European Patent Application EP 4 678 733 A1 - sequence listing, part 3

SEQ ID NO: 4 - DNA, 5305463 bp, Variovorax sp. (residues 3,536,977-5,305,463 of 5,305,463)
  source 1..5305463: mol_type = genomic DNA
  gene 3283935..3288059: gene = rpoB; note = CDS of the gene; part of the gene of SEQ ID NO:3; note (original language) = CDS del gen; parte del gen de SEQ ID NO:3
  gene 2014365..2015895: note = From 2014425 to 2015865: Complementary fragment to SEQ ID NO:1; note (original language) = De 2014425 a 2015865: Fragmento complementario a SEQ ID NO:1; product = 16S ribosomal RNA; product (original language) = ARN ribosómico 16S
  misc_feature 1..5305463: note = Part of the genome (contig); note (original language) = Parte del genoma (cóntigo)
gacaggcagcttcagcatcgaccagggcgtcggcgtgcgtgcggtcagcggcgaaaaaaccgcgtttgcctattcggacgacatttccgaggcgtcgctgctcgatgccgcgcgcaccgtgcgctccatttcttccgcgggccgcaccggccgggtgaagacggccacgcgcaagattgcgtcgagccgctcgctctacagcggcatcgaccccatttccacgctcgacagcacggccaaggtcaagctgctcgaaaaggtcgaaaagctcgcccgttcgcgcgatccgcgcgtggcgcaggtcatggcgggcctcgcgagcgagtacgacgtggtgctggtggcacgcgccgacggcacgctggcggccgacgtgcggccgctggtgcgcctgtcggtcaccgtgattgccgagcagaacggccggcgcgaagtcggctcaggcggcgggggcgggcgcttcgggctggcctacttcaccgacgagcagatcgctgaatacgtcgaccatgccgtgaaggccgcgctgaccaacctcgatgcgcgtccggccccggctggcgagatgaccgtcgtgctcggttccggctggcccggcatcctgctgcacgaggccatcggccacggcctggagggcgacttcaaccgcaagggctccagtgcgttctcgggccgcatcggccagcgtgtggcggccaagggcgtgaccgtgctcgacgacggcaccattgccgaccgccgcggttcgctcaatgtcgacgacgaaggcaacgcgagccagcgcaacgtgctcatcgaggacggcattctcaagggctacatccaggattcgctcaacgcgcgcctcatgaaggtcaagcccacgggcaacggccgccgcgagagctacgcccacgtgccgatgccgcgcatgaccaacacctacatgctgggcggcgacaaggacccgaaggaaatcgtcgcgagcatcaagaagggcctctacgccaccaacttcggcggcgggcaggtcgacatcacgagcggcaagttcgtgttctccgcaagcgaagcctactgggtcgagaacggaaagatccagtacccggtgaagggtgcgaccatcgtgggcaacggcccggacgcgctcacccgcgtgacgatgatcggcaacgacatggcgctcgattccggcgtgggcacctgcggcaaggaaggccagagcgtgccggtcggggtgggccagcccaccctgcgcatcgatggtttgaccgtaggcggaacggcctgagcttgctaagctccgctccttatttttacaaagaggagcattcgatgaggatcaggatcaattcgtccgcggccctgtgggccgcgactgctgcagtggcattgctggcaacggccggctgcgcatcgcgcggcggttcgggcaccagccaaccctcggccgcacccgctgccgcgcctgctgcaccggcccgtgcaggggccaaggccggcatggatgcccagggcaacgtgatcgaatcctccaaggtcgaagccggcagcggccgcacggtcaagggcctgaacggctacgaaggcgagatcaccggcaacccgacgcgcaacagcaggttcaaccggctgcagatcggcatgagcgcgaggcaggtcaccgacattgccggccagccgaccgaccagggcggctatgtgacgggcaaggccttcatccccttctatttcggcggcgaccgccaccgctacgagatgacctacaagggccagggccggctggttttcgcgggcggtggcatgggtgactactcgggcggcaacctgatctggatcatccacaaccccaacgaatccggttaccgctgaccttcggaagcccggcttttgccgggcctcctattttccgtgctacatttcgcccacatgtccgccctccgcgcttatttttttgctttcttttggttcccggtttccggcggacgagaggcgagcgcgtaaagcaaacgaacaccctcccaaaaccgccggcgcttccagccccggcggtttttttatgccctgacgatcttcacacccacaaggaaagcaccatgagcacgaacactgccccgaccagcgacagctggtatgcgagcgtcgaaaaaaccagcaagaccgacgacgaacgcatcaaggacatcaacgtgctgccccctcctgaacatctgatccgcttcttcccgattcgcggcacgccggtcgaaacgctgatcgaaggcacgcgccgcaacatccacaacatcatggccggcaaggacgaccggctgctggtgatcatgggaccctgttcgatccacgacccggccgcggcgctcgaatatgcccgccgcctgaaggtcgagcgcgaaaaatacgccggcacgctcgagatcgtgatgcgcgtgtacttcgagaagccgcgcaccacggtcggctggaagggtttgatcaacgatccgtatctcgatgagagctttcgcatcgacgagggcctgcgcatcgcgcgccagctcttgatcgacatcaaccgcctgggcctgccggcgggcagcgagtttctcgacgtgatctcgccgcagtacatcggcgacctgatttcctggggcgccatcggcgcgcgcaccaccgaaagccaggtgcaccgcgaactggcctcgggtctatcggcaccgatcggcttcaagaacggcaccgacggcaacatccgcatcgcgaccgacgccatccaggcggcggcgcgcgggcatcacttcctgtcggtgcacaagaacggccaggtcgcgatcgtgcagaccaacggcaaccgcgactgccacgtgatcctgcgcggcggcaaggcgccgaactacgacgccgcgagtgtcgaggccgcctgcaaggatctcgaggccgccaagctgccgcccacgctgatggtcgattgcagccacgccaacagctccaagcagcaccagaagcagatcgacgtggcgaaggatatcgccgaccagatcgccgggggttcgaaccgcgtcttcggcgtgatggtcgaaagccatctgcaggccggcgcccagaagttctcgccgggcaaggaccagatctcgggcctcgaatacggcaagagcattaccgatgcgtgcatcggctgggacgactccgtgcaggtgctcgacaccctgtcgcaggccgtcaagcagcgcaggggttaattaaacgggggtcaaagcatcccggccagctcgggccagtggtgccgcatggcagtggcttcgtcgctgtcgggcggcaccagggagaagtcggcaaagtcgaagcccggcccgaccatgcaggcgaccagcgtgtagtcgccgctggtgtggccttggatcgggcgggcagcctgccactggccggccggcaccacgtgctggggccgcgtgccgtgcgcatcgaccgggcccagccgcacgtgggccggcacggtgcgcagggcggcgtcgcaggtccagagtgccagcggcacgccttccaggtgcacccagacttcgtccgacagcacccggtgccagcgcgaatgctgccccgcctcgagcagaaagtagatgctggtgagcgcgctgcgcggcgcgcggccatcggtgggaaccacgctcgcggccgagcggaagacctcgctgtaccagccaccttcggggtgaggctgcagcttcaggctctcgatcagttcccgcgcgcgcatggcggtcatgatgccggcgtggcacgcagcgccgcaagcagtttgtcgtgcacgccgccgaagccgccgttgctcatgcagacgatgtggtcgccgggccgggccgcggcgacgatctgcgcgatcagcggctcgatggcgccggccacctgagcgcggtcacccatcggcgcgagcgctgccgcggcgtcccagtcgagccccgccgtgtggcagaacgaccggtcggccgactccaggctccacggcagctgcgcggccatgacacccagcttcatcgtgttgctgcgcggttcgaaggcggcaaggatgcgctcgccttgcttgccggcggcatcgagcttcttgcgcaggccgtcgagcgtggtgcggatggcggtcgggtgatgggcgaaatcgtcatacacggtgatcgcgccgccgctgcgttcgacggtgccgcgcagttccatccggcggcgtacgtttctgaagcttgccagcgcgcgggccgcatcggccggcgccacgcccacgtgctcggcggccgcgatggcggccagcgcgttcatctggttgtgcaggcccgagagttcccactcgacccggctcactgcttcgccattgcgcagcacgtcgaaggcgtcatgcgacccggaagcctgccattcgccgcccgcgccaaaacgcgcgagcccgctccagcagccttgcgccagtacgcgctgcaggctttcttcggtcgcgttcaccaccagccggccggtgccgggcaccgtccgcacgagatggtggaactgtcgctcgatggcggcaaggtcgtcgaagatgtccgcgtggtcgaactcgaggttgttgagaatcgcggtgcgcgggcggtaatgcacgaacttgcttcgcttgtcgaagaaggcggtgtcgtattcatcggcctcgatgacgaaggccgggccgtcgccgaggcgtgccgagacgccgaaatcgagcgggaccccgcccacgaggaagcccggcgccttgccgcccttttcgagcacccaggccagcatcgacgtggtggtcgtcttgccgtgggtgccggctacggccagcacgtggcggcccagcagcacgtgctcggccagccactgcggaccactggtgtagggcttgccggcatcgaggatggcttccatcagcggaaacttgggcgtgccgtcgggaagccgggccctcgacaccacgttgccgaccacgaacatgtcgggcgaaagtgcgagctggtcggctgcaaagccttcgatcaggtcgatgccgagcgagcgaagctggtcgctcatgggcgggtacacgccggcgtcgcagccggtgacccggtggcctgcttcgcgcgccagggcggccaatccgcccatgaacgtgccgcagatgccaagaatatgaatgtgcatcaggtgattctagggaggccgcatgcaccgcctcggcctgcggcctggcctttgtaccgatgttcgtgtgaagcgcgccatctgcgggcaaaatgtgtcgatggacacgtccaagcgtgagattgccgctgcagcagcccgcctcgtggtcgaagaggggctggagtacggcccggccaagcgcagggcgctgcgcgacctgggcctgtcgtcacgcacttcgctgcccaacaacgacgaggtcgaggccgaggtccgcgattacatcgcgctctactgcgccgacacccagccgcaagaactgcatgccttgcggctgctcgcgctcgaatggatggagcgcatggccgcgttccgtccgcatattggaggcgccgtctggcacggtaccgccacgcgtctgtcagacatttatattcaattgttctgcgatgattccaagtccgccgaaattgcactgatcgaccatcacgtggactacgagccgcggatggtgaccggttttcatggcgaacaggtggaggcgctcagcgtgcacgccgcgagccgtgcgctgggtgaggagatcggggtgcacctgctggtgtacgacctcgacgatctgcgcggagcgcttcggcccgacgcccagggccgcgtgccgcgtggcgacctggctgcgctgcgccggctgattgaaagagaaaaggacaagtgaatgacttcttcgcccacacggcgccgccttctttacggcggcgtggcggttgcggccgcagcggcgggcctgggcggcgcgtggtggcgtgagcgcggcagcggcgcgaagggcgaagccctcgacgccgctttctggacccagcgtttcgagcgtcccgagggcggcgaactggtgtttgccgatctgcgcggcaagccgctcctgcttaatttttgggcaacgtggtgtcctccctgtgtggaggaaatgccgatgatcgaccgcttctttcgcgaaaatggcgcgaacggctggcaagttgttggcttggcaatcgatcaaccgagcgctgtccgcaagtttctccagaagatgccagtcagctatcccaccggattggctggcctgcagggaaccgaactggtaaaaagcctcggaaatacggccggcggtttgcccttcacgctggttctcggcagtgatggaaccgtggcggctcgtaaaatgggcaagctcgaatccgctgacttggatgcttggcggcgtgaactggttcacggttagaatcagatacacctcggcattcgccgccaatcgctaaaaatcaccgatttttagcccagttacatcctaatgaccggcaaagtcggcactggagcctcatggatctgcgcaaactcaagacactgatcgatttggtgtcggaatccaatatttccgaactggaaatcaccgaaactgaaggcaaggttcgcatcgtcaagggcggcggtgccgcccccgtgcagtatgtgcaaaccgtggcggcagcaccggcagcggcccccgcggcaggcgctccggcggtgcccgcgattgccagcgcgccggcgcccgaagccgcgcctgcaggccacgcggtcaagtcgccgatggtcggtaccttctaccgctcgtccagcccgggcgctccggctttcgtcgagatcggcagcaaggtcaacgagggcgacaccatctgcatcatcgaagcgatgaagatcctcaacgaaatcgaagccgacaagtccggcacgatcacccagatcctcggcgaaaacggtcaggcggttgaatacggccagccgctgttcatcatcgagtgaccatgttcaagaagatcctggttgcaaaccggggggaaattgccctccggatccagcgcgcctgcagtgagctcggcatcaaggccgtgatggtctattcggaagccgatcgcgacgcgaagtacgtcaagctcgcgcaggaggccgtttgcatcggcccggcgccgtcgtcgctcagctatctcaacatgccggcgatcatctcggcggccgaagtgaccgacgccgaggccatccaccccggctacggcttcctgagcgaaaacgccaacttcgccgagcgggtggagcagagcggtttccagttcatcggcccgacgcctgaaaacatccgtgtcatgggtgacaaggtctcggccaagcaggccatgatcaaggccggcgtgccatgcgtgccgggctccgagggcgagctctcggacgacgccaccaccaacaagcgcattgcccgcgccatcggctatccggtcatcatcaaggcggccggcggcggcggtggccgcggcatgcgtgtggtgcacaccgaagcggcgctgatcaacgcgatccagatgaccaaggcggaagctggcgctgcattcagcaatccggccgtgtacatggagaaatttctccagaacccccgccacgtcgagatccagatcctcgccgacaagcacaagaatgcggtctacctgggcgagcgcgattgctccatgcagcgccgccaccagaaggtcatcgaggaatcgccggcgcccggcattccgcgcaagctgatcgagaagatcggtgagcgttgcgccgcggcctgcaagaagatcggctatcgcggcgccggcaccttcgagttcctctacgaaaacggcgagttctatttcatcgaaatgaacacgcgcgtgcaggtggagcacccggtgaccgagttcaccaccggcatcgacatcgtgaagacgcagatcatggtggcggcgggcgagaagctgccgttcacgcagcgccagatcgagatgcgcggccacgccatcgagtgccgcatcaacgccgaagacgcctggaagttcaccccgtcgccgggccgcatcaccatgtggcacccgccgggcggccctggcgtgcgcgtcgattcgcatgcgtacaccaactacttcgtgccgccgaactacgactcgatgatcggcaagatcatcgtctacggcgacacgcgcgagcaggccatggcccgcatgcgcacggcgctgaacgagaccgtgatcgaaggcattcagaccaacatcccgctgcaccgcgagctgatggtcgacgccaagttcatgagcggcggcaccaacatccactatctggaagagtggctggcggcgcacaagcgctgaatggcaccacggcatgtttgaactacgcctcatggcgccggaagaccgggtcgagatgctcggcgatgcgctcgacgcgctcgatgcgctgagcgtgtcggtcgaagacgccgacgcccagaccgatgccgagcaggcgttgttcggcgagcccggcatgccgccgcccaaggaaggctggcagcgctcgcgcgtgatcgcgctgtttgccgacgaagcgcttgccaaagaggctgcgtcggtgctcgcgctgcaggatttcttcgaaggctgccaggtgctcggcgtggcgtcggtgcccgagcaagactgggtgcggctcacgcaatcgcagtttgcgccggtcgagatcacgcccgagttctggatcgtccctacgtggcacgagccgcccgaacaggcaaagcaggtgatccgcctggacccggggcttgccttcggtaccggcacgcaccccaccacgcgcatgtgcctgcgctggatcgccaagcagggcgcgtttgccggccagcgcgtgctcgactacggctgcggctccggcatcctcgcgattggcgcggcgaagttcggtgcgcccgacatcgacgccgtcgacatcgacgaagcggccgtttcgtcgacccgcctcaacgccgaagccaacggcgtgcgcctgaacgccggcctgcctgaagcagccaagggccagtacggcacggtgctggccaacatcctggccacgccgctcaaggtgcttgcgccacttttgtgcagccacgtggcgcccggtggatcgctggtgctggccggcatcctcgagcgccaggccgacgagctgaagcaggcctatgcgccgtatgcagcgctcgaagtcagcgacagcgaggacggctggatcctcatgacggcgcgctgctgaggacgcagcgagccgttcgtgtcgccctgattcccctggcgcggcgagggcccaaccctacaatcgcccggtcatgagccttgtcacgcgctgccccgcctgcaccaccaccttcaaggtggttcgcgaccagctccgcatctcggatggctgggtgcgttgcggccggtgcagccacgtgttcgacgccacgctcgatctgcacgaggcacccgacgccaccccggtggccggcgcggcttcgctgccgccatcgtcggcgcctgctgccaaacccgagccactcgagcggccttccgaggagtcccggcgcgcagtcgaagacgcggacttctttgacgacgagcccgagcgtggcgaggcattgggagcttccgccccggtgccgcccggcgagcagatcgaggcgccatcggcggcgccggtgtccgagtccgaatcatcgccggctccagcgcccgcatccgcttcggcttccgcgttggcctctgcctcggtcctgccggcacacggcatcgtcgcggacgagctgtggtccgacttcgaagccaacgagcccgagtggcgtcctccgcccagctcgctgccgccgtttccgaacatcgacctgaatcttggggctcctccctcgcccccgccgcctccgtcgccgcccttgccggccctgcgcctcaaggcccgcgagctggtggcctcggccagcgacgagaacgagaagcacgaacctgcgctggaccgcgaccaggtgcagatgcagaaggcgctgcgccgggcgcgcatcaagtccgccaagatcgccggcgccaaggcgcgggacgagcgcgccgccgccaaggcatcggcctcgatggtgcgcgaggcgagcgagcccgacccggtcctcttgccgctcccatcgctgcgcgacgacgcagaagaagattccgaacggcttccgctcttcggcggcgaggagccgggtcgcgatgccacgggtttctggcagcgcagcgcggtgcggcgttggctctggcttcttgcggtgcttgccgtcctgctgtttgccgtccaggtcttgcggcacgagcgcgacggcatcgtggcccgccagccgaaccttcgtccggcgcttgccgcgctgtgcggttttaccggctgcgagctcacggcattgcgccagatcggcgacgtcgtgatcgagggcgccgccttcgcgcgcgagaagaccggcaacaacgactaccggctgagcttcaccctgcgcaacggcgccacggttccgctggccatgccggcggtcgagctttcgctgctcgactcgcaggagcgcgccgtgctgcgccgcgtgttgacggccacggactatggcgcgccggcggtgcttccgccgcgcgccgagcaggccgcgtcgctgccgctggccttgtccgccacggaggcggcaacgctgccgcccattgccggctaccgcgtcgaagcgttctatccttgagccgggctcgcgttcgccccgctcttttttcatcccttcccaaccaacggttcacccatggcagcagtgatttgcggttccctcgcgttcgacaccatcatgactttcgagggccggttcgccgaccagatccttccggaccagctgcacatcctcaatgtgtcgttcctggtgccgggcctgcggcgtgacttcggcggctgcgccggcaacattgcctacagcctgaacgcgctgggcggcacggcactgccgatggccacgctcggcagcgatggggccgactacctggagcgcatgcgcgggctgggcatcagcaccgagttcgtgcgccagctggacgacaccttcacggcgcaggcgatgatcatgaatgacgtcgacaacaaccagatcaccgcgttccaccccggcgcgatgcagcaggcgcacctcaccaagatcgccgcccgagaagacatccgcgtcggcatcatcgcgcccgacggccgcgaggcgatgctgcagcacgcagaacagttcgccgccgccggcatcccgttcgtgttcgacccgggccagggcctgccgatgttcgatggcgaggcgctgaagcatttcgtcgagctggcgagctgggtcgtcgtcaacgactacgaaggaaagatgctgtcgcagcgcaccggctggagcctggccgagatttcgaagcgcgtgcgcggcctggtggtcacgctggcgggcgaggggtgcgaggtctggaccgacggcgaacgcgagcatgtgccgggcgtgacgcccaccgccgtggtcgagcccaccggttgcggcgatgcctggcgtggcgcgctgctgttcggcctggaaaaggaatggccgctcgcacagtgcgcggcattgggcaaccgtatcggcgcgctcaagatcgcgcagcgcgggccgcaaaactaccagatcgacaggcaggcgctcggcctctgagtcgcctctctgttaggcgcccacaaaaaaaaacccgacaccgtgaggtgccgggttttttgccgacaaggccgctgagaagctcagggcttgctggccgtaggaaacggccaggctgcctgcgggttcagcgtcgtttgcgcagcaggagcaggcgctgcggcaggggctgcctttgcagccttcttcgcagcaggcttcttggcagcagcggcaggcttggcagcgggctttttcgcggctttcttggccgcagcctttttggcaggagccttcttggcggcagccttcttcgcaggggccttcttggcagcggccttctttgccggagccttcttcgccgccgccttcttggcaggagccttcttcgccggagccttcttggcagcggccttcttggccggagctgccttcttcgcggctaccttcttcgcaggcgccttcttggcggctaccttcttcgctgcgaccttcttggccggagccttcttcgcagctaccttcttggcgggagccttcttagcggccgcgaccttctttgccggagccttctttgcagcggctttcttagccggcgctttctttgcagttgccatttctatttctccttgatcaagttgaaaaaatcaacctattgaagcactccacgcacgttggtagcgtgaagcgattcatggcgttggaatctgagccccagcaccatgaacacctgagccctcgtccatgccgcgctcttcggcgcgatcggtggcaagggcaattcttgaattcattaattcttgtcggaaagattcaatcccacgagagcgcgccgcccgattggtactcgatcacgcgggtctcgaaaaagttgcgctctttcttcaggtcaatcatctcgctcatccaggggaacgggttttcctcgttcgggaagagcgtttcgaggccgatctgctgtgcccgccgattggcgatgtagcgcaggtagcccttgaacatggaggcgttcatgccgagcacaccacgcggcatggtgtcttcggcgtatttgtactcgagctcgacggccttcatgaagagggccttgatctccgccttgaactcgttggtccagaggccggggttctcgagcttgagctggttgatcaggtcgatgccgaaattgcagtgcatcgattcgtcgcgcaggatgtactggtactgctcggcggcgccggtcatcttgttctggcggcccagcgcgaggatctgcgtgaagccgacgtagaagaagaggccctccatcaggcaggcgaacacgatcagcgacttgagcagcgtctggtcggtttcgtgcgtgccggtcttgaagtgggggtcgctgatggcgtcgatgaacgggatcaggaactggtccttctcgcggatcgacggcacttcgttgtaggcgttgaagatctcgctctcgtccaggccgagcgactcgacgatgtactggtatgcgtgcgtgtggatcgcttcttcgaatgcctggcgcagcaggaactggcggcattcgggcgccgtgatgtggcggtaggtgcccagcacgatgttgttggcggccagcgagtcggcggtcacgaagaagccgaggttgcgcttgacgatgcggcgctcgtcttcggtcaggccgttcgggtctttccacaacgcgatgtcgcgcgtcatgttcacctcttgcggcatccagtggttggcgcaggtggccaggtacttttcccaggcccacttgtacttgaacggcaccagctggttgacgtcggtctggccgttgatgatgcgcttgtcggaagccttgacgcgctgcgcagcgacgggggctgcggtgggctgctgtgcaatcgacgaagtcggagcgtccaccggtcggcctgcggtcatgccgctggtcgatgcgtggtgttgctgcaatccttgttgcatatcctttgataaggagggcttgacttcttcgtcccaggtcaacatagaaaaatccaatgctcgattatcggagcaacgatgtgagttgcaaagtgctcgttcacatcgcgctccatttatgtggttgttatgttgctctcatgcatcgcgcgatgtcagtcgatgccgtgatcgactgagagttcgcgcgtcgtgcatgcacctctctctgacttcactgacgcgtcattggcatgcttcgcaagtcggatcgtcgacgccgcagaacgcgatgtcggtcgcaggcatcgcactcatctgcgcctttgctgcggctgctgcggcttcgagcgcgctcatgcccgaggatgcatcgctgcccgacgacaccgcgttgaggcggcccgattgcacggtcgacttttcggcgtgcgtcgcgctctgtgtgcgcaggtagtaggtcgtcttcaggccgcgcagccatgcgagcttgtaggtgtcgtcgagcttcttgcccgatgcgccggccatgtagatgttgagcgactgcgcctggtcgatccacttctggcgacgcgaggcggcttcgaccagccacgtggtctcgacttcgaacgcggtggcgtagagcgccttcacgtcttgcggcacgcggtcgatcgggcgcagcgaaccgtcgaagtgcttcaggtccatgaccatcacgtcgtcccacaggcccaggcgcttcaggtcgcgcaccaggtagtggttgatcacggtgaattcgcccgacaggttcgacttgaccgagaggttgccgaagcagggctcgatggacgcgtcgacgccgatgatgttggagatggtcgcggtcggtgcgatggccacgcagttggagttacgcatgccgtcggccttgatcttctggcgcagcgcgtcccagtcgagcgtggacgagcggtcgacctcgacgtagccaccgcgggcctgctcgagcaggtcgagcgtgtcgatcggaagaatccccttgtcccacagcgagcccttgtagctcgagtacttgccgcgttcgcgggccaggtcggtcgatgcccagtaggcgtggtagcagatggcttccatcgactcgtcggcgaactgcacggcttcctgcgaggcgtagggaatgcgcagttcgtacagcgcgtcctggaagcccatcaggccgaggcccaccggacggtggcgcaggttcgagtcgcgcgccttcttcacggcgtagtagttgatgtcgatcacgttgtcgagcatgcgcatcgcggtcgagatcgtccgcttgagcttctcctggtcgaccttgccgtccttcagatgctgcagcaggttcaccgaacccaggttgcagacggcggtttcggtgtcgctggtgttcagcgtgatctcggtgcacaggttcgacgagtgaaccacgccggcgtgctgctgcggcgagcgcacattgcaggcatccttgaaggtgatccagggatggccggtctcgaacagcatcgtgagcatcttgcgccagaggtccgacgcctggatggtgcgggcgggcttgatctcgccgcgcgcggccttttcttcataggccacgtaggccttctcgaagtcggcgccgaacaggtcgtgcaggtcgggcacgttcgagggcgagaacagcgtccaggtgcccttttccatcacgcggcgcatgaacaggtcggggatccagttggccgtgttcatgtcgtgcgtgcggcggcggtcgtcgccggtgttcttgcgcagctccaggaactcctcgatgtcgaggtgccaggtttccaggtaggtgcagaccgcgcccttgcgcttgccgccctggttcacggccacagccgtgtcgttcaccaccttcaggaacggcaccacaccctgcgattcgccgttggtgcccttgatgtggctgccgagcgcgcgcacgcgggtccagtcgttgcccaggccgccagcgaacttcgacagcagcgcgttttccttgatcgactcgtagatgccgtccaggtcgtcgggcacggtggtcaggtagcagctggacagctgcgagcgcagcgtgccggcattgaacagcgtgggcgtgctcgacatgaagtcgaaggacgacagcacttcgtagaactcgatggcgcgggcttcgcggtcgatttcgccgagcgagaggcccatggccacgcgcatgaagaaggcctgcggcagctcgatgcggttcttgcgcacgtgcaggaagtagcggtcgtacagcgtctgcaggccgaggtagtcgaactggttgtcgcgctcggccttgagcgcggcgcccaggcggggcaggtcgtactgcagcagcttttcgtcgagcagctcgttctcgacgcccttcttgatgaactgcgggaagtaatcggcgtaggtctgcgcacgctcggtgggcatgacttcgcggccgatgatctccttgaagatcgtgtgcagcagcaggcgggcggtcgcgaaggtgtagtcgggatccttctcgatcagcgtgcgggcggccaggatcgaggccttgtagacctcgtcgagcggcacgccgtcatacaggttgcgcatcgtctcggcgacgatcggcgcggcggtgatgccgtcgccgaggccctcgcaggccgattcgatcaggcccttgagttcgttcaggtcgagcgcgacgcgttcgccgccgtccagcacgtgcagcagcggcgtggccggcgcttcctgcgcgacctgcttggagcgctcttgcgtgcggcgttcacggtacagcacataggcgcgcgcgatttcgtggtggccgccgcgcatcaggccgagttcgacctggtcctgcacgtcttcgatgtggaaggtgccgccgcccggacgcgagcggaccatggcgcggatcacgccttgcgtgagtgcgtcgaccgtctcgcgcacgctggctgaagccgcgccctgggtgccgtgcaccgccaggaaggctttcatcatggcgatggcgatcttgttgggttcgaagggaaccacggcgccgttgcggcgaatgatctggtagttcgcgaggttctgggcggtggtggagcccgcggtgtcgcgttgctgggacggcgtggagggaacggcacgcggggtcgatggggtgttcagggcagtttgcattcgcttcctctcggttggcaattcttgttgggtggcagcgccttggtcgggcgttgcgccggcgttgttggccggacggaggacactatatctagggtgtagagggtctacaagccactacaggtagtgttttgtggaagtttaacccctacgggtatttctctaggattcggcatacggccatcggtgccgcgtgaatactggcttatggtcgcgcaggccgcatggggcgtggcctgccggacgatttgggcctgcaaggcgcatggttgctacgctgcgcgtcggcgtttgagaaacggagtcgacgcaagcacagcgcatcgcagggcgccgcgcgattaaaaaaattaacgcgggaccgcctgctcgggaaacatttgcaagtcccagccgagttgtccgcgcagcaactgccagtcgaagcccgcgccagggtcttgcttgcgacccggtgcgatgtgctcgtggccggcgatgtgggcaatggcgtagtgctgcgcgatggcggcacagaggctggccagcgtttcgtattgcgcctcttcgaaacgttcgccttccaggccttcgagttcgatgccgatcgaatcgtcgttgcagttctggcggccgcgccacgacgacgcaccggcgtgccaggcacggtcgtcgcagctcacgaactgccagagctcgccattgcgccgcacgtagaaatgcgaggaaacctcgaggccgcggatggattggaagtaggggtgcgcgtcccagtcgagctggttggcaaaaagctgttgcaccgcatcgccgccgtattcgccgggcggcaggctgatcgaatgcagcacgatcagatcggtctgcgcgcccgcgggccgcggaccgaaattcggcgagcgcagcgccttggcgaagcgataccagccggcgtgccagaggccgtcgccgtggctgcccgcgctggccggtgcgtcagtcgtcggcatggctggcggcaccttcgtcgccgttgggcgtggtgatgcccagccgcgcgatgcggtagcggatctggcgcaggctcatgccgagccgcgccgcggccgccgtgcggttgaagccgctttcgcgcagcgcgcgcacgagaatctcgcgctcctgctggtcgaggtaggcctgcaggtcggagggaagggcggcgggcctggactccgcaaccgcgcttgcggccgtagcgggtgcgggaggggattcgccgtcggccgccagcgaagaagacaggggcgaaggcgcggttgccgcaccggtcgaatcggccggcgccgcggcaggctgtcctcccgccgtcaggtcgaggtgcagttcgtcgccgtcgttcagcgccacggcgcgatgcagcaggttctcgagttcgcgcacgttgccgtcgagcggatgctgtgccaggcggcgcagcagatcggcggacaggtggggcaccggcaagccgccgtcctgcgcaatgcgcgcgagcagcgcggcgcaaagcgcgggcaggtcttcgcgccggtcgcgcagcgcgggcaccgcaatctcgatcacgttgagccggtagaacaggtcttgccggaagcggccggcctggactcccgcatgcagatccttgtgcgtggcactcacgatgcgcacgtcgaccgcgtcttcctgcgtggaaccgatcgagcgcacgctgcgctcctggatggcgcgcagcagcttggactgcattgcgagcggcaggtcgccgatctcgtcgaggaacagcgtgccgccgcgcgcggcctggaagtagccgtcgcggtcttgcgacgatccggtgtaggagcccttgcgggcgccgaagaattcggcctcgagcaggttctcgggaatggcgccgcagttgaccgcgacgaagggaccttcgctgcgctggctgcaggcgtgcacggcgcgcgccaccagttccttgccggtgcccgattcgccgcgcaccagcaccggtgccatgccgcgcgccaccttggcgatgcgcgacttgacgagccgcatcggctccgagtcgcccaccagccgttggagcgccgcgatgccgctgcccggaatggcgggcgcatcggtgcgttcgcccgtttccgcgggcgcggcccgcaccgccttggtgggcaacgcctgctgcgcctgcacggcggaggcgaccaccgcgcggaactgcttgagatcgaccggcttggtcaggtagtcgaacgcgccggccttcaatgcctcgaccgcgttctcggcggagccataggccgtcatcacgacgcaacgctcgctgcgctggttcttctggatgcgatggatgatttccatgccctgcccatcgggcagccgcatgtcggtgatcaccgcatcgaaatgcgcagcctcgagatgctgccaggcttcggagacgctcccggcggcctcgacgcgatagccttcgcgcagcaacgtcagctcgtacagcgtgcgcaggtcgggttcgtcgtcgatgaccaggatgttggccggacgctgcagggaaggaggaggagtgctcacggcgctattgtgtcagccggttttcgcttggcgcaaagctgacgaagaattcgttgccttcaggcccgcccgcgacgagcgcgcgccgttcgtagccgatggtggcgccatggcgccggcacagctcgcggcacaggaagaggccgagcccgctggagcggctctcggatgagaagaaaggttcaaacaggtggcgttgcaccgccggctccagcggcgcgccgtcgctccaaacttgcaggctgggtcggctggagctgccgcgctgcatggtggtgacgacctggatcgagccttcccggttgccggcgtagcgcgccgcgttgtccagcaggttcacgagcaggcggcgcaggtgctcgacgtcgaagcgcacttcgctgtcggcggcatcgagcgtgatcagcacgccctggcggtgcgtctggcgcacccattcttcggccagcgcgcgcaccgcagggtcgagcgcgacctgctcgccgagcgagagcacgcgctgctggcgcgcgcgcgaaacatcgagcacgtcgtccacgatgcgagcgagccgctgcgcgttgtgctggaccatgctggtcaacttgcggtgcgcgggatcagtgaggtcttcgttgagcagggcactggcctgcgtgatcgcggccagcgggttgcgtatttcatgcgccaccgcggccgacatgcggcccatcgcggcgagcttttcggtgcggatgcgggcctccagttcgcgcaggtcctgcaggaacatcacgcacaggctgtcgacgcgctggtcgctggtgggcgtgagccgcgtgcgcacccgcacttcgcgcgcggcgccgcgggcttgcgccacggggatttcttcgctttgcggggcgcggcgcgcaaaggtctggcgcgccaacgccgccagtgcgtgccaggccggctgcgcatgcagtgcaaacgggagggcgagccgggccaggccttgtccgaggatggcgtcggccgccggattggccgcatgcaccatgccctcggcgtcgatcaccagcacgccttcgctcagtgtctcgatcaccaggtcgttgacctgcgcctgcatctgcgcgctgctgcggttgcgcagcgcggtttcttcttcgcgcgcgagccggcgcgccaactcgtgcgccagcagggccacgacgaaaaggccggtgccggtcagcgccgcctgcacgaagcgggtggaggaatcgccgggctgctgcagccagtgccagcccgcgtcggccagcagcagcagggtgaccgtggccgtggtgcccaggcccacggtcaccgtgccgagcaccgcgctcatgagcaccggcagcgcgaacagcggcgtgtagttgatgttgccgccctggagcacctggagcgcggtgaaggtgccgaggtcgatgccgatggtgatgaaccacagcgccgcgaagccccggatcggtggcgcgaaatgcgcgtagcgggcgcccagccaggtggcgatcaggtagccggccgaaagcgcgatggccaacggttgcatcgtctggccgagcgccagtgccacgccctgtagcagtacgagcaccactgcaacgaagcagcgcgccgccatgaagccgcgccacaagcgcagcagcgcggcgctctcgctgcgccccggctcgagcaagtcccagtcggtggcggcctcgccttgcggccagagggaagaactcatggaggcgcggcgctcgttcagccgcgctcggcggcctggcggtgcgccgcactgcagtagaccgcgtcgcctgggcccccgatcgcgtcgctcgcgggcaggtgcaaaccgcaatgggcacagcgcagcatggcctgcggagccgccggtgcggcaggcggccgctgggcgcgggccgcctcctgctcgcgctgggcctcgcgcatttcctcccggcggttcttgcgccagagccagatggccacccagagcaccgccaaaacgagcaggtacttcatgatgtgccgcgcgccagcaccacttcgagcacgaagcgcgagcccacgtaggccagcagcaacaggacggagccggcgtagagcacgcgccgcgccgtgcggccgcgccagccgaagcgcacgcggccgatcagcagcaccgcaaagctgatccaggcgagcaccgagaacaccgtcttgtggtcccacttccacccgcggaacgacgcgccatacagcgtttcgctgaacagcaagcctgcgagcagcgtggccgaaagcagcacgaagccggccatcacgaagcggaaggtgagccgctcgagcgtgagcagcggcaggcccgcctgcggctcggtggccaggcggatctgcttttcggcccgcgtgatcagccacgcatggaccacggcggcgccgaacaagccataggacgcaatgccgagcgcaaggtgcagcggcagccagggcgatgccgagacgtgcagcggcgtgcctggaaacagcacgccgagcaatacggccgccgcccccagcccggccagcgcgcggcggaccttcatctgcgggtacatgctgctttcgaccgcatagacggtgagcaccagccaggcggtaacagagagcgcgggcgcaaagccgaagtggggctggctgccgaccaggccgtggcccagcaccgcggcatgcagcagccacgccagcccgagggcccattgggtggtttttcggctcagccgggcacctgcggcagcggcaaacccgtaggcagccgcggtggcgatgcccagcgccaccgcgagtggggaggggatcgctaaaatcatcgctagagtttatctcccccaggcgtgcgcactttcctcgtgccgcagtaaccggccgatctccagtttccgactttccattgacccgccgcggcgggcagcaaggcatccctttcatggccaccgccctcacagaaaagttctcccgcctcgtcaagacgatgagcggccaggcgcgcatcaccgaaagcaacgtgcaggacatgctgcgcgaagtgcgcatggcgctgctcgaggccgacgtggcgctgcccgtggtgcgcgacttcgtggcgcgcgtcaaggaaaagtcgctcggtcaggaagtgctgggctcgctcaagccgggccaggcgctcgtcggcatcgtgaaccgcgaactcgccgccaccatgggcgagggcgtgtcggacatcaaccttgcagcccagccgcccgcggtgatcctgatggccggcctgcagggcgcgggcaagaccaccaccaccgccaagctggccaagcacctgatcgagaagcgcaagaagaaagtgctcaccgtgtccggcgacgtctaccgtcccgccgccatcgagcagctcaagatggtcacgaagcaggccggtgccgaatggttcccgagcacgccggaccagaagccgctcgacatcgcgcgcgccgcgctcgaccatgccaagcgccatttctttgacgtgctgctggtcgacacggcaggccgcctggcgatcgacgaagtgctgatgaccgagatcaagcagctgcatggcgcgctcgatccggtcgaaaccctgttcgtggtcgacgcgatgcagggccaggatgcgatcaacaccgccaaggccttcaaggacgcgctgcccctcaccggcatcatcctgaccaagaccgacggcgattcgcgcggtggcgcggcgctgtcggtgcggcaggtgacgggcgtgccgatcaagtttgccggcaccagcgagaagatcgacggcctcgaggtgttcgacgccgaacgccatgcgggccgcatcctgggcatgggcgacatcgtcgcgctggtggagcaggtcacggccggcgtcgacgtggcggcggcgcagaagctcgcggccaaggtcaagagcggcgccggcttcgacctgaacgacttcctcggccagctgcagcagatgaagcagatgggcggcctctcgagcctgatggacaagctgccgcagcagatggccgccaaggccacggaggccgacatgacccgtgccgagcgcgacatccgccgcaaggaagggatcatccagagcatgacgccgctcgagcgccgcaagcccgagttgctcaaggccacgcgcaagcgccgcatcgcggccggcgcaggcgtgcaggttcaggaagtgaaccgcctgctcaacgagttcgagcagatgcagggcatgatgaagaagatgaagggcggcggcctcatgaagatgatgaagcgcatgggcggcatgaaggggatgggcgggatgggcggcccgggcggtccgaagctgccgttctgagtctccgcacacacatatatatagacagaagcccgccggggcatgccacggcgggcttcgtcgctttcaggtctgcacttcgtagaccatgtcgtgtgcctcgatcggcgccggcagctcccagcgatgcagcatccgctcgatgcccgcgttcgagagcgtcgtgtcgcgctcgcggttgcggcgcatcagttccgggtgcggcacctccaggtacaccagctcgatctgcgcgtggtacgcccagagcaggtccagcgtcttggtgcgcatctgctggctcaggtgcgtggcattccagacgaagcgctcgtgcttgcgcagcagcgccttggcctgatcgacggcatggtgcgcggccatgccatcgttttcgccatgcttgaggcccaactcggcacgcgcatcgtcgaaggacacgaccggccagcccttgcggtgctgcgccacccagtggttcttgccgctcgcgggcaggccgcacatcaccgtgacctgcgcgcccggctgctggaacagtgggtagtcggggctggtgtcggcgccgcggaaataggcaaggcgcgtgtgtgcatcggccatcttgcgcgggccgttccagcagccttcttcctgcgccagttgctcgaagagcgcgatgtcggccaggctgtcggcgcgcttttcatagtggcgcccgagcatgtcgcagcgcgccacgcagcacaggtcgggcagactcagctcccacgagagcctgtgcaccagccattcgggccgctcgcccttgcgcgaggcgaaggcgtggaacggcacctggtgcaccgcgatgatccggcacacggcttcgcgcagcgcgaacggcacgcgggccttccacatcagcacgcgcacgtcgactgcaccgcggcgcgaatggccgggctggccgatgcggccgctggcttcgtcgatcacggtggtgtcgggcttggcgatgtcgtgcagcaggcaggccatgaagagcacgaagcggccgtcggcgtcggcgcgctggaagtgcgcgtctgccgtcagcgcatcgagcaccatgcgcgtgtgaatgccgacgttgccttcggcgtggtagtacgggtcttgcggcgtctcttcgaggcgcagcagggccggcagcaggtcgcagcactgggcccagtcatagccctgcgtgcgcatggggaccagcgcgcgcagatcgtcgtaggtcatcgcggcctccttgtcgttgttgtcagatcgatggggtcgcgcagcgtgcgcagccccaggtcttgccagcgcacttgcggcgccggtgcatagagatccgcgcccggcgcgagctggttgggcagtaccggccggcggctgtggtgcgagcccgagtcgaggatggtctgaacgaaatccggacgcacccacttgtagcggccggtcacctggccgtgcgactcagtcttgaggtacaggccctcggccaggtcggacaggtcggtctgttgccgcaccaggtcgagcggctggccttcctgcgtcacggcttgttcgaaagcctccttccagccagcgctgcgcgcgagcgacggttgcacgagcgagcgcaatgctttcgcgtggcgcggcatctcgccgtcgtagagcaccggaactgaaaggaccgggctgccctcgagcagcgcatgccgcgccggcgtcgacaggaagcactgtgcctgccggtcgtagaggtcgaactccagaaagaacgcgggcagccggtcgtaccagcagctgtgcttcgcaaagcaccactcgccgtacatcacgtagcggtcttcgagccgctccagcagcaccgcttcatgcgcggctgcccagtgcttgaacaggttgaactggcgctcgccggcgccgcccgcaaggtagtggccgcgtgactgcagcagcagttcgcccgccgaggtgaacgacaccgccgcgttggcgccatcgagcttttcctcgatgaccacgtgctggccgtgcagcgcggacaacggcgtctggccgtcgtcggtatcgccggcctgcaggcgcgagccttccagatgcgcggtacgggggtacttgagcagcggaatcgatgagagagaagagagagggaacacgttgttctccagatgcaaatcaggaagaaccgacaacgtgcgggagcgaagctggaaagagggtcgacttcagcggccggtgggccgtgcctggtcagcgggatgcgcagcttggcgcccgacatgaccagtgaagtggtgttgtcggcgtcagaaggtggtgacggcgaatcggggcacttggcgctccaggggatcgagggatccgtgggttgaaaaagaaaggcgcgattctagccacgcgccatgaaaaaagccgaccctgaggtcggctttttgcgagcttgtgtcttcagcgcatcaggcagtcgccagcgccgcggggcgcgccaggcgcagcgcatgcatccaggcgcggcgcagcacggccggcgaacgcgattcctcgggaatcagcagatagccgcggtcgcgcagcgacgtgcccagtgcgatctggctggtcagcaccgtgagcggaatggccagcagcagcggcaggcccaccggcatgagccagatcagcgcgctcggatcgatcattgcgacgccgagagccagcgcgccgaccaccaggctcatgggagcgagctgcgacatggcgaccttccacggcaccgcagcggcttcgcgcgggggcgacttccagtcgagcttgatgccggtgagggcgaccagcacgaacagcgagtgggccagcatgcgaaccggcgcctgcacgatggccaggccgctttcgagcgccgagctcttcaccaggccccacaagccgccgtactggcgttgctcgccgcgcatcagcacggcagcgatgccgagcacgcggggcaggaacaagaggcacagggtccagacccacaggccggccagttccgccggcagcacgctccagctggagatcaggctcgagccgctcagccacagcgcggtgccgagcgtcaggaacgcgagccacagcggtgccgagacgtacgccatggtgccggtcacgaacatcgcacggtgcaccgggtggatgccgggctcggccatcaggcgggcgttctgcaggttgccctggcaccagcggcggtcgcgctgcagttcggccagcaggtctggcggttgctgttcgtagctgccgaccaggtcggcgcagagccacacgttgtagccggcacggcgcatcagcgcggcttcgacgaagtcgtgcgacatgatgccgcccgacatgccgccggtgcccttgatgggagccagtgcgcaatgcttcatgaagggctcgacgcggatgatcgcgttgtggccccagtagtgcgattcgcccagttgccagaactgcatgcccagcgtgaacaggcggcccgtcacgcgggaagcgaattgctgtgcgcgggcatgcagcgtcacgtggccgatggcctgcgtggcggtctggatgatgccggcggtcggattggcttccatcagcttgaccatcgaggtcaggcagtcgccgctcatcacggagtcggcgtcgagcacgaccatgtagcggtagtccttgccccagcggcggcagaagtcggccacgttgccggccttgcggtgcgtgcggcgggtgcgcaggcggtagtagacctcgacctgcggctggttcgggctgtcggccagcgcggcgcgcaggtcttcccaggcggcgcgctcggcggcggcggtttcggggttgtagctgtcggacagcacgaacacgtcgaactgcctggcgtggccggtggtcgcaaccgattcgcaagtggcgcgcaggccggcgaacaccgtggcaacgtcttcgttgcagatcggcatgatgatcgcggtgcgtgcttcggggttcatcgggtggtgggccacctgcttgaccgagagcgcgtgcttgtcaccgcgcaccgagacgtagaagcccatcagtgcggtgacgaagccggtgacgacccagcccgaaagcagaccgtacaggccgatctggccgtattcgagccagacgttgtcgtagtcgggttgcacgccggcaaacagcgcggacgcgatcacagtgctcagcagcgtgagcgccatgaatgcgaagcggcgctgcgccgcggcacgctgccacggctgcttgatctgtgcgccggcttcggcggtctcggcttccggcttgccgccggcgccgagcttgaccagcacggcggtgcccaggctgttccagaagccgcgccaggggcggggcgccatggagccgcggttgaccggcggagcggtcacggcattgggatggcgttcttcgcgcaccgggctgcggtgcgaaaagtcggcttcggtcagcacgttcagttgggagaagtcgtttggcttcatgtgtgatttaccaacgttgcttgtcgagggaaggggtgtcgccaatggcaggaaagcgcttgatgacgcaatccggttcggcgccgcctgcgcttgcgagtgcggccgccgaatgacccgcggcacggggccgcgagagggaaaactgcttttgacgcaggccgtcgcgctgctggcgcagtgcgaaagatgggctggtgagtgctgtcatgcctgtacaggggcaaaccctgtgccaggctggaaaaatgctttcagatcaatgacttacgtcgatctgaatgcggttttggcggctcgggccgtttggaaggccccgaaacccctgtttttgtcgccgaatcccgacaagcccgggaggctggtggaaaatagcgttttgaatcaacgacttaggggcgtcgctactcggcgacaggctcactgccgggagcgacagcgtcggccttgaagtgccccggcgtgagttcgtgcttctgcagcaggcggtagaactcggtgcggttgcggtccgccagccgggcggcatcggccacgttgccgtcggtcagcttgagcaggccgacgaggtagtcgcgctcgaagcgctgcttggcctcggcataggtctgaacctcgaccgtcggcacgcgcagcgcccgctgcacgagcgccagcggaatcagcggggagctggacagcgcgcagacctgctccaccacgttgtagagctggcgcacgttgccgggccaggccgcggtggccagggccttgagcgcctcgggcgcgaagccggaaagccgcttgccgtatttggtcgacagcttctgcagaaagtggttggccaaaagcggaatgtcttcgcgccgggccgacagcggcggcagcgtgagcgtgaccacgttgagccggtagtagaggtcttcgcgaaactggcccgccgccatggccgcgtccaggtcgcggtgggtggccgagatgatgcgcacgtcgacctcgatcgactgactggcgccaagcggccgcaccgcgcgctcctgcagcacgcgcagcagcttgacctgcagggcaggcggcatgtccccgatttcgtcgagcagcagcgtgccgccgtcggcttgctggaacagccccttgtggttcgcatgcgcgtcggtgaaggcgcccttcatgtggccgaacagttccgattcgagcagcgcctcgggaatggcaccgcaattgacggccacgaagggcttgtcggcgcgggcgctggcgcggtggatggcgcgcgccagcatttccttgccggcgccgctgtcgccgcgcagcagcaccgaggcgtccgacttcgcgaccatgcgggcctcggccagcagctcggacatgcggttgctgcggctcacgatttcggcgcgccagctttcgtcgccggccttggcgggcgtgctggccggtgcgccgagcgccagcgcctgggcgatcttgtccagcagctcgcgcccgtcgtagggcttggtgaggtaggtgaacacgccgcgcgccgtggcctcgaccgcgtcgggaatggtgccgtgggcggtgagcaggatcaccggcagcgaagggtgccgcttcctgatttcgtcgaacagctggagtccgtcgcgcccgggcagccgcacgtcgctgagcaccagctgcggatgctcgatttccaactgcgtgagcgcggtttcggccgaggtcacggccgtgacctggtagcccaccgaactcagccgcatcgagagcagccgcagcatgtctgggtcgtcgtcgaccaccagcaggcgcgcgccggtcgtgctcatcggaggggccctttgcgcgatcgctggatgttcatgggctgggcttggtgctgctgggtggcggaagggtcggcaccggtgcgttgttggggcgggcgaagctgcgctcgatggcgcgcaacgcctcgatgcggtcgttgagctggtcgatgcggcgctggctctcgcgcagctgctgcacctgcttgtcgcgatcgtcctcgacgcggcgctgctccacgtagcgcgcggccagtgcgcgcgcaagcggctgcagcggctgggcctcgggcgaggggtttgacatcacgcgctgcagcaggccctgggcgcgcaccaggtcggccggaacgcgcgtctgcgccagcagcagcgcaagctgcatctgcgcggggggcgaatcgcccgggtcgccggcgcgggtgatttcggcgctcagctcggtgccgcccagcgggcggatcttgtcggcgtacgccagcatggccgccacgggcccctgggtgatcaacgtgaagagcgacgccggctgggtggcgggcgccttgggttcggcctcgaccggaaccacgcgcggcgccgcgggcggcggaggcagggcatcggcctcggcggttggcttgggctgcgtcgtacacgcggccagcagcaggaccaaaggcatggccaccgcgctggacagggtcgaactgcggacgaacggaaaaagcatgggtcgaaaaaaggacaagaggcggtgtttcaggtgggtgcccgggttcgcggagcttcaggaagggatcaggccgtgcgcggcagttcgatgcgaaagcgcgcgccgggcccgcctggctgcagggtgatgcggcccccatgggcagcaatgtactcctgcacgatggaaagaccgatgccggtgcccttgaccgcgtgctcgggctggcgctcgcccctgtagaaaggctcgaaaatgcggtcgcggtcgctttcggcaatacccgggccggcgtcgttgacatcgatgcacgccgaatccgccgtgccggacaccgtgatggtgatcacgccgccgggcgccgaatagcggatggcgttcgacagcaggttggccaccgcggtacccagcttgacacggtcgaccgtgagcgcaagcgcctcgccttcggcccgaacgcgcagcccgtgggcttgccattgcagtcgctgggcctcgatctgttcctcgatcagcggcagcagctcggtgcgttcgcggcgcagttcgcgcgcctcgaaggcggccgcattgaagcgcagcagcgcctcgatctgcccctgcagcgacacggtgttctggttcaggatctgcgccacttcgagctgcgccggattcagcgggcccgtcacgccgtcttcgagcagcgaaacgccttcccgcagcgcggccagcggcgtcttgagctcgtgcgacacatggcgcaggaagcgggccttgtcggcgtccagctcggtcaggcgcaggcgcagccattcgagctgctgcgacacgcgccggacgtcggccgggccgcggatgtcgatcggttcgtcgagccggttctggcccagcccgacgatggcgtgctcgagccgcttgaacgggcgcgcgagccagatgccgaaagccagcgccagcgaaaccgcgagcacgctcgccgccaccacctcgcgcatcaggcgtcggcgcgcgttctcgatgcgcttggcgagcgcgtcgttctgcatctcgatcaggaactgggcctgctgcgcgatgttggtgttgagcgaatcgagatcgcggaactggatggccatgctgttctcgcgcgagagcgcggtatcggcgctgccgctcatcaggccctcgatcacgccgagctgggtgcgccacatctcgatgcccgtgggcgcaaggccgttcctctcgagccgatcgagcacctggtgcgcctcgcgcgcggcgtcgtcgaagcggcgccgcagcacggcgtcgttcagcaccagcgactggcgcccggcacgctccatggccgcactgcgctcggccagcgactgggccgcgcccgaaagccgcagcgcacgcgcggccgcatcgcggctctgggtcatgagcgcgtcgtactggaacaccgagcgcaacgccacgcccaccaggagcgcggtgatcaagaggaaagcgaaaagaaggagctgctggaacgagccccgtgtcgacggccgtttcgccatcaggcggcgagcgcggcgggagccggcgccgtcgacgattcgcgcgtggccacttcgccgcgcagcgtgtaggccagcgagcgcgtgatgcgcaggtcggccatctgcccgacgaggcgtgcatcgccttcgaagttgacgacccggttgcacgcggtgcggcccatcagttcgttcgcgtccttgcgcgaggcgccttcgaccagcacccgctgcgtggtgccgaccagcgcatcgccgaagcggcgcacgttgccgtcgatcacgcgctgcagcgtctgcaggcgggccagcttcaccgcatggggcgtgtcgtcgtgcagcgcggcggccggcgtgccggggcgtgggctgaagatgaagctgaagctgttgtcgaactggcagtcgtcgatcagcttcatcatcttggcgaagtcttcgtccgtctcgcccgggaagcccacgatgaagtcgctcgacagcgcgagttcgggccggatggcgcgcagcttgcgcaccgtgctcttgtattccatggccgtgtagccgcgcttcatggccatcaggatgcggtcgctgccgtgctgcaccggcaggtgcagatgcgacaccagttgcggcaccttggcgtaggcctcgatcagccgcggcgtgaactcgttggggtggctggtggtgtagcggatgcgctcgatgccggaaatctcggccacgtattcgatcaagagcgcgaagtcggcaatctcggccgtgtcccccatgcggccgcgataggcgttcacgttctgccccagcagcgtgacctcgcgcacgccctggtcggccaggcccgcaatttccaccagcacgtcgtccagcggacggttcacttcttcgccgcgggtgtagggcaccacgcagtagctgcagtacttggagcagccctccatgatcgacacgaatgcggtcacgccctcgacccgcgcgggcggcaggtgatcgaacttctcgatctcgggaaagctgatgtccacctgcgggcgctccagccgctcgcggtccttcagcatctcgggcaggcggtgcagcgtctgcgggccgaacacgatgtcgacgtagggcgcgcgcgcgatgatggcttcgccctcctggctggccacgcagccgcccacgccgatcttcacgcccttggccttcaggtgcttcacgcggccgaggtcggagaacaccttttcctgcgccttctcgcgcaccgaacaggtgttgaagaggatgaggtcggcctcgtccacgttctgcgtcggctcgtagccttcggcggcgttcagcacgtcggccatcttgtccgagtcgtactcgttcatctggcagccgaaggttttgataaagacttttttgctcatggggtgctctctgggcctcccgctacgggaaaggcgaaatgcagggcggggcaatcgctcctgcggcgcggcgggcgacggcccgccggcttcttcattgcgtgttgacggtgtcgttcgacgtgaacggccagatgttcaggaacggcttgctcagcgactcgcggctggccgtggcctcgctcggcgtgaggatccacacctcgcgcagcaggcccgcggcatcgcgcgtgtagttcaccaggtatttctggccgacgatgccgcccgccatcaccagcatgttctgttcgctgcggatgcgggcgccgggcgccagccggtcagcgtggccgtcgagttcgacgtcgggcgcactgatcaccatgaacttgccgcgcagcgtgccgatggggaaggtgcgcccgcccaccagcgactcgttctgggtctgtggccggggcacgtcggcctgggcggccgcgtcaagggaaaaaaggcttgcagctactgtgcaaagcgctatgaaagtgagagcattcgtgggtttcttgcagcggttcatggggtatatccagaggctgtggagcggcgattttaccgagggggtgaaatcccccttggcgcccgccacagcgggttgtgcatgggcccttgaaaggcggctttacttatctttacggcactcgtggacactgcaagccgaccgctgctccaatagctgctgtcagcccaaagtgctcaaaaaaccatgaagaaaaaactcgttctcgcccttgcaggtgtgttgatcgtagccgtcgcgggatggtggtggaacggggctggcgagcgcatgtcggcaaagaacgccaagccggccagcacggccggcggagcgcctgcgggcagtgcaccgcccgcgctcgtcaccctggccacggccgagcggcaggacgtgccggtgacggtgcaggtcaacggcagcgtggtgtcgctcaacagtgtcgacctgcggccgcaggtgaccaacacggtggcggcggtgcacgtgaaggaagggcagttcgtcaaggaaggccaactgctcttcacgctcgacgaccgcaacgaccaggccaacctggcccgcgcccgcgcccagcagaagcgcgacgaggccaccatggccgacctcgagcgccaatacaagcgcagccaggagctgctggcgcagaacttcatttcaaagagcgctacggacgccacgctgtcgcagctcgaggcgcagcgcgccgcggtggcggccgaccgcgccgccgtgcagtcggcgcaggtggcgctcggctatgccacgctgcgcgcgcccatcgcggggcgcatcggcgccgtcaacatctaccccggcacgctggtgcagcccacgctgtcgctggtcaccatcacgcagctcgaccccatcgcggtgagtttcccggtgcccgaagccaacctgcaagacctgctggcggcggcgcgcagccgctccaaggtcgaggcgctcgtcagcgggcgcaaggagccgctgaccggcgtgctcaacttcgtcgacaacacggtcgacccgcagatcggcaccgtgcgcgccaaggcggtgttcgacaacgccgaccagagcctctggcccggccagttcgtcggtacgcgcatcacggtgcgcaccctgtccggcgccacggtggtgccggcggcggcgctcatgatgctgtccgacggtgcttcgctctacgtggtcgacgaggccaaggacgccaagcgccgcaaggtgcaggtgctctacaccttcggcaccaaggtggcggtgagcggtgtcgcgccgggcgagcaggtggtcatcgagggcagccagaacgtgcgcccgggcggcaaggtccgcatcgacaagaaggccgcaccggccggcaccaccggggccacgccgggcagcgcggcctcctcggacacccagactccgcgggaacgcgcatgaacatctcggagctctgcatccgtcgtcccgcgatgacggtgctgctgtccgccgccgtcgtggtggcgggcatctttgcgtacttcagcatcccggtcgccgcgctgccgagctacaacacgccggtcatcaacgtgaacgcgcagctgccgggcgcaagcccggacaccatggcgtcgtcggtcgcgctgccgctcgagaagcagttctcgaccattccgggcctgcagaccatcagctcggtcaacacgcagggcgtgagttcgatcacgctggaattcgtcagcagccgcgacatcgacgccgccgccgtcgacgtgcaggccgcgctgctgcgcgcccagcgccagttgccgcaagagcttacgcagctgccttcgtaccgcaaggtgaatccggccgatgcgccggtgctgttcatcgcgctgatctctccgtcgatgaacccgtccgagctcaacgactatgccgagaacctgatctcgcccacgctctccaccatcgacggcgtggcgcaggtgggcgtgtatggccgcaaggccttcgcggtgcgcatcaaggccaatgccgacctgctcaatgcgcgcaacatcacgctcgacgaactggccaaggccgtgaactcggccaacgccaacacgccggtcggcacgctcgacggaccgcgccagacgctcaccatccaggccaaccggcagctcaccaaggcggaagatttcgccaagctgatcgtcgggcagcgcaacggcgcgccggtgcggctcgacgaagtggccaccatcgaggacagcttcgaatcggtcaagaccgcgagcagcttcaacggccagagctccatttcgctcgccgtgcagcgccaacccaatgccaacacggtggaggtggtggacgcagtgcgcgcgctcattccgcgcttcaaggctgagctgccgcaatcagtagagatccacatggtgaacgaccgctcgctgtccattcgcgaggccgtgcacgacgtgcagctcacgctgctgggcaccattgcgctggtggtgctggtgatcttcctgttcctgcaccggctggtggccacgctgattcccgccgccaccattcccatctcgctgatcggcgcggtggcgctgctctatgccttcggctacagcctggacaacgtctcgctgctgggcatcacgctggccgtgggcctggtggtggacgacgcgatcgtggtgctcgaaaacatcatgcgctacgtcgagaagggcatggagccctttgccgcggcactgcgcggcgcgcgcgaggtgggcttcaccatcatttcgatctcgatctcgctggtggcggtgttcattcccatcttcttcatgccgggcgtgatcggcctgctgttccatgagttcgcggtggtggtggcgctggcggtgctggtgtcggccgtcgtctcgctcacgctggtgccgatgctcgcgagccggctgctcaagcacgtgccccgcaaggaaggcgtgctcgaccatgaagaggagcatccggagcccggcaccgccattggccgcgccttcgagcgcggctaccgctgggtgcatggcagctacatgcgaacgctcgactggacgctgggacaccgcatggtgatgctgctgatcgccggcagcaccttcatcgtcaccgcgtggctgttcgtctccattccgaagggcttctttcccgaggaagacatcgggcagatccagatcaccaccgaagcggccgaggacatttccttcaccgccatgaacgcgctgcaggaacgggtggccgcgtcgctcctggccgacccgagcgtggcctacgtgaactcgttcgtcggcgtgggtggccccacggccacgcagaacgccggccgcctgttcgccgtgctcaagccgcgcggccagcgtcccaagatggccgtggtgctcgagtcgctgcgccagcgttttcgcgagattccgggtattgcggtctacatgcagccggtgcagaacctgcgcctgggcggccgccagagcaaggcgcgcttccagtacacgctgcaaagcgtgaacgcgggcgagatggtgccctgggccacgcggctcatggagcgcatgcgcgccgaccctgtcttccgcgacgtcaccagcgattcgcagaaccgcggcctgcaggccacgctggaggtcgaccgcgacaaggccggcgtgctgggcgtggccgtgggcgaccttcgcaccgcgctctacaacgcctacggcgaccggcagatcggcagcatctacggcgcgagcaacacctaccaggtgattctctcggcctccgacaatgaccgccagttcgaggacgacatgtcgcgcctgtcggtgcgcagcaccacgggccggctggtgccgctctcggccttctcgaccgtccagcgcaccgtgggaccgacctcggtcaaccaccagggccagctgcaggcggtgacggtgtcgttcaacctcgcgcccgatgtgccgctgggcaacgcgaccgcgaagatcgaccagttcaaggaagagctgaagatgtcgccgtcgatcatcaccacctacggcggcgatgcggcggtgttccagagctcgcagtcgagccaggccgtgctgctggtgctggccgtgctggtgatctacgtgctcttgggcgtgctgtacgaaagctacatccacccgctgaccatcctggccgggctgccgtcggccgccgtgggcgcgttgctctcgctcaagctcttcagcttcgacctgacgctgatcgccactatcggcatcctgctcctgatcggcatcgtgaagaagaacgcgatcatgatgatcgacttcgcgctcgacgcgcagcgcaccgaaggcatgaagccggtggatgcgatccgcgaggcctgccggctgcgcttccgccccatcatgatgaccacgctggccgcgctcatgggtgcgctgccgctcgcattggggctgggcgccggcgccgaactgcgccagccgctgggcgtggcggtggtgggcggcctcatcttctcgcaggtgatcacgctctacatcacgcccgcgatctatcttgcgctcgaccgctacagcggtaccgggccgatggtcgaactgccgggcgaggcgacaaaggccgaggccggtggtgccgccgcggggcacgcggcctcctcgcacgcctaggtcgttgtttcgtcgaggatgtcgtcgtccgccgccaggtgggcggtgtcgctccagcccaccaggctgaagccctcgggcgtccacagcatgcggttgatggctgcgttgccgagctgccaggtgcgcggcgcctgcagctcctggcgcgtggcggcgcggtagagcacgtccatcacgccgccgtgcgccaccagcgccaccagctggcccggatggcgtgcggccagtttcgacgcaatgcgcgtcacgcgctcgcgaaacaccagcaggctctcgccgccctcgggttcgaactcgggatcgcgctcgcgccagcgcctggcctggtcgggcagggtggcctcgatctccgcgaagctcattccctcgaaacggccgaaggcgcgttcgcgcaggccaggctcggggtgcaccgtgaggccgtggggctgggcgatctcctgcgcggtctgccaggcgcgcgacaggtcgctcgcgtagatcgcgccgatgtcttcgtgcgccagcgcctgccccacgcgccgggcctgccagaggccggtggcgttgagtccgacgtcgagctggccctggatgcgagtgtcgacgttccaggcggtctcgccatggcgaacggcaatcaggcgggtgatttcttccatctgccgggattctagaagcgcgtcatttcttcgctgtcgacagctcgatgttcacgcggcgctcgccctgcggcggattcgggaacccctgcagcgcggcctggaacatcaccggcaggatggtcgagctcacgttgtacggcccgtcgttgcgggcccgcgtttcgtagaccacgcggttcgagccgatgtcgcgcagcacgatgctcacttcgcgctcataccaggggttggccgcgggcgggatgaagccaggtccaccgtaccagccgccgccataccagcggcgcgcgtagccgtggtagccatagccataacctccccaggggccgtcgaagagccacgggtccgcccagggcgaaaggccgaccgacacgcgcgcgccgatctgcgcgctgtactgcggcctggcgtcgtcgcggcgcaggccgactttctcgagtgccgcggcggccatcgcctcgagcgattcctgccgggcggcgtcggcctgctgcgacggcaggcgatcgaaacggtaggtggcgccgggcggcaccgcggcgagcgacgaaaaactcttcacatcgctgtcgaccacccaggaggtggcgcagccgctcagcaatgctgccaaaaagagagcaaaaaacgcacgtttcatgaggatctccgggctccgtggcccaaaattcccctgggttgcccgctcagccctggaggatgcgcagggctgcaggtgcctgggagagcaggtcgaaagaaggcgtgtcgaaggccttgtcgccgtcttcgtcggccacgccggtggccttcagacccttgaagtcgtgccgcgttccgtcgagcaggtgggagggcaccacgttctgcagcgcggtgaacatgttctccacgcggccggggtgcttcctgtcccactcgcgcagcatttcgccgacctgcttgcgctgcaggttttcctggctgccgcacagcgtgcacggaatgatcgggaactcgcggtgctgcgcccagcgcaccaggtctttctcggccacgtaggcgagcgggcggatcacgatgtgcttgccgtcgtcgctcaccagcttgggcggcatgctcttgagcttgcccgcgaagaacatgttgaggaagaaggtctgcagcatgtcgtcgcggtggtggccgagcgccaccttggtggcgccgagctcgtccgccacgcggtacaggatgccgcggcgcagccggctgcacaggccgcaggtggtcttgccctccggaatcacgcgcttgacgatgctgtaggtgtcctggttctcgatgtggaagtccacgccgagttcgctcaaatactttggcagcacttcttccggaaagccgggctgcttctggtcgaggttgaccgcgacgatgtcgaaatggatcggtgcgcgcgccttgagcttgagcaggatgtccagcatggcgtagctgtccttcccgcccgagacgcacaccatgaccttgtcgccctcttcgatcatgttgtagtcgacgatggcgcgccccacctcgcggcacaggcgcttttcgagcttgtgcgtctcgcgttcgatcttcagcgaattggcaggggtggcgccggcgacgggcgcctcgtcgatccagacggcgttcatgggtgggctacttcaggcaggacagggggaggagggccccgattttgccttggatcaccattccccggcttccatgcggatagccacctcgcagtcgtcgaagatttcgagcttggcgatcttcacccgaacgccgaccacgccgggcagctgcagcaggcgctgggcgagcttgccgatgagggtttcgagcaggttcacgtgctcggccgtgcactcgtcgatgatgatgcggcgcaccttgcggtagtccagcacgtgaaagatgtcgtcgtccttcggcatcagcggctgcgcgcccagatgcagctcggcatcgacctggatcggctgcggcgccgtcttttcccggtcgaggatgcccaggttggcgtcgaagcgaagcccttgaagggtgagggtctggcggccgatgggggtagagggcatggggggctcacatcagcgagaagtcgcggtcgaatttcatgaggtgctggcccccgtccaccaagagcgtggtgccggtgatcgagttgttctccagcgcgaacttcaccgtggccgccacgtcggccggcgtcgaagagcggcccagcggcgacagcttgtgcagctgtgaaaacttggcctcatcgagcatgtggctcggcagcgtgaggccgggcgctacgcccaccacccgcacgcgcggcgccagcgccatggccagcatgggcgtggccgcttcgagtgcggccttggacagcgtgtagctgagaaagtcggggttcgggttccagagcttctggtcgagcaggtgcaccaccgcgccctgcgcgtcacgcagcgccagatggtcgcgcagcgcctgcgccagcaggatggccgcgccggtgttgctgcgcgcgtggcgctccatcagcgcgtagctgaagctggccgcatcgtcgtgctcaaagagggccgcgctgtggaccacggcatcgaccccgccgaaatgcgccgccacgcgcggcagcaaggcgcgggtggcgccttcgtcgaggaggtcggcctcgaagaccgccgaactgcccgagaggcccgcgcaatcggccgccgtttgctcggcctcggcgcgcgagctgcggaagtgcaccgccacctgccagccccccgtggcgagcgccagtgcgatctcgcggcccagccgccgtccggcacccgtgaccaggacgatgcggcgggccggcgtaacaggagatggaggcactgtgctcatgcggagagagaagggagaatcggggggtgacgacaaagacgacgaacagtttacccatcgccctcgataccttgattgcccgcgccgtggatcgcgccggcggatggatcggcttcgaccgcttcatggcgctggccttgtacgcgccggggctgggctactacgccaacagctccgccaagttcggccacatgccgtcttcgggcagcgactttgtgacggcgcccgaactcacgcccatgttcggccaggcgctcgcggcccaggtggccgaggcactggaaaagaccggtaccgacaccgtctgggaatttggcgccggctcgggcgcgctggcggtgcagctgctgcacgcgctcgacgaaatgggccgcggcgacgtgcgctaccgcatcgtcgacctctcgggcaccttgcgcgaacggcagcagcaggcgctggtgcgctacgccgaccgcgtcgattggctcggcgagctgccggagtcgatgcagggcgtggtggtcggcaacgaagtgctcgacgcaatgccggtgcagctgctggcgcgcgtgggcggccagtggcacgagcgcggcgtggtgcgcaatgccagcgccgatggttggacctgggccgatcgcaccaccgaactccggccgccgttcgaggtgctgggcgaccacgactacctgaccgaaattcatccgcaggccgaggccttcgtcgccacactggcggaccgtctggcgaaaggcgcggcctttttcatcgactatggttttccggaacgcgagtactaccacccgcagcgccacatgggaacggtgatgtgccaccgtgcgcaccaggccgatggcgatccgctgtccgacgtgggctacaaggacatcacggcgcacgtcaacttcactggcatcgccctcgcgggacaggaagcggggttcgaggtgctgggctacacgagccaggcgcggtttctgctgaactgcgggttgcttgcgaggatggagcagggctctactgcggagcggggaatggcggctcggctcattcatgagcatgagatgggggaactgttcaaggtggtggggtttgctgttggtgagccttgggatgcgatggggtttgtggagggggatcggagtcatacgctctgactctttgggctgttggccttgtttgcttcccgaggccgggactcgccccggcgggcgactcactttcttttgcttcgccaaaagaaagtaagcaaagaaaaggcgaccccactgtctgcgacccttcgcttcgctgcgggcaacctgcggtgctcgggtttcgcggggtctcgcagaactcgcttcgctcaaacagctgcgagccctgatccgcgaaaccctgcgctcctcggcgcatacagaggggcttggagaccgaacgggcctttgcttcgctcggccaccaggccaccgcggcgctatgcgccgcggtggttggtattggcgtgggcttcggtattggctgttggggttggggccgagcgaagcgatggcctgtcggctcccaccccttctgtatgcgccgaggagcgcagatgcaggcgggatcagggccgcagctgtttgagcgaagcgagttctgcggacccccgccggagtcgagcaccgcaggttgcccgcagcgcagcggagggacgcagacagtaggggtcgcctttctttgcttactttctttggcgaagcaaagaaagtgagtcgcccgccggggcgagtcccggcctcggaacccaaaaaaaagatccgcaaataagctaccaacgaagagttcgttgatcaaacgccccgcgaaacctacattggcggaatgaccgcttcttcaaagaccgaagcccctccgcagcacttcgaagtgcgccccttccccgcccccgtaggcgcagaaatcctaggcctggacatctccaagcccatcaacgacgaagatttcgcccggatccatcgcgctcacctcgaccaccacgtcctggtattccgcaatcagcagatcacccccgccgagcacatcgatttcagcagtcgcttcggcccgctcgaaatccacgtgctgcaccagttccatctgaagaaccatcccgagatcctgatcgtctccaacatcaaggaaaacggcgagcccgtcggcctcggtgacgcgggtgcctattggcactccgacctctcctacaagccccaaccgagcctcggctccctgctgcatgcgcaggagctgccgagcgagggcggcgacacgctcttcgccgatcagcacctcgcctgggaagcgctcggcccggatctgcagcaacgcatcctgccgctccaggccgagcacagctaccttgccaagtatgaagagctgcgcgccaagaacccgtggcggccgaagctctcgcaggcgcaggtcgaccaggtcacgcccgccgtgcagccggtggtgcgcacccatcccgagacgggccgaaaagcgctgttcgtcagcgagcatttcacgacgggcatcgtcggcctgccgcaagaggagagcgacgcgctgctggccgagctgttcgcgcacagcgtgaagcccgagttcgtgtaccggcaccggtgggcgccgcacgacctggtgttctgggacaaccgctcgctgatgcacctggcggccggcacgcccgaccacctgcgccgccggctgaaccgcaccaccatcgctggcgacacgccgttctgaaaagggacgccggcccgatcgttttcagctggcggcaggcttgccaccgcccttgcgcagcgtgcgcagctcagcggtgaggaattctttggcgtccctcaccgcaccgttcggcatcttcacctggtagggcttgccggttatctcggagcgcgacgcgcagcggtcgatgaagtcttccgcggtgacgatctcgtctttgaagtggtcgaacttggcttgcatgtgcttcgcggcgtcggcggcgttgtgctcgtcgccattgcgcatgaaggtcatcgtcttcatgttcgaaacgcgcaggatcagcgtgtcgatgagcttctgctccgatgcggaaggggtggcctgcgccagcgcggccaccgccgcgagcaaaattgcgaacagggcggtgcgaaaaagtcggaatgaggacggcatggataagcgggagttcggcccatgctaggtccagggcccctggcatgtcaaaccggcccgcctcgggtctaattgcagtttttggcacgcgtgacttctcaatgagccccccgacccccgatctcctgtcgattgccaatgcgctggccgacgcggccgccgcgcaatcgatgcattacttccgcacgccgctcgacatcgtcaccaaggccgatgcgagccccgtgaccctggccgaccgcgccgccgaaacggccatgcgcgagatcctggccgagcgtgccgcggccgatggcatcttcggcgaggagcacggcctcgagcggctcgacgccgagcgcgtctgggtgctcgatccgatcgacggcacgcgcagcttcatcaccggatcaccgctgtggggcacgctgatcggcgtgctgcaaggcgagcgcgtggtgcttggcatggtcgacatgccggtactgaaagagcgctggatcggccaggccggcaagggcgccacgcgcgacggccagccggtgcgcgcaagcagctgcaccgaggtagccaaggcgcgcatcgtcaccacctcgcccgacatcttcgcgccggacgattggcaggccttcgaccggctcagccggcagtgcgcgatgcggcgcttcggcggcgactgctatggctacgcccagctggccggaggcaccatcgatctggtggtggaaaccggcctgcagccctacgactacctcggccccgcgggcctgatcgaggccgcgggcggcgtcatcaccgactggcatggccagccgctggggctcgaatccgacggccgcgtgattgccgccgccacgcccgaactccacgcgcaggcgatggccatcctcgcggcgcaggcttgaatcggcctagactgtttccatgatccgctggctgatcgtcgtcgtccttgccctggtgctcatgagcggcctcaccgcctggctgcgccggttcggctttgggcggctgcccggggatttcgaatttcacgccttcggccgagactggcagctgccgatctcgagcaccctggtgctcagcatgatcgcggcgctggtggcgcgcttcatttagctagcgcaaccgatgaacccaacgtccgaaaagagaagaaccacgcaatgagagtctgcgtcgacatcggcggcaccaaggtggccgtgagcctttccccctcgagcgatgcgccgctgcttggccgccgcagcgagccgaccgccaagaccggcgacaacgatgccgtcgccgtgcagatcatccggatgatcgaggaagcctgcgccgaacacggcgtcgatgccgcctcgatcgatcgcgtgggcgtgtcgtcgaccgggcccttcgagctgcgtgacggcctggtggaactcgccacgccgaacatctgcggcggcattgcgggcccggcgcgcggcctgcccaacaactggatgacggcaatcatcgaagcaccgctggcccggcgcttcggcagcgtgcgggtcgagaacgacgcggtggcggcgctcgaggccgagcgccagtggggcgctctgcaagggctggaccactgcgcctacgtcacctggagcaccggcgtgggcgtgggcctgtgcgtcgatggccgtgcgctgcgcggcaagaacggcaacgcggggcatgcaggccacagtttcgtggcggacgacgccagtggtgcgctctgcggttgcggcaacctcggcgacgtggaggcactggtggcgggcaattccattgcgcggcgcctggggcagccggcgcccgagctgttcgcggccgcgtcgggcggagaagcccacgccgtcgagatcgtcgatgccttgtgccgtgtcatgggccggatgatctacaacctggtggccacgctcgatctccagcgcatcagcctgggcggcagcgtgttctggcaccaccgggactttctgctgccgcggctgcaggcgcaggtcgacggcaagctgctgccgctcacgcgcggcgtgatgctggtgcccgccgggctcggcgaaaaggtcggcgactacgccgctcttgcgctgctcgactgaagcctgcgtgcttcgggcggtgagggggacggtgccgtccctgcgccggtgccgccgcggctcagcgtctcgatgatctggcccagccggcgcaggccggtgtcgacggcttcaccgtaaggccagccgcaattgatgcgcaggtagtggtcgaagcgcgacgagttggagaacagcgtgccgggcgccaccacgatgcgctcgaccagcgctgcatcgaagaccctcgaagatgaaagccgctcaggcagctcgacccacagttgcagtccgccgggcggcaggttgatgcgcgtgccggcgggaaagtagctggcaattgcatcggcggtctgctcgcgctgcgtcttgaggcagccgcgcagatggcgcagatggcggtcgtaggcgccggtgcccatgaaaagacccgccgcgccttgcgagagcccttcgttgttgcgcgtctgcgcaaacttgagcatctccacccgcgcctgccagcgtccggccgtgatccagcccagccgcaggccgggcgcaagaatcttgtgcagcgaggcgcaatggatcacgttgccgctggtgtcccacgacttgagcgcgcgcggcggcgttggggcgtcgaccagttcgctgtaggtgtcgtcctcgatcaacggaatggcatgccgctcgcacagttgcgccagccgggccttgtgggcgtcgggcatgacgctgcccagcgggttctgcaggtgcggcaccaccaccacggccttgatgttgtcgtaggcgctgatcgcaagctccagcgcctcgatcgacaggccggtctgcgggctggtcgggatctccagcgcgcgcatgccgaggctttcgagcacctgcaaaaggccatagaaggtgggcgactccaccgccaccgtgtcgcccggctgcgccacggcgcgcagcgcgaggttgagcgcctcgatgcagccgttggtgaccaggatgtcgtccggcgagatcgccatgcccacgcgcaggctgcgctgcgcgagcacctcgcggaactggcgatggcctttcagcggcgacgcgactgtcagcatctcgggctgctggcgcagcatgcgcgtcatcgcattgcgcagcgcctcggcggggtaaagctccggcgcgccgcgcgcgatcgagagattgagcttttcggcaatctgccgccggcgcgccacgaagtccgacaccttggcgtggatgcccacgtactgcgccggatccggcggcacgccggctgcgggctcctccatcggcgcaatggccagccgccgcggccggcgcacgaagtaccccgagcggtcccgcgcctcgacccatccgtcgctctccatcgtgcggcacagctgcagcgcggtcgaaaggctgatgtcgtgcaggcgcatgaggctgcgcagcgaaggcagcttgtcgccttgcttgagcgagccggtgtggatcgcgtccacgtagtgcgcggcgagctggcggtagagcggtagcgagtccatggcgtcgatgctccctctatcgcgcatcggaaaacagatgcagttgcaaaggaaaacgaccataacagatgcgccgtgcccgccactgttccggtgcgaatcgccttgccgtgtgcctgttttttgagcgcccgaattcctacgatgaccgcatcaactccggaaggtgcgtccatgtcccccctcactctcgaccgactgcccgatacggtctccctgcaaccgggccaggccttgcgcacctcgctcgatcccgccacctggctcgagatgctggagggcagcgcccagctcgtgtcgccgccttcatggttcggcgacaccgtgttcaccgtgaagaccgcgctggccgaaggcgacgtgcatcgcctggaacgcggcggctggatcgagctgtcggcgctcacgccggtgcggctgcgggttcatgcgccgcaacaggcgccggcaccggcggcccggcctgccgagacccggcccgtgatgcgtctggtgcggctcttgaccggcacctgaacgggctgccgcgttctgtctggctagcgctggctcgcggcgtgtcgcagcgcttcgagaaaggtgcgccgccaccaatggatgtcctgctcgcgaatgcgcgacaagagcttctggtgccgctcgcgccgctcttccagcggcatctgcagcgcctgctgcacggtttcggccgtgccgtgcgtgtcgtacggattcaccagcagcgcctccttcagctgctccgccgcgccggcaaagcgcgacagcaccagcacgcccgggtcggccgggtcttgcgccgcgatgtattccttggcgacgaggttcatgccgtcgcgcagcggcgtcaccaggccgaccgccgccgcgcggcacagccccggcacgcgcttgcgcgccaccatgcggtggatgtagcgcaccggcatccagtcgagctcgccgtagtcgccattgatggcgccgcacagcgactcgagctcgcgccggatgtcgccgtaggcatcgaccgtttcgcgcgtgggggacgcaatctggatcagcgtggcgctgcgccggttctcggggtagttggccagcagttcgcgaaaagcccgcacccgctgcggaatgcccttggagtagtcgagccggtcgatgcccagcagcaaccggcgctgcgaatattcgcgcttcatggtctcgaacatgtcgcgcgactctttcgcgtgcgtgagcgccgcgaactcgtcgacgtcgatgccgatgggaaaggtactgcagcgcaccgtctgtccgtaggcgcggtacatctcgtcgcccaggtattcgccatgcgcctcgttgcgcacgtagtgctcgaaatgctgcacgtcctgctgcgcctggaagccgatcaggtcgtaggagaacagcgagcgcatgagccattcatgctgcggaacggccgcgatgatgatctgcggcggcagcggaatgtgcaggaagaagccgatgcgctgcctgcagcccatggcgcgcaactcggccgcgagcggcatcaggtggtagtcgtggatccagatgatgtcgtcgtccttcaggagcggcatcagcttgcgcgcgaacagctggttcacgcgccggtagccgccgatgaagccggcatcgaaatgggcgaggtcgagtcggttgtggaacaccggccacagcacgtcgttgctgtagcccaggtagtagctgtcgtggtcctcgcggctcaggtcgatggtggccagggtgaccttgccggcctgcagcacgtgcagctcgccttcgcccgtggggccgtcctcgacgatctggccgctccagccgaaccacaggccgccgctttgctgcaggctttcgccgagcgcaacggccaggccgcccgcggccggcttgcgtggatccgccacgcggttcgaaaccacaaccaagcggctcatatgcaggagtcccagggagccgacagccgcacggccgcattgatgatgccgaccatcgaataggtctgcggaaagttgccccacatctcacccgtgaccgggtgcgtgtcttcagagagcaggccgagcgggttgcgcgccgcgagcatggtctcgaagatctggcgggcctcggccttgcggccgatcttggccagtgcgtcgatgcgccagaaggtgcagatgttgaaggccgtctcgggcttgccgaagtcgtcggccgcttcgtagcggcgcatgtaggggccgtcgcagagcgacttttccatggcgtcgacggtggaaatgaagcgcgggtcgcgcgcgtcgatcaggcccacctccaccatcagcaggatgctggcatcgagttcgtggccgccaaagctttcggcaaaggcctggcgctcttcgcaccatgacttggcgaggatttcttccttcatgcgtgcggcatggccgtgccagtaggcggcgcgctcgggcaattccagcgcacgtgcgattttggcgagccggtcgcaggcggcccagctcatcagtgccgaactggtgtgcacgcgggcacgcgtgcgcagctcccacatgccggcatcgggcgtgccgtatacgcggatcgcctgttcgcccacggcttccagatgcggaaactccgccacgcccgcgcgggcgagcaggcggtggtcgtgaaaggcctgcgccgcaccgagcacgatgttgccgtagacgtcgtgctgaaagtgctcctgcgcctggttgcccacgcgcaccggacccatgccgcggtagccctgcaggcctcccaccatcgactcgggcagctcgcgctccagcccgatgccgtagagcggctggatgtgctcgccgtgcgaaccgatcaccacgttgccgagccagcgcaggtagtcttccatggtgcccacctcgctcagcgagttgagcgcgcgcaccacgaagaaggcatcgcgcagccagcagtagcggtagtcccagttgcgctggctgcccggcgcctcgggaatgctggtggtcatggcggcgacgatggcgccggtgtcttcatagagcgagagcttgagcgtgatggccgcgcggatcaccgcgtcctggtattcgaacggaatggccaggcgcttgctccaggtgcgccagtaggcgatggtttcctgctcgaaggtgcgcgcggtgtcggcaatgccgtcgagcagggtttcgtcgacgccgaacatgaagttgtattcgcgcgagatcacgaaaggctggcgcgaaagaatgtgcgagatcgaggcgtcggtgttgagccgcagcgtcacgtcgggccccacgtagcggatgtggttgctgccgcgcgtcacctccagcggtgccgtggcaccccactggaagcgcgggtcgagcgccacgcggatgcgcggcgcgccggcaatcggccgcacgcggcgcaccatcatcagcggccggaagtagcgcgagcggctgtagaagcgcggcgcaaagtcggtgatctcgatgccctggccggcgctgtcgtaaagctgcgtgcgcagcaccgccgtattgggctcgtaccactgcttgctggaggcgaagtcctcgatctcgatggcccaggcggcggcatcttcgccggggtgcagcagggcgttgaacaccggatcgccgtcgaagcgcggcaggcagcaccacacggcgcgcccgcgggcgtcgatgagcgcactgtaggcgcagtttccgatcacgcccacgttgagcgaaggctcggccgacggcccgaagccgccgcgcggcacggcctgcaccgcggcatgcgggtcgacgggcgccgtctcggcgggcctggctgcgccggaaagggaagcgcctgcgcgatcttcgggtgccttcgacaattgcatctcgctcattcagggttccttggggactcgtctttcttctttttcggtgcggccagcaggtcgcgcatctgcaccagccattcgtagacggcgcggggcgactccagccggtgcagtgccaggctcgggcccgaaccgaccttgatgccgacgccgccgcgcggctgcacgaccgcgaaaccgctctcgtcggtggtgtcgtcgcccgcaaagaccggcacgcgccccgcgaacggagcctcgttcatgaaggcctcgatggcaatccccttgttgacgcccgtgggcttgacctcgaacacgaacttgccgtgcatcagctcgagatacggccggcccgcgatggcgcgcgacatggcgtccctgcacacggcctccaactgcggcgccagccggtagtgcagcgcgatggccgcgtgcttgcgctcgaccaagaggccttcgtgcacgcgcgccagctcgttggcgatgtcgagaatgggcacgaggtcgggcgcgtgctgttcctgcatgcggccctgcgagtcgcggcgctgcacgccgtgctcgccggccgccggcagccgcagcggcgcaagaaaacggtcgatggcgtcgatctggcgtcccgacaccacggccagggcaccgccgagctggtcgcgcaggtcttgcagcagtgccaccagcgcaggggggacctcgatggcttccggggtgggcgcgagcgcgaccagcgtgccgtcgaagtcgagaaagagggcggtgtctcggcccagcgggggaggcgtctgagagggcattggcatcggtgaaaaccataacacgggcctggcatttgccgtgtcggccaaagtcccgcgcgcgttgggacggcgacagggcgccggcgcattcgaaccgggcttcagcccagcgacgccgccacggcctcgacccgggcgcgatggatcgcctcgccgatctgcggcccggtggcgcccgactgctgcgccgcccgagccaccgcgtcggtggccacgccggcggccgcggagagcaccgcaagcagtcgctcgcgctgcggatagggctggtcttcgaatccgagccggccgcgcgagtcgcactcgcaagccaggagcacgtcggcaaagcgcgccggcttgcggaaggcgtcgcaacgctccagcaggcgcaccagctccggcgcctcgagctcgccgctgccatggatgttgccgtgctcgcgcgccaccacctcggccagttcgcggacgtcgaccggcacgcgccagcgatcgcacaccgcgtgcagcagatcgacgctgcgtttctcgtggccggcatggcgcggcagctcctcgggattcgtcgtgcccttgccaaggtcgtgcatcaggcaggcgaaacgcaccggcagcggcgcctcgagccgggcgccggtgtcgacgaccatcatcaggtgcacgccggtgtcgacctcgggatgatgctccgcggcctgcggcacgccccagagccggtcgacctcgggcagcagcacggccagcgcgccgcaggcacgcagcacctcgaacatgcgcgacgggcgggtttccatcagaccgcgcgccagttcctgccacacgcgctcggccaccagcgcatcggtttcgccggcctcgaccatctcgcgcatcaaggccatggtttcgggcgcgaccgagaaatcgtcgaagcgtgccgcaaagcgggccacccgcaagatgcgcaccgggtcttcgcgaaacgcatcggtgacatgccgcagcagcctttgctgcaggtcgcgccggccatggaaagggtcggccagcttgccggggtcgggctcgaaactgccatcggcctgcacgaactccgcaggcatcgcaatggcgttgaccgtgaggtcgcgccgcgccaggtcttgttccagggtgacgtcgggcgaggcgtggacggtgaagccccggtagccgggagcgctcttgcgctcggtgcgggccagggcgtattcctcgcgcgtgcgcggatgcaagaacaccggaaagtcgcgccccacgggcaggtagccgcgcgagaccatttcttcgggcgtggcgcccaccaccagccagtcgtggtccgacaccggccgcccgagcagccggtcgcgcagcgcaccgccgacgagataggttttcatgcgcccagtgtagggatactcaggctcccctgaacccgacgcgcattagcgggcggtgcggtagggctcctcgaactgcaggaagtccttctcggccagggcgtcgtcgatccatgccttgatgccgggcagggcctgcacccgctcgatgtaggccgagacggcggccggcaccggcagcccataggtcttgatgcgcgtgccgaccggcgcgaagtaggcgtcggcaatgccaaattcgccgaacagcatcgggccgccatgggcgtcgagcaggccggtccacatctgcacgatgcggtcgacgtcgccttgcaggccggggttgtccttcagcagccgggcgccgacgtcggtcagcgaggcctcgatgttcatgacgcacaggctgcgaaggctgccgaagcccgaatgcatttcggcgcagatgctgcgcgcgcgggcccggtcggccatggcgcggggccagagctgcttttccggaaaggtctcggccaggtattcggcaatggccagcgtgtcccacaccacgaggtcgccgtcgaccagcaccggcaccttcgccacgggattgagggcgccgatggtgttcttgaactgcgaattggcgtcgaacgagtcgaagcgcaccttcacttcttcgaacggaatgccggcctgcttcatgagcacccagggccgcatggaccaggaagagtagttcttgttgccgacgtagagcttgcgcatcgtgtgatcctgcggttcagataaggagaaagccttcaatgctagccgggccgtgcgtgcggattgatgccgaagcgcgggcgaattgatgcatgccgtgcgccgctttctctctttctcttcttcagcgcggcggctggtcttcaggcgaggcgatcacacggggtttgccattgccgttgccgcggggcggcccgaccatgcgctcgatcaggctcaccaggcgcggcaccagcgaaagcacggccagcgccagcagcgcgctcaacaccgcggtcacctcgcggccgagcccgcaggccatgccgatggcggccgtcatccacagcccggcggcggtggtgaggccttgcacctggtgttcgtcccggccttgcttgaggatggtgcctgcgcaaagaaagcccacgcccgccaccaggccctggatcacccggctcatgtcggccggcacgatgccggtctgctgcggaatcagcacgaacaacgccgagccgatggccaccagcatgtgggtgcgcacgcccgccgccttgccgtgctgctcgcgctcgaagcccagcatgaagccgagcaccgccgccagcatcaggcgaacgacgatgcgcgtgagctgggcgacgtcgcccacgtccgagaactcggccgcaacggtgtcgagtacctcgcgggcccagctcatctcaggggaggtccttgttgggttccggctccgaggcgtcgcgcgggccgacccggccaaggcgttctttcagcgactgcgggcgtccgctgatcagcgccgcgtagttggtggtgttggccagcaccttcttcacgtagtcgcgcgtctcgttgaagggcacgttctcggcccagatcgcggcttccatcaccgggccgttgcgccagttgcgcggccggcccgggccggcgttgtatgcggcggcagccagcgccatggaaccgtcgaagtcgtcgagcgcgagcttcaggtagttggtgccgatggtgatgttggtctcgcggtcgttgatctgccccggcgtgaagtcgttcatgccgatcttgcgcgcggtccagcgcgcggtggccggcatcacctgcatcaggcccgaggcccccacgcccgagcgcgcatccatgatgaaacggctttcctggcggatcagcccgtagacgtaggccgggtcgagcccgatgtcctggctcttgcgcagcaccgtgtcatggaacggcatagggaagcgctgctccacgtcgatcgtgcccttggtgcgttcgctggtgttgatgcagcggtcccacacctcgcgctggcaggcgaagtcggccgcggccagcagcgcgcggtcgtccatgccgcccttgtcgtgcaggttggtggcgtagttccattcgcgcgtgccctcggggcgcaggccgatggcaatggcatagagcgcgcggttgagcgcgatgttgctgcgcgcggcgcctttctcttcgggcgtgagcggtgccggccgggtgggcaccacgatgcgttggccgagctcttcgagcgccagcatttcatagaagccgcgcgtgccggcaatggtctggtagagctcgcgtgcctgcgcgcggcggtcgtcgccgccggcggcgctgagtgcgcgggccttccagtagacccaggtcggctcttgctgggcggtttcgctcatcgcattgatggcgggcgccacttccttccattggccggcgcgcagcgcggcacgcacgcgccagccgagcatgtcgtcggacaggtcgccgttcttcgtgacgttggcaaagtagctgccggccagcggcgagagcttgccggcagcctggcggccgatggcgccccagagccagttgcgctcttcggccgacagcatcggcccccacttggcgtcgacttgggaggcggcctggtccgggtcggccatggcgatcttgatgagcgccagcaccaccagttccttgcgcgacttggcggccacgaaggcgcggccggtcaggaacttggccgcgctggcattgagctcttcgaacagaggcagcgcatcgggcgcggcaatggtcacggcaccgcgcgcggcctgcgggcgattggcctccatggccaggcgtgcttttttccacgcgtcgttgggcgacatcagccgggctgcgaccatgcggtcggcggcggtcaggcagccgtcgtccgcctctttctggctgaaccagctgcggcgcacttcgtcggcctgggcttgcgtggcattgccggagcgcagggattcgaccaggatggcgtagcagcgcacctgcgcgtcgtcgcccatgcggaagccggccacggcggatgagaaaccgtcccagtcgcggcgctggcccagcagcagcagccagtcgttgcgcagccggtcttcctggtaggtgccggggtagcgggcgaagaagtcctgcacctcgttgggcgcggcctcctgcaggcgggccttgagctcccagtaggcggcccagggttcgagcgcatggccgcgcgcctgcggcagcaaggcggccaggcgtgccttgtcgccgcgctggaacgcctgcttcatctggaccagcacgtcgtcgttgctgttggtttgtgctgccgcgggctgctgcgaaagcagcgcggcggcggccagaacggcggaaaaaaccagcgcgggcgctgcattgcgcgggcgacggcgcatgggtgccaaaatgcttgggaactgcatcgggggattatggacaagtcaaaggatgccgacacctcggcgaccacgagttttctcaagggtcaggtgcgaaaagcgctgatcgagcagcgcctggccatgcccgaccggctcgccagggccgacctgctgcagcgggtgatgcggatctggctggtcggccggcccgacaccgtgatcggcgcctactggccgatcaagggcgagttcgatccgttgcccgccctgcaccgctggaaagaagacggcgagctcatcgacgaaccgcagcgccgccgcatcgggctgccggtgatgaacaaggtgcacaagacgctgaccttccatgcctggtacccggggtgccagatggaggaagacgcctacggcattcccaagcccaaggacacggagctgatcgtgcccacgctgctgttcgtgccctgcgtgggctacagcgcgggcggctaccggctgggctacggtggcggcttctacgatcgcacgctggccgcgctggagccgcgccccttcaccgtggggctgggattcaccaacggctttctcgaagacttcgagcccgaggcgcacgacctgccgctcgacgccatcctgaacgacaacggcgtggtctggccgacgtcctgaccgatttcagtcgatgttgtcgaccgtatccgggtcgggcacctcgccgatggtctcgcgcgtggtgacggcctgggtctgcagccagtcccagaaggccttgatctccggccgcagcgcattgcgcggcccggcgatgagccagtagcccatcggcgaatccatgcggtgctgcggcagcacctccaccaggtcgccgttggccaggctttcggcaatgagtgaactgcgcgcgagcgtcacgccctggcccgtgagcgcggcctgaaccatctggtaggcatagttgaaatagagccagcgcttgggctgcgcccgttccaggccattgacttcgaaccagcgccgccaggtcagccattcgaggtgcgtgcggtgcgcatcgccggcctcgatcagcgtgaagccggcgatgtcggcgggcgtcttgatgggcgggctgcttttcaagagccaggggctcgccaccggcgtgagggtttcgccgaacaggcgcaccgccgtggccggcatggcttcgcgcgggccgtagcgcagggcaatgtcgacgtcggccacgtccaagtcgaccgccacgtcgctggcgtcgatgcggatgtcgatctccgggttgtcgcgctggaaggcctcgagccgcggaatgagccacatcgatgcaaaagatgcaaaggtggtgagcgacacgctcttgcgcccggcgctctggcggatctggcgcacggccgtatcgatgcgcggcagcgactgctgcaccgccagcagcaactgcgcgcccgcgctcgtgagttccaccgcccgtgtgtggcgcaggaacagcgacacgcccacttcttcctcgagcgactggatctggcggctcacggccgactgcgtgagcgccatttcttcggcggcggcccggaagttgagatgccgggcgacggcctcgaaggcgcgcaggtggccggccgagatgggccgggagcgcaggtgggtctgggaatgctgcatggatgacggcggcggcggcctcggtttcgattgatgcgaattcggaatcagtaggctacctcgttttcattggactgccaacggcacaaaaacgatcattcattcccgaactgcgctattgcctccgtctgtgccatcgcaattcggcaacgccaaggagtttcatatgtctaccgctgtctgcaccaaccaatcgctcgccaccctggcgcccgccgcccgtaccgctaccgccgttccgccggccgtgcgccgcggtgcctggcagattgcgcccggcgaggcgatgagcctgaaggcgcggtcggccagcctgctgcgcgtcaagcagggccgcgtctggatcacgccggacgccacctcggccgcccccagcgaagacctggcgctggcaccgggtgagtcgatgaccgtggccgccggccagcgcatcgtcatggaagcgtgggacggctacggcgccacctactcgtgggatccggcctgagtgccaggtttcccacagacggaaaggcggcttcggccgccttttttgttttcagacgctgatgtcgaagctggaccgcagcgccaggaagtgcttgagcgcggcttcgccctccagcgcatggacgcccgccatgaggtcggggccctcgctttcggccaggcccatgccgaagccggtgtagcggcgggcggccagcgggccgcggtagaccaccctgacgccggtgtgcctgggatcttgcgcgatgcggtgcatcaaggtttccaccgcgccctgcggtccttccaggtgctggcagaagcgcatgccgtcgaaaacgagcaggccggtgatgctgtgctgggcgttgcgggcgcgggcctgggtcacgatcgagccgaccgtggccggcggcaggtcctgcgtgagcatgctgcaataaaagacttcgtggagagttgcttcttctgtcattgcggtcgagagcggaaaacgtgcgaagtgtatgaacctccggtcccgtgcgaaatgtaaaaagacacagccgaaaagcctatagtggtgcgtgaaattcgaggactatctgcctacagcgtcgccgccccagggcccgaatccctgcgacgactgtgccttgcgccaactcgaagccttcttgccggcctcggcggaagaactgaagaccatcgagtcgtttcgcatcggctcccgccgtgttccggccggcggcgcgatcatcgaagagcatcggccgagcgcccagttgttcacgctctatgcgggatgggcgtttcgctacaagacgctgggcgacggacgtcgccagattctcaacttcttgctgcccggcgatttcatcggcctgcaggacgagtttgccgacggccagacgcacggcgtggaggccgtgaccgacaccacgctctgcgcgttttcgcgcgacaagctctgggagctgttccatgcgcagcccaggctgggctacgccatcacctggctcgccgcgcgtgaggaaaagctggtcgacgacaacctggtcaccgccggccggcgcaacgcaagcgagcgcgtcgccatgctgttgatgcacctgtaccgccgggcccagcgcgtgggcatggagcgcgacggctgggtcgagtttccgttcaaccagcagcacctggccgatgcattggggctctcgctggtgcacaccaacaagacgctgcgccggctgcagaacctcgggctctacaagctcgatgcgggatggctgcgcatactggagccccgcgcactcgaagcgcttggcgactacttcgagcggcccatgcgcccgacgccgctgatctagcagcgcggcggcttcgcattcatcgcgcggccatcgccagctgctgcaaatcgtcctggtaggcctgcagccgccgcaccgcccgttcgcgctggctggcgctggtggtgttgtgcagggcggccaggttgcggcagccttcctgcagcaggccctgctggggtcctggcggcgggtcggccatgcgcatcacgtaggcacggatggcggcacgcgcttcagccgcggggggcttggtggcattgaagccgcgcagcagttccagcgcctcctgctgccgcctgcggcgcccggcatcgatcagccgcgggtcgaacgccgattgcgccacctgacgccgcaccaggtcgcgctgctccggggtcagccggccatagaaatcttccaggcgatcgagatatttctcatagcgtttctcgtggacctcggccacgctgcggttgagccaattcttgcggtattcggcgttgttcttggcgtacttgcgttccagctgcaacagttgggcctcggtcaggctcagggccagctcggtgcccgcgggctccgcgcgctcggtcaccgccagcaggcgctcgcggatctggtccgccatgcggcaggcctgtgccgccgtcacgtcgcccggcgccattgcttgcgcttcctgcagcaggccgaccacgcgggggagctcgttctgccggtgccaggcccacagttgcgcgagttcgtcgcgcaccttgggcgtctgcgaaccgtcgaagtcgaggtaggcatcgagccaccaatagctcacctcgggaagattgttgtaggccagcttgaccgcactgcacgccccgagcacggcggccaccagcagcacaccgataattcgcgccaagttggcgccactcattcgggtagaaagaagcatgaatcagattccgcaggacaaccagggacccatcgacgtcgtcatcatggcggccggcaaaggcacgcgcatgaagagcaggctgcctaaagtgttgcatcgtttggccgggcgtgcactccttgcgcacgtgaccgacactgccgcccgcatcggcgcccgccatgtggtggtggtgaccggccatggcgcagccgaggtcgaggccgccatgtccgccagcgccgtgggcgccggcttgcagtttgcccggcaggagccgcagcttggcaccggccatgcggtgcagcaggcggttccgctcctgcccgacgacggcacggtgctggtgttgtcgggcgacgtgcccctgatcggcgaggaaacgctgcgcgcgctgatcgccgccagcgcgggcgagcggctcgcgctcctgaccatcgagttcgacgatcccacgggctacgggcgcatcgtccgggccgaagggcaggacgggcagggcgccggcgaagtcacggccatcgtcgagcagaaagacgccaccgaggcagagcgccagatccgcgagatctacagcggcgtgatggccgtgcccgcgggcctcctcaagggctggctctcgcggctggacaaccgcaacgcgcagggcgagtactacctcaccgacatcgtcaagctggccgctgccgacggcgtgccggtggttgcgcacgtcatcggcgatgcgctccaggttgcgggcatcaacagccccgcgcagctggcggcgctcgagcgggcgtggcagctgcgccaggccgatgcgctgatggcgcaaggcgtgcggctcgccgacccggcgcgcttcgacgtgcgcggcacactggcctgcgaggccgatgtcgagatcgacgtcaactgcgtgttcgagggctcggtgtacctgggcgaaggcgcgcgcatcggcgccaactgcgtgattgccaatgcacgcatcgaagcgggcgcggtgatccatcccttcacccacatcgacggcgaaaaggccggcgtgaccgtgggcgaaaggtcgctcgtcggccccttcgcccggctgcggcccggcgcccaactgggtgccgaggtgcacatcggcaacttcgtcgaggtcaagaactcgaccctggccgacggcgccaaggccaatcacctggcctatctgggcgacgccagcgtgggccagcgcgtcaactacggcgcgggcagcatcaccgccaactacgacggtgccaacaagcaccgcaccgtcatcgaggacgacgtgcacgtgggcagcaactgcgtgctcgtggcgcccgtcaccatcggcgcgggcggcaccattggcggcggctccacggtcaacaagtcgaccgagcccggtgcgctcaccgtggcgcgcggcaagcaggtgagctttccgaactggaaacgcccgcagaagacgcccaaggcctgatcgcctgcagcaagcgaacaagctgcgcgctcagggcgcgagcggcaccttgggttcgaacttcgcgcgcttgaggctgaaaaaagccttcacgttgcgcacgttggcatcggcggtaaagagccgctgcgccagcgcgccgtagcccggcatgtcgcgggcggccaccaccagcacgaaatccggtcccggcgagacgcgccagcactgctgcacggcgtcgtccgcgatcacgcgcgcctcgaaggcgtcgagcgccgccgcgtcctgccggtccaacgaaatctcgatcaccgcctgcagcccgtggcccagcaccgcggccagccgatcgggtgagagcagtgcaatctggcgctcaatgagcccctcttgccgcagccgctgaacgcggcgcaggcaggtgggcggcgaaatgccgacctcggcggccagacgctgattggtctgcgaggcgtcctgctgcaaggcgtcgagcaggcggagatctattgcatcgagggaaattgattccataaatgaacaaattatggaataaaaaaccgggaagatggacgggtgaaataaaaattcaaaatcaatgaaattgcgagcgcatatttttcacgctgctctctaccatcaggcctcctcttcattcaaaggcagctcaccatgtgcggcatcgtcggcgcagcgtcccatcgcaacatcgttccggtcctcgtccagggcctccagcggctcgaataccgcggctatgactcctgcggcgtggcggttcatgcgggcggcctggcgcgggcgcgaaccacctcgcgcgtggcggatctcgtcacccaggtgcgcgaagaccatgtcgaaggcctgaccggcatcgcccacacgcgatgggcgacgcacggcgcgcctgccgtgcacaacgcgcacccgcatttcagccacggccccggcaccgacgcgcagggcacgcggcccggccgtatcgcgctggtgcacaacggcatcatcgagaaccacgaagtgctgcgcgcggcgctcgaagccaagggctacgtgttcgagagccagaccgacaccgaagtcatcgctgacctggtcgacagcctctacgacggcgacctgttcgaggctgtgaaggccgcggtgctgcagctgcacggcgcctacgccattgccgtgatctgccgcgacgagccgcagcgcgtggttggtgcgcgtgcgggttcgccgctcatcctgggagcgggcaaggagggcggcgagaactttctcgcgagcgatgccatggcgttggccggtgtgaccgaccagatcgtgtacctcgaagaaggcgacgtggtggacgtgcagcccggcaaatactggatcgtcgaccgcgaccacaagcccgtcgagcgccaggtgcgcaccgtgcaggcgcacagcggcgcggccgagctcggcccgtaccgccactacatgcagaaggaaatcttcgagcagccgcgcgccatcggcgacacgctcgaaggcgtggccggtatcgtgcccgagctgttcgacggcatcgggcaggacggcgccaccggtgccagtgcataccgagtcttcaatgacatcgacaagatcctcatcctcgcctgcggcaccagctactacagcggctgcaccgccaagtactggctcgaaggcatcgcgaagatctcgacgcaagtcgagatcgcgagcgaataccgctatcgcgattcagtgcctgaccccaagacgctggtggtcaccatcagccagtctggcgaaaccgccgacacgctggccgcgctcaagcatgcgcgctcgctcggcatggagcagacgctcaccatctgcaacgtggccaccagcgcgatggtgcgcgagtgcaagctcgcctacatcacgcgtgccggcgtggaaattggcgtggcgtcgaccaaggcattcaccacgcagctggccggcctctttctgctcaccctggcgattgcacagagcaaaggccgcctgagcgaagccgacgaggcgcgctacctgaaggagatgcgccacctgcccgttgcgctgcaatcggtgctcgctctggagccgcagatcatcggctgggccgaagacttcgcgcgcaaggacaacgcgctgttcctcggtcgcgggctgcactatccgattgcgctcgaaggtgcgctcaagctcaaggaagtgacctacatccacgccgaggcctacgccgccggcgaactcaagcacggcccgctcgcactggtcacgagcgagatgcccgtggtggccgtggcgcccaacgacatgctgcttgaaaagctcaagagcaacctgcaggaagtgcgcgcacgcggcggcgtgctctatgtgctggccgacggcgacaccaagatcaagggcagcgaaggcctgcacgtgatccgcatgcccgagcactacggcgcactctcgccgctgctgcacgtggtgccgctgcaattgctcgcctatcacacggcctgcgcgcgcggaaccgatgtcgacaagccgcgcaatcttgcgaagagcgtgacggtggagtgattgcgaggggcggtgggtgggccgggtggttgttctttgccacctgcgtccgcggcagggagcggtccacttacaggggagacaacacccaagggctcctgtcatcagtcatgagatcttcagcaataccggtaattccgcctagcgtcatgttctggcctgcccaactggcccgaccaatgatgtagctctttgcaaattgtggccaagacgaaaaattcgaacgtaattctttatccacatgcgcaagaatacggctgaattcattcggttcaatgtatttgcagtccagtgccattcttgcaacagtgacgagtcggccgagatcccaggcaagtattccagcaccgtaatccttgggaaggtacgagccattaaccttgtcttcgagaaggcgaaaaacggatcgcagattctccagcatctccatagcctgctccaaggccgagaaaacgagatctttttcctcgcatggcccctgtgccgtaatccgattgcgcactgtttccggggagccgtatcgaccgctggcgatcaatgcctcgagaacctcttggcgcccctctcctgaagcaccatcgctgtaaactcgaaaaacaatgtcgtaaaaaaagcgatggccatagcgaccgagtgactccagagtttcagcagcctgctgaggtgagcttatattccaatgtgagccaagcccctcggcgagagtattgtgagacagtccagttgtgcaactgtcgcaatacgccatgatctgctcggagttgatgagcccagcttgaagtgctcgctgcgctatcggatccaccgcggccccgtcggggcaacctctgtattttttcccagaaactatctggaatagtttcttcaagaaacccataaattagatttgcttgaaggcggcattaacggcgcgatgcttgagtgcattcacaagaatatcaaagtccgaatctttcgccatgtgaatggcatcgaattcatgctttttagatgccattgacggcgcactaatttctactgttttctctgcgctcgatgttgaggtttccgggatatctgtgatggtgattttatcgattgcgtcatagctcagagtagtcagtacgccagcgaattttttaacggtcgtgaaagacatgctcttctcatcaagaacaatgctggcgccttggctattggcggcgcgcttcttgaaaagtgttccaactgtaagatacgtggcataaaccccgaatagcatgagggcgccattggccacgcctgccggcaggtgaagccgcagggttcctattttcagatcggcaatcggataaaaaattgcggcaatgataattgccgggccaataagaccgaaaacatactcgagaatcgagtattccattttatagttaatggtttgcatgtagtatatttacttatattgtgattttgactgggcggttggcctggtcggtaatcggtcctgaaaaccgcagactaatgtaacaaatcgcgtccctgtgccgccagcctgctgtacctccaacacgcctacaagctcagcgacgaagagttcatgcagggctgggccaagaacgttgcgcctgtgcagacaaccctggggtcgccggagaacgtgcctagcccctggattgagcggacatgctccggcagaggcttcgcccacctccgcatgccgctcatgtcgaccgccagacaccaggaacacccaatgagaaagctatccactggcagcattgcctttgccaagactcatgtcagcgcaacgcgagaccatggtcgatttcttcacgtctcccctgttgatcaatgacagtaagacgatccgtgcgcaatatgtgcatcgcgatggcggtgagctcacttctggctgcttgcggttcacacgatccccagccgcccgagcgaatctcacccgcgcctgcggcctacaacacggtgatagtggcgccagtcgcgtacgggtattaccaaggccgccagatgtctgaatccgatgacgcgtgcggcgtgccggacctgttgcgtcaggcggtgcaagatcagttgaaggcgcgagatgaggtcgtgctccccgtgctgagtcccggtagggatgcggcccctttgctgaggatcgaaatcatggacatggtgaccgtcagcgccggcggccccacgatggtggtcatccatgctgtgctcgaacgaccgggactgccaactgcgcagttcaaaggcctgcgccagatgcacacccaatactctgatatcacggcggacaccaccgaatgcagctcaatggatgaagtgattcacgggttgggtgcggacgttgcgaaatggatgctcaagccggtggacggggtgtctctagtgaacggagagtgagcaacagccgtcattcacagttccatttctccttctgaccactcgccccactcatacacaaggaccaccttgatccatcacgttcgtacggtcctcgtggcctgcgcattgggcaccacggtgctggctgcttccgcccagataaaaattggcttcatcggcacgctgtccggaccggcggcagcgctcgggcaggagcagtacgacggcttcatgttggcggtcgagcaacgacaaggaatgctcggcggtgtccccgtgacggtcatcaagcaagacgaccagcacaaccctgagctcggggcgcagctggcgcagagcctgatcgagaaagacaaggtcagcttcatcaccggcgtgacattctccgacgtgatgatggccatggccaagccgatggccagagcgggcatgctgttcgtcggctcgaatgccggccctgcgtcgattgccggcaagcagtgcaacagaaaattcgtcttcgcctcgtatcaggacgagtaccaggccgggatcgtgggacggtacgcggtcgatcagcgttactggaagacgctgttcctggcgcccgacggcccgtcgggcaaggatcagctgcggggcttcaagcgctactactcgggcgaggtggtcagcgaaatctacgtccagccccaccagaccgactacgcggcagcgctggcgcagatcaagcgcgtcgcgcccgatgcggtggttgccttcttgcctggcgacatgggcgtcaacttcatccagcagatgaatcgctcgggcctcctgaacaaggtgcccctgctgacggtcggcacggtcgatggcacgacactgccgctgctcaaggacgccgcgctcaatgtgctggcaggcgcggtctggggccccgacctgccgagtccgaccagcaaggccttcgttgccgccttcgaaaagaaacacggacgcatcccatcgcactacgctgcgcaaggtttcgacgcggcgctcttgatcgacagcgcgctgaaggagaccaagggctctgtcgccgatcgcgatgccttgcgcaatgcactcaacgaagccgacttttcgtcggtgcgaagtggcttcaagtttctacgcaacggtttcccggtccaggacgggcacgtcttcgttgttgcgaaggacgcgcagggccgcgcgtcgctcaagcggatcgccacgccgctggaggcgaatcctgattggtactgggacgagtgtcggtagggttggtgatctcatcatcggcaggcgaggtcgaggccatcgatgacaaccgggcgcagagggcgcatggcatttgaggtggacctctcggccaatgagcggacgcatcgggcggtaaagtcgcatccgaggatgccgcctcacgttgccaaagagttaaaccaggagcttcaccatgtcgttcgtccttgacagtggctgcctctgcggagcggtcaggttccacgtcaatcaggcgccgctcaaaacccttgtttgccactgcactttctgtcagcggatgacaggctcctcgttctacgccaactctgtgttccccgttgaggcagtcgagttcaacgatggcgaggtacgcaagtacgagcacacatccgatggaagcggcaggaaggtctacgttgagttttgcccaacttgcggaaccaccatcggccttacctttgagcgctggcccgatctccgagcagtgtcgcggggctgctacgacaaccccaacgtggtggacgtaacttcgaacatatggacccgctcggctcagtcaggagtcgctctgcccgccgaggttgattgcttcgcaagggcaaggctgacccccgaggggcagcccgagcaggcttccaagtacccaaatccagtcatggcccggtagtacttcagcgatgccttagccagcgtcgcgagattgggccgcgctgttctcgcgttccttttgcagccccggcggttcccctccgaaccacatccatttcggatcggtcccaccgtggttaagtccgaactgattccagccttgccctatgacgatggccatcgccaacaacgccagcacgatcacgatcgcgcatccggcataggcgatcaccgtgagggtgggggtagcggggaatagatcggcccctgccaccgcgacgatcgcagcgagtgcgacgcatgcaatgagggacttgagcaccagctttgcattcatgcgaatgttcctttccgcgtagagaggtgaaacaattatcggcgcggtggccgttcgaccgtcattcaggttgcgattaggggcgcgtatctactgatcagttgctcgcctggtagcggccggtcgcgacctcggagtttcgggcctgctgcagacattcgttctcctcaaccggacttggctttggcactactcgcgaaggtcggctttgcggccgcctaggccgcagcggtaaccgacgggttctggccgcttgccgctatgacgcttgcggagatgccggatggcctgtgaccagaacgaccagcgcatcggtctcgtagaagtcgctcagcgacgcggtcggttcgctgtgcatcgctggcatgcacgcaagaacgcatgcgggtgctgctaacagaactgccgcaagtgatcggcggaaagccgataggttggtgctgccccctgagggagcggcaaggctctcagcacgattcttcatgatctccttgatgaccgcctggccggccgggttcagcctttagcccccaggctgcgggtccgcctcaaatttctcgcgcatctcgagatatgccttcttgcaatgttcgaagtacgcccgctcgtcatccgccatgcgctcagcctcgcgccccgaaatcaccgggtcagcttggtcagtctcgaggatgcgtatcgtcaccacatctccggtctgcaaatcggcacgcagccagtccaaatgctcgtccgccgcaccgttcgcgcgtgccgtcagtccgcccacgcgcagcgtgaaatcaacggttccgtcagatcgccgaggcgccgcttcaggacccagctttcccaatagggaaatgccggcagagagcacacacaggtcagaggcgccacccgtcaccgtcttctgtccgttaatcgcgatttccaaggcgtacatgtgcgaaattttgaatgattgaaggacgacttgagcgtccgactttggccgactgtagcctcacgaaaggtcggcgcaaagggctcgttgccaacgttctaactcgacattgccattcaaacgactgatagatcgggcgagagtagatcgcacggcggcggaagatgctccgctcgtgtgctccatatagaacctcgctgcacaaagcaagccaaacgagcgctagccacagcgtctcagactttatttattggcaaacaacggccggttgttgcggccgatcgacttgtctcggtatcgacccatgcacccgccggtcgcggccgttgcgccttctcgcgttggatatcctgcacacggcgagggtgtgcatactgcgcccatgctcgtgccgtccctgatatcgcaccttcggcccgcccgctgggtgggtgcccttctggcgttcacaagcctgtccgtgcatgcggatcccgccgtggatttctttcgcgtgctgggctggactgtggccatgggtttgggagagatcgtggcttgggcgctggggctggggttcgtcttcctgatgacgatcctcgtgcccggcgcgatcgtccgggcactggtgcgcgcgccgctgctctgggcgctatgcctgctgatggtgcctcgctggcgcgcgggaccatggggctggagcagcatcctgctggggctggcaaccgccgctttgggcgcctggctgatcgagcgccgttggcatgacgacgacgtggatgttgaccttcttgattgacacattgggaccaaacgatggatttgcttcgcagggcaattgcgcttgtcatcttcctcggtgcgacctacgtcgcgatcgagatgcgttcgggcggttctgcgctgggagggatctttttcatccccgcagtgcttgtcgccttctttgcgctcgccgtcgtcatattcaacctcccgatcctgggacaagcccggttcgaggacagcggtttcgagcgcaccgtgctgtcgccgtggcagttgaaggtcttcggcattttcctggcgctcctcttcgggggagcgcctgtctacattgccgtgcgaggcctcttcaaaggcatcatccccgctccgtggagcgctccggacatcgtgctggcgcaggcgccactgcaattcctgctcgcgtgtgccgtctttgccggaggaggcgtactgctcgcagtgctgatcgtgaagggaatctggcgaaccagtgttccgtcccggtgattcggccgcatgggcgggcaagcgcaatgaccacaggaagcatctgaatctccgggtctcaaggcataccaggtcaacggctgcagcgaatggtccaaaacgcaactttgccaacagccgttggtggggagaggccgctcaactgccggctcagaccccttcgatgatccgcaggtcccgttcggccccgtcgcccagcgcggccagtgcggcctggtagtcggggctgtcgtgcgcggctctggcctgctcgacgctgtcgaactcgatcaacacggtgcgttggagcagaccgaactcgtagacctcggcgggcaggccgcgcgcaagaaagcgcccgccggcggcggtgagtgccggcccggccagttttgcgtacgccgcaagtttgtcggcgtccttgatggcacggtacgcgctgacccaataggcttttgccatggtgatttctctcagttgctgagcgagcaatatagcctgcgcttgacgttggctgctgccatccgtcagcgcttctcgtcctcccagtccacccaatccaccgcatgggtctcgagatatcggctgacggtggtaccgatggtcggaaagaacgccgcatccccaagccgctcgaaaagcccgaaccgcttcagcttgtccttgacgggatccttcatctcggcaaagcacaactgaatgccggtcgcgtgcagggtttcgatcaactcggccagcatgtcggcggaggttacgtcgacgctggtgattggttctgccgcaacgaccagccagcgcacaggcgtaggcgacgaagccacggcgtccagcacccggtcgtggaacagctcggcgttggcgaagaacagcggcgcatcccagcgaaacaggacgaggccggggataaggcgcgcgtcgggatagcgcgtgatgtcgtggtagcccttgacgccgtcggcgcgccccaggaccgcggagtacgggcgccaggcatcccacaggaattcgatgatcgcaatcacgatggccaggccgatgccttcgaccgcgcccagcacggccacgccggcggtacaggcgatcgacagccagaactcccagcgctggatgcgataaattcgccgcaggtcggagacctcgatcaggccgatggccgatgcgatcaccaccgcggccagtgcgctggtgggcaggtttttcagcaggtccggcaccgccaccagcagcagggcaacagccagcgcgccgacgattccggtcagctgggtcttggcgcctgcggcctcggccacgggggtgcgtgacgaactgctgctgacggcaaagccctgaaaaagtccggccgccaggttggcggcgccgagcgccaccatctcctggttcgggtcgacatagctgcgggtccgcgccgcatagacacgagagagcacgctggtgtcggcgaacgagacgagagcgacggcaccaccgccgatcaggacggggacgatgtcggcggtggtgatccacggaatggcgaacgcaggcaggccttgcgggacctcgccgaggaccgacaccccggcgcgtgccgcaaggtccagcacgccaacgacaacggtcgctcccaccacggcgatcaggatgcccggcaagcgtttgcggcccttgagcagcaggatgacggccagggtgcccgcgccgaccatgaaggtggtccagtgggtcttgccatccatcacggccgtagcgatggccctcaggtttcccaacggtccgtcgccctcgatcgaaaagccgaaaagcttgggcagttggctgatcaatactgtcagcgcaatgccgttcatgtagccgtagcgaatcggcttggagagaagctcggtgacgaagcccaggcgcgcgattccggcaaggatgcacaccgttcccgacacgatcgccatcatgcccgccagggcgaccgcgcgatgcgggtccccgccagacaatggaaggacgacggccagaatgacggcagccaacgaggaatccgggcccagcaccagaatccggctgggcccgaacacggcgtacgcgagcaacgcaacgatggttgcgtagaggccatagatgccgggtacgcccgatgcctccgcgtaggcgatgccgacgggcaccagcatcgtggtcagcaccagtccggcaacgatgtcgtgccgcagccaggccacctggtactcgcgcagcgtgcgcagccccggcaaccagcggctccagccggcctgatcggcggccttcgtccgccgcgcaatacggcccggttcggggaggggggacgaaggatccgtattgctcataagccgctgccgcttggtagagcgtgcagatgcgcgcaaagaaagacaagaggaaagatccgggtgctgccggcccctccgcttcgacgcgatggtccatcgacggacagggtcttgatgaagattccgattgcgttgaaaataatggtgtaaatcatttacaccataatcgaaaatcctcaatgactgactttggcatgaccaacaacgaaatgacttccgcgcccagcgacgcaaccgacccgacagtgaccgcctcgacggtccagccaccggcagagtcgacaacgcctgccgcgccgcaactgccgtcgaacccgccaaccgccaagccggttgcacgcaaaaggccagcggccaagaaggcgccagtgcgcgaacctgaagcagccgcaacgaagaaggcggccgccaagaaggtctcgcctcggaaggccacgccggcaaaaccggtggttacgaagtcctcggcaaaaaaggcagcggtgaccaagaaggcagcggtgaccaagaaggccgcagtcaccaagaaggcaacgccgaccaaagccggcgccaagaccaccgccgcacccaaaaagttgacgtcagtgaagaaagcatccgtgaagaaggcactagtaaagaaagcatcagtaaagaagacagtggcaaagaagaccgggccgctgaaggccaagacggtgcaggccgtcgtcgcgccgcctcaggtcacccggcctgccccccgcaaggaactggcgacgtctttccaggccacttcctccgagtccgcccgcgacgcggccaagaccaaaggcaaactcgtgcgagacagcttcacgatgccccagcaggacttcggtctgattgccgtcctcaaggaccgcgcgctaggtttcaaacgcccggccaagaagagcgagctgctgcgagccgggctgtacgcgcttcagcaactcaccgacacccaactgcgcggtgcgctggattcgctggcgccgctgaaggctgggcgcccgaagaagtaagccaaccgaaggccgcgcggcgttcctcccggcatcggcgatgcctgtgccaggagggcctgggaaaagcggatgcgtgggtacacaatgctttcatggcgcagaagaaacctcccgctttccagcccctgaccggcatctatgagccgtcggcgatccagcagttgccggatgggcgctttcttgtggtcgaggacgaaaagggccatcccttcagcctggtcgtgctcggcgccgacggaagtgtcgacagcaccgaactcaccgccgggctgtttcagatcttcagcgacttctggaaactggatgatctcgagggacttgccttggaccgcgcaggcttcgtctacgcgatcacatcgcattcccgagacgacgaaggcaacgaaaagaagtcacgtgaacggctggtccggttccggatcgaggggaatcgcgtcgaggaccccaaagtcgtcgacggattgaagcgcgccctgatggcaaagcatcctgaactggcctcggcagcccagatccgcgacgtcaagaccggcggcgggctcaatatcgaagcgttggagatcggcccggaccagcaacggctgctgatcggctttcgcagcccgttgcgcaacggccgcgcgatcatcgccagcgtcgaaaatccgcaaggcctcttcgaggcggatgaggccccccgggtggcggctgatctcgatgagctggatctgggcggccacggaattcgtgggttgtcttacgtccccgccattggcgagtacctggtcatcagcgggccgatttcgcgcgacccgggccagttcgccctttggcgctggaatggtcggcaaggtggcgcggcgcgtcgagtcacggttccaggccttcagggcctggggcgcgcagaaggggtgagcccggccgtcatcgacggggtcgaccgaatcatcatcgtcagcgacgacgggagccggaaggcaggacgatctgcgaattatcttctgctggacctcgatcagctgcaaactgcgcattgaatgggcggctcggcaggagcctcgcatcttgccgccgggcggtcgaagtcacatgcacgtcagagtgcaatgcgaggatatgcattgacggtcgcggacgctggtagggaatgcaatttgcacctcgaatcctgaggttcccgatgttcgcggccgtctctacaacaagtctctgtcctggctcacgcgcgccaggcgcgttgcccggtcggaaaacaggggcgcattggaatagcgcagggttccgcacgtgcgggactcgtcgagctgcagttgctgcaccgcgtcacgaagctgaagaacatcggcatcgtctgctccgtacaaggcctgcattcgcacgagaaggtgctgcaggcgggcttgatccttgctcatcgaatcgtccttatgggaaagatgggaaagttcccggcgagattgaactgccacccctgcgctaagctccactctatatgtcaacagtggacaaggtccgagtcatttttgtttcgaagcgcaactcgcttcgaagcgttcttgcacatgcgtgcctcgaacacgtaggcggtgaccgttatgcggccctgtcgtgcggctctccaaagcacctcgccagcgaaattcatcccgctgcgctcggcgcgctggcaagcgcccggatgcgaccgcctctcggaattccaataagttgggagaggttgaaggagcggggtgccgccagagccgcgttcatcatcacgctggacgaggagacgatcggggcccagccggcatggccggggcaaccggataccgcactttggtcgatgccggacgttgccgcatcgggagatccagaaaagacggcctacggtgcgatccaggccctctacgctctgcgtcgaagactcgagttgttcgtcaacctgccgctgaccaagggcgaccgggtgtctctccgagccgatgtccgggatctgggaaccatgagataggccggttggccctcagccccacgcaggaaggttctgcaacgcgtcgttggggcggccgacaatgtcgacgccggtgatgccggttccgcccggcaagaggttgacgtcgcaaatgacttcccaggcgtggctttcagtgcgccgtgcaagacacacttcctcaccggcggcaatgagctctgcgcactcgccgacgctgattcgctgtgccgtgccaagggcgaactctgtcgaaccgaactccttctccacaaccgggtgaatggcgacgagatcgatcttttcgtctttgaagtgaacagcggtaatcgcatgctgggacatctttcgacctccattcgtggagagccccgacatggccgcggcggctgccggcaccggtgggctcgatcatcgactgtacgccagctcccgcttgctcgcactcggcagatgaacccaatcaggaggtgggcgggtcatcgccagtgagcagcaacttcgtttcgatgccgtagagcgcaagcatgcccagcacgtgcccgatggcgacgcccggttcacccgattcgattcgcgcaaccgtctggacatgcacgccaagtcgggcggccgctgcggcctggccctcgccggcattggtgcgagccaacttggccgcagcacccatgtgcttgatcgcctgaagggcgccgctgtcgatgtccgccgagatgcgtttgccttgggccataggaatattgtcgctgcacaatccgggccatgcctcgaaccttgaccgacaccgggcccgtgccttactggctctacctcctggaatgcgaaggcggcgtgtactacacggggatcgcgctcgatgtggagcagcgcttctttcagcatgtctttggactgggcgccaaattcacgcgcgcgcgtcctccgttgcgagtgctcgcagcccgcgcctaccctgacaagggggctgcgctgcgggcggaaatcaaggtcaaggcacttcctcgcgcccggaagcttgccttcttcgaagccctggcgtgacgcgccggattcgagtctgcagcccctctgcatcccgagaaatacgcgattgaccgactgcgctttcgcctgaaattcgctaggctttgctggcgagcgatcccatcgagcgcggagacaacgcgatgagccagggcgcatctcttcgtctgcatgtgccggagcccaccgggcggccggggcacgagaccgatttttcctacctccatctgtcgcgtgccggcgaggtgcgaaaacctccgatcgatgcattgccagccgacaccggcgacctggcctacacgctggtgcgcgtgctcgacgacgagggccgcgccgtcggcccatgggtgcccgaggccgaccctgaactgctgcgccgaggcctgcgcgcaatgatgaagacgcgcgccttcgatgcccgcatgctgatcgcgcagcggcagaagaagatctcgttctacatccagtgcctcggcgaggaggccatcgcgaccggccacgcgctcgcgctgcagcagggcgacatgtgctttcccacctaccgccagcagggcctgctgctggcgcgcgaagacgtgacgatggtggagatgatctgcgagctgatgtccaacgagcgcgacccgctcaaggggcggcagctgccggtgtgctattcgatgaagagggccggcttcttctcggtctcgggcaacctggccacgcagttcatccaggcggtgggctggggcatggcttcggcgatcaagggcgacacacgcatcgcctcgggctggatcggcgacggcgccacggccgagtccgacttccacaccgcgctgactttcgcccacgtgtaccgcgcgccggtgatcctcaacgtggtcaacaaccagtgggcgatctcgaccttccaggccatcgccggcggcgaggccaccaccttcgcggcgcgcggcgtggggtgcggcatcgcctcgctgcgcgtcgacggaaacgacttccttgccgtgctggccgcctcgcgctgggccgcacagcgcgcgcgcagcaacctcgggccgacgctgatcgaatgggtgacctaccgcgccggcgcgcactcgacctcggacgatccttcgcgctaccggccggccgacgactgggcgcactttccgctgggcgatccgatccctcgcctggcgcagcacctgacaacgatcggcgcctggtcgcagcaggagcacgaccagacgcgggcagacctggaggcgcaggtgagtgccgcactgaaagaggccgagcgcttcggctccatggccgacggccacgttgccggcgccgcgaccatgttcgaggacgtctacaaggacatgcctgaacacttgaagcggcagcgcgaacagctgtcgtcggagggatgacgcccatggcctcgatgaccatgatccaggccctgcgctccgccatggacgtgatgctcgagcgcgacgacaacgtcatcatctacgggcaggacgtgggctacttcggcggcgtgttccgctgcaccgagggcctgcaggccaagtacggccgctcgcgcgtgttcgatgcgccgatcaacgagggcggcatcgtcggctcggccatcggcatgggcgcctacggcctgcgcccggtggtggaggtgcagtttgccgactacgtctatccggcctatgaccagatcgtgtccgaggcggcgcgcctgcgctaccgctcggcgggagatttcaccgcgccgatcaccattcgcatgccttgcggcggcggcatctacggcgggcagacgcacagccagagccccgaggtgctgttcacgcacgtctgcgggctgcgcacggtgatgccctccaatccgcgcgatgccaagggccttttgatcgcctccatcgagaacgacgatcctgtcatttttctggagcccaagcggctgtacaacggccctttcgacggccaccacgaccggccgctggtgtcctggtcggcccacccgctgggcgaggtgcccgaggggtactacacggtgccgctcgaatcggccaccgtgttccgccctggcgccgacctgacggtgatcagctacggcaccatggtcttcgtctcggaagcggccgcgcaagagaccggcatcgatgccgagatcatcgacctgcgcagcctgtggccgctggacctggagaccctcgtcgcctcggtgaagaagaccggccgctgcgtgatcgtgcacgaggccacgcgcaccagcggcttcggcgccgagctggcggcgctggtgcaggagcattgcttccactacctggaggcacccatcgggcgcgtggccggctgggacacgccctatccgcatgcgcaggagtgggcctatttcccgggcccggcacgcgtcggcgccgcattccggcgcgccatggagaactgaatggccacgcatgcaatcaaggtgccggacctcggcgaaggcattgccgaggtggaactggtggcgtggcgcgtgcagcccggcgacacggtggccgaagaccaggtgctggccgacgtgatgaccgacaaagccaccgtcgagattccctcgccggttgcgggcaaggtgctcgcgctcggcggcgaagtggggaagcagatggcggtgggcgcggagctgatcaggatcgacgtggtggaccgcggcggggcggaggcgatgcggggtgcaccagcgccggcatctgcacctgcaccaacgcaagtgccggccccggcgccggccgcgcgtgcgcgcccatcggctggcaagccgctcgcctcgcccgcggtgcgccatcgtgctgcgctcctcggcatcgatctccagcaggtgccggccagcggcgcggagggccgcatcctgcacgaggacctcgatgcctggctggtgcggcggcccggtccgcaggcgccgggtgcggcgcgccatgcagagcgcaatgacgaagaggccgtgcccgtggcaggcgtgcgccgccgcatcgcgcagcgcatgcaggatgcgatgcgccgcatcccgcacttcacctacgtcgaagaggtcgacgtgaccgagctggagctgttgcgcgcgcggatcaacgaacgctggggcgccgagcgggcgcacctgacgctgcttccgctgctggtgcgcgcggtggtgctggcggtgccgcgcttcccgcaggtcaatgcccgattcgacgacgaaaagggcgtgctcacgcgccacggcgcggtgcatgtcggcatcgcgacccagacttcggccggcctcatggtgccggtgctgcgccacgcggaagcacgcgacctctggtccagcgcaaccgagatcgcgcgcctggccgatgccgcacgcgccggccgggccacgcgcgacgaactgagcggctcgaccatcacgctcaccagcctcggcgcgctgggcggcatcgcctccacgccgatcatcaacgcgcctgaagtggcgatcgtcggcgtcaaccgcatcgtgcagcgcccggtgatgcaaggcggcgcagtggtcgcgcgccgcatgatgaacctgtcctcctccttcgaccaccgcgtggtcgacgggcagctcgcggctgaattcattcaggccgtgcgggcttcgctcgaatgcccggcgctgctttttatcgagtgagcgtcgagtgagggaggctggagcgcgagcctcaattcgttctcctccagagggttcagctcgagcaccaggcgcctgaaatcagcccggtagcagggcagcatcagcgccgccgtgaacgcatgaacgccgtcgccgcgcgccatgcattcatcgcacgcggcaatgcttcggtagaggccgatcgcctgtgcgactcggctgtcggtggtgctgctcttgcgggtcatcgccggctccttgtagcgcgccctggatggcccgcgaggcgactctatgcactctggagcgcagcggtgagtaacaagatcgtcgtgaattgaggcattggcacccggtgccgcgacaatcgaaggctccttgcaatgattgcctccatgcctcccgatcagttcaccgatcccgtcgaaccgacgcctcacgattccgacgcgcaaagcgcagccaaggccggccgcctgcgcgcggaagccgacaagctcgaagcattctgtgtcgtcgttcgcgcggcttcggccgcagtcgatcacgccgcgtttgtcgaggtcagccgcgcagcgtcccaggcgctgcacgccaagttcggcggtggctcaatcacttcggtgttcacatggttgaccgggcctgcgggaagcgccgcgctaaaaagcgttcttgccggcgaagtggagctggccgggccgctttccatccagcagatcgtcgaagcgattgagctggccaaaaaggcggagttcctgcgccagaagcgctgagggcgcaccgcccgtccgtccgccgcgcggttcagcccgccatcgcgcggcaagcggccgcgcagtcccggcatgccttggcgcacgcctggcagtggtcgtgcttgtgcttgccgcattcgtcgccgcaggcttggcagatgtcggcgcacagcgcacagatggccttggcaaactcgctgccacgtgccatggtggcagccgcaaactggcaggcggccgcgcagtccatgtcgagcgcgatgcacctggccatcatcttgacgtcggcttccttcaggcaggaggcggcgcagtggttgcacgcggtggcgcagccgttgcaggcttcgatgcatgcggcgtaggtttcatgtggcattgctttctccttttgggttggacgctggcgacggcaagggacttgcaggaagcagcgatcaacgcaatgtcgagctgagcgagcgggcggcctccagatgcgagcgcagcgtcggcagcgtcttgcctgcccaggccctcaactcggggtcgcgggcctcgcggctcgcacgctcgaagagcgcgatgtccgtttggtggtcttcgatacccacgagccggatgtacgtgcgatcgaactcgtcttccgtggccgaagccaggcggttcagcttggcgtatttgccacgcggcagcacgccggggagtcgcattcccctgtcgcgcaccagggccctgagttcgttgttggcgcgtgtgtggtggtcgacgagcatctgcgcatagcctcgcacctcggggctggcggcgcggtacatggccaaccgcgaggcctggatttcgtaccggccattgcccaccgccgcggtgatgaactgcgggtcttgaaggccgctcgtccgcgccgcgcccgcggtgccggcgcgcgcaaggggctccggcagagtcgagcaccccgcggcgagcgccgccatgccaacgagcgtgagcgctcgcagaagggtttcgagcgttttcatggttctccttgtcagcccgcaatgcgagccttctcggcgagacgcagaaaatctaagccaggcacgcccggtgccctgtcggacggtagctgcatctgtggcctgacaaccactcgtggttgccgcacttcgctcactgcggagggcagggacgcgcctcagggcttccggtgcttcagaaagcccggcgcgttttcgcccttgccgggctgcgcttcgtcgctggccgtgtcttccacgttggtggactcatccagctcgaggtctctcgcgcgcacctcggcttcgagcggcagcccggatgccggctggtgcgtcatcgggtccgccgatgtggcgggcgcttgtttccgattcatgtctggtgctcctgttgatcgccagtaaccatcctctctgccgcggggctgtacgggcaatcggacggaatgagcacgcggtgcaggcgatgtcctgcgcagcgtctggtaacagcgcccgcgagccagcggtgaaaatccatcgatgcatccaatcagtaccctctttctgcgttccggcagcttcgcgctcctggctgcgtccgcggccatggccgcgctgctggcaggctgcgcggccgctccgtcgacaccggccgcctcaggcgccaagccggcggaatcgacaacaggtgcacggcctgcaattgcgcccgctgtgccagggcaggcggcgccggacgatgcggccatcgaacagcggttcgcaaaatgggttgccgatttccgcgccaccgcgcgtgcgcaaggcatcggcgaggcgacgctgcgaagcgcgctcgatcaggttcaatatctgccgcgggtcattgaactggaccgcgcccagcccgagttcacgcgcaccgtctgggactatctcgacaacgccatcacgccccagcgcgtggccaccggtcaggacaagttgcagcaggttcgcgctgaagccgatgcggccgccgcgcgctacggcgtaccgcccgccgtggtggttgcgatctggggcatggaaagcaactacggcggcaactacggcaacaccccggtcatcgatgcgctggcaacgctcggcttcgaagggcggcgcgaagactgggcacgccgcgagttgcttgcggcgctgaagattctcgacagcggcgacatcgcgcgcgaccggatgatcggctcctgggccggtgccatgggccagacccagttcctgccgtcgaactttctcgcctatgcggtggatgccgacggggatggtcggcgcgacatctggggcagcatgcccgacgtcgtcgcatcgactgcgaactttctctctcgttcgggctggcaggccggcgtgccctggggcgcggaggtgcggctgccggcgggcttcgactacggccgcgcagacatggctgtgcgccagtccagcgcgcaatgggcggccgaggggctgcgcgccatcgacgaccagccgctgccagagcttgccgatgccagcatcctgctgcccgcgggtgcccgtggcccggcctttttgatcgggcccaactttcgcgctgttctgcgctacaacaactcgaccaactacgcgctcgcggtcagccttcttgcgcaacgcctgggcggtgggccgggcgtgcagtcgccgtggcccagagattcggcggcgctttcgcgcagccagatggtcgagctgcaaaccgccctcaaccagcgcggctttgccaccggcgcggccgacggtgtggtggggcccgccacgcgcgacgggctgcgccgctaccaacgcagcgtcggtttgcccgcggatgggtatccgagcgcagagctgctgcagcgcctgcaacggccgtagcgggcccgccgcgcgttccgcgcccgttaaactggggccgggtgcggagccgcttgtcttccatgcggtgccgcaggttcatgcgatggtcgggccgccacgcggattcgtcacgccaatcccatgcaagaacccgccatccagtacattgccgcagccatctttgccgtggccctcgtccatacctttgccgtcaagcagttcgaacggctgtcgcatcgctatccacgccacgccggcctgttccatctgctgggcgaggttgaagtcgtcttcgggttctgggccatcgtgctcgtgctggcgatgggcctggtgagcggcggcgacggcgcgctcggctatgcggagtcgcgcaactacaccgaaccgctgttcgtttttgtcgtgatggtggtggctgcctcccggcccgtgctgcgcacggtcatgtcgggggtgagcatcgtcgcccgggtgctgccactgccgacgcccgttgccgcggcatggctcgggcttgcggctgttccgctgctgggctcactggtcacggagcccgcggccatgacgatcgcggcgctgatgctcgcgccccagatcttcaggccgcagctgcccgaagcggtgaagtacctggccctgggcgtgctgttcgtcaacatatcgatcggcggcaccctcacgtcgtatgccgcgccgccggtgctgatggtggcctcgacctggcaatgggacagcgccttcatgctcgccaccttcggctggaaggccgccgtggccgttctcgtcaatgccaccgtggccaccttcgtgctgcgcaaacatctggccgccgcgccgtcgccagcgaaccccgaactgtccgaggtgcctgtgccggcggccgtggccctcgcgcacctggcattgctcgcggggatcgtgctgttcgcccatcatccggtggcattcctcggcctgttcctgatgttcctcggcttcacccaggcctatgagcgccaccagagtccattgatcatcaaggaagcgctcctcgtcggattctttcttgccggcctggtggtgctcggcggcatgcagcgctggtggctcgagccggtcgtctccagcctggagccgctggccttgttcttcggcgcgctgggcctgacggccatcaccgacaacgcggcgctcacctacctgggctcgctgatcgcgaccatctcggacgaatcgaaatacatgctcgtggccggcgcggtggctggcggcggcttgacggtgattgccaacgcgcccaatcccgccggcgtcgcgctgctgaagcgcggcttcgccgacgagagcatcggcgccggcggactgctgctcggcgcgctcggacccacgctggtggccggcgcggcgttcatgcttttgtagcgggcgcgcgctgcgcgcggaaccaaaggagacaagaacatgcacgcgttctctcgcacgggcctggccgcaggcgcgatgctcgtggccctggccatcggcggttgctcctcgcacgggaacgccgtttccagcagcgccagggcggagccgccgcccaccgattgccgcgcctgggtgggcaccgaccgcaaccaggaactgcccggctaccggctgccgcagtccaacggccagaccgtgtgcgtgccgctcggcgtcaacgcctttcgcccgcccgcggggtatgccggaggcgactaccacgtcgacgaattcaccgatgcgcgcctgaaggagcgctggcgcgcgtgcaaggccgacaccgcctgctttgcgcgcatcgatgcgcaaatgcagcgctggctgccgccgaacaaggcacgctcgacccgcacgaccggcatggtcgatccttcgggaaagatcgatcccgagggcaccgtggatctgcggcagatccgacgcccggccttctttgccaaagcgccttacgaggaaggcattgcgcgcgccgatgccagcacttacgtggtcgagttcaccgtgccgcgcgacaccttcgagcgcatcgacctgaagatgaccgatccgatcaagctgcgcggctggtacatcgaaggccgcggcgtcgacgacggcaagggcggcaagatacgcgcgctggtggtcatggcgcccggtggcggcggtcagctcaccgccatccagcacccgggcgagaaggcctaccgcatcgacccggccacgggcagggcggtggacgtcaagtttccgaacgccaccacggagaccatgggccagcgctggtggcgcgagaacctcgatgcgctcaaccaggcgggcttcgacgtgctggcctacgaccggcgcggcgagggcatttcggggggattcagcgacaccaacacgctggagcagggcgaggacgtctttcgcgtgctggcgcagctcgacaccggaaacggcctgcgccttctcacgcccgacgcgcgcgtgctcgcgggcagcgaggcggccggcaagctgctgggcggcatggcgtcgacgcgcattcccatcttgctcggcggttattcgcgcgggtcgatgtcgaccgcatgggccatggcgaagaatttctcgggctcgtgcagctacgacatgccggtgcccgaatgcgtgccgcccaaagggctctcgaacatcaagggcgccatcctgttgtcttcgtttgccagcggcgcggggtacctgcccgcgtcgccagacctggccgaccgcaacctgtttctgggcggcatggcggcggaccatcacatccttttctatcccaactcggcgcccctggcgggcatgcacaagtggccggccgcgttcttcggcaagggcctgtgggatcgcgcggaaacgctgcaaggcaccgtggccgcctacgaccgcatccgcggcgcgcgcgagatcgtggtggctcgcgccccccattcgatcgagacctggcccgaaagcgaccggcagtacctgcgcgagcggatgattgccttcgccaaggtggcaattgcgggcggcaccacggtgccgggcgcaaagccgtggtccaacctcaaggagctggtcgcgaccacgcccgactcgtgggagtcctcgtcccggccgaagcctgtcaacggctcgccttgacttcttatccggtatgttggatatttggtctgacatcatggataagcagtcaccaaccctgaatgagcgcatcgcgcagcgggtgcgagacctgcgcgccgaccgcggcctttctctcgatgcgctggctgcgcattgcggcgtcagccgctcgatgatctcgctcatcgagcgcggcgaaagcagcccgacggcggtgctgctcgagaaattggcgacgggcctcggtgttccgttggcctcgttgttcgaggcgccacagcctgacggcggccctgtagcccgcctggccgaccagccccaatggcgcgatccgcattccggctacgtgcgccgtaacgtgtcccccagcagcgctgcatcgcccatccacatcgtggaggttctgtttccgcccaaggcgcgcgtggcctacgaaaccggtgcgcgggaaccccaggttcaccagcaggtgtgggtgctcgaaggaaccatcgaagtcactgtcggcgaagaccagcaccggctcggcgcgggcgactgcctggcactggtgctcgaccgccccatgagctactacaaccccacccggcaggccgcacgctatgccgtcgtgatcgcaaccttgccctcttcgtggagatgacatgacgctcgaccttgcaacctccgcgccgagcattcgcgttctttccagcatggacgacgcacatgcccggcagctggccgacgtgctcgtcgattgcgtggagggcggcgcatcggtcagcttcatgctgccgctgacccgcgagcgcgcttcggcgttctggcgacgcgtgggcgagggcgtggcatgcggcgaccgcgtgctgctggtggccgaagacgcgcaaggcatcgtcggaaccgtgcagctgctgctcgaaatgccggagaaccagccgcatcgcgccgaagtggcaaagatgctcgtgcaccggcgcgccaggcgccagggtatcggcgcgctgctgatgcaggccgccgagcagctcggccgcgaacgcgccaagaccttgctcgtgctcgacacctccagtgccgaggccgagcgcctgtatgcccgactcggctggacccgccttggcgtgatcccgggctttgcgttgctgccgggcggcgagccgtgcgacaccacctacttctatcgcgcgctggcctagcgcatggcgccaaaaatgcggtagcccgggatttgcggacgcggcgcagcctgtcatcattcgcggctgaatgacccaagaaccgacgcccctcatcgatctgttgttgaaccgcgccaggcaggtgctggcgggcacggacggcacgctgcagtgcgccgccgccacgcccgaagccggctgcgtggtgttcatcgccctcggcgaccaggcgagccgcgcacgcgtggtcgtggggcgcgggggcagcgccgaggaggcctggcgcgaggcatgcaatgcggcgctcgcgctcatccagcgcatcggcatgcagcctggccgcgtgcgcgtggagctcgtcgaacaggtcgaggccatgacctggggcgcgctgaaggctcgcctctcgcgaaccaagcgcaactacttcaaccagggcgtgtcgttcgacgcgaggttcgaagcggcgctgctcgcgcaggagatcagcggcagcgccatcttctacaacggcaccgtggaacacgcagagcccaacgccggcaacctgcgcctgcacgcccagaggcgcttcggcgccgagatcgattttccgtccgacgatgcggtgccggtgtggtgcttcgtcacgcgcggtgcctatgccgatgccgagggcgcctggccgctgacggccaaggggcaggccgcgggctatcgcacgctgcccgaatggaacgcgggccaggtgcgccgcctcgtcgacaccgcgagcgactatctcgccgcgcaggtccagcccacgggcgagttccactacggctggttcccgtgcttcgaccgcgcgattcccacctacaacaccctgcgccacgccagctcgacctatgcgctgctcgaagcctgggagctgacccgcagcgatacgcaaaaggcggccatcgaccgttcgctgggcttcctgacggcccggctcattcgccaggtcgaactgcccggcggcacgcgcgcggcgtacctgctggatgtcggcaacgagatcaagctcggtggcaacgcggtgtgcctgctggccttcgtcaaatacaccgagctcacgggcgatacgcaatacctgccgctgatggagcagctcgcgctcggcatccaggccatgcaggacccggcgagcgggcgcttcgtccacgtgctgaaccacccggcgctcgacgtgaaggatgcgttccgcgtcatctactacgacggggaagccgccttcggcctcatgcgcctctacgggctcacgcgcgatccgcgttggctcgcggtcgtcgagaaagccttcgaccatttcattgccgcggagcactggcgcgcgcacgaccattggctgagctattgcgtgaacgagctcacccgccatcggccagaaacacgctactaccgcttcggcctgcagaacgtggccgactacctggacttcgtgctcgagcgcatcaccacctttccgacgctgctggaactgatgatggccgcgcgcgacatggtggcgcggcttgccgccgaccccgcgctgcgcccgctgctcgaaggcttcgaccgcgacaagttcgaccgtgcgctcgagcaccgcgcgcgctacctggccaacggctacttctggcccgagctggcgatgttctttcgcaaccccgaacgcgttgccggctcgttcttcatcaagcaccacagctttcgcgtgcgcatcgacgacgtggagcactatctctccggctacgtggcctatctcaagttcctgcaagcgcgggagaacgacgactcccacgacgatgccggccatgcggaggggagcgcccccgcaccggtggtggcatggggcggcgacgtcaacattggccgcaggcagcactacctgacagcgcaactcggcgtgccgtcggtgctcggcggcgtgccggtgctggccgaggcggacctgcgcatcgtcaatctggagtgcgtggtttccagccgcggcgagcagggggtgccgaaaggcgaggccggcccgcactactaccgcgcgcggcctgaaatgctgcgcgtgctcaccggcgccggcatcgacatggtcgccaccgccaacaaccacagtggcgactacggcgcagcggcgctcgcggagcaggcggccttgctcgatgccgccggcatcgcgcatacaggttcgggtccgacgctggacgccgcgctcgcgcccgtgctgcggcgtgcagggcacctgaacgtggcgctcttcgccatcgacaccacgcagcggcgctttgccgccggcaaggccacggccggcaacgcctacctgccgctgtcatcgcccgcggagtggacggcatgcctttcgccccgcatcgtcgccgcgcgccaaaaggcgcatgtggtgctggtggccgtgcattggggaaagaaccgggagccttgccccagtcccgaagaaatcgccgtgggccacgccatcatcgaggccggcgccgacgcggtgctgggtgcttcggcgcatgtcgtgcaaggcgtcgagatacacaagggccggcccatcctccatgacgccggcgatctcctgttcgacgccatcggccgcagcagcaaggacagcgacgaaagcggggtgttctcgctgcacctgggcatcgacggcgtgcggcgcgtggtgttcacaccggtcgccacgggcttcggccagacgatgcagctggaaggcgagcgcgcggtggcggcggccggccgcttcctgcagaaatccgccgcgctcggatcggacttcgcgctcgcacccaacggccagtgcacgctcgacctgcatccgcccgccaggacgccaaggccgccaccatggccggccctgccgcagatggcgcgcaggcccgaggcgatccagcctctgcagcagccacgcgaagagtggctgccggcggtggtgccgccagaggcggcgctcgagcagcccctgtcgctggggccgctgcgcctgctcggcgtgcgaaccacgccagcggccattgcaggccgcggcatgctgtacgtcgagaccttctggcaaatcgacgaggcgaccggcaccgactggcggctcgacatccgcgccgtgccggcagcgccggccaccatgccggcctggggcgtcgcgatggatcacgacccctgcgactggatgtggcccacgagccgctggcagcccggccgcatctatcgcgatttgcatggcttgcggccaccagcgggcaagcttctgcatgatgcgcggctccagatcgaagtcgggctggtgggcgatgccggtcgggtggagcgggtccgactgccaagggacgtttcgttcgcggtgcgagcggaccgtgtggcggcatgaggcgcgagagctccacagccagcggaaccgaaggcatggctgccggacgctggcggcttgttcccctcgcgctgctggcgctggcacagaccgcatgcgcgcaacgcggcggcccggagccgcaggtccctgtgcttgcagccgaaggcggaacactgcggtggaaccagcccgccgtgcgcgccaactgccccgaccgcgccggctatctctgggtgcagccggtcgaagggccggcctgcatccgctacttcgcgagcagcgacatcgacgatgcgcgcatggccatcgtgcagttttcaggtgaccgcgacggtgtcatgaaccagtcgcccgagcgcattcccggcaacaccgaggccctgcgcatgctcgacgcccagcgcagccgcgatcgcgcgggcgtgccatgggtcttcgtggcgcggcccggcacttacggatcgtcgggcgaccatcgcaggcggcgcgaactggccgagttccacgcgctggatgcggcgctcgatgcgctgatgcagcggcaccggatccagcgcatcgtgatcctcggtcacagtggcggcgcgaccgccggcgcggcgctgctcacgctcggccgcacgcgcatcgcctgcgcggtgctgacctccggcgcctacggcctgctggagcgtgcacgccggctggggcaatcgcgcgacggccgcagcgacaccaccggcagcacgcagttctacgatccgctcgaccacatcgacggcattgcgcgcgatccgctgcggcgcatcgtgctgatcggcagccgtgacgacaggaacacgcccttcgacttgcaggagcggtttgccgatgtgatcgccaaggcgggccatcgcgtggaagtcaagacccatgcggcagagccgccgcagaatcacgacctcaaggaccgcatcggcttgcagaccgcatcgatctgcgcacgcgaagcgatgtttcaataacgacagagaccttcaagacaatgccctcgccgaacagcagcactagcaatagcagctccaccgcccgcatcgccacgcaggagttcggccgcatgcccgacgggcgcgcggtgaccgaatacacgctcgacaacggtcgcggccttcaccttagtgccatcaaccttggcggcatcgtcaccgcattgcacgtgcccgaccgccacggccaaagcggcaacgtcgtgctcggcctgccctcgctcgatgagtacctgaagccgcatccgcacttgggcaccatcgtcggccgctatgccaatcgcatcgcgggcgggcgcttcacgctcgacggtgttgggcatcaactcccgctcaacaacggcgccaactcgctgcatggcgggcacaacggcttcggcacgcgcttctggcagatcgaagcggtgccggcgcgcgaggatggcgatgaggtcgccatcgacctctgctacaccagcgccgacggcgaagagggctatcccggcgaggtgcaggtgaccgtgcgctacgcgctcagcaccacagagaacgcgtggcgcatcgactaccgcgccgtggccgaccgcgccaccgtgttgaacctgagccaccatgactacttcaacctggcgggcggcggcgcggtgctcggccatcgcctgtcgatccccgcaagccgcttctgtccggtggattcgggcctgattccgctgagcctggcgccggtggccggaaccccattcgactttcgcgcggccacgccaatcggcgagcgcatcgacgatccgcacgatcaactgcgggtggccggcggctacgaccacaactgggtgctcgaccgcgagccgacgggcatggcgctggcggcacgcctcgaacacgagccctccgggcgcgtgatggaagtgcatacgaccgaaccggcggtgcagttttattcgggcaactttctcgacggcacccttcgcggccgcgaaggcgagagcttcaagcggggcgccgggctgtgcctggaaacgcagcactaccccgactcaccgaatcagccggactttccttcgacggtgctccggccgggagaagtgttcagcagtgccacggttcaccgcttcggcatttcggcctaggctttgaccgcgtcggcgccgaactcggcagcgggcaggccggggcttgcgatgcgaaccgagaacagtgcgccggccagcggctctgccttcagttcttcgtccgagagcccgctgcgcgcggtggtgatgtagagcgtgcacaggtcgtcgccgccaaaggcgcagtccgtgacgttgctcgcgggaagttcgatgcggcacagctcggcggcgctcaccgggtcgtggcagctcacgcaatggccgccccagcgcgcgatccacagccgcccggccgcgtcggtcgtcatgccgtcgggcaggccgtcgcctttcgcaaagcgaagccacacgcgcttgttgctcacggtgccggctgcgctgtcgaagtcgtaggcatacacgcagccttccacggtggcgttgaaatacatcgtgcgttcgttgagcgaccaggtcggaccgttggtcaccgcaaagccgtcgtcgtggcgcgtgcagcggccgtcggcgtcgaagcgatagagcgcgccggtcggcgccacgcaatcgaagtccatgctgccaccccagaagcggccctgccgatcgcacttgccatcgttgaagcgattgccgggccggtcgggctcgggctggtgcaggtagcgcggcggcgcatccacggccgggtcgaagtaggcgaagccgcggcgcatcgtgacgatcagccccggcgcatcggcgcgctcggcgagcgcggtgatctcctcgtcgaactgccagctctgccgcgcgccgccggccgggtcgtggcggtacaggcgacggccgaggatgtcgagccagtagagcgcctgttcgcgctgcgaccacagcgtgccctcgccgagcgtggcgccggcgggccacaggcactcgggttggccgaggacggtgggtgcacccaggggtgcaagaggagatgcggagctgccgttctgagtcattgttttgcgccttcgttgtctcggtccttgacgcggcggatcgtatcaaggcatattgataatagaaaccaaactatttggcatcaagtgatattcattttgcaatgtcacagccagctctctggagacgcacatcttgaaggattccccgcagctttcgattcatcccagcctgaagggacgcaccgtgttcgtcaccggcggcggcagcggcattggcgcggccattgtggcggcgtttgcggcgcagggcgcgcgcgtggcgttcgtcgacattgccgaaagcgccagcgccgcgctcgtgcaacagatcgtcgagcaaggccacgccgcgccgtggtggcgcacttgcgacgtgcgcgacatcggcgcgctgcagaaggccatcgacgacgcggccggcgagctgggcgacttcgccgtgctggtcaacaacgtggcgagcgacgaccgccacacgctcgaatcggtcacgcccgactactacgacaaccgcatggccatcaacgagcggccggcgctgttcgcgatccagtcggtggtgccgggcatgcgtcggctgggcttcggctcggtggtcaacctgggttcgacgggctggcagaccaagggctcgggctatccttgctatgccattgcgaagtcgtcggtcaatggcctcacgcgcggcctggccgtggagctgggcaaggaccgcatccgcatcaacaccgtgtcaccgggctgggtgatgaccgaccggcaggtgaagctctggctcgacgacgagggcgaacaatcgctcaagcgcaaccagtgcctgcccgacaagctcctgcctgaggacatcgcgcgcatggtgctgttcctcgcgtcggacgacgcgaagatgtgcacggcgcaagagttcaccgtcgatgcaggctggacctgatcagtccatctcgagtttgcgcccgtagacgctgaggctggctgtcttcagcgctttcatcatcaccttggcagccggcgacggcagccggtcggtgcgggtgatgatgccgaaggcgtccatgtggcagggcatgtccagcggcagcagcgacacgatgccgtgtgcggcgtagtagcgcgccacgtcggaggcgagcacggccaccatgtcgctctgctgcagcatgcgcgtgatgaagagcagggccgagctttcgatgatgttgttcggcggcaccaggccttcttcctggaacatcagctcgaagcggtggcgcagcacgctgcccgcgggcggcacgatccagccggcgcccaccacgtcgcgcagcgtgaggccgctcacgcccaggagcggatggccggggcgcaccagcgcgcacacgggctcctcggccagcgcttcgtagcgaagctgcgacttgtcgtgctcggcgaaaagccgcgccaccaggatgtcgagcttgccctgttcgagccgctcgatcagcaccgcgctggtctcgatctccagcgacacgcgcaggtcgggctgttcgcgcttcaccatggccaccgccggcggcatcagcgtgaggccgggcgcggtgatggcgcccacgcccacctggccgaagcggccggccttgagcgcggtgagctcgtcgtgcgcctggttcaggctggccagcgccacgcgggcgtggcggatcatggtttcgccgtaccaggtggggcgcatgccgcgcggcagccggtcgaacagcggcacctccagcacgtcttccaggtctttcagcagcttggaggcggcgggctgggtcatgttgagcacctgcgccgcgcggtggatgttgccttcctccgccagcgccaccagcaaaagcagttgccgcgtcttgaggcgcgcgcggatgaaccagtggttgtagttggtcatggttgttgttaaggctttgggctgaaagggttttccagaatccggcgattgatatccattttgtcgaaaaaatgattggatcgatatcaattctgttcctagacttcgccccacttccaaaaaccagagacaaggtcggcgcacaggtgattcacggcgagatccatcagaacgtgcggcaatacatcaacggccgctgggaaaccagcgcgaccacgggtgtgagtgccaatccttcggacaccagcgaagtggtggccgaatacgcacgtgccgatcgccgccaggtcgaatccgcgatccgcgcggcggccgacgcctttccgcactggagccacagcacgccgcagcgccgggccgacgtgctcgaccgcatcggcaccgagctactggcgcgcagggacgacctgggcctgctgctggcgcgcgaggtcggcaagacgctgcccgaagccgtggccgaagccacgcgcgccgggcaggtgttcaagttctttgcgggcgaggcgatgcgcggcgggggcgagaacatggcatcgctgcgcgctggtgtgcaggtcgacgtcacgcgcgaaccggtcggcgtggccggcctcatcacgccgtggaactcgccgcttgcagtgccggcgaccaagattgcgcccgctctggcccatggcaacagcgtggtgttcaagcctgccgaactggtgccggcctgcggctggacgctggccgaaatcatcagccgcgccgcgctgcccgcgggcgtgttcaacctggtgatgggcagcggccgcgaggccggccaggcgttggtcgacagcccgctggtcgatgcggtgagcttcaccgggtcggcccgcaacggcgaacgcattctccaggcggccgccgcgcggcgcgccaaggtgcagctcgagatgggcggcaagaacgcgctcgtggtgctggccgacgccgacatcgaccacgcggtcgactgcgcggtgcagggcgcctacttttccaatggccagcgctgcacggcgtcgagccggctcatcgtcgaggccgccgtgcacgacctgttcgtcgcgcggctccgtgagcggctcaaggcgctgaagatcgggcatgcgctcgaacgcggaatcgacatcgggccgctggtcgacgaagagcggctggcgcgcagcctggcctgggtagccattgcgcgagaagagggtgccgagcacgtttggggcggcgagccgctcaagcgcgcgacggcaggccactacatgagtccggcactcttcctggccgagccagggcaccgcatcgcgcgcgaggaaatcttcggcccactggcctgtgtgctgcgcgttgccgactacgacgaggcgctggcgctgtgcaacgacacgccctcgggcctgagcgcgggcatctgcaccaactcgctcaagcacgcgatgcatttcaggcgccatgccgaggtcggcatgacgatggtcaatctgccgaccgcgggcgtggacttccacgtgccctttggcggccgcaaggggtcgggctacgggccgcgcgaacaagggcgccacgccgcggagttctacacgacggtcaagaccggctatatgctggcctgaccaccacggacggttttcatcagcaagcaaacagagaaagaaggagacattcccatgaaactcaatcgccgcaccctcaacatcgcactcgccgccgcctcgctgggcgggcttcttcccgccgccgcgctggcgcagaagaagatcgtgctgggcttcagccaggtcggggccgagagcgaatggcgcaccgccaacaccgagtcgatcaaggcatcggccaaggaagccggcatcgagctcaagttctccgatgcgcagcagaagcaagagaaccagatcaaggccatccgctctttcattgcgcagaaggtcgacgtgatcgccttctcgcctgtggtggagtcgggctgggaaaccgtgctgcgcgaagccaaggccgcgaagattccggtggtgctgaccgaccgttccgtgaacaccaaggacgacacgctctacgtgaccttcatgggctccgacttcgtcgaggaaggccgcaaggcgggtcgctggctggtcgagaagatgaaggaccagaagggcgacgtgaacatcgtcgagctgcagggcaccgtgggctcggcaccagccatcgaccgcaagaagggcttcgaggaaatcatcaaggccgatcccaagttcaagatcgtgcgctcgcagaccggcgacttcacgcgcgccaagggcaaggaggtgatggaagccttcctgaaggccgagggcaagaagatcaacgtgctgtacgcgcacaacgacgacatggccatcggcgccatccaggccatcgaagaggctggtctcaagcctgcgaaggacatcaccatcatctcgatcgacgccgtgaagggcgccttcgaagccatgatcgccggcaagctcaacgtgtcggtggaatgcagcccgctgctcgggccgcagctgatgagcgccgtgaaagacatcaaggccggcaaggcgctgcccaagcgcatcgtgaccgaagaaggcatcttcccgatggaagtcgccgccaaagagtttcccaatcgcaagtactgagagcccatacccatgaaacgcaacttcctcaaggcctcgctcgcaggcatcgcgctggccgtcgccggtatcgcaccgctcgcgcatgcacaggacaagggaccgatcgccatctccatgcccacgaagtcgtcggcccgctggatcgccgatggcgccaacatggtcaagtacttcaaggagaagggctacaagaccgacctgcagtacgccgacgacgacattccgaaccagctcgcgcagatcgagaacatggtcaccaagggctcgaaggtgctggtcattgcggccatcgacggttccacgctgtccgacgtgctgcagaaagccgccgacaagggcgtgaaggtcatcgcctacgaccgcctcatcaagggctcgaagaacgtcgactactacgccaccttcgacaacttccaggtcggcgtgctgcaggcgcagtcgatcgaggcggccctcggcctgaagagcggcaagggcccgttcaacgtcgagctgttcggcggctcgcccgacgataacaacgccttcttcttctacaacggcgcgatgtcggtcctcaagccctacatcgacagcggcaagctggtggtgcgcagcaagcagatgggcatggaaaaggtcggcacgctgcgctgggacggcgcggtggcgcaggcccgcatggacaacctgctgtcggcctattactccaaggaccgcgtcgatgcggtgctgtcgccgtacgacggcctgtcgatcggcatcctgtcgtcgctcaagggcgtgggctacggctcggcttcgcagccgatgcccatcgtctcgggccaggacgcggagatcccgtcggtcaaatcgatcctgcgcaaggaacagacctcgaccgtgttcaaggacacgcgcgagttggccaaggtcacggtggccatggtcgacgccatgctgtcgggcaagacgcccgaggtgaacgacaccaagacctacaacaacggcatcaaggtggtgccctcgtacctgctcaagcccgtgagcgtggacggcggcaactggaagcaggtgctggtcgacagcggctactacaaggaaagccaggtcaagtgagcatcggcatggcggcagtggacacgcgcagcatcctcgagatgcgcggcatcaccaagacgtttccgggcgtgaaggcgctctccgacgtcaacctggcggtgcgcgcgggggagatccacgcggtggtcggcgagaacggcgcgggtaagtcgacgctcatgaaggtgctgagcggcgtctacccgtgcgactcgtacaccggcgagatccacttcgagggcgagctgcgccgcttcaggagcattgccgacagcgagaagctcggcatcatcatcatccaccaggagctggcgctggtgccgttgctgtccattgccgaaaacatctttctcggcaacgagattgcgcatggcggcgtgatcgactggttcgccgcctatgcgaagacccgcgacctgctcgccaaggtgggcctcaaggagccgcccaccacgctggtgacggacctgggcgtgggcaagcagcagctggtggagattgccaaggcgctggcaaaggaagtcaagctgctgatcctggacgagcccaccgccagcctcaacgagaacgacagcgatgcattgctgatgctgctgctcgaactgaagcggcagggcatcgcgtcgatcctgatctcgcacaagctcaacgaaattgccaaggtggccgactcgatcaccgtgctgcgcgacggtgccacggtcgagacgatggactgccgcggccggccgatcagcgaagaccgcatcatccgcggcatggtcggccgcgacatggcgcaccgctatccgcagcgccacccgaagatcggcgagacggtgttcgaggtgcgcgactggcgcgtgcaccatgcgctgcacgccgaccgcgagcagatcaagggcgtgaacctgcatgtgcggcgtggcgagatcgtcggcatcgcgggcctcatgggtgcggggcgcaccgagctcgcgatgagcgtcttcggcaagtcctacggccagcgcatcagcggcacggtgctgatgcacggccagccggtggacgtgggcacggtgcgcaaggccatcgaccatggcattgcctacgtcaccgaagaccgcaagggcctggggctcgtgctcgaggaagacattcgcaagaacgtgagcctggccaacctggaggcggtctccaacgccatggtgatcgacgacgcacgcgaattcaaggtcgcggtcgattaccgcaaggcactcaacatccgctcttcgggtgtggaacagctggtggtcaacctgtcgggcggcaaccagcagaaggtggtgctcagcaaatggctcttcaccaagcccgaactattgattcttgacgaacccacgcgcggcattgacgtgggcgccaagtacgagatctacaccatcatcgaccagcttgcgagcgagggcaaaggcattctcatgatttcttccgaactgccggaactgctcggcatgtgcgaccgcatctatgtgatgaacgagggccgcttcgtggccgaatttacggcagccgaggcttcgcaggaacgcatcatgcacgccatcgtgagcgcggggagttccgttcatgtcgcagcctgaagtcaacgcggcggtgaacgccgccgtccccatctcggaggctggccccaagctgcacgccggcttcctgaagaacaacctgcgcgaatacggcatgttgatctcgctcgtcgcgatcatggtgctgttccaggtgctgaccgacggtacgctgctgcggccgctgaacctcaccaacctgctgctgcagaacagctacgtcgtcatcatggcgctgggcatgctgctggtgatcgtggcgggccacatcgacctgtcggtgggctcggtctgcggcttcatcggcgcgctggcggcggtgctgatggtcgagtacgaatggcacttcgtgcccacggccatcatcagcattgcggcgggcgcggtcatcggcgcggcgcagggctggttcgtggcgttccgaaagattccgtcgttcatcgtcacgctcgcgggcatgctggtgttcaaggggctcacgctggcgctgctggcggggcagtcggtggggccctttccggtcgagttccagcggctgagctcgggcttcattcccgatccgctgggcggcgacacgttgcgcaccacctcgctggtggtcggcgcattggccgcggcggcgctggtgttcttcaagctgcgcggccgggccaagctcgcggcgcacggcatggaaacggagccctatgcgttcttcctcgtgaagaacctgttcttcgcgggcatcatccttttcttcagctacctgctctcgacctacaagggcctgcccaacgtgctgatcgtgatggcggtgctgatcgtggtgtacgacttcgtcaccaaccgcaccaccatcggccggcgcatctatgcgctcggcggcaacgagaaggcggcgcggctgtcgggcgtgaagacgcagcggctcgcgttcctgaccttcgtcaacatgggcgcgctggccgctctcgcgggcctggtgttcgcggcgcggctcaacacggccacacccaaggccggcctcggcttcgagctcgacgtgatcgcggcctgcttcatcggcggcgcctcggcctcgggcggcgtgggccgggtgatgggggcggtgatcggcgccttcatcatgggcgtgatgaacaacggcatgtcgatccttggcatcggcatcgactaccagcaggtcatcaagggcctggtgctgctggccgcggtgttcatcgacgtctacaacaagaacaagtgatcgcatgagccagagcagcatcagccccgtgctcgaactgcggggcatccacaagcagttcggcggcattccggtgctgcgcgacgtgcagctgcggctctatccgggcgagattcatgcgctcatggggcaaaacggcgcaggcaagtcgacgctgatcaaggtgctcacgggcgtgctgccatcgagcggcggcgagatatgcctggacggaaaaaccattcaccccgcgtcgccgctcgaggcgcagaagctgggcatcagcacggtgtaccaggaggtcaacctgtgtccgaacctctcggtggccgagaacgtgtttgcgggccgctatccgcgctgtggtgcggcgcagggtttccgcatcgactgggcggccgtcaaccgccgtgccgaggaactgctggcgcgcatcggcctggacatcgacgtgacccggctgctgtcgagctactcggtcgcggtgcagcagatggtggcgattgcgcgcgcgctcggcgtgtcgtcgaaggtgctgatcctggacgaaccgacctcgagcctggacgatgacgaggtggagaagctgttcgaagtgctgcggcgcctgcgcggcgaagggcttgcgatcgtcttcgtgacgcactttctcaaccagatgtatgcggtgtcggaccgcatcacggtgcttcgcaacggcaactgggtgggtgaatggcgcgcagcggaccttggcccgcaggcattgattgccgcaatgctcgggcgggaactcgcggcccagtcggcacggcccgctgcgcttcccgcgctcgacgaggcggcgccagcgttgctgcaggccgagggactgggacaggccgggcagctgcaggcgaccgatctgcgcgtgcgcgccggcgaggtcgtcggcatcgcgggcctgctcggcgcgggacgcaccgagctagcgcgcctgttgttcgggctcgaaacaccggatcgcggcatgctgaggatcgacggccgttccgtcagcttctcgaaccccgccgacgccatccgcgaagggctggcgctgtgccccgaagagcgcaagaccgacggcatcgtggccgagctgtcggtgcgcgagaacatcgcgctggcgctgcaggcgcggctaggcacgcggcgctttctgtcgcacgccgagcagaccgcgatggccgagcgttttgtggcgtcgctgggcatcaagaccgcgagcgtggaaacacccatcggcctgctctcgggcggcaaccagcaaaaagccgtgatcgcgcgctggctcgcgaccgagccgcgcctcttgatcctcgacgagccgacgcgcggcatcgacgtggcggccaagcaggaaatcatggaggagatattgcggctcgcacgcgcgggcatggcggtgatcttcatttcttccgagatcagcgaagtggtacgcgtggcgcatcgcatcgtggtgctgcgcgatcgcaagaaggtgggcgagctgccgggcggctcgaccgaggacgaggtatacgaaatgattgcagcagcatgatgcacgcgctgtctccgcgttgtcccctctcccgcttgcgggagagggctagggtgagggcagaggccctcgacaagccaaaggcctttgcgtgggccgcaccccaaccctctcccgcaagcgggagagggagaaagaccgatgcgttgcgctgtgttcggtggagcctgacatgaccaacgccagaaatctcttggcccgcgcgatgagccaccgcctcgcttggcccatcgtcacgctgctgctcctgctcgcagtcaacaccgcgttcaacgccagcttcctgcacctcgaatggcgcgacggccatctctacggcagcctgatcgacatcgtgaaccgcgcggcgccgctcgtgctggtgtcgctcggcatgacgctcgtcattgccacgcgcggcatcgacatttcggtgggcgcggtggtggccattgccgcggcactggcggcctggatgatcggcggctcggtggcgagcgacgtgagccgctttccgatgtggctggccattgcggcggccctcggcattgcgctgctgtgcggcctctggaacggaatgctggtcgccaaagtcggcatgcagccgatcatcgcgacgctgatcctcatggtggcgggccgcggcatcgcgcagctcatcgcggatgggcagatcatcacgatctactacaagccgttcttcttcctcggcagcggctacctgctggggctgccgttctcgttgttcatcgtggcggcggtcttcgtgctgctctatctcgccatcacgcgcactgcgctgggcctgttcatccaggcggtgggcatcaacccgacggccgcgcgcgtggcgggcgtgcaggcacgccggctcgtcgtcggcgcctatgcgttctgcggcgtctgcgcgggcattgcgggcctcttgatcagctccaacgtcaagagcgcggacggcaacaacgcgggacagctgctcgaactcgatgcgatcctggcggtgacgctgggcggcacggcgctcaccggcgggcgcttcagcctcatgggcagcgtgatcggcgcgctgatcatccagacgctgacctatgcaatctattcgctcggagttccgccggagatcaacctcgtcgtgaaggcggtggtggtgttcgcggtgatgctgctgcagtcgccggagttcagggctgaagtgcggacgctggttcagcggcctgcgcatgagggagcaagttcatgagcctccgcccggccgttccgaagggggctcgcaccgcagtgcgcagcacggaggttacccaatgagcgcggtgatcgaaacggcaccctcaccccagccctctcccgcgcgcgggagagggggcaaggcagggctcaatccgaagtacttgccgttgacggcgaccatctcgctgttcgtgctgatggccacgctgggctcggtgttctacgacggcttcttttcggcgcaggtgttcctcaacctgctgatcgacaacgccttcctgatcgtcgttgccgtgggcatgaccttcgtcatcctttcgggcggcatcgatctctcggtgggctcggtgatcgcgctcaccacgatggtgtcggcctcgctggtcgagaagcacggctggagccccctggtggtgattccgctggtgctggccatgggcacggccttcggcgcgttcatggggctgctcatcgaacgcttcaggctgcagcccttcatcgtcacgctggcgggcatgttcctggcgcgcgggctgtgctatctgatcagcatcgattcgatcagcatcaccaacgcgttctattccgaggtctcgcagatccgcattccggtatggggcgaggcttcgctgtcgatcagtgcagtgatcgccatcgtcgtgctgctggcggcggtgttcattgcgcattgcacaccgttcggccgcacggtgtacgccattggcggcagcgagcattcggccatgctgatgggcctgccggtgcgttccacgctcgtcggcgtctacacgctgtcgggtttctgctcggcgctggcgggcgtgatcttcaccttctacatgctgtcgggctacggcctgcatgcgctcgggctggagctcgatgccatcgcggcggtggtgatcggcggcacgctgctcacgggcggcgtgggctacgtggcgggcacgcttttcggcgtgctgatgctcgggatcatccagacgctgatttccttcgacggcacgctgagctcgtggtggacacgcatcgtcgtgggcgcgctgctcttcgtgttctgcctgctgcagcgcttcttcacttcgcgcacgccacggcgctgactttttctttttctctctcgcttttcaggacacccccgcatgccggacgatacccccaagaagaagcttcgctcgaccgaatggttcggctcggccgacaagaacggcttcatgtaccgcagctggatgaagaaccagggcataccggaccacgagttcgatggccggccgatcatcggcatctgcaatacctggtcggagctcacgccctgcaatgcgcacttccgcaagattgccgagcatgtgaagcgcggcatctcggaagcgggcggctttccggtcgagtttccggtgttctccaacggcgaatcgaacctgcggcccacggccatgctcacgcgcaatctcgcgagcatggacgtggaagaagccattcgcggcaacccggtcgatgcggtggtgctgctcacgggctgcgacaagaccacgcccgcactgctgatgggtgccgcaagctgcgacatcccggccatcgtggtcacgggcgggccgatgctcaacggcaagctcgacggcaaggacatcggctcgggcacggccgtgtggcagcttcacgagtcgctcaaggccggcgagatcaatctgcaccagttcctttcggccgaaggcggcatgtcgcgttcggcgggcacctgcaacaccatgggcacggcctcgaccatggcctgcatggccgaggcgctgggcacttcgctgccgcacaacgcggccattccggcggtcgatgcgcggcgctatgtgctcgcgcagatgtcgggcatgcgcgcggtcgagatggcgaaggaagggctcacgctgtcgaagatcctcacgcgcgaggctttcgaaaacgccattcgggtcaacgcggccattggtggatcgaccaatgcggtgatccacctgaaggcgattgccggtcgcatcggcgtcgacctcgagctggaagactggacccgcatcggcagcaatacccccaccattgtcgacctgatgccctcgggccgcttcctgatggaggagttctattacgcgggcggcctgcccgctgtgctgcggcgcctcggcgagaacggcctgctgccgcaccccggcgcgctcaccgtcaacggccagtcgatctgggacaacgtgcgcgaagcgccgagcctcaacgacgaggtgatccgtccgctcgacaagccgctgatcgccgacggcggcattcgcatcctgcgcggcaatctctcgccgcgcggcgcggtgctcaagccttccgcggcgtcgcccgagctgctgaagcaccggggccgcgcggtggtgttcgagaacctcgagcactacaaggcgcgcatcgtcgatgaatcgctggatgtcgatgcgagttcggtgatggtgttgaagaactgcggcccaaagggctatcccggcatggccgaggtgggcaacatggggctgccgccgaagttgctgcgccaaggcgtgaaggacatggtgcgcatctcggacgcgcgcatgagtggtacggcctatggcaccgtcgtgctgcacgtcgctcctgaagccgcggacggcgggcctttggccgcggtgcgcgacggcgactggatcgagctcgattgcgatgcgggtcggctgcacctcgacatcagcgacgaagaacttgcatcgcgcctggcttcgctgtcgaacaccgacgcgcagcccatgagcacgcgcggcggcggctaccagaagctctacgtcaaccacgtgctgcaggctgacgaaggctgcgacttcgactttctggtgggctgcagaggttccgccgtcccccgtcactcacactgatccatccatcatgactcccagataccgcggcatcttcccggtggtgcccaccaccttcactgaacagggcgcactcgatctcgaaagccagaagcgctgcgtcgatttcatgatcgacgcgggctccgacggcctctgcatcctcgccaacttctcggagcagttcgtgctctccgacgaagagcgcgaggtgctcacgcgcacggtgctcgagcacgtggccggccgcgtgccggtgatcgtcaccaccacccactacagcacccgcatctgcgctgaacgcagccggcgtgcgcaagacatgggcgccgccatgctgatggtgatgccgccttatcacggcgccaccttccgcgtaccggagccgcagatcttcgagttctacgccggtctttccgatgcggtgggcattccgatcatgatccaggatgccccggccagcggcacggtgctgtcggcgccgttcctcgcgcgcatggccaaggagatcgaacacgtcgcgtacttcaagatcgagacccccggtgcggcctcgaagctgcgcgagttgatccgccttggcggcgatgccatcgaaggcccgtgggacggcgaagaggccatcacgctgatgcccgacctggatgcaggtgcgacaggttcaatgaccggcggcggctacccggacggcatccgcccgatcatcgaggcccaccgcgcaggcgaccgcgacaaggcctttgcgctttaccagcagtggctgccgctcatcaactacgagaaccggcaggctggcctgctggcgtgcaaggcgctgatgaaggagggcggcgtgatcgcctgcgaggcaccgcgccatccgctgccgacgatgcaccccgacacgcgcgcaggcctgatcgaaaccgcgaaacggctcgatccgctggtgctgcgctgggcgcgttgaagagcgagaaggactgaacgagaagagagagaaaagggcgctcagctcttctcgagttcactgacctgcagcgacaggtcgaacagcttcgacttgctcgcgtaatagcggtcgagccgccattccttcaggatgtccatggcgagttcgaagctcttgtagtccaggctgtagagcgtgaccagctcgaagctgcgttcggattcgagcgccaacacgagctgcgccaggatcttggccgattcgttggccgggtccgtttcgatgaatcggcgagcgaccttgatggcattcatgggaaagagttcctcgtaggcagagaccgcgaactatagctagcacgccgctttgctttgtgacaattgtgtgacaaacgaggttatcactgcgcggcttgcgcaatgatggatgcggcccaccgcccacgcgaatgggcggcggtgctgcacgaagaggcaactctgcgcgtcagcgaatcggcgtgggcatcggggccggcatcggctccatgggggcgggagccatgggtgccacaggggccatcggcgccatggccggtggcggcaggcgcgaaggctcgggcgccggaggcggcatcacggcgggtgccggcatgaccacggtggtgacggactcgcgaatcacgccgccgcccatcacgctgccatcgacattgccactggtgttgccgctgccgccgagcacgcgggcttcgcagtcggcgcgatctgccggcggctgcaggctgcatcgcgcgagggcattgcggcggtagtcgggcgcactggtcaacccgccgcgcgcagcttcatggcgtgcggcgccggcctcgcgaatgcaggctgcgcggtcttgctggttgcggccgcagaccgagagttcctgctggtaggtggaatcgccgcggcgcggctgggccgaggccgacgtggccgcggcaataccgcccacggcaatgagggcggcaatcatcgaacgggtggtgctgttcatggtgtgctccttggagtgacctgaaacatgaggtgaaatagttggaaggggcgggccgcgccaggttccgcgcggccgacgttcaacgcgtgggtgagacgggttgcggcggcagcggcgtgaccgtttcgcggatgatgccgccgcccatcacgctgccttcggtgctggtgcgtgcgccgccctgcaggcgcgcttcgcaatcggcgcggtcggccgctggctgttcgcggcaacgcgccatggcgttggcatcggcacggccggggccaacgctggtgagcccgttgcggcctgcttcctgccgcgcggcgccggcttcgcgcaaacatgcggcgcggtcctgctgcacgccgtcgcaggtggcgcgctcctgctgcgcacgcgcggcggaacctggctcgggtgcctgtgcctgtgcaatcgacgcgccgaacactgctgcaaaaagcgcggcagcagaaagggtggaacgaactgttgttgtcatcgggtgctcctgattgaggcgcgccctccgaaagcgcgaccggacccgcagtgtggtccggtgcaccccttgcagggtgtgggactgcgcagacagcagacccggccagactcgcccctgtgtgtgggacgtgtccggcatggggccggcggcagccggcccgtggcgggtcagcccgccgcgatgcgctgcgcgaggtgcgcgagcgcttcctcgacctggtcgaccaggatcagcgacaaatcgccaggctgcagccgcgcgagcgcggtgtcgatggcaacgaactcgccgcggatctcgtcgatgtagcgcgtacgcgccgcgtcttgcaagccctggcgcaacagcgccatcacctcgccgtcggcacggccgcgctgggccgcgtcctggtacaggatgacgtcgtcgaaggcctggcccaggatggcggtctggtcgcggatgtcggaatcgcgccggtcgcccgcgccgctgatcaccaccgagcgcttgttggccggcatggtgtccacggccgacaccagcgcgcgcatcgcgtcggtgttgtggccgtagtcggcgatcacggtggcgccgcggtagtccatcacgttgaagcgtcccggcacgccggccgcgtcgttcatgaagctcgcgaggccgctgcgaatggtgtcccagtcgagccccacggcccatgctgccgccaccgaggccatcacgttgtcgacctggaagccgatggtgccgttgcgcgtgatgggcacgtcgcgcagcgcaatgcgttcgcgccacgagccttcggccgccaccagcgtgtcctggtcgacatagacggtgcgcttgccctgcgcgcggtgcgtggccatcaccgggtgctggcggtcggcggtgaagaagatcacgtggccggggcagcccgcggccatggcggccacgttggcgtcggcggcgttgagcaccgcatagccatcgggcgcgacgttgcgaaccaccacgcgcttgagcaccgcgaggtcttcgaccgtggtgatgtagttcaggcccaggtggtcgccgctgccgatgttggtgaccacggccacctcgcagcggtcgaagccgaggccttcgcgcagcacgccgccgcgcgccacttcgaacacggccgcgtccacgtcggggtgcatgagcacgttgcgcgcgctcttggggccgctgcagtcgccgctgtcggtctgccggccgtcgacgtacacgccgtcggtattggtcatgccggtgcgcaggccgctcgatgcgagcaggtggttgatgaggcgcgccgtggtggtcttgccgttggtgccggtgacggccaccaccggaatgcggccatcgtcgccgggtgcgaagagcgtgtccatgatggcctcgccaaccgcgcggccgcggccgaacgaaggcgagatgtgcatgcgcaggcccggcgcggcattcacttcgaccacgccgccatgttgttcttcgagcggacgcagcacgttctcgcacaccatgtcgacgccgcagatgtgcagcccgaccatctgcgcggcatcgaccgcgcgtgcggccacttcggggtgcacggtgtcggtcacgtcggtggcggtgccgccggtggacaggttggcgttgttgcgcagcaccacgcgctggccgcgttcgggcacgctgtcgggcgtaaggccctgggcttcgagacggccgacggcgatgtcgtcgagccggatcttggtgagcgacgtggcatgcccttcgccgcggcgcgggtcgaggttgacggcgtccaccagttggcgcacggtggagctgccgtccccgatcacgttcggcgggtcgcgccgcgcggcggccacgaggcggtcgcccaccaccagtaggcgaaagtcgaagcccggcagaaatttctcgaccatgacttcgccgtacacggcggccgagtcgtaggcggccgtgagctgctcgcgcgtcgtgatgttgaccgtgacgcccttgccctggttgccgtcctgcggcttcactaccacgggcaggccgatttccatggccgcagcccagccgtcttcggcatcggagacggggcggcccagcggcacgggcacgcccgcggcattgagcaactgcttggtgagttccttgtcctgcgcgatcgattcggccacgccgctggtgctgtcgatctcggcggcctggatgcggcgctgcttggaaccccagccgaactgcaccaggctgccgctggtgaggcggcggtacggaatgccgcgcgccacagcggcatcggcgatggagccggtgctcgggccgaggcgctcggattcgtcgaggtcgcgcagctcggtgatggcggcggtggcgtcgaagggcgtatcggccagcgcggcggtgatcagctcttcggccagttcgagcgcgcggcgcccgacggcttcttcgctgtattggaaggcgacctggtagacgccatcttcgaccgtgggtgcggtgtggccgaagttgacggcgcagccggcctgcgactgcagcgccacggcggcgttctcgagcacgtgcgcgagtgccagcggctggcccagcaccatcggatgcagttcgccgatggtgggaaaccgcgcgcgcaggcggccttcgaagcccggcagccggctgatggcgttctcgttgccttcgcaggcaaccacggcttcgatggcggtgtggcggctccagagattgggaccgcgcagggctcgggtacgggtgactttcatggggcgacgcgcatcaggcaaattgtggttgtgacgaaagcggctgcgtctgcgagagctgcagcgaggccagcgccgcctgcaggtcggcctcgaaagcctcgacgccggcgccgatgaggttcagcggaatgcccagcgcccaggcggcggccaccgcggccagcaggctctccaggctgacgcccgcgtgggtggcgcgccagatggtcaggcggccgaggcccggcaggaacgattcgctgctgccgttggccagcaccacgcggtcttgccgcaccagcacggctttgccgccggcggcctggtgcgcgctgagcgcggcggcttgcggatcggcggcgtaaagaatgacggcaccgtcgcacagcggcgccaggccggccacgcgcggatcgcccgcgttcagcacggccgtgccttcgccgagcaccacgtcgacctgcgtgcgcagcaccttgaccatctggtcgctctcggtgatgtcgtagtcggccagtgcttcggcgccttcgaggtcggtcacgatgccgacttcgcagcggtcgtaggcgaggccgtcgcgcaggatggtctcggcgccgttctcgatcaccaccgcctgcacggcgcggttcacgagcaggcggtggcccgcctcccaattggcgctgttgcgcgcatcgacgcggcggcgctcgaggaacaggccgtcgcggcaggccaggcccgtgtggcgcccgcccaggttgatgagccaggcgaccaggcgcgcgagcacggcggtgtccttggagccggccacgccgaccaccggaatgcggcctggtgcgtcattgggaaacaggtggtcgcagatggcgcggcccaccgggcgcggcgagccgacggccggcttcaggtgcatcaagaggccggggccggcgttcacttcgacgatggcgccgcgctgcgggccgagcggcttgccgatgtcctgcgccacgaggtcgatgcccgcgatgtcgaggcccaccacgcgcgcggccagcacggcggcgtgcgcgacttcggggtggacctggtcggtgcagtcgttggccatgttgccgttgcgctggatcgtgaccacgcggccggcggacggcacggaagcgccgtcgagttcctggcgcttgagttcgagctgcagcttggcgtcggtgtccagcacgatcaggtcgagcgggtattcctcttcggcgccgcggcgcggatcgctgttgagctgcttttcgatcagctcggccacgttgctcttgccgtcgcccgtgacggtgatgatttcgccgcgcgcggccgccaccacctcgccgcccaccaccagcaggcggtgttcgtggccgcggatgaagcgctcgaccatcacgtcgctaccctcgggctcggcgaccgcgaaggcggccatgacttcttcgcgcgtggtgagttcgagcgacacgccgcggccgtggttggcgtccgacggcttcaccgccaccggcaggccgatgtcctcggcggcttcccaggcttcttcggcgttggccaccacctggccctcgggcaccggcacgccgcagctcgcgagcagcgacttggtcagctccttgtcgctggcaatggattcgccaatggcgctggtgtagtcggtctcggcggtccagatgcgctgctggttggcgccgtagcccagctgaaccaggttgccgctattgagccggatgtgcggaatgccgcggtctgtggcggcggctacgatggccgcggtgctcgggccgaggtagcagtcttcgaccttggccttgaccgcatcgacggctttttgcacgtcagcggcagtgaacgggtcgttgttgatggccgccatcagcaggcggtggccttcggccagcgccacgcgggccacctgctcgtcgcgcgcccggaacaccatgcgatagacgccgtgctccgaggtgctgcgggtctggccgaagccggtcggcatgccggccaggttcaaaagctcgatcaccacgtgctcgagcacgtggcccgaccaggtgccttcggtcagccgctcgatgaagccgccgcgctcgcccacgccgcagtggtgctcgatgagcgccggcagcagggccgtgaggcggtcggtgaagccgtcgatcttgttggacgggaaatcctccagctggcccagatcgagccagacttccagcacgggccggtacgtccagaggttgggaccgcgcaaataattgatgcgcagcaggcggatgtcgtcgaaacgggtcatgcaaacgttcgatgtgctttggccgagcaccacggcgccttcaagcgcgcccatggcaatcggtcagaatcggcgcccgacaaaggacgccatgaagcggtccatgcggcccgcgacgggcaagagtcaaagaaacacaatgcaacatcacgatccagtcggcgcccgggagggcgaaaccgaggcggcctcagacgcgctgaaaagccggctcgcagtcgcggaaaacgttctggtcacattaccggttgacctcgacgatgaacttctgtttacctttgggctcgtggctctcaccgatcggcgcctgctggcgctgcaaccgggcggccagtggtgtgagtggacactatcggatttgtcgctcggtttgcaattgagcgaccattcgggcgtcggaacgctcgaattggtgggtgccggggggcttttggcgcgctggcgttacacgctggccaaccagccggccgcgctgcggctgctgaagcttttcggccagcgcgaaaacggaactgtcgccgaggtgacagccgagcccgacggcgacgaactggccggtgccgacgccgagctgcagaaacccccctcgacctgggtgctgctgcggctggggcgctttgccaagccctatcgcaagcagctgatcacgggctttctgctgacgctgatttccaccgcggcgaccctggtgccgccctacctgaccatcccgctgatggacgacatcctgattccgttccagaacgggcagaagatcgatccggcgcgagtgggcctctatctgagcgggctgctcggcgcggcgctggtcggctggggcctgggctgggcgcgcacctatctgctggcgctggtgtcggagcgcatcggcgccgacctgcgcaccaccacctacgagcacctgctgacgctgccgctcgactatttcggtggcaagcgcaccggcgacctgatggcgcgcatcggctcggaaaccgaccgcatcaacgtctttctgtcgctgcacgcgctcgactttgcgaacgacgtgctgatgatcgtgatgaccgcggtcatcctggtctcgatcaatccgctgctcgctgtggtcaccctggtgccgctgcccttcatcgcctggatgatccacgtggtgcgggatcgcctgcgcaccgggttcgagaagatcgaccgcgtgtggtcggaggtcaccaacgtgctggccgacaccatccccggcatccgcgtggtcaaggcctttgcacaggagcgccgcgaggccgagcgctttcgcgtggccaatgcctacaacctgcaggtgaacgacaagctcaaccgcacctggtcgctgttcacgcccaccgtgtcgcttttgaccgaaatcggtttgctcgtggtctggggcttcggcatctggcaggtggcgcgcggaagcatcaccgtgggcgtgctcaccgcgttcatcgcgtacatcggccgcttctacacgcggctcgattcgatgagccgcatcgtgtcggtcacgcagaaggcggcggccggcgccaagcgcatcttcgacatcctcgaccacgtgagcaacgtgcccgagccggtcaacccggtgaagatcgagcgcgtgcaggggcgcatcgacatgagcggcctgggcttccgatacgggtcgcgcgccgtgatccgcgacctcgacctgaccatcgagcccggcgagatgatcggcctggtgggccacagcggctcgggcaagagtacgctggtcaacctgatctgccgcttctacgacgtgaccgatggcgccatcaaggtcgacggcaccgacatccgccgctttgccgtggccgactaccggcgccatgtcgggctggtgctgcaggagccgtttctcttcttcggcaccattgcgcagaacatcgcctacggcaagcccgacgccacgcgccaggaggtggtggccgccgcgcgcgccgcgcatgcgcacgacttcatcctgcgcctgccgcacggctacgactcgctcgtgggcgagcgcgggcaggggctttcgggcggcgagcgccagcgcatcagcatcgcgcgtgcgctcttgatcgacccgcgcatcctgatcctcgacgaagcgacttcggccgtggacaccgagacggagaaagagatccagaaggcgctcgacaacctcgtgcagggccgcaccaccattgccattgcgcaccgcctgtcgacattgcgcaaggccgaccggctggtggtgatggaccggggcgaggtggtcgaggtgggcccgcacgacgccctgatggcgaagcagggcgcctattggcggctctaccaggcgcagctgcgccaggccgacgaagaagcgagcgaaggtgcgatcgacgaacgcgccggcgcccagttgccgctggtcagccatgcggcccacccggcgggagacgcgtgatgagcaacgacgacaacacccccattcccgttttcggccttgaacgcgacagctttggccgcctggtgctgaccgatgcggagggcgagcgccacgcgggtgtgacgccggtgcgggcctttccgctcagcgcgcccggcgagggcgtgtcgctggtcggcagcgagggccgcgagctggtctggatcgatcgcgtcgacgcgctgcctccgcagacccgcgctttgatcgaggaggagttggcggtgcgcgatttcgcgcccacgctgctgaagctgcacggcgtgtcgagcttcggcgtgcccagcacctggacggtgagcaccgaccgcggcgacaccagcttcgtgctcaaggccgaggaagacatccgccggctcgagggcggcgcactgctgatcgccagcgcgcacggcgtgcagttccgcattcccgacgtgaaggtgctcgaccgcgcctcgcgcaagctgctcgagcgctttctctagcaaacggccggcctgggcgagcaggcgacggcaggcgccgtaccgcgcaggctgcgaaaattgcagtttttgaaccggcaacggctctccgttgaagtgaaatgcccttgcacaccaccgccctcgtcctgttttccggtggccaggattcgaccacctgcctcgcggaggcgctttccaagtaccagcgcgtcgagacgctcggattcgactacggccagcggcaccgtgtcgagctcgacgtgcgcggcaccatcctctcgaagatgcgcgagcgctttcccgattgggcgccgcgcctgggcgaagaccatgtgctcacgctggcggcgctggcccagctcggcggctcctcgctgacggaagaggtggccttcgaaatgcaggccgacggcctgcccaacaccttcgtgcccggacgcaacctgctgtttctgaccctggccggtgcactggcctaccggcgcggcctgcaggtgatcgtcaccggcgtctgcgagaccgacttttccggctaccccgactgccgcgacgacaccatgaaggcgatgcagctcgcgctgtcgctgggcctggagcgccgcctggtcatcgagacgccgctgatgtggatcgacaaggccgagacctggcagatggccgagcgcctgggcggcgcggcgctggtcgacctcatcgtcgaagaaacccacacctgctacctgggcgaccgcgagcatcgccaggcctggggctatggctgcggcgagtgccccgcttgcgacctgcgcaagaagggctgggagcgctacgtctcccgcgcctaggcggcggctggggagaccgaggtttcgagccggtagcgcgcgctgccggccggtgcgtcgtcggcctggggcaccagtgtccagcgctggttgtggaagtcgcccaccgccgcgcggtgcgcaatcgacaccatggcgccgcccgcggccttcacccggtcggagagccgcttgtagagcacgccctcggcctcggcatcaagcgcgctggtgatctcgtcggcaaagagccatgacggcttcttcagcagcacgcgcgcgatggacaggcgctgctgctcgccgcccgagagcttctggctccagacgtcgctgtcgtcgagccggttcaccaggtcgggcagcagcgcgtcaacgagggcctgtcgcagctcggcgtcgctgtagttctcggccggattggggtaagccagggcattgcgcagggtgccatccggcacgtagggccgctgcggcatgaacaccgcgccttccggcaccttcacgtggccgcgcgcaaacggccagatgccggcaaaggtgcggaacagggtcgacttgccgctgcccgatgggccttgcagcagcacgctgtcgcccggcttcacggccagcgttgcgcccgagagcagcgaggtgccgttgggcagtgccacggcgagatcgccggtctgcagcgcgggcgccgtgccgtcgcggtcgagcgcctgattctgggccgcatgggcgcgcatggcatcgtcgaagctggtgagccgatcggtggtggcgcgccagacggcgacgcggtcgtagttgtcgacgaaccagctgagcgaatcctgcaccttgccgaaggccgacgagatctgcatcagctggccgagctggatcgcgccgctgaaaaaccgcggcgcggccacgatgaacggaaagatcaccgcggcctgcccgaagaaggcggtgaaggtgatcaggttcttctgctgcttgatgagcaccagatagttgcgcagcacgctgccgaagcgcaggtcgagttggccgtgctcgaccttctcgcccttgtccagtgcaatggcttcgctgtactcgcgtacccggaccaggtggtgccggaagtcggcctcgaagcgctgttgccggaagttggtgccgatcagcgggcggccgatgtagtgcgtgatgaccgtgcccaccacgcaatacaccaccgccagccagaccatcgcacccgcgatctggtaggtggttccgctcagcgtgagatcgaagttgcccgacagcccccagagaatgcccacgaagctcacgagcgtgaccaccgcgttcaggaggcccatggacagcgacatcgtgtagtcggtgaacatctgcatgtcctcctggatccgctggtcgggattgtccggagtcccgtcgttctgggcgtagcgcgcgagttcgaggtgatagaaagtgcggtcggacatccagcgcgacaggtagtcgcgcgtcatccaggtgcgccagcgcagctgcagcagctgcgtcacatagaacttgagcacttgcaccgcgatgttggcgaaggcgatccagccgaagacgccgacctcgcgccagaagacagccgaatccttgttctgcagcgcatcgtagaagcgcccgtaccactggttgcccagcacggccacgtacacatagaacaggttcagcgcgacgatgcccagcagcatggcgcgtgcgcgccatttctcctcggaacggaagtagggcgccgcaagcgcgaaaacgcggcgcaaaacctgggcgaacgtggcggcacgcgccgtgacggataaagacatgcagatttcctcggtgggcgcgggtgcgccgagacttcgtgaggaaccatggtagtcaaatgttccttaaacgggcctgaagcccgtcccggaacctcgaaaagtgctcagcgcagcatcacccgcgccgcgatttccaggaagtgcttgagcgttggcgtctcgagtccggccacttttgcgtcgtcgtcccaaaggcgcagccgcaccgcgtcgccggcccagcgctgttcggcaaagtgctgcgcggcctgggcgtccatcacgccgccctgcaacgcgaggctgcgcaccgaatccggggagagccgcgagaagtagccgggccgcgtcgcgcaaagatagcgcttggcgtccacatgcaggcggatcggctcgcgcacctcggcgccgaaggctccgcgcagcaggggcatggcgatgtattggtggcggtcgtcgatgccgagttcggtgggcgagcccgacagcgtctggtgttcggcgatcagcaggtgcccgaggtcatgcagcagcgaggccgtgaccagcgcatcgcccgcaccggcctgctcggcaagccatgcgcactgcagtgcgtgttcgagctgcgacaccggctcgcccgcatacgcgaccccgccgcgctcggcgaacaggcgtgcgatctcggcgaggtcgagtgtcatggatctgaaacgaaggcgggaatcgcgaggcggcagcaccccagcttcgcgcattgcagtgacaaggacatgacgaagcctccacaggcgccgcgcaggcgcgtgccttctgacaaatgcctgtcacacgccgctgccagcatcgccgcgttcatggcgcttgccgtgggtactttcttccgcgtacgtcccgctccgtcttcttttccgaggtttccccatgctgcgtcgttctatccgctggtcttgcgtgccagccgctctgctctcgctggcctttgccgcttcggcccaaggccgcaccgagctgctggtctacaccgcgctcgaagccgaccaggtgcaggcttacaaggcggccttcgaaaaggagaacccgagtgtcgaactgaagttcgtgcgcgactccaccggcatcgtcaccgccaagctgctggccgaaaaggccaacccgcaagccgacgtggtgtggggcctggccgccacctcgctgatgctgctcgacaaggaaggcatgctccagccctacgcgcccaaggggctcgacgccatcaagccgacgatgcgcgatccggccaacccgcccaagtgggtcggcatggacgtgtggtcgtcggccatctgcttcaacaccgccgaagccacgaagaagaacctgcccaagcccaccagctgggccgacctgaccaacccggtctacaagggccagatcaccatgcccaacccggccgcatcgggcaccggctacctgatggtgtcgggctggatccagatgatgggtgaagaaaaggcgtggaagtacatggacgcgctgcaccagaacatcggcatctacagccagtcgggcagcaagccctgccgccaggctggtgccggcgagttcgcgctcggcatgtcgttcgaataccgcgccaacaagaccaagcgcgacggcgcgcccatcgacatcgtgctgcccaaggaaggcctcggctgggacatggaagccaccggcatcatgaagaccagcaagaagcaggacgccgccaaggcgctcgccgattgggccgtgacgaagcaggccaacgagctctacgcgaagaacttcgccgtgctcgcgctgccgggcatccaggagaagctcgagttcgtgccgggcgacgtcgagaagctgctcgccaagaacgacttcacctgggctgccgcaaaccgcgaccgcatcctgacggagtggtcgaagcgctacgaatcgaagtcggaaaagaagccgatgtgatcgtgcgtcccggctgcagcacatgacgagtttcctttcccttcgcggcatcggcaagtcctttggcgccacccgcgtgcttgacggcatcgatctcgacatcgagcccggcgaattcgtgtgcctgctcggtccctcgggttgcggcaagaccacgctgctgcgcatcgtgtgcggcatcgagcgtgccgacggcgggcagatcctgctcggcgggcaggacatcgcgggcctgccgcccgcggcgcgcggctttggcgtggtgttccagtcgtatgcgctgttccccaacctcacggcggcgcagaacatcgcctacggcctgcaccccaccggcgcactcgcacgcgagatggccaagcgctcgcgcgagatgctcgacctggtcggcctcgccgcgcacgccgacaagtaccccgtgcagctttcgggcggccagcagcaacgtgtcgcactggcgcgcgcgctcgcgcccaacccgcgcctgctgctgctcgacgagccgctctccgcgctcgacgcacaggtgcgcgccagcctgcgcagcgagatccgttcgctgcagaagcgactgggcatcgtcaccatcatggtcacgcacgaccaggaagaagccctctcgatggccgaccgcgtggtgctgatgcacaacggccgcatcgagcaggccggcacgcccgacgagctgtaccgccagccgcgcacccgcttcgtggcgggcttcgtcggccgcatgaacatgctgcccgcgaccgtgctggccgatggcaaggtgcgcgtgcgcgacagcgaactgttttgtgcaccgggcaacctgagtgtcggttcgcaggccaccgtgggcattcgccctgagcacgtggtggtcaggcgcttcggcaccgagctcggcgccaacagcttcgcggcgcgcctggtcgataccgaattcttcggcaaccgcacctccgcgcggctggtctgcgaaccgctcggcatcgagatcgaggccgagctgcccgccgatgcgcgcaacggtggcgacgagccgttggtgcccagcagcatggtgcacatccaactgcccctgaatgcactctcggtgctggcgcactgagccatgagcagcctccccgaagccatcgccgctcggccgatggcgatggcgcgcagcagcgccttcgaccgcgagcgctggctgacgggcgcggccgtctcgctgctcgtgctgctgctggtcgtgatcgtcgcgctgcccgtcggcgcgctggtcggccagagcttcttcgaccgcgcgggcgccttcgtcggcctcgcgaatttcgcgcgctacctcgacaaccccgcgctcgtgcagtcggccttcaacagcctgtggctcgcggcggtgagcgccgtgatctgcacggccatcgcctatgtgtacgcctatgcgctcacgctgtcgtgcatgccggccaggggcatgttgcgtgccgtggcgctcattccgctgcttgcgccttcgctgctgccggccatcagcctggtctacctgttcggcaaccaggggctcttcaaggggctgctgggcgacgtgtcgatctatggcccgctcggcatcgtgctcggttcggtgttctggacactgccgcatgcgctgctgattctcaccaccgccatggccacttccgatggccgtctctatgaagcggcgcagacgcttggcgcctcgcgctggcgcatcttccgcaccgtgacgctgccttcctctcactacgggctcatcgtggccgcgatggtggtattcgtgctggtcatcaccgacttcggcgtgcccaaggtggtcggcggccagaccggcgtgctcgccaccgacatctacaagcaggtggtcggccagcagaactttcagatgggcgccgtggtcggtctggtgctgttgataccggcggtgctttcgttcctggtcgaacgccgcgtgcgcataaggcaggccgcggcgctctccgcacgcgccacgccctaccagcccgagcccgtggcatcgcgcgaccgcgcgctgttcgtgttctgcgggctcacggcctgcgccatcctcgtgatgatcggcatggcggtgttcgcatcgctcgccacctactggccctaccagctcgcgccgtcgctgaagaactacgacttcagcaacatggacggcggcggctggggcagctacctcaactcgctgcggctcgcgttgtgcgccgcggtcgcgggcgcgctcgtcaccttcatctcggcctatctggtggagaagccgcggcacttcggcctgctgcgcgagctgctcaacctgctcgccaacctgccgctcgcggtgccggggctggtgctgggcgtgggctacatcttcttcttcatctcgccgtcgaatccgctgcacgggctgtatggcggcatgacgatcctcgtcgtctgcaccgtcgcgcacttcttctcggtggcgcacctcacctcgctcaccgcgctgcgccagctcgatcgcgaatacgagctggtgtccgagtcgatgggcgtgcccttctggcgcaccctctggcgcgtgcacctgccggtggcgctgcccacggtgctcaacgtcggtggctacttcttcgtcaacgcgatgaccaccgtgtcggccgtggtgtttctctactcgccgcagaccacgctggccgccatcgccgtgctcaacatggacgatgccggcgacgtggcgcccgctgccgccatggcctcgctgatcatgctcacggccgccgtcggccgcggcgtgttcgcgctggccggacattggacgctcgaacgcacccaagcctggagaaaccggtaatgcccggaacacctgacaacaaagacagtttcgacctgatcgtcgtcggcgccggcatcgtcggcctggcccatgcctacaccgccgcgcagcgtgggctcaaggtctgcgtggtcgagcgcgatgcggcctgcatcggcgcatcgatccgcaacttcgggttcatcaccatcaccggccaggcgccgggcgacacctggcgccgcgccatgcattcccgcgaggtctggcaggacatcgcaccgcaggccggcatcgacatcgtgcaccgcaatctctggcttgcggcctaccgcagcgaggcacacgacgtgctcgaagccttcatgcgaacgccgatgggcgaagcctgccagctgctcgatgcggccgacgcgcaggccaaggcgccggcgctgagcctggccgatgcacgctcggttctcttcagcccgcacgagctgcgcgtcgaatcgcgcaccgccatcggcctgctcgcgaaatggctggccgaagtgcacggcgtggtgttccgcttcggggagaccgtgcacgaggtggaaacgccgcgcgtgcgcacctcgcgtggcctgctccgcggcgagcgcgtggtggtctgcaccaacaccgatctgcacggcctctttgccgaccgcattgccgcccacgacctcaccctgtgccgcctgcagatgctgcgcgtgaaacccgaggcgggctttcgcctgccgggctcggtgatgatggacctgagcctggtgcgctacgagggctatagcaccttgcccgaggcggccgcattgcgcgcgcggctgcaggaggaagaggccgcatccctcgcgcacggcattcacctgatcgtggtgcagagcgccgacggctcgctggtggtcggcgactcgcatcactatggcgacgcgcccgagccgtttgcaatggaagaagtcgaccggctcatcctgcgccacctgcgcggcacactgaatctcgaatcagcgcagatcaccgaacgctggaccggtgtgtacccctcgtccaagaccacgccctgcgtgatcgatgcgcccgacgaggccacgcgcgtggtgctggtcaccagcggcaccggcgcgagcacgggcttcggcattgcgcacgacgtattcatgacttggtaagtatcttcatatgaacgcccacaaccactccaagctccaggccgtcgtcttcgactgggccggcaccatcatcgacttcggctcttgcgcgcccatgggcgccttcgtgaagctgttcgagcagttcggcgtggacatcagcattgctgaagcgcgcggccccatgggcatggccaagtgggaccatatcaaggcgctgggcacgctgccgcgcatcggggcgcagtgggaagcgaagcagggccatgccttcaacgatgcggacgtggaccacctccatgaagtgttcacgccgatgaatgccgccagcgtgcgcgaccatgccgacttcattcccggcgcgctcgacgcggtgaacgccgcgcgcgaacgcggcctcaagatcggctcgaccaccggctacaaccgcccgatcatggaagtggtcgcgcccatcgcggcggccggcggctacgcgcccgacaacctcgtgtgcgccggcgacctcgcggaaggccgtccgtcgccgctcatgatgtaccgctgcttcgccgaccttggcgtatggccgccgcacaccgtggtcaaggtcgacgacaccggcgtgggcctgcaggaaggcctcaatgccggcacctggaccgtgggccttgcggtgagcggcaacgcggtcggcctcacgctcaccgaatggctggcgctcgatgctgcacagcagcaggagcaccgcgagcgcgccaccgaccagctccaggccgcaggcgctcactacgtcatcgacagcgttgccaacctgccgaacgtgctcgaagacatcgagcgccggctgcaaggcggcgagcggccggcagccgcctgacggtcgcccgacgttccgattcggcacggcgtccgacttgacttgcagggcggcgggcatagcatccgccgcatgagaagcacagcctttgttcttctgttctgcatcggcctggtgatggccggctgcaacgacaagcccaagccgggcgggccggtgcccaaggcttcggtggatgtcgtgatgccggcgcggatcgtgggttgattcgccgccatcgggcgcgcgggcggccacgtgccgcctgccattgcgcgcccgcgcctatgcgcctgcgcttccgggggtatcctcggcgcggagaaaaacaatgaagacctcggagacgaccacccatcaggcggactcgcgctatgccatgctgcggctcggcctcacgctgctgatcatgacggtcggcagcagcggcatgtacgtggtgtccgtgatgctgcctgccgtgcaggccgagttcggcgttgcccgcgccgatgcttcgctgccgtacacgctgctgatgctgggctttggcgtcggcggtgtgctgatgggacggctggccgatcgcttcggcgtgatgtggcccctgctgggcggtgctgtcagcctgggcctcgggtacgtcgcctgcggcatggccgacggcatcgtggccttcaccgtggcgcaggcggtgctggtcggcctgcttggcagtgccgcggcctttgcgccgctggtggccgacacctcgctctggttcgtcaagcggcgcggcattgcggtggcggtgtgcgcgagcggcaactatgttgccggcgccatctggccgcctattgcgcagcatttcatcgaaaccgtgggctggcggcagacctacatcggcatgggtgtgttctgtggcttggcgatggcggcgcttgcgctcttcatgcgagcccggccgccgggcatcgctatcgagcctgccggttcggcgcctgccatgggggtgggcgcagtgcgcaagcgcgacatgacgcggccattcggccttagcatgggcacggcgcaaggcctgctgtgcgtggccggcgttgcctgctgcgtggccatgtcgatgccgcaggtgcacatcgtggcctattgcagcgacctgggctacggggccgcgcgcggcgcgcagatgctgtcgctgatgctggccttcggcgtggtgagccggctggtatcgggcgccatctgcgaccgcatcggcggcctgcgcacgctgctcctgggcggcgtgctgcaatgcgtggcgctgctgctgttccttcccttcgacggcctcgtgccgctctacgtgatctcggcgctgttcgggctgttccagggcggcatcgtgccgtcttacgcgatcatcgtgcgcgagcactttccgcccgccgaagccggcgcgcgcgtgggcacggtgctgatgttcacgctcttcggcatggcgctgggcggctggatgtcgggcaaggtgttcgacctgaccggcagctaccacgcggcgttcctgaacggcatcggatggaacctgctgaacgtgagcatcgcggcgatgctgctgttcagggttcggcatcttcggcttcgcaccgccgcggcgtagcgccctcagagatcggccaggcccatcgccggatcgctcaccgtgtgccggccggtttccacccggccggcgaagcggcgcgagtagctggggtcggcatcgcaggtgaccgcgaagtcgtaccactgtccgctggcggcaagctcccagtgctgttcggcggcggcgccggcggcgactgtcgcgatccacgggccgtcatcgcgataggccttggcgcgcaccgtgaacttgcaggccttggtgccgccgctgcgcatttccaggtagacgttgccgttggcaatgtcgtagcacacgcgcacttcagggttggcgccgttcgtgcgcagcgcattgagatcgcccttgaagtggcggtgaaagccattggggccgagcacccagaggtcgtagaagccgctgttgtcggttgctgcgttccatgtgtcgtcgagcgtcttgccgggctcgaccatgtagcggcgcggcaggcggccgaggttgagcatgtcgtacacatggaacaccgcgcctgccttgcccgtgttggcgaacagcaatcgaacggtgcctgccgcggcgtcggcgcgtgcgctggtgtgcagctcatagggcagcgcacgcgagggccgcgtgccggtggcctggcgcggcaactgcggatcgagcggcagcgggacctggcccagcgcctcctggctgagccgcagctggtcggcttggtcgcgggtgctgcggccggcgagcgtgggcagcggctcgtcgttgggattggcaaagttgaaggcgctcgtgaggtcgccgcacaccgcgcggcggaaggcgctgatgttgggctccttcacgccgaagcgcgcctccaggaaacgcagcacggaggtgtggtcgaaggcttgcgagttgacccagccgccgcggctccatggcgacaccacgtacatcggcacgcgcgggcccgggccgtagacacggccgtcgggcgcaggctgcacgatgctgccgggcggcgccgcatgcgtgaagtattcggggcccaggtccgaatcgggcagcgtggtcctgccggcaaggctgccatcgccgaccggcgagggggccgagggcgagggcaggtggtcgaagtagccgtcgttctcgtcgaagttgacgaagagcacggtcttgctccacacctcgggcacggcggtgagcgcatccagcacctcttgcaggaaccacgcgccctgcaccgggctggaggggcccgggtgctcgcagtagatggacggcgcgttcatccagcagacctggggcagcttgccctcgcggatgtcgcgcttgaaggcgtcgaggtagttctcgggccgggtgcccggcagcgtattggccacgcccttgtacagcgggttcttcgcgttgtccgtcgccgcgtcgtaggcgcggtagggcagcggctggccggtatcggcatagggtgtgttcggctcgccgccgctcgacaccggaaagcccgaatcgaggtttgcctggcggaactgccggaaggcgccgagcatgttgtcgccccattcgtcgggcatgttctggtagctgatccagcgtacgcctgctgcttcgagacgctcggcataggtcttccacgtgtagccggtgcccaccgacccggggaggccgtcgatccagtcccactcgttgcgcacgaaggccgtgctggtcgcgcccgcgccgttggtgccggtgagatggaacgagcgattggcgtcggtgccggtgtgcatgctgcagtggtacgcatcgcaaagcgtgaaggcgttggccagcgcgaactggaacgggatctccgcttgcttgtgatagcccatggccttggcggtcttgtagcgcggccactggtacatgcggccgctgtcccaggcgttctggctgtcggcccagtcgtggggcgtgccgccgtcgcgctgcgcgttgcccttgctgctgtccaggtggtagggcagcaccagcttgccgccggcatcggtctgctgccacacgttcaatcccttgggcaacgggatggtgaagcggtcgccgaagccgcgcacgcccatgagcgtgccgagtagtggtcgaacgatcggttctcctgcatcaggatgacgacatgctcgacgtcctggatggtgccggtcttgttgttggcgggaatggcaagcgcgcggcgaatgcttggcggaaaggccgagagtgcgagcgcggcggcaccggtggtggcggtgcccgcgagaaattggcggcgggaggtcattgccgtgcagccatcacagatcggccaggcccatggccgggtcgctcaccgtgtgcctgccggtttccacccggccggcaaagcggcgcgcatagcccgcgtcggcatcgcaggccacttcgaagtcgtaccacgcgccgctcgaggccaggtcccagtgcagctcggccttggcgccgccctgcacggtcgcggtccacgggccgtcgcttcggtaggctttggcccgcacggtgaacttgcaggcgctcttgccgccgttccgcatttccaggtagacgttgccattggcgatgtcgtagcacacgcgcacttcgggcgcggcggcatcgcccgcgcgcagccggttgaggtcgcccttgaagtggcggtgaaagccgttggggccgagcacccacaggtcgtagaagccgctgttatcggtcgccgcgctccacgtgtcgtcgagcgtcttgccgggctcgaccatgtagcggcgcggcagccggtcgaggttgagcttgtcgtagacgtggaacaccgccgccgccttgccggtgttggcgaacagcagttgcaccttgccgccgatgctgtcggcgcgcgcgctggtgtgcagctcgtagggcagcgcgcgcgaggggcgagtgcccgtcgcctgccgcggcagctgcggatcgagcggcagcgcaacctgggccagggcttcctgggacgcgcgcagctggtcggcctcggccttgctcttgcggcccgccagcgtgggcagcggctcgccgttggggttggcaaagttgaaggcgctcgtgaggtcgccgcacaccgcgcggcggaaggcgccgatgttgggctccatcacgccgaagcgcgattcgatgaagcggatgaccgaggtgtggtcgaaggcctgcgagttgacccagccgccgcggctccagggcgacaccacgtacatcggcacgcgcacgcccgggccgtagacgcggccgtcgggcgcaggctggctggtggtgccaggcgggttcggatggttgaagcgctcgaaggcaacgtccgatgcgggcagcgtggtcttgccggcggccgtgccgtcggcgttgagcgatggcgccgcgggtgaggggtagtggtcgaagtagccgtcgttctcatcgaaattgatgaagagcacggtcttgctccacacgtcgggcacggcggtgagcgcgtccagcgtttcctggatgtaccagccgccctgcaccgggctcgacgggccggggtgctcggaataggttgccggcgcgatgatccacgacacctgcggcagcttgcccttcttgatgtcctggcggaactgctcgagaaaaccgccatcgggcatggtgttggcaatgcccttgtagagcggattgccggcgtcgtcgctggccgggtcgtaggcgggcgaggccacgtcgttgctcacgggcttgcccgaggcctcgttggcgagccggtattgcttgaagccggccagcgggttgtcgccgaagttctcgggcatgttctggtagacgatccagctcaccttggcttcctgcagccgctcggggtaggtcttccactcgaagcccttggccgagctgtcgatcgagtcccactcgttgttgaccgaagccacgttcgcgccggtggggccgttggtgccggtccagaggaacatgcggttcgaatttgtgccggtgtgcatgctgcagtgatagccgtcgcacagggtgaacgcgttggcgagcgcgaactggaagggcagctcggcctccttgtagtagcccatggccgcgttggtcttgtagcgcgaccactggtaggtgcgcccgccgtcccaggcgttctggccatcgatccacgagtgcggcgtgccgctcacgcgctgtgcgttgcccttgcggctgtccaggtggtagggcagcaccgggttgtccgtggcatcgccctgctgccagacgttgcggcccttgggcagcggaatggtgaagcggtcgccgaagccgcgcacgcccatgagcgtgccgaagtaatggtcgaacgagcggttttcctgcatcaggatgacgatgtgctcgacgtcctggatggtgccggtcttgttgttggccggaatggcgagcgcgcggcgaatgctcggcggaaaggcggcgatggcgagcgcggcggcaccggtggtggccgtgccctgcaggaatctgcggcgtgagttcatggtcttgttgtcgtgttcggtcatgaggtttggcaatgggcgcttcgatggacgctcaaggcgcgcagcgcatgtcgggcttggtgccggtgtcgggcgggttgccgggcgttgccggcgtgccggtagccggcgttcccgagccgggcaggaagcccgagaagccgccgccgccatcgccgccgccgcaggcggaaagagcgcaagccaggatcagtgcgggaacgagccgcacgggcagggatgaaagtcgcatggtgggttccttggagttgtcgcgtgtgggcactcggatgcggcagaaaaatggcgcctcgaaggcaccgcgcaccggacagacacaagactagggagaacccgttacatcgccatgaacgagcgatgacaaggcgaaaggcgccgaaggcgccaggaggacgaagcactgcgaaggtgcccgccccggacgaggctcaatgctcgttgctgatgccgctggagacgtggccggcgggcacgtggcgtgccgcggcgtcgacgtggccggtctggtcgtcgaagaagaaatcgggttcgaactcgcgcaggaattcgcccttgggcaggccgccgaggaacatggcttcgtccacgcggatgttccacttcatgagcgtgcggatcgcgcgctcgtgcgcgggcgcgctgcgcgcggtgaccagcgcggtgcgtatgcgcatctgcgcattgccggccatctgcaggcgatgcagcgcggtcagcaagggcttgaagggaccttcgggcaagggcagatcggccttgctgagttcgtgggcctggaaggcatcgaggccctccgcctggaacacgcgctcggcttcgtcggagaacagcaccgcgtcgccgtcgaaggcaatgcgtacttcgttgggccacgcatcgctggccttcacagattcgacgagcacccgtgcggccggaaagcctgcgacgagggcctcgcgcacgtcttctgcattgaccgacaggaacaagtgcgcgcgcagcggccgcaggtagccgaagggcgggcggccttgcgtgaacacgccgcgctgcagcttgatgtcggccgccgcgctggagcggaagatgcgcatgccagagaccgggtcgttgcgcgagaggatcaccacctcgacgcgctgcacgccgtcgtcgttgaagcgcagcagtttgcggatcagcgagtacgcgatgcccggcgcggccggcacgtcgatgcggtcgagctgcagtttcatgtagccctcgttgtcgccggcctcgaagatcctgttttcttcttcgaggttgaacagcgcgcgcgacgagatcgcgaccacgagtttgtcttcgagcgtgacgggcatgaggtgcggtgcttcctggcggcgttacttgacgaactggttcagctggatgataggcagcatcaccgccagcacgatgagcatcaccacgccgcccatggccacgatcagcaagggctcgagaatggtcgccaggtgcatcgcgcggcgctgcacttcggcgcccagctggttggcggcgcgctgcagcatcagcggcagcgtgccggtctgttcgcccagccgcgcgaacatcgagaccagtcccggaaaacgttttttctgcgccagcgccgaggccagcggcgcgccttcgcgcaccagcaccagcgcatcgagcgcatccgcgcgcatggcgcggttgcccaaggtttcggaggccgcctgcagcgcgcgcaggatcggcacgccggcggttgcgagcatggccagcgtgctggcaaaacgcgccgcgttgtagccgcgcgcgagcttgccgaccagcggcagcttgagccaggcggcatcgaacttcagccggaaagcctcttgcgccagcgcgagccgtacggcaattgcggcgaacagcacgccgccgagcatccaccacccgtaattgcgcaccgccgcactcagcgacagcatcaccgtggtgagaaaaggcagcgaccgcttggtgcccgcgaacacctgcgccacctgcggcaccacatagctcacgaggaagatcacgatcacgatcgccacgagagtgacgatggccgggtagagcgccgcgccgacgagcttctgctgcagcgcctgccgttcctcgaggtcgtcggcgagccggtcgagcacgaggccgaggttgccgctttgctcgcccgcgccgatcaccgcggtgtagatgggcgaaaactcgcgggggtgagccgccagcgcacgtgcaaacggcgagcccgcgttgacttcggcgcgcagcgatgcgaccaggttgcgctgcggctcggtctcggcttcgtcggtcagtgcggtcaatgcgcgttcgagcggcaggccggaggacacgaggcccgcgagctggcgcgtccacaccgcgaggccggtggagctgaaaaccctggcaccgccgccgagccatcggcgcaagcccccgttgccggtgccgttgacgtggctgctgccgactggcgtgaccgacagcggaatgagcgcctgcgcgcgcaacaggctgcgcgcgctgcgcgcggtgtcggcctccagcacgccttcgcgcgactggccgctggcatcgatggcttcgaaggaataggcgggcatggcgaagtgaaggactgcttattcgcgcgtgacccgcagcagctcggcgcgcgaggtgatgccgccctgcaccagccgttcgccgtcctcgcgcatcgagcgcaggccgccgcgcgcgccggcttcgaagagcaggctctcggccgccttgccatgaatgagcgcctgcacttcatcgttggccaccagcagctcgaagatgccggtgcggccctggtagccggtctggccgcaggtctcgcagccggcgccgccgcagctggtgcagaccttgcgcaccaggcgctgcgcgagcacgcccagcagcgacgagctcagcaggaagggctccacgcccatgtcggtgaggcgtgtgacggcgctgaccgagtcgttggtgtgcagcgtcgccagcacgaggtggccggtgagcgaggcctggatggcgatctgcgcggtttcgaagtcgcggatctcgccgatcatgatcacgtccgggtcttgccgcaggatggcgcgcaaggccttcgcgaaggtgagctcgatcttggcgttgatctgcgtctggcccacgcctggcagctcgtattcgatggggtcttccaccgtcatgatgttgctgcggcccgcgtcgagccgggccagcgccgcatacagcgtggtggtcttgcccgagccggtggggccggtcaccaggatgatgccgtgcggctgcgcgatgaggcgctcgaagcgctcgagcgtgtcgccctgcatgccgaccgattcgagcgtgagcttcgattcggtcttgtccaaaaggcgcagcaccgcgcgctcgccgtgggcgctgggcagcgtggagacgcgcacgtccactgcgcgcgtgccgatgcgcagcgagatgcgcccgtcctgcggcagccgcttctcggagatgtcgaggtcggccatgatcttcaggcgcgagatcagcgcggcgtgcagcgcgcggttgggctgcaccacttcgcgcagcgtgccgtcgatgcgaaagcgcacggatgaggtgcgctcgtagggctcgatgtggatgtcgctcgcgccgtcgcgcgcggcctgcgtgagcagcgcgttgagcatgcggatgatgggcgcgtcgcccgcgctttccagcaggtcttcgacggccggcagttcctgcatcatgcgcgagaggtcggcgtcgctctgcacctcgctcaccaccgcggctgcgctcgactcgccctgtgcataggccgcgctgatgcgctgcgccagcgggccgtcggccagcacctcgaaagcctgcacgccgtacttgcgcgtgacctcgccgagtgcgctgcgcgagggatggctcgacatccacagcgtgtagtggccgtcgtcggcttcctcgagcaacagttgctggctgcgtgcgaatgcgtagggcagaggatggcgcatgggcgggtcagggcagttcgcgcgaggtggtcgggtcggccgtgggcggcagggcgccgcgcaacgggctcgggcgcagggtgcgcgtgtcggccggcgggcgcggcggcggaatgagctgcgtgccctggatgcgctcgctgctggtgttgctgctgctggtgcgatcggccgagcggggcggcggtgcttcgggcagcacgggcgcggagtcgacgccgcgcagcatgatgttgtcggtgttcggctgcgtgcgctgctgcatgccgcggatctcgtcgtagcgatcgtaggcaaacgcttcggtggaggcgccgtcgcgcatgacggcagggcgcaggaacatcatcaggttgctcttggtgcgcgagcggatttcgttcttgaacaggttgccgagcaccggaatatcgccggccacgggcaccttctcgatcgtgttgttgtagtcgtccgaaagcaagccgccgagcatgatgaggccgccgtcttccaccagcacgctggactcgatggagcgcttgttggtggtggggccgttggggttgctgaccgtgttctggtcgaccgtcgaggtctcctggaagatcgtcatcttcacggtgccgttctcgttgatggtcggtcgcacgcgcagcgtgaggccgacgtccttgcgctccaccgtggtgaacgggttgatgcccaccgagcccgaggtgctcgcgtactggccggtgacgaagggcacgttctgcccgatgacgatcttggcctcttcgttgtccagcgtcagcaggttgggcgtcgagagcacattggcgtcgccgtcgctgttgaagaaattggcgatcgcgcccaggatgtactggccgccgatcttgccggcaatgccgaggttcaggccggtcgatggccgcacgttggccacgtcgcgcgtggccagggcctgcgtcagcgcgaggatgttggcgctggccaggctcgagttggtgccgatgaccgcgttgttgcccagcgcgctctgccactggacgccgaagttggcggccttcttggcgctgacctcgacgatcagcgcctcgatcatgacctgggcgcgccgtccgtcgagcttgtcgatcaccgcgcgcatctggcgatattgcggctcgggcgccgtgatgatcagcgagttggttgacggatcggcctggatctgtccgccagtcgacggctggttggcgttgttcagcggcgcattggcggccgccgagccgctttgcccgccgaggctggcctgctgcatggcctgcggtgcgctggcctgcggctgcacctgcccgccgccacctgcggcccccggcgtgccctgtgtgcccggcagctggttggcggccatggcggcgcgcagcgtggccgcgaggcgcaccgcgtcggcgttcttcaggtagaccacgtagatgttgccggccgcgccgttgctgctctcggccggggcgcggtcgagcttctcgaccagcgtgcgcaccagcgaggcccgcgccgggttggctgcgcgcaggatgagcgagttgctgcgcggatcggccagcaaagtggtgcgaaacgacgcgtcggccgcgcccggtgcggcggcgcccggcgttgcgcctgaaccgctgccgtccaccagccgcgtgatcagcggcagcatgtcggtggcgacggagtgcttgagcgggatcacctcgatgtcggacgcattgggcacgtcgagcgccgcgatgatgcgtgccagccggcgcatgttgtccgcgtagtcggtgatcacgagcgagttgttgcccgggttcacgttgatagtgttgttgggcggaatgagcgggcgcagcaccggcagcaggctgttcggcgattcgtagttgagcctgaagatctgcgtgacgatttggttgccacccacggagcctgcgctgggcgtggcggtgttgacggtctgggtctggagcttggcgtccgcttcgggcaccaccttgtagagcccctcggcctccaccaccgcaaagccctgcaggcgcagtgcggacgcgaactggttgaacgcggcggccggggcgatggctcggtcggtgacgaggttcatcgtgcccttgacgcgcgggtcgaccaccacgtcgcggccggtgaccacggccatggtgcgggccacggcctcgatgtcggcgttggcgaagttgagcgtgatgggctcgccccggcgcggcgcatcgggactgccggcctgtgcgaacgcggtcggcacggcctgcatgaaggtggcggcaatcagcatctgcgctgcgagtgcaacgatgccgaggcggctgccgtgcgaagtcagtggcttcttcatgatcaacccagggtgatgatcgaacgcgcgttctcgcgccgcccgatgatgttcaacaaattggaaagcgcgtcttcgcggccggctgcagcgttggcttcgccattgaagcgaaaggcggtgccgttccagctgccgctgccgttcagctgcaggctgccttcgcgcgtgctcaagagcaggctcggccggctgccgccttcgagcgtgaggcggtagctgcccatcggcttcagggtcgaaaggctcgacgacacgtcggtggcgtcgagcgtcgcctggcccgcgatgcgcagcacggggccgtcccactgcatcgacagggccttggtggaaaggtcgagcgtgccctcgagcttgagcgtgttccagggcgcgcccaggccggccagcaaagtggcgggccagcgcgaactgccgtcgccccattgcagctgcatgccgtccgcgcgtgggctggccttgagttcgagcggccgggccgtgcagcagggcaggtcgagcaccgcgaacatgccgttccaggtgggccgcatgcgccagttgagcgacccgggcagcgacaccgcctcggcgccgccggtaccgcttgccagcaccaccgcggccgcaccgttccagaccgtgccgcgcgggttgacgagcagcagccggccctggctccagctcgacagcgccgcggccagccaccgggccggtgcgaacagaacgagcgcgagcagtgcgccaatcacgatgccgagtagggcccagcgccagccgcggcgcggcgccggatcggaaagggaagggcgcgtcaccatggcgggtgtgctcaacgggccgcgggcagcgccatcaccagcgtgccctcccagcgcaccttggcgggttcggggtccttgttgctcgcggccggcggcgcggcggccgcgcgggtcaggtgggcttcgcgcggcacggcatgggcattgccgcgcgcctgcgcgagccattgggccagggcatcggccggcaccgcgcgcagcgtgacggtggcggcgccgtcgccgctggccgtcatgagctgggcattgcttcccaggctctggcgcaccgaggtttcgagggcgcgcagtgcgtcgtcgcgggtcaggcggggctgggcttgcagcgccttggcgcggttctgcaaggtggccatctgctgcaattgcgcatcgagccgcgcgtgttcggcccgcgccgcggccagcgtgcgcagtgcgggagcgagcgcaatccaccacagcagcgcgagcacgacgagcccggccgcgatggcgagcatgcgccgctcgcgcagatcgagggaagcccagcgggcgcggagttgttcggcgaagttcatcgggaagcctcggcctgcaccagcagcagatcgccctcggcgcgcacgctgtagccgcgcgggcccatggcgcccgaaagccgcgtgagctccgaaggctgcagggccaggccgcgcaggcgcagttggccggcgctgtagtcgatggcgctgggcgtgcggcccggcggaaggttggtggcgagcgcgccgatcatcggttcgaagtcgctgcccgcgacgtcgcccaccgcctgctgcagcgccgcgacctcgcgtgccatctgcaccggcgcatcgaccaccagtttcacggcaggaaaggtctgggtcagcatggtcttgacggcctgccgcttggcctcgagtgcattgcgctccttccaggcccaggcgttgaggccgatcagctgggtcagcagcaaggcgatgacgccccagcgcgcggcgcgccactcgggtgcatagcgcagcgtctggaccacggatgcgaatttcttgccggcgcgggcgcggcccgtgacggcaaggtcgaactgcgcgagctcccacggcgagcgcgcagcctggagccagcgttgcggtgcctgcacgatgggcaggcggcgctcgagcagatgctcggcggcctcggcgacggcgggttcggcggcgatgacggcggtgtcgagcggcaggctgccggcgagagccagcccggcacccgccagcggcagcgagaccacgccgtcggcatcgcacaccgtgagctgcggcgcctcggcctcgccggtgacctgcagcagcggcgggccgtccgcaggctgcggcgcgaattcaggaacgatgcgcaccacgcgccgccccgccgattcgaggccctggacgaggctgcgcagccagatgcggttgcaggccgccacccagaccggcgggccggccttggcctcgggttcgagcgcgaaatgcaaggcttcgggctcgtccagcaactgctcctcgagcagtccgtcgagcacggcgcgcagtttcgaggtgctgcccatgctgcccttgggcagggtgacccggtgccaggaaagcgccgccgcgggaatgccgagcatgacttccgtgcttgccggcaacagcgcgagcaacgcgcggccgtggtcgtgcaacgcgatgccgtcgtcccctgcctgggcccagtcgtactcgccggcggtatcggccggaggaaggggggcaatgagcagcagcggggtcatttcgatttgggaagggcgggtgattgtagggtcgcgcttattgcatgagtgctactttatttgtagcgtgtgacgtagatgcgacgggggttggacgatttttttggtgcaagaaattggcagaggaagccgtgactcagggtttagccggagaggcggtcatgccggccccgcgattgcgccagatcgtcttcacggtaatgccgtcgcgttgcaggagcgagcgttcttccacccaggtgcggtcgagccgcagcttgccgtagacctcgaagaactgggtgctcacgctgtgctggttggcgttgaactgggtgccgccgttgggaagggcggtgttggcgtcggcgatctgcttgaagaacgagcgggtgcgtttttccaccacctggcgcgcatcgctgatgctcagcgaaggcaggctggcgctgatggcctcggcactcgcggtgttgatgttgagcggcgtgcgtatcgggaggatcgtcacgtagggctcgagggcggccgcggtggagggcgaaaggccgagccacaccagctgcgaaacctcctgcggcatcagcggcgccgcgccggcatcgccgccgcccgcggcgtcggtaccggtggcgagcgcgcgcaccagcgaggcggtcatcacgctgagctccgaagccggcaggccgaggatgttgaacagcttggtgaaggtggcgacgctcgcgggcaccggcttgttgccgtcgaccagcgacagcacgttgagcttggattgcgcatcgacgatgcggcccgacagaaaggcgtcgggcagcccttcgaggttgtcgctggccacgtttttctcggccgagagaaagctggcgagccttgcttccgcgagcggcacggcccagggttcggccaggtggtcgggcccgccggtgagggcgtcttcgcgcaggatcaggcgcgaccagtcgagcgcgccgaccagcacccacgccgcctgcacgcgtccgcgctcggcggcctcgacttcggacgagcgccattgctgccacagcgcggcggcggaaaaggtggcgaccagcatcacggtcagcatggctgcgagcagcgcggcgccggactggcggccggcacttgcgcgcgggcggctcgcagaggaagggagaggcgtcgtcacgatcgcggcgctcccaccgtcggcttgacccagtcgcgcgtgatggcgcccgccagtccgtcgccgggcgacaggttcagcaccaggcgaacgccgtcgggcatgttcacgatggcgcctgtggggttggccgggttcgcagggttggacgtgccgctcggcaattcgcccgccggagtccaggtgttctcgcggaaatagaagagctgccagccgtcgaccggcatcagggcggtttctccgccgccgccttcctgtgcccaggaggcggccatgttccaggcctgctgccattcgccgcgcgtgctgaagggctgcgattgccagcgccgccagcgggtgccgtcgactcccgagcgcagcgtccacgccaccaccagcatggccggtgcggccgcatcgctgctgcggcgcgtgagccgcagcacgcggccgttccaatcgatggggcgggtttgcgcgagcgcggtcacggcgtcgaggtcggcgctccattgcgcgagcgtggtctgcagcgtcagcaccgcgtcggcgcgctgctggttctgcgtggtggcgcgcgacatggcgtcgagcccgcgccagctcacgatcgcaagcagcgccatgacggcaatggccaccagcagctcgatcagggtgaaacccccgcgggttcgccggtttgcgaagcggtgcatcagaagcggcccaccacggtcgagatgcgcagcaccggcgcgttggcctcatcgcgcacctgcacgtcgacgcgccggaagttcgggttgagcgtggcgatggtggaggtggtcacgttgaaggaaacgccggcctgcacgcagatggagcccgaatcgcccacggccggcatttgccgagccaggcgcgccttggcgagttcgttttctgcgcacaggtcggccagcagcaggtcggactggcgctgcgcgttgcgggtcagcgacatggtggcctgcgacccggccgccagcgccagcgcgacgatgccgagcgcaatcagcacttcgatcagcgtgaatccgccgcatgccgaccggcgcccggttgtcatggcgtgctcacggtgaagggtcgcaggccgtcggtggcaacgcgcagcgaacgtgcgggcgggccttcggaataaagaacgatctgctgcgcggcaatgatcggatcgggcccgagcagcacggccggaatcggcgcgccgttggccagcgcggcctgggcgctgatgccgctggtggcccagccgttgggcaaggcgtcgggcggcaggccctcgaacacgaagctgccgccttccaccaggcgccatcgcaccgcgacgccgcttgcgcgcgactgggcgcgcgccgattcgagcagcgccgccagccggtcggcctcgcggtcgagccgggccgcgctgctgtcgcgcatcgcgaaggtcacgctggcggtggccatcgcgatgatcgcgatcaccacgatcagctcgagcagcgtgaagccgccggtgcgcctactgccagctgccgatgtcggcattcttgccctcgccaccggcctggccgtcggcgccaagcgagagcacgtcgatttcgcccttgatgcccgggttcatgtattggtacggatggccccacggatcgttgggcagcttttcgacgtacggcttccagttgggcgcggccgggccggcggtggggcgcacgagcagcgcctgcaggccttgctcggcggtgggatagcgctggttgtccaggcgatagagcttgagcgcctgcatcaggttgttgatgtcggtccttgcggcggtcacgcgggcgtcgtccgcgcgctcgatcacgtttggcacgatcagcgcggcaaggacgccgatgatgaccagaaccaccatcaattcgatcagcgtgaatccgcgctgggcggtgcgggtggcggcgcgaaggatttttttcatagcttggatgacatggttcggaaggcgcgctgcatgataatccgcggccatgacaagtccctattccgccgcgcgctggcacgcccccgttgcaaccacgggactctgggcgctggccgccggtgcggcggtgttctggggactgcggctcgcgagtccggcccagcccgtggcggcggcggccacgatgccccgggcgtcggtttcggccgatgcggatgcggtggcgcggctgctcggcgcggtttcggcatcggaagcggcacctacgatgccggaggccgccagccgctttgcgttgtcgggcgtggtggcggatccgttcaaccagggagcggcgctgatctccatcgacggcaaacccccgcgaccgtttcgcgtcggttcgcgtgtcggcgacaactatgtgctgcagtcggtgggggtgcgctcggcgacgctgggcgccagcgttgggggcccggcggctttcacgctgcaattgccggtgcgggcgccgatcagcgtcgggagcccgattcagccgggcatgacgccatcgccgcgtcccagcgggctgtttcctgccacggtgcccgccgtggtggcgccgccgtctgccgatgcggctgctgcgccgcagcagatgcctccaccggcgcctgcgccgcaacctcctgcccaactcgcgcagtagggcgagggggcgcaggccgccgctcggtcaggcctgcaggaacagccggtacgccgggttcgccgtttcctcgacgtacgggtagcccagcgtttcgaggaacgcatcgaaggccgccgcatcgctggcaggaacctgcagccccaccaggatccggccgtagtcggcgccctggttgcggtagtgaaagaggctgatgttccagttgggccgcatcaggctcaggaacttgagcagcgcgcccggacgctccggaaagacgaagcgcagcagccgctcgtcatgcgcaaggctcgtgcgcccacccaccagatgccgcagatgttccttggcaagctcgtcgtgcgtgagatcgagcgcatcgaaaccgtggtcaatgaaggtctgcgcgatggtggtcgattcaccgcgtgtggacgtggtcaagccgacgaacacatgggccttggtcgcatcgctgatgcggtagttgaactccgtcacgttgcgtggcgcgccgccggtggagtcggtttccttcgattcgatggccggcatttcgccgaccagttcgcagaagcggcgaaagctgccgcgctcttcgggaatggtcaccgcaaacagcgcctcgcgctcctcgccgacctccgcgcgttcggccacgaagcgcagccgatcgaaattcatgttggccccgcacaggatggctgcgtaggtctcgccgtggcggccatgcccggccacgtactgcttgatggcggccaccgcgagcgcgccggccggctcgacgatgctgcgtgtgtcgacgaagacgtccttgatggccgcgcaaaccgcatcggtatcgaccgcgatgtattcgtcgaccaggttgctggcaatgcggaatgtctcttcgcccacgagcttgacggcggtgccgtctgaaaacagcccgacgtcgggcaggctcacgcgctggcgcgccgccaccgattgcatcatcgcgtcagagtcgttcatctgcacgccgatcaccttgatctccggacgcaccgccttgatgtagttggccacgcccgagatgagcccgccgccaccgatcgcaacaaagaccgcgtcgagcgggccctggtgctggcgcaggatctccatggcgatggtgccctggcctgcgatcacgtcgggatcgtcgaacggatgcacgaaggtcaggccttgctgggcctgcagttccagcgcgtgcagataagcatccgaatagctgtcgccatgcagcaccacctcgccgccgaatccgcgcaccgcatcgatcttgaggcgaggcgtggtcacgggcatgaccaccacggcgcgcgtacccagcttgcgagcgcccagcgccacgccctgcgcgtgattgccggccgatgcgcagatgacaccacttgcgagctgctcgggcgtgaggtgcgccatcttgttgtaggcgccgcgcagcttgaagctgaagaccggttgctggtcttcgcgcttgagcagcacggtgctgccgagcctttcgctgagcgcgttggctttctccagcgcggattcgaccgccacgtcgtaaacgcgggcgttcagaatttttctgagatagtcggcgggcgatagtgccggaacagggacgtcgcgcacggttttttccaaggggagtttcaattgataaatgacgatgataagaggcatcgggattgcatacgggccatgacatggacacaaatgtcataaacctcatcctgagagccccagcggcgaacgattccggtttttttgagcgcacctatcccgcgatccatccgtccgccagtcagttaacaaatgagcaaaatttgttatcagtttctgtcagcgacctttccaaaggattgatgcaggcagaagcggcgcgtgtacagcgcggcgaaattgggcgacctacctggcaagtgatgggcaacagattgcgggcccatgtcgtccctttgctgggtgccgttcaagcacaggcgtttgccaccgccgatgcgcaacgcctgatcgaccatctcggagagcagggcttcaccagcacgacgattgcgcaataccttgtgttgctgcgaaaggtggtgacgcacggcgtcaacatcggtgtgcttcgcgttgcgccggcctttccgaaggtcaaggtgcgcagccagccgcgcggcagcttcagcgttgcggaataccgggccgtcgtggcagctgcgcgcagattgcgcgggcagtcgcatcccgtgctcgaccagctgacatccggcgagcgcttctggattgcgcgcgagttgctcgtcatgccggaggagttgccctggttgattcgctggatggtgaacacctttgttcgtccgagcgatatcaaactcatgaagcacaagcacatagaaatcgtgcgcggcaagcacgtctatctgcgaatgaacttgcccgaaaccaagcggcacagccagcccatcgtgagcttgcgtcccgctgtgcgggtctatgaatgcttgctcgatcgtcgtcgcgagcaaggctctggtggcgcggaagactacatcttcatgccgcaattgaagaaccgtgaacacgcgctggcggtgctcaactttcttttccattgggcgctcgaggtgattgcgctcgagaaggggccgctcggtcaatcgagaacgctctattgcctgcgccacaccgcgatcacattgcggttgttgtacgggcagggcatcgacatgctgaccttggcgcgcaatgcacgcacgagcgtgaacatggtcgagcggttctatgcgtcggttctgaacggtgaaatgaatgtgggcctgctgcaaagcaggcgtggccgtgcaagctgaacaaagccaaaaagccgcccggcttgcgctgggcggcttgacactgaatcgactcgaactggctggagccagcatcggatcagacccgtgatcgatcagaaggcgtggcggatgccgaagtcgtagccggtcgaattgcggggttcgtagccagcggcagtggagaatcggggggcaccaccgacggtgatcggcgcgccgttcttgttcgcgacccgggcaaccgtggtgtacagcgcggtccgcttcgacaggttatgcacgtagccgattgcaaacttgcggctgcgtggatcgtcgttgccatcgaagttcgctttggcctgggagtaggcaacgcggatcaatccagcgccgaccggtgcagtggcaccgatcaagaatccattgaggccgatcttttcagagcccagctgagatgcatagaattcgttggtgacgcgggacaattcggtgaagagcttcacaacaccgaagtcatacgaagcgccaaggttcaatgttcttgcgtcgatacccgttcctgcgccgttgttgaagacatcgctcttgccatatgcaagcccaacgtccagcggcccgtttgcgtagccgactcgaccgcccacgtagcggcccgtcttgcttacttgaacgccactggtcttcacgttctcgtgcagtccgtattgcacttgaccatagaagcctcccagattgggcggcagaaaatagccaatggtgttgtttgcacggacatagttcgagtcggaggggagtcccaagcccgtcaggatggcactgtgtgatgagttaatgacattggtgccaacgccgttggtgccgaacggatcgaacacggtgtcgttccagaaggtcggggtgtagtcacggccgaggcggacttcaccgaaaccacccgacaggctcacggtcgaacgacgtgagaagctgataccggtggaggaagcgccgtcgtcgttggacatcggcgattcgagccagaagctcgctgccaggccaccaccgaggtcttcggtaccacggaagccaaggcggctcgagttgtaacccgagttggccagcgcggtttggctttgcttgaagctggagccggtgatgagggaacggctgctggtttcgtagtggctgatcgacgcgtcgaccacaccgaagagcgtgacggacgactgagctgaggcaacaccggcaacagccagggcagccagagcaactgcccttcgggcgcgaaaacctagagtgggcctggcccgagccgggagcggcgacgccgacaagaaaaaagccccgagctttgcagctcggggctaaatccaccaattggaagggtggaggagacaaccggtgcgcacatgttcgtgcgcgatgaaataaagtatatcgactgtttgttgcgttgcaacaagcaagtgacacttttcccacacacaagttgatttcagcgactttttttgctgaacaccctgattggacctgacgaagatggaatgcacagtaacttggaccggcgacgccggcacccgttcggccatgggttttgtggccgaaacgggcagcggccatgtcttgacgatggacggcgcgccggatacggcaaaaccggagaacggtgggcagaacctggctgcccgccccatggaaaccgtgcttgccggaaccggtggctgtacggcctacgacgtggtcctcatattgaagcgtggccgccaccgcgtggagcgctgcagcgtcaagctgaccagtgaacgcgccgagaaggaccccaaggtcttcacgaagatccacatgcacttcaccgtggccggcaagggcattccggcttctgccgtcgagcgtgccgtcgctctgagccacgaaacctattgttcggcgagcatcatgctcgcgaagacggccgagatcaccaccagcttcgatctgatcgaaacctgagccgcgaaagcttcagatccggtgcgccagcgtagtcatcacgcgggaggcgaaccgcatcagggccttcgcgggcgccggcaattccgccgcaccggcgtcgatagcctgcgcggcatgccgtgcttcatcgaccttcatctgctcgaccaccgccctcgatgcgctgtcggcaggcggcagacggcccagatggctgtccaggtgggcctccacctgacgctcggtttccgcgacaaagcccaagctgagcggatctcccaggcgtccagccaccaggcccagcccgaaggcgcccgcataccagagcggattcaagatcgaaggccgcgcacccagatcgtccagccgctggcgggtccaggccagatggtctgtttcttcatgtgaggcttcgagcaggcggttccggaggacgggatcgcgcgccaccgccgcctgcgcggtgtaaagcgcctgcgcgcagacctcgcccacgtggttcacccgcatcagtgcgccggcctcgcgccgctccgagtcggtcatttcgccgggcgcctggagcggggcaggcatggcacgcgtggcatgcggccgggcaaaaagggtacgcaatgccgcatccgccgcggtcaggacgggatcgagcgaagaagtcatgcctctatttgaacgtatggggaaaagaccaggcgaaacacttgcttcatttcacattgtggttcgtgaggcggcccaagcctttgttgcaggactgcaacgaaacgcacgggccacccgacttttcgggcgatttgttttgccctgccgcagcggctctggtgcaatagcatcaacttcccaaaaggaggttggcccggggtccggtgggagcactaagtgccagtcacagtgagcccttcgcaccggagccctatgtttaaccttggagaaacttgcaatgaaaaaatctctagttgctctggctgccctggctgttgccggtgttgcctcggctcagtcgtccgtcacgctcttcggtgtggtcgacgcgtcgatcagcggctactcgagcacctcgcgtgacctgaacagtgccacgatcctgaacccgttctacctgaaccagggcagcgtcaagacgagccgtcgtgaactggcgaactcgggctacaactccagccgtatcggcttccgtggtacggaagacctcggcggtggcctggctgccagcttctggctcgaagccccgatctccaacgacgacggccagcaaggtatcgcgacgttcgctcgtcgttcgaccgtgagcctgtcgggtggtttcggtgaagtccgcctcggccgtgactacaccccgaccttctggaacgacaccgtgttcgatccgttcggcaccaacggcgtgggtaccaacctggtttcgacggccaacaccgccttcggcaacttcctgaccccggctgcttcgaccgctccgttcaccaacgttgccaacagcaactacgtgcgcgcaagcaacagcatcggctacttcctgccgccgaacctgggtggtttctacggccagctgcagtacgctttcagcgaaaagaccaagtacgatccgggcaccgctacgcctaacgtcgcgaacaactcgcgcgctggccgttacatcggtggccgcttcggctatgcaaacggtcctctggacgttgcagttgcctatggcagcagcacgattggcgatcagttctacgtcggcacgaccaccaaggtcaacacgctgaacctcggcgcttcgtatgacttcggtcccgtgaagctcttcggtgaagtgtcgcgcgccaagaacaagatggacttcgaagtcgagccgttcctgggcggccgtcctgacatcgacctgaccggctacctcctgggtgtgaccgttcccgtcggtgctggcctgatccgcgcttcgtactcgcgcgtcaagaccgacttcaacgctcctgaagtgctgttcgcaccttccgttgctgacccgaaggccagcaagctggctctgggctacgtgcacaacctgtcgaagcgcacggctctgtacgcaacgatcgctcgcgtgagcaacaagaacggtgcagcctacactgttggtggcccggctttcatcagcaacgccgtcttcaccccgaagaactccaccggctacgacttcggtatccgtcacgctttctaatttgaggctggcgtgagccagctttgaatcgaaagactaagaagccactcgacgaaagtcgggtggcttttttatttggtgcgcagctgatgcatcggctcaggtatacgcaccatcggcgtgccccccccggggaacccccgtgcgggcacgcaccttgcactgctagcatgccggttcactctgtttgttgaatgattgcctttgtcctgcgccgcttgatccaagccgtgatcgtcatgatcgcggtcgcgttcatcgcctttcttctctttcaatatgtaggcgatcccgtcgtctttctgcttggccaagacgccaagcctgagcagattcgtgatctgcgcgccgcattggggctcgaccagcccttctttgtgcagttctggcactttctcgtcaacgccgcacagggcgaattcgggctgagcctgcgccagggtgcgaaagtctcgcgcctcatcggcgagcgctttccggccacactcgaactcgcgctcgtggccgccgtgctggccctgttcattggcatcccgatgggcgtctacaccgcactgcgccggggcactttcctgagccaggtgttcatgaccgtgtcactgctcggcgtgtctcttcccaccttcttgatcggcatcctgctgatcctcgtctttgccgtgctgctgggctggttcccgagtttcgggcgcggagaaaccgtgcagttcggttggtggagcagcggtcttttccgggctgatgggtggcatcacatcatcctgccggccgtgacgctcgcgatcttccagctgaccctgatcatgcggctggtgcgtgccgagatgctcgaggtcttgcgcaccgactacatcaagtttgcacgcgcccgcggtctgacgaaccgcgccattcatttcggccacgcgctcaagaacacgctggtgcctgtgatgaccatcaccggcctgcagctcggcggcctcattgcctttgccatcatcaccgagtcggtgttccagtggccgggcatgggactgctgttcatccaggcggtgacctttgccgacgtcccggtcatggcggcctacctgtgcctcattgccttgatcttcgtggtgatcaatctcgtggtcgacctgttgtatttcgtggtcgacccgcggctgcgcgtcggcaaggcgggaggacattgagatgacggttgccgcagcagcaccccggctgcaagcctccggccgggcgtttgcgcacatcgcgagcttctacccggagatcacggcgtttcgccgcgacctgcacgctcaccccgagctcggtttcgaagaggtctacacggcccgccgcgtgcgcgaagcgctgcgtgcctgcggcgtggacgagatccacgacggcataggcaagaccggcgtggtgggtgtcatccgcggcaggtccgcagccagcgggcggatgatcgggctgcgcgccgacatggacgcgctgcccatgcgcgaagacaacgacttcggctggcgctccgccaacgatggcctgatgcacggctgcggacacgacggccacaccgccatgctcgtcggtgccgcgcgctaccttgccgaaacacgcagcttcgacggcaccgcggtgctgatcttccagcccggcgaagaaggttttgctggcgcgcgcgtgatgatcgaagacggccttttcgaccgctttccggtgcaatcggtctatgccatgcacaactggcccggcatgccggccggcaccgtgggcatcaaccgcggcgccatgatggccgcggccgaccgcgtcaccatcgagatcaagggcaagggcgggcatggcgcccatgcgtaccagaccatcgaccccgtggtggtggccgcgcacatcatcacggccgcgcaaaccatcgtctcgcgcagcgtgcggcccatcgatgctgcggtcgtcagcatctgcgcggtgcaggccggcgacctgggcgcgatgagcgtgattccgggcgaggccacgctcgtcggtaccgtgcgcaccttcagcgcccgcgtgcaggcgcaggtcgagcagcgcctggccgagctgtgcacggccattgccgcgggcttcggcgccaccgccaccatcaagtacgagcgcatctatccggccaccatcaacaccgcccccgaggcgatgttcgcggccgacgtggccgagtcgctcgtgggtgcttccaacgtcgaccgcagcatggagcccagcatgggcgccgaagatttttccttcatgctgcagaagaaggccggcgcctacctgcgcatcggccaggacgcgaggaacggtgccttcctgcacaacagccgctacgacttcaacgacgagatcctgccgcttggcgccgcattgcatgcggggttgatcgagcagggcatgccgctggctgctacccgcagcgagcagccaaggaaagacgccgctaccgcggcgccttgatgtatttccgattccaacccgaggagtgttctcaatgagtttccagaagaagaaggcggccgcggtcgcagttttgtgcgtgctgggcaccaccagcctcttggccggcgcgcagaccatccgcatcgcaaaccagggagatgcgttgtcgctcgacccgcattcgctcaatgaatcgttgcagctcagcaccaccgccaacgtctatgaaacgctggtcggccgcaacaaggacctgagcgttgcgcccctgctggccaccagctggaagcagacctcgcccaccgtgtggcgcttcgaactgcgcaagaacgtccagttccacgacggcacgcccttcaccgccgacgacgtgctcttcagctttgcccgcgccgccggcgaaggctccgacatgaagtcgaacaccaccgacatcaaggaagtccgcaaggtcgacgcccacaccatcgagatcgaaaccaagggtccgttccccattcttcccgacgtcatcacccagctcatgatcatgagcaagaagtggtgcgaagagaacaaggccgtcacgccggtcgaccgccgcaagggcatcgaaaacaccgcttcgttcaaggccaacggcacgggcccgttccgcgtacgcgagcgccagcccaacgtgcgcacggtgttcgtgcgcaatcccacctactggggcaagatcgaaggcaacgcgcaagagatcgtcttcacgcccattgccaacccggccacccgcgtcgcggccctcgtgtccggcgaaatcgacgtgatggaacccgtgccggtgcaggacgtggcgcgcatcaacgccagccccaatgcacgcgtcatctccggccccgaactgcgcaccatcttcctgggcatggaccagaagcgcgacgagctgctgtactcgagcgtcaagggcaagaacccgttcaaggacaagcgcgtgcgccaggccttctaccaggccatcgacatcgtcggcatccagcgcaccgtgatgcgcggcgcctcgcgtcccaccggcctgatggtgggccccggcatcaacggctggaccgaagcgcaggacaagcgcctgccctacgacgtcgaggccgccaagaagctgctggccgaagccggctatccgagcggcttcgaggtgacgatgaactgcccgaacgaccgctacgtgaacgacggccagatctgccagagcgtggcttccaaccttgcgaagatcggcgtcaagatcaatcttgccgcggaaaccaagggcacctacttccccaagatcctgcgccgcgacaccagcttctacctgctgggctggaccccgaccacctacgactcgcacaacgcattgaccgcgctgacggcgtgccctgacgacaagaccggtgccggccagttcaacctgggtgcctactgcaatcccaaggtggacgagctgaccaagaagatccagtcggaaaccgacaagcccaagcgcgacgcgatgatcaaggaagccttcgacctgcacgccgcggacgtcggccacctgccgctgcatcagcaggcgctcgcctggggtgtgagcaagaaggtggcgctgacgcagatggccgacaactacatgcccttcaagtggatgagcatcaagccgtgatcccgtcggccgcccgccgatgggcggcctgagtggctcgatcctgggcccgcttcttgcgggcccatccttttttctcacgatgaaaaaaacacttgcccgctggctcgacagcgatgtcggctacagctttcgcacttcgcccgtggcgatggtggctgcgctcatcgcactggcctgcctgttctgcgcggtctttgcaggatgggtgtcgccgcacaatccgttcgacctcgcgacgctcgaactgggcgatgcgcgcctgccacccgcgtggagcgccgaaggctcttccaaatacctgctcggcaccgacgaccagggccgcgacattctctcggccgtgatctatggcgcgcgcatctcgctgatcgtcggcatcgtgtcggtgatgctctcgatcacggtcggcgtggtgctcggtctgctcgccggttttctcggtggctggctcgactcgttcctcatgcgcctgtgcgacgtgatgctgtcgttcccgcccatcctggtggcgctgctgattgccggtgtcggccgcgcgctgttccccaatgcgcatgagtcgctggccttcggcgtgctcatcatctccatctcgctgaccggctgggtgcagtacgcgcgcacggtgcgcggctccacgctggtggagcgcaacaaggaatacgtgcaggccgcgcgcgtgaccggcgtggcgccgctgcgcatcatgctgcgccacgtgctgcccaacgtgatggggccggtgatggtgctggccaccattcaggtggccaccgccatcatcaccgaggcgaccttgtcgttcctgggcgtgggcgtgccgccgacttcgccttcgctgggcacgctgatcagcatcggcaaccagtacctgttctccggcgaatggtggatcaccgtgttcccgggcctgatgctggtgctgattgcgctcagcgtgaacctgctgggcgactggctgcgagacgcgctgaacccgcgcctgcgctgaagtaaataaaaaggacaacgccaacatgacgctgctccaggtcaaaaacctcgtcgtcgagtttccgcaccgccgcggcacgctgcgcgcgctcgacggcatttccttcgacatcgcacccggtgaaatcctcggcgtggtcggcgagtccggtgccggcaagtcgctcaccggtgcggccatcatcggcttgctcgagccgccgggccgcgtggccagcggggaaatcgtgctcgaaggccagcgcatcgacaacctcggtttcgatgccatgcgccccatccggggccgcaagatcggcgcgatcttccaggacccgctgacttcgttgaacccgctctacaccgtcggccggcagctggtggaaaccatccgcgcccatctgccggtgaccgacgccgaggcgcggcgccgcgccatcagcttgctgcaggacaccggcattcccgccgccgagcagcgcatcgaccattttccgcaccagttttcgggcggcatgcgccagcgcgtggtgattgcactggcgcttgcggccgagcccaagctcatcgtcgccgacgagccgaccaccgcgctcgacgtgtcgatccaggcgcagatcatccagctgctcaagcgcatctgcaaggagcgcggcgcggcggtgatgctgatcacgcacgacatgggcgtgatcgccgaaacctgcgaccgcgtggccgtgatgtacgcgggccgcatcgccgagatcggcccggtgcacgaggtgatccaccagcccgcgcatccctacacctccggcctgatggcctcgatccccgacatgacgagcgaccgcgagcggctcaaccagatcgacggcgcgatgccgcggctcaatgccattccgaagggctgcgcctacaacccgcgctgcccgcgcacctttgcgcgctgcctggccgagcggcccgagctcatgcacgcgggcgccacgcgcgccgcctgctggctgcacgatgccaccgatccgcaccagggccaggccgaactcgcagcgcggcaccacgatgcgcagcgcgccggcgaacgcgccacgcccgacgcagccgcaccgattgcggaggtgacccgatgagcgcagtggtcgaaccccgcaaggcagaaggcggcgaaccgctcgtggtcgcccacgacctggcccgcaccttcgacgtgtcgccgccctggctcaaccgcgtgctcgaacgcaagccgcgcgtgctgctgcatgcggtggatggcgtgagcttttccatcgagcgcggcaagacgctggcgctggtcggtgaatcgggctgcggcaagagcacggtggcgcgcctcctggtcggcctctatgcgccgacgcgcggcgggctgcagttcgacgggcaggacgcgcatgccgcgttcaagacccccgaaggccgcaagctgcgccgccgcatccagatgatcttccaggacccttacgcgagcctcaacccgcgctggatcgtcgaggacatcatcggcgagccgctgcgcgagcacggcatcctcagggacaaggccgagctgcgcgagcgcgtgggcgagctgctcaagtccgtcggcctttcgccgctggacatgagcaagtacccgcaccagttctcgggcggccagcgccagcgcatctcgattgcgcgcgcgctcgccacagagcccgagttcctggtgtgcgacgagcccacctccgcgctcgacgtcagcgtgcaggcgcaggtgctcaacatcatgaaggatctacagcgccagcggggcctcacctatctcttcatctcgcacaacctcgcggtcgtgcggcacgtggccgaccaggtcggcgtgatgtacctgggccggctggtcgaggtggccgacaagcagaagctcttcgccaagccgcagcatccgtacacgcgcatgctgctcgacgcgattccgcagatgaagcacaccggccgctcgcgcacgccggtgcagggcgaagtgccgaatccgctgaatccgcccacaggctgtgcgttccatccgcgctgcccgcatgcgaatgcacgctgctcggccgagcggccgaagctgttgagcatcaagggcgtgcaggtggcctgccatgcggtggaagaggggcgcatcggctgaaaagcgtgcgcaaacgcactgaggcgcgcgggaaaccggtgcagagtgcggtgatgacgatgaagaagcccccacgcgcagacagcacagacagcagccacacgcttcggccggagctcggccgccgcggctttctcatgggctccgcgctcggggcgaccgcaacgctggcctcgctgtgttcgttgtcgcacgccgccgccggtgccccatcgcagcggatgccggccatcttcatcggccacggctcgcccatgaacgcgctggccgacaacgccttcacgcgccggctgtcagcatggggccgggagcttccgcgtccctcggccatcctgagcgtttcagcccactggctgagccgcggtgccactggcgttggaatgcaggagcggccgaagacgatccacgacttcggcggctttccacaggcgcttttcgacatcgagtatccggcgccgggccatcctgcgctcgcacgcgaagccctgggcgcggtgcgacagacctcggtgatcggcacggaacaatggggcctggaccacggaacctggacggtgctgaagcacctgtatccgaaggccgacatccccgtttttcagctcagcatcgactacgacaagccggcggcttttcactacgccgtcggccgcgaccttgcggcactgcgcgacaagggcgtgctcgtgatgggcagcggcaacgtggtgcacaacctgcgggccaccgaccgcggcacgcccgatgggctcaaggcaagccggccatgggcgcaatcgttcgacgatgcggtgaaggccgcgcttgcgggccgcgacgaccgggcgctggtcggctacgaaaaactcgagggcgccgccactgcggtcgccatgccggaccactactttccatttctctacgcgctcggtgctgcggggacgggcgaacgcgcgaaaacgatctacgaagggttccagtcgggcacgctcggcatgcgttgcgtccaattcggctgagcgcgccggcctactgctcctcgccccacgagaaaccatcgcgcgcaatcatcgcgctcgatgcgctcgggccccaggtgcctgcggcgtacggccgcggtccaccgtccgatgcccagctgtcgatcagcggctcgacccagcgccaggcttcttcctgctcgtcgctgcgtacgaacaggttcaggcggccatcgatcacgtcgagcagcagccgctcgtaggcgcccacgcgctcggcgccgaagcgcttgtcgaagtccaggtcgagttgcaccggcgccagctgcgcggcgctctggtggccgttgctgcggcggttgtcctgtgcctgcgcgagcatgtgcagctccagcccgtccttgggctgcaggttgatcaccagcttgttgaccgcacccgagggcgcgcggtagatcgcgtgcggcgtcggcctgaagttgacctcgatgcgcgcatcgcgcgacgcgagccgcttgccggtgcgaatgtagagcggcacgccggcccaccgccagttggcgatttcggtgcgcagcgccacgaaggtttcggtccggctctcggggtcgacgccgggctcgtccctgtagccctgcacgcgttcaccgtaggccgtgccggtcgtgtactggccgcgaatggcatgcaggcctagcgtttcgggtgtccagggcttgagcgcgcgcagcaccttgagcttctcgtcgcggatggcatcggcatgcgagttgatcggcggctccatgccgatggcgcagaccagttgcagcgcatggttctgcaccatgtcgcgcagcgcgccggtctggtcgtagaaggcgccgcgcttttcgacacccaggtcttccgcgatggtgatctggatattggcgatgtgctcgcggcgccagatcggctcgaacagcgcattgccgaagcgcatggcaaacaggttctgcaccgaaggcttgcccaggtagtggtcgatgcggaagacctgtttctcttcgagcaccttgcacaccgcggcattgatggcgcggttggacgccaggtcatggcccagcggcttctcgagcaccacccgcgtcgatgggccgttgagccccgccgcggcaatctgctctaccacctgggtgaagagcgctggcgccgtggccacgtacatcaccaccgtgtcggcgttgcgctgcttcagcaggtcggaaagccgcgtgtagtcggctggcttggacaagtccatgcgcaggtagtacagcagcgaggcgaacttctcgaactcttcggccgaagggcgcttggcgccttcgacggcattgaagcgcgactggatcagttcgcggtactggtcgtccgaaaggtcgtcccgcgccacgccgacgatgcgtccgtctttcggcaggctgccgtgcctgaaggcctggaacagcgcgggcatcagcttgcgccatgcaaggtcgccagtaccgccgaacagaacgagatcgaagctcatgtgtcgaatttccttttgtcttggtgccgaggggctgtctgtttcaaccgaatggtacttgtaccaattcatgaaacctgtacgaaagctacgctgcaccccggccgggaggcctatttttgttttggaggcgaggttttcacatgaagaagctatttgccgctgcggccttgctgggtttgtcggccgccgcatcggcccagggcacggtgaatgtcatctgctcggtccaggccgaatggtgcaacgtgatcgccaccgtgtatgcacgcaccaccggcacccgcatcaacatgtcgctcaagggctcgggcgaggcgctggcccagctcatcgccgagaaggacaaccccaagaccgacatctggttcggcggcaccggcgatccgcacctgcaggcggccgaacagggcctcacgctcgaatacaagtcgcccacgctggcgcagcttcacccctgggcccagcagcaggccaggcagtcgggctacaagacggtgggtatctattcgggcccgctgggcttcggctacaaccccgagctgctcgccaagaagaagctgcccgtgcccaagacctgggccgacctgctcaagcccgaatacaagggcgacgtccaagtggccaaccccgcgtcgagcggtaccgcttacaccataatcgccacgctggtgcagctcatgggcgaagacaaggccttcgactacctgaaggcgctgcacaagaacgtggggcaatacacccgctccggcaccggtcccatcaaggcggtggcacgcggcgaaacggccgtgtcgatcagcttcgtgcatgacggcccgggcgagaagatgcagggtttcccggtcgagaccatcacccccagcgatggcaccggcgcggagatcggctccatgagcatcatcaagggcgcccgcaacctcgaggccgcgaagaagttctacgaatgggcgctgacgcccagcgcgcaggaactcggcgccgccaacaagcagttccagctgccgagcaacacaacggccaagctcgatccgcgcatccccgacttcaagaagatcaagttcatcaattacgactacgccaagtacggcgccagcgccgagcgccggcgcctgattgcgcgctgggaaaaagacgtcaactcgctgccgcgctaagtgggcaccgtcgctgccggcgccgcgccggtcaatccggccgctgcggcctcggcccggcggtcgcagcgctggatctgggcctgggtggcgctcggcttcgcggcctatctcctgctgccctggtacgcgatccaggattcgacctggtacgaggccgttccccaagtgttcggccaggccgagggcgccaacgggctgatgcaggcggccatgcagggccgcagctggctcttcgtcggcctcgcgggcctggcgatgtgcgccatcggcgcctggctgccggccggccgcgcgcaggggcgctggctgctggcgggcggtgcgatcggcgccatcggccttgccgttgcaggctttgccatcggcgcgcgcggctggagcttcgcggcactcaacgcgcagttcggcgagctggccgtcaaccagttcggcatcggcgcgggcggcttcatggcgcttaccgcgctcacgctgctggcggccttcggcattgcgcggctcgggctcttcaagggcgacctgttcgtggctgcggcggtcatcggctgtggcgtgctgatggcgctgttcatcgcctatccggtgagcaaggcgctggccggtgcgttccttgacgaagacgggcgatggtcggtcaccgcgttcatcgcgcgcgtgttcaccgagcgcatctgggggctgggctgcattgccggcggggtgcgctgcggcgtggcctggaacacgctggtgctggccttgctcaccgccgctggcaccaccttcctcggcacgctgatggcgctgatggccgagcgcggcagcaagcgcgggcagggcgcgctgcgggtgctggccttgctgccgatcatcacgccgcccttcgtggtgggcctggggctcatcctgctgttcggccgtgcgggcatcgtcaaccagctgctcgagaacgtcttcggcatcgagccgacgcgctggttctacggcatgccgggcgtgctggtggcgcagctcttcgcgttcacgcccattgccttcatgatcatgcgcggcgtggtgcagggcattgcgcccagcctcgaggaagccgcgcagatgctgcgcgccgaccggcgccgcaccttcttcaccatcacgctgccgctgctgaaaccggggctggccaatgccttcctggtgggcttcatcgagagcattgcggacttcggcaacccggtggtggtgggcggccagttctcggtgctgtcgaccgacatcttctttgccattgtcggcgcgcagtacgaccagggccgcgcggcctcgctcgcctgggtgctgacgattttcgcgctgggtgttttcgcgctgcagcggggtgtgctcggcaagcagaactacaccaccgtgagcggcaagggcgacgcgggcatcgcgatggcgctgcccgacggcgtgcgccgcaccatctactgcatcgcgctcccgtggatcgcgttcactgcggtggtctacctgtttgccttcgcgggtgggttcgtgcagacctggggccgcgactacaccttcacgctcaaccacttcaagaacgcctttgcgctcgaatggggccagttcggcctggtctgggccggtacggcgtggaactcgctgatcaccacgctcaagctcgcgggcatctcggcaccgatcaccgcggcgctcgggttgctcatcgcctggctgctggcgcgcaacgagttcaaggggcagggcgttttcgagtttggcgcgctgctggcttttgccattccaggcacggtgctgggcgtgagctacatcctggccttcaacgtgccgccgttcgagctcacgggcactgggctcatcatcgtgctgtgcttcatgttccggaacctgccggtgggcgtgcgggccggcacggcggctttcaagcaactcgaccgctcgctggacgaagcctcgctgatgctgcgggcctccacgtcgcagacgctcttcaacgtggtgctgccgctgctgaaacctgcgctggtggccgcgctggtctacagcttcgtgcgcgccatgacgacggtgagcgcggtgatcttcctggtcacggccgagaatgaactggccaccacctacatcatcggccgcgtgggcaacggcgattacggcattgcgctggcctactgcacggtgctcatgatcctgatgtcgctggcgattgcgctggtgcagtgggtggtcggggagcgcaagctggggcggcgcagggcgggcgtgccgatggtggctgcgcccgtggtgcattgatcgggaaaagaacacatgagcaacggcatcgaattccgcaatgtcaccaagcgctacggcaccgacaggaacgggcccttggcggtcaagggcatcagcttcgaggtaccggtcggcacgctcaccaccatcctcggcccttcgggctgcggcaagacgaccacgctgcgcatgatcgcggggctcgaatcgccgacctcgggctcgatcctgatgggcgggcgcgacgtcaccacgctgggcccggccgagcgcaacgtgagcatgatgttccagagctatgcgctgttcccgcacatgaacgtgatcgagaacgtgggttacggcctgcgcatgagcggcgtgaaaaaagacgaggccacctcgcgggcgcgcgatgcgctcaagggcgtgggactggtcggcttcgacgagcggctgccgagcgagctttccggcggccagcagcagcgcgtggcactggcgcgcgcgctggtgctggagcccgcagtgctgctgttcgacgagccgctatcgaacctcgatgcccgtctgcggcgcgaaatgcgcgaggagatccgcgcgctgcagcagcggctgaaactcacggtggcctacgtcacgcacgatcaaagcgaggccctggccgtgagcgaccagatcatcgtcatggaccacggcgtgatcgcccagcgcggcacgcccgagcaactctatggccggcccgagagtgaattcgtcgccggcttcatgggcgaggcgatggtgtttccggccgttgcgcaggccgatggcagcgtggtgctcggcccgctgcgcctgcagccgcgctatgcggtgggccccggcacggtgaaagtagcggtgcggcccgaagcctgggaaatcggcgccgccgacgcggcggggggccttgccgccacgctgcgcaaggcggcctacctcggcagcttctacgaatacggcttcgatacatcgctcgggccggtcttcgtggtgtcgaccgatctttcgcgcccccttgccgcgggcgcgcaggccacgctgtcgctggcggcgcacggcgtcagcgtggtgcccggcgcatgaaacaatggcgccatgaacgtggttttcgatcttggcgccgtgctgctggcatgggagcccacccggctggtgcaggcccatcttcccgagcacgctcccactgagcttgccgcagcggcgctgggccgggcgctttttcaccatgacgactggatgtgcttcgactgcggcacgcgttcgctcgaagacgctattgcgcgcatggcccggcgcctgtcgcttccggcggcacggctcgacgccatgctcggcaacctgggcgagcgcctggagccgattcccgtcacggtcgacctgctcgaagggctgttcgcgcggcgcgatgccggcgaggcgctgcggctctactacctctcgaacatgcctctgccttacgctcgcgccctcgagcgccggcacgggttcatgcggcgtttcgatggcggcgtcttttcaggcgacgtgaagttcatcaagccgaaccgcgaaatctacgaactgctggcggtgcgccatgcactcgatccgcagcagacggtgttcatcgacgactcggccgccaatgtggaggccgcgcgcgccttcggctggcatgccatccattgcacccaccccgccgcgctggcggcgcagctggcgcgctacgtgccggctgcttcgcctatcggccggtgagcaccaccttggcggtgtcgaatcccaggctggcggcgtagtccagttcggcctgcagcgcgtcgtcttccaggcgcggcgcacgcgaaagaacccacaggtattcgcggtcgggcgtgccgaccagcgccacctggtagtcgcggtcgagcttcaggatccagtagtcgccccacaccatcggcagccagctgagccatgacggcgcaaagcacacttcgagccggcctgccccgggctggccggcgaccggcaccacgcgggccgtgcccacggcctcgtcgaagttgccgtcggggcgcacgcagcgattgagcacctgcaccgtgccgtcgggctgggggatgtactcggcggtgaccgggccggcgcactgcttctggaagcggtttggcaagcgggcctgttcgtgccagatgccggcatagcgttggatgtcgaccggcgccaccacctgcagcggcgcgcgcatcagcggcgcgccgtcggcggggccggccagctgcgcacgtgcggtgcgccccgcgcccagggcgatccaggttgccacgccgccgacgacgaaagcggtggccagcgtgccgatggcggcgctggtgcggcggtcgtcgaaaggagcgcggtttgctgcagcggcgggcactgcggtgcgatgtcggcaaggcatggaaaggcactcctgtggtcgaaagcatcaaggcgggaagccgcaggctagcccgccgacggaatcgctctcgtcagcggcggaccacagcatttgtagggcagggcggccggcgcacgacacggccggttacaggccgatgcagcgcggtgaaaacccgtgctacggtgcgcatcaaaacatcggccccagcgcaattgcgtgcaggacttgtcatcacccgcacaggataatcttcgacatgaatcaactcgatgctctccgtcaatggaccaccgtggtcgccgacaccggtgacttcaagcaactcagcatttccaagccgcaggatgcgaccaccaatccgtcgctcatcctgaaggcagtgcagaagcccgagtaccggccgctgctcgacgatgccgtcaagaagcatgcgggcaagccgctggacgaggtcatcgatcgcctgctggtgcgcttcggcgccgaaatcctttcgatcattccgggccgcgtgtcgaccgaggtcgacgcccgcctctcgttcgacaccgccgccaccattgcgcgcggcgagcgcatcgtggcgctctacaaggccgaaggcatcgacaccggcaagcgcctgctgatcaaggtggcctcgacctgggaaggcatccaggcggcgcgcgtactcgagcagaagggcatccgcaccaacctgacgctgctgttctcgttcgcgcaggcggtggcctgcgccgacgccggcgtgcagctcatctcgcccttcgtgggccgcatctacgattggtacaaaaagtcggccggcgccaaatgggacgaggccgccagtgcgggcgcaaacgatccgggcgtcaagtcggtgcgcgaaatcttcaactactacaagcagcacggcatcaagaccgaggtgatgggcgcgagcttccgcaatgtgggacagatccaggccctggccggttgcgacctgctgaccatcagccccgaactgctggccgaactggccgcgaacaacgacccgctcgaacacgcgctcgacgctgccaaggctgccgccacggcgaatgtgcagaagctgagctacgacgaggcaagcttccgcttcgcgctgaacgaagatgccatggccaccgagaagctcgccgaaggcatccgcgcctttgcggccgacgccgtgaagctcgaaagactcatgcaggaaagcggcaaataaacatggccatgacccttcgctgcgaccgcgcgcccgcctgggcgcaactgcggagctacttcgaaactgcgggccggcagttcgacgtacgccacgccttcgtcgacgacgcggggcgcttcgagcgcttcagccaggaggcgccgtatgtctttgccgacctgtcgaagaacctgatcgacgcgcacgccgaagaactgctgctcgcgctggcaaccgagtgcgggctcgaagcgcaccgcgacgccatgtttgccggcgagcacatcaacaacaccgaagaccgcgccgtgctgcacacgctgctgcgcgcaccagccggcgccgcagtgggcagcaccgcggccgaactgcgcgaagtgcacgccacgctcgacgcgatgctggcctacgccgagacggtgcgcagcgaccacaccatcaccgacgtggtcaacatcggcatcggcggctccgacctcgggccgcagatggcggtgctcgcgctggccgagttcgcggcgccgggcaagcgctttcacttcgtctcgaacgtcgacggccacgaactggcgggcgtgctgcgcgacctggcgcccgagcacacgctgttcctgatcgcgtccaagactttcaccacggccgagaccatggccaatgcgctctcggccaggcgctggtacgagcagtcgggcggcaccgacatcgccggccacttcgcggcgctcaccaccaacgtcgaggccgcgaagcaattcggcatcgacaccaccttcgggttctgggactgggtgggcggccgttattcgctctggtcggccatcggcctgccgattgcgctggccatcggcgccgatgggttccgccggttgctggcgggcgcgcacgccatggacgagcacttccgcaccgcgccgctggcgcagaaccttccggtgcggctcggcctgctcgacgtctggtaccgcaatttccacggcttcacgagccgcggcatcgcgccgtaccacagcgccttgaagcgcctgccggcgtatatgcagcagctcgagatggagagcaacggcaagcaggtcgatgccagcggcgcgccgctgcccgccagcctgggcacctcgcccgtgctctggggcgagcccggcaccaacggccagcacgcctacttccagatgctgcaccagggcaccgacgtgattccgctcgaatttgtggcggtgcgcgatgcggcccacgacctggacggccaccaccccaagctgctggccaatgcactcgcgcaggcgcaggcgctgatggtcggcaagctcgacgccggcggccacaagaattttccgggcaaccggccgagcactttcttcgtgttcgacaagctcacgcccgaatcgctcggcgcctttctcgcgctgtacgagcaccgcgtgttcaccagcggcgcgctgtggggcatcaacagcttcgaccagtggggcgtggagctgggcaaggtgctcgcgaaagacatcgagccgcggctggcctccggcgacgtcacggggctcgacgcctcgacggcgggcctgctgaaacggctgggtagccgggcctgagtctctgaagtgcgaggcaataggccgttggtttgagaaccaatggccgaatttgcagttgaaagacccgccgatatgatcagcccggggaagtttccctgggaacaatcaagaggagtcgatcaatggactttcaaacagcggtcaagacctgtttcagcaaatacgccgatttcacggggcgtgcatcgcgttcggaatactggtggttcgtgctggctgagctcatcgttctgatcgtggcgagcctgatccaccagtacgtttacgtcattgcggcactgggcttcttggtgcccgcgctggccgtgggcgcgcgccgcctgcacgacatcggcaagagcggctggctccagctgctgatgatcattccgctcgtcaacctggtgctgatctatttcttcgtgcagccatcgcagcccgagaccaacccgcacggggtgcccgccacctgaagcggggcacagcgcccgctgcgcgcgctagggaacaatcatcaagggccgcgcaagcggccctttttcatggcttcttacatgctgtattgcgttaactagggaatatcctagccaactggtgcatgaaagtaccaccatgacccggtgcagtaccaaaaccgcaagcgtgcttctccagaattcaggccacggcgacccgacaagagggcgtcgctcacctctaggagacaacatgaagcgttttctgaaagcgggcctcgtcctcgcactcgccggcacggggctcgcctcccacgccgccaccgaactcgtgattgccaccgtcaacaacggccacatgatcgagatgcagaagctcacccccttcttcgaaaaagccaaccccgacatcaagctcaagtgggtgacgctggaagaaggcacgctgcgccagcgcgtaaccaccgacatcgccaccaagggcggccagttcgacgtgatgaccatcggcctgtacgaagcgccgatctggtcgaagaagggctggctccagcccattgccaccgacgccgcctacgacgcggacgatctgctgcccgccatccgcgccggcctgtcgtacgaaggcaagctttacgccgcgccgttctacggcgagagctcgatgctcatgtaccgcaaggacctggccgacaaggtcggcttccagatgcccgagcagcccacctgggcgcaggtgaaagagctcgccggcaagatccatgacccgaaggccggcgtgtacggcatgtgcctgcgcggcaagccgggctggggcgacaacatggccttcctgaccacgctggtcaacaccaacggcggccagtggttcgacatgcagtggaagccgcagatcgacaccaagccctggaaggacgcgatcaacttctacgtcgacctgatgaagtcctacggccctccgggtgcatcggccaacagcttcaacgagaaccttgcgctcttcaacgaaggcaagtgcggcatgtgggtggacgcgaccattgccgcctcgttcatcagcgatccgaagcagtcgaaggtggccgacaaggtcgcgttcgcacaggccccggtggccgtgacgccgaagggtgccaactggctgtggacctggaacctggccattccggcaagctcgaccaagggcgccgccgcgcagaccttcgtgaagtgggcaacttccaaggagtacgtcaacctggtggccaaggagcacggctggggcacggtgcccaccggcacgcgcaagtcgacctatgcgaaccccgagttccagaaggtcgccaagtttgccgcggccgagaagaaggccatcgacactgccaacctcagcgacagcacgctgcccaagtcgccgtacgtcggtgtgcagtacgcggccatccccgagttccaggccattggcgtggcggtgggccagcagatgagcgcggcgctgtcgggcaaggtcacggtcgaccaggcgctgaagacttcgcagacggcggccgagcgcgagatgaagaaggctgggtactacaagtagcaagccgtctttcccctctccccccggggagagggcagggtgagggggcagcgtgtccatgagcgccgccgcatgccctcaccccaaccctctccctcaagcgggagagggggcaacagcctgagaggaacacaagatgaaacgactcctgccccgggccctgatggcgcccgccgtgctcacgctcttcctgtggatgatcgtgccgcttgcgatgacgttgtacttctcgttcgtgaactacaacctcatgcaacccggcgagcgcacgttcgcgggcatcgagaactttcattacttcattaccgacccggacttctggcccgcgacctggaacacgctgctgctgatcggcagcgtgatcgtcatcacggtggtgttcggcgtgctgctcgccctcttggtgaacgagccctttccgggccgcggcatcgtgcgggtgctgctcatctcgccgttcttcgtcatgcccgcggtcaatgcgctgctgtggaagcacatgatgatgaatcccatctacggcatcctggccgacgtgtggcgcttcttcggtgcgcagcccgtcgactggctcaccgacgtgccgctgctgtccgtgatcatcatggtggcatggcagtggctgccgttcgcctgcctgatcttcatcacctcgctgcagtcgctcgaccgcgagcagatggaagccgcgcgcatggacggcgcaagcgcattccagcgctttttctacctgaccattccgcacctcggccggccgatggcggtggtgatcatgatcgagatgatctttctgctcagcgtgttcgccgagatcgccatcaccaccaatggcggcccgggcaacgagagcaccaacatgacctacctgatcttcaagcagtcgctgatgaatttcgacgttggcgtggcttcggccggtgcgctcttcgcggtggtgctggccaacatcgtggccgtgttcctgatccgcatcatcggcaagaaccttgattgaaggaacgaccatgcaacccagcaatttccttccgcaactgctgcgcaccgcgggtgcgtgggcgctcgcactgctgctgttcttcccgctcggctggctgtttctcacggccttcaagaccgagctgcaggccatccacgtgccgccgctcttcatcttcgagcccaccctgggcaacttcagcgaagtgcagcgccgcagcgactacctgctgtatgcgcgcaactcgctcatcaccagcctgggctcgaccatcatcggcctcttgatcgcggcgcccgccgcgtattcgatggccttctttcgcacgaagaagacgcgcgacatcctgatgtggatgctctccaccaagatgatgccggccgtcggcgcgctggtgccgatctacgtgctcgcacagaccgcgggccttctggattcgctcactgcgctcacggtcgtgttcacgctgtcgaacctgccgatcatggtgtggatgctctacagcgcctacaaggacattccgaacgagatcctcgaggccgcgcgcatggacggtgcgaccctgtggaccgagttccgccacgtcgtgctgccgctgtcggtcggcggcctggcatcgaccggcctgctgtgcctggtgctgagctggaacgaggccttctgggcactcaacctcagctcggccaaggccggcacgctggccacgctcattgcctcgtactccagcccggagggcctgttctgggccaagctgtcggctgcctcgctgatggccatcgcgcccatcgtcgtgttcggctggttcagccagaagcagctcgtccagggcctgaccttcggcgccgtcaagtaaagaaagggagacacctcatggcttacctgcaactcaaagacatcaagaagagcttcggcgacgtcaacatcatcaagggcgtcgacctcgaaatccagaagggcgagttcatcgtcttcgtcgggccttcgggctgcggcaagtcgacgctgctgcgcctcattgcggggctcgagccgatcaccagcggcaacctgctgctcgacggcaaggacatcacctgggcgccttcgggcaagcgcgacctggcgatggtgttccagagctacgcgctctatccgcacatgagcgtgtacgacaacatgtccttcgcgctcaagctcgcgggcgtgccgaagagcgagatcaagaccaaggtcgagtacgcggccaagacgctcaatctcacgcaatacctcgaccgcacgcccaaggatctgtcgggcgggcagcggcagcgcgtggcgatcggccgcgcgatcgtgcgcgcgcccaaggtgtttctgttcgacgagccgctgtccaacctggatgcggcgctgcgcggcaatacgcgcgtcgagatccacaagctgcatcggtcgctcggcgccaccaccatctacgtgacgcacgaccaggtcgaggccatgacgctggccgaccgcgtggtggtgctcaaggacggtctcatcgaacaggtcggcacgccgctcgaactctatgaccatccggccaaccagttcgttgcgcagttcatcggcatgccgtcgatgaacatggtggcggcgagcgcgattccgagtttctcggccgcgaccggcgggcgcctgccgaacgacggtttcctgggcgttcgacccgaaggcctgcgcgtgcatccgaagcaggccgctgctgcaggcgtgcccggccgtgtcgagctgatcgaggcgcttggcgccgacacgctgatccacgtcgacgtgggcggcgtgccgctgattgcgcgccagaacgagcgcacgccgctgcatgcgggcgatgacgtggcggtcgagctcgatccctcggtgctgcatctgttcaaccgcgaaggccgcgcggtttccgcctgatttttctatttttcttccggacatttaccgtgatccttgcagcagcgcctcttgcgcccactccaccggttctttcggagttcacggtgcttcaccttggactcggctcgttccaccgggcccaccaggccgtctaccttcagcggctgatcgatgcgggcgacacccgttggtcgctctcgggcgccaacatccggcccgacatggcggatgtcgttgcagccctgcaggcgcagggcggacgctacacgctcgaaaccgtgtcgcctgcgggcgagtaccgctacgaagagatcgaagccattcgcgaagtgctgccgtgggagcgctcgctggccgcggtgatcgcgcgcggcgcggcgccgtccacgcgcatcgtgtccttcaccgtgaccgaggcgggctactacctcgacaccaagggcaagctggacctgtctttcggcgatcttgcggccgacatcgagcgcgcgcgccgcggcgtgacatgggatgagggcggcgagggcgtgaccatctacggcgccgtctgcgcgatcctgcgcgcgcgcaaggccgcagaggccggtgccgtgacgctgctcaactgcgacaacctgcgccacaacggcgaccgctttcatgccggcttgctcgagttcatcgagcgtgccggcgatgccgaattgctcgcgtgggtgcaagcgaataccgcctgccccaacgcgatggtggaccgcatcacgccgcgcccgccgcccgaattgcgcgcgcgcgtgcaggccgccaccggacgcgacgatgcggcagcgatcacgggcgagagcttcatccagtgggtgatcgaagacaactttgcggccggccgtcccgactggggccgcgtgggcgtggaactggtcgactccgtgcagccttatgaagaggccaagatccgcatcctcaatgccacgcacagctgcattgcctgggccggcacgctggccgggctgggcttcatccacgagggcacgcaccacgcggcgatccggaagatggcccacgactacgtgaccgacgacgtgatcccgtgcctcagcccaagcccgatcgaccttgcggcctaccgcgacgtggtgctcgaccgtttcggcaaccccgcgatccgcgacaccaaccagcgcgtggcggccgacggtttctcgaagatcccgggcttcatcgcccccacggtgcgcgagcggcttgccgcggggcagccgatcgacagcgttgcgatgctgccggcgctgttccttgccttcctgcaactctggcatcgcggggcgttgccctatgcctaccaggaccagggcatggacgaggccgtggcgcacgccatctgcgatgccgccgatccggtgcttgcgctgtgttcggacgccggactgtggggccccgtcgcgggcaatgtgcggctgatcgacgccgtgcgcggtgcgagcggtcgtgtggcaaattttgtgagttcaggagcaacgatatgagtgaacgtctgaagaaccgccacgtactgctgaccggcgccggtggcggcatcggtctggccgtggccgaagcctgcattgccgagggcgcgcgctgcagcgtggtcgaccgcgtggcggcggcaccggaggcggtgcgggcgctgcagcagcaacaccccgacaagctcgcctacatcgcggccgacgtgaccgacacgcaggccatcgcgcacatgctggccgaggcgcaggtcgccttcgggcccatccacacgctgttcaacaatgccgcggtgttcgacctcgcgccgctgctcgacagcgacgaggcatccttcgacaagctctttgccgtcaacgtgaagggcatgttcttcgtgatgcagggcgtgctgcgtcacatggtcgaggccggcacgcagggcgcttcggtcatcaacatggcttcgcaggcggggcggcgcggcgaggcgctggtgtcgcactactgcgccaccaaggccgcggtcatcagctacacccagagtgccgcattggccatggcgccgcatggcattcgcgtcaacggcatcgcccccggcgtggtcgacacgccgatgtgggaccatgtcgacagtttgttcgccaaggccgaagggctgccgcccggcgagaagaagcgccgcgtgggcctggaggtgccgctcggccgcatgggcgtgccggcggacgttgcgggtgcggcggtgtttctcgccagcgatgaggcgcgctacatcacggcgcagaccttgaatgtcgatggcggcaatgtcatgagctgaactgaaggcctgcttcttcccggcacgcaatccatgaacgaagattttcatctgtacctcgacagcgccgacatcgccgaactgcagacctgcctgccgcatccggtggtgcacggcgtgacgaccaacccgacgttgctgcagcgcgcgggagtcggccgcggcgaagtgccgggcttgctgaagcgctgcatcgatctgggcgcacggcaggtgcaggcgcaggtgtattcgagcgaggtcgacggcatgctcgaagatgcccgcgccttgctgtcgcacttcgagctgggccagttggtcgtgaagattcccgccacgcgccagggcctcgatgccggcgcgcggctcattgcgcaaggcgtgccggtgacgtggacggccgtctatgcgcccgagcaggcgcactttgcggcgcagctgggcgcggcgtatgcggcgccttacctggggcggctggaagatgccggcatcgacgggctggcgctgatcgcgcagatgcagggcctggtcgctcagcggccttcgtctggcacgcgcctcctggtggcaagcattcgatcgcgcgaggcgtatctttcgttgctggggttgggcgtgggggcaatcacgattccgccgcgcctttttgccgaactgctcgatcatcccgccacgctggcggccgagcgcggcttcctggccgacgcgcgcgccttgtcctgaaagaagagaatccgagaaccatgcgcattgcactcacgggcgaagccctgatcgatttcaccgccagcgaggccggcacgctcgcgttcctgggccacgagggcggctcgccactcaacacggctgtggcctgcgcgcgcctcgggcagcccaccgggtttctcacccagctgtcgaccgacctgttcggcgaacggctgatgcgctttctcgagcgcaatggcgtggacaccagcttcatcctgcgcagcaatgcgccgtcgaccctggcctttgtcgagcgcacgccgcagaccaaccgctatgcgttctacacgcgcggcagcgccgacgcgacctgggcccccgagccgctgccgcagctgccggccgactgccgctttcttcatttcggttccatctcgctgctgcaggagccggcggccacgcgcatcgccgaactcgtcacggccaacgcggggcggcgcgtgatcgtgttcgaccccaacgtgcggccgagcctgattcccgacatggcggagtaccgcgtgcgcgtcatggactggtttgcaatggccgacctcgtcaagctcagcgacgaggatgccgaactgctggcaccgggccagccggccgatgcactggcggcgcagtgcctgcgagccggcgcgcatgcggtgatcgtcacgcgcggcggcgcgggtgccacgctctggcgcacgggacacgagccgctcaccgtggcggcgccgcgcgtcgaggtggtcgacaccatcggcgcgggcgacaccttcacggcgggcctttcggtcgcgctgctggcacatggcgtcgagcacccggcccaactcggccagctggcggacgaagcctggcgccaggtgatgcgcttcgccgcgacggcggccgccctgaactgcacccgcgaaggggccgatccacccacgctagcagcggttcacgccgcgctggcgcaggaagacaatggagccgtcgcttcccggtcctgactccgtgctgccatgaccacgtccacacgcaaacgctcgattccacgtcagcgccaacccgagctggaacgcgacattgcgcgctccccgtcgctgggctacgaagcccccgaaaccggcctggtgcgctgccttgcgcacggctttcccagcccgctggtgcgatggcactttcatgaagactacgaactgcacctgatcaccgagacctcgggcaaggccttcatcggcgactggatcgggccgttccagcccgggcacctggtgctgtgcgggccgcggcttccgcacaactggatctctctcgatgtacccgaaggcggcgccgcggggcgcgaccgggtgatccagttccgccacgagcccatcgaacgtgcggcggaggagattcccgaactgcgcgaggtgatgcagctgttcgaacgggcgcggcacggtatcgagttcttcggcatgtcgcagcaggcgcaaatgcactgggacagcatcaaggccgcgcgcggcatgcgccggctcggcctgttcctcgagttcatggccgatctggcgcaatgcaccgactaccggctgctgtcgagcgtgcagatgcaaggggcacacggcgccgatggcgatgcgcaggtcgaccagatcaacggcatcgtcaaccgcatcaccgccaacctggcagagcccatctcgatgtccgacgtggcggccgagctcggcatgagcgagagccgcttcagccgcttcttccggcgctccacgggcaacagctttaccgacttcgtcaaccgcgtgcgcatcaacagcgcctgccatctgctgatgcagaccgaccactacgtgaccgacatctgctaccaggtcggcttcaacaacgtcgccaacttcaaccgccgctttctcgaaatcaagggcatgaccccgagtgaattcaggcgccaggccgacacccgcttcggctgaggtcgggacgccccgctttcaagacgcaatcagggagcaccatcttgtatctgggactcgacctcggcacgtccgagctcaaggcgctgctgctcacaggcgatcaccgcatcgttggcttggcacgcgcaccgctcacggtcgatcggccgcaaccgctctggtcggagcaggcaccgggccagtggtggcaggcgctggagcaggtcatggccgagctgcgggaggtgcactccggggcgctgtcggccgtgcgcgccatcggcctctcgggccagatgcacggcgccacgctgctcgatgcggcgggcgaggtgctgcggcccgccatcctctggaacgacgggcgcagcggcgcgcagtgcgaggcgctcacgcgcgctgtgccgcgcctgggcgagatcgcgggcaacctggcgatgcccggattcaccgcacccaagctgttgtgggtgcgcgagcacgagcctgaaatcttcaatcgcgcggcgcgcgtgctgctgccaaaagactggttgcgcttcatgctcagcggcgaggccgtcagcgagatgtccgacgccgccggcacgctgtggctcgacgtcggcgcgcgcgactggtccgacgagctgcttgcggccacggggctcacgcgcgaccacatgccgcggctggtcgagggcagtgaagtgtcggcgcagctcaagcccgaacttgcggcgcgctggggcgtcggcagcggcgctgctgtgctcattgccggtggcgcgggcgacaacgccgcgagcgccgtcggcatgggtctggtggagccggggcagggcttcgtctcgctcggcacctcgggcgtggtgttcgtctcgaccgaccgctttctgccgaacccggcgcaggccatgcatgccttctgccacgcgctgccgaagcgctggcaccagatgtcggtgatgctctcggccgcaagcgcggtgagctgggccgccagcacattcaagtttgccgacgaggccgcgctgctcgaagcggccgcgtcggtcgagccggcacggcgcgagcggtgcccgttgttcctgccgtacctgtcgggcgaacgctcgccgcacaacaaccccgatgcgcagggcgtgctgttcggattgacgcatgcacatggagcggcggaaatcgcctacgccgtggtcgaaggcgtgagcttcgggctgcgcgacgggttcgacaccctgcgcctgcctgccgacatgccgctgcgcgaagttgcgctggtcggtggcggcgcacgcagcgtgtggtggggccagttgctggccgacatcttccaggtgccgctcacgctgtatgcgggcagcgaaacgggcggcgcgctcggcgcggcgcgccttgcctggctggccgacggcggcaccgtggccgaggtgtgcacgctgccgccagtgaggcagcagctcgcgccgtcggcggtcgatgtggatttgcacagcacgcggcatgcgcgattccgggagctttatatggcgctgcgcgaccagttccgataacggatacaacgctccgagcgcccataaaaaaagcccgtcgcaagacgggcttttttatttcgcggaacaccgcggaaccgggtttgccgggccgcaggtgttgcccccggtagggggtgggcgtagcggacacgaagtgccgcgcagcctgggggcgagcgaaatttacatccccatgccgcccatgccgcccatgccacccatgtcgggcatgccgccgccggcaccggcttcgtccttcggtgcgtcggcgaccatggcttcggtcgtcagcagcagcgaagagaccgatgctgcgttctgcagcgcggtgcgggtgaccttcgtcgggtccaggatgcccagctcgagcatgtcgccgtacgtgtcgttggcagcgttgaagccgtagttgcccttgcctgcgagcacagcgttcacgaccaccgaggcttcgccgccggcgttgttcacgatttcgcgcaggggggcttcgatggccttgagcaccagcttgatgccggcgtcctggtcggcgttgtcgcccttgatcgagtcgcccacggcttgcttggcacgcagcagagccacgccgccgccagccacaacgccttcttccactgcagcgcgggtggcgtgcagggcgtcttcgacgcgagccttcttttccttcatttcgacttcggtggcagcgccaaccttgatcactgcaacgccgccggccagcttggccacgcgctcttgcagcttttcacggtcgtagtcgctcgtggcttcttcgatctgcacgcgcacttgcttcacgcgggcttcgatgtcggccgcagcgcccgaaccgtcgatgatgatggtgttttccttgcccacttcgatgcgcttggcttggccgaggtcggccagcgtcaccttttcgagcgtcaggcccacttcttcagcgatgaccttgccgcccgtcaggatggcgatgtcttcgagcatggccttgcggcggtcgccgaagccaggagccttcacagccacaaccttcaggatgccgcggatcgtgttcacgaccaaggtagccagggcttcgccttcgacttcttcggcaatgatcagcaggggacgaccagccttggcgacttgttccagggtggggagcaggtcgcggatgttgctgatcttcttgtcgaacagcagcacgaaggggttgtcgagcagcgccgattgcttctcggggttgttgatgaagtagggcgacaggtagccgcggtcgaactgcatgccttcgacgacgtcgagttcgctgtcgagcgacttgccgtcttccacggtgatcacgccttccttgccgaccttgtccatcgcgtcagcgatgagcttgccgatggtttcgtcgctgttggccgaaatggagccgacttgcgcgatttccttcgacgtggtggtgggcttcgaagccttcttcagctcggcgacgagggccgtgacagccttgtcgatgccgcgcttcaggtccatcgggttcatgccggcagccaccagcttgaaaccttcgcgaacgatggcttgtgccagcacggtcgcggtggtggtgccgtcaccggcgttgtccgaagtcttggaggccacttccttcacgagctgggcgcccatgttctggagcttgtccttgagttcgatttccttggcgaccgacacaccgtccttggtgacggtgggggcgccgaacgagcgctcgagcaccacgttgcggcccttggggcccagggtcaccttgactgcgttggccaggatgttgacaccctcgaccatgcgtgcgcgggcttctccgccgaagacgacgtcttttgctgccatgttgatttactccgaatgggatggattgattacttctcgacgaccgcgaacaggtcgtcttccttcatgacgagcaattcgtcaccgtcgaccttgacggtctggccgctgtacttgccgaacaggacgcgatcgccgaccttgacggtcagtgcggtcaggtcgcccttgtcggtgcgcttgcccgggcccacggccaggacttcaccctgatcgggcttttcggcggctgcgtcggggatgacgatgccggaggcagtcttggtttcgctgtcaatacgcttgacgatcacgcgatcggccaaaggacgaagtttcattgcatctcctggataagaaacggggttgtggtcgggcgccggacccgaggccggcgacccatcgactggaagcgaggcttgttagcactcatcagcagcgagtgctaatgataagggcaatcggcggactttcaaggccgggggtgggtgggtgctgtcggttctctgctgctgactccgaactcttctcatccgactcggactgcacgaccgtgctatttaagggctttctcaggaggcgaacagcctcatgtccgttgcttgtgcttcagcgaaaagctttcggtcgccacacgagaaaggccagcacacccgccgccatccgcccgaacgacggcaggccctgcatgaggaaggcgccagtgtcgcgcgcgacgcgccagccggaaaagcctgagttcaggtcgcagcggcacagcgaccaccagcagcgcagcacgtcgagcgagaggaaggtcgcagccaagccgagtgcgagcacggtgcgcgcgcgtccaatcccatggtgcgccgccacgtcggccgcgacgtggccgtgcgcgatttcctcgcgcgcgtgccagcgccacatgcgagagtgagcggagtcatcgtctggcagcaggtcgggatgcgccaggatctcgcgtgagagcacgatcgtcagatgctcgaaggccacaaccagcgccaatcgcatcgtcaagctgcactttgcaatctcgtcggtgacgcgcatcgcgcgctcggctgcgggcgccgcaccgggcgtggctttgatcagtgcagcgttgtagcgatcatgcgcgcgttgatgcgcacgttcttcccggatcagccggctgacctcggcatgcaacgcggtgctggcggagctgccagcgacgcgctgccattcctcgatcgtcgcgatgacgaaggattcgccggtgggcaagatcagcgaaagcgcatcgaacaggcgactgcggggaatcgtgcggttccagatgacggcctcgccggaggtgggcgcggtcatgagtcggcctttgcgacgctggggggcaaccacagacgtggtccttcgcgcagccagcgccgcgcgaaatctgcataggcgaccggcacggcggatgcgtcttcacgaaggcggtccggggcggcgatccacaccgcgttcggctggcgatgatgcacgcggtgcagcgaccgatgcagcatgatccatcccagtccgaacgggagtgtgacgtcatgagccagttcgctcgcgacgcgccgcgtgccggccggcgccactgcggtgccgtagtgctcggcctgcgtcagcggaaagtcgatccaccccgatatgcacagcgggatcgcataggcccagaagaaggcgtgcggcgcgagccagcaggccagcgcgaccgcgctggcgcacagcagccacgagaccgtcgacaggcgacgcgccgctcgacggtctagtggcacaaggccgccgcccacgcggttgatatggaacgcaacccagaatacctccagcggagccagtgcccagatccagcgcgtgcgccaactcagcgcgtacaagctcccttccggatcgtcgtcgttgcaggtcgcgaggtggtgcttgaaatgaaagtagcggaatgcggtgaagttctcaccgatcaaggacgcacaggcattgccggccaagtcattcaggacccggtggctcaggaagcttcgatgcgccgcaaggtgcttgacctcctggcaaccgaggaaaagcaaggcctgaacgatggccagtggcacgtcgatccacaccgagcggaccgtcgccagcaaggtggtgttgacgacgacggcgagcaggaacagcccgccggccaggtcgcaggtgagtcgcaggcccatcgccgggccagttgttgtcgcgcggcccgtactcacagcatcgtcaccaggtggcgggtgacgcgctgcgtagacgtcagcggcatcatcttccagacgggcttgagcagcgacagcggcacggtgccgcgcaggatcacgccgtggtcgagcgagcgtgcgtgagggaagtaatcgggtttcgcgcagacgatgtccttgaagccgcggccatggtagtagcgcagttgcggatcgaccggtacgccggcgcgttgcagcgcgacgtagtcttgcaccgatccatcgcgatgggaccggagccagccttcgaagccggggatcggtgagccgaggtagatgtggcgccagccgctcttgagcgcgtggggccagaagaactcgagcagcgcttcgacgccgctcggatggctgctgctgaggctgatgccgaacagcgaatggccgcgcgcgggccggggcgagtcgacgcagtcaacccacgacgcggcatgacaccagaaatccgcgtggacaggacgcatgaagagcgatgcgagcagcgtgtccgtgttcttgcagaacgcgcctaccgaaaggctcggatagtcctcgaggcgctgcatgagatcgtctggcgatgctgcctggacggtgtcccacttttcgcgttcgagcgtgagcagggccggcaggtcgcggcgggtcaggaaccgggcatgtgtgagaagagggaacggcgagtgcgacagggagacggaagaggacgttgacaacactgggcgtgagagcaggttccggatcgggatgccgattacgcttgtgtcaggttacgtcgcggtgaccgccttgtgacaacgaatcgacagtcacaactggtccgtcggcacgaaccaggagaacagcagcagttgcagccgcgtgagcaggctggagtcgggttcgctgtccagcacctcgttgtccacgtcgccggtgccaatccattgcacgttctcgccgtcgggcatgagcaccacgcggtagacgccctcgatgtcgtccagctggtaggcatacagcagcgcctgggccagttcgaagctgcgcacgcgaaccccgaattcggtgttcaaccgggccgagcgggggtcgaggttcatggagccaagcagcacccattcgcggtcgaccagcgccagcttggcatgcagccggccgcgcgctttcttgagcagggtgcggaactggcggttgcgcttgagctgctgggtactgacctcgtagaggttcacgcccagcttgagcatgtcgacgcggtagcggttgtagttgatgttcaccagcggttcgtcgctgtcggccagcgaattggtgatgacgctgatgcgcacgccgcgtgcgcggccttcccggatgcgcgccatgccgtcctcgcctggaatgaaatagggcgagatcaccaccacgtccgagcgcgcgctcgccgtcatttcatggaaccgcgccgcaagtgattcggccggcgacgcaagagtgccaagcgccttgttggggctgtcggctgcggcatgcgcgtcggcgcgcatccacttcacccggtcaatgtcggccagttgcgtgccgagcgtcgcgtcgcccagcaggtcggtgccggaaagaggggtgggcaggggtgcatggaccggtgaggtggcggcttcgaactgggacttcagcgtctccggggtgtcgctggcgccggcaatccgctgaagcggatagaccacgtcgctgttccagtaggtgtcgaagatgcgcgccgcttccggcaccacgggccccgccatgagcagttcgaaatcgatgaagttggcgccctcgctgcgcaagaaatactcgtcggccaggttgcggccaccggcaatcgccatggcaccgtcggccacgaagagcttgttgtgcatgcgatggttgaggcggcggaaatcgccgaaaaactccagccaccgcgtggccgagtggtcgcgggcgttcacgaaagggttgaacagccggacttcggcattgggttccgcggcaaggccgagcagcaggcggtccatgccggcggtatagaagtcgtcgagcagcaggcgcacccgcacgccgcgccgcgcggcatcgcgcagttcgcgcagcagcagccggccggtcttgtcgttgccgagctggtaggtctgaacgtcgagcgaggtttgtgtccgccgcatcagctcgatgcgggcatcgagcgcaaaagatgcctcgaccagtggccggatgctggacaacccgtcgctcgcggcgtcaaggcgggccgccgcgcggccaagcgtggtggcgggcgaggccgcaatcgagagcgtcggcggctcggctgcgcgcggaggaaggccggcacaacctgcgagagccagcgcaagtccaggaaccatcagccgaagcgccaggccgcgcaacgcgaaaaacgaagaagcaatgaactggagcatggggcctgccgacgcacaaaacgtgcggccggatcgtagccgctttgcgctgtatctccggcgcccgccaaggttcgaatgtggaggactggctaacacccgccacccggcgactgtcagcgagccaggtccgcgatgaaagctgcgtcctgcgccccgctgtagatgcgcaggtcctgcatgcggcccttgaagaatcgatcgcccccgtactgcgatcggcccagccaggttcgcgtggtgtggccgagctggtaaggcgtgatccagatctcgttgttgctcgcgaccggcgagccgtccacgtagagcgtgcccaccgttgcggacagcgtgacggccacgtgcacccaacggccggtgggcagtgggtccgcggacaagggttgttcgggccagaactgctcgcgcgaggccatgaactggagccggttctctccactgcggggggaaagcgcgatgtatgcgacgtcgtcggagccgaaatcgaagatgcgtgtgttgatggctgtggtttccgaatagacccacaccgcgaccgtgaaatcgcccagcgctgacaccgccccgtcggggaggaccacgtgaccgctgtcgccatcgagcagcacggaacctcctcccgcacgcccttcgcccaggcttgcgctgcccgtcagcttgccgtgccgaccgtggccgctgacatcgctggcgttgccgttcagcggcatgtgcagccacagttcgccggggacggccacgcgagccgtctcggcgccaacgcgctcgtcgaggttggcggtcacggcggtgatcctgtagtaccaggtgccctgggcgggggcgtcggtgtaggtgcgggggtcgttcacttgagcgatggtcgtgaacggcccattggacgaactcgctcgttgaacgaggtagtgggtggcgtcggcactgccccaccacgacagcagaaccttgctgccgctgaggaatgcgctcaggccgctgggctttgcgggcggggccggatcgcgcgaatagagcagcgtgcccaggccggggctgtcgcctgtcccgtcgaagcgctcggggcgcactttctcgaccgtcgccttggtccacggcgccgacaagcccttgcggttcacgtagtggttgtagatcagttcgaagcagggccggaagtgcccggtcccggccgtcgcggtgcctgtgccgtggacaccggtgtacggggtgaacggcatcgtgtacgggttgccgttggggtcgctgaggttcgtcttggcgacgtattcggcgccggccagcaggcggttgttccagtacccgtagaggtcttcgccctggttccacgccatctcgcacaacgcgccggccagcgcgatgcccagggtcgagtggccttggtcgcggtggctttcctgccattggcccaaatgaccggggtgcacgaaatagacgttgtgggcgctcgcgccgttgccccgccccgacttgtagtagctgaccgcttcggcggtcaggtcgggccggtcgcagaacaccccgatggcgtagaccgagcagatattgcacagatcccagttggcccagtagtgggtgacctttctgacctcgctgttattgtgattgaccagaaagtcgtggcacaacggatagaacacgttcagcagcatggcctggaagcgtgcaacgtcctcgttcgcccagccgggataggtgcgcatcagttcggcggcattggcccattggtagccgtagaggcccgaggcgaggaagacgttggagttgccgcccagcttggtcaacgtcgacgaccaggcattgagaaactccaccgacttcttggcgtagtcttcgtcgcccgagatcttccagcgcagcgcgagttgatgggcgcgttgcatgtcggagaacatcaggccgaagttctggccgtcgacgccgcggatcacggtttcctgggggcgcggcgccgtggagaggtgcgagcggccgctgccgagcagtgcgccccagccggcgacccatggctgttggctggcggcaagcttgtcccgaatgcgggtcaggtcggcctctgtgctcagcaggccggggtgggtgagcttgcccacttgcgtcacaggggccatcgggtcaggcgcggcggcatcggtggtatcgatggcatcgacagtgtcggtggcaccgggagcagcacccggcatctggtcttgcggctgctgctgcgcgaggggccctcccgccgtcgaaaactccccacctccgccgccgcaacccgtgacccccagagccagtgcgcccgcggtgctgagaaagaaaacacggcggtccagcaacaagccattcttgtcgtcactcggcaaatgtgtcatttatatgaaatatgtaaaaagttgattctgcaaggtacgtgccatttgcttgtgccgctacacagagcgagatcggtagcacggatggatgcattgcatgcgctgtaacgcgcttgaggtgacgtttgttgtcacatggtggtcagcactgccagaaatgtcagcggcaagtgcggtcatgaaccagcttccggagagcttcgtcgatgtgcccgtgcttcacccgcgcccgtcaaggccgaacgcccctcgccgatccagggaaattgaaacaaatgagactttataactattagaatgcgaatcgttcttaataatgtttcggagtggagaaggaatgacgggattcgtggcggggcgcagggtcgcgacagtgctggcaggttgcttggcaatccatgtgcatcaccaggttctggcccagaccacggcgcccggcgccttgcccgaagtgaaggtcgatgcgaatgccgaggccgaaaccgcgacgtcgccggtgatcggataccgtgcccggaacgccgcgaccgcgaccaagacggacacgccgctggctgaaaccccccaatcggtcaccgtggtcacgcgcgaccagatggtcgaccagggcgcctacaacctgcaggacgcgctcaattacgccgccggcgtgcgctccgatgcctatggcctcgattcgcggaccgactccgtgcgcgtgcgcggcgccacgcccgacgtctacctcgacggactgcgccaggcttacggctactacaccagcaccacgcgcaccgagccctacacgctggagcggctcgaagtgctgcgcgggccctcgggcatgctgttcggcgcgggcacggccgcgggcgtggtcaacatggtgagcaagcggccgctgcaggagacgcagcgcgaagtgggcgtgcagttcggcagcttcggccgcaagcagatccaggccgacctgaccggtccgctgaacgccgacggcaccctgtcgtaccggctgatcgccttgcaacgcaagtcggacacccaggtcgaccacgtgcccgacgaccgcagcgtcatcgcaccgtcgctgacgtggcggccgaatgcagccacttcgctcaccttgcagggtttgtggcagaaggacaagagcggcagcagctcgcagttcctgccgtgggagggcacgttgctgccgaacccgaacgggcgcgtgcccaccagccgcttcatcggcgagccgggtttcgactactacgacagcgagcgcaagaccttcggctggcagttcgagcacaagttcaacgacagctggaccctgcggcagaacttccgctatgcgcagaacgagaacgacaaccgctaccactatggcgccgcgttcagcggggccgaaagctgggatgccaccgatccgatcttcaagcgcgtgctcggccgctactacgacagctacctgacgcgcaaccgcacgcagacgctcgataaccacgtcgaagggcatttccagaccggcgcgctcaagcacacgctgctcgtgggggcagactttgcgcgccagcgcgagaacgtctggggcggaacgaccttcgacaccatcgacgtgtacgcccctgtctatggccacgtcgacgtgcccgagcgcaccgcattgccgcgcacccgccagcgccagaacggcttctacctgcaggaccagatcaagctggacaactggatcttcgtggcgggcttgcgccacgacaaggcggtgtcgagcgcggcgggcagcgaggccgaggaaagcagcgcaacgaccaagcgcttcggcctgatgtacgcatcgccctcgggctggtcgccatacctgagctacagcgaatcgttcacgccgcagtcgccgcgcaacggacagatattcacgcctttgcgcggcgagcagtgggaagccggcgtgaagtacgagccgaaggaccgcgcactcgcgttcagcgcggcggtctacgacctgcgcgagaagaaccagatcacctcgccgtcgccgaacgtgtacacgcaagtcggcaagaccaagacccagggccttgaactcgaagccaagggctcgatcggctcgaatctcgatctggtcgcgcactacaactacacggacgcggatgaacagatcgaaggcctgcccaagcaccaggcaagcgtctgggccaagtaccgtttctcgatcggcggcctcagcggcttctcggccggtgcgggcgtgcgcctgatgagttcgttccaagacctgcagttcggtgtcggcccgcgcgtgccgggcgttgcactggccgacctcgtgtttgcctacgaaaccgatcgctggcgctatgcgctcaacatcaacaacgtgacggacaaggtgtatttcagcacctgtctctcgcgcggtgactgctggtacggcgcgcgccgcaacatcgtggccagcgcaacctatcgcttttaattttcaactttcgacgagggcagcaacgacatgaacagccgaaagatcaagacctgggcctgggtgcacaagtggagcagcctcgtgtgcaccgtgttcatgctgctgctgtgcatcacgggcttgccgctgatctttcatcacgagatcgggcatctgctgggcaccgaggtcgaggcgcccaagatgcccgcgaacacgccgcgcgtgagcctggaccgcgtgctcgaaaccgcgcgctccaagcatcccgaccgcgtggtgcagttcgtctcccagcccgaggacgacgacggcctctggctcgtcacgctcacacccacgcctgagcccaccgaagacttcaagacggtggccgtcgacgcgcgcacgggtgtcgtccttgcgcagccgaagttcgatgagggcttcatgtatgtgatgttcaagctgcacatcgacctgttcgcggggctcgcgggcaagctctttctgggcttcatgggcttgctgcttctcgtggccatcgtctccggcgtggtgctttatgcgccgttcatgcgcaagctcgacttcggcaccgtgcggcgcgagaagcgcccgcgcctcaagtggctcgatctgcacaacctgctgggcatcgtcacgctggtgtggctgttcgtggtgggctccaccggcatgatcaacacctgggccgacctgatcatcaaatactggcagtacgaccagctcagcacgctgctggccccctacaagaacgaaccgaccgtgcccgtggcccagcgcgcatcggtgcagcgttcgatggacgtcgccctccagcaggcgcccgacatgaagctgtccttcatcgcgttcccgggcacttcgttctcgagcccgcaccacgtcaccttcttcatgcgcggcaacgagcccttcacttcgaagctgctgcaaccggtgctggtcgatgccaagaccgcgcaggtgaccgcttcgccgaagatgccctggtacctcacggggctgctcgtgtcgcagccgctgcacttcggcgactacggcggcatgccgatgcagatcatctgggcgctgctcgacattgcgaccatcatcgtgctgggcagcgggctctacctgtggctcaagcgcggcaacaccgtgacgtcgccggccgctgcgggcagtgcgggcagtgcgggcagtgcggggcgcgcgccgcagcatggcggccagcagcccgacccggcccctgccatgaaggcgcaggcatgaagcaccggcacgcgttccggcgcatgtggggcgggccgatcgcgctgggcgtgctgaccgccgtcggcctggtttccgcgctgttcagcgatggcgggatgggcgacgtgctggcctggttcgcgctgggcctgccggtcgtcgtgtgcgcctggtacggctggcgcaggaactgagctgcgcccggaagcgcaaatgccggcgcgaggccggcatttgcgttgaagaggggctgaaagccccaggctttacaggccagccgcggcgcgcagcgcggctgcttgcgtggtcgcttcccaggtgaactcgggctcctcgcggccgaagtggccgtaggccgcagtcttctggtagatggggcgcagcaggtcgagcatctggatgatgcccttcggacgcaggtcgaagaactcgcgcacgagttccgcgatcttgctgtcggggatcacgccggtgccttcggtgtagaccgtgatgttcatcggctgggccacgccgatcgcgtaggccacctggatctggcactggcgcgccaggccggccgccacgatgttcttggccacgtaacgcgcggcgtaggcggccgagcggtcgaccttcgacgggtccttgcccgagaacgcgccgccgccgtgcgggcaggcgccgccgtaggtgtcgacgatgatcttgcggcccgtgaggccgcaatcgccctgcggaccgccgatgacgaagcggccggtcgggttgatcaggtagcgcgtgtccttgagccattccttcggcagcaccggcttgatgatctcttcgatgatggcttcgttgaacgaggccttcatcttggtcggcgtttcgctctggtcggggctgtgctgggtggagagcaccacggtgtcgatgctgtgcggcttgccgtccacgtagcgcatcgtcacctggctcttggcgtccggccgcaggaagggcaggcggccgtccttgcgcagctgggcctggcgctcgacgagtcggtgcgcgtagtagatgggcgcgggcatcagctcgggcgtttcgtcgcaggcgtagccgaacatcaggccctggtcgccggcgccggtgttcaggtggtcgtcggacgcatggtccacgccttgggcgatgtcgttggactgcttgtcgtagcagaccatcaccgcgcagcccttgtagtcgatgccgtactcggtgttgtcgtagccgatgcgcttgatggtgtcgcgcgccacctggatgtagtcgacgtgcgcattggtggtgatctcgccggcgagcaccacgaggccggtgttggtcagcgtctcggcggccacgcggctgcgcgggtcctgctcgaagatcgcgtccaggatggcgtccgagatctggtcggcgaccttgtcggggtggccttcggaaacggattcggaagtgaagaggaagtcgttcgccattttgttcaaagctccttgaagtgatttggcgcgttgccaactctgcggagccctggcgaacgctttagcagatgccgatgaatcggcggggcacaatcgctcttgcgcttgtgtttgtcgccctgcaagttgttccgtaactcggcgacaatttgcattctattcgagccgcgccaaacccgtgcgcgcgcgtcctggtattcacactccctgtcagcccatggtcaccttgttccgcctgcttgcccgcgtaccgatgccgttgatgcatcggctcggcgcgttgctggggtggatcgtctggtggtgcgcaccggactaccgccgccgcttcaaggccaatgccgagagcgcgggcgtcacccccgagcagtaccgccccgccatcgcagcggctggccagatggccgccgaactgccctggctctggctgcgcccgcaaggcgaaagcgtgctgcgccgtgtggtgcgatgggaaggcgtggaggccttcgaggccgccatgcaggcaaagaggggcgtgatcctggtggcgccgcacctgggcagctgggagatgtgcggccaggccatcggcgagcgctttctcgaaacctacggcccgatcacggcgctgttccgtcccgcccgcaagaaatggatggccgagctgatcgccgcaggctcgcgcgaccggcccggcctgcaaaccctgccgaccaacaacaccggcgtgcgcggcctcatccgcacgttgcggggcggcggctacaccggcatcctgcccgaccaggtgccgccgctggggcagggcgtgtgggctccatttctcggccgaccggcctacaccatgacgctgctgccgcgcctcgctcagcagaccggcgccgcctgtttcctgagcgtgtgcgaaaggctgccgcacggtgcgggctacgtgattcgattcgagcccatcgtgggcacgccgctcaccgatccggccgcgcccatcgaagccgcggctgccgccatgaacgacgccatcgggcgcctgatccgcagcctgccgggacagtacgtgtgggactacgcgcgctacaaggagccgcgcggcgaaaccgcggcggccgccccgagcggggagcaggcacgatgagtttcggttcccgcctgggcatcggctttatgcgcacgatcgccccgttgcccctgccattgatccgcggattcggcgcggtgctgggccgggtgctccacaccattgccgtgccgcgccgccgcgtggtcgacaccaatctcgcggtgtgctttccccacaaatccgaagacgaacgccggcgcatcgcgcgcgagacttttgtctatgtggcgcagtcgtggctcgaccgcagctggctctggcatgcgcctgaaaaggtggtggccagccggctcaaggtggtgggcgcggcgcaggagatcgacgaaatcgccaacggcgacgagccgatgatcctgttcgcgccgcatttctacggcctcgatgccgcggccacggcgttgaccatgcacaccccgcggccctcggccaccatctacacgacccagcgcgacccgatggtcgacgagtggattcgtgaaggccgcacgcgcttcggcaacgtggcggcgctcaatcgggtcgatggcatcaagccggtgctcggaggcctgcgcaagggtggcctgctgtacctgctgccggacatggacttcggccgcgaccagaccatcttcgtgccgttctatggcgtgcaggccgcgaccgtgccctcgctgtcgcgctttgcgcggctgggcaaggccaaggtggtgcctgtggtttccaggctcacccccgagggttacgagatccaagtgctgccggcctggcagaactttccgacggacgacgtcgaggccgacacgacgctgatgaaccagcgtttgcagggctacatcgacaccatgccctcgcagtactactgggtgcaccgccgcttcaagacgcgtcccgaaggcgagccgcccatctactgagcggccggggagggcgcctcagctccgttgcaggaagccttcgatttcgcgcgcgacgagctgcggctgctcgtgcacgatccagtgggtggcgttgggcaccttcttgacttcgagccggggtacgtactcttccaggccgtcgagcaggccgggcagcagcgcggcatcgtcgagcgcccagaagacgaaggtgggaacgttcacgctgagccgttcgtgcggcagcaccggaatgccctcgatgtcctggcccggcaacggcggcttcatcggcgtgacgcgatagagattgcaggcgcccgtgaggcccgcactccagacttcgcggtactgctgcttcacgtcttctgtgagccagccgaaaccttcgggcccggccttcatcaaggtgaagaagggccacatgcgcttgaagtcgtcggccgcgagcagggcctcggcatcgggcctcgcgagaaagttcatgtaggcgctggcttgctgctgcgccgggttgttgcgcagctcgcgcgtaaaggtgccggggtgcggcgaattgatgatgaccagccggccgacctgctcgggaaaggcgttggcatagccccaggcgaaagcgccgccccagtcgtgcgccaccagtgcggccatggtgccatcggcactttcggtggccaccagttgctggatgtcctggatcagcaggtaggccttgtacgcggccacgtcggtcggcgcgctcgatttctcgaaaccgcgcaaattgggcgcgacgcagcggtagccgccgtgctcggggtcggcaaagtattcgagcagctcgtcccagatgaaagcggcctcggggaagccatgcagaaacaccatcagcggccggccggccgtgccggtggcgcggcagctcagtgtggttccgttgggcaggctgcgctggaacgtctcgatcatgcttttgtctccttcgactttcgtcgctattgttttgatagtggatcacgctgatgaaacgccggcgagccggcttttccctaggtgtcttccggagccgccggttccgccgcttctgtttctgcctttgtgtctccgggtggatgcgcccagcgccagagcaactcggcggcttcccccacaccctgtttcttgagggcggaaaacagtttgacctcgccgccgccggcttgcagtcgcgtaatggacagcgccttggcgccatcgctgcgggtgagcttgtcggccttggtcagcagcacgaggaacttgagcccctgctgcacgcgcgggcggatcacgtcgagcaggatctcgtcgagctcggtgaggccgtggcgggggtcgcacatcagcaccacgccgcggaggttttcgcgcgtcatcaaatagttgcccatgacccgctgccagcgcagcttggcttccttgggaaccgcggcatagccgtagccgggcaggtcggccagcacggcgtcgtcggccttctgcttgccgacgccgaacaggttgatgtgctgggtgcggccgggcgtcttggaggcgaaggccaggcgcgtctgctgggtgagcgtgttgatcgcggtcgacttgcccgcgttggagcggccgacgaaggcgatctcgggcagatcgagcggaggcaaatgctccagttgcggggcactggtcaggaagtgggcggtgtgcatccagccgagcgcaatgcgctcgcgctcggcgacaagagggtccacggcaggggtcgcgcgggaagggggagcggcgtgcttgcgcgacggggaggtcatcaatgagctttcggaacgggctgccattgtagaatcgcggggttttgcgccaataaatcgagcccccgatatgaagttgtttgccaattttctgcttgcagccctcatgggtgtcgcagccagcgcgagccttgcggctgacgatcatgccgccgcaccggctgctgcacccgcggcggccaagccggccaagcccgatcccgccaagggcgacgcggtgttcaactcggccgcccaggcctgtgcctcctgccacaacgcagacggcaactcggccattgcggcaaaccccaagctggcgcagcagcaccccgaatacatcctcaagcagctgcaggaattcaagtccggcaagcgcaagagcccgatcatgcagcccctggccgccaagctgtccgacgaggacatgcgcaacatcgcctggttcgtgggttccaagaaggtcaagtccggcttctccaaggagaaggatctggtggtgctgggcgaaaagatctaccgcggcggcattgccgatcgccagatcccggcctgcgccggctgccacagccccaacggtgccggcatgcccgcgcaatacccgcgcctgggcggccagcacgccgagtacacggtggcacagcttgttgccttccgggacaacgtgcgccagaacagcgctcccatgacgggcgtagccgcaaagctcaacgaccgcgaaatcaaggccgtcgcagactacatcgccggcctgcgctgacgccacgcccttcagcgtgaactaaccgccgataaaaaccccaaacaaagggcgggccgatccagctggatggcccgccctttgctttttcccctattcccttctttccgcccgccgatgtctgtctccacccatggccttcgcgttcatcgcggcccgcaagcgcttcgcgccgcggtggagctgttttcgtcgatgcggttcgcgattgcgctgctcaccatcatctgcatcgcatccatcatcggcaccgtgctcaagcagcacgagtcgatcaacaactacatcaaccagttcggcccgttctgggccgagctgttccgcgcggccaagctcgattcggtctacagcgcctggtggttcctgctgatcctgctgttcctggtgatcagcacgtcgctctgcattgcgcgcaacacgccgcgcatcttcgtggacctgaagaccttcaaggaagggattcgcgcgcagagcctcaaggcctttggccagcgcgccgaaacccgtctggacgaggcgcccgccgcggcggccaaccgcattggccagctgctggtaagcggcggctggaaggtcaagctccagcagcgcgaagccgcggacggccaggccgacgccggctggatggtcgccgcgcgcgcgggcggcgcccacaagctcggctacatcgccgcccacagcgccatcgtgctcgtgtgcatcggcggcctgctcgacggcgacctggtggtgcgcgcccagacctggttcaacggcaagagcgtgttcacgggcggcggcatgattgccgacgtgccgccccagcaccggctgtcgccgcgcaatccgaccttccgcgggaacatcctggtgcccgagggcgcgcagggcagcgtggccatcctgcagcaatccgatggcgtgctgctgcaggagctgccgttctcgatcgagctcaagaagttcatcgtcgactactactcgaccggcatgcccaagctctttgcgagcgaggtggtgctgcatgaccgagaaaccggcgcccaggtgccggcgcgcatcgaggtcaaccacccggccagctacaagggcgtggaaatctaccagtcgagcttcgacgacggcggctccaaggtgaagctcaaggcggtgccgatggcggccgcggccaagcccttcgaggtcgagggcgtcatcggcgggccgagcactgaaattaccaacggcacggaaaagctcacgctcgaatatgccgcgctgcgggtgatcaacgtcgagaactttgccgacggcggcgccatgggcagcggcgccgacgtgcgcaaggtcgacctgcgccacgacatcgaatcccgcctgggcgccgccaacaagaccagcaagccaaaggtgctgcgcaacatcggcccgagcatcggctacaagctgcgcgacgcggcgggccaggcgcgcgagtatcaaaactacatggtgccggtcgacaccggcgacggccagccggtgttcctgctcggcatgcgcgagaaacccgaggagccgttccgctacctgcgcgtgccggccgacgaccagggctcgatggacagcttcgtgcgcatgcgcaccgcgctggccgacgccgatacccgcacccgggccgtcgaacgctacgtcgccaaggccgtggacccgaagcggcccgaaatggccgagcaattgcgcgtatcggccgcacgcgcgctggcattgtttgccggcagcgagcgcgccaaggccgaagccaccaccaagggcggctggcaggccattgcggagttcatggaagccaacgtgcccgaaaccgagcgcgaacgtgccggcgcggtgctggtgcgtatcctgaatgacgtgctgttcgaagtgctcaacctgagccgcgagggggccggcctggcggcattgtcgagcgaccagaagtcgcaggccttcctgacccaggcggtgctggccatcagcgacgcgtacttctaccccgcgccggtcgccatgatgatgaccgatttcacccaggtgcaggccagcgtgttccaggtggcgcgcgcgcccggcaagaacgtggtctatctgggctgcctgttgctgatcgtcggtatttttgccatgctgtacgtgcgcgaacgccggctctgggtgtggcttacaccccatggcgcgagctccggagacaacaccactgccgccaccatggcgttctcggtcaaccgcaagaccatggacagcgatcgcgagttcgagcacctcaagcacaaactgcttgccttgaagaaagaaggacaggccacgccatgaacaccaccaccctcacgctccacgaaagctggttttcgcgccgcaaccttttcgactgggtgtttgcggcactggtgctggcaggcggcctttttgcctttgcccggtatgcgggcgcgatggactcctacgagaagcccattcttgccgccgccatgatctcggtcattgccatcggctggttctggcgtccgctgcgggtgctggccatcgtggtggccgcggcctcgctgctggccatcgtgtcctaccagggcgacctggcgcgcgcggacacggtgttctggctcaagtacttcctgtccagccagtcggccattctctggatgagcgtgctgttcttcatgagcacgctgttctactggttcggtttcttcggcggcaagcagggcgacaccttcgacctgatcggctcccgactggcctgggccgccgttgccatggcgctgatcggcaccatggtgcgctggtacgagagtcatttgctggggccggacatcggccacatcccggtcagcaacctgtatgaagtgttcgtgctgttctgttggctcacgacggccttctatctttatttcgaatcgcgctacggcacgcgcacgctcggcgcgttcgtcatgctggtggtgagcgcggcggtcggcttcctgctctggtacacgctggtgcgcaacgcgcacgagatccagccgctggtgcccgcgctgcagagctggtggatgaagcttcacgtgcccgccaacttcatcggctacggcaccttcgcgctcgcggccatggtggcgtttgcctacctcatcaaggagcaagcacaagagacgcgctggtacaagctcacgccgatctggctgctgggcgtggcactgtgcttcgtgcccgtggcgttccgccagcgcgtgcaggaggccggcggcagctactgggtgatctacgcgggtatttccgcactcatcgccgcgggcatcctgctggggcgcaaacgcattgccgccaggctgcccgccaacgaggtgctcgacgacgtgatgtacaagtcgatcacggtcggtttcgcgttcttcaccattgccaccgtgctgggcgccctgtgggcggccgatgcctggggcggctactggagctgggacccgaaggaaacctgggccctgatcgtctggctcaattacgcggcctggctgcacatgcggctggtcaagggcttgcggggcacggtggccgcatggtgggcgctgggcggcctggccgtgaccacctttgcgttcctgggtgtgaacatgttcctgagcgggctgcacagctacggtaccttgtagcgcgggcggccggcttttcgcgaagaattgaaaccacgcgccgccattgcgcgtaaccgaatcagggaattgcacgaactaccctgagcacaacgattcacgcgaaaggccaccaccatgtcgtttcattcccgtccgcagggtcgcagcagcggtttcattcatccgctgtcgagcgagatcacgccgcgcgccgtctacgagggccggcgagacctgctgaagctgatggccggcggtgcggcgggcgccgcgcttgcgagctttgccgggcgagaagccttcgcccaggccacgggtccgcacaagctggcactgcttccgggcgccaagtcggccgtgccgggcgcgcaaaccatggaaaagctcaccgagtacaaggacgcgacgagctacaacaacttctacgagttcggcaccgacaagggcgatccggtcaagaacgccggcacgctcaagacgcgtccatggaccgtcgaagtcgaaggcctggtcaagaagcccggcaagtacggcatcgaagacctgctgaagctcagtgcgcaggaagagcgcatctaccgcctgcgctgcgtcgagggctggtccatggtcattccgtgggtgggttattcgctggccgagctcatcaagaaggtcgagccgcagggcaacgccaagtacgtggaattcgtgaccctggccgatcccaagaccatgcccttcgtgggctcgcgcgtgctcgattggccttacaccgaaggcctgcgcatggacgaggccatgcatccgctcacgctgctggctttcggcatgtatggcgaagtgctgcccaaccagaacggcgcgccggtgcgcctcgtggtgccctggaagtacggtttcaagtcggccaagtcgatcgtgaagatccgcttcgtcgaaaaggaaccgagcacggcctggaacaaggccgcggcgcaggaatacggcttctattcgaacgtcaacccgaacgtcgaccatccccgctggagtcaggcgaccgagcgccgcatcggcgacggcggtgggctcttcgccaagcgcaacaagacgctgatgttcaacggctacgaagcccaggtcggccagctctatgcaggcatggacctgaagaagaactactgagcccgcaccgccatccggcctttgccccatgaacaagctgctcatgcacccggcggccaagccggtcatttttctgttgtgcctgctgccgttcgcgcggctcacctacggcgcgttcaccgacggactgggcgcgaatccggccgagttcctgattcgcgccaccggcgactggaccttgcgcttcatctgtatcgtgctggcggtgacgccgctgcgcgtgatcgccaaggccaatgcgctcgcgcgctttcgccgcatgctggggctgttcgcgtacttctacgtggtgctgcacctgctgtgctacagctggttcgacatgggcttcgaatggggcgacatcgccaaggacatcgccaagcggccgttcatcctggtggggttctcggccttcgtgctgctgacaccgctggccgccacctcgttcaatcgcgccatcaaggcactgggtgccaagcgatggcagatgctgcacaagctggtctacctgatctccggccttgggctgctgcacttcttctggatgcgtgcgggcaagaacgacttcgccgaggtgttcgtctacgccgcgatcattgcggtgctgctcgggtggcgggtgtggaactacgcgagcaagcgcaagccgaagccgtccgccggtgtgcgcggcagcagcgagaagtcgctgcgcagcaccggctgaccggcggatcagctctcgatctgctcgctgcgcaactggtcttccatcgtctcgcggcggcggatcagcgtggcgcgctggccgctcaccagcacttcggcggcgcggccgcgcgtgttgtagttgctggacatgctcatgcagtacgcgcccgcggacaggacggccagcaggtcgccggcaaccacgttgagcgcacggtcgcggccgatccagtcgccgctttcgcagaccggcccgaccacgtcgtaggtcgttgcgttgccggcgcggattcgcagcggcacgatcttctggaaggcctggtacatcgcgggccggggcaggtcgttcattgccgcgtcgacgatgcagaaattcttgtcttcgccaggcttggtgtagagcacctcggtcacgcacacgcccgcgttgccgaccagcgaacggccgggttcgatgaccagcttgcgctgcccgaagccgcgcgcatcgagccgtgcgagcagttgctgccagagcgcatcggccttgggtggcacttcgccgttgtagtcgatgcccaggccgccgccgaagtccagatgatgaatgggcacgccggccgcctcgatggcctcgaccaaatcgagtatccggtcgcaggcatctaggtagggcgaggcttcggtgatctgcgagccgatgtggcaatcgatgccgaccacctcgagtcccggcagcttcgcggcgtggcgataggcctcgaccgcgcggtcatgggcaatgccgaacttgttgcccttgaggccggtggaaatgtaggggtgcgtcttcggatcgacgttcggattgatgcggatgctgatgggcgcgcggcgcccttcggccagtgccacctcgttgagtacgtcgagttcggcttcgctctcgacgttgaagcaggcaatgcccgccgcgagcgcctgccgcatttcggcgcgagtcttgcccacgcccgagaagatgatctttgcgggatcggcgcccaccgccagcacgcgcgccagttcgccgcccgacacgatgtcgaagccgcagccggcctcggcaaacacgcgcagcacgcccagcgatgaattcgccttcatcgcgtagcagatgagggcgtcgcggtcctcgaacccgcgctggtaggcggccagcgcgtccagcatccattgcttcgaatagacgaacagcggcgtgccgtgttcgcgcgccagcgcatccaggcggaggccctcgacgtggagcgagtcgtctcggtgcgcgatatggggatgtccggggagagatgcgttcgtcattatttgggcgctccgctgccggtggtggcgccggtggccggtgccggtgcgctgctggccgcggcaggcttgggcgctgcggcgtcggcgtcggaggtggcggcgcgcggcccgcccggcgtgagcagctgcggcaaggtggcgcgctgggcggctgccggatcggtcggaagaaaaagcggcccgcgctgcccgcaagcagccaaaccgcccgctgcggcagcgaggcagaccatgagcgcagcgcggctgggggcgctcactagaatttgacgaacattcaacatagcgaaattgtaatgaccgactccgaatacatggaccgcgccgaagccgcgctcgccgccatcgagcaaggctgcgaccgcatcaacgacgcgaccgatgccgatatcgacaaccagcgcgtgggcgggatgatcacgatttcattcaagaacggcagtcagttgatcgtgaatctgcagaagcccctgcaggagatatggcttgccgcgcgctccggtgggtatcactaccggtacgacggcaaggcctgggtcgacaccaagaccggtgaagaattctttggcaacctgtcgcgcgaagcgagctcgcaggcggggcagccgctggagtttgcggccgcctgaaccgccgttttctttttcagttcctgaagaggtcgaggatgcgattgcgctcttccggtggcgggggcgggctcaccggaaccccgctcagagactccgcaggcggcgtggccgcgctgtccacacccaggctggcaacgccgcggcccggcgcgtagtcgtcgtagtaccactcgccgcccacgctcacgacgccttgcggcggcgtggccgacagctcggtcacgggcacgcccttgatcgcggtctccatgtagttgatccagatcggcaggctcaggccgccgccggtctcgcggtcgcccaggttgcgcggcgtgtcgtagccgatccacgagatggccgtcatcgtcggctggaagccggcgaaccaggcgtcgagcgagtcgttggtggtgccggtcttgccgtagaggtcggtccgcttcagcatggcctgggccttggccgcggtgccggcgcgcgtcacggattgcagcagcgtgtccatgatgaatgcattgcgctggggaatggcgcggatcgtctcgttgagcagcggcggctgcttgtcgaccaagaccttgtccttgtggtcggtgatgcgggtcacgaggtacggattgacacggtagccaccgttggcgaacaccgaatagcccacggccatctgcatcggcgtgaccgagccggcacccagcgccatcggcaggtaggcggggtgcttgtccttgtcgaagccgaagttggtgatccagtcttgcgcgtagcgcgtgccgatcgattgcaggatgcggatcgacaccaggttcttcgatttcatcagtgcggtacgcatcgacatcgggccgtcgtagccgccgccgtagtttttgggctcccagggctggccgccggtggtgccggcgtcgaagaagagcggcccgtcgttgatgaccgtggatggcgtgaagcccttttcgagcgccgccgagtagatgaacggcttgaagctcgaccccggctggcgccaggcctgcgtgacgtggttgaacttgttcttgccgaaatcgaacccgcccaccagggccttgatggcgccatcgcgcgggtccatggcgacaaaagcgccttccacctcgggcagctgggtgatttcccaggtgttcttgggcgtcttgaccacgcggatcaccgcaccgcggcggatcttgatgttgggcggcgccttgtcggacaggccggactgggcgggcttgaggccgtcgcccgtgatctgcaccgggtcgccattgccgcgcacggccgtgatttccttggcggtggccttgagcaccacggccgccatcacgtcgccgttgtcgggatggtcggtcagtgcgtcgtccaccgcttcgtcgagttccttgggatcgttgggcaggtcgacgaacttctcgggaccgcggtagatctggcgccgctcgtaatccatgatgcccttgcgcagcgccttgtatgcggcggcctggtcggcggccacgagcgaggtgtagaccttgagcccgcgggtgtaggtgctgtcgccgtattgcgcgtacatcagctggcgcacggtttcggccacgtactcggcatgcagccggttcgggtcggccgcgtcgcgcaggtgcaattcttctttcttggcctcggccgcctgctcggcggtgatgaagcccgcgtcctgcatgcggtcgatcacgtagaactggcgaccgcgcgcgcgctgcggattgttgaccgggttgtttgcacccggggccttgggcaggcccgccagcatcgctgcctgcgcaatggagagctcttgcagcggcttgccgaaatacgcctcggaggcggcggcaaagccataggcgcgattgcccaggtagatctggttcaggtagatctcgaagatctggtccttggtgagcaggtgctccagcttgaaggtgagcagtacctcgtagatcttgcgggtcagcgttttctcggagctcaggtacacgttgcgcgccacctgcatggtgatggtcgacgctccctggctcttcacgcggttcatgttggccaggcccgcgcgcaccatgcccttgtagtcgacgccgccatggtcatagaagcgagtgtcttcagcggccaacaccgcttccttcaccagcttggggattgccgcgatcggggttagattgcggcgctcttcgccgaattctccaatcaggatgccttcggcggagaacacccgcagcggcagcttcggacggtagtccgacagttccgagatgtcaggaaggttggggtaggcaacggcaagggcaaccgcgatgacgcacaggaccgccaaagcgctggctgcgacgatgccgaatccccacactgtgaaacgcagcagccatttcagccaggctggtcgtgcgggtggaggagtcttggctggccctttggggcgtgaagtttcttgcatgtgggcccggagagtcaccgcacattataaaaagccgccctcttgccgggagccgaacttaggtgcatcgttgcggcctaaaccaaaagttactgaatgtggcttcaacgtcagcttttgacaacgttcccaggatttgccggctcgggttgcttggttgccgcaacgcctgctgctagcatgcaaccgaacgcacttttttccaatagttacaaatgcaggggtaaagggacctaacttggctgctttcggatcattgtttcgccgtcagaacgctcccatgctcggcctggacgtcagctcgtccagcgtcaagctggtcgagctcggccgagaagccagcggcaagctggttctggagcgctgcgcgatcgaacccctggaacggggctggatcactgacggcaacgtcgaaaagttcgacgaagtggccgaagccgttcgccgggtggtgcgcaagagcggcacccgaacgcgcaacgtcgcgctcgcgctgcccccttcggccgtcattaccaagaagatcattcttcctggtggcatgagcgagcaggaactcgaaatccaggtcgagtccgaagccaaccaatacattcccttttcgctcgacgaggtcagcctcgacttttgcgtgaccggacagagcaccgcctccgccggcgatgtcgaagtgctgattgccgcgtcgcgcaaggaaaaggtgcaggatcgcgaaggcctggccgaagcggccggcttgaaggcggtgatcctcgacgtcgagtcctatgcctcccgcctcgcgaccgctcgcctgatcgagcagctgccgggcaagggcgtcgatgccgtcgtggcgcttttcgaagtgggcgccttcaccaccagcatgcaggtgctgcgcaaccaggaggtgctgtacgaccgcgaccaggccttcggcggcgcccagctgacccagctcatcgtgcgccagtatggtttttccgccgaagaggccgaagccaagaagcgcagcggcgacctgcccgacgactacggctcgggcgttctgaagcctttcgttgaaagcatcgcgcaggaaatcgcacgcgcgctgcagttcttcttcaccagcacgccccacaaccgcgtggactacgtgctgcttgcaggcggatcggcttcgttgcccagcctgaccagcgccgtcacgcgccagacctcgttcgcctgttcgctggtgaacccgttcgatggcatggaaatgggctccaacatccgcgagaagaaggttcggcgcgaagcgccttcctatctgacttcctgcggtctggccatgcggaggttcgtgcagtgattctcatcaatctgcttccgcaccgcgaggccgcgcgaaagcggcgtcgcgaggccttctacggcacgctcggcgcagccgcggtcctgggcgtactgatcgccggcctggcctttctctggttcgaggcgcaaatctcggcccagcaagccaagaacaccttcctgaagaccgagatcaccaagctcgacgccgagatcaaggagatctcgacgctgcagcaggaaatcgcagccctgcgcgcacgccagcaggcagtcgaagatcttcagggcgaccgcaacctgccggtgcacctgctcaacgagctggtccggcagttgcccgacggcgtctatctcaccagcatgaagcaggacaaccagaccgtcacgctgcagggcatggcgcagtcgaacgagcgcgtctctgaactgctgcgcaacctgggcaacaacagcccctggctggtcaagcccgagctggtcgaaattacttctgcgacggtgagcctgagccagcgcgatcagcgccgggtggcgaacttcacgatgcgcatcggcctgaagcggccgaccgacgcgcagaaggccgcggctgacaaggcgctggccgcatcggcgcaagtcaaggggtagacggatcatggcaagcaatcgcccctcccaaaaaatcgacgtcgccgcggcaatgcgcggcttcggcgatcagtttcgcaacctgaacgcgaacgacccggccagttggccgccggtgccacgctatgtcctgtgcctggtggtgaccgcgctggtgttggtcggactgtggttcgtgtggctgaccaattcgaacgacgagctcgagagcgagcgcgccacggaagtcacgctccgcgccgactaccagaagaaggtggccttggccgccaatctcgacctgctgaagaagcagcgcgagcaggtgcagcagtacgtgacgctgctcgaaaagcagctccccagcaaggcagaaatggatgcattgctgtccgacatcaaccaggccggcctcgggcgcagcctgcagttcgaactgttccgtccgggacaggtttcggtgaaggactactacgccgaactgccgatcgccgtgcgcgtgaccggccggtaccacgacatcggctcttttgcggccgacgttgcgagcctgtcgcgcatcgtgacgctgaacaaccttacgatcgctccgcaaaaagacaaggacggcacgctgacgatggatgccacggcccgcacctaccgctatctcgatgacgaagagcgggcggcccagaaacgcgccgcggcgccaaaggcccagaaatgaggacgaccgccaaaatcctgtggctggtcatggcagccctgggcctgagcgcctgcgccgattcggagcaggaagacctgcgccgctggatggtggagcagcgcgcccaggtgaagcccaacgtgccgccgatcaccgaacccaagaagttcacgccccaggcctacaccgaagggtcggcgttcgagccgttcaacctgctgaagctgacccaggcgctgcgccgggattcgaaccagcccagcacgtcggaactgatcgcccctgaactggtgcgccgcaaggaggcgctcgaagctttcccgctcgactcgatggccatggtgggcagcatgaaccgcaacggccagccggtggcgctggttcgggtcgacaagctgctctacaaggtgcgggtcggcgagtacctggggctcaactacgggcgcatcacccgtatcaacgaaaccgaagtcgccttgcgtgaaatcgtgcaagacgctgccggtgaatggatcgaacgcgtggcgacattgcagctgcaagagagtgcgaacaaatgaatcacaaaaaatcaacgatggcacagcggctgcgagccgccgggctgggtctcttggcatttggcgcgttcgcgattgcccatgcgcaaaacgccatcgaagcggtgaccagctcgacgcaatccggcgccgaggtgatccgcatcgacctcgcacagccgctcacggccgtgccgaccggttttgccgttcagacgccggcgcgcatcgcgcttgatttcccgggcgtgacgaacgccatcggccgctcctccatcgaggtgaaccagggcaacctgcgttccgtcaacgtggttcaggccggcgaacgcagccgcgtggtgctgaacctcaaacaggcaaccgcgtacaaggccgagatccagggcaagtcgctgctggtgattctcgagcccgtggccggtacggccctggcttcgtccacgcccaacgtctttgcggaaaaccgcaatcgcgacaccctgccgctgcgcgatgtcgacttccgcctgggcacggacaacaccggccgcgtgatcgtcgatctgcccaacaaccaggtgggcgtcgatgtgcgccagcagggcaagaacctcgtcgtggagttcaccaagtcgaccctgccggaggggcttcgccgccgcctcgacgtggccgacttcaatactccggtccaactgatcacttcgcagcagtcgggcgaccgcgtgcgcatgacgatcgaggccaagggcgactgggagcacagcgcctaccagagcgaaaaccagttcgtggtcgaagtccgcgcccgcaaggtggacccggccaagctgacccaaggcgtcggctacaacggcgagaagctctcgctgaacttccagaacatcgaaatccgttcgctgctgcaggtgatcgccgacttcacgaacttcaacatcgtgacttccgactcggtcaccggctcgctgacgctgcggctgaaggacgtgccttgggaccaggcgctggacatcatcatgcaggcgaagaacctgggcatgcgcaagaacggcagcgtgctgtggatcgcgcccaaggatgaaatcaacgccaaggaaaagctcgatttcgaggccaaggccgcaatcgagaacctggagccagtgcgcacccagtcgttccagctcaactacaccaaggcgattgcgattgcgcaaggcctgaccggaaccggcgcctcggcaggcggcggtggcggctccggcaccaccacgcgcatcctgagcccgcgcggcagcgtgatcgcggagtcgcgcaccaaccagctgttcgtgtcggacatcccgtcgcgactggcacaagtggccgacctgatccagaagctcgacattccggttcgccaggtgctgatcgaagcccggatcgtggaagcctccgacaccttcggcaagtcgctgggcgtgcggctgggcggcggcattgccggcgagcgcttcgcctcgtcgtcgggcaaccgcgcctttgccaacctgggcatgatgccggcggtgacctcgggtgcgagcggcaacaccgccaccaccacctggaccaactccaacttcatcaacctgccttcgggcgatgccggtggtactggtaattctccaggcaccttcgcgatctcgctcttcaattcgagcttctcgcgcatgctgaaccttgaaatctcggcactcgaagccgacggcaagggcaaactggtgtccagcccgcgcgtcatcacggccgaccagacgaaggcgctgatcgagcagggcgaagaaattccctaccagcaggccacgtcgagcggcgcaacgtcgatttcgttccgcaaggccgtcctgaagctcgaagtcacgccgcagatcacgcctgaaggcaacatcatcctcacgctggatgtgagcaaggacgcacgcggcgtcaatacttcggcaggtccggccatcaacaccaagcacgtgcagaccgaagtgctggtcgagaacggcggcacagtcgtcatcggtggtatcttcgaactcaccgaaaccaatgacgaatcgcgcgtgccggtgctgggtgaagtgccctacctgggtgcactgttccgcaagcgcgaacgcgttgccaacaagaccgaaatgctcgtctttatcactccgaagatgattaccgaccgcaacgccgcgcgctgacgcgcgggcgtagcagccaccgcgtggcggtcgcactcgtcgggttgcccggcgccggcaaatccgcagtgggccggcgccttggcgcgcgcctggatcttcccttcgtcgataccgaccatgtcatcgagcagcgcatcggctgctcgatccgcgactacttcgaccgcgagggcgaaaccgccttccgcgatctcgaagagaccgtcatcgccgacctggccgcgcattcccatggcgtgctggccaccggcggcggcgcggtcctgcgggaggccaaccgcaagcagctgcgggatcacttccacgtgatctacctgcgttcttccccggaagatctgttccggcgcctgcgccacgacgtcaagcggccgcttctgcaggtggcggatccgctcggccgcttgcgcgagctgcacgatgcgcgcgacccgctctaccgcgagacggcccacgacgtagtcgacaccgggcgcccgtcgatcgccatgctggtgaacatcatcgtgatgcagctcgagcttgccggcatcgtcgtgccgggatcccggcccgaagagcccacgggctgagctggcctggctgcagcgcctaaactcgctgccatgtcattgtccgcaccctccgccacgcccgaacgcgtcgacatccagctcggcgagcgcagctatcccatcctcatcggcaccgccctgctggacgatccccagagctttgccgtcgttcccaccgctgccagcgcgctgatcgtcagcaacaccaccgtggcaccgctctacgccagcgccttgcgcaccgcgctggccggccgcttccgcacggtgcacatgctcgagctgcccgacggcgaagtgcacaagaacctgcagaccctcaacttgatcttcgacgccctgctgggccacggcagcgaccgcaagacggtgctttttgcgctgggcggcggcgtggtgggcgacatgaccggctttgcggccgccagctacatgcgcggcgtgcctttcgtgcaggtgccgaccacgctgctggcgcaggtcgactcgtcggtgggcggcaagaccgccatcaaccacccgcttggcaagaacatgatcggcgcgttctaccagccgcagctcgtggtgtgcgacctgggcacgctgcagaccttgccgccgcgtgagttgagcgcgggcctggccgaagtcatcaagtacggcccgatccacgacatggcgttcttcgactggatcgaggcgaatgtcgatgcgctggtggcccgcgacccggccgcgctggcctacgcggtcaagcgcagctgcgagatcaaggcgctggtcgtcgggcaggacgagcgcgagaccggcctgcgcgccattctcaacttcggccacaccttcggccacgccatcgagtcgggcctcggctacggcgaatggctgcacggcgaagcggtcggttgcggcatggtcatggcggcgcacctgtcgcagcggctgggcggcatcgatgcggcattcgtccagcggctcacgcggctgatcgagcgggctggtctgccgaccgtcggccccgcgctgggtgccgaccggtatctcgaattgatgcgggtcgacaagaaatccgaagccggcgagatccgcttcgtggtgatcgacaagccgggctcagccgcggtcagcagcgcgcccgatgcgctcgtgcgcgaagtgctcgcgcagtgctgccgcgcggaatgagcgcagcgccaagggtgcagccatgaacctcgcggcctatgcctgccaccctgcgcggtcgcgcgggaggcggcataccgagccgccggcgcccacgcgcgatgccttccagcgcgaccgcgaccgcatcgtgcattccaccgcgtttcggcggctggtctacaagacccaggttttcctgaaccatgagggcgacctgttccgcacgcggctcactcattcactcgaggtggcgcagctgggccgttcgatcgcgcgggccttgcgaatcaacgaagacctggtcgaggccattgccctcgcgcacgatctcggccacacgcccttcggccatgccggacaagacacgctcaacgcctgcatggaaggcgagggcggcttcgagcacaacctgcagagcctgcgcgtggtcgacgccctggagctgcgctatccgcaattcgacggcctgaatctcagcttcgagacccgcgagggcatcctcaagcattgctctcgcgcaaatgcggaacgcctggaagccgcagaacccaacggcgtggcgcggcgcttcctggaccgcacgcagccggggctcgaagcgcagctctgcaacctggccgacgccattgcctacaacgcgcacgacatcgacgatggcgtgcgctcggggctcatcagcgtggagcagctcggcgaggtggatctgttcgagcgctaccgctgcgaggcgctggccgaatatccccatctggaagggcggcgcgtgctctacgaaacgatccgccgcatgctgagcgcccaggtctacgacgtgatcgatgccacccgcgcagcgatcgaaacggcgaagccggccgatgcggacggagtgcggaactccccgccgctcgtcgcgttcagcgacaccatgcaggtgcagtccaacgcgctcaagggcttcttgttccgcaacctctatcggcatccgcaggtgaggcagaccaccgagcaggcgcagcaggtggtgcgggagctgttctccgcctacctcgagcgccccgccgagatgcccggttcctatgccgagcgccgcgaccggcaccgtgccgtggccgactacatcgccggcatgaccgaccgttttgccatgcgcgagcatgaaaggctgaccggccggcgaggcattgcatgagcgcccgcccggccgttccgaagggggctcgcaccgcagcccgtcagggcgaaggtgctccgatgagcgcaacggccgtggtgcccgctcgcgttcccgccgctgccttcgcggtggtgctgggcggcgtcagcgcagcgctgcacctgggcaagctgccgcccgctgtgccggcgcttcaggcttcgctcggcatcggtcttgtcgaggcgggttttctgctctcgctggtgcaggtggcgagcatgacgctggggctcgcggccgggctggcagccgacaccatcggcttgcgccgcagcatgctgacggggctcctggtgctgacggcggccagcctgctcggcggcggcgtgggcgccggccttttcggcagcgcgcatgcggtgcaatggctgctgctcttgcgtgccgtcgaaggcatcggctttctcctggcggtcatgccggggccggggctgatccgcgcattgactccggcgggcgccgacaaggcagcgctgggcgtgtggggcgcatacatgccgctgggcgtggcgctcgcgctgctgctggggccggccttgatcgcctggggcggatggggcgactggtggtgggcgctgtccgccgtttcggccgccgcggcgctctggctctggtcggccgtgccggcggacgggcttcgttccgttgcggcaggcagcggcatgccgggcggctggtcgtcgcgcctgcgcgccaccgtcggcgcccgcgcaccctggatggtcgcgtcgagcttcgcggtgtattcggcgcaatggatggccgtgatcggcttcctgccagccatctatgccggcgccggcgtgccggccggctggaacgcggtactcactgccatcgcggccgcgatgaacatcgtcggcaacctggcgggcggacgctggcttcagcgcggcattgcgccagagcgcctgctgcaatggggcttcctggcgatggcgctgggcggcgtggccgccttcgcgcaggtggggcagggggccgacgcaatcggcctgccgccagcgctgcgctatgccgcggtctgcgctttttcgctgggcgggggcatggtgcccgccaccctgttcctgctcggagttcgcctggcgccggggcccaccaccgtttccacgacggtcgggctcatgcagcaggcctcttcgctggggcaattcctggcgccacctgcggtcgcgtgggtggctcaccgtgtcggcggttggcactggacgtgggcggccacgctggcatgctcgctggccggcatggccattgcgcggcgcctggggcgaatacgcctggcggcggaggtggcatgagcggcgcggcgacaatcgacgccattcaggccgaagccgatacgcggcgctggctcgagcgcgcggtgatcgggctcaacctgtgtccgttcgcgaaggcggtgcatgtgaaggcgcagatccactatgccgtgtacctgcctgccgacgacgccgcgctgagcgacgctttgttggcagaggccgatgaactcgccgcgctcgatgcctccgtgcgcgacaccaccttgctgatagcacccaacaccttggcggattttctggacttcaacgatttcacggcgcgcgccgaacgcaagctcgcccgggcgggtttcgacggcgtgttccagctcgcgagctttcatccgcactttcaatttgcgggatcgcagagcgatgacatcacgaacgcaaccaaccgcgcgccgtaccccacgctgcacctgctgcgcgaagacagcgtgagccgcgcggtcgaggcgtttccagaggccgaagccatcttcgagcgcaacatcgaaacgctcgaagcattgggtccgcatggctgggccgcgctcgacgtgggcccagggagcgcccgatcatgatgaatgcacaagcgaccaaggcggtgaagaccgccaaggcctccaaggccgaagccgagctggcggaggttctgcgtccggggcagtccgtcgagctgctcaaggagctgcacatcctcacgcgcgagggccgtctcaaccaggattctcggcgcaagctcaagcaggtctaccacctgttccagttcatcgagcaattgctgcgcgagctgcccggtggcggagccgaggccacgctggccgaccatggcgccggcaagtcgtacctcggcttcatcatctacgacctgttcttccgggcgcgccagggcggccatgtctatggcatcgaaacgcgaagcgaactggtcgagaagtcgcgggcattggcacggcaactcggcttcgatcgcatgtcgttcctgaacctcacggtggccgaatcggcccaggcgagcgagctgccggagcggatcgacgtggtcaccgcgctgcacgcctgcgacaccgcgaccgacgacgccatcgccttcgggctcgcgaagaaggcgcgctgcatggtgctggtgccctgctgccaggccgaggtggcggcgtgcctgcgcgaaaccaaggcgctagccctgtcgcgaacgcccttggccgaactctggcgccatccgctgcacacgcgcgagataggcagccagctcaccaacgtgctgcgctgcctctatctcgaagccaatggctacagcgtcaccgtcaccgaactggtgggctgggagcacagcatgaagaacgaactgatcctggcgcgccacaccgggcagcgcaaggccgccgccgcgacgcggctcggcgagctgctgtcgcaattcggactcgatgccttgggcgatacgcggtttcgcctgtcctgaaaacccgcgagagcgcgctcgttcgattgacgccatggcccgcctgccccgcctcacgctcgccgacatgccgcaccacgtgatccagcgcggcaacaaccgccaggtgatcttcgtcgaccgcgcggaccacgagcggctgctcggcctgctggcggacgcggccgcgcgctttggcgtggcactgcacgcctacgtgctgatggacaaccatttccatttgctggcaacgcccagcaccaccaccgggctgccgcagttcatgcaggcggtagggcgcagctatgtgcgctacttcaacgaccgccacggccgcagcggcaccctctgggaagggcgctacagatcgacgctgatccagaccgaccgctatctgctgacctgcatggcgtacatcgacctcaaccccgtgcgggccggcctggtatccgacgcgcgcgactttccgtggtccagccacgggcactacgcggggctgcggcacgacaagctgctgacaccgcacccgctgtactgggaactcggcaacacgcccttcgcgcgtgaagcggcgtatgcggagttggtgcgcgccggtgtgcggcctgccgaccaaggtgccctcaccgaggccactttgcggggatgggcggctggcgatgcaaattttctcgcgtcgcttcaaaaatccaccgagcgccgggtggccaagaccaaggccgggcgtccgccttccgcctcccgttcctgattcgattggcgcctgttgggctgcagtggtcggccttttgctattttttttgatatgtccctaatttatttctgacaagaagactcaggatttaatgggaatctgacccccaataaagtatttggcattctttgtgcatcgcaatatccttcacatccctgcgaaaaactgatgaaggagtgcgccatgacgacggctgccgagatcgaacatctccaacaacacggtctgtattccggtgccgacgagcacgatgcctgcggcgtcggcttcgtggcgcacatcaagggcgagaagagccatgccatcgtgctgcagggcctcaagatcctcgaaaacctggaccatcgcggcgcagtgggcgctgacaagctgatgggcgacggcgcgggcatcctgatccagctgcccgaccatctgtaccgcgaagaaatggccaagcagggcgtcacgctgccgccgcccggcgaatacggcgtgggcatgatcttcctgcccaaggagcacgcgtcgcgcgaagcctgcgaacaagagatggaacgcgccatcaaggcggaaggccaggtgctgctgggctggcgcgacgtgccggtgaaccgcgacatgccgatgtcgcccaccgtgcgcgccaaggagccgctgctgcgccaggtgttcatcggccgcggcaacgacgtgatcgttcaggacgcgctggagcgcaagctctacgtgatccgcaagaccgccagcgccaacatccagcgcctgaagctcaagcacagcaaggaatactacgttcccagcatgtcgagccgcaccgtggtctacaagggcctgctgctcgccgaccaggtcggcacctactacctcgacctgcaggacaagcgctgcatctcggccctcggcctcgtgcaccagcgcttctcgaccaacacttttcccgaatggccgctggcgcacccgtaccgctatgtcgcccacaacggcgaaatcaacacggtcaagggcaactacaactggatgaaggcacgcgaaggcgtgatgtcctcgcccgtgctgggcgccgacctgcagaagctctaccccatcagcttcgccggccagtccgacaccgccaccttcgacaactgcctcgagctgttgacgatggccggctaccccatcagccaggccgtgatgatgatgattcccgagccctgggaacagcacgccaccatggacccgcgccggcgcgcgttctatgagtaccacgccgccatgctcgagccttgggacggcccggcctccatcgtgttcaccgacggccgccagatcggcgccacgctcgaccgcaacggcctgcgtccctcgcgctactgcgtgaccgacgacgacctggtcatcatggcgtcggaatcgggcgtgctgcccgtgcccgagcagaagatcgtgcgcaagtggcgcctgcagcccggcaagatgttcctgatcgacctggaacagggccgcatgatcgacgacgaggaggtcaaggccaccctcgcgaacagcaagccctacaagcagtggatcgagaacctgcgcatcaagctcgacagcgtcaaggccgagccggccgcatcgacgatcaaggcgcccgtgagccaggtggcattgctcgaccgccagcaggctttcggctacacgcaggaagacatcaagttcctgatgagcccgatggcgcaagccggcgaagagggcatcggctccatgggcaacgacagcccgctggccgtgctctcgaacaagaacaagccgctctacaactacttcaagcagttgttcgcgcaagtgaccaacccgccgatcgatccgatccgcgaggccatcgtgatgtcgctggtgtccttcatcggccccaagcccaacctcctggacatcaaccaggtcaacccgccgatgcggctcgaagtgagccagccgatcctcgactttgccgacatggcgaagctgcgcgacatcggcaagtacacccagggcaagttcaagagctatgcgctcgacatcacctacccgctcgcctggggcgacgaaggcgtcgaggccaagctggcctcgctgtgcgccgaagcggtggatgccatcaagggcggccacaacatcctgatcgtgagcgaccgcggcgtgagcccgacgcaggtcgcgatccccgccgtgctggcgctgtcggccgtgcaccagtacctggtgcgtgagggcctgcgcaccacggccggcctggtggtggaaaccggctcggcgcgcgaggtgcatcacttcggcgtgctggccggctacggtgccgaagccgtgcacccctacctcgcgatggaaacgctggcggccatgcatgccgacctgccgggcgacatgagcgcggagaaggcggtctacaactacgtcaaggccatcggcaagggtctctcgaagatcatgtcgaagatgggtgtcagcacctacatgagctattgcggcgcccagctgttcgaagccatcggcctcaacaccgagacggtgaacaagtacttcaccggcaccgcgagccgcgtcgagggcatcggcgtgttcgagattgccgaggaagccatccgcatgcacaaggcggcattcggcgacgacccgattctttccaacatgctcgatgccggcggcgaatacgcctggcgcacccgcggcgaagagcacatgtggacgcccgacgccatcgccaagctgcagcacagcacgcgctccaacaactggaacacgtacaaggaatacgcgcagctcatcaacgaccagaaccgccgccacctcacgctgcgcggcctgttcgagttcaagatcgatcccgccaaggccatcccggtcgacgaggtcgagtccgctgccgaaatcgtcaagcgctttgccaccggtgcgatgtcgctcggctcgatcagcaccgaggcgcacgccacgctcgccattgccatgaaccgcatcggcggcaagagcaacacgggcgagggcggcgaagacccggcgcgctaccgcaacgagctcaagggcatcccgatcaagcagggcgatacgctcaagagcgtgatcggcgcggccaacgtcgaggtcgacctgccgctcaaggacggcgactcgttgcgttcgcgcatcaagcaggtggcttcgggccgcttcggcgtcacggccgaatacctgcattcggccgaccagatccagatcaagatggcgcaaggcgccaagcccggcgaaggcggccagctgcccggcggcaaggtcaccgaatacatcggcaagcagcgctatgcggtgccgggcgtgggcctgatctcgccgccgccgcaccacgacatctattccatcgaagacctggcgcagctgatccatgacctgaagaacgccgcgccgcatgccagcatcagcgtcaagctggtgagcgaaatcggcgtgggcaccatcgcggccggcgtggccaagtgcaagagcgaccacgtggtgatcgcgggccatgacggcggcacgggcgcatcgccctggtcgtcgatcaagcacgcgggcagcccgtgggaaatcggcctggccgaaacgcagcagacgctggtgctcaaccgcctgcgcagccgcatccgcgtgcaggccgacggccagatgaagaccggccgcgacgtcgccatcggcgcgctgctgggcgcggacgaattcggctttgccaccgcgccgctggtggttgaaggctgcatcatgatgcgcaagtgccacctcaacacctgcccggtgggcgtggccacgcaagacccgatcctgcgcaagaagttctcgggcaagcccgagcacgtcgtcaactacttcttcttcgtggccgaagaagtgcgccagatcatggcccagctcggcatccgcaagttcgacgacctgatcggccgcgccgacctgctcgacatgcgcaagggcatcgagcactggaaggcttcgggcctggacttcagccgcctgttcgcgctgcccatcgtgccggccgacgtaccgcgctaccacgtcgagaaccaggaccatggtctcgagcgtgcgctcgacgtcaagctcatcgagaagtcgcgcccggcgatcgagcgcggtgagaaggtgcagttcatcgaggtggcgcgcaacgtcaaccgctcggtgggcgccatgctgtcgggcgcgctgaccaaggtgcatccgcaaggcctgcccgacgactcgatccgcatccagctcgaaggcacgggcggccagtcgttcggcgccttcctggcgcgcggcatcacgctctacctgatcggcgatgccaacgactacaccggcaagggcctctcgggcggccgcgtggtggtgcgcccgagcctcgacttccgcggagaagcggcgcgcaacaccatcgtcggcaatacggcgctttacggtgcgaccaccggtgaagcgtatctttgcggcgtggccggcgaacgcttcgcggtgcgcctgtcgggtgccacggccgtcatcgaaggcaccggtgaccacggctgcgaatacatgaccggcggtacggtcgcggtgctcggcaagacgggacgcaacttcgcggccggcatgagcggcggcgtggctttcgtctacgacgaagacggccagttcgccacgcgctgcaatctctcgatggtgtcgctcgacaaggtgctgacctcggccgagcagttggcaagcgtgcaccgcaagatctggcacggcggcgaaaccgacgaggcccagctcaagaagctgctcgaagagcatcaccgctggaccggcagcaagcgcgcgcgcgaactgctcgacaactgggccgtgtcgcgcaccaagttcgtcaaggtgttcccgaacgaatacaagcgcgcgctcgccgagctgcacgaccgcaaggtcgaactcacgagcagcggcaacaacgcgcacgtgggccttgagccgcacgcgctggctcccgcaccgcagacgtcgccggcttcggtctgagcgcccacgagaacgcagagagaaaaaggacatcacgatgggaaagatcaccggcttcatggagcatgagcgcgtcgaagagggctacaagcccgcctccgagcgcgtcaagcactacaaggaattcgttgtcggcctgacggtcgagcaggccgaggtgcagggcgcacgctgcatggattgcggcacgccgttttgcaacagcggctgcccggtcaacaacatcattccggacttcaacgacctcgtgtaccgcaacgactggcagaacgccttcgcggtgctcgactcgaccaacaactttccggagttcaccggccgcatctgccccgcgccctgcgaagcggcctgcgtgctcaacgtgaacgacgacccggtcggcatcaagtcgctggaacacgcgatcatcgatcgcgcctgggacgaaggctgggtggcgcctcgcgttgccaagcacaagaccggcaagaaggtggccgtggtgggttcgggcccggccggcatggccgcggcgcagcaactcgcgcgtgccggccacgacgtgacgctgttcgagaagaacgaccgcatcggcggcctgctgcgctacggcatccccgacttcaagatggagaagacgcacatcgaccgccgcgtcgagcagatgaaggccgaaggcgtgaccttccgcaccggcgtgatcgtcggcgccgcgaaagacccgctgggcaagggctccaaggtaaccaacctcgccaaggaaactgtcacgccggaacaactgcagaaagagttcgacgccgtggtgctcacgggcggtgccgagcagtcgcgtgacctgccggtgctgggccgcgacctcgacggcattcactttgccatggagttcctgccgcagcagaaccgcgtcaacgcgggcgacaaggtcaagggccaactgcgcgccgacggcaagcacgtcatcgtcatcggcggcggcgacaccggctccgactgcgtgggcaccagcaaccgccatggcgcagccagcgtcacgcagttcgaactgatgccgcagccacccgaggaagaaaaccgtccgctgacctggccctactggccgatcaagctgcgcaccagctccagccatgaagaaggctgcgagcgcgagttcgccatctccaccaaggaattcatcggcgaaaagggcaaggtcaccggcctcaagaccgtccgcgtggagtggaaggacggcaggatgcaggaagtggccggcagcgagcagatcctcaaggccgacctcgtgctgctggccatgggcttcgtgagcccggtggccaacgtgctcgatgccttcggtgtcgagaaggacgcacgtggcaacgccaaggccacggtcgatttcatcggcggctacgttaccaatgtgcccaaggtgtttgccgctggtgacattcgccgcggccagtcgctcgtcgtgtgggcgattcgcgaggggcgccaggcggcgcgctccgtggatgaattcttgatgggttttagcgacttacctcgctgaattttgtttcagtttggcggaggccccccacggccccgctatcattcgcggaaaccgcatgccgggatgcctgagaaggcgcccggcttttttattgagatggacccagccgcactgccacacccttttgtagagtttcgcgacgtttcgttcggctacggcgcgcgcgcgatcctcgaccgggtgtcgttcgcggtcccgcgcggcaaggtcactgcgttgatgggcgcctcgggcggcggcaagaccaccgtgctgcggctcattggcgggcagcagcgggcgcagcacggcgaggttcttttcgacggccgcgatgtcggcaaactcgacgccgccggcctgtatctggcgcggcgccgcatgggcatgctgttccagttcggtgccttgttcaccgacatgagcgtgttcgacaacgtcgcctttccgctgcgcgagcacacgcagctctcggaagcgctggtgcgggacatcgtgctcatgaagctcgacgcggtcggtttgcgcggcgcgcgcgacctgatgcccagcgaagtttcaggcggcatggcgcgtcgcgtcgccttggcacgcgccattgcgctggaccccgacctcgtcatgtatgacgagccgtttgccggcctggacccgatttccctgggcacggcggcacggctgattcgccagttgaacgacacgctcgggctgaccagcatcgtggtgtcgcacgacctcgaagaaaccttccgcattgcggatcacgtgatcatcctggccaacggcggcatcgccgcgcagggcacgccgagcgaggtgcgcgaaagcgccgatccgctggtgcatcagttcgtgaacgcgctgcccgacgggcccgtgcattttcactacccggtcgtcggcattgaagaagatttcggcaatgaaggggggcggacatgagcgcagcgctgggccgccccgagcaagcgaaggccccctcggggggcagcgaggacacgaagtgccgagagtgggggcagatatgagctggttgaagcccgctgatgccggatttgccgtgcgcagcaaactggccgacctcggttatggcgccaagcttttcctgcgcctcctggtacagggggcacaaagcttgcgtcgcttcgggctggtacgcgaccagatccatttcctgggcaactactcgctcgccatcatcgcggtgtccggtcttttcgtcggtttcgtgctgggtctgcagatgtattacgcgctgcagcgctacggttcttccgaggctttgggcctcttggtcgccttgagcctggtgcgggaactcgggccggtcgtggccgccttgctcttcaccgggcgcgcgggcacgtccctgactgcggagatcggactcatgaaggccggcgagcagctcagtgccatggagatgatggcggtcgacccggtgcagcgcattctggcgccgcgcttctgggccggcgtcatcaccatgccgctgctggcggcggtgttcagcgccgtcggcatcatgggcggctacgtggtcggcgtgctgatgctgggtgtggacccgggggcgttctggggccagatgcagggcggtgtcgacgtgtggcgcgacgtgggcaacggcgtgatcaagagcatcgtgttcggtttcaccgtgaccttcattgcgctgctgcagggctacgtggcacagccgacccccgaaggcgtgtcgcgtgccaccacgcgcaccgtggtgatggcgtcgctttcggtgctcggcctcgacttcctgttgaccgccatgatgttcagtatttgaaggagctccgctccaatcgttctagagagtgcaaaccatgcaacgttccaatagcgacatctgggtcggcctgttcgtcctgatcggcggcgcggcactgctgttcctcgcgctgcagtcggccaacctgctgagcctgagcttccagaagacctacaacgtcaccgcccgcttcgacaatatcggcggactcaagccgcaaaccgcagtcaagagcgctggcgtggtggtcggacgtgtggaatccatctcgtttgacgacaaatcctttcaggcccgcgtgacgctggctttgcaaaaccgttacagttttcccaaggacagctcgctcaagatcttgaccagtggtttgctcggcgagcagtacatcgggatcgagccgggtgccgaggagaagagtctgcaagccggcgacaccatcaccgcgacccaatcggccgtggtgctggaaaacctgatcagccagttcctctatagcaaggccgccgaaggaagcaatacgccttcgacgccgggaacagccaacaagaaatgaaaaccagtcttttttcgtccattgctatcaagaaggtagcaaactccgcccgcgtggtgggcgctgtagcaacttttgtgctgcttgcaggctgcgcgagcggcccccacgccaatccggccgatccgttcgagccgttcaatcgcggcgtcacccgcttcaacgacacggtcgacgacgcggtgctggtgcccgtggccacggcctacacgcgcgtgctaccttccatggtgcgcaccggcgtgagcaacttcttcggcaacctgggcgacgtctggagctttgccaacagcgtggcccagctcaagctgcagaacagtgccgagaccttcatgcgggtcaacgtgaacaccttcttcgggctgggcggcctgctcgacgtggccaccgaagccggcatcgatcgccatgaggaagatttcggccagacgctcggccgctggggcgtgggtgccggcccgtacgtcgtgctgcctgtttttggcccctcgaccctgcgcgacaccgcggcattgccggtcgaccgtgccggcggcatcgtctcgaacatgaacgacgtggcctggcgcaattcgctgtcgttcctggaagctgtcgatacacgcgcaaagtacctgcgcgccggccgcctgctcgacgacgcggcactcgacaaatacaccttcacgcgcgacgctttcctgcaacaccgccgcaacgacgtctacgacggcaatccgcccgacgacgaaggcggcaagtaaggggccggggtgatggcggccggtagaaaagcttttgcttgcatccggtttcaaggcttcacctgtgcttcaggaacccggtcggcgtggaacccgtcgaacacgttctttccaggagccgcgtcgatctatcgcgtgtctcctgccgatttcaaaaatttaagggaattgccatgaacaacaatatcttgcaacgacgcggctttggccgcctggtactggccagcgcactccttttcggcgctgccaccgctttcgtgcgcccggccctcgcggccgacgaagcgcctgacgcgctggtgaagcgcctgtcgaccgacgtgctcgaaaccatcaaggccgacacctccatcaagtcgggcgacgtcagcaagatcatggtgctggtcgacagcaagatcatgcccaacgtcaacttccagcgcatgacggcttccgccgtgggcccggcatggcgccaggccacgccggagcagcaaaagaggctgcaggaagaattcaagaccctgctggttcgtacctatgcgggcgcgctcgaccaggtgagcgaccagaccgtcacggttcgtccgttccgcggttcgccggaagacaccgaagtgctggtgcgcaccgaggtcaagggccgcggcgacccggtccagctcgactaccgcctcgagaagacgcccggccagggcggcggctggaaggtctacaacctcaatgtcctgggcgtctggctggtcgacacttaccgcacgcagttcgcgcaggaaatcaacgcccgcggcatcgacgggctgattgccgcgctggccgcgcgcaacaagggcaacaacggcaagagctgacgccatgctggtgctgccgaccaaactcacccacgacgatgccccggcctgcatgcgcatgctgcagcaggggttgaagggacagaccgacacctccaccgtcgtggacgccagcgccctgacgcagttcgattcctcggcgctggcggtgttgctggagtgccggcgtgaatcgagcgcgcttggccgcggctttgccgtgaaggggctttccccccggctgcgcgagcttgctgccctgtacggcatcgccggcctcctgccggccgcaccctgagggcgggtggccccggcgggcgccgcgtcagggcatcccggcgccgcccagcggcttgtaacgcaggcccgtaaaatcgccggctctcatgcccgcgatctcattccaatcggtctccaagacctaccctccctccagacagcaacgggcccaaggcaagcagggcctgcgcgccgtcgacgaggtcagcttccagatcgagccgggcgagttcttcggcttgctcggccccaatggcgcgggcaagaccacgctcatcagcatgctggccggcctgtcccgtcctacggccggcgcgatcagcgtccacggcttcgacgtgcagcgcgactatgccgaggcccggcgccagctcggcatcgtgccgcaggagctggtgttcgaccccttcttcaatgtgcgcgaatcgctgcgcatccagtcgggctacttcggcatcaagaacaacgagccctggatcgacgagctgctgcaaagcctcggcctggccgacaaggccacggccaacatgcgccagctgtcggggggcatgaagcgccgcgtgctcgtggcgcaggcgctggtccacaagccgccggtcatcgtgctcgacgagccgaccgccggggtcgacgtcgaacttcgccagacgctctggcagttcgtcgccaggctcaacaaagagggcagcaccgtgctactcaccacgcactacctcgaggaagccgaggcgctgtgcagccgcatcgcgatgctcaagcagggccgcgtgattgcgctggaccgcaccagcgaactgctgaaatcggccaccagcaacgtgctgcgcttcaagaccgacgccatgctgccgtgggccattgcccagcatgcgcgaattaccggacgcatcgtgcagctgccggcgcagaacgcccatgaagtcgaacaattgctggccgcgatccgcgaagccggcgtcgcggtggaagacgtggaaatgcgcaaggccgatctggaagacgtgttcatcgacctgatggcgggcgagcagacgccgttggaggtctcgcgatgatggcggttactggttggcgcgcgctgctctacaaggaaacgctgcgcttctggaaggtcggcttccagaccgtcggtgcgccggtgctcaccgcgctgctgtatttgatggtgttcggccacgtgctcgaagaccacgtgaaggtctacggttcggtcggctacaccgccttcctcgtgccgggcctggtgatgatgagcgtgctgcagaacgcctttgccaacagctcttcgtcgatcatccagagcaagatcatgggcaatctggtgttcgtgctgctcacgccgctgtcgcactggggctggttcttcgcctatgtgggctcgtcggtcattcgcgggctggccgtggggctcggcgtgttcctggtcaccatgttctttgcgatgccgagcttcgttgcaccgctctggatcctcgtgttcgcgctgctgggctccgcaatgctgggcacgctggggctcatcgcaggcctgtgggccgagaaattcgaccagatggcggtgttccagaacttcctgatcatgcccatgacctttctctcgggcgttttctattcgatcggatcgctccccccgttctggcagggcgtgagccacctgaacccgttcttctacatgatcgacggctttcgctacggcttctttggcgtgagcgacgcctcgccctggctcagcctgggcatcgtcggcgccgcctggctggccgtgagcgccatcgccgtccatttgctgagaatcggctacaaaatcagaggctgaaaggccctttcaaatcccatgaccgccgaagaactccaggccttgatccagtcccacctcccgtgcgagcacatctcgctggagggtgacggccgacactggtacgccaccatcgtctcggccgaattcgagggcaagcgcgccattcagcgccaccagcgggtctacgccaccctgggtgcgaaaatgcataccgacgaggtgcatgcgctctcgatgaaaacctacacccccgccgaatgggcggcgatcgacaagtaagtaactggcggccgaagcggccctaaattcgctggattcctgatggacaaacttctgattcgcggcgggcgccggcttcgcggcgaggtactcatttccggcgccaagaatgccgcgctgcctgagctgtgcgccgcgctgctcaccgaccagcccgtgacgctgcacaacgtcccccgcctgcaggacgtgtcgaccatgctcaagctggtgcgcaacatgggcgtgaccgccgagcgcgaccacaacggcacggtgcaactcaatgcgggcgacctcagcaaccccgaggcgccctacgagctggtgaagaccatgcgcgcttcggtgctggcgctgggcccgctgctggcgcgcttcggccatgccaaggtgtcgctgccgggcggctgtgccatcggctcgcggccggtcgaccagcacatcaagggcttgcaggccatgggtgccgagatcgcggtcgagcacggctacatgatcgccagcctgccggcgggccgcactcgcctgaagggcgcgcgcatcctgaccgacatggtcaccgtcaccggcaccgagaacttcctgatggccgccgcgctggccgagggcgagacgctgctcgaaaacgccgcgcaggagcccgagatcgtcgacctggccgaaatgctgatccgcatgggcgcgaagatcgaaggccacggcaccagccacatccgcgtgcagggcgtcgaaaaattgcacggctgcgagcacgccgtggtggccgaccgcatcgaggccggcactttcctttgcgccgttgcggccacgggcggcgaggtgttcctgcgccacgcacgagccgaccacatggacgcggtgatcgacaagctgcgtgaagccggctgcacggtgacgccggaagagggcggcgtgcgcatcagctccaaggccccggcctgcgagcacctcaaggcgcagagcttcagcaccaccgaataccctggcttcccgaccgacatgcaggcccagttcatggcgctgaacgtgatcgcgcgcggggcctccatggtgaccgaaaccatcttcgagaaccgcttcatgcacgtgaacgagatggtgcgcctgggtgccacgatccatgtcgagggcaaggtggcgatggtcgagggtgtccagcagctgtcgggcgccaccgtgatggccaccgacctgcgcgcctccgccagcctcgtcattgccgggctcgtggccgacggcgagacgctggtcgaccgcatctaccacctggatcgcggctacgaccgcatggaagccaagctgcgcggcctgggcgccgacatcgaacgggtttcgggaaccgccgcatgatcacattggcatcacaggagtcgcaatcgtgatcacgcttgctctgtccaaaggccgcatcttcgaagagacgatgcccctgctggccgcggccggcatcgaggtcaccgaagaccccgaaaaatcgcgcaagctgattctcgcgaccacgcggcccgacgtgcgcgtggtgctggtgcgcgcctccgacgtgcccacctatgtgcagtatggcggcgccgacctcggcgtgaccggctccgacgtgctgctcgagcacggcaaccagggcctgtaccagccgctcgacctgcgcattgcggcctgccgcctcagcgtggccgtgcgcgccgactacgactacgcgtcggccgtgaagcagggctcgcgcctccgggtcgcgaccaagtacgtgggcctggcgcgtgaatttttcgcgagcaagggcgtgcacgtcgacctgatcaagctctacggcagcatggagctcgcgccgcttaccggccttgccgatgccatcgtcgacctggtctcgaccggcaacacgctcagggccaaccatctggtcgaggtcgaacgcatcatggacatcagcgcccgtctggtcgtcaaccaggccgcgctcaagctcaagcgcgagccgatccgccgcatcatcgacgccttcgcctccgccattcccgcggcagccacgccctgagttcttcaccgcagcgccatgacactgaaagcagcacccatccgcctctccacggcttcagccggcttcgacgctgaattcaaggcgcggctgcattggtccgctgatgcggatgcggccatcgagaaggtggtggccgacatcctggccgatgtgcagaagcgcggcgacgatgcggtgctggagtacaccaaccgcttcgacaagctcgatgcgaagacactgccggaactggagctgacgcaggccgaactcaaggccgcgttcgattcgctgcctgccgcgcagcgcgatgcgctcgaatctgcggcccgccgtgtgcgcagctatcacgaagcccagaagaaggcgagcggcgagagctggagctaccgcgatgccgacggcacgctgctcggccagaaggtcacgccgctcgatcgtgtcggcatctacgtgccgggcggcaaggcggcctatccgtcgagcgtgctgatgaacgcgatcccggcgcacgtcgcgggcgtcggcgagatcgtcatggtcgtgcccacgcccaaaggggaaaagaacccgctcgtgctcgcagccgcctacgtggccggcgtcacccgcgccttcaccatcggcggcgcgcaggccgtggccgcactggcctacggcaccgccaccgtcccggcagtggacaagatcacaggccccggcaacgcctacgtcgccgccgccaagcgccgcgtgttcggcaccgtgggcatcgacatgatcgcgggcccgagcgaaatcctcgtcctggccgatggcaccacgccgcccgattgggtggcgatggacctgttcagccaggccgagcacgacgagctcgcgcagagcatcctgctgtgccccgacgcggcctatatcgatcgcgtgcaggccgaaatcgatcgcctgctgcccaccatgccgcgcgccgaaatcatcgcggcctcgctcaatggccgtggcgcgttgatccacacgaagagcatggaagaggcctgcgagatcagcaaccgcatcgcgcctgagcacctcgaagtgagcagcagtgagccgcagcgttgggagcccttgctgcgccatgccggcgcgatctttcttggtgcctttaccagcgaaagccttggcgattactgcgctgggccgaatcacgtgctgccgaccagcggcacggcgcgcttctcgagcccgctgggcgtctacgatttccagaagcgttcgagcctgatcgaagtgagcgaagccggcgcacaggtactaggccccatcgcggtgacgcttgccgaaggcgagggcctgcaggcgcacgccgaagccgcgcgaatgcgcttgcataagatctgagactttacaaaaaccgcttcggggaggagccagccagatgattcaccgtctatacagcaggtcgcgttttttcagattcgccgcaggcctcgttgcaggcgcagccttgctcgccgcttgcagccagatgccgcaggcgccgcgcaacgagtcggccgccttgtccgcaacgcccagcgtcgccgccgccgccgccgcgcccgcaccggcacagctcggcacccagtggggcgagggcatcgagtcgaagacccgcgcggtcagcgccaagcggctgtccgcgcagcctgacgaagtggcctcgctgggctacaacgacgcggccagcgtgcgtcgcgacgcgggccacaatcccgagcgccggctcaacctgctgctggcccagggcgatgtcgaatggtcggtgctcgacgagaccgaccgccccctgccgatgcagcgcgcgcgccgcagcgccgacatgttccgcctcgccggcatcgaaggcgcgcgctacacgctgcgctttcgcaatctcagcgaccgaagctacgaagtgatcgccacggtcgacggcctcgacgtgctgaatggcaagcccggcagcctgcgcaatggcggctatgtgttgcgtccgcagcaggtgctcgacatcgaaggcttccgcaagagccagagcgaggtcgctgccttccgcttcgccgcaccgggccgtgcctatgcggcgaacaccgaagccggcgacgtgcgcaacatcggcgtgatcggcgccgcattgttcgagctcgagcagcccgaggcgccacgccgcccgcgccgcgacgccacgccgccgcagcccagcgcctttccggccgacgcctcgtacgcgccgccgccgcgctatcgcaagtgacgccatgagccgtgctgccgtcctgctgctgctgccgcgcctgccggtgctgttgttcgcactggcggccggtgccggtgcgcaggcgatgagcatccgcgaactgcggctgctcgaagccaacgagaaggacggcaaggcgtacgcgagctactacctcgtcggcgtgctcgagggcttgcgcgaaggcgtggaagcatcgcagcgcaacggccagaagccgatcttctgcgtcgaaggccgccgcatcgagccatcgatggcgcgctccctttatcaaaccgagctgacgcgcaacgccgacagctatgaagccgacatgcccgtgcaactggtcatgtccggcgcccttaaaaacagcttccgctgcacccgatgacaacttcttccaccgtccgcccgatcgatcgcatccgctccgatgtgcagtccatgcatgcctatgcggtgcaggacgcacgcggcttcgtcaagctcgacgccatggagaacccgttcggcctgccgcccgcgttgcaggccgagctgggcgcccggctcggcgcgctggcgctcaaccgctatcccggtgagcggggcagcgatctgaagcgcgcactggccgcgcacgcgcacatgcccgaaggctttgcgctgatgctgggcaacggctccgacgagctcatctcgctcctggccattgcctgcgacgtgcccggcgccacggttcttgcgcccgtgcccggtttcgtgatgtacgccatgagcgccaagctgcagggcctgcgcttcgttggcgtgccgctcacggccgactttgaactcgacgaagccgccatgctcgccgccatcgcgcgggagaagccggccatcgtgtatctggcctatccgaacaatcccaccgccaacctctgggacgacgccgcggtcgaaaagatcgtgcaggcccagggcgagcagggcggcctggtggtgatcgacgaggcctaccagcccttcgccgccaagagctatatcgaccgcatcgcacggcacggccatgtgctcctgatgcgcacgctcagcaagttgggcctggccggcatccgccttggctacctcatgggcccggccgcgctgatcgccgagatcgacaaggtccgcccgccctacaacgtcagcgtgctcaactgcgaatgcgcgctcttcgcgctcgagcacgccgaggtgttcgaagcccaggcgaggcagatccgcgaggagcgccatcgcctcatgatgggactgggccgcctttcgggcgtcaaggtgtggccgagcgacgccaacatgatcctcgtgcgcgttccggatgccgccaagaccttcgagggcatgaaggcccgcggcatactggtgaagaacgtttctaaaatgcacgaactgctggcaaattgcctgcgcctcaccgtcggaacggccgacgagaatgcgcggatgttcgcggcactcgaagcctcactatgaccaccccccaaacagccgacacgggcaccgctgcgcgcaccgcatcggtcacgcgcaacaccgccgaaacgaagatcaccgtcagcgtcaacctcgacggcacgggccgcgccaggctctccaccggcatcggctttttcgaccacatgctcgaccagatcgcccgccacgggctgatcgatctcgagatcgattgccagggcgacctgcacatcgacggccaccacaccgtggaagacgtgggcatcactctcggccaggcggttgccaaggccgtgggcgacaagaagggcatctgccgctacgggcatgcctacgtgccgctcgacgaggcgctgagccgcgtcgtcatcgatttctcgggccgcccgggcctggagatgcacgtgcctttcacgagcggcatgatcggcaccttcgacagccagctcacctacgaattcttccagggctttgccaaccacgcattcgtcacgctgcacatcgacaacctcaagggcgtcaatgcgcaccaccagtgcgaaacggtgttcaaggcttttgcacgcgcgctgcgcggcgcgctcgaactcgacccacgctccgtgggcgtcattccctcgaccaagggttcgctctgaattcctccagcgaacagctatgaaatctgtagcaaataccgtcgcggtcgtcgactacggcatgggcaatctccgctccgtttcgcaggcggtgcagcacgcggccgaccaggtgggcgtgcaggtcttcgtcacgtcggacccagaggtggtgcgcaaggccacgcgcgtggtgctgccggggcagggcgccatgcctgactgcatgcgcgaactgcgcgactccggcttgcaggagtcggttctcgaggccgcggcgaacaagccgctcttcggcgtgtgcgttggcatgcagatgctgctctcccgcagcgacgagggccccaccgacggcctgggcctcattccgggcgaggtcgtcaagttcgaactggccggccggctgcagcccgatggcagccgcttcaaggtgccccagatgggctggaaccaggtgcgccaggcccagccgcatgccgtgtgggcgggcgtgccggacatgagctatttctatttcgttcacagcttctatgcgcggccggccgacgcccggcacagtgtgggcgaggcagattacggtgcgcgctttaccgcagccatcgcacgcgataacatttttgccacccagttccacccggagaagagtgcggaccatgggttgcagctctaccgaaatttcctccactggaatccctgaacttatattcccgcccgggccgacccttcctcagcccggattccgcacactcgcgtcacttccatgctcctcattcccgccattgatctcaaagacggccactgcgttcgcctcaaacagggcgacatggaccagtccaccatcttcagcgaagaccccgccgccatggcccgcaagtgggtcgaggcgggggcgcggcggctccatctggtcgatctgaatggcgcgttcgccggcaagccgcagaaccacgcggccatcaaggcaatattgcgcgaggtgggcgacgacattccggtgcagctgggcggcggcatccgcgacctcgacaccatcgagcgctacattgacgacggcctgcgctacgtgatcatcggcactgccgcggtcaagaatcccggcttcctgaaagacgcctgcgtggccttcggcggccacatcatcgtgggcctcgacgccagggacggcaaggtggccaccgacggctggagcaagctcacgggccacgaagtggccgacctgggcaagaagttcgaggactacggcgtcgaatcgatcatctacaccgacatcggccgcgacggcatgctgtcgggcatcaacatcgatgccaccgtcaagctcgcgcaggcgctgaccattccggtcatcgcctcgggcggcctgtcgaacatggccgacatcgaccagctttgcgccgtcgagcccgaaggcgtcgaaggcgtgatctgcggccgcgccatctattcgggcgacctcgatttcgccgccgcgcaggcccgcgccgacgaactcgccggcgcctgacgccttcccacagcagcagcgcgtgctttccgcgctcgccattgccaattaccgctcgctgcgccagctgacggtgccgctcggtcggctcacggtggtgaccgggcccaacggcagcggcaaatccagcgtctaccgcgcgatgcgcctgttggccgatatcgccaatggtggcgtgatccgctcactggtgcgcgagggcgggctttcctccaccctctgggccgggcccgagcgcttttcagccgccatgctgcgcggcgaggtgccggtgcaggggacgagacgcaacgaccccgtcgccctgaagcttgggttcgccagcagcgaatccgacgaattcggctacgccatcgacatcggcttgcccccgccgcccccgcctccgccgcccactcccacagctttctcgcacgatcccgagatcaagcgcgaggtgatctggagcggcccggtgctgcggcctgccgcgcagctggtcgaccgcaggggcgcggcgcttcgtctgcgcgaaggcaagagctggcaggccgtcggccgccccatccccgccttcgccagcatgatgaccgagtacgccgatccgcacaccgcgcccgagatgctcacgctgcgcgaacagatgcgctcctggcgcttctacgaccacttccgctccgacgccgatgcgcccgcgcgccagccgcagctcggcacctacacgccagtgctcgccaacgacggcgccgaccttgccgccgcactgcagaccattcgagagatcggcgacggcgaggcgctcgatcgtgccgtggacgatgcctttccgggcgcccgcatcgaagtgtgcgtggccgaagcccggttcgagacgctgatgcaccagcacggcctgctgcgcccgctgacggccgcagagctttcggatggcacgctgcgctacctgctctggattgccgcgctgctgacgccgcgaccgcctgcgctgctggttctcaacgaacccgagaccagcctgcacccggacctgctgcctgcgctcggccgcctcatcgcccgagctgcacgcgaatcgcaggtgatcgtggtgtcgcatgccgcgcgcttgatcgccgcgttggacgacagcgaaggcctgcgacaagtggtgcttgaaaagcagttcggcgagacccgcatcgcgaatctggacatgggcgaaatcccgcgctgggagtggccaacgcggtagcgggaaagcgaaggcctactcggccttcaccgccatcgtctggatgatcgcttccagctgcgcgctcatcggcaggttgatgctctctccggtgggcagcttgcgcaggaaccagcgcttgtactggcgctcgacctcgccgtcctcggccagcacctggaaggtgtcgttgatcaccttgcgaagctgtgcatcccccttgcggtacatgatcccgtaggggtcgtaggagagatagtcgccgaccacttcgtactccgccttggcggcgtcccgcgcgatcaggccgtagagcagcacgtcgtcggtggcgaaggcgtcggcctggccgctcttcacgagcccgaaggaatcagcgtggtcgcgcgccaccagcaggttgatgccgagcttgaacttctgcgaaagctcgcgcagcgtcttctcgttggtggtgccggcggtcaccgccacccgcttgccggccaggtcgcggaacgacttgatcggcgaacccttcttcaccagcaccttggtgcccgagacgaagatcgtgggcgaaaaactcacgcgcttctgccgctcgagattgttggtggtcgagccgcattcgagatcgaccgcgccgctctcgaccgcatcgatgcgcgaatcggaagtcacgggtgcccacttgatcgtgaggctcttgttcaccgcgtcttcgatggccgtgaccagcgcgcggcaaagttcgatcgagtagccgatgggttccttgcgcgcgttgagaaaggaaaacggcaccgacgattcgcggtagccgatggtgatggcgccggtctcccgcaccttggcgagggtgccggtcaatgtctcgggggcctgcggctgtgccagcgcaggcacagcggaaaccagcgcagcggctgccagcaggccggccaggaaaaccgacagcatggccttgggcttcacggttggcctcacgcgtgcgctggatgggccagggtggccgcagcctcggcgtccagcgccttggcattgaccgccgcgtcgctttcggagagcaactggccctcccacttggcaaccacggccgtggcgatggagttgcccaccgcattggtggccgatcggcccatgtccaggaaggtgtcgacgcccaggatcagcagcaggccggcctcgggaatgtcgaagtggttgagcgtggcggcaatcaccaccagcgacgccctcggcacgccggccatgcccttggaggtgagcatcaggatcagcagcatcgtgatctgcgtgctgagcggcatgtggatgttgtaggcctgcgcgatgaacagcacggcaaaggtgcagtacatcatcgagccgtcgaggttgaacgagtagcccatcggcatcacgaagctcgagatcttgcgctttacgccgaagcggtcgagcgcttgcaggatcttcggatacgccgcttcggagctggcggtggcaaacgaaagcaggaaggcttccttgatgagcgtcagcagcttgaacacgcgcggccccaggaacgaaaagcccgcgaagatcagcacgccccacagcacgaagaggcccaggtagaagtcgcccatgaaaacggcgaacttgagcaggatgcccaggccgttgaccgcaaccgtggcggccatggcggccatcactgccagcggggccagcttcatcacgtagccggtgatcttgagcatggcgtgcgagagctcgtcgatggcggacaccagggtcttggccttgtcgccgagcgaggcgagcgccacgccgaagaacatcgagaacacaacgatctgcaggatctcgttgttggccatggcctcggcaaaagacttgggcaccaggtggctcacgaagtccttgagcgtgaacttcgcggtggcgaggtttgccgaagagccgatgtccggcagcggaagcccgaggttctcgccgggcttcaggaggttggccatcaccaggccgatgagcagcgaaatcagcgaagcggtaaagaaccagccgagcgacttgccgaacacgcggcccaccgatttggcatcacccatgtgcgcgatgcccaccaccagggtggagaacaccagcgggccgatcagcatcttgatgaggcgcaggaatacatccgaaatgatcgacacgtagcccgcgatctgagcggccgccttcttgtcgggaaagctcgtgaagatcatgtagccgacaagaatgccgagcatcatggcaatcaggatccaggccgcggcgggcagtttctttctcatgtttgtccctttgacgtatgtgtggttccggggcgcgggcgcatcggccggcagcctcttcttgtgcggcaggcgaagggtatccaagaaggtcccttgcgtgcaaccggcgcgggcgcattggcgatgaagccttaagtgtccaatgccaattccgtgccacgcgatttcgctgcctacaattctccgatggatatcagctcgatcgagttttgcggacagcccgcgcttcgtgccgccgggaccgatggcagtgctttcatcgtgtcgctgcacggggcgcagctgctttcctggaccacggcggacagggtggaacgcctctatctgagcccgcgcgcggtgttcgacgggcaggctgcgatacgcggcggcgtgcccatttgctgcccccagttcaaccagcgaggcatgctgcccaagcatggattcatgcgcaatctgccttgggaaaaccggggtgccgacgccgcttcgggcgaactggtcttgcggctgcgcgacaacccggccactcgcaagctgtggccgcactctttcgaggcgcgcctgcagatcggcatgggcccgggacggctgcgcaccacgctggcgctgctcaatgtggaccatgcacccttcagctttgccgcggcgctgcacacctacctgcgcgtcgacgatattgcccaagtgcggctggaaggcctccagggtgccaaccgctgggattccctgcgcgacgaccgccacgtggagacggcgccggcgctgtgcttcgatgccgagttcgacagcgtctatgccgctcccgcgaagccgatgcggctggtgcagccgagcggcacgctcgagatcacgcaaagtgcgagctgcagcgaaaccgtggtgtggaaccccggcgcggtgctcggtgcgaaactcgccgacatgcccgaagatgggtatcggcacatgttgtgcgtcgaggccgcgcgcatcgacgagcaggtgctgctcctgccgggcgcgcaatggcagggctggcagcagctccgcgtcctctgaatgaacttttccttacgaccgaccatgctcgcaaaacgcatcattccctgtctcgacgtcaccggcggccgcgtcgtcaagggcgtcaattttctcgagctgcgagatgccggcgacccggttgaaattgccgcgcgttacaacgcgcagggcgccgacgagctcacctttctcgacatcacggccaccagcgacggacgcgacctgatcctgccgatcatcgaggcggtggcgtcccaggtcttcattccgttgacggtgggcgggggcgtgcgcaccgtggccgacgtgcgccggctgctcaatgcgggcgccgacaagaccagcttcaactccgcggccatcgccgatccgcaggtgatcaacgacgcatcgcagaaatacggttcgcaatgcatcgtggtggccatcgacgccaagcgccgcagccccgaagaagccgccacgcgcggcgcagggtgggacgtgtacagccatggcggccgcaagaacaccggcctggacgccgtcgaatgggcgaccgagatggtgcgccgcggcgccggcgaaatcctgctcacgagcatggaccgcgacggcaccaagagcggcttcgacctggcgctcacccgcgcggtgagcgatgccgtcaacgtgccggtgatcgcctcgggcggcgtcggcagcctcgacgacctggccgacggcatccagacgggcggcgcagatgcggtgctggccgccagcatcttccactacggcgaacacacggtcggcgaagcgaaagcccgcatggccgcgcggggaattccggtgcgaatcgagtcctgaggggtctttgcctatccccgacaatatcgcgatgaattggctcgatgaagtgaagtgggacgcgaacggcctggtgcccgtgatcgcgcaggagcagggcagcaacgacgtcctgatgtttgcctggatgaaccgcgaggcgctcgaaaagaccgccgagctgggccgcgccgtgtatttcagccgctcgcgcagcaagctctggttcaagggcgaggaatcgggccacgtgcagacggtgcacgagatccgcctggactgcgacaacgacgtcgtgctgctcaaggtcacgcaactcggccacgagcccggcattgcgtgccacaccggccgccacagttgctttttcagcaaatacgagaacggccaatggaccgcggtcgagccggtcttgaaagacccggagtcgatctacaaatgacggccacagtgaacacctcggacgcccttgcacgccttgccgcggtcatcgaaagccgtctgcccgcgcgcggcggcgactccgagaagagctacgtggcgcgcctgctgcacaagggccccgatgccttcctcaagaaaatcggcgaggaagccaccgaagtggtgatggccgccaaggacgccgaccatggcggcgaccgcacgaaaatagtgaacgaagtggccgatctgtggttccacaccatggtggcgctcgcccactacggcctctcgcccgcagaggtgattgcggagctcgagcgccgcgagggcaccagcggcatcgaggaaaaagccctgcgaaaggcagaggcccgcgaggcatccaacgattgaaaggacatccaatggccaacgacatcgtgaacgtggaacccgacgactccctcaagacctggggctgggtcagttatatcctgcacctgatcgtggccatcggcgccgtcctgcccggagcgcaggcttccgtggtccttttgctcgtcgccctggtgatcgacttcatcaagcgcgacgatgccgccgggacctggcaggccacgcacttcagctggcgcatccggtcggtgctgtgggccggcctgctgtacatcatcacttcgtggctctggctgctgtttctcgtgccgggctggattgcctggagcctgatttcgctgtggtttctctaccggatcgtgaagggcatgatccgcatgaaagacaaccgccccatggaacccaaagatgtcatctgatccgaactgcgtcttctgcaaaatcatcgaaggcaagatcccctcgcgcaaggtctacgaagacgacgaactgtttggttttcacgacatcgcgccctgggcgccggtgcatttcatgctggtgcccaagcggcacatcgcctccatggcgcagctcacccccgaagacgccgcgctgatgggcaagatcatgacgctggcgcccaagctcgcgctggagctgggctgcaggccctatccggagggcggctaccgtgtgctggtcaacaccggcgccgagggcgggcaggaagttcaccatctccatgtccatgtcatgggcggtcccaggccctggcttcgcggctgaacattaggccaaactgtcacattccgcccgactaaaatcggacacattcttaggagtcttccatgggttcattttcaatctggcactggctgatcgtgctgctcgtcgtggtcatgatcttcggcaccaagaagctgcggaacatgggttccgaccttggtggcgccgtgaagggcttcaaggacggcgtgaaggacggcggcaccaccgccgatgcgcctgccgcttcgtcggcccctgctgcccaggttaccggtcagccggccaacagcgacaagtcggcgatcgacgtcgaagcgcgtcagaagtcctgagcgcgggtcataagtgctcgaccttggcattgagaagctggcgctgatcggcgtcgtggcgttgatcgtgatcggaccggaaaagctgcctcgcgtggcgcgtacggtcggcaccctgctgggcaaggcgcagcgctacgtgaacgacgtcaaggccgaagtcaatcgctccatggagctggacgaactgcgcaagatgaagagcaccgtggaggatgcggcgcgcgacgtcgagcacagcatccagaccggcgcaagcgatctcgagaagcagttttccggctcgggcgaaacgctttcggccctggccgaacccgagccctcggtgccggagtaccggcatccccgcaagaactggcgcctgaagcagggcgccacgccgcagtggtacaaggcgcgcaacggcgtgcgcaccaaggcgttgtcgggtgccgcgcgggttgcgcgtttccgcccccacaagatcaactagcggctttcccactccccgcgttcctcgtgcgccgcacgccggccgaagccacgctttctcctgctctttttctctcccaatggccgattccgacaacaagaacaaagacgcagaagacgagttggcgggcaccgaacaaccgttcgtccagcatctggtcgagctccgcgaccggcttctctattgcgtctacggcttggtggccgcgggcgtgctgctggccatctggcccgggccgagcgggctgatcgaccttatcgccatgccgatccaggcccacatgccgccgggcgccaagctcatcgcggtgggcgtgttctcgcccttcttcgtgccgctgaaggtgctgggtatgacggccgtgctgctggcgctgccttggctcatgtaccaaatctggatgttcgtggcgccggggctctatagccatgaaaagagattcgcgctaccgctaatcttgttcggcagcttgctggcctatgtcggcatcgcctttgtgcagttcttcgtgctcgacaagatgttcggcttcattcagaaattcacgcctccgagcgtgagtgccacgcctgacatctcgtcgtacgtggaggccatcttgtcgctctacatcgcgttcggcgtggcgttccaggtgccgatcgtcgtgatgttgctggtgaagttcgagatggtgacagtcgaaaagctgcgctcgttccgcggctacttcatcgtggtggccttcatcatcgccgcggtgctcacgccgcccgacgtggtgtcgcagctcgcgctggcgattccgatgtgcctgctctacgaggtcggaatcatcggcgcccgctacttcacaggcggcaagaagacggaagaggaagaaagcgccgattcatcggcctcttcctgatcggtcattctggctggttgggcatctgccgcaccgggctcctgggccgaaggcccggcgtcacgtccagctccatcttgtcggtgccgcgctgcagcgcgaagcgggcggtgctgccgggcttcaggccggccacggcggtcagcagggcctgcacgttgtcggtctttttctcgccgaccgaggtgatcacgtcgcccgggcggatgccggccttggcggcagggccgttctgcagcacgccggtaatgatgaccccggcattcgccttcacgccgaaggtctcggccagctccggcgagagctcgttcggctccacgccgatccatccgcggcgcacctggccctctttcacgatgccttcgagcacgatcttggccatggaaaccggaatcgcgaaaccgatgcccatgctgccgcccgagcgggagtagatggccgtattgatgccctgcaggttgccattgacgtcgatcagcgcaccgcccgaattgccggggttgatggccgcgtcagtctggatgaagttctcgaaattgttgatgccgagctggttgcgccccagcgccgagacgatgccgctggtgaccgtctggcccacgccgaaggggttgccgatggccagcacctggtcgcctacctggagctcgtccgaattgcccagcacgatcgcgggcagcttatccatttcgatcttgagcacggccaggtcggtgtccggatcggtgccgatcaccttgccgcgcgtgtggcggctgtcgttgagcgtgacctcgatttcgtcagcgccttcgaccacgtggttgttggtgagcacgtagccctcggcgctcacgatcacgccgctgcccaggccgacctggggctggtcgccctggtcgccgaagaagaaccggaaccacgggtcgttgctgcgcggatggcgctgcgcggccttgctggtgttgatgctcaccacggccggcgacgctttcttggccgccgcgctcaggctgccggggaccggtacggacgaggcgccggccggtgcctcgacgatcgacaccacgccgcccagtgaggtggagcgccgattgatccattcgggcttgagtgttgcaacgacgaagtaggccgccaggaggacggtcacggcttgggcaaagagcagccaggtgcgtttcatgaaactttgattgaacgaagaggacacgccgcccacgcggcgccacggcccattgtccctcaacccccaattgcataaaccgcgcgctgcggtcgagattggcaaagccgtcagcaccaataagggataacccttagcatcgctgtgcgagcccacacggctccgagctccggccttccgcatcgcctacccggctcacgcggcgaggtgtttcgccggcgcgccgccttccgcatggatccttctgcggccggcgtgcggcaacgaccttcctgccagccatgacttctcacgcaatttccccggacggtgcccagccggcgccggcccgcacgctcgatgcgcgcgactacaagacactgggcctctccgcccttggcggaacgctggagttctacgacttcgtcatctacgtgttctttgccaccgtgctgggcgcacttttctttcccgccgacatgcccgactggctgcggcagctccagaccttcggcatctttgccgccggctacctggcccggccgttgggcggcatcgtcattgcgcattttggcgacctgctcgggcgcaagcgcatgttcacgctgtcgatcttcctgatggcggcacccacgctggtcatcggcctcttgcccacctacgccagcatcggcattgcggcgccgctcctgctgctggccatgcgcgtgctgcagggcgcggccatcggcggcgaaatgcccggcgcgtgggtgttcgtcggcgagcacgtgcccgcgcagcgctacggtttcggcatcggcgcgctgacttcgggcatcaccggcggcatcctgctgggatcgctggtggccgtggccatcaaccgccactattcgccggcggaggtgagcggttttgcctggcgcattcccttcgtgctgggcggcgtgttcggcctcgtctcggtgtacctgcgccgcttcctgcacgagacgccggtcttcagggagctggcgggccgcaaggccgtggcgcgcgagctgccgctgcgcaccgtgctgcgcgagcatcgcgcggccagcgtctacgtggcgctgctgacctgggtgctgtcggccgccatcgtggtggtggtgctgtacacgcccacctacctgcagaaggtgcaccacattccggcggccctggcgctggaagccaatgccctcgccacgctgaccctgaccatcggctgcgtgctggtcggctgggccagcgaccgcatcggcacgcgcgcggtgatgctcatcggctggggcgggttgttcgcgacggcctatctcttctacacggggctgcccggcacgccggccacgctgttctggcactacggcctggtgggcttgttcgtgggcaccatcgccaccgtgccgatcgccggcgtgcgcgcgttcccggcgccggtgcgcttcaccgggctctcgtttgcctacaacatgtcgtatgccgtgttcggcggcctcacgcccgtcatcctcacgctctggctgcagcacgacacgatggcgccggcgcattacgtcgccgtgctggcggggctgggattcctgctggccctgtggccactcgcggcacgcggccatgccatgcgcaacgcagacgggagcgcgacaatgtcgcgatgagcaccacccgccatgaattgctgcatgccttcgacctgcttcttgcgccctcgcgcttcaaggactacggaccgaacggcctgcaggtcgagggccgcaccgtggtgcggaagatcgtttccggcgttaccgcgagccgcgcgctgatcgaagccgccattcatgccgaggccgatgccatcttcgtccaccatggcctgttctggcgcggccaggacggctgcgtcaccggctggatgaagcagcgcctgggcttgctgctgggtgacgacgtcaacctgttcgcgtatcacctgccgctcgatgcgcaccccgaactcggcaacaacgcgcagctcgggctgcaactcgggttgctcgcgcatgccgggtcgaccgggcgcttcggcgaccaggagctcggttttcttggcgcgcgcgacaacggagaaagctttgccagcgccaaggaactggccgcccacgccgaaaaggttctgaagcggcccgtcaccctcgtggacacggcgcaccgcccactcaagaacatcgcatggtgcacgggcggcgcccaaggctatttcgaagccgccattgccgccggtgccgatgccttcatcaccggggagatctccgagccgcaggcccactatgcgcgcgagatgggcgtcgctttcctcgcgtgcgggcaccatgccaccgagcgctacggcgcccaggcggtggccgcgcacgtggcggcgcagctcgggctgaagcacgagttcatcgacatcgacaatcccgcatgaccggacaggctcccatcgctcccaccactcccgtcgccatcacgctcggcgatcccgcgggcatcgggccggaaatcattgccaaggccttccgcgaggcacccgacgccacccgcggcgccttcgtggccggcgacgtggccacgatgcgccgcgcatcgcaagccttggcgttgcccggacaaccggcctggccggtggccgaaatcgagcagatcgccgaagcggccgccgtgccgccgggctgcatccccgtgctgcaggtggtggcgccgcccaaggacatcgtgcccggccggatcagcgccgaagccggccgcgtggctggcaattgcgtggtctgggccgcacgggccgccttgcaaggcaagatcgccgccatcgtgaccgcgccgcttcacaaggaggcgctggccgcggcgggttttccgtatcccgggcataccgaactgctgcaggccgaagctgccgcgcatgcgggcctcgcggtggacggcatgccggtgcgcatgatgctggccaacgacgagttgcgcaccgtgctggtgagcatccacatgtcgctgcgcgacgccatcgccgcggtgagcttcgccggcgtgctggagacgctgcgcatcacccaccgtgccttgcaccgcgtgctcggacgggcgccgcgcatcggcgtggcgggcctcaatccgcatgcgggcgagggcggattgttcggttccgaagagcgcgacatcattgcgccggccatcgaggctgcgcgcgccgaaggcatcgacgccgatggcccccacgcgcccgacaccgtcttcatgcgcgcgcgggacaaggccggcgtgccgggaagcggcgaattcgacgtggtgatcgcgatgtatcacgaccagggcctgattccggtcaagtaccttggcgtggaaaagggggtgaacgtgacgctgggcctgccactggtgcgcaccagccccgatcacggcaccgcgttcgacattgcaggcaccggccgggccgatgcctcgagcctcgtcgaggccctgcgcatggccagaaagctgtcgggcggctgagaagacgcgttcagggccgcttcaggctgtcgcggatctcgcgcagcagggcgatgtcctcaggcggcgccaccggtgccgcgggcgcatccgcctggtgtttgcgcagcttgttgatctgcttgaccatcatgaagatgatgaaggccaggatgacgaagttgaccgcgatggtgatgaagttgccataggcgagcaccggcaccccggccttcttgaggtcgggcagagtgctgggcacgcccgccggcacgctgcccagcaccaggtagagattcgagaaatcgagcttgccgaacaccagaccgacgatcggcatgatgatgtcggccaccagggagtcgacgatcttcccgaaggccgcaccaatgatcacgcccacggcaagatcgatgacgttgcccttgacggcaaattccttgaactcgctgatgatgctcatgatcaatatgctccgggacgctggtgttgaactgccgccagtatgcctgcggattcgccagttcgaatcgtgaagccccttggtgggtaatgcaaaagaattcttttcttcgatgatcttctttaatggtgcctgatcgatcggcgccggcgcaccaataaaggcgcgcaatccctcttcaaataaatgaatagtttctggttaattgccaccggattcggtgacagcggctttctgttgcctgccgcatttggggttgcaatctggctcgcaatagatcggggcacacgcccggcggcggtgcattgggtgcttctatttggcgcttgcggtcttgtcgtgatgctttccaagctcgctttcatgggctggggaattggcagcgcccgctttgatttcactggcttcagcggacataccgcattggcgaccagcgtctggccggtcattttctggctcgtggcgctgcggcgcgcaccattggtgcgcatggctgccgcgatatcgggatgggtatgggccgtcttcatcggcgtgtcgagactggcgctcgaagttcactccccggccgaagtcgtcgccggtgccgcactcgggaccctggtgagcgcaggctttctgagactgcagtggcaccggcacctgcgggtgcgaacacctcgatggctcgcgctgggcttggtgctgccgctattgtttttgatcattgggcggccggcacccacgcagttcgtgctcgagaggatggcggtctggatggcgggcatcgagcgtccgttcatgcgcgccgacctgctgcaggcccgcgagcccgcccgcagcccggcctgagcaaacaactgtttacaaaagagcaaaccttttcgcaaagccgatcgggcccggcttttgtagtttcagcgccacaattcgccgatttgagctgttaattaatagttcacattttcaaatcgcaaggcgcggcttcgcttgtgcaatccaaggcttcgctcccaatgaaaaagggggctcagctattgatcttcgggataacccctagggccttggggttgatccgcaaatggacacattttttgcacctattgcacggaaagtgggtgccacggccgcagcgacaattcggcccagcccgtctgccgttcatgcgcaggcttgctttgacgaaccgtgacaaaaagggtgggcccaaataccaactgggctcgggccttgcatatgaaatcgcggttgccgaaaaccaatttgtgcaatggggatcaatttgacacgcttcgtgtacccgatggggtggggttttgccctaatgggcgcgttattgctgcagggctgcgcaccgggcttcagttctgtggctgcctatgaggcagaccagagcctgccgccggagttccagtacctgccagccgatggcgcgccggatggagtcatcacctccatttcgcccgcgctcatccgcgcgatggcggaggcgcagccggcctccgtttcgccggacgtgaagtcgctcttcggcgaagcgccggtctacaccatcggaccgagcgacgtggtgggcgtggtcgtctacgaccatccggaactgctgcccaacgcgggcgcggtgatctcgcagcaggccgacccgaccggcatcagcgtggcgcccggcttcatcgtcggtgcggacgggcagatctcctttccctacatcggccgcgtcaagctccaggggctgaccgaaatcgaggcctccgacctcattgcgcgccgcattgccgcgtacatcaaggatccgcaggtgacggtgcgcatccagtccttcagaagccgccgcgcattcgtcgaaggcgaggtccgcacccccgggctgcagatcttcaccgacgtgccgatgacgctcgcggaggccatcagccgcgcgggcggcatcaccgccagcggcgaccgctcgttcgtgaccttgacgcgcggcgacaagaccacgctgatcaacctgcccaacctccaggaactgggttccgatgccagccgtattccgctgcgcaacggcgaccggatccaggtgcggcaccgcgacgagagcaaggtgttcgtgatgggcgaaatcgcgcggccttcggcgctgctcatgcacaacgggcggctcagcctcaacgaggcgctgggcgaggcaggcggccccaacctgaattcggcccacacgggccagatcttcgtcatccgcaacaacgcgagaggcttgccggccatcttccacctgaacgccaagaatccggcggcactggccctggccgagcgctttccgctgcagccgcgcgacgtggtctacatcgattccgtgccgctcgtcacctggaaccgcctggccagcctgatcctgccggcggcccaggtcatcaatgcgggcgacgaagtctggagccgccacagatgaaatcgatcctgacagtctgcatcggcaacatctgccgaagcccgatggccgaaggcatcctggccgcgggcctgccgcatcttcgcgtggtgtccgctggaaccggcgccctcgtgggcaagccggccgatgccacggcgcagaagctcatgcaggcgcgcggcatcgacatttcgggccacgtcgcgcagcaggtcagccagatgctgtgccggcaggccgacctgatcctggtcatggacatggcccagcgccgctacctcgagtcgacctatcccttcgtgcgcggcaaggtctttcgcattgccgaggccgccaagcaggacgtgcccgatccctaccaggaggacgaggcggccttcgcgcacgccctgtcgctcatcgatgtgggcgcccgaacgtggatcgaccgcattctgaaaattacgaaacccgagcagcaaccgacatgaacgcaacccagcaagccgccctgccgatgccagcgctggaagaagagggcgaaaagttcagcctcgtcgagtacctggacatcctgatcgacaaccgctggctcattgccatcgtggttggcgtgatgctgttgctgggcgtggcctacgccttcttcggcaggcccatgtacgaaaccaacgtggccgtgcaggtcgaggactcgggcaattcggccggcagcttcctgggcgatgccgcatcgtcgctgctgagcgtgaagacgccggccgcgggtgaaatcgaaatcatcaagtcgcgcgccatcctcggccaggcggtggagaacaccaagctgtacatcagcgccgtgccccgctatgcgcccgtggtgggcagctggcttgcacggcgcgccaccgatctgtcggaccccggcttcatggggctttcgggctacgtcaccggggccgagaagatcatggttccccagttcgacgtgcccgcggatttcgaggcgaagccattcacgctgaccctggggccggacaaccgctacgagcttgccaaccccgagctcaaggccccgctcaagggcacggtgggaactccgctgctcgccaacctgccgagcggcaatctgcggctgctggtgagttcgatcagtgccaagcccggcgcgcagttccagctcgttcgctattcgaagcaactgacgctcctgacgctccaggacagcctcaaggtcgtcgaaaaaggcaagcagtcgggcgtgctcgacgtgggctggaagagcccgagtcctgaaaagctgacacagctcctcaacgaaatcgggcgcctctacgtgcgccagaacatcgagcgcaaggcggccgaggccgaaaaaaccctgggtttcctcgatacggctctgccccagttcaagaagcagctcgagcaatccgaggatctctacaaccgctacagaaacgagaacggcacggtcagcctggacgacgaggccaagaacgccctgacccagacggtcgacctgcagtccaagttgctcgaggcgcaacagaagcggcgcgaactctccgcgcgcttcaccgacaagcatccggccctccagacgctggatacgcagatctcggcctggaagggcgaaatcgcctcggtcgattcgcgcatccggaaaatgccgctgctgcagcagaacaccgtgcagatgcagcgcgacatcaaggtcaacaccgacctctacgtgtcgctgctcaacagctcgctgcagatgcggctggccaaggaaggcaaggtcggcaacgtgcgactgctcgacgaagccatcgttcccgaagaacccgtgtggccgaaaaggccgctgatcatcgcggtggcgctgctgctggggctgatggcgggcgcggccgccgccattgccaagaacgcgctcttcggcggcatccgcaatccgagcgagatcgaaatgcacacggggctcaacgtctacagcagcattccgctgagccccgcccagcggacgatcgacaagaacatcgaaaacagggcgcccggcacgcacatcctcgcgcttcagcattccgaggatcccgcggtggaaagcttgcgcagcctgcggaccgcgctgcagttcgccatgctggaagccgccaacaatcgcctgctcatttcgggcgcgacacccggggtcgggaaaacttttgtttctgtgaatttcgcggcgatcaccgccgcgtcaggaaaaaaggttcttctgatcgacgccgatttgcgcaagggccgggttaatcaattcttctccatgtcgcgatcgtccggcctgtcggaattgattgcgggcacgctgagctacgacaaagccgttcgcccgtcggtcttgcccaatctggacgtcatcacgaccgggatgcttccccccaatccagcggaattgctactgagcgattccttcacgcagatcctggaaaaactgtcgcccgattacgaccttgtgattatcgacaccgccccggtgctggtcgctgcggataccgcttcggtggcgccgctggcgggttctcttctcctcgttgcacgggcggaaaagacccaactcggcgaattgaacgagagcgtcaggagattggcgcacgcaggctgcactgccaatggcgtaattttgaatgctatggacttatctcggagacatgccggcagcagcagttataaatatggcggttaccgttacacacactataaatacaaaaacaacagggataccacctagtccaaaggcggtttctgagaaaattcattgaaattgtgatgattttcacgtgatgcactaattcggtgctgccgattaaatgctaataaaaaaggcctacgaccatatgcgtcattcttttgtattaggtatttcaatcgctccgccagcgcgctgatttccgcgctgcaactttcaaggccccacgctgcaaagcccttttgggcttggcatggagtcgacacgtgtcactgaacccgaaaggggcaagcgcttgcttgtaagacgaaaggtgctcctgcaatgagagttctcaaactatcaattcgctttcgttacaaatgtggaaacggggcgtacgtatgaccaatttctctcgcgaggagtcgatggcacctccaggcgaagcggtgggcggcgcaattgcggacgacctggcttggatcaaggttcgtcatccggccatactgcgtgccggaaaaagagcggtcgatatcagtgcatccctgttctttttctgcgtcttcggttggctctatgtgctgatcgccatcggtgtattcatcagttcgggcgcaccaatcttgtactcgcagccgcgcttcgggcgaggcgggcgggtgttcaagttctacaagttccgctcgatgctgccgaactcggcccagatcctcgaggaacacctcaggaacgaccccgtggcgcgccagcagtgggacgactatcaaaagctcgagaacgacccgcgcatcacccgcttcggcaggttcatccgcaagaccagtctggacgaactgccgcagttctggaacgtgctcgtgggcgacatgagcctggtcggcccccggccctgcatgctcgaccagaaaagcctgtatggcgcggactggtcgttctattgcgccgtgcggcccggaatcaccggcttgtggcaagtcagcggccgcaaccagctcagctacaagaagcgcgtggcactggatgtcacttacgtggagacgctctccgtcggcagggacatcggcatcttcatcaaaaccatctgggtggtggccgtcggccatggttcacggtgaaacccaggtcaacgatgaaaaagatcctgatctgcgcggtgcccttcagcgacaacctcggcgacggggtcattgccgcatccctggcccatattgccggcctgaagtatccgcaagcgaaggtcgagtttctggatattgccggccgcgtcggcttccaggaagaaaacctgcggggcggcggcgcattcgaggtttttgcaaaactgccgtcgctgctgcgttcgctgatcgtcttcttgtactgcctcaagggctattttctttcttggcgaaaaaactggaaggccgcggtcggcgacgccgatctgatcgtcattggcggcggacagctcttctgcgatgtggcgctcaattttccggccaagctgtttcttttgagcaggctgctgcgcggcaagcgcgtggtggtcgtttcggtcggcgtcacggccaaatggtcattctggggccgcttcctcgtcaagcgcttcatcaggaatgcaaggccggttttctacgcgactcgcgacaaggaatcggcaagcaacctgcacacccacttcagaattccgaggggcagcatacgggtcgttccagatccggcgcttgtttgcgccgatgcgttctcggaagagctctcgcccgaaaagaactgggatatcggaatttgcgtgagcagcctcgatgcgctggtcatgaactccgaatactcgaactccaattcaacggagtccgcgaggtttttttcgacgcttgccgaatcattgcaggcccaagggaagcgggtgctttatttcaccaatggcgcgtccgaagacaacaaggtattgagcgagatttcttcgggaaccggggccatgaaatcggggtttttcgttccccggcatcccgatgaactcgtttcactgatcagcgcctgttcctgcattgttgcccatcggctccatgcaaacatcgttgcctacagcttgaacattccatccataggaatgaactgggacaaaaaggtcgaatcgttcttcgaattgacgaagcgaaagcgctatctcttcgatttgtcgccccgcatcgaaaaaatcgaggcttcggtgctgagcgtgttgagcgaaaagaccccggaccgacaaacactggatttgctgagaggcgaagtggttgccggagttcatgccttgatctgatggagcgggccatgaaaatattgcacattgccgaaacactcaagggcgggctggaaacctatcttcggatggtctccggtttccagcagaactctccggtgatcagccaggcgaagttcattcttcccggccccgtggactggctgagctcgcaggacacccacgtggtccccacggcgcgcagtccgttggcccttgccacgtacgccgccgaagttcgcaagatcatccgcagggaacgtcccgcggtgcttcatctgcacagctcgattgcgggcggaatcgttcgggccatggcgctgctgggccaggtgccgcaagagacaaaaatcgtctattgctctcacggatgggcgttcgaccagatcgggccttcgtacaagaagtcgatctatcggtggatcgaatggctgctttcgtactggagcgacgccatcatctgcatcagccaccatgaactgcggattgcggagaagttcggcatcaagcgctgcacctgcattccgaacggaatcacccctgcgctggccacccaggaacaggtcgcccttcccaaggcttcttcgccgcaccccagaagaatcctgttcgtgggccggctggaccggcaaaaaggcatcgatgcactgctcgagtcctatgcgcgggttaggcccgacttcaagctgatcgtcgtcggcggcgccgttcgaaacgatctttctctcgcccattccgaagacatagagttcaagggatggctcgaaaaagacgagctcgacgctgcctacaggtcttgcgacgcgatcatcgttccctcgagatgggagggcttcggccttgtcgcggtcgaagccatggcgcggagcaagccggtgtttgcatcggcggtgggtgggctcgtcgatatcgtcgaagacacccggagcggacggctgtttccgctcgatcggctcgacgaaatgctgcgcgagatcgaccagatttccgaccaagacatggtgcggatgggccgggcagggcgggagattttcgaaaagaaatacaccgctgaccggatgaactccgccatcgtcgatttgtacagggagtcggtactctgatgaagttttcttccgttgttcccgtctcggagcgcctcgccggtctcttcaggttgctctgcgcttcggcggccattgctgttttttcgtgcgcggcccaggcccgggggatcagcgaactgagcaccgattacccgacggcgctgagcgtgcagatcgacccgagcgacatttcggatgaagacctgaacgaaatcagggcggcgggattcgagttcgtccgattcggcgtgcggccgcctttgaagagcgtcaaccccggacggatcgactactcgaaactgatccggcgcgtgcggaacgcgaggctcgacgccatcgtgacgctgttcggaggcagggagatctggggccacgaaccaggggagctcggcggcggccaacgggaaaagctgttcgcgaacttcgccgctgaattcatgaacgcccacatcgccgatgtggcgatgtgggaactgtggaacgagcccgactacaagacctttctgaacccggcgcttttctcgaacttcgaaaccgcgaccgcggagttttgcagcagcatcgcgcagctgaagaacccgccgaagatcgtcatggggttcggctttgcgaagcttcccttcaaccaggggcaggttccgccgcaactcgaaaatgccttcgtattgggggccaaggccaataattgcctgacggacatatcgatccacccctaccgctcgattccggaaacggccattgccgactacggaaagctgcgcgccaagctggaccagatgcaactcggcaaggtcggcatcgttgcctccgaatggggttacgcgtcgtacctgccggtcagggaccgcaacacgcaggcttcgctgatcttgcgtgaatacctgaccaacgtggccgccggcatcaagctcttgaacctctatgcctggaaggaccggggaacgtccgtcatttcgagagaagacaacttcggactcaagtcgaaggccggcgaaaagaaggaggcgttttcgagcctgaccgaattcctcaagatcgcccggacttcgaagaaggtttcgtacgacagcaacggaagcctgaacaagctggtgctgagccgtggaacgaccttgctgcacgtggtgtggacgcaaagctccgagcaggacgtgctgattcccgcagccaagggaaagaagtgcacgcgggtcgacttctttccgcaggtgcgccacggaacctgcggcagtccggtggaggggggcgttgctgccaaggcttcgagctatccggtcctgttctccattgcggactaggggatggcgtccggaattcgaaagcgcctcggaggtccgatctatgccgttgcagaccaatgcatctatagcgcaagccagctgctgctgagctttgcgctcgcacgggcgttgtcgccctcggatttcggtattgcgtcggcgttcctggcgatcgtcagtttccagtacatcctgcataccgcggtggttcatgagccgctgctgatcaagcgccattacgcaaatcggtccgccgcctggtggagctgggcgctcgtgcttgccgtctcgttggccggcttcctggcctggcagttcacgagcttcccggggccgctgcgctgggcgggcgtggcgctcatcgtgggctacgaaatattctggctctcccgcagcgtcttgctggtgggacgccgatacctggttctctgcatctccggcgtcctgatcagcatcggatacgtggcggtcttgatcgggttgaagccggccacgtggacgcaggcgctgctgtggatcgccgtgatccagctgccttttgccctcttgattgtgaggacgctgaaaagcgtgatcgccccgctgccggcacccgccgatgcccaggcgctgaccgtgaaggaagccgccagctatggctggaaggccagtctttcgcagctcatgagctggatcatgacgggaggtgcgatcctgctgctggggtcctcggcagattctgtgcaaggcggcctgctgaagatctacatcacgttcttgctgcccatgcagtacgtgctgctcgcgctgggctactacatcctgcccaagctggcggccagctggaattccgagggccgaagggacgctttccgtctcttcgtcaagttcgtgatcttcggcttcatggtggccgagctcggtggtgtgctgctgggcctgctcgggccctacctggtggtgctggcgttcggcaagaactacagcggcatggatttttcgccgttcttctacgcgcccgcgatcttcggcctcacgatgtgcctccgaacgggtttcagggcggctgcgcggcccggggctcttctgtggtgctcgattttcggcgcgctggtcttcgcggcgtgcatgctcgtggccaagccgcccatctcctacatccagaccatcaacgccatgacgattggctttgcctgcatggcggccatgatgatcggctggctgttcgtcatcatgcgcggccccagggtcgccgcgcaggtccgctgaccgttcttccagaggttccgctgcgggggtaggcgattgcgcccgattgcgcccgggcaaccgggcgcaatcgctcgccgatcaccgtgggcgttcgaaattcaggatgttgtcgcccgccttcgggctgccagtgtcgggcggctcgaacttgtaggcgctcgggtcgcgcgcggaagtcatttcgtagagcgggtggatccgggccagtcgcgcaccgccgtcgcgcaccaggggcgcccacgcgaaattggcggtgaacttgttcgagcgcggcagcagcgcgtcgaaggggatggaaagatagatgcccttgtcgaagctgccttcgccgaactgcctggccgacacattggtcttggtgacgtaggcgccaagcaccacgccgttgtcgaagcggcggctgatgtcgatggtgaccccgcgatcgcccgccaggtactggcccgcgctgaccttggccaggacgccgttccagccggtgtcccagtagagggttgcgtggccggtgttgaccttgtagtcgcgcaggccgaagtcctgttcgaagtcgcgttgccgcacgtggttgaagtcgacgccaatcgccatccggctgcgccacgggcgatagagccattccccgccgacgcccgcatacatgctttcgagtgcgccgccgtagacgctgtagtactggttgtccgtcagccggccgacgtgggtcagctgaagcaccggcatggtcagccgcttcgaggtgacgtactcgcgctgaaaggttcgcacgcggggcaggttgctgggcgccgtataggtgaacttgtcgaagttgtcgacgaggcgcaggttcagcgcgccgttgacccaggtgctcggcgtgaagcggtattccgcaaccgcctgcacgccgacctggaaaagcacgaaggagttggggccgccgagaatctggccgaggctgggcgtgaggccgatgctgaacttctgcaccgggcgctcccatggggccagcgccttgtcgtccgcggcctccttggccgtagccggagtgccggcgcccttcgcaacattgagggcgggtgcgtcggcgccgagcggcgggggcgcatagtcgcgctgggtcgccgcccgaagttcacttggcgcctgcgcctgatagtgcgctgtcacccactcgttccggtcgaccacttgcgcgtgcagcgccaggccccgttccgagtagtgaagaacaaaattcttgatcgaagcgggcgcatcgcgatgcagcacggcaatgatctgctcgacccgggcactccggtagacagtggcgctttcggtgatccacacgtgcagcatcgggccttgcggcgcaatgcgctgaacggcccaatcggtgcggctttcgatatcggccgcggtcgccgcccaacctggtgacgtggtggggggcgtcggcgaaaagcgcggcgccggagggtccgccgtcttgggcatctgcatcgtcgcgaggttggtctgcagcgtgaggccgaccatcaccttgtttccgcgctcgaagccggccgagaaagtcacgccgggggcgtagcggtactccaggccgatattgaagggcgagcgctgcggctgggcgttgttgagcggctcgttcttgtagtcgttgccttcgtactcgagcttgagcgtcaacgggtcccagggcgtgcgccattgcacgccgccaaagagcgcggcgggtccgcgaaagagccggccgaagttggcgccaccccatgtggtctcgctgacgcgggtcttgaaacggctgctcagcagattgaacggattaccgatgtttccgctgcttcccatgtagccccagccgatgccgaggctgaaatccaggtcgccgtggcgcttgctcgccaccaggtactcggacgaaaagaggccggtgccgccgatgtcgcgaaagcccagggccacttcaggaaggtaggccgactctttccacaaccgcgccttgaggtcgatgctcttgtccttgtagccctggttgctgaggccgatgccgtagatccggttgctgatggacgtgtagcggaaacccgcttccagccagtccagcggctggaacatcacgttcagccgcgtgtagggcgaaacatgcgtgagggacgtgcgcatgtcccccgcctggcccatgcgggccgtgggtgtctgcagcaagccggtttcgccccagtcgttgccgctggactggagcgcgcggtactgcggcgccgcctctgggcggaccgatatggcggtcggcgcgaaggcatcggccggtgccggtgccggggccacaggggcgggcgaggcctcggccgagggcgcggctggggcttctgccggagcggcaacgggtactgccgcaacgggcgttcccgacatcgtgttgccgccttgcggcgacggcccttgcgtggccagaaacttgatcaggccctcggaaatcgcgttcaggtcatccatgccgcgaggcgctgcccagacccatgcgccaggtgccggttcatcggagggatgtgcgttccatcccgccacgcccacgcgggcgatgcggccgtcgggttgcgcgacccatgcccagtcgtgcttgcccccggggtcgcaggccgtcacgtagtcccatgccgtgcgccccggttcgtggaccacctggcagagctgcccgtcgggctgcacgaccgagatcgtcttcaggacgggcggaggcgcaacgagctgctggccggccttcagcaccgggtcttcctccggatgcgcctcgagccagcgcgggtcgacgatgccgagcgcgacgcggccggtcacggggaggccctgcagccatttgatcagctgctggcgctggccccgttgttccgggcgcgcgcgccgggtggcggcgtcgagccgcagcagcagctggttcttcagaaactgttgcgccaggcgctcctgcggaatgcgccaagccagcccgggcgccgcggtttcggccggctggcgcagcagccaggcgctcagccgctcgccggggcggatgtcggcgtcgttggccggggtcttgttgtcgacagggctgctgccgaggggctgggccccggcggcgcagctcgccgccagtgcgcaggccaccgcggcgcgaaggggccagggatgtctgccaaagccacggggaagcaaactgctcatgtaccagcgctcgccgctgcgacgggtgctgggggggaaggcgtccactgctcgaagctcatacacaggtcattggaaatacattgctcggaataaacgacccggggcgtgccgcccgcctgcgaaacgccaaagcgcgcgggaggcagcgaggcgctcgaaggatgcgaaacgctgcgctcctcgtaccagcgcaaggacgaggcggccgcgccggccacggcggcttgctgcggcacggcaatgggcgtctgcacgatctcgtcgcgaatgccgaaacggtagcccggcatcatgtcgcgctcacgctgataggccctgggctgcgaggcgttcgcggcgtcggcccacgccggcagcctggaaaagcgcacctcgcgccagtcggtggtgaggccggtcgttcccatgaggcgcccgtcgagcagcctgacgacttcgccggcattgctgtaccagacctcgacggcaccttcggggcgcttgtcgatgtagccaagcaccatgtagaccgtctggccgccgacgactacgcgcaggtaacggtaattcgggttgaaagtgggcccgggcgccgcggcgccgccgctatagatatgccgcgccgtggccagcatggccgaagatccggaagaacagccgccaacgcccaaaagaaatgctgacaaaagacagcattcaataagtcgcgtggcgagaccaacgcgcggagccttcagcgaatgccctcccggcaggagggcccgcacgattaattcgtgccggtcgtgcccgtgccgcctgtgccgctcgtgccgcccgtaccgctgccgccaccgctgttgccgccattgccgctgccaatggcagcggccaatccgacgctggctgcgacgcccccggcctgctgggccgtgatgcggccggatgaagaattggctgcacccgtggcgctggcgggctgcgggccgggcgtttgaacgggtggcggattctggggtgggttttgagccagcgccgaagaaatacccagggcggcaataaaggctgcggaaaccaatgacttaattttcatggcggatatcctcgtaattagcaattgacagttgcgtcaagattagcagctagcgaagtgtgccgcaactaagttagccttttttacaatcgatgtgcgtgcaattccttgtgtccaaatgtcttgcaaatcaaaattaattcattgttcttaattggtctttgcggggggtcgagatgggcattcgcacacgctccggccggcgccgttgaatatgcgcgcaacagcccgctacaatcgccggttgaccctgctccagcgaagaagacttagaggatccccatgagtgacatgacctccggctccccccggatcgacacaagcaagcggacgtggttgatcgcatccagctgtgccggcgtagcgggaggcgtggccaccgcgattccctttgtgagtacgttccagccttccgagaaggccaaggccgcaggcgctgcggtcgaggtggacattgcaggcctcaaggtcggcgagaagatcaccgtcgaatggcgcggcaagccggtgtggatcctcaagcgtacgcccgagcaactggctgggctgcccaagctcgacggccagctggccgatccgctttccaagcggcaccccgacgaattcacccccaagtacgcgcagaacgaacaccgttcgatcaagcccgacgtgctggtggtggtgggcatctgtacccacctcggctgttcgccggtcgaccgcctccagtccggcccgcagccctcgctgccaagcgactgggacggcggcttcctgtgcccttgccacggttccacgttcgacctggccggccgtgtcttcaagaacaagcccgcgcccgacaacctgcctgtgcccccgcacatgtacctgtcggacaccaagctcctgatcggtgaagactccaagaaggcctgaggcagaagaagaacatggctgaattccacgaaatttcccccaatgcgcccacgggcgaaaagctgctcaactgggtcgacaaccgcttcccgctgaccaagctctggaacgaccagtggggcaagtactacgcgccgaagaacttcaacttctggtacatcttcggctcgctcgcgatgctggtcctggtgatccagatcgtgaccggcatcttcctcgtgatgcactacaagcccgatgcgaaccaggcgttcgcttcggtcgagtacatcatgcgcgacgtgccctggggatggctcatccgctacatccactcgacgggtgcctcggcgttcttcatcgtggtctacctgcacatgttccgcggcctcatgtacggcagctaccgcaagccccgcgagctgatctgggtcttcggctgcgcgatcttcctgtgcctgatggccgaggccttcatgggctacctgctgccctggggccagatgagctactggggcgcccaggtgatcgtgaacctgttcgccgccattcccttcatcggccctgaccttgcgctgctgatccgcggcgactacgtggtgagcgacgccacgctcaaccgcttcttcagcttccacgtcattgccgtgccgctggtgctgctgggcctcgtggtggcccacctgatcgcgctgcacgaagtgggttccaacaaccccgacggcatcgagatcaaggccaaccgcggccccgacggccatccgctcgacggcattccttcgcacccgtactacacggtgcacgacatcttcggcgtggtggtgttcctcaccatcttctcggccgtgatcttcttcgcgccggaagcgggcgggtacttcctcgagtacaacaacttcattccggccgattcgctcaagacgccgaaccacatcgctccggtctggtacttcacgccgttctattcgatgctgcgcgcaaccaccgacgacatggtcaacgtgttcgcgctgatcatcggcctggccgccgtgctgaacttcgtcaagggcaagtcgagcacggcactgaagatcgcgctcgtcgtggtggcggccgtggcgatcttcctgctcaaggccttcgacgccaagttctggggcgtgctcgtgatgggcggctcggtcatcatcctgttcttcctgccctggctggacaagagcgaggtcaagtcgatccgctaccgtccgagctggcacaagtatgtttacggcgtcttcgtgttcctcttcctgatcctgggctacctgggtatccaggcgcctggcgtctggggcaacctggtcatcggttcgttcgtgctggacatcgcgcagaccatttcgcagatcggcacgcttttctacttcggtttcttcctgctcatgccgtggtggagcagcaagggcgagttcaagaccgtgcccgaccgcgtgaccttcgccgcccactgaaaagcccaagagagcttgagagaaacacgatgaagaaaagcatttctggctggctcgcggttgtgggcctggcattgggcctgaccttctccgcagccgcatcggccgagtccggcggccttgcctgggacaaggcgcccaacaagaccaccgacgtggcctcgttgcagaacggcgccaagctgttcgtcaactactgcctgaactgccattcggcagccttcatgcgctacaaccgcctgcaggacatcggcatcaccgagcagcagatcaaggacaaccttctgttcgcgaccgacaaggtcggcgagaccatgaaggccaacatcgacgcgcgccaggccaaggattggttcggcaccacgccgcccgacctgacgctggtggcacgttcgcgcgccggccacggcggtaccggtgccgactacctgtacacctacctgcgcacctactaccgggacgacaccaaggccaccggctggaacaacctcgtgttcccgagcgtcgccatgcccaatccgctgtgggagctgcaaggcgaacgccgtccggtctacagcaaggtcgtgcagcatggccacgagaccgaagtgttcaagggttgggagcaagtcacccccggcaccatgacgccgctgcagttcgacacggcggtcggcgacctggtgagctacctgcaatggatggccgaaccggcgcagaacacgcgcatccgcatcggcgtgtgggtgctgctgttcctgctcatgtcgttgcttttcgtgtggcgactgaacgcctcgtactggaaagacgtcaagtagttccgtccacgccgaccggacgccatgcgcgcccggtcccacagagtgggttgccaacgcgacccactctttttgatttttaggagtctctcgccatgatggtcttgtattcaggaacgacctgccccttttcccaccgctgccgcttcgtgttgttcgagaagggcatggacttcgaaatccgcgacgtcgatctctacaacaagcccgaagacatcggcgtgatgaacccgtacggccaggtgccgatcctggtcgagcgcgacctgatcctgtacgaatcgaacatcatcaacgagtacatcgacgagcgcttcccgcatccgcagctgatgcccggcgacccggtcgaccgcgcgcgcgtgcgcctgttcctgctcaatttcgagaaggagctgttcgtgcacgtggccacgctcgagaaccgcacgaccaagggcaacgagaaggcgctcgaaaaggcccgcgcgcacattcgtgaccgcctgacgcagcttgccccggtgttcctcaagaacaagtacatgctgggcgacaacttctcgatgctcgatgtggccattgcgccgctgctctggcgcctggactactacggcatcgacctcagcaagaatgcggcgccgctgctgaagtacgccgagcgcatcttctcgcgccccgcgtacatcgaagcgctcaccccgtccgaaaaggtcatgcgcaagtaagactgcgtccaaccgttctccgctgctttcatgatcaacgcgctcgagtcgtcctccacccgcccgtacctcatccgggcgctgtacgaatggtgcaccgacaacgggttcacgccctatgttgcggtgcaggtcgacgacaccgtccaggtgccgcgcgagtacgtgaaaaacggcgagatcgtgctgaacatcagcttcgacgcgaccagctcgctcaagctcggcaacgacttcatcgagttcaaggcccgctttgcgggcagcgcgcgcgaaatcgtcgtgcccgtgggccgggtgattgccatctacgcgcgcgagaacggccaaggcatggcgtttccggcgcctgtacccaccggcagcaatgccgatggcagtggcgccgcatcgccggcaggcggtgtgccggcagtccaggggcctgcccgcatgccgctgcgcgacgcgtcgcgcggtagcgagggcgatgccagcaagatcgttcacctcgtgacggacgaagcggccgatggcggcaacgacatcggctcgcccgtcgaccccgacgacgagccgccgcgcccgccggccggaggcggcagccgtccgtcgctcaagcgcgtgaaataggacaacagcaggacggacctgaaagggcggcttctgccgccccgttaaaatccgtaaagagaattccgtgccgctttagctcagttggtagagcacccgccttgtaagcggaaggtcgtcagttcgattccgacaagcggcaccatacatttccccactggggatcagcaacggcccttcttggcctgtcccggtgggcagtggtgaccaccaccgccatggccttcgcgctcggcatggtgcggttgctccgcgcgccgccagttgccctccatccatcgccagccaccgtctgcctggacccatcggcccggtgcatacgcgtggtcgggccgagccgcctgccagtagccggagcgccaggcgtaggcgcgttcgttccaccgccaatgaccgggcacccagacctgtcctgcgcgcggccctggcatgggctcgtagcggggcgcgggaggtgcgacctggatcaggccaggcacatggatattgaccgagacctgtgccgcggcgggcagggcacaggcggcgagcgctgtggcaatcaggagagccgagattttcatttgaaacccttgaagatgagaacacgcatgtacaacgcgggccggcgcaaagtgtaatcagaacattcctcagggccttgggcagccgaaccgtggtacgcaaaggccgcgcccgtttcatcaggtgctagagttcaggcgcacgctgcatgccgatgcgcagactacgcttcctgacccaccgccaccgcgccccttccacaaaccgggtgctcggcctgctgctggccttcaatgccggcgcggtgaatgcggggggcttcctgatgctgcacatgtacacctcgcacatgacgggcttcgcgtcgcagtttgcggacgggctggtgctcggcaacacgaagctcctgttgaacgcgctgggcgccatcctcgcgtttctgtcgggcgcggccgtctgtgcaattctcgtgaactggggccgccagcaccgcttgcgcagcgtctacgcggtgccgctgctgctcgaggcggcactcatgtttccgttcggcctgatgggcgccatcacgttgacctggtcgacgccgtttgccgtgccgctcactgtgctgctgctctccttcatcatgggcctgcagaacgcggtcggctccaagacctccggaggcagcgtccgcaccacccacatgacgggcaacatcaccgacatgggcatggagctgggcaagctgatctactggaaccggcatgccacgccggcgcatgccatggttcggcacgaccgccggaggatgcggatggcgggcgggctgattggcatgttcgtgctgggcggcatcgtcggcgcgctcggtttcagctctatcggcttcgtgtgcgtggtgccgctcgcggcgttgctgctcgccatttcgataccgccgctcatgcgcgacctgccgcgctcccggacgctgcagaagcttcttgccgccatcggtgtgaaggtgccttccaggcacccgccggcgcacgccgattcgtcgcccgaaagctgaaggctctcccgggtcaactgcgggcctcagatcccgcccacgctgcccgtgatcggcagcacgatgccggtgatatagctggcgcaactcggcgccgcaaggaacacataggcgggagacagttcctctggttgtgccggtcgctgcaggtcggtgtgcttgccgaagtccttcaccttttcgggcgggctgtcggcggggttcaagggggtccataccggtccgggcgccaccgcgttcacgcggatacccttgggcagcaagttgctggccagcgacttggtgaatgcgtggatggcgcccttggtggtcgagtagtcgagcaggtgggcgcttccttccaggcccgtgaccgagccggtattgatgatcgacgcgccctggcgcaggtgcggcaccgcggcgcgcgccatctggaagtagccggtgacattggttctgagcgtgaggtcgaagcgctcgtcggtgatgtcctcgatcgaagccgcgtgcaactggaacgccgcgttgttcacgaggatgtcgagcttgccgaaggcctcgagcgtcctgtcgatcgcctcgcggcagaacgccgggtcagagacgtcgcccttgatcatgatgcagcgcgcgccctcgttctcgacatggcgccgcgtttcctcggcgtcctggtcttcttccaggtagacgatggccacgtcggcgccttcgcgtgcgtagagcactgccaccgcgcggccgatgccggaatcgccgcccgtcaccagcgccgtcatgccctcgagcttgccgctgcccttgtaatccggcgcctcgaaacggggccgcagcgccatctccgcttccacgcccggcttgcggaggtgctgcgccggcatgggattgaccggctgggaccgcggccccgcttgagcgggttggctggatttcctggaggccggctttgcgctgtcctttgcgtcttgtgcacgctgaaccgcgcggtgcctggaggccgtgtgggctgcgcctcgggatttggcggatccggagggggatgcggtggtcgatttcatggtgcttgggctcctcatgtgaacgaccaccgtaaaactccggggctcggctcgcgtaggaatccgtctcgaatgcgcgcccgccgtgtcgcgcggcgatttccgcttcgcttgcaaagggtaacgatgcacgcctacgcaccggccatggcggcgtgcgcattgtcatggcttcccgactctggagcaggggcgatgcagcctgaaaaggacacgaaggaatccgccggcaaacgcaatggcaacggcgaaagcagcagtggcaacggcaagccgcaccggccgccccgccgcaagcatccctcgctccaggcactgacgcaccggaacatcgagtcgattctgaggctggaagaagaaaaccggcgcgccaagccgctgctctacaggctggtctcccgcgtagcgcgctactgcggaacggtggctttcctgtggtggaacctggccttctttgccgcatggatcctgctcaaccagtttgtctggcagatcgatccctatcccttcaccttcctgctctgcctggtttccatcgaggccatcgtgctggcgatcatgatcctgatcagccagaacatgtctgccgaagaaagcgagcgccggcaccacctggacctgcagatcaacctgctgaacgagcgcgagatgaccgccttgctgcgcctcgccacccgcatggcggaaaagatggaggtgccgcaggagtcgcacagcgaggtcagggcgctgaccgagcgcaccgaccccggcaaggtgctgcaccagatcgtggaggccgaggcttcgcacgaggagcgccgctgacgggcaaccggcgccgctagggcagttccgcgccttcgaccaggaagcgcacgcgccgcacgccctgccattcgtccgcatcgagccggaaggccagcttcacgcgcgcgggcagcggatcggtatggccgaaccagatgccgtcgaccggctgcccctggtgccgcagcttgagcgcgaggtgcttctcgcccaccaagcgctgcgacaccacctccacctcttcgctgaaggtgggcggggcaaaaccctggccccacacctcgcggtgcagcgtgtcgaccaggtcgatgcgcatgtactcgcgggccagcggcccgtcggtgtcgaggcggcgcgtcagggtggcggcgtcgagccactcgtgcgccacttcggccagcgcctgctcgaacacctcgaacttctcgcgcgcgacggtgcagccggctgccatcgcgtggccgccgaagcgcagcagcacgcccgggtggcgcttggccaccaggtcgagcgcatcgcgcaggtgaaagcccggaatcgagcggccggaacccttgagctcatgcgccttgcccggcgcgccgctcgcggcaaacacgaaggtcgggcgatgaaaacggtccttgatgcgcgaggccacgatgccgaccacgccctcgtgaaagtcggcatcgaacacgctgatggcggccggaggtgcctcgccgccatcggccgtggggccgaacagcgactcagccagcagcagcgcctggtcgcgcatgccgccctcgatgtcgcgccgctcgcggttgatgccatcgagcatgcgcgccagttcgtcggcgcgtccggcatcgtcggtcaagaggcattcgatgcccagcgtcatgtcggccagccgtccggccgcattgatgcgcgggccgagtgcaaagccgaagtcgaaggtggtggccaccgcggcgttgcgtcccgcggccttgaacagcgccgcaatgcccgcaggcagcgcaccggcgcgaatgcgccgaaggccctgcgcgacgaggcggcggttgttggcgtcgagcttcaccacgtcggccacggtgcccagcgccaccagaggaagcagcacgtccagcttgggctgcgtggctgcggtgaagaggccgcgtgcgcgcagttcggagcgcagcgccagcagcacgtagaacatcacgcccacgccggcgatgctcttgctctcgaagccgcagccgggctggttgggattcaccagcacctcggcggccggcagttcggggcccggcaggtgatggtcggtcaccagcacctgcaggccgcgcgccttggcggcagccacgccctcgacgctggcaatgccgttgtcgacggtgatcagcatgtcggcgccgctgtcggccacgcgctcggcaatcggcggcgtgaggccgtagccgtcgaccacgcggtcgggcaccaggtagctcacgttcttcgcgccgagcaggcgcaggccgcgcacggcgacggcgcaggcggtggcgccgtcgcagtcgtagtcggccacgatgcacaggcgcttgtcctgtgccatggcatcggccagcaacaccgccgcctcgcgcgcgccgtgcagcgtgtcgggtggcaacaggcgcgccaggccgtcgtcgagctcgtctttggcaagcacgccgcgcgcggcgaagaggcgggcgagcaggggatgcacgcccgcctgctcgagcgcccagaccgtgcgggggggatctccctggcgatgatcttcatagggcctcgagcacgctggcggcgcgcggccggtcgaacaggcttcgggcccagcccaccaggccgcgctgctgcaccgcgtagcgctgcgccgcgcggtcgccgcacagcgtgagcgtgacgtcggcaccggcggtgtagtcggccagcaggctggcgagggtgcttgcatcgagcgcgtgccaggcttcggcccagcccgggccgtcgtcgcgcagcgcggccacgcgcagcgcttcgctcacggtcggcggggtcgtgtcggccggaggaatgcctgtttgcagcgcgccggtgccgctgagccagaaagagttgatcggcggcacgccgcgggcggcgcggtcgtcgttcacgcgttgggtatagagcagcatctgcatttcgttctggagccggcgcagcggccgcgccgcttcggccaggggggaccattgcgaaatgggatggcccactgcgcggtcgatggacgccgtggccagtccattgaagatgggtgcgcgcgccaaccatcggccgggcgtcgcggaggggtgaagggcaatgccgtcttcttcgaagaaaggatgcgcggcggacagcagcgccgccgattcggcggcgtcgatctcgatggcggacgggtcgcccagcaccacgtcgtcgatgcccacctgccagttgcacagcgaaaccaggccccagccttcgctgtcgccgggttcggcgatgctgctctgcctggcttccagcgcggcccagggaacgcagccgtcgggcgccgagatgcccagcgccttggcgagcgcccgttcgtgaggtggtgagcgcgtgctttcgtcctgcgtatcggtctccgccagcgagagccgggagagcagtgcttcgaggttgggcagacgaagcgaaggcaatgccgcgcggcatgccggggaaccgcggccggcaaaggggatcaacagatgacgtgggagaggttcggccatttccctattgtccgggatgctaggatgaaacgccctccgaagcgcctttggcgctcctcccactggagggcgcacccggcgggtgcacctggctgagctcaaactgaaaatatgcgacttccttacgaactgcagctcggctggcgctatacccgcgcaggccgggcgacgcggcgcaacggcttcatctccttcatctcgggcgtgtcgatgctcggcatcgcattgggagtggcggcgctgatcatcgtgctgagcgtgatgaacggcttccagaaagaggtgcgcgaccgcatgctcggcgtggtgtcgcacatcgagatcatttcgcgcgacgggcaggcactgcccgacatcgacgccatcacggcggccgcgcgcaagaaccccgaggtgatcggcgctgcgcccttcattgccacccaggcgctcatcgcgcgcggcgaggacatgaaaggcacgctggtgcgcggcatcgtgcccaagctcgagcccgaggtgaccgacatcgactccacggcgcagaagggcacgctcgacaagctggtgccgggccagttcggcatcgtgctcggcggcgagctggcgcgctcgctgttcgtgcagccgggcgaccaggtcacgctggtggcgccgggcgggcaggtcacgcccgcgggcgtggtgccgcggctcaagcagttcaccgtggtgggcaccttcgattcgggccactacgaatacgactccgcgctggccatgattcacgaggaagacgcccagcgcgtgtttcggctcgacgggccttccggcatccgcatcaagctcaaggacctgaacgaggcgcgcgaggtggccgaccagatggccgtcacgctgccgggccagttcctcattcgcgactggacgcgccagaacaagacctggttcgcggccgtgcaggtcgagaaacgcatgatgttcatcatcctcacgctcatcgtggcggtggccgccttcaacctggtgtccacgctggtcatgaccgtgaccgacaagcgcgccgacattgccatcctgcgcacgctgggcagctcgccgcgcagcatcatgggcatcttcgtggtgcagggggcgatggtcggcgtgatcggcaccgtgggcgggctgctgctggggctgggcattgcctacaacatcgacgtgatcgtgccggcgctcgagcggctcttccatgccagctttctgccgaaggacatctacctgatcagcaagatgccgagcgatccgcagcgcagcgacatcatgccgattgccatcatttccctggtcctggctttcctggccacgctgtacccgagttggcgcgcgagccgcgtcaaccccgccgaggccctgcgctatgagtgaacaaaaaaatgccgccacgccgggcaatggcgtggtgctgaaggcgcgcggcctcaccaagcgctttcatgaagggcgcatcgacctcaccgtgctgcacggcgttgacctggacgtgcgcgccggtgaaacgctggccatcgtcggcgcctcgggttccggcaagagcacgctgctgcacctgatgggcgggctcgacggccccacggccggcagggtcgagctgctcggcaaggacatcgcgcatgccgatgcggccgagcagggccggctgcgcaaccagcacctgggcttcgtctaccagttccatcacctgctgcccgaattcagcgcgctcgacaacgtggcgatgccgctcaagatccggcgcatggcgcccgcgcaggcggcggccgcggccacgaagatcctcgaaagcgtgggcctgggtgagcgactgcaccaccgcccggccgagctctcgggcggcgagcgccagcgcgtggccattgcgcgtgcgctggtcacgcagccggcctgcgtgctggccgacgagcccacgggcaacctcgaccgcaacacggccgacacggtgttcgagctgatgatcgagctggcgcacaagcaccgcacggccttcgtgatggtcacgcacgaccaggagctcgccaagcgctgcgaccgcgtgctgcagctggtggcggggcggctcgccggctgagttgcagctgccgcttgccacggtgcctgcaatgtcgcgaaactgtctgcctgtccggcaagatgccgttcaatcacaggagcgctgcttcatcatggaaaccgacgacgacaccccacccgcggccactgcggaaccgcgcaattcctacctggaagagaaggccttcaagtcgcgcacgctgctgattttcggcagcatcaccgacgcggtggccgccgacgtgacgcgccggctcatcgcgctggatgccgacagtcccgaaaaaccgatcgacatcctcgtgagttcgcccggcggccacctggagtcgggcgatgccatccacgacatcgtgcgtttcatcagcgcaccggtgaacatgatcggcaccggctgggtcggcagcgccgccacgcacctctacctggcggcgccgcgcgagcggcgcgtgtgcctgcccaacacgcgcttcctgatccaccagcccagcggcggcgcgggcgggcaggcgaccgacatcgcgatccaggcgcaggaaatcatcaaggcccgccatcgcgtcgcgcacgagatcgcgcgcgaaaccggcaagccgatcgacgtggtgctggccgacatcgagcgcgaccgctggctctcggctgcggaggcggtcgaatacggactggtctcgcgcatcatccagcgcaagaccgagctgctgtagttgctgctgtagttacttgggcttgtaggccaccacgtcgatctcgaccttggcgtcgaccatcaaccgcgcttcggtggtcgagcgcgccggcttgttttcaccgaagtagctcatgtagatgcggttgaaggcaccaaagtcgcgcgcgtcctgcagccagacggtgctcttgcagacgtcgtcgagcgtggcgccggccagcgccagcacctttttcaggttttccatcacctggcgcgtctgcgcctcgatgccgcccaccacgatctcgccttcggcattggcaggcacctggcccgacacgtagatgaaatcgccggcgcgcacggccggggagaaaggacgtgcctggcggtcagaggcgacgggcggggcgccgaggtattcgagcggcatgagaggactcctgaagtgaagacaaagaagaaaaagggggatcgcaagtatcggcccaatctgaaaatctctttcagaataaccctcaaacaagggttaacacggatgattttgcatggatagtgcttcaaagtgcgggccgaagagaaaatttctttcacaaaccgcctgccccatgaaggagttccccatgttccacgccggtcttgtccagcgcctgccgaagctgtcgaagcgcagcctgctgggcgcttccctgctcgcgatgctgtgtgccgcgttgcctcaccagcaagcgcatgcccaggggccgcgcaacttcgccacgctggccatggtggccgaaccgcagacgctcgacccgatggcctccacggccgacctggtcggaaccatcatgcagcacgtgtacgagacgctctacaccttcgacgccaagtggaacgtggtgcccatgctggccgagagcagccctaagatctccgccgacggcaagagctacgccatcaccctgcgcaagggcgtgatgctgcacaacggccgcgaactcaacgccgacgacgtggtggccagcctgcagcgctggatggaccagtcgccgcgcggcaaggccgtgggcaaggaaatcgagagcctcaaggccaagggcccgctgggcgtggagatcgtgctgaaggcgccgtatgcgccgctgctctcgcagctcgcgctgcccagcggcatggcggccatcatggccaaggattccatcgcttcgccgctgaaggagttcatcggcaccggcccctacaagttcaaggagcgccgtcccgaccagttcgtgctgctcacgcgtttcgacaagtacgccgcgcgcaaggagccggcaagcggctacggcggcaagcgcgaagccgccatcgaagaactgcgcttcgtgcccgtgcccaacgccagcacgcgggtcgaaggcgccctggccggccagtacgactttgccgacctgctgccggtcgaggccctgccgcggctcgagaagtccggcggcaagaccgtgccgatcatgacgccgtcgttcggctttccgtacctcgtgctcaacaccaaggaaggcgtggccgccaaccaggccctgcgccaggcgatccagtccgcgctcggcgaaggcgaaatgctcgctgccggcttcggcgacacgcgcttctttgtcgccgaaggcaaccacttccccaagggctcgccgttctattcgaccgccggcaccacgctctacaacgagcgcaacgcgtccaaggccaaggaggccgcggccaaggccggctacaagggcgagccgatccgcgtgctcaccagccgccagtacgactttcactacaacatgtcgctcctgatggccgagcagctcaagcgcgccggcttcaaggtcgatttgaacgtggtcgactgggccacgctggtgcagcgccgcaacgacccgaagctgtgggacatctacgtcacccactcgggccagtttcccgagccgatgctctcgccgccgcagctcggcgacggcgcgcccggctggtgggattcgcccgccaagaagtcggcactgcaggccttcaatgtcgagagcgatccggccaagcgcggcgcgctgtggggcaaggtgcagcaggtggtctacgaagaagtgccgtacatcaacgtcggcaagttcaacggcctgtcggccaagagcccggcgctggacaactaccagcccgcgacgtggccgttcttctggaacgcaagaatcaagtaagcccccgggtcgccacggagccaaccactcatgtttcgctatctcgcctcgcgcgccgccggcatgctcgtcgtgctcgccatcgtggcggtgctcgttttcgtgctcacgcgcgcggcctcgggtgatccggtctcggtgctgctgggcgaccaggccaccgcggccgacatcgcccgcgtgcagaaggaatacgggctcgacaagccgctgcccgtgcagttcggctactggctgcgcgaagtgctgcagggcaacctcggcacctccatcttcctgcagcggccggtgacgcaagcgctgtgggagcgctccgaacccaccacgctgcttgcgctgatggccgtggccatcgcggcgttgatcggcgtgccctgcggcatcgtctcggccgtgtttcgcgggcgcatggttgaccagctcttcaccggcatcgcgatgctgggcgcgagcattccgagcttctggctcggcatcgtgctgatccagatctttgcggtgtcgttcgggtggtttccggtgtcgggctatggcgcgcccgatgcgccgttcgccgagcggctgcatgcgctggtgctgccggccacggtgctgggcttgctgaactcggcgctcatcatccgcttcacgcgggcctcgatgctcgacgtgctgggcgaagactacgtacgcaccgcgcgctccaagggcctgagcgaaagcacggtggtgctcaagcatgcgctgcgcaatgcgctggtgcccatcgtcacggtgatcggcctcacggtcgcgctgatgatcggcggcgccgtcatcaccgagaccgtgttcggcctgccgggcgtcggcaacctggtcgtgagcgcggtgctgcggcgcgactatccggtgatccagggcgcgctgctcgtgatcgcggcgatctacgtgctgatcaatttctcgatcgacctactgtacgccgtcgtcgatccgcgtgtgaaggtctgagagcaacaccatgcaaatgccccgaatgctccgccagctgatgcaccgccgcatcgtgatggtctccgcgctggtgctgctggtcatcgcggtgctcgccatcggcgcgccgttgttcgcctccatcgaccccaacgacacggccgtgctgcaacgcctgaaagggccgagcgccgaacacttgctgggcaccgacgaactcggccgcgacatgtactcgcgcatcgtgcacggcgcgcgctattcgctggccattgccgcgctcaccgcccttggtgcggtgatcgcgggcacggtgctgggcctcatggccggcttctttcgccggctcgatgcgccgttgatgcgcgtggtcgacgcgatgatgtcgttccctgacatcctgctggccattgcgctcgtggccatcctcgggccttcgctcatcaataccgtgcttgcattggtgctggtctacaccccgcgcgtggcgcgggtggtgcgggcctcgacgctggtggtgcgcgagctgctgttcgtggaggccgttcgtgccctgggcgtgcgcacctcgcgcatcctgtggcgccacatcctgccgaacctgatgtcgcccatcctcgtgcaggtgtcgttcatcttcgcctacgccatcctggccgaggcggggctgtcgttcctcggcgttggcgtaccgcccgaaattcccacgtggggcaccatggtcgcgggcagccagcagtacgcgcaccaggctttctgggtggtgctgttcccggggctcgcgatcatcttcacggccctgtcgctgcaactgctgggtgacggcgtgcgcgacctgctcgaccccaaactgaagaagaccctgtgatgacgaccacgaaaacaccgcgtctccaggtcagcaacctgagcaccagcttccccaccgaggacggcctgatccgctcggtggccgacgtgagcttttcgatccagcccggcaagaccacggcgctggtcggcgaatcgggctcgggcaagtcggtcaccagccttacgctgatgcgcctcctgcccaagaccgcgaatgcgcaggtcagcggctcggcttccttcgtgacgcgggaaggcaagtcgctcgacctgctgcagatcggcgagcgtgagatgcgaagcctgcgcggcaaccagctgtcgatgatcttccaggagccgatgaccagcctgaacccggtcttcaccatcggcgagcagattgccgagagcgtgcggctgcacaaggggctggaccgcaaggcggccatggcccatgcgctgcgcatgctggagctggtcgagattccggccgcggcgcagcgcatccacgagtatccgcaccagctttcgggcggcatgcgccagcgcgtgatgattgcgctggccatggcctgcgacccgacgctgctgattgccgacgagcccaccaccgcgctcgacgtgaccatccaggcgcagatcctcgaactcatgcgccggctgcaggccgaaaccggcatgagcatcctgttcatcacccacaacctgggcgtggtcgcgcaccatgcggacgacgtggtggtgctctatgcgggccgcgtggtcgagagcgcgcccgtgcggccgctgttcgcgcagcctgagcacccgtacacgcagggcctgctggcctgcctgccgggcaaggcgcgcctgccggggcagcccaagcccaagcgcctgttcgcgattcgcggccaggtgtcgagcccgctcgcgccgccgccgggttgcgctttcgagccgcgttgcgatcttgcgctggcggggtgcagggaagcgattccgccgctcatcgagatccgtcaggaccgccaggcgcgatgcatccgtgtacaacccgacgcccaacttgcgagggtcgcatgacgggcgcgctgctcctgtcttgctccctctcccgcgtgcgggagagggctggggtgagggcggcccccgcatccctcgcgagcaccctcatcccccgccttctcccgcaagcgggagaaggagccaatacaacatccccatgaccaccgccgcccccctcatcgaagtccgcggactcaagaagtacttcggcagcagcgaccgcccggtgcgcgcggtcgacgatgtctcgttcgccatccaacccggcgaaaccctgggcctcgtcggcgaatccggttccggcaagagcaccatcggccgcaccgtgctgcggctggtcgagcgcaccgagggccaggtgctctatcgcggcgatgacatcggtgcgctctcgggcgagcgcatgcgcaagctgcgcagcaagctgcagatcatttttcaggacccgtatgcgagcctgaacccgaagatgcgcatcagcgccatcctcggcgaggcgctctccacgcacggcctgcacaagggtgccgccgcgcgcgacaagcgcattgcggagctgctcgaaaccgtgggcctgcgcgccgagcatgcgagccgctttccgcacgagttctcgggcgggcagcgccagcgcatcggcgtggcgcgcgcgcttgcggtcgagcccgaattcatcgtggccgacgagccgctatcggcgctcgacgtgtcgatccagtcgcaggtcatcaacctgctggccgatctgcgcgagcggctcggcctcaccatgctcttcatctcgcacgacctcgacgtggtcgagtacctgtgcgaccgggtggtggtgctgtacctgggcaaggtgatggaagtggccactaccgacgagcttttcgcacggccctcgcacccttacacccaggcgctgctggccgcgagcccgaagcccgacccgacgctcgccacagagcgcatcgcgctcaagggcgacattcccagcccgatctcgccgccatcgggctgcgtattccgcacccgatgcccgcatgccatcgaggcctgcgcgcagaccgtgcccgcgctggatgagatttccgtcggacactacagcgcctgcatccgcaaagagctgctctccaacattgccgcatgaccatgaccgacatcaccgccgccgacaaggatttcaccgacccgctgctgggcagcaacttcaagggctacccgcgcacgcagccgccgcgccgccgcagcgaggtcggcgccgcgggctggaacgtgctcgccggcgacctgccgctgccgctggccgtgctcaagcgcgaggcgctggagcacaacctggcgtggatgcagtcgcgcgtgcgcgagtggggcatcgacctcgcgccgcacggcaagaccaccatgtcgccgcagctcttccagcgccagctcgatgcgggcgcctggggcctgactttcgccacggtgacgcagcttgccgtgggcgtggcggccggcgcgcgccgcacgctcatcgccaaccaggtggtcagcgacgaagacctggcgggcatgcaactgctgttgcaggcgcatgccgacctgcgggtggtgttcctggtcgattcgctcgcgcagctcgcgctgatcgaagactggtcgaagcgccatcccgagagcgtgcccttcgaggtgatgctcgaaatcggcgtcgaaggcgcccgcaccggctgccgcacgcatgaagaggcggtggcgctcgccacgagcctgcgcgccagcgacgcggtcaagctcgtgggcatcgagacgtatgaagggcagggcgccaccggcgccagcgaacccgacaccacctacgccaacgcgctgatggaccgtgtggaagccatcgcacgccactgcgacgtgcagcagctgttcgagaccgacgaggtgctggtctcggccggcggttcggccatcttcgatctcgtggccggccgcctgaagcccgcgctcggtgcgccggtgcgcggcctgctgcgttcgggctgttatgtcacgcacgaccatggcttctacaagcgcatggtgagcgcagtggacgagcgcctgggctgcgattgcggcgagagcctgcgccccgcgatggaagtgtgggccacggtgcagtcgcggcccgagcctggccttgcgattcttgccgtcggcaagcgcgacatctccttcgacctctcgatgccggtgccgatcgcgcgcgccgcacgcggcatgctcgaagcagaggccgtgcccgccggctggaagatcaccgcccttaacgaccagcacgcctacctgcgatgggataccaacgaagaagcgcaggccccggtggttggcgaccgcgtcggcctcggcatttcgcatccgtgcaccaccttcgacaaatggcattggatgccggtggtcgaagagaactaccgcgtgagcgacgccgtcgccatgcacttttgaacacgtgccgatgactccctcattgcttcagaagatcgccgagctccgcagcagcgcgcccgccacgcggcgcgcgattctcgacctgatcctcgaagaccccgaccgcgcgctcgaagagagtttcgagcagctggccgagcgctcgcgcagctcggtgcccaccatcatgcgcacctgccgcgacctcggctttgcggggctgcgcgagttcaagctcgcgctcgcacaggagctggcgctcggcggctcgcccctgcaccggcgcgtgaacatcgaggacgcggccgatgaggtcgtcagcaagatcgcgcgcagcgccgcggcctcggtttcgggcgtgcgcggacagctcgacatgaaagtgctcgaaggggcagtggccgccatcgcggccgcgcctcacgtggacctgtatggcgcgggtgccacgtcgtggttcatggtcaacgatcttcaggcgcggctcttcaggctgggcctctcggccaacgcctgggccgactaccacctgcagcaggtggcgggcgcggcgcagcgtccgggtggcgtggtcattgccatctcgcacgtgggcggcatgccctcgctgctcgatgccgtggacatcgcgcgcggacaaggcgccaaggtggtcgcgctcacgcggcccggcaccgcgctggcggccaaggccgacttcctgctgggtctctcggtgcccgacgacgccgtgatgcacgtgggcatcgacgcctacctgacgcacctcactgccatcgaaattctcacggtgctggtggcccagcgccgtggcgaacccgccgtgcagcgcctgcagcgcgcccgcgaggcctttcagcgccatggcatcgacgcctccacgcacccgctgcaaagctgggacggcggcggcatcaacaccggaggccgcgcatcgtgagcgacgccaaagccatcctgctcgaagccggcctcgtggtcgatggttcgggcggaccctcgtggtccggcgacgtgctgctgcagggcgaccgcatcctggcgctcggcgaagggctgcgcgagcggttgccaaaagggctcacgctggccgacatcgatgtcgtcgattgccgcaccaaggtgattgcacccggcttcatcgacgcgcatacgcacgacgacgccatcgtgctgcgcgacccgctgtgcctgcccaaggtgtcgcagggcatcaccacggtggtgacgggaaactgcggcatttcgcttgcgccttaccgcacgccgcagtccaagccgccgctcacgctgctgggtgcggagtcgttcaagcacgccaccatggccgagtaccgcgcggccgtcgatgctgcgcagccagcgctcaacgtggcggcgctggtgggccacaccaccttgcgcttcgcggccatggaggtgctcgaccggcccgcgagtggcgacgaactcgcgcgcatggcggcgctgctcgacagctgcatggccgaaggcgcgcatggcctgtcgtcggggctgttctacgaagaagcgtttgccgctccggccgcagaagtgactgcgctcgcgcgcatcgtggcaaggcacggcggcatctacgccacgcacctgcgcagcgagatgcagcagatcatcgaggcgctgcacgaagccggcgacacggccttcagcgccggcgtgccgctcgtcatctcgcaccacaagtgcgccggccccgccaactggggccgcacgaaggaaacgctgccgctgatcgagacgctcgccgagcggcagaagatctcgatggacgtgtacccctacgtggccggctccaccgtgctgcgcgaagacctggtcgacggcgtcatcgacgtgctgctgacctggtcggacccgcacccggaaatgacaggacgcctgatctccgacatcgcccgcgaatggggcaccaccgagcaggaggcctgcctgcgcctgaagcccggcggcgcctgctatttccagatgcaggaagaagacgtggagcgcgtcatcgcgcacccgctcaccatgatcggcagcgacggcctgccgcacgaccgccatccgcatccgcgcctgtggggtgcctttccgcgcgtgttcgcgcgctactggcggcagcgccgcctgttcacgctggagcaggccgtgcacaagatgaccggcatgaccgcgcgcaacctgcgcattgccgaccgcggcctgctgcgcgtgggcgccatggccgacgtggtggtgttcgaccccgagaccattgccgacaccgccacctacgacaagccgcacggcgtgagcctgggcgtggagcgggtgttcgtgaacggcgtgctggcgtattgcggtggcggcgctgaagcgaaggtgcttgcgcgggcgggacggatgctcactcgcgggagttaggcgaacacaacgcgttcgggaacaacaagccccggataggatgtgcgccatctccatgttcctcctttccatgcacgcagccgcacgccatctcgtttttcacgcagcagtgatcctgcttttcggacttttgctgggcgcaccctatgcgaaggccatcaagcgcaatgcgccggcccacatcgtcaactcctggcgcgtggcgcacttgagcctgcccatcggtgcaacgttgatgctcgcgacagctgccgtgctgaccttgcttgcggtctccgcgccggtcatctgggtcattgccgttgcgctgatcgtttcaggctacggcttctgcgtttccacgcccctggccgcgatcacgggccagcgcgggctgtcttccgatggcgctggcctgggcaagctcgtctatgctggaaacatggtcggtgcgtggggctcgatcgtcggtgccgtcgcgttgctctgggcggcgttcgttgcgctctgacgggcggatcggcaacacgtcgcgggcgggcatttcatcgtcgatggcgaggccgtcgatgcgcggccgctgccgcccgcgcgcccctaggtttttctcggacggccggttccgggtccgtcagggcacgggcccgcgtgccaccggcaccacgagcatgcggcgcaatgccagcacgccgcacccaccggccagcaagaccagcagcaaggcccacgccgcgtccgccgtcgaggcggattccggccagtcgccgatgaagatcgtgccgctgttgtaggccgcatgcagcgcgatgcacggaatgagcgaacgggtccgctcatagagccaaccgagcactgtgcccatgaccagccccacgacgaactggtagatgttcaggtgcgcggcgccgaagagcagcgccgagcccaggatggcctgccaccgcgaatagcgcagcagaaagccccgcagcacgatgccgcggaacagcatttcttccagcaggggggccatgaggcacaccgccagcgtggccgcgacgctgccatccgccatgcggctgaacatcgactcctcccaggccgagagcggcgcgatgaacaccagcaggttgagcacggccgtcatcaccaccatcagccccggcacgagcagcagcaccggcggcaccaccagcatcagcgtggccctcgcggaagccggcgactcgtgaaatagttcgcggtaggtgagcttctggtggtgcatgaccacggcgaatacgcagccgttgcccagcaccgcggacagcacgccgagctgcatgccgttcaggcccagccaacggttggcgtcgcgcagcgcaacgccaatgacgaattcgcagaggaacaccgccaggaacagcagcgcggcctgcgtggcagaaggaaaagccgtgcttttcggggagggcatgggggtcttcgggcgccgagggggatagacgcatattaccgttgagcgcccccggacggctcgcgggcggcgctccgccaccgcaggatcgcccgctacagcccgctacagcccgccgcaacccgctacagcacgaacggaatgaagcgccgggtgctgcgcatgtactcgcggtaggcgtcgccaaaatgcgcgatgcattcctgctcgtcgcgcagcgccgtcaggaacagcagcaccgtggcggccagcaccagcgccagcgtgagccaggtgaactgcttcaggaaggcgccccaggcgagcagcatcagcgccgtgtacatgggatgccggatgtagcggaaggcgccggtggaaacgatggaagaagtcttctcgaaaccgtagagggccgggtcgtcgttgcgcgcctcggtcggcttgccttgggccttgagcagtttgaccgcgtggatcggcagccagatcgacagcgcgaggaacacgcaggagagcagttgggtgagcgacagcggatcgacatgccacaccggcaggttcacgatgatcagcaccagcatgcattcccaggcgaagaagcggtagaagccgtgcgagccgggctggctcaacggcccgcgcgagacgtacagcagcgcggccgtgccggagataaaaaggaagatctggaaccagagaagcatggcggccgaatttacacggcctgcccggcttcagccagaggtagaaaacccgccgaccaccggaatcgctgtgccggtcttcaggtggcgtgcggtttcttggagacgagggtcaggatgtcgtagctcgcgacgagctcgccgtcctggttggtcacctccacgtcccatgccaccacgccctggccgtggccgctcgcgtccttcttgttgcggtcggtcttgcgcttgcaggtcagccgtgcccggatggtgtcgccgatgcccacgggcttgacgaagcgcagcgtatcgaggccgtagttggccagcaccggccctggcgcgggtgagacgaacaggccggccgcggccgacagcacgaagtagccatgcgcgatgcgcttgccgaagggcgactcctttgccgccacctcgtcgaagtgcatgtagaaatagtcgcccgagatgccgccgaaggccacgatgtcggcctctccgacggtgcggcgatgggtgagcagcgagtcgccgatccgcaagtcttcgaagtaacggcggaacggatgcacctcgctctcgcgcacggccgcgccgcgcacatgctccccggtgatggcggccagcatggtgggcgagccctgcaccgcggcgcgctgcaggtagtgcttcacggcgcgcaggccgcccagctcttcgccgccgcccgcgcggcccgggccgccgtgcttgagttgcggcagcggcgagccgtggccggtcgattcggcggcggcctcgcggtcgagcaccagcagccggccgtgccatgcggcggccacgggaatggcccgggccgcaatggccgggtcgcgcgtgaccagcgtgccgacgaggctgccgcggccgcgcgcggccagcgcgagcgcttcgtcgatgccgtcatagggcatcagcgtgctgaccgggccgaaggcttcgacgtcgtgcgcggcatcgtgttcgagtggcttgcggctcaagagcagcgtgggcgcgaagaaggcgccttcgccaacgccatcgcccaccggcgagaagccgtcgcgttcgccatggaccagctcggcctcctgcagcagcgtggcgacgtgctccgccacgtcggccttttgtgcgtgcgaagcgagggcgcccatgcgcacctcttcgcgcgacgggtcgccgacgacggtcttggcgagccgcgcccgcaggcgttcggccactgcgtcgagatgctggcgcggcacgatcgcgcggcggatggccgtgcatttctggccggccttggtggtcatctcgcgtgccacctccttcacgaagagatcgaactcctcgtcgtcgggcgtcacgtcgggcgccaggatcgcgcagttgagcgagtcggcctcggcattgaacgggatcgactggcgcaccaggttcggatgcacgcgcagcctggccgcggtgtcggccgagccggtgaaggtgaccacgtcggcgccctcgagccggtcgagcaggtcaccggtgccgccgacgaccagctgcaggctgccttcagggagaatgcccgactgcacgatgagccgcaccagcgcttcggtgagatagctggtggccgtggccggcttgccgatgcagggcatgcccgcgagaaaactgggcgcgaacttttcgagcaggccccacaccggaaagttgaacgcgttgatgtgcaccgccacgccgccgcgcggcaccaggatgtgcgtacccgcgaagccgcccttcttgccgagcgcgaaggccggaccttcgtgcaacaggttgcccgacggcagctcgttggtgccgatgccggcataggcgctgagcgtgccggcgccgccctcgatgtcgatccagctgtcggcgcgggtcgcgcccgtgtgggccgagatggcgtagagcgtttccttgttcgcggcgagaaacttggcgagggccttcaggcgctccgagcgttgctggaagtcgagcgccatcagcgcggggaggccgacacggcgcgcgtggttcagtgcttcggcgaagtcgatggcttcggcatgcgtgctggccacggctttcccgttgatggcgctgcgcagttgctgcgcgctttccttgccgatccagcggcccgcgatgtagctttgaagaatggtcataaggtgtcctttcgctgtcttggtattgctccttccccttccgggggaaggctgggatgggggcaggcggcgctcattcggcgcagtgcgttatcgaacgccgcctgcccccatcccgaccctcccccggaaggggagggagaaaaacccccgggtcattccttccttccgatgcccaggtaggtatcgatgattcgctggtcgtgcatcaattcgcgcgcgttgccgtcgagcgccacggcgcccatctcgagcacgtaggcgcggtctgccacctgcaatgcggcgcgcgcgttctgctccaccagcagcaccgagacgccgtggctgcgcaactgcgaaaccacgcgcagcacttcgcgcaccaccagcggcgccaggccgagcgagggttcgtcgagcatcaggagccgcggacgcgccatcagcgcacggccgatggcgagcatctggcgctcgccgccggaaagcgtcgaggccagctgcgggcgccgctcgcgcaagcgcggaaagatctcgaacacctcgtccatgcgcgcgcgctggtcgcgcttgcccttgcgccactggtagaagccgcccagcagcaggttgtcttcgaccgacatgtcgccgaacagctcgcgccgctcgggcaccagcgccacgccgcgcgccaccatggtctccacgcccggccgcgcgatgcgttcgccatgcagcgcgaggctgccggtggacggcagcaggcccatcgtcgcgcacagcaacgtggtcttgcccgcgccgttggggccgatgacggtgacgatctcgccttcgttcacatgcagccgcacgccgtgcaccgcttcgacggcgcggtaggcgacgcagaagccgtcgagttcgaggataggagtgctcatctcgcgtcctccagcagttcgtcgtccgcgccgccaagataggcctccagcacgcgcgggttggcctgcacttcggccggcgtgccggtcgcaatcacggtgccgaattcgagcaccgtgatgcggtcggcgaggttcatcacaaattccatgtcgtgttccaccaccaggatgccgaggccttcggcgcgcagctgccccagcagcacggagagcgcgcgcttctccagatgccggagacccgcggcgggctcgtcgagcagcagcacggagggctgaccggccagggcgcgcgcgatttcgaccacgcgctgctggcccagcgagagcgatgcggccggcgtgtcggcatgcgcgccgaggccgcagcgctcgatctggcggcgggcttcggccatcagtgccgcttcctcggcacggtccagcctgagcatggcggcaagccagccacgcttcgcgcgcaggtgcgcgccgagcgccacgttctcgaccacgctgcgctggccgagcaggcgcacgtgctggaaggtgcgcccgaggccgagcgccgcgaacacgcgcgaaggctttgctgtcatcgtctggcccgcaagccgtacttcgccggcgctcgggtcgtccacgcccgagatcatgttgaagaaggtgctcttgcccgcgccattcggtccgatgagcgcgtggatctcgccggctttcagcgtcatcgagatgtcgttgttggccaccagcccgccgaagcgcttgctgacgctggtggcctggagcagcacctcgcccttggcgggcaggttgcgctgcacaagctgcatggtggaggtcgcaggccgcgcggcatcgggtgcagcagccgcatgcgggcgcacccagcggcccgcgattcgcgccagcgtgggccacaggccttctgcaaaacgctgcagcacgaacagcatgagcagcccgaacacgatcacttcgaagtttccgctgctgccgagcaacgaaggcagcacgtcctgcagcttctccttcagcagcgtgatgagcgcggcccccagcaccgcgccccacaggtggcccgcaccgccgaccaccgccatgaacagcagctcgatgccgatgttcaggttgaaaggcgtggggttcacgaagcgctgcaggtgcgcatagagccagcccgacacggcggcgagcagggccgcgagcacgaagagcttcacgcggtggcgggctgtatccacccccatcgattcggccatgagccggccgcccttcagcgcgcggatggcgcggccctcgcgcgagtcgagcaggttgtgcagggcccagagcgcaagcagcagcacggcccagatcacgacgccgagtgcgcgcggcgtggccagcgagaagcccgcgatgaccagcggcggcacgccggtgatgccggtctgcccgccaaggaaatccatgttgccgaacaggtagtacaggctcaggccccaggcgatcgtgcacagcggcaggtagtggccctgcagcttgagcgtgaccgcgcccagcgcccatgcgagcgcgaaggtcagcaacaggccgagcagcagccccgcccatggcagcaaggcgggcgccacgaagccgcccatccacgccgccgcggcgggcgaggtgcagatccatgcggtggcgtaggagcccacgccgacgaatgcggcctggccgaacgaggtcatgccgccgacgccggtcagcatgaccaggccggccgcgaccagcgcatagagcccgatgttgctgagcacagaaaccgtgaactcgggcaggaagccccaggccagcgccattgcgacgacgagcaccagcgtgagctggcgcgaggtgaccagcggcttgccagcgggcggcaggtgggcggtgatgggattcgacggagcgctcattcctcgtcctccacatggcggctgtgcagcgagcgccaccacagcaccgggatgatcagcgtgaagaccagcacctccttgaacgggctggcccagaacgaagcaaaggcttcgagctgcccgaccagcagtgcaccggccagcgccagcggatagctcgcgagcccgcccacgatggcggcgacgaagcccttcaggccgatcaggaagccggtgtcgtagtacaccgtggtgagcggcgcgatcaacaggcccgacaccgcgccgatgagcgccgcgagcgcgaagctcaggtcgcccgacaactccgtcggaatacccgacagccgcgcgcccacgcggttgatggcggtggcgcgcagcgccttgccgaccatcgagcggccgaagaaaagaaacattgcaatcaccagcagcagcgtgatgccgatcaccaccagcgactgcccgctgaccggaatgccgccgatgtcgaagcgctcttccgagaacgcggtggtgcggtagccctcggcgccgaagaagagcaggcccagtcccaccagcacgccgtgcagcgcgaccgagacgatcagcagcatcagcacgctggcatccgccagcggccggtaggcgagacgatagagcaacggaccgagcggcgcgatcagcaccagcgtggtgatcgactgcgccgccatcgaagtcggcttgagccccaacacgagtgcagaggccagccccggcagcgccacgcaccaggtgagcgccgagccccagtccaccaccgtgccgcgcttccagcgccaggcttccaccaccagcaccatggccgcgagcgcgatcagcagccacagcgtggccggcacgcggccggtctgcagcatggccatcgacagcgcgccgaaggcgacgaactcgccctgcggaatgaagatgacgcgcgtgacggagaacaccagcaccaaggcgagcgccatcaatccatagacggcaccgttcacgatgccgtcctgccccagcaaaagggcgatctgcagatccataaaaaaccttcgggctcggcccttgtatcgaatcagtgtttgccgcaaacgcctacagccacgctgcattgctccttccccctttgggggaaggttgggatgggggcagcccctgcgttcacgccgcgtggacgtctatgccggcgtgcccccaccccaaccctcccccaaaggggagggagccgggatccttcagggctggtatttccaggcgccgttttcgatcttcaccatgacgcgggcgcgttggtccaggcccagatggtcgttggccgtcaggttgaatacgccgtgagcgcctgcaacgtccttcacctgctccagcgcgtcgcgcagcgccgcgcggaactcgggcgtgccgggctgcgcctttttgagtgcgaccggcacggccgaggtcatcaggaggcccgcgtcccaggcgtgcgcgccgaaggtcgacaccgtgttcttgccgttggcaccctcgtaggcggtgacgtaggccatggccgatttcttcacgggatggctggccggcagttgctcggccacgagcacgggaccggccggcaggaaggtgccttccacgtccttgccgcccacgcgaaggaagtcggcattggccacgccgtgggtctggtacatcttgccggtgtagccgcgctctttcagcgtcttctgcggcagcgcggccggcgtgcccgagcccgcgaccagcaccgcgtcggccttggcggccatgatcttcaaggcctggccggtcaccgaggtgtcggtgcgcgcatagcgttcgttggcgacgatcttgagcttcttcagttccgccgccttggcgaattcctgcgaccaaccttcgccgtacgcatcggagaagccgatgaaggccaccgtcttcacgccgttggcggccatgtgttcggcaatggcgagagacatcatgatgtcgttctgcggcgtcttgaagacccactgcttcttggggtccatcggctcgacgatgcgagctgaggcggcgatggaaatcatcggcgtcttggcttcgctgaccacgtcgatcatcgcaagcgagttgggcgtggtggtcgatcccagcacgatgtcgaccttgttctcggcaatgagcttgcgcgtgttggccacggccgccgtggtgtcggaggcgtcgtcgagcacgatgtagttgatcttctggccggcgatggtcttgggcatcagcgcgatggtgttcttttcgggaatgccgagcgaggcggccggaccggtggccgagagcgtcacgccgacattgatgtcggcccatgcggccacggcggtggcgcacagcgctgcgatcagcaggggcttgaagaatttcatttgggtttgtctccggttgaaaagttgttatggggtcagcgctcgtcgaaggacagggtcacgcgttcggtgagagggtgcgcctggcaggtcagcacgaagcccgcggctacttcattcttgtcgagtgcaaagtttctttccatgcggacttcccccgccacgagcttggcgcggcaagtgccgcacacgccggaggtgcaagagaacggcacctcgagcccggccgcggaagccgcgtcgaggatgctcggctgcccttcggtgaaagtgatctctcgctgcaggccgtcgcgcacgatggtgatgcgcgcctgcttggcatcgccgggcagggcctcgtgcaccaccgcgccgacctcgccggccgaagcgccggaaggcgatgcgacgccgaagcgctcgatgtgaatacgctcttcgggcacgcccgcggcgagcagcgccgcttcggcctcgtcgttcatctggaacgggccgcagatgtacacatggtcgatgcctgcggccggcaccagcgtgctgaggaactcgccgatcttctcgcggttcatcacgccgaagcccagcggcgaatcggtgtgctcgtcggagaacacgtgctgcagcacgaggcgcgtcatgtagcggttcttcaggtcctcgatttcttccttgaacatcgtggagtgcaactggcggttgccgtagatcagcgtgaagcggcttcggggttcgcgcgccagcacggtcttcatgatcgacaggatcggcgtgatgccgctgccgccggcaatgccgacgtgatggcgcgcggaagccggctcgatgggtacgaagaagcggccctgcggcgccatcacctgcaccgtgtcgccgggctgaaggtgcgcgttgatccagttggagaacacgccgtcccgcaccttgcgcacgcccacgcgcagctccccgtcgtcgaggccggcgcagatcgagtacgagcggcgcaggtcctgcccgtcgatgtcgcggcgcaatgtgaggtactggccctgcgtgaagccgaagacttcccgaagctcgggtggcacctcgaacgagacgacgacggcctccgaggtgtcgggctcgacagccttcacgcgcagcgggtggaagagggtgctcatcgcttagatcggcttgaaatgttcgaagggttcgcggcagcccatgcagcggtagagcgccttgcaggcggtggagccgaaggcggacaggcgctcggtgcgctcgctcgcgcagcgtgggcaggcgatgctttctttcacgccggcgatgcggccgaagaggcggatgggcatcgcggtgccggcggccgcttcgggggtgaggtgagccggcggcgcgatgccataggccttgagcctggctcggccttcttcgctgatccagtcgctggtccaggccggcgcgcggcgcaaggtggcgcgtgcgcggccaaggccggcgttctcgatggcggcgagcacgtcgtgctcgatggcttcggtcgcggggcaacccgagtaggtgggcgtgagcacgatctccagcccgtcgtcatgttcgatcacctcgcgcacgatgcccaggtcgcagaccgacacggccggcacctcgggatcgggcacggtgtgcagcacggcccaggccatgtcgacgcgcgatgcgacggtgttgttcaccacacacccccggggtaagagcgctgcaggtgctgcatctcggccaggatgtagcccatgtgttcggtgtgaacgccctgcttgccggtgctgcggaaggcggcctccttcggcatctcgaggccggcggcgtcgagcacctgttgcatctccgagaaccagggctcgcgcagctcgctccacgcggggccgaggcctgttgcgctggcttctgcatcgacggcatcgctctcgaacagctccggcacgtagagccagagctgcttcaaggcgcgctcggtgcggcggcgcgattcgtcggtcccgtcgccgagccgcacgacccagtcgcccgagtgctgctggtggtagcgcgcttccttcacggccttgccggcgatggcggccacctcggcatcgttcgatgcggcaaggcgttgccacagcagcttgagcagcgtggcgaccatggtgttgcgcaccacggcaaaggcgaagtcgccgcgcggcagttcgacgagcgtgaggttgaagtagtcgcgctcgtcgcgaaggtaggcgagctggtcttcgtcatgcgcatgtgcagcaccctcgagcttgccggcgtgcgtgagcagcgcgcgtgcctgccccacgaggtcgagcgcgatgttggccatcgcgatgtcttcttccagcacgggcgcatggccgcaccattcgcccaggcgctgcgcgagcaccaggcaggtatcgccgatgcgcagcaggtattgcacggcgggggtgcggttcagttcgatagaggcttgcattcagtggctccaactctgtcttgctccctctccccatggggagagggtgggggtgagggcgtgggcggtggaagaaacctgtcggtagcgaaggccggcggccctcaccctgaccctctcccagagggagaggggacaacacgaagtccattcgcgggctctcatcacggtctcacatgtggtcgactgacttgggcagcgaatagaacgtcggatggcgatacaccttgtcctccgccggatcgaagaacatgtccttgtcacccggatcgcttgccacgatctggtcggagcgcaccacccagatgctgctgccttcctggcggcgcgtgtacacgtcgcgcgccatctggatcgccatcttcggatcggccgcatgcaggctgccgcaatgcttgtggtcgaggccggccttgctgcgcacgaacacttcccacaggggccactcttgttggatatcggcgctcatgcggcctccttgatcggttgcttgttggcgtgggccatcgcggcttcgcgcacccacgcgccttcttcccacgcgtcgacgcgggcctgcaggcgctcgcgattgcacggaccgtcaccgccgatcacgcgccagaactcgctccagtcgatggcgccgaagtcgtgcgcctgccgctcttcgttccacttcaggtcggggtcgggcaaggtcacgccgaggatgcgcgcctgctcgacggcggcgtcgatgaacttctggcgcagctcgtcgttgctgaagcgcttgatgccccagcgcatcgactgcgccgaattgggcgactggtcgtcgggcgggccgaacatcatgatcgagggccaccaccagcggttgaccgcgtcctgcaccatcgccttctgcgcctcggtgccacgggtcatcatggtcagcagggcttcatagccctggcgctggtgaaaactttcctcgcggcagatgcggatcatggcgcgcgcatacggcgcatacgagcagcggcagatcggcacctggttcatgatggccgcgccgtccaccagccagccgatggtgcccatgtcggcccaggtcagcgtggggtaattgaagatcgagctgtacttggccttgccggtgtgcagcgcgtcgaacatctggtcgcgcgaagtgcccagcgtctcggcggcggcatacaggtagagcccgtggccgccttcgtcctgcaccttggccagcaggatggccttgcgcttgagcgtgggcgcgcggccgatccagttgccttcgggcagcatgccgacgatctcggaatgcgcgtgctggctgatctgccgcaccagcgtcttgcggtagtgctcgggcatccagtctttcgcctcgatgaaatcgccggcgtcgatgtgcgcgtcgaagcgctcctcgagccgcatttcgtcagccgagcgcacggctttcttcttgccgtcgtcgcctgcatccttgcccatggtgtccattgcctgggtgtacatgtgcgtgtcctttgaaaaaaggttgtgttggaacggcgcgcgctcagcgcgggcgcgtgtcgatcacgcggcgggccttgccggtctgcgtgcgttcgatggaatcggggttgaacacgcgcaccgccgtcgagatgccgaccagcgtcttcacgcgttcctgcacccaggcggcgatggccttgcgctcggcctcgtcgatggcggcgttgcggtggtcgagttcgcagtgcacctcgacctcgtcgagcaggccgtcgcggcgcacatgcacctggtagatgccagacagatgctcgtgcgcgagcacgatttcttccacctgcgtgggaaagacattgacgccgcggatgatcatcatgtcgtcgctgcgcccgacgatctttcccatgcggcggaaggcgcgcgaggtcggtggcagcaggcgcgtgaggtcgcgcgtgcggtagcgcacgatgggcatggcctccttgctgagcgaggtgaagaccagttcgccttcttcgccgtcggccttcaactcgcccgtgtcggggtcgatgatctcggggtagaagtggtcttcccagatcaccgggccgtccttgctctcgacgcattcgctggccacgcccgggcccatcacttctgagaggccatagatgtcgaccgcatcgatgccggccttgccctcgatgtcgcgccgcatggcttcggtccaaggctcggcgccgaagatgccgatcttgagcgagctgtccttcgcatcgaggccctggcgttcgaactgctcgatgatcacctgcatgtagctgggcgtgaccatgatgatgtcgggcttgaagtcctggatcagctgcacctgcttctcggtctggccgcccgacatcggaatgaccgtgcagcccgcgcgctcggcgccgtagtgcgcgccaaggccgccggtgaagaggccgtagccataggccacgtggatcatgtcgcccgcgcggccgcccgcggcgcggatggagcgcgcgacgaggtcggcccaggtgtcgatgtccttcagcgtatagcccacgacggtcggcttgccggtggtgcccgacgacgcgtggacgcgcgcgacctgcgtgcgcggcacggcgaacatgccgaagggatagttgtcgcgcagatcgctcttcaccgtgaacggaaacttcgacaggtcggcaagcgacaccaggtcttccgggtgcacgcccttggcatcgaaggcgctgcggtagtgcggcacgttgtcgtaggcgcgctgcagcgtggcgcgcaggcgccggatctgcagcgcggtgatttcgtcgcggcttgcggtttcgatgggttcgagctcaccgggcgcgggatgtctggctgtcatggtcttgtctcctcaggcggcaacggcggggcggcccttggcggtgtaggagcggccgcgaaagatcgcgatgcgctcgccgcgctgattggtgatttcggcgtcgtacacgccggtgcggccggcttttgaaacctcgaagcagcgcgcggtgagcacgtcgccttcgcgcgccggcgcaatgaagtcgatcgagaagcccgaggccaccgtcagctcgttgtacgagttgcaggcgaaggcaaaggtggaatcggccagcgtggccatgaagcctccgtggcagatggcatggccattgagcatgtcggggcgcacgcgcatctcgagcgtggcctcgcccggtgcgatttcgacgatgcgcatgccgaggcccttgctcgcgttgtcgttcgcgaacatgccgtcgcggacgtactccgcggtttgctggggtgtgcgggtggtgtccgtcatggcttcagcggtccttgaaaaccggcgcgcgcttggcgcggaaggcctcgacgccttcgcggtagtcgttggcgttgcccaggtcgcgctggatgcgggcttcttcggccagtgccgtttcaaggtccgagtcctgcgccgcagtcatggcgagccgcgtggctatgagagcgcgcgtcggcatgcccgccagcttcagcgcgagcgcggcggccgtctcggccagcgccgcgtcgtccacgcactgccagatcaggccgatgcgcgcggcttcttcggccggcagcttgtcgcccagcatcgcgatccccagcgcgcgcgccgagcccacgagccggggcagcagccacgtgccaccggtgtcgggcacaagaccgatcttggtgaaggcctggatgaagctggccgagcgcgcggccaccaccaggtcgcaacacagcgcgatgttggcgcccgctccggcggcgacgccgttgacggctgcgatcacgggcacgggcatcgagcgcaggcgcgctaccagcggggcgtagtaagtggagatgacgtcgcccaggtccttgggcgcggcaccgggcgcggggtcgggcgcgaccgcagggtcggcgaggtcctgcccggcgcagaagccgcggcccgcacctgtgagcacgacgcagcgcacggtctcgtcacgcgccgcaaggtcgagcgcggccatcaactcggcatgcaactccgtcgtgaagctgttgagcgccgcggggcggttgaggctcagcgtgcgcactgcgccggcattgctggtgagaactaaaggttcaggcatgggcttggctctcatccttgaagaggggtgaatcggcctgcaaacactattgaccgaccgtccggtagattttaagatcgtctcccgtgacgacacaagcgggttgagtcggggcaaaccctgagcccgcatccaaggagaccgaacgaatgcccagctactccatcgacggcgtgattcccgtcgtcgacccgacggcctacgtgcaccccagcgccgtcttgattggcgacgtgatcgtcggccccggctgctacgtgggcccttgcgccagcctgcgcggcgacttcggccgcatcgtgctggaggagggctccaacgtgcaggaccattgctgcatccacggctttcccgaccaggacacggtggtcgaggtcaatggccacatcggccacggcgcgatcctgcacagctgcatcgtgcggcgcgacgcgctggtgggcatgaacgcggtggtgatggacgaggccgagatcggcgagcaggcgatcgttgcggcctgcgccttcgtgccggccggcatgaaggtgccggcgcgctcactggtggccggcattcccgccaaggtgaagaagatgctgagcgacgaggaaattgcctggaagctcgaaggcacccagacctaccaggcgctgaccgtgcgcagcctggcaagcctgcgcgaagtggcgccgctggctcagacggagccgggccgcccgcgcctgcccgccacggacgtgcgctcgctgattgcgacccggcgcggttagccggcgcgcttcatgcaagatcgagggttgcccgcaaccgccaatcaaggaagaaagaagacccgatgccgcgtggaagatccgccacctacgacgaccagcgtgaactgatcctcgcgcaggccgcccagctgttcgcgcgccgcggctacccggccacgtcgatgaaccaggtggccgaggcctgcaatctctcgaaggccacgctctaccactactacagggacaagagcagcctcctcatcagcattgccgagacgcacgtctcgcggctggccgcgctggtggccgaggaagaggcctcgacccacaccgacgaagagcggctgcgccgcttcatctaccgcatcgtcgaggaatatgcgggcgcgcaagacgcgcaccgcgtgctgaccgacgacgtgcgctttctggaagaagccgaccgcgaacgcgtgctcgaccaggaacggcaggtggtggcgggctttgcacgcgcggtgtcggccttgcgtcccggcgctccgagcgacgacctcgccaagccgctgaccatgctgctgttcggaatgatcaactggatgttcacgtggatgaagcccggcggccggctcgaccatgcgtcgattgcgccgatcgtggccgacctgttcctgggcggcatcggcgcggtgaaggcgcctgcgccgcgcgccgatgcggcgccgccggcaaatcggccggacgcggtcaaagaatccggttgaaccagagcagcgacagccccgccgacagcagcgtgagaatggccgcgccgagcgcgaagagcgcggagacctcggtttcctttttctcgaccgtgagccgcgagctcagcgtttcgtacaccttcttcaggtcggcggcggtgccggcgtagaagtattcggcctgcgtcttgttggccacggccttgagcgtttcctcgtcgagccgtacgcgcatcgaccagccttcgaaaccgatggtctcgccatcgaccgtgcccacgcccaccgtgtagatgcgcacgccgcggtccgccgcggccttggcggcgtcgagcggatcgacgcccgtggtgcgctggccgtcggtcagcatgatgatggcggccgaggtgtaggagcccggcgccaccggcgtgaattccttggcctgcttctccgtctggtcgatgggcgtgccgcgctggcggcttggcgcgctgaactgcgagacgtcgatgcccgcgtcggggaacaaggtggcgagcgacaccacgatcgcattgcccgtggccgtggcgcgctgcagctggaagctgtcgatggcggtgatcaggtcgtcgtggttggttgtgggcaactgcgccacctgcgcgctgcccgcaaaggcgacgatgcccactttcacatgccggggcaggtccttgatgaaggtcttggccgcctcctgcgccgcgaccaggcggttgggcagcacgtcggccgcgcgcatgcttccggaaacgtccatcgcgaggatgatggtctgctggttcgacggcagcatcaccacggccaacggccgcgcggccgccaccagcatggcggccatggccaggaggaacaggaaaggggggatgtgccgtcggatgctctggccggtgcccatggcctcgcgcacgatcgacaggctcgcatagcgcaccgccagcttcttcttgcggcggatcagccagaggtagagcaacaccagcagcggcagggccgccagcaaccaaaggaattgaggccagagaaaagtcatgctgccaccgccttcactccgctgatgccgatgcgcgtgcggcgcttgcgcatgtcggcaaatcgaacgatggcttccaccaggtcgtcactggtcgaaagctcgagcgcgtcgacgcccgcccttgcgagcgaggcgcgcagggttgcttcgcgctcggccgccaggcgcgcaaagcgcttgcgaaagcccgcatcgtgggtgtcgacccagagctgctcgccggtttcggcatcgcgcagcggcaccaggccgaggtcgggcaggtcgagttcgagcgggtcgaacaggcgcacggcaatgacctcatgccgctgcaccagttggccgagcgggcgttcccagccgggctcgctcagaaaatcggacaccacgaagacggtggaacggcgcgtcatcagtgtgccggcggacttcagcaggtcggccagccgcgtcatgcctttttgcgtgggcgcggcctcgatcttgtcggcgcggcgctccatggcgtgcagcaggtgcagcacatgccggcggccactgcgcggcgggatcacggcctccaggtcggtgccgtagaccagcgcgccgacccggttgccatggcgcgtgagcagtcgcgcgagcacgccgacgaagccggccgagatctcgcgcttggccctctggccggatccgaaatcgaccgagcggctcaggtcgagcacgaaccacgcggacatctcgcggtcttcggtgaagacgcgtacatgcggcgtttgcagccgcgcggtcacgttccagtcgatgtggcgcacgtcgtcgttgtgctggtattcgcgcaggtcggccaggtcgaggccggtgccgcgcatcagcgtgcggtagtcgccctgcagcaggccgtccaggcggcggatcaccgtccattcgagccggcgcagcgcgcggtctgtcccgccggcttcagcgatgagccgttcgtcgttcgcggccgcgggggccttacgccaccagcttttcatgttcgagcggttttgggggagcggggacggccttcatgatcttctcgatcaggctgtcgggggtgagcccttcggacaagccttcgtaggaaagcgtcacgcgatggcgcagcacgtcgggcaccagcgccgtcatgtcttcgggcagggcatagctgcggccgcgcagcagcgcaagcgcgcgcgcgccttcggtgaggctgatgctcgcgcgcgggctggcgccgaaggtgatgaagcggcgcatgtccttcaggccgtgcttgtcgggcgtgcgcgtggcggagaccagcttcacggcgtactggatgagcgaagggtcgacgtacacgcgccgcgcctcggcctgcaactctgcgagctgttcggtggtcgcgaccgggctggcgccgacttgcgggccgatcacgcgctggacgatgacgaactcttcctcgtcgctcgggtagtcgaccagcaccttcatcatgaagcggtcgacctgcgcctcgggcaggggataggtaccctcggtctcgatggggttctgcgtggccatgaccaggaagggccgcggcacccggtgcgtttcgccggcaatggtgacctggcgctcctgcatcacctcgagcagcgcgctctgcaccttggccggggcgcggttgatttcgtcggccaggagcaggttggcgaacaccgggccgagcgaggtgctgaactcgccggtcttctggttgtagatgcgtgtaccgaccaggtcggccggcaccaggtcgggcgtgaactggatgcgcttgaactggccgcgaacggtgtcggccagcgtcttgacggtgagcgttttcgcaaggcccggcacgccttcgaccagcaggtggccgcccgcgagcatggcgaccatcacgcgctccaggaagcgatcctggcccaccaccacccgcttgacctcgtagaggatctgctccatcagctcggccgtggcggaagacgtggaaaagggggtctcggtgctcatgcgatggtctctcttggatgaatgaacgatcgaaagctggtacgtggtgcaggtcctgcgttcctagaacggcggcgaaccggcggccgaggccgcgttttcaatcggcacagcaaatccgatgccaatgaaggtgcgctgctgcgtgggattgaggatggcggtgacgatgccgagcacctcgccatccatgttgatcagcgggccgcccgaattgccggggttggctgccgcgtcgaactggatcaggttgccaagctcctgcttgccctcgggcgagcggaacgagcgcttgaggcccgacaccacgccggccgatacagatggcccgatgccgaacggaaagccgaccgccgccacctggtcgccgggctgcagatcgccggtcgagcgcatcaccgcgggaatcaggtcgtcgggaatcttctgggcctgcagcacggcgaggtcgttctcgggctgcacgccggtgatggtggccacggcttcgagcccgtcggagaacgtcaccttgatggtttcggcgccggccaccacgtgcaggttggtcaggatcacgcccttgtcgacgatgaccacgccggtgccaacgccgcgctcgacttcgcccggcggggcgtcggcttcaggcggcttgccgttggccagattgcggccgcgcttctggatcttggcctcgggcgtggctttctcggggccgtagccgaccacccgtacgatggagggccgcacgatttcggccgccttcgcggccggggagggcagcgtctgggtctgcagcgtgcgcagcaccgccgcatcgatgtccttttgcgtcagcgccttgacgctgtgccggggccaccaggtggcgccgccggcagcgagcgcggcgctcagcaccaccatgaacgcaaaactgcgccggcccggctgccagccggccttggcgggttttgcagaagaaggaggaggggagtctggagaaccgggcggcgcgccgttgcctgcgccctcgggcgatggcacggcagcctggtcggccgtggagtcggccgcttgcggctgcgtgccgggcgaacggctgtacaaagcgggcctgcgcatcggggcacctccggcaagggatgacgggtgatcagggagtcacagtagcacgctttcttctgccttgcatcccttcgggcatcatctcgccatggctgcattcgtcgatacccactgccacctcgatgcgcccgaattcggtgcagagatgccagtcatccgcgcacgggccgccgagcggggtgtggcactgtgtgtcattcctgccgtggccgtcttcaactttgccacggtgcgcgaactggcgcgggtgcaaggcgatgcgtacgcgctcggcatccacccgctgtgcaccggcgacgcgcaagagtccgatctggaaacgctggacgccgaactcgccgcgcgccgcggcgatccccggctggtcgcggtcggcgagatcgggctcgactacttcgtcccggggctcgacagcgacaagcaagagcacttttttcacactcagttgcaactcgcgcgcaaatacgatttgccggtgctcatccatgtgcgccgctcggtcgacaaggtgctcaagcatctgcggcagaccgcgggcggccggccctggcggggcattgcccatgcattcaacggcagcgagcagcaggccaaggcctgcatcgacatcggtctgaagctgggcttcggcggcgccgtgaccttcgagcgtgcgttgcagctgcggcggctggccgccacgctgccgctcgaatcgatggtgatggaaaccgatgcgcccgacatccagccgcactggatctaccgcacgcaggcacagcgcgcggccggcgaaccgcagggccgcaacgaacccggcgaactgccgcgcattgccgaagtggtggcgaaattgcgcggcatcggactcgacgagttggcccaggccaccaccgcgaatgcgcttgaagcgctgccggcgctccaaagtcttctccccttgtcggaagccaggccgcaccacgcgtaggccgatgtcccgtattgcggttgcgcaagcggagcgtgcctttttactgtcatccttggtgttcgacgtggcgttgcttgttcagtggcaactccgtcactccaacacttcatccaaaaggagtcttcacatgagcagatctttcattcgcaccgtgcccgttgtccttgccctcgcgcttgcctccatcggcgtttccgccgtggcgcaaaccgcggcgcccgcaaccgccgaacccaccaccactgaaaaggtgaaggaagccggcaaggacgcggtcgatgcgaccaagactacgaccaagaaggccgtgaatgccaccgaacgcggcaccaagaaggcctgggacgccaccaagcgcaccaccaagaaggccacgaccgccaccaagaatgccgccgtcaagactggcgacgctgttgaaaccgccggccacaagacggccgacggcatgcgcagcaccggcaaggcgatcggtgaaaaggtgcccggcacggccgaaaacgaagccgccaagaaataatcggccttcgccttcagcacaaacccgcttcggcgggttttttcatgggcggtcgacagtgccaagatagagcccattcatgaatccaccagccgcacccgacgcgggcagcgcggtgttgaccggccttgcgcccatcgtctcgcccgctaccgccgtactgatcctgggcagcttcccgggcgctcgctcgctcgagctgcagcagtactatgcgcatccgcaaaatcagttctggaaaatcttgcaagccgtttggcccgaccacccgctgccgaccggcgcagacagctacgtgaaaaagaaggcgtggctgctcgaccgcggcctgggcgtgtgggatgtgtacgccgcctgcgagcgcgagggcagcctcgactcggccattcgcgcacccgtggccaacgacatcgccgggctgcacctgccgcggcttgctgccatcgtgcacaacggcggcgagagcttcaagcatgcgcgccacacgcgcaccctgggcgtgccggtctaccagctgccctccaccagccccgccaacgcgtcgtggagcttcgagcgcaagctcgcagcctggcgcgaggtctttgtcgcccaccaccttctttgatggccacgagcaaaactcccgttctccccgaagtcaatttttccgactggggcgacatccgctacctgcatctcgggaccgaatgggtccagggctccatgaagctcgatgcgcctttcgaaatcgagctcgaatacgtgcagcgcatgatggcctggctgctgttcgccgaccccaagagcgtggcaagccgccacgcgatgcagctcggcctcggcgcggccacgctcaccaagttctgccgcaagaccctgcgcatgcggaccaccgcggtcgaactgaatccgcaggtggtgtcggcctgccgcggctggttcaaattgccggccgacgatccgaagctgcgcgtggtcattgccgatgcggcgctggagatccgcaagcccgaatggcatggcacggtcgatgccctgcaggtcgacctgtacgaccatgaagcggctgcgccggtgctcgacagcgaagatttctacgccgattgccgcgcgttgctcaccgaagacggctgcatgacggtcaacctcttcggccgctcgtcgagctacgagcgcagcctggagaaaatcgccggcgcattcgggcccgatgcggtctgggccttcaagccgacgcgcgaaggcaacacggtggtgctggcgcagcgctcgccgagccgcccgaagcgcgaagcccttgccgagcgcgcccaaacgatccagactcgatgggccctgcccgcgcctaaatggctgcgtgtcttcaaaccgctgaatcccactctcacccgaccttccggcccatgagcgctgttcccgctgtttccgcccccgccccgctggccgcgcgccacgaaggcccgctcgacctgcgccgcctgatcgaatggctcgccaccgacggcgtgatctctccagtggaagccaagcgcaccatcgcgcgctgcgcccaggccgagagccggcaggcgccgctggtgcggctggccaacgtggccatgacgcgcgaaagcgacggcaagccgctcgacctcgaaatgctcacgcagtggctcgccggccgcgcggggctggcctacctgcgcatcgatccgctcaaggtcgacgtgggcaaggtggccgacaccatgagcgcggcctatgccgagcgccacaaggtgctgccggtgcaggtgctgcccaatgaggtggtggtggccacggccgaaccctttctcaccgactggatcgccgaagtggagcgccagtcgcgccgcacggtgcgccgcgtggtggccaacccggccgacatccagcgctacacggccgagttctttgcgcttgccaagtcggtgcgcgccgcgcagaaggccggcggcaacaccggcggcgcgagcttcgaacagctggtcgaactgggcaagagcaccaagcagctcgacgccaacgaccagagcgtggtgcaggtggtcgactggctctggcaatacgccttcgaccagcgcgcgagcgatatccacctggagccgcgccgcgagcagggcgtgatccgcttccgcatcgacggcatcctgcacccggcctaccagatgcccatgggcgtgatgaacgcgatggtctcgcgcatcaagctgctgggccgcatggacgtggtcgagaagcgccgtccgctcgacggccgcatcaagacccgcaacatgcgcggcgacgaggtcgagatgcgcctgtccaccttgccgaccgccttcggcgagaagatggtgatgcggatcttcgaccccgacacggccgtgaaggacctcgacgcgctcggcttcgcgcagcacgatgcgcatcgctgggagcagctcgtcacgcggcccaacggcatcatcctggtgacgggccccacgggttcgggcaagaccaccacgctgtactccacgctcaagcgcgtggcgaccgaagaagtcaacgtgagcacggtcgaagacccgatcgaaatgatcgagccctcgttcaaccagacgcaggtgcagccgcagctcgacttcggctttaccgaaggcctgcgcgcgctgatgcggcaggaccccgacatcatcatggtcggcgaaatccgcgacctggccacggccgaaatggcggtgcaggccgcgctcaccggccacctggtgttcagcacgctgcacaccaacgatgccccgagcgccatcacgcggctgatggaactcggcgtgccgtcgtacctcatcaatgccgtgatgctcggcgtgctggcccagcggctggtgcgcaccctgtgccccaactgcaagcagcccgacgacacggtcacgcgcgagaagctcgaaaccatcgtcaagccatggcagatcaccggctcggtgcgcgcctacaagcccgtgggctgcgtcgattgccgcatgaccgggtacatgggccgcatgggcctgtacgaactgctgagcatcagcgaagacttcaaggcccaggtcaccaaggagccgaacctcgcagggctgcggcggcaagccgtgatcgacggcatgcggccgttgcgcctggcgggcgcgctgcgcgtggccgaaggcgtcaccaccatcgaggaagtgctgagcgcgacccctccgctcgagtgagggccgatggcccgagccctgggggttatccctagcccttcggttagtggaatccacatcgggctgaccaccggctgactcgacaatctcgcatcgaaatttgttcgaggagactgttcgtgaaaatcaagagtcagaaagactttttctcgggcctgatgtttacggtcgtaggaacggcgttcgcatggggcgccaccacctacagcgtaggcaccggcgcccgcatgggaccgggttacttcccgttgatgctgggcatcctgatggccgtcattggcctggggatcatgttcagtggcctgacggttgaaaccgccgacggcgaaaagatcggcaagtgggcctggaagcaggtggtgttcatcctgggcgccaacctcgcattcggcatcttgctgggcggcctgccgagcatcggcgtgccggccatgggaatgatcatcgcgatctacgcgcttgtgatcatctcgagcctcgcgggccacgagttcaagctgccaagcgtgctggtcctggccacggcgctggccatcggcagctatgtggccttcatctgggcgctcaagctgcagatccaggtctggccgaccttcatcaccggttgagaaagcgcgcaaatggaattgtttgaacacctctcgatgggttttggcgttgcctttaccttcaccaacctgctgtactgcctggccggctgtattttgggcacgctgatcggcgtgctgccgggcatcggcccggtcgcgaccatcgcgatgctgctgcccgccacgtacgcgctgccgcccgtgtcggcgctgatcatgctggccggcatctactacggcgcgcagtacggcggctcgaccaccgcgatcctggtcaacctgccgggcgaatcgtcctcggtggtgaccgtgatcgacggctaccagatggcgcgcaagggccgcgcaggccccgcgctcgccgctgccggcctgggctcgttctttgcgggctgcgtgggcacgctgatcctggcggcctttgcaccgccgctgaccgagctggccttcaagttcggcccggccgagtatttctcgctgatgatcctgggcctgatcggcgccgtggtgctggcctcgggctcgctgctcaaggccatcggaatgatcgtgctgggtctcctgatgggcctggtcggcaccgacgtgaactccggcgtggcgcgctacagcttcgacattcccgaactgaccgacggcatcggcttcgtggccattgccatgggtgtgttcggctacggcgaaatcattgccaacctctcgcgccccgatgacgagcgcgaagtgttcactgccaaggtctcgggcctgttcccgaccaaggaagacttcaagcgcatgcttcccgcggtgttgcgcggcacggcgctgggctctgcgctcggcatcctgcctggtggcggtgcgctgctggcagcttttgcggcctacaccatcgagaagaagaccaagctgcagccgggcgaagtgcccttcggcaagggcaacatccgcggcgtggcggctcccgagtcggccaacaacgccggcgcgcaaacctccttcatcccgctgctgacgctgggtattccgcccaacgccgtgatggcgctgatggtgggcgccatgacgatccacaacatccagccgggcccgcaggtgatgaccagcaaccctgagctgttctggggcctcattgcctcgatgtggctcggcaatgcgatgctgatcgtcttgaacctgccgctcatcggcatgtggatcaagctgctgtcggtgccctacaagtacctgttcccggccatcgtgcttttctgcgccattggcgtgtactcgaccaacaacaacaccttcgacatctggatggtgggcatcttcggcctggtgggctacaccttcttcaagctgggttgcgagcctgcgccgctgctgctgggcttcatcctcgggccgatgatggaagagaacctgcgccgttcgctgctgctgtcgcgcggcgactggagcgtgttcgtcacgcgcccgatctccgccagcctgctggccgccgcggcgctgctcttggtgatcgtgctgctgccggccgtcaaatcgaagcgtgaagaagccttcgtcgaagtcgactgagcctcgcgcaccctagcgaaaaaacggcgtcttcgggcgccgtttcttttttcagggcttggcagcgcgtggcgggctcatgtgctgtcttgccatcgcgaggaaggccatcgccgccgggctgaggggatgcttggccaggcggatcgcgaccaccgggtactcgaggacagggcgtgtcacggccacggcgcgcaggttgcccggcatcaacacctcgacgtagcgcggcagcagcgccacgcccgcgcccgcctggatgagcccgaacgccgtcgacagcatcgacacgtggtgcaccacgcgcggatagacgttggccacgctcgagagctggcggctgacggcgcgccacacattggcatcgggattgacgtggatgaagggcagcgcctccaggtgtttggcgtcgaccaccacgcgctgcgccagcggatggtcgtcgcgcacgaacagggccatgcgttccgagaaaagcggctcggtcgccagctccgagtgcttctgcccgatgtcggagccaaagcccaggtcggcctcctgcgagaggatgcgcgagatcatctgctccgccgtgctgtcgagcagcgtggtggcgagcgtgggatgcttgcgggaaaagcggccgagcatcggcggcagcagggcgcccgccgtgaggtggcccaccgccagcaccacccgcccttcgcgcaactgcgattgcgagcggcaggcgtccacggattcatcgatgagccgcagtgcacgcacggccgtctcgaccatcacctggcccgcgctcgtcaagcggatgcggcggccccgcaccaccagcggctgcccgagctcttcttccatgcgcttgaccaggtggctgatggcgggctgggtcagctgcagggtttccgccgcgagcgtgaagctgcccgattcggcaacggccgccagcgcccgcagttgctgcagcgagatttcttccgaggcgtttcttgtcataaacagcgctcatagttgaataagcagaattatctggcttgatgtccggccgctgcatagcatgcaagctttccaccggggccagaattcagaccatgaaacgaatccagttccttcaaggggttgccgttgcgctctgcatggccgcatcgacggccagcctggcccagggctacccgaacaagccggtgcggctcatcgtgccgttcccggcggccggcgccacggatctttttgcgcgcaccctcgggcagaagatgagcgaaaagctgggcgccacgctgatcgtcgacaacaagccgggcgccggcggtgccatcggctccgacatggccgccaaggcgccacccgacggctacacgctgctgctggccaccaccagcacgcattcgatcggcccctccatcaccagcaagctgccctacgacacggtgcgcgacttctcgcccatcgcgcacgtgggcgatgcgccgagcatcatgctggtgccggtcgactcgcccgccaagacggtgcgcgaatggatcgcctacgcacagaagaaccccggcaagctcaactacgcgtcgagcggcaacggcaccatcgtgcaactcaccgccgagctcttcaaggcgcaggccggcgtgttcgtgacgcacattccttacaagggcaccgcgctcgccattcccgacttgatcagcggcaaggtcgacgtgctcttcgactcgctgcccaccggcatgccgcacgtgcgtgacggccggctccgcgcactcggcgtcaccacgctgaagcgcagcccgctcgcacccgaactgcctccgatcgcagacacgctgcccgggttcgagtcgaacacctggttcggcttctatggcccgaagggattgccggcggacatcgtggcgcgcgtcaacaaggccgccaacgaggcgctggccgatcccgaagtgagagaaaagctttcgcgcctgggcatcgaacccgcggctgccggaacgcccgagcagttcgcgaagatggtggccgcggacgccgccaagtggaaaaaaatcatcgtcgagcgcaagatcagcaacgaatagcaagcactttccaatgaacttcgacttcagcaatccctacctttccacccgcattccaatctttgcgcgcaacgtggtgtccacctcgcacccgctcgcctcgcaggccggactgcgcatgctgcagcaaggcggcaatgccgtcgatgcggccattgccacggcggccgtcatgaccctggtcgagcccgtgagcaacggccttggcagcgatgccttctgcatcctgtgggatggcaaggagctgcatggcctgaacgcctcgggtcccgcacccaaggcctggacgccggaatacttcagggccaagtacggtgccgacgccgccacgccgcccatgcgcggcatcgattcggtgaccgtgccaggcgcggtgcgcggctgggttgcactgagcgatcgcttcggcaagctgcctttcgccgacctgctggcgccggccatcgacatcgccgagcgcggctacctggtgccgccggtggtgcagggcaagtgggccgcagccacgtcgctgctgcagtcgcagcccggctttgcgcagaccttcctgccctggggccgcgcgcccgaggtcggcgagctgttccgcttcaccgcggcggcgcgtgcgctcaaggccattgcccgcaccaagggcgaggcttactacaccggcgagatcgccgaggcgcttgcaaagttctcgaccgagcagggtggctcgctcacggtggcagacctctcggcctaccagcccgaatgggtcaagccgatctcgcgcgactaccgcggccacacgctgcacgagattccgcccaacgggcagggcattgcggcgctgatcgcgctcggcattctcgagaaattcgacatcgcgtcgctgccggtcgactcggtcgcttcacagcatctgcagatcgaggcgatgaagctcgcctttgccgacgtgtaccgctatgtctcggagccatcgtcgatgacggtgaccccggcgcaaatgctcgatgactcctacctcgcatcgcgtgcgaaactcatcgacgtgaaaaaggcgcaggacttcaaggccggcaaccccgtgaagggcggcaccatctacctcacggccgcggacgagagcggcatgatggtgagcttcatccagagcaactacatgggtttcggctcgggctgcgtggaacccgaattcggcatcagcctgcagaaccgcggccacggcttcagcctcaaggccgagagcccgaacgtcgtggcaccgggcaagcggccgttccacaccatcatcccggccttcctcaccaaggacggacagccggtgatgagcttcggcgtgatgggcggcaacatgcagccgcagggccacatgcagacgctggtgcgcatgctcgactacaagcagaacccgcaggctgcctgcgacgcaccgcgctggcgcttcaacgcggggctcgagatcaacgtcgaggccgcgatgaacccgaacaccgtgcagggcctgcgcgagctcggccaccacctcgatgtgatcgacgactcctaccaggacttcggcgccggccagttcatctggcgcgcgggcgatccgtcggtggaaggctacgtcgccgccagcgatccgcgccgcgatggcgtggctgcaggcttttgaaggccgcgcaatgatgatcgagggatgaacaagtccgccgcacagaccggctttccctcttcagcaagcggcgcaaaaaagagcattggggccggcctcgtccttgcctcgctgggtgcggtcgctttcagcggcaaggccatcatcgtcaagctggcctaccgctatggcgtggatgcgatcacgctgatcatgctgcggatgctgttcgcgctgccgctgttcgcgctcatggcgtggtgggccggccgcggcaagcctgcactcaccttccgcgactggctcggggtggtcgggctcggcttctcgggctactacctcgcgagctttctcgacttcgcgggactcgcctacatctcggcgagcttcgagcggctgatcctctatctcaaccccacgctggtgcttctgttcggctggctcctgtaccggcgccgcgccacgcggccgcaggtgctgggcatgatcgtgagctatgccggcgtgctgctggtgttcgggcacgagctctggatcggcagcggcggcaagggcggcggggcggcggcctggggcgctttcctggtgttcctgagcgcggtgagctatgcgggctacctcgtctacagcggagagttcgtcaagcgcctggggtcgctgcggctcgtggggctggccaccaccgtggcctgcgtgctgtgcatcctgcagttcgtgctcacgcggccgatgagcgtggccatgcaggtggcgcccgaggtgatctggctctcggtgctcaacgccacgctgtgcacggcggtgcctgtcctgatggtcatgatggccatcgagcgcatcggccccgccatggccgcgcaaaccggcatgatcgggcccttgtcgaccatcctcatgggcgtggtcatactcggcgagccgttcaccgcgtggatcgcggccggcacggtgctcgtgattgcgggcatcttcgttttcacacgcacggggcgctagcgcccctgcagatcaggagcaacaaaaatggatctgggcattgcaggcaagaccgcgctggtgtgcggcgcgagcaagggtctcggctacggctgcgccgaagcgctggtgcgcgaaggcgtgaacgtggtcatcgtggcacgcggcgccgaggcgctggaagcggcagcgaagaagctggccgtggcgaccgtcgcggccgccggttcgccaacgcctttcgtcaagcacgtggccgccgacatcaccaccgaagccggccgtgcagcggtgttcgcgctgggccatgacttcgacatcgtcgtcaccaacgccggcggtccgccacccggcgattttcgcaactgggaccgcgaggcctggatcaaggctgtcgatgccaacatgctcacgcccatcgagcttatcaaggccacggtcgacggcatggccaagcgcggcttcgggcgcatcgtcaacatcacgtcgagctcggtgaaatcgccgatcgacatcctcggcctgtcgaacggtgcgcgcagcggcctcaccggcttcgtggccggcgtggcgcgcacgcccatcgcggcgcagggtgtgaccatcaacaacctgctgcccggttcctttgacaccgaccgcctcaagggcacgatggccggcgcggcccagaagaccggccaggatttcgacaccgtgtgggaagcccgcaagaagaacattcccgccaggcgcttcggcacgccggccgagttcggcgccatctgcgcttttctctgcagcatgcaggccggctacatgacgggtcagaacatactggccgacggcggcgcctacccgggcacgtactgagctcgcccacaggggagctggtgaatcagcgccgcgacgacaccacgatcccgcccacgatcagcgcgaatgccgcgccgtggtaccagtgcggcggctcgcccaggaaggccgcggacaagagcgcggcgaacagcggcgtgaggttcatgaagaagctcgccgcctgcggccccgcatgctgcacgccgctgccccagcagcgataggcgagcaccgcggggccgatgccgatgaaggccagcgccgcgaacagcggccagccgggcacgatgcgggcgtcggtcagcgtccattccccggccgcgaacacgcccgaccacgcgaggccgaacaccagctgcgccatcaggaacgcggcccagtcctgccgcacggcctgcggctcgcgcgtgcgcgccagtatccaactgtagaaggcccaggcgatggtgcccaggatcatgtagagatcgcccggcaccagccgcagcccgagcagctgccgccattcgccgcggctcagcaccagcagcacgcccagcatcgaaagcagcgagccgccgatctcgcgcgcgctgatgcgggcaccgaagaagatggcgcccgtcgccagcatccacagcggcaggctggagcccaccagcgtgacgttgatcgggctggaggtctgcagcgccaggtattgaaacgcgttgtagcagccgatgccgagcagccccagcacggcgtagcgcttccagtgcgcccacaaggggctggtcggccgcaccaccggccatgcgagcggcagcagcagcgcgaaggcgatgacccagcgcacgaagttcagcgtgagcggcgacaccaggtcgcgcaccagccggccgaccacggcattgccggcccacagcagcggcggcacggtgagcaggaggatggtggaaggcgtgaggcgctgctgctgtgtctgcatggccgccgactctaccgggcattgccctctgccgccgcggcaaggccaaacgtggcaggatgcgcttcttcttttttccgcgtgcctggagactgcaaaaatgatgagcaaagccgtccgtatcgaccgccacggcggtcccgaagaactgaagatcgtcgacgtggaggtcggcgaacccggccctggtgaaatacgcatccgccacaaggccgtgggcctgaatttcatcgacacctaccagcgcagcgggctctatccgttccagatgccgctgcagctgggcatggaagcctcgggcgtggtcgaggccgtgggcgaaggcgtggcgcacctcaaggccggcgaccgcgccgcctacgcgagccagccgcccggcgcctacagcgagctgcgcgtgatgccggccaagaacgtgtgcaagctgcccgacgccatctcgttcgagaccggcgcagccatgatgctcaagggcctgaccacgcaatatctgctgaagaagacgctgccggtggagggcctgcagcccggcgacttcatcctctttcatgcggcggccggcggcgtcgggctgatcgcctgccagtgggccaaggcattgggcctgcagctgatcggcaccgcgggcagcgacgccaagtgcaagctcgcgctcgaccacggcgcggcgcatgccatcaactacagcaccgagaacttcgcggcccgcgtgaaggagatcaccggcggcaagggcgtcaaggtggcctacgactcggtgggcaaggacacctgggaaggctccatcgagtgcctgcgcccgttcggccttctggcggtgttcggcaacggctcgggccccgtgccgccgatcagcctcggcacgctggcctccaagggctccctctacgtgacgcggcccacgttgttcacgcacatcgcaacgcgcgaaagcacccaggccatggccgacgacctgtttgccgtggtgcagagcggcgcggtgaagataccgatcgaccagcgctatgcattggccgacgtacagcaggcgcatcgcgacctggaagcgcgcaagaccaccggctgcaccatcctcacgctctgaagccgtgcacggctggcgcgccgatggcggcgggccagccttgtcctaccctcggtggggtgtcatgccttcgtcttgccaagagtgcactttgtagccttcaacaaagttgggaaggccagcgccatggacaccgtcagaaccttcatcgtcgaggacaacccggccatccgcgaagccctggccggcacgttgcgcgaagtggcccgggtcgatccggtgggtcaggctgagacggaactcgaaggcatacgctggctcaccagcaatctgtcgcagtgggatctggccgtcgtcgacctgttcctgaaggacggcacgggcttcagcgtgctcgaagcctgccgcaaccgcgagcccacgcagaagatggtggtgctcagcaaccacctgacgccggagacgcgccgcaaatgcacgcagctgggcgccgatggggtgttcgacaaggccaccgagatcgatgacctggtcgacttctgcctgcgccgccggcaggaatcttgaagccggtcagccttctatttttcccagccgcgattcgcgcagccggcttggggccagtgcacccgccgtctccaggatagggtaggcgatggagcagatgtgcgagttgatccgcttcaggtcgctgatcaggtcgatgtgcagcgagctggtttcgatgctcagcgtggtgcggtcggagagccggtccaggtgggtggtggcataggcccgttcgaggtcgcgaaagcgggctttttcttgcagcagcttttgcgcatcgcgcacattgccgttgagaaagacgctcatgctcagccgcaggttggccaccagccgcccatgcagttcgacgatttccgccatgcccgcttcggagaagttgcgctgcggcttgatcttcttgtcctcgatgtcgatgatcacgcgctcgatgatgtcgccgatctgctccatgttgatggtgaagctgatgatgtcggtccagcgccggctttcttcctcgcccagtgcctcgcgcgagatgcgcgtcatgtagtacttgatggccgagtagagctcgtccaccgtgtcgtcgagctgccgcagttcctgcgccaggcgcaggtcgttgtggcggatcacgtcgagcatgccgatgagcatggtctccaccacgtcggcctggtgcagcgcctcgcgcgcggcattcgaaatggcgagcgaaggcgtcgagagcgccgacggatcgaggtggtgcggccgcatggaagtggcaggctgctgcggcaccggcagcatcttcgtgaccagcgtggccacccattgcgtgaggccgatgaagcccacgctgatgaccacgttgaacgccaggtggaacagcaccacgccgtgggttgcatttggcacgtgcggctgcacgtagcgcagccagagcccgacgaatggcgtgacgatggcaacgcccagcgccttgaaaagcaggttgcccatcgtgacctgccgcaccgacacggccgacttggccgtggtcagcaccgccagcaggccgctgccaaggttggcgccgagcacgagcccgagcgcgacgtccagcggcaccacgttggaactggccatggccgccaccagcagcaccacggccaggctcgagtacgccatgatggccagcgcggcgccgatggtgatttcgagcagcacgtcgctggtgagcgaggccagcaacgcacgcatggccggcgcggagaacaggggttcggtggcttccaccaccagctgcagcgccagcagcatcaggcccaggccgatgagcacccggcccacccggcccgccatgctggccgagcgcgaaatgaacagcaccacgcccacgaagatgaacatcggcgaaagccaggacaggtcggccgagaacagcaccgcgatgagggctgtgcccacatcggccccccgcatcaccgccagtgccgccggcagcgtgaccagcccctgccccacgaaggaggaagtcatcagagaggtggcggtgctcgactgcaccagggccgtgacgccgatgcccgaaagcgcggccgtgaagcggttgcgcatgctctgcaccaggatcttgcgcaggttggcgccgaacacgcgcagcacgcccgtgcgcacgaggtgcgtgccccacaccagcaatgcaacggcggccagcaggttcaggagatgcttcatggggggcgggttctatccttttcgtttcggttcgttttcgaccccattttccacatctgtgggctcagtcgatcagtgcgccgttgtcatggaacggaaaagggccctcgaacgtgccggaagccgccaaatgggtcacaagccttcggttccgtgcggaccaggcgtggacccggaagccgggcggctccagtgtccaggccgagggcgcgttggccgaaaggtccaggcagacctggtgcgccggcgcgggcgaggtcgatgcgatggtgccgccaaagcgcacgtcgatggcacggtgcaggtggccgcagatcacgcgctcgacgttgccatgtcgcgcaaccagcgcttccagagcctcggcgccctgcagcaggccgatctcgtccatgtggccgatcagcgtctggaaaggcgggtggtgcatggcgatgacgacgggctcgccgcggctggcgtcgagctgttgttccagccaggccaggcgctcgtcgcacagggcgccgtggctctcgcccgggacgcaggtgtccagcgtgagcaggcgcagcgcgcccacgcgcaccgaatactggatgaagccggccgtgcccacgcccggcgtcagataggcgtggccgggaaagctgcggcgcaactggtcacggtcgtcatggttgccgggcatcaggtagaccggcatcgcgagcggcgccagcaggcgcgccaggtgctcgtattcggcggcgcggccgaagtcgctcaggtcgccggtgatcacgacggcgtcgggccgctgcggcagccgcagcaccgactgcaccgcgcgctccaggtagggcgcggtgtcgatgcggccgtaggccaggcgtcccggctcgcggatgtgcaggtcggtgagctgcacgaggaaagtgctgttgtcttctgccgttgtcgtcatacgctggtctcctgcgacgtcatcaggcggtcgggctggatgcgaagcccgaccggatcgcccgggccgaacggcgtgtcgcggcctacatcggccgtcagcaagggctggtcctgcaggcgcagttgcaattgcacgcggtcgccgaggaaggtgcggcgttcgaccgtggccgcaccccagtcgggccgcggcgcgctcacttcgacgtcttcgggtcggaccagaagcatcgcatggctctgccaggcgggtgggcaaggcagggtgcttccgccgagtcggacaatgccttgcgcaatggcgtcggcctcgcgttccagccggttgacccggcccaggaactccgccacgaagggatgcgccggcgcgcggtacagatcctcgccgcggccgatctgcacgatgcgcccggcactcatcaccgccagccggtcggcaatggccagtgcctcctgctggtcgtgcgtgacgtggatggccgtgatgtgcaaccggcgcagtagctcggccagttcatctcgcagcgactccttgagcttggcgtcgagcgcggccaagggctcgtccagcagcagcacgcgcggacgcacggccacggcgcgcgccagcgccacgcgctgccgctggccgcccgaaagctcggcggggcgtttgttctccaggccgtcgagccgcgtcaggtcgaccagttcgccgaccgcgcgcctttcttcttccggcgccacgccgcggatgcgcaggccatagccgatgttggccgccaccgtcatctgcggaaagagcgcgtagctctggaacaccatgcccacgccgcggtgctccaccggccggtcggtgacgtcctggccgccgaacaagatgcggctgccttcgtcgggtgcctcgagccccgcgatcagccgcagcagcgtcgtcttgccgcagcccgaggggccgagcagggcgagcacctcgccggcctccacgtgcaggtcggtcggcaacaggccgcgcgtgccgtcggcataggtcttggcgcagcgcgagatgtcgatgggaatgcgttcaagttccatggcgtttctgcatcaggttggcaagatattgcaggccccacagcatcgggagaatgactgcgaagaaaaccagcgtgtaggccgatccgatctcgatgcgcatcgacgcatagctgtcggccagccccacgggcagggtgcgcgtgagcggcgtgtgcagcatccaggtgaggttgaactcgcccaccgaaagcgtgaacaccatcaggctgccggccacgatggccgggaacacggcgggcaccaggatgcccatgaagcgctggcggaagttcgcgccgagcgagcgggccgcttcctccagcgcgagcaggtcgtcacgctggaaggccgaactcaccgtgcgcaccatgaacggcagcgtgaacaccatgtggcccacgagaatgaaggcgaagctctggcggaaggcggtgagctggccgtaggcgaggatgagcgccagcgcggtcgcgaggcccggcaccgcgaccggcagcgtcagcagctcctcgaagatgtgcgcggcccgcgagcggctgcgcgccagcgcgtaggcgcagggcacgcccagcagcacggtgccgaccacgcaggccagcgcgagtgcaagcgaccagccgacggtgccgccgtagttctcccacacctcgccgagccagcgcagcgtgagcccgctcttcaggcccgcgctgtagttgttgaccaggcctgccatcaccgacagcagcatcggcgcgatcatgaagaggctcaccagcacggtcacggcgaggaggaagggtgccttgggttgcatgttctttcgcatgaagcgtttccttcagcgcgccaccggattggcgccgaagcgccgcgccgcgaacagcaccagccaggtcacgaggcccagcgcgatcgacagcgacgcggcgagcgcgaagttggcgtagttggtgaactcgttgtagatggtgatcggaatcacctcgaacttgctggccagtgtgaacgcggtgccgaaggcgcccatcgaggtggcgaacaggatcgcgccgcaggcgagcgtggtgggcgcgagctctggcatccacacgtcgcgcgccacccgcaggcgcgaggcgccgagcgagcgcgctgcctcttcgagctgcacgttcatcgcctcggccgctgccgcataggtggcgatggcgcgcggcagcgaaaagtacaggtaggccaggaacagcccgagcaggccgtaggcaaaggtgatgcgctcgccgaacaggctgtcgccgatgtcggccaccagcccttgccgaccgccgagcaggatcacgaagaagccgatgatcacgcccggaaaggacagtggcagcgtgagcagcgacagcagcatgcgcttgcccgtgaaggcatggcgcgcgagatagatgcccacggccgcgccgagcaccagcgttgcgagcgttacgcccaccgacagcgccacggtgttggccatgctctgcaggtagcgcgcgtcggtgagcactgcaaagtaagtggcccaccctttggttgcaggtaatgtgagcaggcgcaccactggcagcagccagaaggccgcgaagaacacggctgcgggcgctgagcaagcgagcaggcgccagcgtgggttccaggcgttgtcgggtttcatttcagctgtgcttgtgtttggagtgctgctgttcagggcgcgtgtgaaggccaccgggtactcccctccgcgaatgtcccccgccttcggctcctcctttatttcgctgcggggagcccccggcgccctgtgcacgccgggcgcggctgtcgtgctggccgatcaaccagtgccctgaacaacgatcccgctggcggggtgccttgcgcagcgaaataaaggaggagcccgaagggcgggggacattcgcggagaaaggtacgccgtcggcgggagcgcgccctgaacacaacaagatcagcgcacttccttcagataccgatcagagaacgaccgttgcgcctcagccatgcgcgcgtagtcgacgctctttgcgcgggcatattcggtagcaggcaggaactgcgcttctacgtccttcggcattgcaccggcgcgtaccggccgcaggtacgccttggcccagatcgcctggccttcgtcggacagcacgaagtcgagcaccttcttgccttcggctgcgtgcggcgccttggcgacgaggctcatcacgtagggcacggccagcgtgccttcgctcgggatgacgaaggcgacattggccttgtccttgtacttggcgcggtaggcgttgaagtcgtagtcgagcaggatcgcgatctcgcccgacagcacgcgcgcgtaggaggtctgcttgggcacgatgggctcgttcttctgcagtgccttgaagtagtcgatggccgggccgaagttgtcgagcgtgccgccgcgcgcctcgttcacggccaccgcgccgacatagccgacaaaggccgaggcggggtcgagatagccgatgaggcccttgtattcgggcttgagcaggtcggcccacgacttcggaatcggcttgcccttgagcgcatccacgttgaccatgaagccgagcgtgccggagtggatggtgaaccagttgccggcagggtccttcaggccatcgggaatgtctttccaggcggccggcttgtagggctcgaccacgccttctttctgcgcctgcaccgcgaaggtcacgcccaggtaggtgacgtcggccacggggctgcctttttcggccacgagttgcgcgagcgactggcccgagttcttgttgtcggccggcacggtgatgccggtcttggccttgatggccttgagctgcgtgccccagtcggcccattcggtggggcagttgtagcagatggcggtctgggccatgacgctgcctgcggcaacgagcgtggcggcgagcaagcccaggcgggccatgcgggagatgcggagggacatgaagaactccttggatggatgtgagaggcggaagcggggtgatcagtcggtggcgatgtcgcacgcggatgcgcacgattcgccgtcgcggaagaagtgaggcagcagcagactcgcatcggcctgcagcgcggtaccgccggccatggcctggatcagcaactcgacgctgtggcggccgatgtcgctgttgggctgcgcgatggtggtgagtgccggcgtgaggtcttcgccgagcgcaatgccgtcgaagccgaccacgctgagatcgtggggcaccgagaggccgctcaggtgcgcggccctgatgctgcggatggcgagcaggtcgttcgagcagatcagcgcggtgggacgggtcttggcctgcagcaagtgcgcgagcatgtccactgcgctttcgacaaaaggtacttcgatgagcggcggcgcatcgagcccggcatcggccatgcctttttgataaccccggtagcgctgttgcgcgcggtcggacgcggccagcgtgccgctgaccatcgcaatccggcgatgccccagaagcacaaggcgtgcgacggcatccgctacggcagcttcgccgtcgacggtcacgcagggatggtcgggatgccggttgtaggccagcacataaggcgtgtcggtggtgcgaagccgtgcgagggccgccgaagtggaggggttggagaccacgaggatcagcccgtcgacattgccggcaagcagcaggtggactgcacgctcttcttcgtcgagctggtagcccgtggtcacaggaatgatcgcgtagccgcctgcgatggcggcacgtgcgatgccttgcaggcactcggcaaaggtcggattcagaagcgtgggaagcacgacacccaatgcacggctgcgctgggtgcgcaaagtgcgcgcgctggcattcggcacatagtgaagctcgcgtgcgacgcgttccaccaactcccttgtagcgggcgtgaccttgtcggggaaattgaaggcccgcgacacggtggccacggagaccccagccttggctgcgacggattgaatgctcatcgtgcggtgttatgtaatcgattacatttcaccgcggcagtatgaccccgctatgacaggcaagaaagccgggaaaaaccctcgcgtggggtttgctccctctccctctgggagagggttggggtgagggcaggcggcctctaacgaatgaccaactacttcccccgccgaacccgccggatctcgtccaggatcaggcagatggcacccagcgtgattgcactgtcggccgcattgaacgccgggaagtaccagttgccggcgtggaagctcaggaagtccacgacatagccgtgcatcatccggtcgatcacgttgccgatcgcgccgcccaggatgcaggccatcgagaacgaaaacagcttctgccccgcgtgcgacttcagcatccagacgatgaacaccgcagccgccacgccaatggccgtgaagaaccagcgctgccatcccgaatggtcggccaggaacgagaacgcggcgcccgtgttgtgcgcgcgaaccacgttgaagaagctcgtcacataggtcgcgtcgccgagcttgtaatagcccaagatcagcgtcttggtgaactggtcgatgatcaggatgatcgccgccagcccgagccatggccagatgctgccgctgcgggaacgcgatgccgacatggtgcgtgcggccgccatcaggcaaagctccgcgattcgccggcgccgaacaggttgctcgtgcaacggccgcagatcgtcggatgcgccgggtcgtggcccacgtcgtcgcggtagtgccagcagcgatcgcacttctgcgccgtgctcggcgtcaccacggtagacagggtttcgctcgccgccagttcaatggcggaagcgatgaagacgaacttcaggtcgtcgccgagcgtgcccagcagcgcaaggtcgtccgccggtgcgctgagttgcaggttggcctgcagcgacgagccgaccttgccttcggcgcgcaccgcctcgatgtccttgttcaccacgtcgcggatctcgcgcaggcggctccacttggcgagcagggcttcgtcgggcgccgcgaattcgctgtacgtctgcgcgaagatcgactcgcccggcttgcccgtgctcacgaacttccacgcctcttcggccgtgaagctcaggaacggtgccatccagcgcagcatcgcttgcgagatgtgccagagcgccgtctgcgcactgcggcgagcgagcgagcccggcgccgtggtgtagagccggtccttcaggatgtcgagatagaacccgcccaggtcttcagagcagtagatctgcagcttggccaccaccgggtggaactcgtacaccttgtagtgcgcgaggatctcggcctggaactgcgccgcgcgcgcaagcgcatagcggtcgatctcgaacagctcgcccagcggcaccgcatccttcgcgatgtcgaaatcgctggtgttcgcaagcaggaagcgcagcgtgttgcggatgcggcggtacgagtcgaccacgcgcgccaggatcttgtcgtcgcccgcgatgtcgcccgagtagtcgctcgcagccacccagaggcggatgatttcggcgcccagcttgctgctgatttcctgcgggtcgatgccgttcttgagcgacttgctcatcttgatgcccttggcatccaccgtgaagccgtgcgtgagcaggccgcggtacggcgcgcggtcttccagcgcacaggcgatcaggagcgacgagtggaaccagccgcgatgctggtcgtggccttcgagatacaggtcggcttcaggccccgtctcgtggtgcacgttggggtgcgtgccgcgcagcacgtgatggaaggtcgagcccgagtcgaaccacacctcgaggatgtcggtgctcttggtgtagtgcggcgcgtcttcggcacccaggatttcttctaccgtgacacggctccaggcctcgatgccacccttctcgacgatgtcggcggcctggtcgaggatttccatcgtgcgcggatgcagctcgcccgagtccttgtgcaggaagaacgggatcggcacgccccagctgcgctggcggctgatgcaccagtcgggccggttggcaatcatgtcgtgcagccgcgccttgccgttctccggatagaagctcgtttgctcgatggcttcgagcgcggtctggcgcagcgacttgggcgccttgtccttggtgaacacgccctcgccttcgtccatgcggacgaaccactgcgccgcagcacggtagatcaccggcgtcttgtggcgccagcagtgcgggtagctgtgggtgatggtctcggtggtgagcaggcggttggcgtcgcgcagcgccgagatgatgaccggcaccgccttccagatgttctgcccgccgaagagcggaaagtcgggcgcgtagctgccgttgccctgcaccggattcaggatgtcgtcgtaggcgacgccgtgggcgatgcaggagttgaagtcgtccacgccgtaggcaggcgaggagtggaccaggcccgtgccgtcggtggcggtggcgtagtcggccaggtacaccggcgacaggcgcttgtagccagcatccacgtcgtacaacggatgctcgaactccaggccgccgagtttctcgcccttgaccgtggccagcaccttgccgtcgagcgcatagcgcgtcatgcacatctcgaccagcgaattggcgaggatcaggaggccgcgctcggtgtcgaccagcgaatactcgatctccgggttcaggttgatcgcctggttggccgggatggtccacgcggtggtggtccagatcacggcaaagatgtcgccgaggatcgtgtggtcggtctcgaaggccttgagcaccttctcgcgctcgtgcgccttgaaggccacgtccagggtctggctcttcttgtcggcgtattcgatttcgaactcggccagcgacgaaccgcaatcgaagcaccagtacaccggcttcaggccgcggtacacgaagccgcgctcgatcacgcgcttgaacgcgcgcagttcgccggcttcgttcgcaaaatccatcgtcttgtagggatggtcccattcgcccagcacgcccaggcgctggaagtcgagcatctgctgcgcgatctgctccgtggcgtaagcgcggctcttggcctgcatctcgtcgcggctcaggttgcggccgtactgcttttcgatggcgttctcgatcggcaggccatggcagtcccagccgggcacgtagagggcgtcgtagccttcgagctggcgcgccttggtgatcatgtccttcaggatcttgttcaccgcgtggcccatgtggatctggccgttggcgtacggcgggccgtcgtgcaggatgaacttgggggcgccgtggcgggcgtcgcgcaggcggtggtagcggccttcgtcgttccattccttcacccagcccggttcgcgcttgggcaggtcgccgcgcatcgggaagggggtgtcgggcaggttcagcgtggaacggtagtcggtgggggaagcggcgtcagacatgttggggtgcgaaacagaggggcttcgacaggctcagcccgaactgcattgagcggtcggtgcggaagaaaagccgttcgccctgagcttgtcgaagggcggcagcacggtgcgtgcagggctaaattcggtcgcgcgtcgtctggcgatgggtttcggcgtgggtcgatgcaaagaacgcgcgcgcgtcgcgcccatccttcgcgatgcccgcagtgagggcctcgaggctggtgtagcgcaattcgtcgtgcagtttgtgcaggagttccacgcggacgattttaccgtaggccccttcggctcccagatgcgagggccactccaggcaatgcgtctccagcaacacccgtcccgcgttgacgtcgttggcgtccagcgaggggcgcacgccgaggttggccacgccgggcagcggctggtcggccaggccgtgcaccagcaccgcgaagatgccgctggcggccggcttccagtgcttgaagcgcatgttgagggtgcgaaacccgtcatccctgcccggggccgaggcgcccagcgcgcggccgagcttgcggccatggaccacgtggcccgagatcgtgtacggccggccgagcagatgctgggcgtcggccatgcggccctcggccagcgcatcgcgcacggccgagctggaaacgcgcaagccatgcacctcgtagctgttcatgcgcgccacgtcgaagccatgcgtatcgccggctgcgtcgagcatggcgtagtcgccggcccgcttggcgccaaaacgaaagtcgtcgcccaccagcacgtagcgcgcgcccaggccgtcgatcagcacgttctggatgaattgctcgggcgactgggaggccagccggccgtcgaagggcagcacgatggtctgcgccacgccgcaggccgcgagctcggtcagcttgtcgcgcagcgtgccgatgcgcgccggcgccaggtcgggtttcttggtggcggcggcgaaatagtcgcgcgggtggggctcgaaggtaagcacgcaactgggcagcccgcggtggcgcgcctcggtctgcaacagcgccagcatggcctggtggccacggtgcacgccgtcgaaattgccaatggtgagggcgcaggccggagccacgcccgggtgccggaagccacggaaaacctgcatgggtggatatctttttgatagcgcctcgcgcccgtcaattgggcgaatcaggccgttttgtcacaaagccggtatattgtgactcagtgcgttgcctgaagtggtctccggcgcgctccgtgtccctggtctttccgtgattcttccctttttgaggaggcgtgtggtgaaggtcttgaagctgtcggcccaagggctgccccagtcatggatatcgctcgaacaggcggtcatccactatgcagcggacgaagtccgctgggaggtgggcgcgcaggtggctgtgttccgtggcggccacaacgccatcacgggcgagcaatcgcagattgcgatcaacagcatcatcggcaccaagggcgtgccgcgcatcaatcctttcacgcaacgcccggggctcaccaacagcaagctctttgcgcgcgaccgcaacgtctgcgcctactgcggcgggcatttccacgaagacgagctcacgcgcgagcacatcattccgttcgcccagaagggcatcgacacctggatgaacgtggtcacggcctgcaagccttgcaaccaccgcaagagcagccgcacgcccgagcaggcgaacatgccgctcctgtatgcgccctatgtgcccagcctctgggaagatttcattttgcgaaaccgccgcatcctggcggaccagatggaattcttgatggcgcacctgccgcagagctcgcggctgcacgacagttagcagctcgctcagcgcttccagtccggcgagcgcttctcgatgaaggcctggatgccttcgagcgcgctctcgtccatcatgttgcaggccatggtctggctggcgtcggccagcgcggcttcgatgccggtttcgagctggcggtagaagagggccttgcccagcgcaagcggctggcgcggcttggcgacgatgctggcgaccagcgcttcgactgcggcatcgagttcggccggcgcggcaacccggttgactaggcccttctgcttggcctcctgcgcatcgatgaactcacccgtcacaagcatctcgaaagcctgcttgcgcccgaggttgcgcgacagcgtgacgctcggcgtggcgcagaacagccccacgttcacgccgctgaccgcaaagcgtgcttcgctcgaggccaccgccaggtcgcacaccgcgaccagctggcagcccgcggccgtcgcgatgccgtgcacgcgcgcaatcacgggcacggcaaggcgctggatcgacagcatcatggcgccgcagcgttcgaagagccgctgatagtagccgagcgagggctccgcgcgcatttccttcaggtcgtggcccgcgcagaaggccttgcctgctgccgcgatgacgaccgcacgcacgctctcgtccgccgcgatgtctgcaatggcttgctcgagcgcgccgagcatgccctccgagagtgcgttgaacgaggccgggcggttcagcgtcagcgtaaccacgccgcgcgcatcgcgcgctttcagcacgaagggggaggccgcatcgttcatgtccgcagccctcagtaggtcaactcgagcaccgtcacgtgctgttgcgcggcgggccaggtcaggccggtgatgcgctcgctgttgaactcaccggtcaccgcgcgctggggctccgcggcggcaatgcgcaacctggaactcgacacgccggaacccttgggcggcacgcccgctggcgggctctggccgtcgagacgcatggtgtcgcgctgcgcgtcgaaatagccgcgagggcgcgtgaagacgacgaccgcctgggcattggcatcggcgggcgtgaggcgctcggggcgcaggttcacccaaccgctgctgcgtggaaatgcgctgcggtagatgtgggtgatgccatagcccggcgcgctaagaacgaactcgtaggacgtgtccccgcgcgcgctgaaagggccccatcggccgtcggcgccgatgttcctgctgtgcacggcgttgccgcgacgtgcacccgtggcggggtcgacggcatagacggtgacctggccgccattcagcgacaggttttccgcaccgatcgcgcggccgtcgagcacgacgttcgcgtcggccgcaatcgccgtgctgcgtggcggctcgcccgtgaggaattgccatgtcgccgcgaaggcggccggggagaacgaggtctcgcggtgatcgacgcgcggcagcacgacattggttgcgcctttgagcgcaggcccgtcgaagccgatgttcgtcggctggcccggcacgccgatccacagtccgtcgggctgcgcgtacttgtcgttgttgtcggagcgcagcgtgagccatctcacgcccggcgtgacctcctcgccgttcggccccttcggcgcattgagctgctgcatgaagccagagagccccgagaactcgttgttctcgcgaaagcccttcacgacccagatgccgtgcgccggattgccgcctagcaccacgtggctcaccgcatccgcgccgccgccgttctgcacgtagttgcggatcgtgttgccgccgcgcgagttgccgatcagcaccaccttgctggcgcccgtggccttcagcaccttgtcgacctcggccttcaggaagacggccgagtcggtcgtcgaactgcggcccggctgcgccacggcgtcgtcgtcgcgcgccaacggatagggctggtcgaccgcaaagagccggttgcgcggccagccgttcgattcgaaacgccagatcgtggtctgccagagcgcggccgagtcgccgttgccatgcatgaaaacgatcggcgggcgctcgctgtaagagggcgagggcgcggtggcgcaggccgtcagcatggcggtcgatgcgagcccgagggcaagaagggtgcggcgtgatggcatgtttttgttcctggctgaaggtccaagtaaaaacgcccgccggcgcaaagcgggcgggcgttggatgctatgagaaaaacatcgtcaggcgaagacgccagcggtgtcctgcatacgggcagacacttcgcccaggtggtgcagcgaatcgccgaaggtcatttcgagctgcgtgagcttgcggaagtaatggctgccgatgtattcgtccgtcacgccgatgccgccgtgcagctgcaccgagttggcggcgacatagcgcatcgacacgcccaactggtacttggcgcgcgccagcgcctggcgccgctcttcggccggcgcgttgagcttgagcgtggcgtagtagctcatcgagcgtgcgagctctagctgcatcttcatgtcggccacgcgatggcgcagtgcctggaaggtggagatggtcacgccgaactgcttgcgctggttcatgtagtcgaccgtcagggcgagcgtcttgtccatcacgccaacggcttcggcgcaagtggccgcaatgccgacgtcgaccgcgtactcgagtgccgccagcccgtcgatggtgatcagcgtggcgtctgccttgtcgaaaacgacctcggccgcacggctgccgtcctgcgtgccgtagccgcgggcctcgacaccgctggcgctgcgttcgacgagaaagagggcgatcttgccgtcggcctgcgcgggcacgatgtaggcatcggcttcgtcgcccacgggcaccacgctcttggcgccggtcagcgaccagccatcgccggccttcacggccttggcttcgcacacgtcgagccgatagcgcgccttgcgctcctggtaggccagcaccacgatggcctggccgcccgcaatgcggggcagccagttgtccttgatgtcctcgccggcatagccgctgagcaccgcgccggcaatcagcgtctgcgcgaagggctccagcacgatgccacggcccagttcttccatcacgaccatgcccgccacggggcccatgcccaggccgccgtcttcttcggcgatgtagaggccgcccaggccgagttcggccagatcgtcccaggcctcgcgcgagaagccaccaccggcctcgatgctgcggcggcgctcgaagtcatagcccttgtcgacccacttgcgaacggcgtcgcgcagttgttcctggtcgtccgagaaattgaaatccatgttcttgtctcctcagccgagaacggtttgagcaacgatgttgcgttgcacttcgttcgagccgccgtagatggtggtcttgcgcatgttgaagaaggtcgatgcgagcggcgcaagggccgggttgccgccggggaagtcgccttgccagccggcttccatcgcttcgcggatgagaggcagggaataggcgccgccggccagcatcatcagttcgctgtagcgctgctggatttcgctgccgcggatcttgagcaggcccgcgacgtcgagcgagttcttgcccgacgtagcggccgagagcacgcgcagcaccatcatctcgagcgcgacgatgtcgacttcgagcttggcgatctcgtcgcggaaacggaggtcgtcgtacacgccttcgctcttggcgatgcgcttcagccgctcgagttcacgcttggcgcggttcacgtcggcgatgttggtgcgctcatgcgaaagcaggtgcttggcgtaggtccagcccttgttctcttcgccgatcaggttctcggccggcacttcgacgttgtcgaagaacacctcgttcacttcatggccgccgtccagcagcttgatgggccgcaccgtgacgccgggcgacttcatgtcgagcagcagaaagctgatcccggtctggggcttgccctcgttgctggtgcgcacgaggttgaacatccagtcgccgtactggccgagcgtggtccaggtcttctggccgttgacgatgtacttgtcgcctttgcgctcggccttggtcttgaccgatgcaaggtcggagcccgaacccggttcgctgtaaccctggctccaccagacttcaccgctcgcaatgccaggaagaaaacgcttttgctgctcggcgttgccgaaggccatgatcaccggagcgaccatcaccgggccgaacggaacgatgcgaggcgcgccggcaagggcggtttcttcctcgaacaggtggcgctggatggcggtccagccggggccgccgaattccttcggccagccgtagccgagccagcctttcttgccgaggatcttggcccagccttgcaaatcgtcacgcgtcagttcgagcgcgttgtgcaccttgtgcgaaatctctttgggaaggttttccttgacccaggcgcgaatttcttcgcggaactgctgttcttcgggcgtgaagctcaaatccatgcgtgcctcgctgtgttgatcggtcgccgccatcgcgaagaaaagcggcttgtctccggggtttcgagttttagcacggtcgtgctgtgaaacggtgtccgcgcggcgacaagcagcccctcgcaccgtttttcgggcgcgccaggcggagcacagataatcccggcctcccatgaagaacatcgtgatcctgatctccggcggcggctccaacatggcggccatcgtgcgcgccgccgagcgcgaccgctggtccgagcgctttggtgcgcgcattgccgccgtcgtcagcaacaaggccgaggcgggagggcttgcgctcgccaagacgcacggcatcgaaaccgccgtggtcccgcacagggactatccgagccgcgaggccttcgacgaggcactggcgaaggtcgtcgatgcgcattcgcccgcgctggtggtgctggcgggcttcatgcgcatcctgacgcccgccttcgtcggccgctattcgggccgcctggtcaatatccatccctcgctgctgccggcatttccggggctcaacacgcaccagcgggccatcgacgccggctgcaaggtggccggcgtcacggtgcaccaggtgaccaccgaactcgaccatggcccgatcctggcccaggccgtggtgccggtgctgccggacgacactgcggccacgctggccggccgggtgctcgcgcaagagcatcagttgtatccacgcgccattgcggaatggcttgccgatacatcaagtcacataccttaaatttgtttatattcgcgggttttcgggagcatccattgaaaacccaatcgctactgtccacggtcgccgccgccgtcttgttggcggcttgcgccgcgccagcccctgcacccaccgctgcatccacatccgcatccgccgcggcggcggccgagccggtgtaccagtgcaatgcggatggcgcacggttcgctgtcggacagccgttgtcaccgcaactcgaagccgccgcccgcgtgcgcgccggtgcgggcacggtgcgggcactgaagcccggcgaagtggtcacgatggaactcaacggcggacgcctcaacctcgacgtggatgcgcgcggccgggtgaccgacgttcgctgcggctgaggctacgccaggatctggaccggggcgaagcgcaattggcgaattccctcgatctccacggtttcgccgaacatcgcggccgggcggacccagagtccccgggcgccataaagcgcgcggtagagcgtcatcggctccagggtctcgctatggcgcacggtgcccagcacctcgtattcgccgcccttgtagtggcgatagcggccgggaggcgtctctatcaggggtggcaggtcgttgtcattcacggcgttgcttctttcaaactgtggtgtccggttggaggaaagacggatggatcgcgctgattttgttcacctcgtccgactgagcgagcatgccagcgctgacgacagcgcgcgctaccggcgcaacgtcgcggcgtttgcagcgctcggctatgcctgggtgatggcctgcctggcgctgtcgatcggcatcattgcctgggtggcgctggccgccgggcgcggacgcttcggtttctcgcgcggctggctgctgctgtttgccttcggccttctctgggccacgctgcgcgccttgtgggtgcggttcgacgaacccgacggccgcgagctttcgcgcgcggatgcgccggcgctgttcgaggcactcgaccgcatccgcaagaagatcaaggggccgccggtccatcgcgtctacctggacgacgagttcaacgccagcattcggcaggtgccgcgcttcggcctgttcggcggggccgtcaattccctctccatcggcttgccgctcttgatgatgctggaccggcggcggctgctgtcggtgctcgcacacgagtacgggcacttgcgcggcaaccacggcaggctcagtgcctggatctaccgcacgcggctgtcgtggctcaagctggacgccagcctgcagcgcgacgaaagcgtgatggcgctcgtgtcgcaggcttttttccgctggtactttccgcgctttgcggcccggacctttgcgctcgcccggcaggatgagtacgaagccgaccgcatttccgggcggctcctgggcacgcccgtggcagcggccgcgctgacggaaatagccatcaagggcaactggtacgccaatgaattctgggcttcgcactgggcacgcgccgaacgcgagcctcagccgcccggtcccttcaaggcgctgcgggagcttgccgcaacgccgcccagcagtgaattcgcgcgccaggccctgcgcgaagccatgcggcgcgtcagcgacctcgacgacacccaccccgtcttgcgtgaccgcctcgaggcgctcggccagaaagccgtggtgccgccgtggtccaccgaaccggcgctgggcatgctcgccgacagcgcgaagtggatcgagcacttcgacaaccaatggcgccgcgcccacgccagcgactggaagcagcaccatgcgcaccggacgcgcatccgcgaacgcatcgaacttcttgccgctcggggcgagcgcaacacgcccgacgaaatggtcgagtgggccgattccgaacgccggctcgatccggccgcgccggtgcgcgagcgctatgaacgcgtgctgcggctcgcccccgaacatcccggtgccttgcggggggtggcccagatgctgcccacgcgagaccgcgatgcgcgcctggcggtgctcgaccgcttgcacggatccagtgcggccagccgctggtgggctgcgaaaaacgccgtggcggcgctcgaggatcccgatgcgggggcgcacgacgaggaagccctcaagctgtggcgcggccggctcaaggaggccgaagaagccgaggcgcgtgcctgggaagaaatcaccgaaacgcctttcttcagccagatcgtccggcatgacctgaacgaccatgagctgggcgaattgcgggctgacctgtcgcgctgcctcccgatctcgagggcctggctggtgcgcaagactttgcgcgagtttccgtggcgccgggcctacatcgtgttcgtcgacctgcccggcatggacgacgacgaccgctggcagctttgccggcaactcgagcagaccctgagcctgccgggggcggcgctggttctctgggccggccattcgccgacgctggaggacattgaacggcaggctttcgggacgatctggacgcgcacggcgtagggagccgcccggctgagacaatcggggcatgcaccccaaagccctgttggaggccaccgccgatctggtcggccttgtcctgaaattcgatcacccggccgaccaggtcgtttcgcgctttttccgcgaccaccgcgagttcggcccgcgcgagcgagccacgcttgccgagaccgtctacaccgtcttgcgcaagaagctcctgttcgaccatctctcgccctcgggcaccggttcaaaagagcgccgcatggcgatcctgggcttttacggcccgcgcgacttcttgaagagcgccctcaacgacaccgaaaaacgctggctcgacaactgcgatgccgtcaagcaggaagacctgctggagcgccaccgccacaacctgcccgaatggctggtcacgccgctcaaggcccagttgggcgacggcttctggccgttggtcgagagtttgcagcagcccgctccgcttgacctccgggtcaatgcactgaccgacaagcgggcagaagtgaaggcggagcttgccaaggctgctatcaaatctgaagcaaccccgttttcgccctggggcttgcgcatcgaaggcaagccggcgctgaccaagctggatgcttttgcgcgcggcgccgtcgaggtgcaggacgagggctcccaactgctcgcgctgctgctggacgccaagcgcggcgaaatggtggtcgatttttgcgccggcgcgggcggcaagacgctggcgattggtgccaccatgcgcaacaccggccggctctatgctttcgacacctcggcgcaccggctcgatgcgctcaagccgcggcttgcgcgcagcaagctctccaacgtccatccggccgccatcgcgcacgagcgcgacgatcgcatcaagcgcctggccggcaagatcgaccgggtgctggtcgacgcaccctgctcgggcctggggacgctgcgccgcaatccggacctgaaatggcgccagtcgcccaaatcggtcgaggaactgacggtcaagcaagccgccatcctgcaaagcgcggcgcgcctgctgaaatccggcggtcgtctgatttatgccacgtgcagcgtgctgccggaagaaaacgaggccattgccgaggctttcagcgcggccaacccggatttcgtgccgcaggacgcggcggaactgctgcagggcctcaaggtggagggtttcgagaagctctgcgccggcgggccggacggccgccgcttcctgcggctctggccccatcgccatgcgaccgacggcttctttgcggcggtgtggaaccgcaaataggcgcggcactccaaactagggtaaatctgcgcttttgtggaaggacaaaaggcctcattttggccttgtccccttaaaatcgcaggttaactgaaaggttgcaccttcgtgtggccatggagcacttaattcaatgttgattcctgactctgccgttttgagcgcggccatcgactggctcggacacggcttgtgggacctcacatggtggcaagtcgtgctgtacacgctcgtcaccacgcacatcacgatcgccgcggtcacgatcttcctgcaccgcacgcagacgcaccgggccatggatctggggccgatcccctcgcatttcttccgtttctggctgtggctcggcaccggcatggtgaccaaggaatgggtggccattcaccgcaagcaccacgccaagtgcgaaaccgaagacgacccgcacagcccgcaggtcaagggcatcgacgaagtcctctggcgcggcgccgaactgtatcgcgccgagtcgaagaacaaggaaacgatggagcgctacggccacggcacgcccgatgactggctcgaacgcaacctgtacacgcgctacagctggcaaggcgtgggcctgatgctggtcatcaacctggcgctgttcggcgggctgggcctcacggtctgggccgtgcagatgctctggatccccatcacggcggccggcatcatcaatggcattggccactactggggctatcgcaacttcgaggcgcaagacgccagccgcaatgtctcgccctggggcctgatcatcggcggcgaagagctgcacaacaaccaccacacgtatcccacctcggccaagttctcggtcaagaagtacgaattcgacatcggctgggtctatatccagatgatgcagaagatcggctgggccaaggtcaagaaggtgccgccgaagatgcagatgggcgacatccagcccgtggccaacgagaagacgctcgaggccgtcattgccaaccgctacgaagtcatggctggctatgcgcgcgaaatgcgccgtgtcaccaaggcggagctggttgcgctcaagaccaagggcggcgacatctcggtgctcaaggcagccaagaactggctgcaccgcgacgacgacaaggtgccggcatcggcccgcacgcacctcgtgcaggcgcgcgccgcccacccggtcatcgacaagatggtcacgatgcgcgaagaactgcgccagctgtggctcaacacgtcgcagtcgcgcgagcaactggcggccgatctggcggcctggtgccaccgtgcggaagccagcggcattgccggcctgcgcgaattctcgacccgcctgcgcgcagcgcgggcctgagagtccttcaagaatcgcgcgactcgcgcagcacctgcgctccctgaaaagccggcttccaggccggcttttttacgcccgtctttttcctgcgcgagagcgggagggcaaagaaatagaagaacccgcgagttgaaatgagggatcgacgggcaacaaaaaacccccgccgggcaagcctggcgggggttttttgtttgggtaaaccagcgctgaattacttcagcttgatttccttgtattcgacgtgcttgcgtgccttggggtcgaacttcatgatcgacatcttttcaggcatcgtcttcttgttcttgctggtcgtgtagaagtggccggtacccgcggtggattccagcttgatcttttcgcgtccgcctttgctcgttgccatgattcagctccttaagcttggccgcgtgcgcgcaggtctgcgagcacggcgtcgatgccgttcttgtcgatcaggcgcagtgcagcgctcgaaacacgcaggcgaacccagcggttttcagtctcgacccagaaacggcgatattgcaggttcggcaggaaccggcgcttggttttgttgttggcgtgggaaacgttgtttccgaccatcgggcctttgcccgttacgtcgcatacgcgtgccatgaggacactctttcttgaacagctggcaccggcgcaaccgtgaagattgcaggtgttttgcagcttgacctcgccagaaacgggtggcggtaccccggcttgccgaacccacggggagtggtgctgtttcggcaaagccttgaattatagcccttttggccgcagcccggtctagagcgtgccgtcctgctcaaggaagcgctgggcgtccagcgcggccatgcagccggtgcccgcgctcgtgatggcctggcggtacacgttgtcctgcacgtcgccggcggcaaagacgcccggaatgctggtcatcgtggcgaagccctgcaggccggagcgggtcaggatgtagttgtccttcatctccagctggccctggaagatgtcggtgttggggtggtggccgatggcgatgaagcagcccttgaggtcgatctgctcggtctcgccgttctgcgtgctcttgatgcggatacccgtcacgcccgtgtcgtcgcccagcacctggtcgagttccttgtgcagcttcagcacgatcttgccttcggcgaccttttcgtggagcttgtcgatcaggatgggctcggcgcggaacttgtcccggcgatggaccagcgtgaccttgttcgcgatgttggcgaggtacagcgcttcctcgacggccgtgttgccgccgccgatcacgcacacctcttgctcgcggtagaagaagccatcgcaggttgcgcaggccgaaacgccgcggcccatgaatttctgttcggaatcgaggcccaggtacttggcggaagcgccggtggcaatgatgagcgaatcgcaggtgtaggtgccgctgtcgccggtcagggtgaaggggcgcttgccgaggtcgaccttgttgatgtggtcgaaaacgatctgtgtcttgaaccgctcggcgtgttcgagaaagcgctgcatcagctccggaccctggacgccgtgcacatcggccggccaattgtcaacttctgttgtcgtcatcaattggccgccttgggcaatgccggtgatgagcaggggttgcagatttgcgcgtgctgcataaaccgcagcggtatagccggcagggccggagccgaggatcaaaaccttggcgtgttggggagcggacatgattggaaagcctagtatttgcgctgcgtcagcgtgtacattttcagggtggtagccgatatatatggagtatcaccgcccggttcaatgcccgggtgcacggtgttttcaatgcgcgcgattgtagtaatccatcgaaaaccgaaggtggggagggcttgcacgtgcggtatcagggattgataaatgtcgatgctttccaatcttgagctgttgcggcgcgttccgttgttcgcctcgctgacatcctcgcaatctgcaagcattgcggatgcgatcatcaaaaagcgcttcaagcgagcggaagtcattgtcgagcagggcaagaagtccaatgccctctacatcatcctgaccgggcgggcgcgcgtcacgagcgccgacacccgcggccgcgaagtgatccttgccacgctacacaccggcgactacatcggcgagatgagcctgatcgacgacgagccgcattcggccacggtgcgcaccgaaatccagtgcgacgtcctcatgctgggccgcgacgcattcgcacgctgcctgcccgaaaactcctcgatggcctacaacatcatgcgcgggctcgtgcagcgcctgcgccatgcggaccgcaagatcgagtcgctggcgctgatggacgtctatgggcgcgtggcgcgttcgctgctcgagttcgccatcgacgacggcgcgggcaatttcaaggtgcgcgacaagatctcgcgccaggatctcgcgaaaatggtgggtgcttcgcgcgagatggtgagccgcgtgatgaaggatctcgaggagcgcggattcgtccagtcccaggacgacggctccatgatcgtcaaggaacggctcctgtctttgacttgagccgacggggcgggcgcttccagcggccgccttttgttgtagtgttcaggcctccagccgccacttcgaaggctggatgccgtgtttttcatgacctattcgctcaatacgcttcaatcttcttccgccgccgaggggcaaccggtgcgcatgcgcgccatgcgctttgcccacgaaatcacgctgatcgcgggattcgcggggctgctgttctggttgctggccatgctgagcttcacgccttccgatgcggcgtggtccacctccggcaccggaggcgaaatcaagaactggggcggccgcatcggcgcctggctggccgacggcagctacttcctggccggttattcggtgtggtggtgccttgcggcgggcctgcgcgcgtggctctcctcgctcgccaactggctgcgcggcggcgagaccgcgcctgccgagcaaccggtgcgcggccgtttcaaccgcagccgactggcgttctggttcggcctcgtcctgctgctgtgcgcgagcgccgtgctcgagtggtcgcggctgtatcggctcgaatcccatctgccgggctcgggcggcggcgcgctgggctacctggtcggtcccgcaagcgtgcgctggatgggctttaccggctcggcgctggtggccattgccgccggcgtgatcggctcggcgctggtgttccgtttttcatggacccagattgccgagcgtattggcgcgcgggcctattcgctgttcgagtcgcgccgcgaaaagcgcgagatggccgctgacatcgccctgggcaagcaagccgcacgcgaacgcgccgaggccgaggagccgccgttctcgcatggagccgccggcagtatcgagccgacaggcctcgaaggcgatgaagagttgcgcatcgagccgcgcccaaggcgccgggcgccgtcgccgccggtgcagatcgagcccgcgatgaccgaggtgcccaggagcgatcgcgtcgtcaaggagcgccagaagccgctcttcaaggaactgccggacagcaagctgccgcaagtcgacctgctcgacgccgcgcaggtgcggcaggaaacggtgtcggccgacacgctcgagatgacctcgcgcatgatcgagaaaaagctcaaggacttcggtgtcgaggtgcgcgtggtgcttgcctcgcccggcccggtgatcacgcgctacgaaatcgaaccggccaccggcgtcaagggctcgcagatcgtcggcctggccaaagacctcgcgcgctcgctctcgctggtgtcgatccgcgtggtggaaaccattccgggcaagaactacatggcgctggagttgccgaacgccaagcgccagtcgatcaagctcagcgaaattctcggttcgcaggtctacaacgagggcaagtcgttcctgacgatgggtctcggcaaggacatcatcggcaaccccgtggtggccgacctcgcgaagatgccgcacgtgctggtggccggtaccaccggttcgggcaagtcggtcggtatcaacgcaatgattctttcgctgctctacaaggccgaggcacgcgacgttcgcctgctcatgatcgacccgaagatgctcgaaatgtcggtctacgaaggcattccgcacctgctggcgcccgtggtgaccgacatgcgccaggccgcgcacggcctgaactggtgcgtggccgagatggagcgccgctacaagctcatgagcaagctgggcgtgcgcaacctggccggctacaacaccaagatcgacgaagccaaggcgcgcgaggagttcatctacaaccccttcagcctcacgcccgacgatcccgagccgctcaagcgcgagccgcacatcgtggtggtgatcgacgaactggccgacctgatgatggtggtcggcaagaagatcgaagaactcattgcccgtctcgcgcagaaggcgcgcgccgccggcatccacctgatccttgccacgcagcggcccagcgtcgacgtgatcaccggcctcatcaaggccaacattcccacgcgcattgcgttccaggtgtcgagcaagatcgacagccgcaccatcctcgaccagatgggcgccgaagcgctgcttggcatgggcgacatgctctacatgccgagcggcaccggcttgccgattcgcgtgcacggcgcgttcgtgagcgacgaggaagtgcaccgcgtggtggcgtatctcaagagccagggagagcccgactacatcgagggcgtgctcgaaggcggcacggtcgatggcgacggcgacatgctgggcgagggcggcgacgccgagaaagacccgatgtacgaccaggcggtggaagtggtgctcaagaaccgcaaggccagtatttcgctcgtgcagcgccacctgaaaatcggctacaaccgcgcggcgcggctggtcgaagacatggagaaggcgggcctcgtcagtgccatgagcggcagcggccagcgcgagatcctggtgccggcgcgcgccgaataggcggcgaaaacccgccgtcccggaagttacgcgctgacaagctcgttgcaaaagctgcgctagcgttgcaaaacttcatcaagccccgcacatggcgcaacgcgccgcggggtatggtcatgtcaacggcatcgcttgctgaaggaatccaaaatgaaaatgcgtcattggctgttgatcggccttctctcatcccttctctcaacggccaacgcctgggccggcggcctcgaaagcctcgagaccttcgtcaagacggtcaagtcgggccgcgcggaattcacccagaccgtgaccgcaccgccgcgtgaagggcagccgggccgcgccaagacatcgaacggcaccttcgaattccagcgcccgggcaaattcaagttcgactaccagaagccgtttgcccagagcatcgtggccgacggcaagacgctctggctgtacgacgccgacctgaaccaggtcacgcagcgtgcccagtcgcaggcattgggctcgacgcctgcggcactgattgccgcggcccccgacctgcgtgcgctgcaggccgacttcacgctcgaggccgcgcccgaacgtgatgggctccagtgggtcaaggctacgcccaagaacaaggacggccaattgcagaacgtgcatgtcggcttccagggcgacgcgctggccgcgctcgagattctcgacagctttggccagcgctcggtgctcaagttcagcaaggtcgaagtgaacccggcgctccctgccaccgtgttcgaattcaaggcgcccgccggggccgacgtcatcaagcaatagcagcaacccgacaggcaggcttggccaacagttcgcatcaaccccttgccgaacgcctgcgtccgaagacgctcggcgaggtcattggccagcagcacctgctggggccgggcatgccgctgcgcatcgccttcgagtcgggccaaccgcattcgtgcattctctgggggccgcccggcacgggcaagacgaccatcgcgcggctgatggccgatgccttcgatgcgcaatttctcagcatcagcgccgtcctcggcggcgtgaaggacatccgcgaagcggtggagcgcgccacggccgcacgggacggcctggagcagcagcgcaccatcgtcttcgtcgacgaggtgcaccggttcaacaagagccagcaggatgcgttcctgccgcacgtcgaatcggggctgttcaccttcatcggcgccaccaccgagaacccttcgttcgaggtcaactcggccttgctttcgcgcgcggcggtgtacgtgctgcagccgctcacggagggtgatctgaagcagatcgtcgccaaggcacaggccatccaggcggttcccgccatcgaagacacggccatcgaccggcttgtcgcctacgccgacggcgacgcgcggcgcctgctcaacacgctcgaaacactggccgtggcggcccgtgccgagaagctcgacaacatcgccgacgaatggctgctgcgcgtgctcggcgagcgcatgcggcgctacgacaagggcggcgagcagttctacgacaccatcagcgccttgcacaaatccgtgcgcggcagcgaccccgacgccgcgctctactggttcgtgcggatgctcgatggcggtgccgatccgcgctacatggcgcgccggctggtgcgcatggccagcgaagacatcggcctggccgatccgcgcgcgctccggctggcgctcgatgcggccgaggtctatgaacggctcggcacgccagagggcgaactcgcgctggccgagtgcgtcgtttacctggccatcgctcccaagtcgaacgccgtctacaccgcctacaacgcagtgcgtgccctcatcaagaaggacagcacgcgcccggtgccgatgcacctgcgcaatgcgcccaccacgctcatgaaggacctcgactacggcaagggctaccgatatgcgcacgacgaggaaggcggctttgcggccggcgagcgctacctgccggagggtctcgaagggcaggtcttctaccagcccgtcgaacgcggactcgaaatccgcatcgcagaaaagctgcgcgaactccgccggctcaacacccagcgcgaagggtgatacgtcttttcacactgcgggcacgccctgcatgacttcactcgcatacagcatggcgtgagcgggtaaaccccggtgaaggcgcaccaaatcggcgctggtgggtgcttacaatcccgcccacaaatcagccagcgacacatgctggctggttttttgcttatcaagccaaggtgccaaaccggtgccacgctgggtgaacggcaccccgcaacggtgcaacaaataggaacgcgttatggaaattttgctgcagcagatcatcaacggtctggttctcggcagcatgtatgccttgatagccttgggctacaccatggtgtacggcatcatcaacctgatcaactttgcgcacggcgaagtgctgatggtgggggcgctcacgagctggaccatcatcggcctcatgaaggaatcgatgcccggcacgcccggctggttgatcctcatcatcgcgctgatcattgcctgcgtggtggccgccacgctcaacttcgtgatcgagaaggtcgcctaccggccgcttcgcaacagccccaagctcgcgccgctcatcacggccatcggcatgtcgatcctgctgcagacgctggccatgatcatctggaagcccaccaacaaggcctatcccaacctgctgtcgaccacccccatcgaggtgggcggcgcggtgatctcgcccacgcaggtcatgatcctgagcgtcacggcgttctcgctcgtggtgctgatgtggctggtcaactacaccaagctcggccgcgccatgcgcgccaccgccgagaacccgcgcgtcgcggcgctcatgggcatccggcccgacatggtcatttcggccaccttcatcatcggcgccgtgctagcggccatcgccggcgtcatgtacgcctccaactacggcatcgcgcagcacgccatgggcttcctgcccggcctcaaggccttcaccgcggcggtgttcggcggcatcggcaacctggccggcgccgtggtcggcggcatcctgctcgggctgatcgaagccatcggctcgggctacatcggttcgctgaccggcggtgtgctgggcagcaactacagcgacatcttcgcgttcatcgtgttgatcgtcatgctcacgctgcggccttcgggcctgctcggcgagcgcgtggcggatcgggcctgaggagcagaacaccatgaagaacagcaagaacctcgctctctacgtgctcggcgtcgtcgccgtgctcgccctgcccatcttcctgcagagccagggcaacgcctgggtgcgcatcgccgacatcgcattgctctacgtgatgctctcgctcggcctgaacatcgtcgtcggctacgccggcctgctcgacctgggctatgtcgccttctttgccgtgggggcctacctctacgcgctgatgggctcgtcccacctgtccgacaccttcccgtggttcaaggccatgttcccgaacgggctgcacacctcgctgctcatcgtggtgccgctggcgctggcggtggcgggcgtgctgggcgtgatgctcggggcgcccacgctcaagctgcgcggcgactacctggccatcgtgacgctcggcttcggcgaaatcatccgggtgttcctgaacaacctcgaccagccgatcaacatcaccaacgggcccaagggcatcaccgccatcgactccgtcaagttctggggactcgacctcggcaaggcatggaagttcgacggcttcacgatctcctcggtcacgctctactactacctgttccttgcgctggtggtcgccaccatcatcatctcgcaccgcctgcagatgtcccgcatcggccgcgcctggatggccatccgcgaagacgagatcgccgccaaggccatgggcatcaacacccgcaacatgaagctgctggccttcggcatgggtgccagtttcggcggcgtgtcgggcgccatgttcgcggccttccagggcttcgtgtcgcccgagtcgttcagcctcatggagtcggtgatgatcgtcgccatggtcgtgctgggcggcatcggccacctgccgggcgtgattctcggtgccgtgctgctggccgcgttgcccgaagtgctgcgctacgtggccggtccgctccaggccatgaccgacggccgcctcgatgcgtccatcctgcgccagctcttcattgcgctggccatgatcgtcatcatgctgatgcgtccgcgcggcctctggccttcgcccgagcacggcaagaccttgcagcgcaagggcgtggccccagacgcccccgtggcaccgggttcgctccagacccatgcgcccggcatcgagacacccgccgacgaattgccgggtgcggcttcgcgtcccatgtcgatcaatccgtgagccgaaggaagcaatcaacatgacgacagacaccatcctcgacgttcgcggaatttccaagcgcttcggcggcctgcaagccctctccgacgtcggcatcaccatcaagcgcggccaggtctatggcctgatcggccccaacggcgccggcaagaccaccttcttcaacgtgatcaccgggctctacacgcccgacagcggcagcttcgagctcgccggcaagccctaccagccgacggccgtgcatgaagtggccaaggccggcatcgcgcgcaccttccagaacatccgcctgttctccgaaatgacggcgctcgagaacgtcatggtggggcgccacatccgtacccattcgggcgtgttcggcgccatgctgcgcaccggttcgttcaaggccgaggaaaaggccattgccgagcgcgcgcaggaactgctcgactacgtgggcatcggcaagttcgccgactacaaggcgcgcacgctgtcgtacggcgaccagcgccggctcgagattgcgcgcgcattggccaccgacccgcagctcattgcgctggacgagcccgccgccggcatgaacacgaccgagaaggtgctgctgcgcgagctgatcgaccgcatccgcaaggacgaccgcaccattctcatcatcgaacacgacgtcaagctcatcatgggcctgtgcgatcgcgtcaccgtgctcgactacggcaagcagattgccgaaggcacgccgtacgacgtgcagaagaacgagaaggtgatcgaggcctacctcggcaccggaggacactgaaatgaccacgacgacgatgacgagcgcagaagaaacaacagcaacggcaactgcaaccccgccgaagaccgcggccacggccaccggcaagacgctgctcaaggtcagcggcctcaaggtcggctacggcggcatccaggcggtgaaaggcgtggacttcgaggttcacgaaggcgaactggtgtcgctcatcggctccaacggcgccggcaagaccaccaccatgaaggcgatcaccggcacgctgccggccggggcgggcaccatcgaattcctgggccgcaacatcaagggccgcggtgcgtgggacctggtgggcgagggcctcgtgatggtgcccgaagggcgcggcgtgttcacgcgcatgaccatcaccgagaacctgcagatcggtgcctacatccgcacggacaaggccgagatcgccagcgacatggagcgcgtgttcgtgaccttcccgcgcctgcgcgagcgcaaggaccagctcgcgggcaccatgtcgggcggtgaacagcagatgctggccatgggccgcgcgctcatggcgcgccccaaggtgctgctgctcgacgagccgaccatgggcctgtcgcccatcatgtgcgacaagatcttcgaggtggtgcagaccgtggccgcgcagggcgtgaccattctgctggtggagcagaacgccaaccgcgcgctgcagctggccgaccgcggctacgtgatggagtccgggctcatcacgatggacggcgacgccaaggaactgctgcgcgacccgcgcgtgcgggccgcctacctcggcgaataaccttcgaaggggtcaatcgaccctggcgccggtcgccttcacgacggcttcgtacttggagagctcgctcttcatgaacgtgccgaactgctcgggcgaactggccacgggctcggccagcagcgtggcaaaacgggtcttcgtttccggtgcattcagcgccgcgacgaaggcctggttgagcttcacgaccacgtcgtgcggcgtgccggccggtgccaccagcccccaccaggtgtcgatcgaaaagcctttgagcgtgtcggccaccggcggcacgtcgggcatggcgctgctgcgctgcaaggtcgtgacggcaatggccttgagcttgcccgagcggatgttgggcgccgcggtggcaaggttgtcgaagttgaaatcgacctggcccgagagcagcgccaactgcgccggattgccgccgttgtacggaatgtgcagcgcgaagatgccggcctgcttcttgaacagctcgcccgccaggtggccggcgctgccgttgccaccgcttccgtagttgagcttggccgggttcgccttggcgtagcgaaccaggtcggccacggtattgatcttcaggcgctgcgccgtctctgcattcatcaccagcacgttcggcacgcgcaccatctgcgtgatgggcgcaaagtcgctcgccgcgttgaacggcatcttgctgtagagccacggattcaccgcatgggtggcggtggccgcaatgccgatggtgaggccgtcgggcgcggccttggcgacgatgtctgcgccgatgttgccgcccgcaccgggcttgttgtcgatgatgaccgtacccagcgtgtccttcacgcgttcggccagcatgcgggccgtgacgtcgatcggcccgcccgcggcgtagggcaccacgaggcggatcgggcgttgctgctgggccgccgcctggccggtggcaatcagcgtggcactggcaagcagtgcaagaaggaagtgtctcgttttcattttttcgttctgtcgtctcgcggaaatcggatcggagatcagggaagcgctttgtcggcctcggtggtgaatgcgtcggcaaagaactcgtcttcgggcaggccggccagcgccacgtagtcatgcttggccgagtcgaccacgatcggcgcgccgcaggcgtacacctggtgcccggaaaggtcggcaaagtcttccagcaccgcgcggtgcacgaagcccgtgcggccggtccagttgtcttcgggcgtggcattggaaacgaccggcacgtagcgcaggttcggcatctccttcagctgctcgcgcatccagccgtccatgtagaggtcttcgggccggcgaccgccccagtagaccgtggcgggccggtcgatacgcttgaacttcatgtgctcgagcagcgccttgatcggcgcaaagccggtgccggaggccaggaagatcatcggcttggcggagtcctcgcgcaggaagaagctgccgtaggggccttcgatgcgaaggatttccttttccttcatcacgccgaacacgtggtcggtgaacttgccgcccggcaggtgccgcaggtgcagttcgatgcccgtgcccggctcggccagcgtgtgcggcgcattcgccatcgaatagctgcggcgcgcgccgtcgcgcaggatgaattccacgtactgccccgcatggaactgcagcggttcgccggccggcaattgcaggcgcagcttcatcacgtcgtgcgacagccgcgtgagcgccagcacgcgcaccggcattttgcggatcggcagggcgccggcctcggtgacctggcgcgactcgagcaccacgtcgctctttgcgtgggcgcagcaggtcagcacgaagcccgccagctgctcttcggcgctcagtgccttgctctggtgcgggcccagctcgacttcgccagagagctttttgcacttgcaggagccgcaggcgccgtctttgcacccataggggagcccgatgccttgccggatcccggccgcgagaatggtttcatcgccatgcaccacgaagtgacgcccgctgggctcgacggtgatggaaaagcccgcgtcatgcggcgctgcaacagtcatcggtattcttcggcttgtttcagcctgtagcagaaaagagaaaaagggaaaggaacccggattttgccttcaatcaatagcccttccggcgcgctgccggcccgcttccgccgcgaacgcctgctgatcgtcggctgcggcgacgtcggccagcgcgtggcacgcgacctgcgcggccgcatgcagctggtggcgctcacttcgtcggccaaccgggtgccggcgctgcgggcagccggcatccgcccgctcgtaggcaacctcgacgacccgtccacgctgcggcggctggccggcgtggctacccgcgtgctgcacctggcgccgccggcgcgcgacggcggcgcttcgtggtggcgcgaccagcgcaccaccgcattggcccgggcgctgcggctgcgctccacgccattggcattcgtctacggttccaccagcggcgtctatggcgactgcggcggcgcgcgggtgagcgagacgcgggccgtgcggcccgacacgccccgcgcccatcgccgcgtggatgccgagcgcgcggtgcgctggctcggccgcagcgccggcgtgcgcgcgagcatcctgcgcatcccgggcatctatgcgccagaccgcgaaggcggcacgccgcgccagcggcttgcgcgcggcacgcccgtgctgcggcgcgaggacgacgtgttcaccagccacattcatgccgacgacctggcgcgcgcctgcgtggcggcgctgttccgcggccggccccagcgcatcgtgcacgcctcggacgacaccgagctgcgcatgggcgactacatcgacctggccgcagacctctacggcatgccgcgtcccccacgcgtggcgcgcgacgaagcccagcgccaactgccgctgcaactgctgagtttcatgggggaatcgcgccggctcgacaacacgcggctcaagcgcgaattgcgcgtgcggcttgtgcatccgacggtgcacacgggactgcgcgaggaagcctgagctaccagggaaggggtcttttttcagggataccgaggaaccggcttcgccgggccgccggtatcgcccccggtagggggttggcgaagcgacacgaagtgcgcgcagcctgggggcgagtcaaagtgtggtgcccggggccggaatcgaaccggcacacctttcggtgggggattttgagtcccctgcgtctaccaatttcaccacccgggcagggttctgaagcaagcccaaaattatggcacagtggctgccatgaattatccgacgatcgaagacgccatcggcaagacccccctggtggcactgcaacgcatcgatgcggccgaaaatgccaagcgtggcaacgtgatcctcggcaagctggaaggcaacaatcccgcaggctcggtgaaagaccgtccggcgctctcgatgatcaagcgcgccgaggagcgcggcgaaatcaagcctggcgacacgctgatcgaagccacctcgggcaacaccggcatcgcgctggccatggccgcggccatcaagggctaccgcatggtgctgatcatgccggaggatctgtccgtcgagcgcgcccagaccatgaaggccttcggcgccgagctggtgctcacgcccaagagcggcggcatggaatacgcgcgcgaccttgccgaacagatggtggcgcagggcaagggccgcgtgctcgaccagttcgccaatgccgacaacccgcgcatccactacgagaccacaggccccgagatctgggccgacaccaagggcaagatcacgcatttcgtgagcgccatgggcaccaccggcaccatcaccggcgtctcgcgcttcctgaaggaaaagaaccccgcggtgcgcatcatcggcgcgcagccggccgagggctcacgcattccgggcattcgcaaatggccggccgaatacctgcccaagatctacgatgcgagccgcgtcgatgaagagatcagcgtgagccaggacaacgccgaagaaatgtgccgacgcctcgcgcgcgaggaaggcatcttcggcggcatctccgcggccggcgcgctatgggtggcgctcgaggtggccaagacggtggagaacgccaccatcgtgttcgtcgtgtgcgaccgcggcgaccgctatctgtcgaccggcgtgttccccgcctgataaagccacaaccccatgccccatcccaagttctgccaggcctgcgccacgcccctcgaatggatcgcgctgatggaagacggcggtcccaaggagcgcctgcgctgcccgtcctgcggccacacgcactggaacaatcccacgcccgtgctcgcggccatcgtcgagtaccgcggccaggtgcttctggcgcgcaatgcggcctggcccgtcaagatgtatgcgctgatcaccggcttcatggaggccggcgaaacgcccgaggaaggcattgcgcgcgaggtcaaggaagaaaccaacctcgacgtgagcgcggccaagctcgtcggcgcgtacgacttccagcgcatgaaccagatcatcatcgcctaccatgtggtggccgatggcgaggtcaggctctcgcccgagctggtggactatcgcctctacgacctgcccgacctcaagtgctggccggcgggcaccggctatgcattggccgactggctgcgcacgcggggccacgagcctgtgttcttcaccgcagccgagaacgacgaccgccgccgcgggctcaatctgccgcccgaggagcccaagcatggaagctgatcgcgaaatcgatacgcgcgggctgaactgcccgctgcccattctcaaggcgaagaagtcgctcaacgacatggcgagcggacagttgctcaaggtggtgtcgaccgacccgggctcggtgcgcgacttccaggcctttgcgcgccagaccggcaacgagctggtcgaacagcagaccatcggcagcgacttcatccatgtgctgaagaggcgctgaccagaaagaaaaagaaaagggccccggttggggcccttttttttcagagctccaggctcttcagatactcgcggaactgcgcgcccacttcggggtgcgccagcgcaagctccaccgaggcttgcagaaagccttccttgctgccgcagtcgtagcgaatgcccttgtaggcataggcatagaccgattctttcttcatcagcgccgcaatgccgtcggtgagctggatctcgccacccgcgcccttgggctggttgcgaatttcgtcgaacacgccgggcgtgaggatgtagcggcccgccacgccaaggcgcgagggggccttgtccggcgagggcttctcgatcatgcgatcgaccttcacgagatcgtcgccgatggattcgcccgccacgatgccgtagcgcttcacgtgctcgagcggcacttcctgcaccgcgagcagcgaggcgccgagcttgccgaaggcggcggtcatctgtgcgagcaccggtgcaccgcccacggggccgaccatcaggtcgtcggccagcagcacggcgaagggttcgttgcccaccaggtgttcggcgcacagcaccgcatggccgagccccagcatgcgcggctggcgcacgtaggagcaggtcatgtcgtcgggcatgaccgagcgcgcgatgttgagcagttcgagcttgccgctggcctcgagctggctctcgagttcgtaggcggtgtcgtagtgatcttcgatggcacgtttgtttcggcccgttacgaaaatcatgtcgcgaatgcccgccgcgtaggcttcctcaaccgcgtattggatgagtggcttgtcgacaaccggcagcatttcctttggctgcgccttggtagcgggcagaaagcgggtgccgaaacctgcaacaggaaatacggccttgcggatgcgtgtcgagggagtgggcatggacaatttgggcgtctgttcgttcagttgaagaagaaggttttacagtcagcaaacggtaccgaaataccgtctttgtcatgctaaaccctgccccgatccatgtgtgtcagccaagacgcacaagctgatcgcgaagacgttccaacgttgcactgaaatcgctcaggcgcttgcgctcctgttcgatgacagccggtggtgccttagctacaaaggcttcattgccgagcttgccgttcactttcaggatctcgccttcgatgcgagcaatttccttgcctatgcgcgcacgctcggcggccttgtcgatctccatgtgcaggcacagccgtgccgtgcccaccacggccacgggcgccgcttcggccgctgccgaccatgaggcctcgtcgtcgaacactttcacttccttgagcttggccagggcctgcagcaccggtgccgcatcgcgcaagaaagccgcgccctcggcatcgtcggccaccgcatagagcggcaggcgcaccgcgggcgacacgttcatttcgccgcgcagcgtgcggcacgcatccaccagcgccttcaggcgcgccacgtgcgcttcggccgcttcgtcgatcttctcgggctggctcttcggataggccgccaccatgatcgattcgccctcgcgtcctgcgacgggcgcgaccttctgccacagctcttcggtaatgaacggaatcaccggatgcgcgaggcgcagcagtgcttcgagcgtgcggatcagcgtgcggcgcgtggcgcgcttttgcgaatcgtcgccggtctggatctgcaccttggcaatctccaggtaccagtcgcagaactcgtcccacgcaaactggtagatggcgttggccacgttgtcgagccggtattcctcgaagcccttggccacttcggcctcgacgcgctgcagctgcgaggcgatccagaagtcggcgcggctgaacttgaggtagccgtgggccggtccaccgaccgcgcactcttccttggtgtgctcgcgcaggccgcagtcctgcccttcgcaattcatcagcacgaagcgcgtggcgttccagagcttgttgcagaagttgcgatagccctcgcagcgcttgctgtcgaagttgatgcttcggccgagcgacgccagcgaagcgaacgtgaagcgcagcgcatcggcgccaaaggccggaatgccttcgggaaattctttctgcgtgttcttgcgcaccgcgggcgcggtctcgggcttgcgcaggccctgcgtgcgcttgtcgagcagctcgggcaatgcgatgccgtcgatcaggtcgaccgggtcgagcacgttgccttccgacttgctcatcttcttgccctgcgcatcgcgcaccaggccatggatgtacacgtccttgaacggcaccttgccggtgaagtgcttggtcatcatgatcatccgggcgacccagaagaagatgatgtcgtagcccgtcaccagcacgctcgagggcaggtacagctccaggtccttcgtcttctcgggccagccgagggtggagaaaggcaccagggccgccgagtaccaggtgtcgagcacgtcttcgtcgcggcgcagggtcttgcccggggccttggcctgcgcttcggcttcgtcgtgcgccacgtacacattgccttcgtcgtcgtaccaggccgggatctggtggccccaccagagctggcgggagatggtccagtcctggatgttctccatccagtggttgtaggtgttgacccagttctcgggcacgaagcgcacttcgccggtcttcaccacgtcgatggccttctgcgcgatcgaggtgccgtcggcgccgggccgcgtcatggccacgtaccactggtcggtgagcatcggctcgacgatggcgcccgagcgcgcgcagcgcggcaccatcagcttgtgcttcttcacctcgaccaggaggccgagtgcatcgaggtcggccacgatggccttgcgcgcgacgaagcggtccatgccgcgatatttttcaggcgcgttgtcgttgatggtggcgtccagcgtgaggatgccgatcacctcgagcttgtggcgctggccgacggcgtagtcgttgtagtcgtgcgcgggcgtcaccttgaccacgccggtgccgaactccttgtcgacgtagtcgtcggcaatgatgggaatcaaccggtccaccagcggcagcttcacgcgctggccgatcaggtgtttgtagcgctcgtcttcggggtgaaccatcacagccgtgtcgcccagcatggtctcgggccgcgtcgtggccacggtcagcgtggcgctgccatctgccagcggataggcgatgtgccagagcgagccgtcttcctcttcgctttcgacttcgaggtcgctcaccgaggtcttgagcaccgggtcccagttgcccaggcgcttgccgcggtagatcaggccttcttcataaagcgagacgaaggtttgcgtcacgacctgcgaaaggtcgtcgtccatcgtgaagtattcgcggctccagtcgaccgtatcgcccatgcggcgcatctggccggtgatggtgttgccgctcttttccttccactcccacaccttggcgacgaagttcttgcgggcctcggcgggcgtcgggcccatgtcgtggcggctgatcttctgctcctgcagctgccgttccaccacgatctgcgttgcgatgcctgcatggtcggtgcccggcaaccacagcgtgttgtcgcccttcatgcggtggtaacgcgcgaggctgtccatgatggtctggttgaacgcatggcccatgtgcagcgtgcccgtcacgttgggcggcggcagctggatcgcgaacgaatcggcgccttccttcggctcctgggtgccgcggaagccggccttggcatagccgcgcttttcccactccgggccccagtccgcctcgatggcggcgggttcgaacgatttggacaggctgtccagaccaggctgggcggaaggggtggtggattcgctcattggagatgcaggagatgcagggagatgcagaacggcgccttcgggggagccgtggagacaagggtgggatagccggcgattttaccggggcggccccgggcgagccccaccccacataattccgggatgctcttcttgctttcccctgcgaagtcgctcgactacgacacccccgttcccgccgaaatccccgccacccaaccccatttcgaatccccgcgcggcccttcggtcgaactgatcaagctgctgcgcgagaagtcgccgctgcagatttcggagctcatgcacctgtcggacaagctctccgccctcaacgtggcgcgctaccaggcctgggccggcaagagcacgccgaagaatgcccgccaggccgccttcgcattcgacggcgacgtgtacggcggcctcgatgcccgctcgctcacgcccacccagctggcctgggcgcaggagcacctgtgcatcctgagcggactctacggcctcctgcgtccgctggacctgctgcagccctaccggctggagatgggcacggcactggccaaccgccatggcaaggacctgtatgccttctggggctcgcgcattgcggaacacctcaacgagcgcctggcggcagaccgcacgcctgtcgtggtcaatgtcgcctcgcaggaatacttcaagtcggtggacctgaagacgctcaaggcccgcgtggtcgaatgcgtgttcgaggaatggaagggcgacaagtacaagatcgtgagcttctacgccaagcgcgcccgcggcctgctcgcgcgctgggcggtgctgcacaaggcggccacgcccaaggcgctggaaaaattcgatctcgagggttatggtttcgatgccaaggcttcaacggccgaaaggctggtgttcaggaggaaggcttgatatgtcacaggcgatcagtcccgagctgagggagtggctggtgtcgcagctagcggccgggcattcggtgcccgcgctgcgcgcgtcgatgcgcgccgccggctggaaggatgcggccaccgatctcgcgctggctcagctcgaagccggctttccgcacttggaagtggctgcgaagacaccgcgcaccgacatgcccggccccgacctcgaaggcgcgccgctctacatcgatgcgggcgaccgccgcgtgcaggtgctgcacaccatgcggcatccgcgcgtggtggtgttcggcaacctgctctcgcccgaggaatgcgaaggcctgattgccgccgcgcgggtgcgtctggcgcgctcgctcacggtcgaaacccgcaccggcggcgaagtgctgaacgtcgaccgcaccagcgaaggcatgttcttcgagcgcggcgagaacgagatcgtcgcgcgcctggagcagcgcattgccgcattgctgcgctggccggtcgaattcggcgaaggcctgcagatcctgcgctatgcgcccggtgcccagtaccgcccgcattacgactacttcgacccgggcgagcccggcacgcccaccatcctcaagcgcggcggccagcgcgtggccacgctcgtgatgtacctgcaggagcccgagcagggcggtgccaccaccttccccgacgtgggcctggaagtggcgcccgtgcgcggcaccggcgtgttcttcagctacgacgaacccgaccccgccacccgcacgctgcatggcggcgcgcccgtgctcgcgggcgagaagtgggttgccaccaagtggctgcgcgaacgcgaattcaaatagccgcaaggaaccgatgaaagtcaccgccaacgggctgcagatcgaggtcgacgataccggcggcgagggacgacccgtcgtcctgctcatcatgggcctgggcatgcagctggtcgcatggccgaacggcttcgtgcggcaactggtcgacgcgggctttcgcgtggtgcgccacgacaaccgcgacatcggcctgagccagggcttcgaccatgccggtaccggcaacatcgtctgggaaaccgttcgccaccgcctcgggctgaaggtgcgctcgccctacaccctgcaggacatgacgcaggactcgatcggcgtgctcgacgcgctgggcattgccaaggcccacatcgtcggggcctccatgggcggcatgatcgcgcagcgccttgccgccagtgcgccgcagcgcactgccagcctcgtgagcatcatgagttcgagcggcgcgcgcggcctgcccggcccgcgccgcgaagtcacggccatgctcatgcgccggcccctgggccgcagcgaggccgagctcgtggcgcacagcatcaagctcctgcgcctgatccagagcccggcctatccccagaccgacgaagagctggccgaacgcctcaccttcagcatgcgccgttcgtaccgcccggccgggctgatgcggcagatgctggccattggcgccgatgacgatcgcccgcaaatcctgccgcgcatccagagacccacgctggtattgcacggcgaagccgatgccctcgtgcccattgcctgcggcaaggattcggcggagcgcattccgggctcgacgttcatcggcattcccggcatgggccacgacctgccgccgcaggtctgcaccatcctcgccaaccacattgccccgttcgcgcatgccgtggacgccaaggaaaagccatgagcctcgacaacgcccccgacaaccccaacacccccgagcagtcgcaactgggccgtgcctcggcctacgccgacaagtacgacccctcgctgctctttccgatttcgcgcgccacccagcgcgaggccatgggcatcatcggcgcccagctgcctttcttcggcgccgatctctggaccgccttcgaggtgagctggctcaacctgcgcggtaagccgcagctggccattgcgcacttcaccgtgccttgcgaaacgcccaacatcgtcgagagcaagtcgttcaagctgtacctcaacagcttcaacagcaccgctttcgcgagcctcgatgccgtgcgcgaccgcctgcgcatcgacctgtccgaagcgctctggcgcggcagcgaccagtccgccggcatcggcgtgaagctgctggcgcccgacatgttcgaccgcgagccggtgcacgaactcgacggcctggatctcgaccggctcgacatcgagtgcacgcactaccagcccgcgcccgaactgctgtccagcgacaccacccagccgccggtgaacgaaacgctcaccagccgcctgctcaagagcaattgcctcgtcaccggccagcccgactggggcagcgtgcagatccgctacagcggcccggccatcgaccaggccggcctcctggcgtacatcgtgagctttcgcaaccacaacgagtttcacgaaccctgcgtcgagcgcatgttcaccgacatctggcgccagtgccagcccaacaagctcgccgtgtacgcacgctacacgcggcgcggcgggctcgacatcaatccgtttcgcaccagctggccgcaggcgctgccgccaaacatccgcaccgcgcggcaataagcaaagcgcgtcgccgaagcccctcttcggaaatcagaaactcgcagtcccggccctgtggcattctggatctgcccgtgaaccgcgggcggatttccggagcagacacacatggttgaaggaaaaacagtcgtcgtcaccggcgcgggcggcggcatcgggcgcgacattgcgctggccatggccagccacggcgccaaggtggtggtgaacgacatcggcgccgcgctcgacggcgagggcggcagcgccggcccggcgcagcaggtggtggacgagatccgcgccgccggtggccaggccgtgccaaacaccgacagcgtggccgatgcggccagcgcggcgcgcatcgtcgaatgcgcggtcgagagcttcggccgcatcgacgccgtggtcaataacgccggcatcctgcgcgaccgcttcttccacaagatgtcggtcgacgagtgggacgctgtgctcaaggtgcatctctacggcgcctattacgtgagccgtgcggcggccacgcacttcaaggagcagaactcgggcgccctggtgcacatgacctccacttcgggcctcatcggcaactacggccaggccaactacgcggcggccaagctcggcatcgtggcgctgtcgaagtcgattgcactcgacatgctcaagttcaacgtgcgctccaactgcatcgcgcccttcgcgtggagccgcatgatcggcgccattcccaccgacaccgacgagcagcgcgcccgcgtcgacaagatcaagcagatgacgcccgccaaggtggcgccgctcgcggtgtacctggcgagcgaggcggccagcgcggtcaacggccagatcttctcggtgcgcaacaacgagatctcgctcatcagccagccgcggccggtgcgctccattcatcgctccgaaggctggacgccggagagcattgccgagcacgccatgcccgccatgcgcgcgagcttctatccgctggaccgctcggcggacgtgttcagctgggaccccgtctgaagcccggcatctgaggtcaaaccctgagaagggcgcagacaacgccattcgccggacaatgcacgctccctttctttctggcgcgctcgtccggtgaacctgcacttcgatctgttcgacctgaaactgttcgtctacgtggcggaggcgcgcagcctcacgcgcggcgccgaaaaagcctgcatctcgctcgcggccgcctccacgcgcatcaagcagatggaagaagccgtgggcggcaagctgctgcaccgcagcgcacagggcgtgagcctcacggccgcgggccaggcggtgctctaccacgccaagcgcgtgatgcagcagatggagcacctgcgctgcgacatgcaggacttcggcaagggcatcaagggccatgtgcgcgtgttcgccaacaccacctcgatcaccgaatacctgccgcaaaagctggccggctttctcacccagcatccggccgtgcaggtggatttgcgtgaatacctgagcgaagaaatcgtgcgcgcggtggccgacggcgaggccgacatcggcatcctggccggcgacgttcacaccggagaattcgatgcgcgccccttcggccgcaaccagctcgtgctggtggtgcccgtcacccaccaccttgcgggcgcaccctcggtggcctttgccgacacgctcgacgagcagcacgtgggcctgcaccacggcagcgcgattcaccgcttcttgcagcgccgtgccgagctggccggccgcggcttcaatccgcgcatccaggtcagcagcttcgaggcgatctgcctgatgatcgaggcgggcgtgggcgtcggcgtgctgccggcctcatccgcgcagcggctgtcgatggcgatgcggatctcgaccgtcgccctcagcgatgcatgggccgagcgcgaactcaagctcattgcgcgcgaccgcgaacagctgcccgcctcggcgcgcgagctgttcgatcatctcgtcgcgccttagccggcgcttgtgccgtgctgccctcagggcagccagcgttccacgcgcggtgcgtcggccagctgccagatgcgccggcacaaggccttggcctcgtcggccgtggcgccttcgccgtagtgcgccaggcgctgcatcttgtcctcgagctctgcgcggctcaggctgttgcccgggtcgcccttgggctcgtccacgcggccttgcagcgtgcggccgtcacgggtctgcacgctgaccttgccgatccagcgcgcggggtaggcggtgtcgacctcggcatcgagttccatcgccaccctgtcgcggaaagcggccacctcgggcgcgagaaagtcgcggtcgaattcgcccaggcccgcgcggccgtgaactgcgatgagccccagcaccgtgcccatcgagaacttgccctggtgcacggtggccggcaccgcgacacggccgagcacgtcgatggcaccttgatgcacatgcgtggtcacgtgcgccacgtcatcgtgcttcaggttgttctgcgccatcacctgcagcagcgcgtcggccgccggatgcgtgtggcggcacgaggcgtggtacttgaacgaggtttctgccagcgcccagcgcgtgccgaggccgtcggtaagcttcgcgggatcggcatcgctcgacatgcccacgccgaggccctgcgcaccttcgagcaccttggccgcaccggtgaaaccatcctgcgcaagataggccgacatcagtccgctcgcggccgcatgcgcgcagtgcagctgcttggaatcagccgcatcgcgcaagaactcccacacgccggccgactgcgtaccggccgagccgaaggcgtgcagcatctgctgcggcgtgagcttgagaaggctgcccacggcagccgcggcggccagcgtgcccgccgtcgcggtggtgtgaaaggtcctgtagtgagagcggcccaggaactcgccgacgcgaatgccgacctcgtagcctgcgaccacggcggtcagcaactgcgcaccgcttgcacccaggctctgcgccacggccagcgcgggcgcgatgaccacggccgcggggtggaacaccgagccgttgtgcacatcgtcttgttccacgtagtgcgaagccgccgcgttgaccagcgcggcgaacaccggcgagctggtgcggcgcgaagtgagtatttcgctcggcccttcggcgggccccatcatctgcgcgaaacgctcgatgctgcgcaccggccgcgccgtgcgcgccgcgagcacagagcccagccagtcgagcatcaggtcttcggcgcggcgcagcaccggggcgggaatgttcgcgaacttcagctcggcagcgaaagtggccagggtttggctgggatgattcgatgaagtcatgagaggccttcagaacgaacgtggcaagccgagcatgtgttcggcgacgtagctgaggatcaagttcgtcgagatcggcgccacctggtagagccgcgtctcgcggaacttgcgttcgatgtcgtattcgcacgcaaagccgaagccgccatggaactgcaggcaggcattggccgcctcccagctggccttggccgcgaggtatttcgccatgttggcctgcgcgccgcaaggctcgcgcgcatcgaacagtctgcaggcttcgtagcgcatgaggttcgcggcctcgatctcgatgaaggcctcggcgatcggaaactgcacgccctggttctgcccgatgggccggccgaacaccacgcgctccttggtgtaggccgttaccttgtcgatgaaccagtagccgtcgccgatgcactcggccgcgatcagcgtgcgctcggcgttgagtccgtcgaggatgtacttgaagccctggccttcctcgccgatcaggttctccgccgggatctcgaggttttcgaagaagagctcgttggtctcatggttcaccatgttcaggatgggccgcaccgtcatgccgttgccaatggcttcgcgcaggtcgacgatgaagatcgacatgccctcggacttcttcttcacgtccgcgagcggcgtggtgcgcgccagcaggatcatcaggtccgaatgctggatgcgcgagatccacaccttctgcccgttgacgacgtagcggtcgcccttcttcacggccgtggtcttgatcttggtggtgtcggtgccggtgctgggttcggtcacccccatcgactgcagccgcagctcgccggtggcaatgcgcggcaggtagttgcgcttctgcgcctcgctgccatggcgcagcagcgtgcccatgttgtacatctggccgtggcaggcaccggagttgccacccgagcggttgatctcttccatgatcaccgaggcttcagtgagcccgagaccggagccaccgtattcctgcggaatgagcgcggccatccagccggcctgggtgagcgcatcgacgaactcggcgggatagccgcgcgcctcgtcgatcttgcggaagtattcgttcgggaattgcgcgcacaggtcgcgcacggcgtcgcgaatgtcggcaaagcgggtgtcgttgtggctgttcatgggtgctcaatcctggcgcgggccgccggcttccttttctacacgttgccagatctcgatcgccatcgggtcgtcgatctcctcgaggatgtggcccacgagcccgatggcgcgcgccatcacgccgaagccgcgaatgatcttccacggaaagccgaactcggcggcaatggcgccgatggcgccggtcgcgttgatgggcagcgacttgcccgagacgcgctcggcctcctgctgcaccgcctgcatcagcgccacgtagtggcccgagaggccgttctcctcggcaatctggaacaggcgcggcgtgcgcggatcgatgggcttgtgcagcggatgcccgaggcccggcacgatctgcttgcgcgcgcgatggtcgccgacgatctcctgcgccatctcggcgagcggccgcgtcggtttctcgccgaagggaatggcctcgtagagcatcttcgccgcgccctcggtgctgcccacgaacaccgtgcccagcccgcacaggccagctgccacggcggcctgcaaggcttcgggcgcacccgcataggtgaggcgtgcggccagcgcgctcggcgtcacgccatgctcgaccagcgtgacgacgatggcgttgaaggtgacggattcctgcggcgtcgggatgcggccggtcagctccaggaaggccatgtcgccgaggttcaggtggccgaggatctcggagggcaggtcgcgcccgcgcacggtgatcttgtcgggcgtgctgtggccgagttcggtgtgcagggatttcttgatctttgtaggcatgcgccgaatctatgccgctctcgcgcgaggtgggtctgtgattgcgaaaccctcccttcggcaaatgcaaatgccgcgcggcggggtgttctgtcacgctgcggcgatggatatcgaatcactctcagccatgcgcgacgccgcgctcgactacttcgtgcgcagccgttcgatccagcggcggcgcgagcgcatggagcggcccgatgccgacgaggcgcagggctggagcgccatcgccgaactggggtggaccggcatgctggcacctgagtccgcgggcgggctgggcctggagctggcgggcgccgcgcaaatcctccgcgccgcgggcgagcacgtcgcgcccgagccgctgttggcggtggccggcctgagcgcgctgttgctcgcgcggctcggcacaccgggcgcgcacgcgctgctggtggaactcgtcgcgggccgcagcctgccggcactggcctggcaggagagcgcgggcgacctgagcgcggtgcctctggcctgcggctgcgagccgcgcgcggggcacgccggcggcgtgctgctgcagggcgaaaagctcatggtgctgcccggcgcggcggccagtggctggctggtgtcggcgcgcggcagcgacgatgcggtgttgctgtgggtgccgcgcggcacagagggcgtgagcgaaacgctggtgccgctggtggacggcagccaggccgcgaacctgcgcttcgagcaggtggcgctgccggcggaatcggtgctggccgaaggcccggccgcgcaggacgcgctgcgccatgcgctcgcggcgggccagatcctgcaggcggcagagctgctgggcgtggggcaagccatgctcgcgcagacgctggcctacctgcgcacccgttcgcagttcggcaaacccatcggcagctttcaggcgctgcagcaccgctgcgtggacatgttcattcatctcgaagtggcgcaggccgcgctcgacgaggtgctggcactggcgggccaggcgctctccgccgagcggctcgaagccgaagccagccgcgtcaatgcgcgctgcaccgctgcggcgctgcaggcctcgcgcacggcggtgcagttgcatggcgccatcggctatacgcaggagtgcgacctgagcctgtactacaagcgcacgctgtgccttgcagcgtggctcggcaatgtcgccgcgcaccagcgtcgccatgccgcgctggccgatggcgcggaagcgcggccggccaccgccgtatgggagggcgagttcccacgcagcgccgactgggccgcgatgcccgaagccgagttccggcgcatggtgcgcgcctttctgcagcagcgctatccgcagcagctgcgctacctctcgcaccgcgcgcgctggagcgagatccgcgagtggtatctcacgctgtcggggcagggctggatcgcgccggcctggcctcaggcgcatggcggcatggggctgccggccgacaagctcattgcatggatcgaggaactcgagcagtacggcgtcgcgcgcgctccggaccagggcatcgtgatgatcgggccgctcttgatccagcacggcacgcccgaacagcagcaacgctttctgccgcgcatcgtgagtggcgagcatgtgtggtgccagggttattcggagcccaacgcgggctccgacctggccgggttgcgcacggaggccgtggccgggcgcgatgcagagggcgatcacttcatcgtcaacggccagaagatctggaccacgctcgcgcaggatgccaaccacatcttcatgctcgtgcgcaccgacaaggccgcgcgcaagcaggagggcatcagtttcctgctgtgcgacctgcgcacatcgggcatcacggtgcggcccatccacacgctcgcgggcgagccccagttctgcgaggtgttcttcgacaacgtgcgcgtgccggccgagaacctcgtgggcaagctgcacggcggctggaccattgccaaggccttgctgggcttcgagcgcatctttctcggcagtcccaagcagtcgcagtacgcgctgggccagctcgcgcggctggcagaggcgaggcgtctctttgccgaccccgtgttcgcgcagcgctttgcggcgttgcggctcgacgtgctcgacctgtcggcggcgtacacgggctttgccgacatcgtgcgcgcgggcaagccgctgccggcttcggtttcgctgctgaagatctgggccagcgaaacctaccaccgcattggcgcactgctggtcgaggcgggcgaagagcagggggccgtagccggcgaccaggtgctggacgggcagagcttcaacgtgctgtccccgttgatcggctcgacggccgcaatgatctacggcggcaccaacgagatacagcgcaacatcctcgcgcggcaggttctggacttgccggcctgagcgatgcgagccgctgaagaaatacacaacaggagacaacgctcatgcaatcgatcgacttcacacgccgtcatgccatggccgcgctggcaggcagcgcactggtggccgcaatgccgtcgcgcaccctggcacagcagcagcagcaacaacagcagctgccgccgctcatcaagctcgtggtcggctactccgcgggcggcccggtggacggcgccgcacggctgctcgcgccggcgctgggccaggagctcggcacgcaggtcatcgtggacaaccgccccggcgccagcggttcggtgggcggcgatgcagtcgccaaggccgcgcccgacggcgcgctgcttttcttcggcgcgagcccgacgatcaccatcaatccgaacgtccagcgcaagatgcccttcgacccgatgaaagacctggtgcccatcgccccgctggtcgactacaccaacgtgctggtggtcaacaaggacctgcccgtgcacagcgtggccgagctgctggcctatgcgaaggcgcggccgggcaaggtgttctatggctcggccggcatcggtgcatcgaaccacctgagcggcgcactgctcgagaagatgaccggcgtgcagctgacgcacgtgccgtacaagggcagcgcacctgcgctggccgatgtgatgggcggcaccgtgaccatgatgttcgacatcatcgccacctcgcggccgttcatccagtcgggcaagctgcgcgcactggccgtcacctcgcgccagcgcaaccgcatgctgcccgaggtgccgacgatgatcgagtcgggtgtggccggctacgacgtgggcggctggttcggcctctatggccctgcgcgcctggatccggcgctggtcgcccgcatcaacgcggccgcgcacaaggcgttggcgcgcgaggacattgccaatcgcctgcgcgaacagggctacgaggtctggagcggcagtgcggacctgctcgcggccaagggccaggccgaccgcaagctctgggctaccgcgtccaagggcatcgaggcggaatagccgatggcaatcacgcgaatccacgaactgctcgaggcacgcgcttcgcgcacgcccgaagaggtctttctcttcgaaccggcgggcggcgtgtcgtatgccgggttgcaggccatggccgaagcggccacgcaagacctgctggccgccggcgtgcggccgaccgaccgcgtgctgctggtggccgagaactgcgccgcgcacattgcgctgctcatggcgtgcagccgcgtcggtgcgtggtcgtgcggcgtcaacgcgcgcatgtcgcccggcgagatcgtggccattgccgagcgcgccgacgcgcggctgtgctacttcaccaccgccgcatcggacgccgcgcgccagcatgccggccgcgccggcgcggtgccctccgcgctgcccggcgtgatgcgctcggccgtgcgcgccgaggcccggcccgaagccgaccccgcgctggcggatacggccgccatcatcttcacgtcaggcacatccggcacgccgaagggcgtgatggtgtcgcactgcggcctgctgcatttcggccgcgtatcggccgccgtgcgctcgctgactgaacgcgaccgggtctacgccttcctgccgatgacgcacatcttcggcattgggacggtgctcatggccgcgctcaccggcggtgccgcgctggtgctgcgcgcgagcttctcgccggccgacatgctgcacgcgctggcgcatgaagaggtgtcgaacctgctggggccgcccacgatgtatgcgcgcctcctggcccacgtcgaggcggagcgcatcgtgccgcgccttccggcgcttcgctatgtgtataccggttcggcgccgctcgacctggggctcaagcagcgcgtggaggcactgttcggccagccgctgcactatggctacggcctgtcggagtacgcgggctcggtgttcctcacgcgcgtggaggcaccgcgcgcggacacgtcggcgggctacgtggtcgaaggtggagaagcccgcatcgtgagccccggcggcaaggatgtcgcgccgggcgaaacgggcgagatatggctgcgtggacccggcctcatgctgggctacttccgcgatgccgcggccaccgcgctggtcatgcgcccgggcggctggtatgcgagcggcgacctcggccgcttcgatgcggacggcgcgctgttcgtggtgggcaggctcaaggagatgatcatccggtcgggcttcaacgtgtatcccgcggagatcgagaccgtgatcggccgcttcgcaggcgtgcacctttgcgcagtggtgggtgtgcccgaggccgacggcaacgagcagatcgtcgcgttcatcgagatgaagcccggcacggtgctggacgagccggcgttgcgcgcctacctggcggagcatctgtcgccgtacaagcggcccgcgcgcatagagaccgtccaggcgttgcccaccacggccaacggcaaggtgctcaagcgcgaactgcaggcacgctgtcgttagcccgcgctggtttcggacatttcctgcaaggagccgcgccgccgtccgccagtgccgcggaggaagagcgcgcatcgttcgtgcatcgatacaggagacacaggacgcacgccatggcagacgacccgaacaagcgcggccccgaggaccggacccgcatcaatgtcaacgagccgcacgaggtgcgctactggacccagacgctgggcgtgaccgaggcgcagctgcgctcggccgtcgcggccgcgggtgtcgaagtgaaagacgtgcgggtctatctcggcaagacctgaccacgatcgcggtcatttgccgcggatctgcagcctcgagcgatcccagcttccgaatacgtaggtacgctcctacactcggtcagggagggggggccgatacttcttgcatccccgcttcaggacgcgaaaaagtgaacgtgccgaacgtgcccattgccgacccccgacccacaggccccggtcgcctgcaggcctgcccacccaacgaggcgaagccttcgtctcccgccgcgcaatgaaggcctcgcccggagcccgcagctggattgcagctggcgtgcggcacgaactgctcacccgcgccttgccggcattgcggcacgacatggcggcgccggtctccgtggtacgcatggccctgctcatgctcaagcgccagatgagcgcgccgtccatcgatgtggccgcctgcgaggaacgcgtcgcgctcatcgacaaccaggtgtccgaattggtggaaggcatccgttcgctgcgcgactgggagctggccacagtggacgacggcatcacgcgcagcgcgctggtgtcgcaatgcgtgggcctgatgcgggctgccttcgacatgcacggcgtggcgctcgatgtggaccccgcgctcgaaccgcaggcgcacgaacctcgacggccgcaaggggctgcgctgcgctatctgttcctgggcgggctcggctatctgcacgatggcgcgtccgacgccggtgcaatccgcatcgaggccgacggtgacgatgcgctccggttgagcgccttgccgcgcgagtccagcggcgtgagccccgtgctcgacgcgcaccgcgcaccgcgcgcactggccatcgatgcgatcgcgctgcaaagcctggccgaagacctgggttacaccgtggcgctcgagcgcgacagcgtgcggttcccgctcgccacggcctgaagcctcggcgctccgctttgcctcccgggcggcgcggcctttgcgctgcgatttgggctgcgcttggcgctggccctctgcgtcttgccaagttcacgaagctcgcgcgcctgggtgtgccgatgcatccgcaagaaggcgagcaagcgctgttccgcggcgtggagtccgcgcgccttgcgtgccgcgctgcgggccgtcatctttcgcagcacttccgacgaggcgtcttcgcggtcgcccgcgagcgcgctgcccagcgccagcacggccgggtggacataggccttcttgcacacggcgggtgtgttgccgagctgcctggccaccgcggccaggatctccttggcgctgtagcggttgccgtcggcggccacacggtccggctcgcaggccagccgcgtgagttccagcgcctgtaccgtgccgtgccaggtccggaagtccttcgccgtgaagcgctcgccgggcgaggcttcggcgatgtagtcgttcacgtcggtggacgacacgctgcgcagctgcccgtcttcttcttcctggtactggaacaacgcctggccgggcaactgctggcactggcgcaccaccttcgccacgcgcggatcgtcgagcagggcctcgtgcatcacgccgctcttgccccgaaagcgcagccgcagcgccgccccccgcacggccgcgtgccggttgcgcagcgtggtcaggccgtaggagccgttgctgctcgcgtactcctcgtttcccacgcgcagcagcgtggtgtcgagcaggcgtaccagcgccgccagcacctgctggcgcccgggcgccgacgtggccgcgcccgcgccttcctgcaggtcgcgcgccacgcgggcacggatgcgcggcagcgcgagcccgaaggcctcgaggcgctcgaacttggtctcgtccttgaagagccgccagtcggcgtggtagcggtactgcttgcgcccccgggcatcgatgccggtggcctggaggtggccgttgggcagcgggcagatccagacctggctgtaggccggcggaatcgccagcatgcggatgcgcgagagctcgtccgcatcgcgcacccagcggccctccgcatcgcggtagcgaaagcggtcgccctgcttcaggcgccggatgcccggcatgtccggattcacgtagaccaggccattggcgatcggcgtcggcttcgaaggcggtgtgggcgacgagagcggtgtggagcgggccggcatgtggttcgggtggtgactgtacccagcgcttgtgcctgcaccggccattgcttcctgtaggacgccgcaatcgacgctggtgcgatggaggctctttgttcccgtgcgtcagggccgcaccggctgcaggtgccacgtcacgttgaagtcgaacggcgtccagcggctcaccgtgacacccgcgcgccgcaggccgcggccggtccaggtgttgcaggtctcgaagaggtgatagccgccttcggcttcatagaaggcgtcgtcgttgccgtagtgcgcgcccgcaatgggcaccgcgcggcccgagggcagcgaggtgcgcacgtagtccacgagctgcgtgtactgcgcctgcgagagcggcagttggtaggcgccgtgccgcagctgcgcgcggcgcaggtaggtcacgtgcagcagcgcacggttgccgccagacagcgcaccgaaggcgcgcgcggccgtcaggtcggcccaggtgggcgtgtgcaggtagaactcgcggtcgccccagccgatggcgatgaattccgcatcgggcggcacggccttgaaatgcgcgaacggaaagagctgccgccagtcgatggtcgccgagcggatcgggaacaccagatcggtgtgcaggccgttgctcagcacccaggcctccacggcgggtgcctccgcgggtgcttgcgccgagggttttgcattggccggccagaacaccatcgcgcaagccacggccgcatacaggcataccgcaaccgtgaaccccagcagcgtgaatgcgagacgccggagccagcgtttcatcacggcttcagaagagcgaggccgtggtcgaagtcgactccacggacgcgcgggaggccgggctgctggcggccggtgccagcgcctccgggcttcccgccttcgcgagcgcgcccacgcgcacgcccagcagccgcagcggccgctcgagcggcacgcgcttcaggcacagcccgccgatctggcgaatcgtcttgccgtcggcggtgaagcggtcgatggtctggtcgcgcgtggcaatcttgaaatcgtcatagcgcagcttgatgccgatggtcttgcccacgtagcccttgcgctgcaggtcttcggccagcttctcgcacaggtgggtgaagatggcgccaagctcggcgcggtcgcgcacggcatgcaggtcgcggtcgaaggtggtctcgcggctcatcgacacgggctcgctttcggtcaccaccggccggtcgtcgcggccccaggccacctcgtgcatccacgcgcccgtggatttgccgaaattctggatcagccagtcgcggtcgcgcgccgcgagttcgcccaccgtctcgatgccgaagcgcttgagcttctcgtcggccttgggcccgatgccgttcaccttgcggcagggcagcggccagatgcgggtctgcaggtcgttctcgtagaccaccgagatgccgttgggcttgttgaactcgctcgccatcttggcgatgagcttgttgggcgccacgccgatcgagcaggtgaggccggtggcgtcgaagatcgctttttgaatcagccgcgccagcgagcgcccgccttcgcgctggccgcccggcacgtcggtgaagtcgatgtacacctcgtccacgccgcggtcttccatcagcggcgcgatctccctgatcatctgcttgaaggcgcgcgaatacttgcggatctcgtcgaaatccaccggcaggatgatggcctgcgggcagagcttggcggccttcatgagccccatggccgagcccacgccgaactgccgcgccgggtaggtggcggtggtgatcacgccgcggcccacgtagtctcgtaggcgcggaaaggcgtcgaccggaatgtcggccagcgtgccgccttcgggcacatggcggatcgcctcgtccacgctgcgccgcccgccgccgatcaccaccggcaagcccttgagctgcggatagcgaagcagttcgaccgacgcgaagaaggcgtccatgtcgaggtgggcgatgcggcggatcggaggcttggtcacgggctgggaactcacggctgcgattgtctcgcggccgggctgtgtccgcccgcgcggggcacgcatgccagaatgcggcggaccgcggtttttgaccgtccgatggcaattgcgacatgggaaggaaggggatctggcatggatgacgaagtcgaaggattgagcatcgcgctgacgccggtgcagatggcggcggtgctgggcgggcaggacgtgcccgaatccgcgagcctgagcaaccggctctgggggaccgtcgggctggtgggcggggtggtggaactggtcggcgccggcgtgctctgcctggcgcccgagcccaccatggtgaccaaggccggctgcgtggtgctgggcgtgcacggctacgataccttggcaacctcgagccgccaggtctggaccggcaccccgcagcgtacggctaccgccgtcactgccagcgcggcggccgaggcgctgggcgcctcgcgcgaaacggccgacggcatcggccttgcggtggatgtggcggtgccgctggtcgtggcttccgggctggtcgccgcgcgcgtgatcgcggtgcgcgccagcaggtttcgcctggagccagtcaatctgcggctgcatgaaggaccgccaggcacaaagatcggcggccacgcgatccgggaacatgtcggcaagaccgaggcggaacttttccagaggttggcgaacaagccgtcgctgcccaaagtgtcgtcgttccacaatctcgacgtcgcagagcgcgccatcagcgccactgttcgtgccaacgccagagccatcagggcgtggtcgcgttcggccgccgtgggctccaagcccgtggcgttcgaccacaacgtgggcagcgtggtgggcatcggcgtgcagcggggcgccaccaccgtcagccagctgaccaacgtgcgcgtgatcctgaacatgaagagctacaacggaatgccgtactacatcctcacggcgcaccccttctgaaaccagcagccggattgccatgaagcgctacgaactcatcgacaacctcaccaaggtttacttcggccaggattacgaatacttcggcgagaccggtgccgaagtcatggccgaataccggaaggcctgcacgcccgccgaacttgaggcgttgcgcgtcgagatcgtcgatttcatgcgctcgcacccggacctggaaaccgacttcccgcgccggttcgagcggccagcccagccggaggacttcggaaccaccatacgcgaattcctggacagcgtgctcgccgcactgaaatagcggcgggcgccccatccgattgccttggtgcgcggtgcgggcaattttcatcagcgcagatcgagtgtcccggccggttgcacctcgccgccaagccacacatccggtccaagttctttcgccagacaggccacgagcttcgcggtgcgcttgcgcagcggggcaatgcgggcctgcagaccggccctgggcagtgcaacggcttggccgggctcatcgtcggaatcggggttgctctcccggatgtagagcgtgccgttgcaggcccagacctccaccgcccacccttggtcctggtcgtcgtagaccatgccttggtcattcccggccacggcggccaggaaatggtccattgcggcgaaggtgtcgtaccaggggaacgacaggtgaacgtccgcctcctcgttgtcgagccgcagatccatccagaaatactggcgcacctgatggagtttcagcgcgtgctgctgggccagcgtggccacccggccgtaatacgcggcaagttccgcctcgtgcccaatggcctcggaggtgcgcgccagcaggcgcgaagcgcgcgggaattccggcaaggcgagcggctcgggctgatggcccggcgcgggacgaaattcgtcccacaaaagaaacgcgatctccggctccagcgagttgatcagcttggcatgggcgaaccagggttccacttgcgtgctcctctgaatggtcgagcctacgaacgtcagctctccatgatgatgcgaacggggctttcggcgagaccgccctgcgctcagcgcgtctccaccgtcgtcagcagcggcgagtcgaacatcgccactggcgagatcacgggctcgtccatcggcaccttgtcgccgtagcgctcgcgcatcttggcgcgcaccgcggggtcgtccaggttgaagctgcgaatcttctgcagttcgccgatgcgcacgccttcttcatgatccggggcattgtgacaaggcttgcctgttgcgcccgctggggtcatcatccgcgccatgcaaaccgtcgcttccattctgtggcgcaggctcgatgcaccgggccatgacgcctgccggctcgagcgcaacgcgaccgcgtggcagctcgacggagctgccgtgttccgcctcgaggaccaccgtatcgcgcaactgcactaccgtgttcgctgcgaccagcactggcacacgcagtggggcacggtgcgcggctggatcggcggcagcgctatcgacctgtccattgctcgcgatgcgcgcggccactggaagctcaacgacgaggccgtgccggacctgtcgcattgcgtcgacctcgacctgggcttcacccccgccaccaacctgctgcagctgcgccggctcaatcttgccaagggcgaaggcgccgatgcgccggccgcctgggtcgatattgacggcggcgtgctcagcgaactgatgcagcactacgagcggaccgcagacgacacgtacgcctacgaggccaagcgcttcgactatgcggcgacactgcgcgtcacggcggacagcttcgtgcgtgactatccgggcctttggatcgccgaggcgtagcgcctcggtcgaactggtgcctggcttcgtctccgcatcgggggccgccatggcgctggaacccggagcaggacattgacatcattgatgagtcacggcaaaccacttcttcgcaccttcgctttcgcgctgctcggcaccctggccccgctggcggcccaggccgccgcctgggggcccaagcccacggcctgtccggcgccggtgcccgaggccacgcgctgctataccggcgaagacggcacgggcgccttctactggatcgcgatccccaaggattggaaccgcgtgctcgtgatgcacgcccatggcggtcccgagaccggtccgcccaagctgtcgcgaagcgaggaagacctgaagcgctgggccgtcaccgtgaaagccggctacgcatgggccggctccacctaccggcgcggcggctatggcgtgaccatggccgcggaggacaccgagcgcctgcgccgcatcttcgtgcagcgcttcggcccaccgcgccgcacgctgctgcatggccagagctacggcgcgggcgtggccgcaaaggccgctgaactccatgcgccggcgggcgatgcgaagagcccgtacgacggcctgctgctcaccagcggcgtgctcggcgggggcaacagtgcctacgatttccggctcgacctgcgcgtggtctaccagtacgtgtgccgcaaccatccaaagcccgacgagccgcaataccccttgtggcagggcctccccatggattcgcagctcacgcgcgccgaactggctgcacgcgtcaaggagtgcaccggtgtcggcctgcccgccgcgcagcgcacgccggagcaggcggcgcggctcaagaccatcctgtcggtggtgaagatccaggagcgctcgctgcagggccacctgaactgggccacctggctgttccaggacctggtgcagcagcgcctgggcggacgcaatcccttcggcaacatcggcgtggtctatcagggctcggcggacgatgcgacgctcaacgccggcgtggcgcgctatgccgccgatccgcaggccaagggcgcgctcgccgccgacagccagcccaccggccgcaccgcgctgcccaccgtggccctgcacgccatcgacgaccccacggctttcgtcgaactcgagaacgcctaccggcgcattcgcgatgctgcgggcacgggtggcaccctggtgcaaagcttcagcgccgagcgcgagcacagctacctgagcgattcggaatacccggcgctcttcgatgcattgatggactggatcgacaagggcgaaaaacccacgcccgcgagcctggcgcaacgttgcgcggcgctgatgccgcgctacgacaccgacggcaagaacggctgccacatcaagcccgagtggcaggcgcccgcgctcgaaacccgcgtgcctgcgcgggctccctgattttcccccgggcctagaacgtgcccggcagcaggatgctcgaatccacgttctcgatatcggtgcgaccgcagaaggccatggtgatgtcgagttccttgtggatgatctgcagcgcgcgcgtcacgcccgcctggccgtaggcgcccaggccgtacagaaagctgcggccgatgagcgtgccgcgggcgccgagcgcgcgggccttgagcacgtcctggccgctgcggatgccgccgtccatccacacctcgatctcgctgcccacggcatcgacgatggcgggcagcgccgcgatggaagagggcgcgccgtcgagctggcggccgccgtggttggagacgatgagcgcatcggcaccgctcgcggcggcaaggcgcgcatcttccacgtccatgatgcccttgaggatcagcttgccgccccagcgcttcttgatccattcgacgtcggcccagctcagtgccgggtcgaactgctcggccgtccacgacgcgagcgacgacaggtccttcacgcccttggcatggcccgcgatgttgccgaaggtgcggcgcctggtgcccagcatgcccatgcaccagtgcggcttggtcgccaggttgatcatgttggcgatggtcggcttgggcggcgtcgagaggccgttcttgatgtccttgtggcgctggccgaggatctgcaggtcgagcgtgagctgcagcgccgacacgttcgcggcgcgcgcgcgttcgatcagccgctcgatgaagtcgcggtccttcatgacgtagagctggaaccagaacggatgccggccggtgtgctcggcaatatcctccagcgagcagatgctcatggtcgacagggtgaacggaatgccgaaggccttggccgcgcgcgcgcccaggatctcgccgtctgcgtgctgcatgccggtgagcccggtgggtgcaatggccaccggcatggccacgtcctggccgatcatggtggtgcgcgtggagcggccttccatgttcacggccacgcgctggcgcagcttgatcttttgaaagtcgctctcgttggcgcggtaggtgctctcggtccacgcgccggagtcggcgtagtcgtagaacattctcggcacgcgccgcttggcgaccacccgcaggtcttcgatgcaggtgatcttggaaaggtctggcacgaggcggtctcctgaggggtcttcggttgttcgtttttttgcgaaggcccgccattatgggcaggcccgcagcggcccgagtgtgatgcgcgcggccacggccgatatgaaaattacccggtccgcggctgaaaagaattcagttcagttcaatcgcgcagcgcctggcgcagccattcggcgaaggtcgcgcactcccaccgctccatggcgcccggccgccagcagatgaagtaggcgttgggcgagggcacgctgcgtggcgaaagccgcacgaggcggccgctgtcgagccacgcgctgccgagcttcaggtgcatgagcaccacgccgaagtcttcggccgccgcgtcgagcgccaggcccaggtcgttgaactggtggcccgtggccggctcgggcaggccgatgccgcaggccttgaaccaggtgcgccaggattccagcggcgtacgcagcaactgggcgcgcgagatttccgcatcggtggcaaagccgtcgaaggggccgtgccgctccaggtaggccgggctgcacacgggcgagacctcgtcggccagcagctggaaaaactcccggtcgtgaaagggcccggtgccaaagcgcagctcgatatcggcctcttcggccgtcatgttgcgcaccggcgtggtcacctgcagcatcagttcgatgttgggataggcatcgcggaacacggccagccggggcagcagcatctggcgcgagaaggtgggcgtcacggccacgcgcagccgccgcacctgcgatgcgggctctcgcccgggcacctgctgcagcgccgcaatggcctcgcgcacgcgggccaggtaggccacgccatcggcgctcaggctgaagtcgttgcccacgaagaacttgagttcgagcagcgtttcaagctggcggatgcggtggctcacggcactgggcgtcacgctgagctcttccgccgccaggttcacgctgcgcagccgtgccacggcctcgaaagcctgcaggccctgggtcgaggggagtcgcgttgaagccatgtgtcgttccgggctggatcttatcggggcactgcggggtgtgacgcggcggccaatgcctggagaaggcgccgcaagtcgtcgatggcttcgcgcgccagggccgcgtcgcccatctgcgccttgacgatggcgccgtccacgccgagcgcggcggcctgtgcaagcgccatgcgcgagggtgattccgcgggcaaaaggcccgcgatgacttccaccatctcgcgcttgtgttcgcgcgcacgctgcgctgcaccttcgacgctgccgcccacctcggccaccgcgttgatgaaggcgcagccacgaaacaccgggtcggcgaaccattcggccatcacgtcggcgagcagaagcaaggccccggcatcgccggcccgttcgtgcgcgccgcggcgtcccagtgcgtcgacgaaccaggccatccaccgcgcgtggcgatggtcgagaaattcgcgcaccaggtcgtccttcgacgggaagtgccggtagaaggtgaccttggtcacgcccgattcggcaatgacgcggtcgatgccggtggcgcggatgccgtctgcatagaagaggtcgtgcgccgtgtgcaggatgcgctcgcgtgcgggcagtgcggagatgtccatggcgctattgtaggcatgtagacagatctgtctacatgtggcacattgcgggctcgcaccgctccttcatccactccgcttcaacgaaagacgctcatggaatcccgcccgccgctgcctcccttcaccctcgaaagcgccacgaagaaagtccaggccgccgaagacgcctggaacacgcgcgacccggttcgcgtgagcctggcctacacgcccgataccgagtggcgcaaccgcgccgacttcgtcaacggccgcgagcaggtggtcgaatttctcacccgcaagtgggagcgcgagcacgactaccgcctgaagaagcagctctgggccttcatggacaaccgcatcgcggtgcgcttcgaatacgaatggcacgacgaggccgggcagtggtttcgaagccatggcaacgagaactgggaattcgccgagaacgggttgatgcaaaagcgctttgcgagcatcaacgaccagcccatcgaggagtccgagcgcaagttccgctgggagcgctgatcggccctgtccttcttcaggaacatttgttgcttgcttttggtgcatggaaacgcccgtactgaaccccaccgccagccacccgctctggcagcaccaattggggctgctgctggagtccaccggcgagggcatcttcggcgtcgacctcgacgggcactgcatgttcatcaaccgggccggggcagagatgctgggccacgaggcgcgcgacgtgatcgggagcaacatgcacgagctcacacaccactcgcacccggacggttcgcactacgccgacacggactgtcccatcttcaatgcctttcgccgcggcctgccgtgccgcatcgacaccgaggtgttctggcgccgcgacggcagcgcctttgcggtggagtattcgagccatccgatcatggacggcgcgcaggtgcgcggcgccgtcatcacctttgtcgacatcaccgagcgccgccgccaggctgaggcgctgcagcaggccaaggacgaactcggcctgcgcgtgcaggagcgcacgcgcgaactcagcgatgcgctggtgcaattgcgcgagctctcggcctggctcgacaaggtgcgcgaagacgaacgcacgcgcatcgcgcgcgaggtgcacgacgaactcggcagcctgctggtggcgctcaagatggacgtcaactggatcggcaagcgcctgggcgagcagcaggagcgcgcacccgatgccgcgcaggccatgcgcgaccagatgcgcggcaagtgcggcaacatgagtcagctgatcgagcgcgcggtcgacaacgtgggccgcatcatcaccgacctgcgccccagcatcctcgaccaccagggcctgtgggcggcgctcgaatggcaggcgcacgagttcgtgcagtctgctgaactggcgctgcaatggcacttcgacgtgcctgcgggcgtggagctgcccgagcctgcggccattgcggtgttccggatcttccaggaaatgctcagcaacgtcgggcgccatgcgaaggcgcgcagcctcgacatccgcgtcggcgtggaacagcggcaactgaacatcagcgtgcgcgacgacggcattggcgcaccggcagaggccttcgaagcggccacctcctatggcgtattgggcatgcgcgagcgcgcgcgccacttcggcgggcgcatcgacatccacagccaggtgggcgagggcagcaccttccgcctgcaactgccgcttccgctgccggtgtaggcttggcggcatgaacgagatccgcgtgctcatcggcgacgaccaccgcatcgtgcgcgagggcctgaagcagatgctgggcgatttgtcgaacggactgccctcgatggccgttcgcgcggaagcgcagaccggccccgaggtgctggccgccgtgcaggaactcggcggccccgagggcctcgacgtggtgctgctcgacatcgcgctgccggggcgcgacggcctcgacgtattgcaggccctgcggaaagactggcccacgctgccggtgctgatgctcagcacctatcccgagaagcagtacgcggtgcgctgcatcaagcttggcgcttcgggctacctgaacaagagcgccgatgccgacgacatggtgagcgccgtgcgcaaggtggcggcgggcggcctttatgtatcggcggccacggcggaagcgctggcggccgcagtgggccgcaacgtggggcagggacccgaacagctctcgcatcgcgaacaccaggtgtaccggctgctcagcgccgggcacagcgtgagcgaaattggtgcgcagctgggcctggcgcccaacacggtcagcacctaccgcgcccgcatcctcgaaaagaccggcaccaagaacgacgtggagctcgcgctgtatgccgagcgccacggcaaagcggcgcccgcagcatgaaaacgaagccggcgggcatcgccttgtagtgccagccctacaaggcctcgacaagcgcggcacgatctgcggtcggcaagcctttgggcctcgctttcggcccggcccttgcatcgtgcaagcatcttttcaccgaggtgcaccaccatgtccagcccatccgattcgaccgcctgcgatctctacgatgccgaccggccactgaacatgcgatgcgcctgcggccgcagccacggccgcggcgccgacatcgaggtgagccccgacgacaagctcgaggccagcctcatgaaggcgctgtttccggtcgacagcgtgcgccgcaacttcctgcgcgccgtgggtgccaacaccgcgcgcgccgccattgcttccgtgctgccgctgggcgcgctgcaggccatggcgcaagacaaggcgccgctcgaaaagaccaacctcaagatcggcttcattccgatcacctgcgccacgccgctcatcatggcgcacccgctgggcttctatcagaagcaggggctcaacgtcgacgtggtcaagacggcaggatgggcgctcatccgcgacaagatgctcaacaaggaatacgacgccacgcatttcctgtcgcccatgccgctggccatttcgatgggggccggctccaaccaggtgccgatgaatgtcgcgaccatccagaacaccaacggccaggcgatcacgctggccaacaagcacaaggacaagcgcgacccgaagatgtggaagggcatgaagtttgccgttcccttcgagtacagcatgcacaacttcctgctgcgctactacgtggccgaggcgggcctgaaccccgacaccgacatccagatccgcgtggtgccaccgcccgagatggtggccaacctgcgcgccggcaacatcgacggctatctgggccccgacccgttcaaccagcgcgccgtgttcgaggaaatcggcttcctgcacctcttgacccgcgacctctgggacggccacccctgctgcgccttcggcagctcgaccgaattcatccagaagaaccccaacaccttcgcggcgctggttcgctcggtgctcaccgcatcggccatggcgcgcgacccgaagaaccgcgagctgatcgccaaggtaattgcgccggcgcagtacctgaaccagcccgagaccgtgatcagccaggtgctgaccggcaagttcgcggacggactcggcaacatccgcacggtgcccaaccgcgccgacttcgatccgattccctggcagtcgatggccgtctggatgctcacgcagatgaagcgctggggctacgtgaagggcgacgtcgactacaagcagatcgcggagaaggtgttcctgctgaccgatgccaagaagcagatgaaggcgctgggccagccggtgcccgagggggcataccccaagttcaccatcatgggcaaggtgttcgaccctgcgaagccggacgactacgtcaagagctttgcgatcagcaagctggcggcctgacacgccatgcgcaagaacctcacgctcaaggcggcgctgctgtcggtgctgctgctcggcctggtgctggccgtgtggcagctcgccaccctgccggctgccggcaccacggccgccgccggcatgaccgccgagcagatcgaataccagaagatgctcggcaaggacccgggccaggtgaagagctcgggctttccgtcgccggccgagatgggcggggcggcctggcggcacctgtccgatccgttctacgacaacggcccgaacgacaagggcatcgcgatccagcttgcctggtcgctcggccgcgtggcgctgggcttcctgctggcctgcgcggtggcggtgccgctcggcttcgtcatcggcatgtcgccgctgctgcacaaggccttcgatcccttcatccaggtgctcaagccgatctcgccgctggcgtggatgccgctcgcgctctacaccatcaaggattcgtcggtcagcggcatcttcgtgatcttcatctgctcggtgtggccgatgctgctcaacaccgccttcggggtggcctcggtcaagcgcgaatggctcaacgtggccagcacgctcgaagtgaagccgctgcgccgcgcgttccgcgtgatattgccggcggccgcgcccaccatcctcacgggcatgcgcatcagcatgagcatcgcgtggctcgtcatcgtggcggccgagatgctggtgggcggcaccggcatcggctacttcgtgtggaacgaatggaacaacctctcgctcaccaacgtgatcttcgcgatcctggtgatcggcgtcgtcggcatgctgctcgaccaggcctttgccgggctgcagagaaaggtcacctatgtggagtgatcgattggcacaaggcgctctcatgacacctgttcccgcccctttgcccgccgccggcggcttcctgcgcatcgagcggctggccaaggccttcgcgcccgcgcggccggtgttcgccgacgtgtcgttcacgctcgaccgcggcgagttcgtctgcatcatcggccactcgggctgcggcaagaccaccatcctcaacgtgctggccggcctcgacgaagcgagcgcgggccacgtgttcatggacggccgcgaggtgtccggcccgagcctggaacgcggcgtggtgttccagagccatgcgctcatgccatggctcacggtgcgcaggaacatcgcgttcgcggtggtctcgcgctggcccgactggtcggccgctcaggtcaacacgcaggtggaacgcttcgtggacatggtgggcctgcaggcggccatcgacaagaagccctcgcagctttcgggcggcatgaagcagcgcgtgggcattgcgcgcgcctttgccatacagcccaagatgctgctgctcgacgagccctttggcgcgctcgacgcgctcacgcgcggcaccatccaggacgagctcatggccatcgtgcgccggacgcagcagaccgttttcatgatcacgcacgacgtggacgaagccatcctgctggccgaccgcatcctgctgatgaccaacggcgtcgaccagccgggtggcggctggcggcccggcaacatcgccgagaccgtggtcaacccgctgccgcgcgagcgcacgcgggcttcgctgcaccacctcgatggctactacgcgctgcgcaaccacatcgtcgattttcttgtcacgcgcgccaaggcgtcgtgattcccacctcattcattcatccaactcatcaggagccaacccgcatgaaccgcaacgacgttaccgagaagatcatcaccgtgaaggtgtccaagggcatccagtgggccgacgtggccaggaaggtgggcctctcgaaagagtggaccaccgccgcatgcctcggccagatgacgctcgacgacaagcaggccaagatcatcggcaagatcttcggcctcaccgtcgaagagcagaagtggctccaggtggtgccctacaagggttcgctgcccacgcccgtgccgaccgatccgctcatctaccgctggtacgaggtggtgagcgtgtacggcaccaccatcaaggaactgatccatgaagaattcggcgacggcatcatgagcgccatcgatttcagcatggacatccagcgccaggccgacccgaagggcgaccgcgtcaatgtggtgctctcgggcaagttcctgccttacaagacctactgataagacctactgacgcggcccctcagaacgcgtgctcggccggccgcgggcgccatgccgtgcgccggggcgccgagatgctgctgccttcgatggcgcccgcaatcgagcgggccacggcctccaccggcaccgcgatgcgccgccgcgtgaccatgcgctcgaacgagctgcaggccgcgatgcgatcggccagcgtgcggtccgcctcgctcacgtcggggcgtaccaccgtcacgcgcacgcggcccgcatgctcctgccgcaacccttccgaaatggcgtcgactgcgtactgcgtgccgcaatacaccgctgaattcggcgacacgccatgcgcgggcaccggcgccacgttgacgatgtggccccagccctgctcctgcatcgtcggcagtaccgccgcaatgcccagcagcacgccacgcaggttcacgtcgatcatcagttcccactcgtcgaccttgcgtgaccacagcggcgagagcggcatcacgcccgccgcgttcaccagcacgtcgatgcggtcgtgcgtctcgagtgcgaactcggcaaaggcttccacgtcgggccgataggtgacgtcgagccgctggaagctcgccgttccaccggcggccgtgatgtcgtgggccagtgcctcgagccgctccgtgcggcgcgcgccgagcaccaccttggcgccgcgacgtgccaagagccgcgcggccgcctcgccgatgccaccgctcgcgcccgtgatgaggacgactttttcctggattgcgctcatgagaaactcctcgtgcgggttggtgtgaaccatggcgcaacgctgcgccgggcatggaggcaagtctcgcgcggatggtgcttcgggcgttatccggatcgaacaaggttcttgcctgatcctgcagaagtggtgcccgccgcggccggccgggtgtcatacgctttctggcagatggccgcgtgcgcgcgcagccgcgacactccgggcatggataccgcaccgcccccattccctttcgagatccaactcttcgacacgccgaccggagccgcgcgcgcggcgctcgaagccgtgctcatcgagtccatcgaacggcgcaaggagttcggcggcatgatctgccagtggggcaccaaatacttcgccatgcccccacgcgagggagacaccaacaccgtcgacgtgggccaccgcggtggcaacaagggctgccccgaaggcaccagcgccgtggcttactaccacacgcaccccgcggtcaaaggcgccggcttcaagatggagcccaacaagttctcaccggaagaccggggcgtggcggacgatttcggaatcgatgcctatgtcggcagcgtgtcgggcctgttcctcaaatacgaccacaggacgaagaagaccgcagtcgcggggccgaggctgaagaactgccgggatgaaatgatcctgcgcgatccgcccaaggtcacgcccagatcgaggacgcgtgcacggctgaacgccacgtagccgcaaccgaaaacccactgccgccggtcaatagggcggagccttctgcgcccgctgcgtgcgcgcggcttcggtccaccaggccaggtcgtcggcgaatcggccgaacgagcgctcgagcgattcgcccgggccgccggtgggcttgccgtccgtatccagcgtctgcgagatggggccgacggccagggtgctcgagatgacgaccattcccatctcggacaggatcgaatgccacaaggtgcccgagcgcacacccgaaaaacgccccgccgaatagctggccacagcggcgggacgccagaaccattcctccaggaagtggtcggtcaggttcttcaagccgggctgcgggccccagttgtattcgccggtcacgaagacgaaagcatcggcgccgcgtatcttctgcgccagcgcttccatcgccgcgggcgcggtacctttgggatattccttgtacatgcggtcgagcatcggcaggccgacggcctgggcgtcgatcagttcggcctcggcgccgcgcgcggtgaggccggccaccacgtagtccgccaggcgaatgcccatgcggtccgatcgatacgagccatagaacaccaggatcttgtcagccatcttcgctccgttcgagaggccgggggcggccacgcagcgaaggctacagcatcgaggccctccctcatgggtcatttggtagcagcttcttccaggcagtctggctaccattcccgtccatgaaaaagccgccgccagccctttgcaccgtcgccccgatgctcgccctgctgctggccggccaggtctttgccgcacccgccgcgcagccgttcgacgtggtcaggaagccggagtccgtcgaccccgaatggcgcgcccgtctgtgtgcgctgctgccgcagccttgcgatccgcagtcccttgggttgtaccggccgcgtggcgctgccgcgggcgactacgcggtgttgtccgacgaaccgctggccatggcgatggtgcgcatcaagcgcggcgcagattccagaacctggcagctggctcgcctgcatgacttcagcagctatgccgccgcgttgaagaaagacggcgccggcatgcccgaggcgcgtgtctcgctcgcgccggccctctacccgctggccgaagggcaatgggccgtggccgtgctccagacggtgtccgagatgtattcgggcggcggcgcctcgttcaccaaggccgacttcgttccgctcggcgaaagcaaggccgcgtacgacgacattcccttttcctgctcgaagatggtccgtgcctgcttcagcgaaaaggaatacaagcagtcgaagcattgccacgacgagagcagcggcagcctgcgcatcgcctatggcgaacctgcccggccgggcgagccctacaactggcaattcacgtggctgcaaagcgactggccggcgcacacgcccgcgagcgccgcgaccaccacgcgcctgcatttcgccgccaggaccaccgaacgtgcggggttctgcggcggtccgcagtagcggccgggtggccgctttgcccggcgcggcgcgcttgcgtttcttccctcttcttcttcagtgccgcggaatcgtgaccgtgcccacgtgcatggtgcgccccgcgccgatgccggccatcaccagcgcgatacccagcccgatgaagagccatgacgacgcgcggaagctgccggtccatccgtgcagcaggccggccatcagcgggccgcaggccgccacgacatagcccacgccctgtgccatgcccgagaggtgcgccgccacgtgcgaatcgggcgagcgcagcacgatcagcgtgagcgccagcgcaaaggtgccgccctgcgcaatgcccagcagcacggcccacaaccacacgccgccgagcggcgcgaacagcatggccagcatggcggccacggtgagtgcggccagcaccaccgccagcccgcgctggttgcgcagcctcaccgccacggccggaaccacgaggcaggtcaccacctgcgtcatgaccgacagcgacaccacgtagcccgcggtctcgccgccgagcccgcgttcgcgcaggatgggcgcgagccagcccatcacgatgtacgccagggccgactgcagccccatgaagaacgtgacctgccatgccagccgatcgcgccacagcccgcgcacggtgaagcccgattcgctggccaccggcctgaggggcagggcctgcggcgcccagatcagcgtgacgagcaaggccggcaccgcccacatggcgagcgcataggtccagctcccgccgagcgcatgttcgagcggcaccgtgaggcccgcggcactggccgcaccgccgcataccgccatggtgtagaggcccatcatcagcgccgcctgcctggcgaagtcgcgcttcacgaggccggagagcagcacgttcgacaccgcgatgccgctgcccgcgatggccgaggccaggaacagcagcgggatgttgcccgtgccccgcagcagcgtgcccaccaggatcagcaccatgcaggcgagcagcgtgcgctcggtgccgaagcgccggccaaggcccggcgccagcggcgcgaacacgcccaggcagacgatgggcagcgtggtcaagaggctcgcggcggtggcggagaggccggtggccgcgatgatctcgggcagcaccaccgacaggctggcgaacaccggccgcaggttgaatgcgatcagcaccacgcttgcgcccagcaggatgcgccggcccaggctgcccgccggcgtggcgcgcggcgcgggcatgctgtcggcctcggcgtcgatcagcaggtcgtcggccgcgcggcctgccccgatcggcactgcgctcatcggacgggcgccgcgtcctgcgccagcgcgtcgatcatgggcgacatgaaggcacgcaccgcctccgcggcgcggtcggggtcgcggcttgcaatggcttcgacgatggtggtgtgcacggccgtgtcgggttccggcaggccggtgttcatcgtgctcgcaatggtctccttgatgtagccggcgatgaagcggcaggtctcggccagcgcgagattgccggagatgtcgacgatcgccaggtgaaaggccaggtcgcgctcgatgaagctcgcgccgccgtcctttgggtcgggcacgccgcgcttttcgagcagggttttcaggttgcgcaagtccttggcggtgtggcgcagcgctgccaggcgcgcggcctcgacctcgagcgcgcgccgaacttcgaactggtctcgcaggctcgcgcgccgcatcttctgcaagctgagcgaagggtcgaagccggagcgcacgtaggtgccggagccctgccgcacctcgagcaggccgcgcgagaccagcgtcttgaccgcttcgcgcacggtgccgcggctcacgccgagcagcagggccagttgcggttcgatgggaatgcgcgaaccgaccgtccaccggccggctgcgatctcggcgcggatgctgtcggcggcgctgtcggccagggaggtgcggggagcttggaggagcatatgaataagaaaggcctaattcattgaatcatttgacgaattttcgcgcagatggattgtcgcagtcggccgcaggggtttggggaccggcgcagggatgggagctccagccggtgcggtcgcttttcagcctcagacaccgaggcttctgcaagtgcgatttacacaattgccgccaaacagtgaactattcccggatcggcaaagccttgtttacaaaggttaaccaatcttgtcttatcgttcgaaaatgatactaaaggccgctgcgcttattgcgtgagggcttcatttgcgaagcggcgcggccgcccaaaacgccgatgagagcgttcattaagaaaacaaacagggttcccggaagtcgaaatgaaggatttttctttgtcggatgtccggcttttcaccaaagccgcccagctcggaggactgactccggcagccgacgtgctgaacgtgcccaaggcgtccgcatcgcgccagctccagcggctggaggcgacggtcggacaccagctgctgcatcgcggctccacgcgcttcgcgctcacggaggagggccgggagtttctggtcgcggcccagcatgtgctgaccatcctcgatgacgtcatgctgaacctatcctccggcagcggtacggtgggcgggcggctgcgcgtggcggttcctcactactacggcagggaactgctcggggcgcatctgcccgatttcatggccgcctatccgcagctcgaggtcgtggtcgaaacgggcaatgacagggccgatctgtatcgcgacgaggccgatgtggccatccggcgcggacgggaaggctgcgacgagatggtggcgcgccatctgaagaacgagccgatggtgctgtgcgccgcccccgattacctcgcagcgcaccccgtcctcgagggggttcccgatctggcgtcgcatgcctttctggtcaccgagggcgagggacgcaaaaaggaaatcagcctttcgaccgcgggcaagatccaccgggtgcgcgcgggcagcgtattccaatccgacgatctggaattgatcctgaaattgacaatagccgccaaaggcatcgggctggtccctctggcgatcgcccaaccgcacatcgacagcggacttctggtttccgtgctgccggcgatcaaattgaagccgcaggaaatcaatcttgtctatttgccgtctcgccgcaattctccaaagatcaaggtttttgtcgattacgtcttgaatatcttcaagttttcttgatacggcaaggacgattggctcgcaaccgctgagccaggcatgggcttttttcccatttttctttgcatcccgtcgaacgccgcgagagggttttcggtcgctcgcgtatggccttccgaggggaaagcgaggctccctcggcctccggttgtcgaaaccggaactgttgttccgaatgcacggttgtcggtttcgattggtaccaaagtatcagttttgaactacacttagtaaccaaaaagcgatagttggtaacagttgatcgactgaccgcgacagagaaatcgcagcagtccagagggcagcgccgcagcgatgcaaatcgaaaaggcgctgatcgctcatccaaatgccggcgcttgcaatgccggcgattcctcccgcggcccgagccgcttatttcatgccggcatgcgccggggtgaactcctgtgtgtcttgaatctggagcaaccatgtttattaaaaaactgactcaaatcctgaattgccgccttgccggcctgggcgccagcgcgttcctgctggccgggctgaccggtttcgccggtgctgccgcggcccagtccgcacccgccgccgccgaggccgcccagaagaaggccgttgccgtcgtcctcacccagtccaaggtggtgaaggacgcacagggcaaggaacagctggtggacgccagctcggtcaagcccggcgatgtcgtcgagtaccgggccacctacaccaacaacaccggcaagccggtcaccggtcttgtggcggatcttccgattcccgaaggcctggagtaccagccgcgcagcgccaagccgggcgcaggcctggtgcaggccgcgacgaaggacgccgtgttcggcgccgagccgctgatgcgcaaggccgctggcaacaagtccgagccggtgccctatgccgactaccggtcgctgcgctggacgctgggccaactgcccgccaacggcagcaccgccgtgagcgcgcgcgccaaggtcgaggtggttgtgccgccgcccgctgtggcggtgcaggccgcgtccggcgctgcgcgctgatccggcacttcgctccgtccacccgtgccatctgatttctttcgagtgcaacccgctcgccgcgttttcgagcaacgaaacacggcagccgggttttttcctgttcctgaccttttttgacaaccgaggagaaaccacgtgatttccaccctgccaacccggcgcagcatcggcctcaggccgtctgcgtcgtgggccggcgccgcagccttgacgctgggcttcctgttcggaagttcgaccgcactggccgctgcaccaccagccaataccgtcatcggtaaccaggcttcggccacttattccgacgcagccggcaccacccagctggccacgtccaacctggttcagaccacggttcagcaggtagggtcgttcacgctcgactcggtcaaccaggtcacgacggccatcgtcaacaccaagatcggcgcggcaggctccatcgtctacgcaccgcacacgttgaccaacaccggcaacggcaccgacaccttcacgctgacggtcgatgccgacaccgacaagttctccaaggtcgaggtctaccccgacgccaacggcgacggcgtgcccgacggcaccaccccgctgtgcacggccgcagccgcgggcgtctgctccgtgcccgcacagagcgtggccggcaacaacggcgtgttccgcttcgtcgtggcctacacgattcccggtacggccagcagcggcgccggcgctttcgacacggcgaccatcaccgccactccgggtaccgcggcgctgtacaccgcgccgaatacctcggcggccgacaaggaccagatcacgctgacgacagcggcggcgttcaacgtcaccaagtcgatcggcattccttctgtggccggtccgggcaatggcgcctggccgaccgcgaccaacggcggtccgcgctcgacctcgacaacttgcgccgcgacctggtcggccggcctcgcttccagcgcgacctgccagtacacggtctacacgctcaccttcaacaacacgggcggcgccgcaggcaagttcgcgatgtccgacacgctgccgagcggcatgacctacgtcgcgggttccgcggtgtggagcagcttgcccggcaagggcttggtcaatggcgacattcccgccactcaacctggcatcgactttcaggccagcggcaacaccgtgaatgccgtgatcaagtcgctgggccagaacgtgacgcagaccgtgagcttcgtggtgctggtgaacagcaccgccgcgatcggcacgtccaccaccaccaacgtgggccagttcaatccggcggattcgcccacggccaccgcagcggccatcggcacccttggctccagcaccaacccgtcggcctacacggtcgtggcgagctacagcatcgcggtcggtaccaacccgtcgaccgccgccaccgccgtcgacacgacggccggcacgcccaacggcaccgcagccgacctgaccacgcgtccttcggtcgtggccggcggcagcgtcaagttcgcgcagtccgtgttcaacgcgggcaccggtaccgacaccgtgaacctcacgatcgcaacaggcaccttcccggcgggcacgaccttcgtgctgttcgcggccgacggcgtcacgccgctgctcgacaccaccggtgacggcgtgcccgacaccggccctatcgcggccggcggcagcgtcaacatcgtggtgcaggccaacgtgccctccgccacggcggtgggtgcgggtccgttctcggccacggtgacgggtcgctctgcgggcgacaccaccaagatcgacgccacgcgcgacacggtcaccatcgtcgtcggctcgctggtcgacctgaccaacaccgcggcaggcacgggcacgggctcggcggcaggcggcgacctcggccctggcccgagcccgaacccgaccacgaccaactcgacggatgccggcaccggcacggtgttcgcgctgttcgtcaagaacaacgactcggtcaacaacacctacaacctggctgccagccagtcgaccagcttccccggcaccctgccgaccggctggacggtgaagttcgtggcctcgggcggcacttgcgcatcggcagcgatcaccagcgtggccgtcaatgccggcgcacaagcgcaggtcgctgcctgcgtgacgccgcctgccacgcagttgcccgtcaccgcacagaaggtctacttccaggtgcagtccaccgccgtggcttcgaccggtgtgatcgtttccgacacgaagaccgacgccgtgaccgtgaccgctgcacagacgctgagcgccacgctcacgccgaacaacagcggccaggtcgcaccgggcggcaccgtggtgtacccgcacacgctgaccaacaccggcaaccagagctgcggtgcgtacacgctgacggccaccgtgcctgcggccgacgccacgctcggctggaccaccgcgatctacctggacgtcaacggcgacggccagatcgacgcgggcgacacgctggtgaccggcccgcaagccggcccgctggccgtgggcgcatcgcagaagctgctggtgcgcgtgttcgcaccgggcggcgccagcgccggcgcaaccgacaccacgaccgtgaccgcgaccttcaccgacgcggcgagctgcggcgcaccgtcggccaccgacatcagcaccgtgatcaccggccagatccgcgtcctcaagacgcaggcagccgacctcacctgcgatggcacggcggacggcgcattcgcggcagctccgctgtcgctgaagcccggccagtgcatcgtctacaaggtcgtcgccaccaacgaaggcacggcatcggtcaccaacatcgccatcaacgatgcggtgcctgcgtacacctcgctgagcgccacgcaacccgcggccgcgtcgcgatgcacctcgaccggcgtgaccggcacggcgctcgtctacgcacagaccgccaccgcggtgagctgcggcagcgccgccaacaccgtggccccgagcggcacggccacgctgaccttcgccgtgaagatcaacgagtgacgacaagggtttgagtcgctggcgggcctcggggtccgtcggcttttcgcgaggcgctgcctgtcggcatgcctcgcttttttcccttgccgctttcacccagcacgcgaccgcgcctgaccagcaggcggcagaggaaaaagttctttgaggtttagacggcccgcgccgcgcgcgggccgacggaaggttcgtggcgtgcaatttcttctggcgtatctgagcacctgctcgcagcgatggcgaggcggcatggccgcagccgtcgtggcgacggcggtcctcggctgcacgctcgccggaactgccgcgcacgccgcgcccccgtccggcggcaccgtgatccgcaacgtcgccaccgccacctacgtgccggccggcctttcgcagaccgagacgtcgagctccaatggcgtcagcgccaccgtgctgccggtcgaggcgctggtgctcacgcaggaccagtcggtcagccgtccgccggccgtcgtcgtcacgctgagccacctgctcgccaacaccggcaatgtgccgtcgagctacaccatcggccttgtcaacggcggcgcgggctgcccggccggcgcgctcgacatgtcggcgctgcgcgtggtgcgcgacaccaacaacaacggcgtggccgatgcggccgacccggtgctgccgctcggcgccggcggcgccatcgcgctgcagtccggcgagaccgcagcgctgctggtgcagggcaccgtccctgccgcggccagcggcaatgcctgcgtggcgctcaccgccaccaccgcgctgcagaagctcagcgcggtcaaccgcgacaccgtcaccgtgggcgacgtggcggtgctggccatcaccaagtccgcgagctatccgggcttcgtggttccgggcaccacgcgcatcgacttcaccgtgtcgggcaccaacatcggcgcgcgcgacgcacgccctggcaacaccgccgcacccgccggaacgccggtgctggtgaacggcacgcccacccccctgctgctgttgcgcgacctcgtgcccgcgggcacgcgctacatcgccggcagcctgcaaagcacggcagccggcgcggtgcgcctgttccgcctgccgggcgatccggacttcagctaccgcaccgccgaagacgcctcggccgtcgaagtggccatcggcgtgccgaccgcgctgtcgcgcaacgcatcgatcgccatgcagttcgcggtgcaggtcaaggccgaccagagcggcgacatccgcaacaccgcgcagggctactacaacgacggcgcagcgcccgcggtgtcgccgtcgaacacggtggtcatcacccccagccagagccgcatcggggtggccaaggcggcctcgacgccgcgcctgaaccgcggcaccgacggccagctcgacggcaccgccaccgtgagcttcagcgtcaacgtgcgcaactacggcgccgtgtggctctacggcgtgcaggcgaccgacctgctcgaaggcagcggcgccacgcagttcggcacctacacgtcggccgcggtgcccgccgccaaccagtacaccatcgtgcccggcacgctggccatcgcgggcaaccagggcaatggcgtgggtggtaccgtggccgcggccgacagcgcgttcaacggcaccgccgccgcgcagaacctgctggcgcccggtgccgttctgccggtgggcgggcagttcaccgtgcgcttcgatgtgcgcttcaacgtcggcggccgcgccggcacgctctacaacaccgtgcgcgcccagggcgcgctcaccgccggcggctcgccggcggccttcgacgactcggtcaacggcagcaaccccgacgccgacggagacggcaatccgaacaacgacagctcgccgacgccggtgtccacgcaactgcccgcgctcacgctggccaagaccgcctcggcgccgcggcgcgtgtcgcagggcgtgtacgagctcgactaccgcctcaaggtgagcaacaccggcgtggcctcggcgccgaacgtgcgcatcatcgacaacctcaattgcaccttcgacatggacaagcccgacggcctcgttgccgcctgggaactggccgctccgccgaaggcgcgcaacggcatcctccatgccgcgggtggcttcaccggccgtgccccctgcgaccgcgaagcgctcgcaagcagcgatcccttcaggctgccgaccgaagccgtgctgagcgtcaccgacggcagccgcccgctcgcgccaggccagagcgaagaactctccttcaccgtgcgcgtcacgcagaagcctggaatcgtcggcggccgaatggcgcttaccaacaaggcctgggcggcggccttcgaccagaacaccgtcaacgtcacgccggccatgctggtggccgccagcgccagctcggcgcagtcgctgctggccgacccgcagggcaccgtctacaacgccgtcacgcgccagcccgtggccggtgcggtcgtcaccttcacgcgccagtcgtgcagcagcgggccggtcacgccgatcaccgcggaagagctgtatggcggctcgtcgggcatctacacggtcaacgccaacggcagcgtctccatgaccaccggcgccgacggcggctaccagttcttcctgcagtcgccgccggtcaccggctcgtgcacctacgccctcggcgtggtgccgcctgcagccagcggctatgtgacgccgtcgcagctcattccggtcacggccggcaccttcaacagctgcggcgccatcgtgccgaatgccggcccgccgcagggcgcagacccgaccacctactacttctcggtcaacgcgggcttcaacgcatccggcgccgcctgcgacgtggtgcacaaccacatcccgctcgacccgggcaatgtgctcgggctggtgctgcgcaaggaaggcagcaagcgccaggtcgagttcggcgacttcatggactacgccctggtcgtcaccaacaagacgggcttcccggtcaccggcgtgcgcctggccgacagcctgccgccgggctttgcctacgttgcgaacagcgcgcgcctgaacggttcggccgcggtcaacccggccggcggcgcgggcccgcagctggtcttcgactacccggcgctggcgctgggcgtggaccaatcggccacggtgcgctatcgcgtccgcatcggcgtgggcgcgcccaccaatggcgacgccgtcaaccgcgcccgtgcgagttcgggtccgatgcagtcgaacctggccaactggaccgtgcgcgtgaccggcggcgtgttttccgacgacgccttcctgttcggcaaggtccacatggattgcaagcgcgacggccggcaagagggtgacgacgagatcggcgtgcccggcgtgcgcctctacatggaagacggcacccacgtcatcaccgacgtggaaggcaagtggagcctctacggcctgaagccgatcacccacgtgctgcgcgtcgaccagaccacgctgcccgccggcgcgcggctcgaggcgctcgacaaccgcaatgccggccgtcccgagagccgcttcgtcgacctgaagaagggcgagttccacaaagccaacttcatcgtcgccaactgcgacacgcccggggtgatggacgaggtggcggcacgccgtgccgccatcgccgccattcccgacaccgaagccgaggcgcaggtgcgcatgcggctcgaccccgaaggcaagatcgtgccggtgggcgacgcgcgctcgctgcccgccagcggccaggcgctcgcgacgggcagcacaggcagcgccggctcgacgctctccaactcggccccgctgatcgcgatgcccgtggcgcccgccaacgcgagcagcttcgtcaacggcgcatcgagcaccttgagtggcacgctcggcgccagtgcggcaccggcgcccacgcccgcaggcagcctgttcgcggcgctgagcggcctgcccaccaacgcgcagggcgcatcggccacgggcggcggcgccaccggcgtgggcgcattcgcgagccgtccggtcaacacgaacaccgccatgctcgagccgcgccagaacgcggtggcaccgctgctgccgcaggccgtgcccagcccggtcgaactcgaagccctgttgccgcagatcgaagacaacgcgctcggcttcatcgacctgaaggacggcgacacgctgccgggccagtcggtcaacgtgcgcgtcaagggccaggccggcctggcgctgcgcctcacggtcaacggcaaggccatcgaggagcgccgcgtcggcaagaagaccgagctggccggcaagaagctcggcgcctgggaatacatcggcgtggtgctgcagcccggcgccaaccgcctgctgctcgagggcgtggacccgttcggcaacgcgcgcggcacggcgcagcagatcggcgtgatcgcgcccgacaagctcggcgccatccggatcgacgtgcccgaatcggcgaaggccgacctgcgcacgccggtgatcgtgaaggtgcgcctgaccgacgcggccggcgtgccggtgaccgcacgcacccagctcacgctcgaagccgaccgcggccgctggctggacgaagacctgaatcccgccgaacccggcacccaggtgttcatggaaggcggcgcggccgagttccgcctgctgccgcccggggagcccggcgatgcacgtctgcgcgtgacggcaggcagcttcgtgaaggaagtgcgcctcgcgctcttgcccgagatgcggccgatgatcggagtcggcatcgtcgaaggtgtgctcgatctcaccaggcgcggcggcgtgcccctgggcgcgatgcctgcgggcgccgccttcgaggcggaactcaccggcctggccgacgagagcaacagcaaccgccgcgccgccgctcgcaccgccttcttcttcaagggcaccgtcaagggcgagtacctgctcacggccgcctacgactcgaacaagacgcgcgacgaccgcctgttccgcgacatccgccccgacgagttttacccggtgtacggcgattcctcggtcaagggcttcgacgcgcagagcacgcagaagctgtacgtgcgcatcgacaagaaccgctcctacctgctgtacggcgacttcacgaccgccagcagcaccgaggtgcgcaacctgagccagagcaaccgtgcgctcaccggcctcaagcatgtgtacgacgacggcaccgtgcgtgccaccagcttcttctcgcgcaccgcgcagacgcagcaggtggaagagttccgcgcggtcggcacctcgggcccgtactacctgagcgccacgagcggtgagttcgtcgacaacagcgagcaggtcgaggttgtggtgcgcgaccgcaaccagcccaacctggtgctgcagcgcacgacggtggcacgcttcgtggactacaccatcgagccgctcacgcgccgcatcctgttcacgcatgcgatctcgtcggtcgatgcgaacctcaatccgcagtcgatccgcgtgacctacgaaatcgatgccggtgggccgaagttcaacgtggccggtaccgacgtgcaggtgaaggtcggcgacaacctgcagctgggcgtggtcgccagcaccgacgagaaccccgagaaccgccgcaagctcggcgcgctcaccgcggtggcgcgcctgggcgacaacaccaccatggccggcgagtgggtgcgcaccgagtccgacaagaacggcaagggcaacggcggccgcgccgagctgcgccaccagaccgaagacctcgccgtggtcgcgcttgccagcaagaccagccccggcttcgacaaccccggcgcgagcttctccgccggccgcaccgaagcttccgcgcgcgccgagtaccgcatcgacgccaccaccgcggtgcgcggcgaagcgctcttcagccaggacgctctgcagggtggcagccggcgcggcttcaccgccagcgtgcagaagaaattcggcgagcagatggccgccgaagtgggcctgcgccatggccagagcggcgcgggcctgggcaccagctcgggcttcgactacggccagatctcgacctacagcgggaacctcggcagcggcgtcggtgccagcaacgtcaccgcgctgggcagcgcggcaagcgcgaacgccagtgcgaatgccgaagacctgacgaccgtgcgtgcgcgcctgtcggcgcaggtgccgggactgccacaggccaacgtgttcgtcgagggcgagcaggacatccgcaagtccgaccgccatgtgctggccgtcggtggcaactatgccgtgaccgacaagacccgcatctacggccgctacgagctggtctccagcctttacagccaggaccagctcggcacgaccggttcgaacaacgtcggcatcctgggcgtcgagagcagctacatggaaggcgggcgcgtgtacagcgagtaccgcctggccgacagcatcgacggccgcgccgcgcaggcggccaccggcgtgcgcaacaccttcaagctcaacgaccagtggcgcctgaccggcggcatcgagcacacgcgccagctcggcggcctgcgcaacagcggcaacaccggcacgggctattcgggcgggctcggccagtcgacggccatcaccggcggcgtcgaatacatcgccgagcgcatcaaggcgagcggcgtgctcgaaggccgccgcggcgacgatgcgaacacgcggctcttcagcgccggcttcggctacaagatcgaccgctcgtggagcctgctcgcgcgcagcgtgatgagcgacagcgaagggcagggcaccaacgccggcaacgcgcaccacctcgcgcgccaccaggtcggcctggcgtaccgccccgtcgataccgaccgctggaacgcgctgatgcgctacgagcgccgttcggagcgcgtggtgggcgcgggcagcacgaccggtgcgctcgacggttcgagcgtcttcggcgcgggctccggcaacgccagcctgcccggcacgacgggcgccgacatcgtctcggcccacttcaactacaacccgcggcccggcaccgtgatcaacggacgctatgcggccaagtggtcgcgcgccgacgacggctggctcaagagcacctaccgggcccacctgctgcaggcgcgctacacgcaggacatcaacagggactgggacttcggcatccaggccggcctgctccacggcaagggcggcgcgctgcagaagacgctgggcgccgaggtgggctaccaggtcatgaaggacctgtgggtgtcggccggttataacttcgtcggactcaaggaccgcgacctcacggccaacgagtacaccagcaagggcgcctacatccgcctgcgcttcaagttcgacgagacggggctgggcttcgcctctgccggcgctgcggcctcggcgaacgccaaatgacaagaattgattcggccgcagtggcagaacagatgactcgatttccatcttcgatcgcccggcgcatgcgcgttctgctggtgctgctggcgtcgttcgtgtcggcgccgacgctggccgcacaaaccgcctgcacgccgcagtcgggcttcaactcgtgcgtgcgggtgacttactccggcggcgaccagaccttcaccgtgccggccggcgtgacctcggtattcatcaaggcctggggcgccggcggcggcggacccaataccagctactaccccacgcagcgcggcggcggcggcggcgggttttcctccggcacgctggcggtgacggcgggcacggcgctgggcgttcgggtcggcgagggcggcggtgtcaacgacgcctccacgacctacggcggcggcggtgcgggcggcaacgcgcaggccacggccatcggcgcaagcggcggcggcctgtcgggtgtgttcgccaccacgacttacacccagggcaacgcgcggctcattgccggcggcggcggcggttcgtcgccgggcgcggacgtgggcacgccctccgccggcggcggcggcggtgcgagtggacgcgacgacaacgtggctgccagcgggcggcccggcacccaggcagcgggcggcgcggcgggaacgggcggcacctgcaacctcggcgcgccgacgggcggcaccgcgctgcagggcggcaatggcggctccaccaacgagaaccagaacgaaggcggcggcggtggtgggggcgggttcttcggcggcggcggcggcctgtgccaggggacttcacccaacggcatgggcggcggcggatccggctacaccggtggcgtcaccagtccgaccacggccgtgggattgaattcgacgtccgacaatgtcggcggcgcagcggccaccactggcgacgctcactatgcggccggcatcggcactggcggaggcggcgatgccagcggcggcaacggtctggtggtgatccagttcaacgcgccgccgtcgatcacgctgagcaagaccgcgccggccacggtggcgccgggcgcggccatcgcctacgtgctgagcctgaccaacagcggccccgccgccaccggcacttcggtggtcgtgcgcgagcagcttccgccgggcgtgatcgccactggggccacggccggcaccggcgtcacctccgtgagctgcggcacgatgccgagcgcagccggcgcgttgctgacctgcacgatgacgctgcctaccgccggcattcccgccagcggcggggttcgcagcttcacgctcaatgccacggcgccactggtggcggcgggcacggtgctcaccaactatgcgaacagcaacgtggccggcagcggaacgccggccacggcgcccggcgcggcctgcgtgtccaacaccaccgtgagctgcgccagcgccgccaccaccgtggtcgccggcgcagccgccctggcgcgttcgggcgaacgcaccgccaccgacaaccaggtggccaacggcagcgcgcaggacgtgctcgaagccatcgtgcgcgacgcggccgacaacccggtggcgggcacggtggtgaccttcgtcgccaccaccggcgtggccttcaacggcggcgcggtcggcgcggccggcacttgcactaccgccgccaacggcatctgccaggtcaacgcgaccagcaccgtgccaggtgcaaagagcaccgcggtcagcattccggccggcacgctgaccggcgtcttcaccgcgaacggccagagctacggcgcgagcccggcgacctacagcttcgtggtcggcacgccgagcgccgcgcagtcgggtctgcgcatcgccaccgacggccaactggccaacggcagcgcacaagacgtgctggaggccttcgtgcgcgatgcgaacggcaacccggtcggcgccggcgtggtcgtgagcttcggcgccacgcccaacgtggccttcaacggcggcaccgtgggcgcggcggccagctgcaccaccaccgcctcaagcctctgccaggtgacggcaacgagcaccgtggccgcgacctacagcaccaccgcggtcacgctgggcggcgtggcactgggcggaaccttcacggccagcggcaacagctacctgccgagcccgcaggcctacaggttcctgtcgctgccgacggtgaccatccgcacgatttcggtcaacggcgtcggcactttcgatttcaccggcaacaacggcctggccgcgcagagcatcaccaccaccgtggccggcaccgccgccagcgcggcgccgcagacgctcacggccgcgggcaccgccaccaccatcaccgagagtgcgccgccggcaggctacacgctgacgggcgcctcctgcaccggcctgccttccggcggcaccgccacgctctcgggccgcacgctcacgctcaatgccgcggccaccgcgccgggcgccaacctggtctgcaccttcaccaacaccggcgccaccgacgccacctcgccgccgattccaccgacgttgagttgcctctcgaacgccgcgatcttcaacaccgcctacaacggcgtcaacggcccgccgctcaccagcggccgcgacacggtgtgggagtcgggcgtgggcgctgccagcggcggcccgggcaccgtcgcctcgtggcagcgtgcctacgtgggcaacaaggctcccaccgcctgggtcaattcgccctttggcaacgccaactggaattccaactacgacccgaaccacacgggcaacgtcgacgtctaccaccgcttcactttcaacatggcggcgtcggtgaacccggcgagcttctcgctgaagctggacttctattccgacaactcggtggccgaggtgttcgtcaacggcgtgctgcagagcgtgcccggcgtgccgcaaggcggcagcgatccctacaattttcgcgggtacctggcgggcagccaggcaagcgcgacgctgtccagcaactggcgcaccggcagcaacaccgtggtggtgcacatcaagagcggcgcgaacgccgaaggcttcctggcgcaggccaccaccaccgcggtttgcgctccacccaccttgaccctgtcgaagaccaccaccggcggcgctggcggccccttcaacttcacgctgagcaacaccacccagaccaacggcgtggtcagcaccgtggcggcgggcacggcggtgcaggtcgacggcaacacggcgacggccggtacgcagcccttctcggccacggcccagggcgccgcgatcaccattgccgagccggcggtgccgggctggaacctggcgggcgcggtctgtaccgatgccggcacgccggtcggcagcctgggcaccggcaccaatgcgcgcacctacacgattcccgcagccagcgtgcagtacggcaggccgctttcgtgcaccttcaccaatgcggcctcggccacggtgacggtcagcaaggtgagcaacggcggcgtgggccccttcggcttcaccggcaacaacggcctcgcggcgcagacgatcaccaccaccgcggccggcgccgcggtcgcgggcgcgatccagacgctgaccgcacccggcgtcgccaccaccatcaccgaagatccgctgcccgccaactacgcgctcaccggcgtgagttgcaccgggctgggcgcgggcggcaccgccacgcccgacctgcccaaccgcagggtgacgctcgatgcggccgccaccgcggcgggcagcaacatcgcctgcaccttcaccaataccttcacgccgccgttcccccgggtgcaaatcgtgaagaccaccaccggcggcagcggcgccaacctgttcggctttgcgctcagcgggctctcggccgccaccgacagcatcaccgtcaccggtgccggcagcgcgagcggtgccgccaacctgaccggcacggccggcgcgctcgcgacgatcagggaaagcgtgcccgccggctggcccgccaacccgatcagcgcgagctgcctggatgcagccagtgccacgcccaccgtgcccttcggcacgctggccggcaatgagctcaccattcccgcggccaacatggtggccggtgccaacatcacctgcaccttcgtcaacggctttggctacaccgtgacgggccgcgtgttcctggacaacggcacgggctcgggcgtcgcgaacgacgggttgatcaacggcagcgagggcggcattgccggcgtgggcgtgcagctcaccaactgcagcgccacggtgctgtcgaccgccaccaccgacggcgccggcaactacgcgctcgacgtgccctttgccaccgccgcgaacgcgccgctgtgcgtggaagaaaccaacaccgcgttgcgcctctcgaccggcgcttcgttcggtgccgtcccgctgccttcgggctcggcggtggcgagcggcggcaccagctacacctacacgcgcaccggcacgcccgaccgcattgccttcacctggaacggcgcaggccacaccggcctcaacttcggcgacgtggaccgcaacaccttcgcagccgacggcgccaagagcggcatgccgggcagcaccgtcagctatgcgcacaccttcattgcgcggaccggcggcacggtgagcttcagcatctcgaactcggtcgacacgccggccgtcagcggctggagcggcaagatctttgccgacaccggctgcaccggcgcgcagcaggccggcgctgcgctgctgtatccgcccgcggcgccggtcacggtggctgccgggcagaacgtgtgcatcgtgatgcaggagttcattcccgccaatgcggccaacggcaacaacaaccagagcacggtgcaggccagcttcagcttcaccaacgccggcccggccctgagcgcgagctacacggtgctcgacaccacgacggtgtcgaacagcgcgctcgaactcaagaaggaagtgcgcaacgtcacgcagggcggcagcttcggtgtgaacaaccaggccaagtcgggcgagacgctggagtaccgtgtcacctacaccaacaacggaacgacgccgatctccgacatgaagatcaacgacacgacgccgcagtacaccagtttcggcgctgcgcaagccggcaccacgcccgcttcgctcaccggctgccgcaagaacacgcctgccaacgccattcccgctccctcggtggcctgcgcggtggcgcagaccgccggcggtaccggcacgctgagctgggagttttccggctcgctcgcgccgggcgggtcggggtcggtgctcttcagcgtgaaggtggactgagcggtcgcgatcacttgctatcggcgcgcgcctttcgcgaccacgcccgcgccgcgcacttcgagcttgcgctggtccaccaccttgcccgtggcatcgaccagttcgatcacatggcgccccggccagggcagccattgcgcgctgttgccgcgcgcaaagtgcttgccgtcgatgcgccattgcacgccgcgcccctcggactcgaaacgcacgcgctggtgcaggggcggaatgtccgggtcgagcgcgatgatggtgccgtcggccggcgcggtgatgcgcgcggctgccgcgtcggacgatgtgccggcgccgccgttgtcgagcgcgaagagcggttgctccgtgccctgcaggaaccattcgccgcgcgccgcctcgatcgggttgccgtcggcaccgggtccgaatgtcacgtgcgcttcgacgaggccggcgggcggcctgggtgcgcggctgggttcacgcgcgtgcaggaagcgcatcacctcggcccagaccggcgccgcgccgctggtgccgctcacgtcccacatcgaggccccgctcgcgttgccgacccacacgccgaccgtgtagcgctgcgaccagcccacggcccagttgtcgcgcatgtccttgctggtgccggttttcaccgcggtccagaagcgcgtggaaagaatgctgtccaggccgaaggtgcgcgtgcgcgcattcgcgtcggacaggatgtcgccgacgatgaaggcggcgcgcggatcgaggacgagcgcggccgagtcgtcgccagccctcgctttcgcggttgaagccggtgtcgcaggccgcgcagtcagcatcgtcggtccgtagcgcccgccattggccagcatgcgataggcgttggtgagcgacagcagcgacacctcggcgctgccgagcgcgaggctgtagccgtagtagtcgccgctttcgcgcagcggcaggcccaccgcgcgcagctgccgcgcaaacgactcgggcgacaccatcaccagcgtgcgcaccgccggcacgttgagcgaggcggcgagcgcggtgcgcgccgacacgggccccttgaactggcggtcgtagttctgcggaatgtagaggccgctcgcggtgctgatctgcgccgacgaatcgtcgatcagcgatgccgcggtgagccgccgctcggcgatggcctgcgcatagagcagcggcttgagcgtggagccgggctgtcgcagcgcggtggctgcatcgacctcggccgcctggctcagcgggcccgacgagccgacccaggcgagcacctcgccgctcgcgttgtcgagcaccaccagcgcgccgtcttccacgtgccggccgcgcagttccttcaggtggcgttgcagcgcgccgagcgcaaagcgctgcaatggtgcgcgcagcgtggtcctgacggccgtctccttgtttgccgcttgccgcgcgggtgtcgtggaagaagcggcggcggccgcttcaccggcgtcgcgcaactcgcgcagcgcacgccgcgccgcatgcggcgcaatgccttcgttcgcatcgaaggcgcgccgctgcaccgccgcgctggtgaacatgtcgatcgcatcgcaatcgatcttttgccccggctccatggcgcgcatgagctcgcaagcgcgctgcgccaccagcgctggcttggcgttgggcgcgcgcaccagcgcggcggccacgctggcctcgcgcgcgtcgaggccgttcggcgccttgccgaacagcgtgcgtgagagcgcgtcgatgcccacgatctcgccgcggaacggcacggtgttgaggtaggcctccaggatctggtccttgcgccagctgcgttccagctgcgtggccgccacggtctggccgatcttctgcgtgaaggtgcgtccgctgttggcgcggcgcaggtcttcgtcgagcaggccggagagctgcatcgtgatggtcgatgcgccgcgggtgcgcgtgttccacaggttgccccaggcggcggccgacacggcgcgccagtcgatgccgctgtgctcgtagaagcgccggtcttcgctcagcaccatggccatgcgcagcgcgggcgaaacgtcggccagcgcaatccactggccgcggcgcacggtggcgtcggtgcgcacgcgctgcagcagctcgccgttgcgatcgagcaccgcggtgtcggaagaacggaactcgcgcttcacctcgtcgaagctcacgatgccggccaatgccagccccggctgcgcgcagaggatggtcgtcagcgttgcggtaaggcaacggcggcttgcggcgagaggcgagcggtgcatgaaaagcggtgtgaaggcaggggcggaaatcggcgccccggagcgccattctcggccatgcggccacgggaactgcacctacttgcagacgggcgcgccgccgtctgcgcgcgtaagaacttagcgccaaagtttgcagcacgttccacatccggtaacgaacttcacgccccggcctcattgcagatacggagccgagacggaggtggccttcaatgcagttgccggcttgcggaggcaagccgtctttttagaactccaaggagaaatcaaatgatggtgaagacattggccgttctgcttgccgcatcggccgctctggccggctgcgtcgttgcaccctatgaccggccggcgccgcgtccgcactatggctacggagaccgcgaccgcgacggtgtgcccaaccgctacgaccgcgaccgcgatggcgacggcgtgccgaaccgctacgaccgcaatccgaggaacccgtactaccgctgacgctggcgggagcgcacctcaggcgggccggcgcgcgagcagcgcccacacgcctgccgcgctcagcagcgagccgcccgcaaggttgaagcgccgctgcgcgcgcggcgaggaaagcagcctgcgggccgatcccgcgaacaccgcgtagagcgtggcattgagcgcggccatggccacgaaggtgaccgccagcacccacagctggcgcgtcacgtcggccgtgggactcagaaactgcggcagaaacgctacgaagaacacgatgcccttggggttcagcgccgtcaccaggtaggtgttggcgaacagcctccagcgcgaagcgggcgccgccggcgcagccatgtccgccgatgtgatgcccgcccgcagcagcttgatgccgagatagatcaggtacaggccgcccgcccacttcaccaccgtgaaccagaacgccgaggtggcgagcagcgcccccaggcccagcagtgaaaccaccagcgcggtcgagtcgccgagcgccaccgcggccaccagcggcacgttggcgcggcgtccgtgcgacatggaatagctgatcaccgtgaggatggtcgggccgggaatgatcaagagcacggcggatgcggcaacgaaggcgagccagagttcaacgggcatgaagagtctccaaggttgttgtgatgttcaggcgccgaagcgcgcggccgacctggcccgcgcgcgttcggcctcgatggcgcggtcgcgcggttcggccgtggttaccagcgaatcgatgagccgcgttgcgctggcggccatttcatcgaccgcgcgctcgaaggcttcctggttcgccttcgatggcacgctgaagccgctgagcttgcgcacgaactgcagcgcggcggcgcggatctcctgctcggtggcgggaggctcgaagttgtagagggtcttgatgcttctgcacatgggaactccatacggcaggggatgcgccagtttagagcctgttgacaggccctagcgaagcagcgccatagcgtgggcatcgtgataaatgccgtcgatcaggctggcgcggcggatgaggccttcgtgttcgaaaccgaatcgctcgtacagcgccttcgccttcaggttgtccgcgcgaacggaaagctcgatgcgggtcagcccgcgcgaccacgacctgtcgatggccgcctgcagcagcgctgcgccgagtccccggccccgtgtctcgggcagcatggcgatgcccagcacaccgatgtgggcccgcgagtggccgaagaccggcgaaacgtcgcaccagcccacgaccttgccgttgccatcgatcgccacgaaatgagggaagcccgctgccagcacgttgcggtagaaggcgagcgattgctcccacggcggcgcctgggtcagcgcaagatacctctgctcgcgcgccacgacatcgagcgccttgtgcaggctctcgaagtgttgctccgcggtgggaacgacggaatggttcatgcgcgcgagacgaagcgcgtgttcattcgacgagcccgcgctcgacggcctgcgccgggttctcgaagatcgccatcgcggtcttcatgcgcctgaagccgaacttttcgtagaagggctccttgccggccaccgcatacagaatgatcttgcggtgcccgctggaggccgccacgagccgcgagacgatctccttgccaaggccggtgccctggtggctcggatgcacggccacgtcgcagatgtaggagcagtcgagcccgtcggccatggcgcggccgacgccgaccagtcggctgtcgtcatacgcaaagcacttgaacatgctgttggaaaacacgagcttcaggccgtccgcttgtttgttgccgagtggcgcggcctggtagagccgcgagagttcttcccaatcgatgtcttcgagcgaatggcgccattcgagtgtcatggagcgtgcctcttgttgggccggtcagccggcggggttcaaccgcaggatggcgtccgccacggcctcgatgccggggtccgtgaggtcggctgccgccacctgctgccgcagcggccacttctcgaaatggcgcgcctgcgagcgttcgtagtgcggatcgtaatgaagcgccatcagttccgcaaaaagcggcggcagatcgccctggagcgcccactcctgccagcgctgcaccaccgccttgccctgcatttccttcagcctgtcgagctgcgccgccagcgcggcgcggtcgtcgccgaggtaggcgtagtcgcgcagcaggtagtcgagccgcgtggccgcatcggcctggatttcgatgcacgctgccgcgcgcatgtgcgcaaccagcggaatcggcaccgagagccggccgatgcgcgcactttcgccttccacatagagcgtgcgcgagaggtcgagcgcatcgaagcaggtggcgatgcgcgtctcgaactgcttttgcgaaggctgcggcacgccgggcagggcgcccaagagcgagcccttgtggctggcgcaatgctccaggtcgagcacctgttcgccgcgcgcggcaagcgcctgcagcacccgcgtcttggcgctgccggtggcgccgcagatcacccgcagctgcagcttgggtacggtggcttcgatctgcgccagcacgtgatggcgaaagctcttgtagccaccggcgagctgctgcgcgtcccagccgacgagacgcagccaggtcaccatcgagccgctgcgcaagcccccgcgccagcaatacacgagcggccgccagttggcgggctgttcggcaaagcgctcgcgcaggtgccgcgcgaggttggcggccaccatggcgccgccgacacgccgcgcctcgaaggcgccggtctgcttgtagatggtgccgacgatgcggcgctcttcgtcgtcgagcaccgggcagttgatggcgccgggaatgtggtcgagcgcgaactcggagggcgagcgcgcgtcgatgacggtgtcgaaccggtgcatgtcggccacgcgcgtgggctggtggcgcgggttgctgtcgtgctcacgcatgggcgtgccccaggttgcgccgcagccggccgctcgccaggtcgacgagggccaccagcccgaacattgcaatcagtacggtcatggcctgctgctgttgaaagatcgacaaatgaaagtagagaagctgccccaggccgccgccgccgacgaagcccagcaccgcggccatccggatgttcatttcccaacgatacagcgcataggccacccattgcggcagcacgagcggcaggctgccgtagccgaaggccgccaccgcgccggcaccgcccagcgccagggcctgttcgggttcgcgcggcgcgttctccaggctttcggcgaacaggcggccgagcacgccggtggtgtgcagcgcgagcgccagcgcgcccgcgaacgggccgatgcccgcggccagcaccatgagtgcggcccacaccagctccggcacgctgcgcaagaagttgaggacaaaacggcagccctgccgcaccagcaggcccgatcgccccgaggccgggagcgcgagcacggcggcgcccgcggccgccagcagcgtgccgagcgccgacacggccagtgtctgcagcgcgccccatgcggtcttggcaagaaaggcgctcgaaagatccggtggaaagaactcggcgatgaacttgcccatgaaaccgatcgattcggccgtgaagagggcgctgtagtcgatggccaggtacgcgaagctggccaccacagccaccagcaccagcgccgatgcggcccagcagcgaatgcatcggggcggacgggcgaattgcgcggcgttgtccttcatgccagcaaccgccgcaacgcattgctcagcgcatcggcgagcagcaccagcaccaggaacaccagcaggatgctgctggcttcgccgccgttgagcatcttcatcgactggtccatgagctggcccaggccgcccgcgcccacgaagcccatcacgaccgaggccctgacggcgcattcccaccggtacaccgtgtacgagacgagttcctgcccgcagtggggcaacaggccgtaaaccagcgcggcgatgcggccgctgccgctttccattaatgcgcgggcgggccgcgtgtcggtggattcgagcacctcggcatacaccttgccgagcatgccgccgtaggtgatggcgagcgccagcaccccggccgcggggccgaggcccagcgcgcgcacgaagaccagcgcccagacgatttccggaatggcgcgcagcaccatcagcacggaacgcccggcctgccgcaccacggcggcctgcgcgcgccccgggccgggcccgatgcgcgagaccgagagcgcgcgcgtggtcacgaaggccaacggcgcaccgatggcgaaagccagcgccgtgcccgccgtggccatggccagtgtctccagcgtggccttggccagcatcgcgaggaagtccggcgcggtctccggcggcatgaagccggccaggaatccgccgatcacctgcaggttgcccggcgcgaacagggcagagggcgcgaagcccgacagctgcagcatcggccaggcgatgacgagtgcggccaggagccacactacgcggcgccgcgccatcggatcgcgcagggcgggcggcgtgcgtggcggcagcgattgcgcagtggtcacaggcaatccggccgttcgacggaattcgcggaagccgcggtgaattttcgggatggcatgtccagcggcagtccaggtgcctgcatcggcaacccgccctcactggcatagagcgccgcgagcatcggttccgtcacgttgccgacgggctcgtcgaacaccacctgtccgctgcgcatgcccacgatgcgcggaaaccagcgcagcgccaggtccaccgcatgcaaggaggccacgagcgtggcgcccgtcgattcgctctgcgccaccagctgctgcagcgcggcgtcggccagcgtcggatcgagcgcggacacgggctcgtcggccagcagcagcgcgggccgctggtagagcacgcgcgcaatgcccacgcgctgcaactggccgccggagaggcgatcgcagcggtcgaacaaccggtcttccagcgcgagccgcgacagcacttcgtgcgcgccttcgaggtccgacggacgcagcagcgagccgagcgcgcgcatcgcgctccattgcccgagccgccccgagagcacggcggtgaccacgcgcaggcgcggtgcgattggcgggctctggtgcacggtgccgatgcgtgaccgcagcttgcgcagcgccggcgcggccaggccccacggcgcttcgccgagcagctgcaccgtgccttcgcccggccgcagcgctgcgccgagcacgcgcagcagcgtggtcttgccggcgcccgaggggccgatgacggccagccgctcgccgtcgcgcgcggcaagcgacacgccctgcagcgcacgatggccgttcgggtgcaccagcccggcgtcgtcgagcgaaaagctcacgcgacggctccggcggtgcgccccgatggcatcacttgaccagaccggccgacttggcggcggcttcgatgccgtcgtagttcgacgacttggtggcaatgaacttgctcgcgcgctgcaggctcatgatctccttcatggccgggtccgcgggatcgagcttcaggaatgcctcggtgagcttcttggtcagtgccgggtcgaggccggggcgcaccgtccagttgtagtcgtagtaggttggggtggtggccaacacgcgcaccttggcggcgttcgggttcttgctttcgaccagcttctcccacaccgatgcgttcagcacgccggcctcggcccgcgaggcggccacgaaggccacggtggcgtcatgcgcgcccgagaaagcgaccgtcttgaagtccttctcgggatcgatgcccgcctgcatcaggaaatagcgcggcatcaggctgcccgaggtggacgaaggcgcgccgaacgcgaaggtcttgcccttcaggtcggccagcgtcttggcggtgctatcgaccggcacgatgaacttgctcgtgaacacctcgtcttcggcgcgctgcacgatcggcaccgcgccgccgttggtgcggatgcgagcctgcacgaaggtgaagccgccgagccaggccaggtcgatcttgttcgtcgccaggccttcgaccacggcggcgtagtcggtcacgggcgtgaactgcacgtccatgccggtttccttcttcaggtagtcgccgagcggcgtgaacttgcgctgcagttcggtgggcgcctcgtcgggaatggcggacacgcgcagcaccttgccctgcgccgaagcacccagggcgaggacggagagcgaaagtgcaagggcgatgcgaaggaggggtttcatggggtggcgcggcatggcgcaatggaggacggacaaccttcgattgtagaaacccgcgcgcgggtgccgtttgcggcccccttcgataatggacgaccgccccgatccgaattgcgccatgaccgacaccccgacgatttctccgctcaaccccctggcgccgctgcggctcaccagcttctcgcatggcggcggatgcggctgcaagatcgcgcccggcgtgctgtcggaaatactgaagaacagcggcggcggcctgattccgccggagctgatggtgggcatcgaaaccgccgacgacgcggccgtgtaccgcctgaacgacaagcaggcgctgatagcgacaaccgacttcttcatgccgatcgtcgacgacccctacgagttcggccgcattgccgccaccaacgccatcagcgacgtctacgcaatgggcggcaagccgatcatggcgctggcgctggttgccatgcccatcaaccagctgccggtggaggtcatcggcgacatcgtgcgcggcgggcaggacgtgtgccgcgcggccggcattccgattgcgggcggccacaccatcgattcggtcgagccgatctacggcctcgtggtgatgggcctggtcgatccggcccacgtcaagcgcaacgccgaggcgcgcgcaggcgacgtgctggtgctgggcaagccgctgggcgtgggcgtgctctcggccgcgctcaagaaagagaagctgtcgcttgccggctatcggcagctcatcgagaacaccacgcggctcaacacgccgggcattgcgctggccaccatgcccggcgtgcacgcgctgaccgatgtcacgggcttcgggctggccggccatgcgctggaactggcgcgcggcgcagggctcaccgccaccatcgactggccgcgcgtgccgctgctcgatggcgtggccgcgatggtggcggacggcttcgtcaccggtgcctcgggacgcaactgggccgggtatggcaaggacatcgagctggcagacggcctgcccgccaccgcgcaggcgctgctgagcgacccgcagacctcgggcgggctgctcgtgagctgcgcggccgaatcggccgatgcggtactgcaggtgtttcgggccgaaggctttgcgcaggccgccgtcatcggccggatggagcaaggccccgcgcggctgcgcgtctcggcgtgaaaaccgcgaaggccacgcggaccggcgcgaggcgcgacttggggccagaatgcggctcagggagacacggtcgtcttcggcagcccacaacggaggtcgcatgatgcgcacatcggttctcttcattccggcgctcgccgctgcagcggtcgtcgccgccatcggcgcgcaggctgccgacgtggttcgctgcaccgatgccagcggaaacaccgtctataccgacggcccttgccccccaggcagccggctctcgcgccaggtacccctcaccgagccggtgagggtggttccgtctgattctcccggcgaagcgcgccggccgtcgtccacgcccccgccgcgcgcggcgctgccgcagccgccgccgcagcagcagcagcagcaggccggcaatgcgccgcaggggccggccatcattccgcgcaacgtcgatgagccgcgccaggtgcccgagccggcaccaccggtctacagctgggggccggagccctactacgacggtggccgccccatcgttcgtccacggcacccccgcccgcaggaagacccgggcccgccgccgggccagcggccctgccagaacctcgcgggtatcaagcgcaacaactgctgagccgccggagccgatgcaacttcgccactggaccgtgtattgcgacggcagcgcgatgccgaaccccggccgcatgggagccggtgcggtcatcaccgagcccgatggcacccgccacaccttgtcgctcgcgagccatgccattggctgcaacaacgaagccgagctccgggcgctgaccctcgccctcgaagaactgaaggcaaggggcgcgacctcggtgctggcctataccgacaacagcatcctcgtcgagcagctcggcgcgcccggtgcgaggccgatcgcacgcatggccggcctgttcgaggatgcccgcgccttgctgggttcgttcgaggaggcgcacctccgatgggtgccgcggcaccgcaaccacgaggccgacgcgctcgcgcgtgcctcgctgggctttgcgcccaaacctgccgccaagaccacgaagaagcggcgctaggacaggccgctggccgcggcccgcgagagaagccatatcatccgcgtcttcaccgccggccccgcagcgaacgagtccggggcggtatcgctttcaggaaaccgtttttagccatgaccgaagccaatccccttccgcctctgcccgatcacctgtccacggacccgcgcagcccccatcacgtggccgccgtcttcgagcacgacatcggcatccgcttcaatgacaaggaacgcctcgacgtggaggaatactgcatcagcgaaggctggatcaaggtgcccgctggcaagacggtggaccgcaagggcaagccgctgctgatcaagctgaagggccgggtcgaggcgttctatcggtaggagaacccactgcgcgaacagccgggcatccggcatggatctggagctgggagtaacctgccaaccattccattcgacgcagatgacgcagatcaaagccatgcagaaagctcttcgcgccgtgcgcggcgacatcaccaggctgcaggtcgatgccatcgtcaatgcagcgaattcatcgctgctgggcgggggcggcgtcgatggcgcgatccatcgcgcggccgggcccgagctggtgcacgagtgccgcctgctggcgggttgcaagaccggcgacgccaagctgacgaagggctatcggctgccggcccggttcatcattcacaccgtggggccggtctggcgcggcggctcgaacggtgagccggagctgctggcgtcgtgctatcgaaagtcgatggaactcgcagcgcagtgcggcgcacggaccgttgcgtttccgtcgatcagcacgggcatctacggctacccgatcgaactcgcggcaccccttgcggtggccacggtccgatcggcgctggcggagagtgccagcgtggaagaggtcacgttctgctgcttctcggacgcggaccttgccgtgtaccaggcggcgcttgcggcagcgggatctccatagaagtgcagatccccgccgcgccttacttcgtcgcctccaccttcacccgcgcattgggcgtctcgccgaacatctccggcgcatacatcgcttcgacgcggctcggcggcagcgcgaagtcgcccacgttgttgaggcgcacggtgtattcgaccttcacaacccccttgggcaggtactcgtagtagctgcggaaggcctcgaagctgcgctcttcgaacgccagccagccggcgcccgactttctctcgccctgcgtggcgatctgcgagtcgcggcccaggccgctgcccaggatggtggcgccgcccgggatcgggtcgctgaccacgacccaggtcatgtcggtgctggcgttcacctcgacggtcacgcgcagcacgtcgccgcgggtgtacttgcccgcgacggcctgttcgaccggcgtgatggtcttcttgatggcatagccggcggcaaacggcgccttcaactgcaccgcggcaatcgactgcatcgtgagccacggcttgccggtgccctgctgggtgaccagcagcgtgtcgcgcaccggcgcgcccgcgggtgatgcggaccagggcaggaacatggtgttgttcttcaggttgcccggcgaagcaggcgcgccgaagaaggtggcctggttcggcgcgccggccgcgtcggtggtcttcacgcgcgtgacgttgcgccagtcgacctgggccttcacggcacccagcgtggcggcggtaacgccggccaccggcgtgctttcgaacaccttggagaacttctcgagcgcgagcccgccccacaggttggcggtggtggtgtgccaggcgccgttctgctggcggccgatgaagccgttggccagcttgccgatgtcgtccttccaggccggatcgtccatcacgctgagcaggaggcgcgcggtgttgacgtcgccgttggtcatgagccaccaccagtagtcgtcctgctcggtgctgaagacgagcttggtgccctggtacgacagccgggccttgagcacgttgttggcctcgtccaggcgctgctggcgttgcggcacgtcctgcacgcgcttcaggatgttgagccagtcgatcacggcgccggtgggccactggttcggcgcaatggtgatgctgccgagcatgctgcccttggccgtgccgtagcgcgacagggcctccagcgcggcgagcttgcgcacgtccaggtccttgcgcgggctccagaactcgcgctggatgcggccttcgacaaaagcgatgaggcccgactccatcggcgcgcgcgcttcgtcgggcagcgcaaaggccgggttcagcgccgccgcctcgtgcgttgccgccagcaggtacgaggtgaggatgtcgctgccgcggttggattcgccgtcgcgcggcggaaagtagctggccaggccgtcgctgtccaggtacgtcggcagctgggccagcacgccctgccacatcttcgcgtcgcggaggcccaccgatttgctggtcttctgttcgaggcagctgaagggatagttcgcgaaccagtcctgcacgcccggcaaaccttcggcgagcttgggttgcagggaaagcttcaggccgccgcggccgggcagggcgtcggcgggcggcgccacgtcgagcgtgaaggggccatcgacctgcaccagcgtagcctgctgcactgtgagcggcaccgagggcacgatgcgctggcgcaccttgagcgcatcgcgcgcgccgccgagcgtgtccttggcctcgatctcccacaggatggcttcggcgcgcgtctgcgcgagctgcgcgggtgcggtcacggtccatgcgacttcgcgcgcttcaccggccgggatgtccacggtctgcgtttcgagcgtgagcagcgtggcgcgcggcgtggcttccaccttcatgggtttttgcgtggtgttgcgcagcgtgatctgggcgcggaactgatcgtcctcgcgcaccagcggcggcaggccgctgatgatctgcaggtcttgcgtggcctggatgctggcctggccggtgccgaagaggctggtgcccgaatcggccacggccacgatcttgaaggtggtgagcgcgtcgttgagcggcaccgtcaccacggcctggccgttggcgtcgagcaccaccttcgggttccacaagaggagggtgtcgagcagctcgcgcgtctgccccttgccgccgccgccgcccgcgggcacggccttgcgcccgtaatggcgccggccgacgatttccatctgcgcggtagacgtgctcacgccccagctgcgccgctgcagcatggcgttgagcaggttccagctgtcgttgggcatcagctccagcaaggcctggtcgaccgcggccaaggccacttcggcaccggccgcgggcttgccgtcgggcagcttggcggagatggtgatctgcgccttgctgcgcaccgggtagctgggcttgtcgctggtcacggtcacgtcgatctggtgcgcgcgcgtgccgacgcggatctcggccatgccgaggcggtaggcgggcttgctcaggtcgaccatcgcggtgggggcgacgtattccttgccttcgtaccagaaggcggtccaccactcgcgcggtgccttgaagccccatgtgaagaagctgtaccacggcacttcgcgcaggcggccgcgcagcgcgagcacgctcacgtaggcgttcggcccccactcgggcttgacctgcaggctcacggtcgggtcttttccgtcgagctgcaccacgcgggtttcgatgatgccttcgcgttccaccgacaccagcgcggtggcaaagcggaacgggctgcgcacctggaacttggcggtctcgccgggctggtagctcttcttctcgggcagcacgtcgatgcggtcgttgtcctcgccgccgaaccagagttcgccctgcttggtcacatacaccgagctggcggcgcggctgtcgcggccttcgctgtcggtggcgctggccaccagttcgacctcgccgggctccttcaactcggactcgcacagcagcaggccgcgcgcgtcgctcttgccgctgcagacggtgccgatgtccttggtctcggtcttgttgtcgtaggtgtagaagccgcccaccatgcgcttgcggctggtggtggtgatgcgcgccacggcgcgcacgttgagcgtgacgccggcctggggcttgcccgaaaggtcgagcgcgagtgcctggtacttgagcttctggctggtcgagacccagccttcggtcttgatgcccgcgatgaccgacgcgggccacagcgtctgcgtgctgcggatggtctgcacctcgccgttcggatcggcataggtggcttcgagcagcagctcgcgcgcggccttgaccttgggcaccttgtcgatcgtgaccttgccggcgccgtccttgttcagcgtgagcggcagcttgtcggcaatcacgcgggtgtcgctggcgctgttgatgtcttcttcgccgcctgctgtctcagccgcggccgcttgcgcgccgtcggcctgcacgcgcggcgggttgaagctgaaggcgtcatggtcggcgaagctcaggctcttgccgcgcaccatggccgacacgcgcaccggcaggttggcggcgccgccgccggccacgtagttgatctgcacgtcggccggcaccgagagcacgttcaccagcggcttcttgtcggtcggggcgatgcggccttcgagcacgggcaggcggaattcctcgacgcggaactggccggtggagaagctccggttgcggccgctctcgtcgccttcgccttcggagtcgccgctgtcggcgtccttgcccttgccggtgcgcagcatcacttcgtacacgccgagcttggcggccggcggtatggcaaaggtgttttccgcgctcaggccgccggtcggcgtcttgcgccaggccagcggctgcgtgaagcgctggccgctgccggtgtgggtcaccaccagcgtgtcgggccggttctcgggcaggccgaagcccttgctggtctgggtgcggatcaggtgcttcatcgacaccgtttcgccggcgcgcagcaaggtgcggtcgaagatggtgtgcgccacgcggtcgggctcgggctgcaggttggtgggcacgttgaagcgccagggctcgatgccgcgctgccagtcgctccaggtgaaggccaggtcctcgacgcccttgtcgtccttggcgcgggcgctgacgaaccaggcgcccgcgttgtattcgtccggcccattgcagttgggcgcctcgggcgagatgcccgtgaggttgacgatgccgttcgcgtcggtggtgccggtggccacggccttgccgtcgcagcccgacacgcgcacctcggcacccgccaccaccttgcccttgtcgagcgtggtgacccaggccatcgagttctcgcggccgagcttgaagtgcacggccaggttggtggccagcgcggtggtgcgcacgtacatcgtgcggctggcgccgtagcgctcgtcgagcagcgcgtcgcccagcttctgcgaggcgatctcgagcacgtggaagcccggcgtcagcggaatgccgatgacttcgaaggggcgcggatcgccgctctcggccttgggcatgtcgagcgccttcacgcccggctggcccgcgagaagagagagcatgcggctctgcacgcggctgcgctcgctggattcaatgaccgcgggcagcgtgcccttgacgtccttgcgtgcctggtcgcggctcacggtgtactcgtcgtagcggcgcaccttgcggaaccacgcgatgatttcggcgtcggtcttcgggttcatgtcgctgaccttgccgggcgtgagcgcctgcaccatgagcgcgggttccacgcgccgcacggtcaccggcatcatggccggcatgccgggttcggcgagccgttcgaccacgccgaagggcgaggccgcgaacttggccagcggcggcatcgcgccggtcgcgaccttcagcggaaaagtgccgggcgaggccagcgcccggcccgaggcatcctcgaacttggcgggcagttcgatggtgaacttggtgtcttccggcagcggcgggctgaagctcgcggagctgaccacgtcgtcttcgctggccgcgccgccgtcgttctcgagcgtggcggcaatcgtcttgccgccgcccttgagctggatctgcgaggccagcttgcgcgtgaccggcgcattgaactgcaactgcatcggccgcagcggcaggcaggcggcctgcgcgttctcgcgctcgcaggtgaaagacaccgcgaacggctcgcgcacctgaaagctcaggcggcgctccacgttgttggccacacccgatggcgtggccacgcccttgccgtagacgatctgcaccttgctgcccggcgtcagcgtgcggttgcattgcagcgcaatgaagcgcagcgggtccttcgcggcttccttttcgcggctgaaggccttgagcagaccggtgcgctgctcgccgtcgagcagcttgaccggaatgcgctcaccgatgccgtcggccgcgcaccagacgttctggcgcacgctctccaccgtggccgcgccgttgagttcgagcacgaacatctgctgttcgtcgatccggccatagctgcccggcatgaaattgcgcacgaacggtccgccgctattgaattgatagcgatccggccccgtcagctcgccgccggcgctgggcttgaaggtagggatgcgcgtgacggtgcagcgcacgccgggcggcaggtcgttctcgaagtcgtagacccactgcttggcgtcggtccagcggcctgtgcccttgccggcttgcgcgtcggtgcagctcaccgtgagcggcgcgggcgccttcgggtcgccgaaattgaccgcgggctggtcgaacttggcgacgatctggcgcacgcgcgccacttcgccttgcggcgtcaggctggtgatctggagcgcatggcccggcgcggccaaaaaggcgctgccggccaggagcaacgctggaatatttcttttcaattttttctccaccttgaagcacgcgcagcgtagccgatttgcacgacgcttcggctgtgccagtcgccatatgcctcgccccgacttcatacaatcggcactgtcgtgcgtgcgccgcgcggaccgccaccaagacctcgccgccgaccgatgaaacgctactgggaaatagacgccttgcgcgggctgatgctcgtgctgatgaccgtcacccacctgccgacccggctcacggacccgctgggccagcccttcggtttcgtctcggcggcggaaggcttcgtgctgctgtcggccttcgtggccgggctggtctacagccgcatcggctacgtgcgcggcgtcgactcgatgcgccaggccttctggcggcgcgtgctcaaggtgtatctctgccaggcggcgatcctgctgtttctcttcaccgtgattgcggcgctggggctgcacatcgaccagccggccgtgaagaacctggtgtcctactacctcgcggagccgcgcgacggcttcctgttcggcctgctgctcatctacgagcccccgctgctggacatcttgccgatgtacatcttcttcatgctgatgagcccgtgggtgctggcctttgcgatgcggcacggctggacgctggtgatgggtgccagcgccctgctgtggacgctggcgcagttcggcctgagcgaatggatctacgagctcgcgcagcgccacctggggctgccggttccgttccacgaaatgggcgccttcaacacctatgcctggcagttcctgtggttttcgggcctttgcctcggcgccagccgcaaccggcccgatgcgcggccgctgcgctttccggcttggctgtgggcgccggcgctggccattgcgctctatgggttctggtggcgccaccacggcatcaacggccaggcgccgttcggcggcgacgtggaactgaacctgctgttcgacaagtggcaactggggccgctgcgcatcgtcaacctggtggcgctgggcatcctggcggtgcgcttcggaccgtggttcatgcgcaagatcccgcgcctgcactggctggaggccatgggctcggcctcgctgccggtgttctgcgcgcacctggtggcggtgctgctggtgctggcgttctatggcgacagccagaccgcgcgcccctggtggggcgacggcctgctgctgctggcggtgttcgtgggcatgtacgcggtggcgcgcttcacgcgcggggccgacgtgccgccgccggcggacgatatgcctgccgagcctgcgcgcgcctgaggccgttcagggcagagaagccgccggggcgggaattgatgccggcaccgcccccggcaagcgcgccgagatgatcgactgccagagccggtagccctcgtcggtcaggtgcagccggtcgccgcgaaacagctcgggccgcggccggccgtcggcgccgagcatgggcgtgaagatgtcgatgaattcgctgtcgggcagccggttgaggtaggccgagatcacgttgttggtttcgcggaccagcggcatcaggtgttcgcgcgagggactcggcttgaccgagatgaagctgatgcgcgtgttgggcagctcggcgcgcacggcattggcaaagcgcgcaaaactttcgagcacctgcagcggcgtgcggccttcggccaggtcgttgtcgccggcatacaccagcacctgacgcggcttgtagcgcaccaccaggtcgcgcgcgaacaggctgcagtcggccatggtcgaaccgccgaagccgcggttgacgatgccgggtacctggcggaaatcctgcgagaggttcttccacatgcgcacggtggagctgcccacgaacaccacgccgccgggtggtgggaactgttgctggtcggcccgggcgaaggcagccagctcgttgtgccagcgcgcctttgcggcgaggtattcggaggaagcgtccgcggcggtggcgccgtccgcctcgtaagggaaggcggccgatgcggtctgggcatgcgaggcaagcgctgccgtcaatagtgcggctgcgagcagcgcggatttcatcgaagacatcgggaagacacgaagcagatcagatggttttctcaatcagggcgcccttgaatacgatggggcccttcggaccactgccgggtggcacgccgcccttggcttccaaggtaacggccagggccggcacggcgtggacttcggattctgacgcaggcagccgcagcgccggcgcgtggtcgagcacgccgagcgagcgcggcgtgccgcccggcggcagggcccagagctgcagcgacttgtcggcgccttcgtcgtagctgcccacgcgctgcagcaccagctgccgcttcctgggatcgaaggtcacgagcatcgaggcggtggccttgtcgtcggacagcaccgccacgtactggacggccggcgcgttctgcaactggtcgcgcaggttcagaccgacccccactgccatgacggtggcaagcgcaccggccgccgcggcgccgcgccagagtgcgaggctgcgcagccagccgccctctgccggagaagcgttgggggccgcaccgcgctgccgctcgatggcgtgctgcgcctgctcggcatcgatcatgttgcggatgcgggtccacacggccgcgtcggggacgaccgggctttgcagctcggtcatgctcgcgagccggctctgccacaccagcgccgcggcgcgcacgggcgcctgttcgcgcgccagggtctcgaaacgcctgcgggcgccgccgcgcaacgtgccgagcgcatggctcgcggctaacaggtcgagcagttcggggtgggcgagaaggttcatggaaagcttgtcgtcggcgtcgcggctaggcgaagcgccccatgcagaggcgcagtttttcgagcccgcgccggatccaggtcttgaccgtgccgagcggcagcttgagctgctcggccagttcgccgtggctcagctcgcgcaggtaggccaggctcacgacctcgcgctggcgggcctcgagctggctcaggcactggtgcagcgcccaggcctgctcgctggcgtcggccgtgtcggcggggttgggcgcgtcggactcgagggtctcggccatcagctcgtcgaactcctgggtgagctgggcgcggtcggcggtgcggcggcgcagcaggtcgagcgagcggctgcgcacgatcagccccagccaggcgagcggcgggctcagcgtgccgcggtagtcgccggccacgcgccagaccgtcatgaacgattcctgcagcacgtcctcggcccactcgcgctgccgcacgacccgcatcgccaggcccatgagcctgggcgccgtctggtcgtagagctggcgcagggcggcctcgtcgcggcggccgatgcgatcgatcagcgcgatcagttcggcatcggggctgggtgctgtcatgcgcggattgtggggcattggcctgcatggaaaagatacggcggggcggcccgggcagattcacttcggcggccgtgaatccatttggccgcggcctccgtacaggcctgcgaggccgtcgaaacgcacgacaccaagcacgggctcgctgtccattcacccgccatcgatacgaaagaaaaaggaaccgaccatgaccatccgcatcctgaccgcgctcgccaccgccgccggccttgccgcctgttccggcatgggcgccaagcccccgatgtattcccaggccggcctgccggatgccgtgaaggtgccggccggccatgcggtggccatggagaccgtgggcgccggcgacatcacctacgaatgccgggccaaggccggcatgcccggccagcacgaatgggtcttcgtcggccccgacgccaggctgatggaccgcagcggcaagcaggtgggcaggtactacggcccgccagccacctgggagagcatggacggctccaaggtcacggccacgcaggtggcggtggcgcccaacggcagcggcaacatcccgcaccagctggtgaaggcgaatccggcgatgggcacgggcgccatgcagggcgtgagctacatccagcgcgtgtcgacgcaaggcggcgtggccccggccgcggcctgcgacgcctcggccatgggccgcaagcaggttgtgaagtaccaggccgactacatcttctaccgcgccatctgagcgtcttcgggccccgctttccgtcacccggaaaacatttggcaacgtatactgcctcgcaaaatcggagcggggcgcaccacggtgcggggcagggaatgaaacaaatagcgatcgttgtcgcgctctgcgtgggcgcgtggtactttttcatcggcgggcgcaagctcgacgatgccatggtgcgccagtactacgagaaagaggcgcacgccatctattcgcgcgacgcggagaagctgtgcaagcagctcagcaagaaggtcgtcctccagagcaagacggtcatgatgggccgcacgcaggagaccaccagcgaccgcgaacaggcctgcgagtccttgcgcaagaccttcaagatgttcgagatggtgggcgaggggatgggcggcattctcaccatcgagtacgagtaccacatcgacagcgtcgagatcgcgagcgaccgcaagagcgccactgtcgccggcaccagcgtgctgaagatgggcgaggccgcgatgcagttcaagagcagcttcacgcagcgtctggagcgcgagatgggccagatgcggctcgtgcgcggcgacgacgtgacggtggtgcgcctgggcgggcgcggcgccatgagccagagcgacttcttcaagtaacggcaggcgccgccatcatgctcgccaacgattcgctgccgcccccgccgcctttctggcatcgcctcaacagcttcttcgcgtttccgttccagctgcggccgttgatgtatggcctcgggctcgcgttctgcagcctgctgttcgaggcgcttcccttcgtccacccggggctgtcgctgctgctgatcgagctgggcatcgtgctcgcggccagccgctatggtttcaaggtgaccgcgctcggttcgcgcggcatctggcgctcggccgattttccgcgcgagctcaacgaggactgggtcaacctgccgtggaagctgttcgccatctcggtggtgcagggcgcgctgatcggctggctggcatggttcgagccggtgctcggcaccgtggcgctgttcgtggtgtcgttcacctttccggccgcggtgatcgtgctggtgcagtcgggcagcttcttccaggccatgaaccccggccacgtgatggatgcgatgcgcatcatcggctggccctatgcgctgctgtgcttcttcctgttcctgctgagcacgggggcgcagatcgccatcggcgtgctgctgccgatgatcgatggggtcatcgtgctgccgatcgccaatttcgcattcatctatttcggctgggtgatggcgagcctgctgggctacgtgatgtaccagcaccacgacgccttcggcatcgacctgttgcccggcggcggcgtggacgacggcgcgccggcggatcgccgcacgcccgagcagattgccgcgcagcgtaccgatgccgaagtggcgcagctggtcaccgagggcgacctggccggcgcgctgggcgtggcctacgaggcgcagcgcgtggcatcgcccgacgacttggcggcgcagcggcgctatcaccgggtgctgctggtctcgcccgacaaggcggccaccttgctcgaccatggacaccgctacataccgctgctgctgcggcgcgacctggcgtccgaggcgctcaaggtcttcagggcctgccgcaaaaaggacaaggcttttgcgatcgacgacgcacccacggtgatgttgctggccaaggccgagtggcgcaatggcgatgcgcatgccgcgctggcgctgctgtcgggtttcgaccggcggtttcgcgggcatgcggccattccgcaagcctatgagctggcagcgcgggtgctggtgcaggggctgggccgcaccgacatggcgcagcccattctcacgacgctcgaatcgcgctttccggacagcgagcagacgcaggaagtgcgctggctgctgcggccgactgcctaggttgcccggctgatcaagcgcgctcgagggcgcgcgtcaccatgtcgttgggcgcgatccgcagcaggtgcggcagccagccgacggccatgtcgcgctcgccggcatgcagcaggccattggcgcagaccgacagcgtgtcggccagctcgggatggtcgggcgcggtcttcagcagcacgcggcacagcttgtcggcatcctggaactggcgcacgcgcgtgaagcggcgcgcgagccgggccatgtcgtcgggcttgagccgggcgcccggcttggcctggtcgaggtaggtggtgtagctggcgtgttgcagggccagcgtgtccggatcggtggccggcaggcggaagatgcggcgcgcggcctggtgaaaatcttcgcccccgggctgcagccgcgcggtgttgaaccaggcgcgcagcgtgtcggtgtcgccggggcgcaatgcggcggcggcacgccattcggccgtggcggcctcgaacttcatggcggcgcccatccggcgcgccgcggccacgtggcgatcgaaatcgccgttgtcggccgattgttcggaggccaccgtctccggcgtcttcacccggcccagcgccgtggcgcaggccatcagcgtggcgcccgccagaaggccgcccaggtgcgccatgtaggcaatgccctggccgcccaccagatgctggagtagctcgttggcaatccaggccggaagcagcagcagggccggcgcggtgacgtagttgaaatagaagaagagctggtagaagaaccggatgcgccgcagccggtacatcaccgcgtacatgcccatcagcgccgacaccgcgcccgaggcgccgaggccgtagctgcccttgcccgcataggcccagtcggccagcatcgaggcgcccaccgcgcccaggatgtagaaggtcaagtaggtgccgcggcccagcgccagctcgaccgagaacccgaacaggaagaggaacagcatgttgcccagcaggtgcccggtgctgccatgcaggaaggccgcggtaatccaggtccagggcttgaattcggcgtccttggtgtagtcctgcgcccagcgttcggtaaacggcgcgggccgcatcgattcgtactgctggcggtcgcgcttccactcggcgtagcgcggattggcgggcgtgacgacggcgtcggcccgcagtttctgcaggaacaccgtctcgtgctgcatgccgtcgagcagcagccctgtttcctcatgcgccagcaggcgccgggcggccttggcgcggggcgagcgcgtttcttcgagccaggccacgaagggcggcagttccagctcgggcagcacgctgtgcgcgtagtagtgggccgcgcgttcgtcggccttttcttcgctgcgctgcgggccccagaacacgatcatgttcacgaggatcagcagcaccgtcatccacggtggattgcgccagctcggtttgttctcgagcggaatggcgtagaacaagtgggctttcgctcaggcgaggcgtgcgcgatggcgcgcgatctgcgccttcacttgcgccggcgcggtgccacccaaaatgttgcgcgcattgagcgagccgcgcaggctcagcacgtcgtacacgtccttttcgatcttcggattgaactgctgcagcacggccagcggcagttccgcgaggtcgacctggtgcgaggtggcggctttcaccgcatgggccacggtttcgtgcgcgtcgcggaagggcaggcccttcttcacgaggtagtcggccaggtcggtggcggtggcgtagccgcgcagggcggcggcttccatggcctcgggcttcacggtgatgccgccgatcatctcggcgaagatgcgcagcgtgtctttcagcgtgtcgacggtgtcgaacagcggctccttgtcttcctggttgtccttgttgtaggccagcggctggcccttcatgagggtgatgagcgccatcaggtggccgaccacgcggccggtcttgccgcgcgcgagttcgggtacgtcggggttcttcttctgcggcatgatcgaagagccggtcgtgaagcggtcggcgatctggatgaagccgaagttctggctcatccacagaatgagttcttcactcatgcggctgatgtgcaccatgcacaggctggcggcggcggtgaactcgatggcaaagtcgcggtcgctcacggcgtccaggctgttctggcacacgccgtccatcttcagcgttttggcgaccagttcgcggtcgagcggatagctggtgccggccagcgcggcggcgcccagcggcaggcggttgacgcgcttgcgcacgtcctgcaggcgttcggcgtcgcggctgaacatttccacgtaggccagcatgtggtggccaaagctcaccggctgcgccacctgcaggtgcgtgaagccgggcaggatgacctcgacgttcttctcggcgatgtccaccagcgacacctgcagcgcgacgagcagttcggcaatcaggtcgatttcgccgcgcagccacaggcgcacgtcggtggcgacctggtcgttgcggctgcggccggtatgcaggcgcttgccggcgtcgcccacgagctgggtcagccgggcctcgatgttcaggtgcacgtcttccaggtcgagtttccactcgaaggcgcccgattcgatttcgctgcgaatctgcgccatcccacgctcgatctcggcgtggtcctgcgtggcgatgatgccctgggcggccagcatgccggcatgcgccagagaaccctcgatgtcggcctgccacagacgcttgtcgaagaacacgctcgcggtatagcgcttcacgaggtcgctcatgggttcggagaacagggccgaccaggcttcggatttcttgtcgagttggttttgagtcatgggagccgttcgagaggcaataatgggttggttacccaatgtatctgtgatgcgcaagccgtcgattttatcggccacctccacccccacgcctgcggccccgccggaaagagggcgtttgcctgcgcgcggcagcgccgggctgttcgacgcctgccagatcggggtggttttgcgcaccgtgctcttcgtggaagcgctggtcgcgaccgccacgctcttcgtgtcgtcctcccccacgggatggctggtgcagaccgccaccgtcacgggcggcgccctgcctgccaccttgttgtggctggtggccacctgcgggctcaagaagccgctcgggcgcctgccgcggcaggcgcagtacgcggccggtgccgcgctgggtgccctgtcctcgctctacggctgcggcctgctgcggctcaccggcgttcttggcacggcgccgtggcttgccagcgccgtggcgggcgccttcatttcgggcctggtcatggccgcgatggtgctgcgggcgcgcggccagacgccggccgccatgacggcccggctggaggaactgcagtcgcgcatccagccgcactttctgttcaacacgctcaacagcgccattgccctggtgcgcgaggagcccgccaaggccgagaccatgctggaagacctggccgagctgtttcgccaggcgctggccgacccgggcgaatccggcacgctggccgacgaaatcgcgctggccgagcgttacctggccatcgagcaggtgcgattcggcgaccgcctgcgcatccgctgggacctcgatgccgccgccagcaacgcccggctgccgccgctgctgctgcagccgctggtggaaaacgccatcaagcacggcgtggagcccagccccgaaggcgccaggctgcgcatccgtaccgagcgccgcggcagcgtggtggtgatcgaagtggtcaacagcctgccgcccctgcgctgggccgacgagcccctgccgcgtggccatggcattgcgctggccaacgtgcgcgaccgcctgcggctgctgcacgacatgcagatgcagttcagcgccggcatggaccagaagaactatcgcgtacgcattgccattcccgccgaaccatgactctcaagaccctgatcgtcgacgacgaagccctggcccgctcgcgactgcgaaccctgttgcgcgactgccgatcgcccgccgccgaagtggtggccgaggccgcgcagggcgccgaggcactgcagcacctggagagcatggcgctcgacctggtgctgctcgacgtgcacatgcccggcgtcgacggcatcgaggtggcgcgcgccctgcgcagccaggccgatgcgccggccgtggtgttcgtgaccgcccatgcggcccatgcggtgaccgccttcgacctggacgcggtcgactacctcaccaagccggtgcgggccgagcgcctgcagcaggcgctgcagaaggccgagcgttttctcaaggagcggcgcgcgctgcaggcgaacgccctgcaggaaagcgtgctcatccaggaccgcggccgcgccgagcgggtgccgctgtccgaagtgctctacctgaaatcggagtacaagtacctcacggtacgcaccgcctcgcgcagccacatcctggacggttcgctgaatgaattcgaggagcggtatccgggacgctttttgcgggtgcaccgcaatgcgctggtagcacgctcggccatccgcgcgctcgagaaatacgacgacggggaagacgccgaaggctgggccctgcggctcgacgcgatccccgaacccgtcgcggtgtcgcggcggcaactggctgcagtgcgcgaagtgctgaaggaaccgcgatgagcgacgacaagaaaacggccggccaggatgcggcggtgcaagaggagccgcaagtcgtggagcccccgccggaactgccccccgcacccgtgcccgagccgctgcgggaagccacggaaccggaaccggaaacaaagcccgaaccggaacccgagcccgaccgcgtgctgctgcacatgccggtcgacgtgcgcagcgcatcgctggtggtgctcgccgtgctggccagcgtctttgccttgcaatgggcgtcggcggttttcattccgctgatgctgagcctcctgatgagctacgcgctgtcgccgctggtcgacgtgctcgagcgctggagggtgccgcgctggatcggtgcggcggtgatcctgctgagcctgggtggcggcctgggctggaccggctattcgctgtcgggcagcgcctccgagcttctcgatgccttgccggtggcggcgcagaagctgcgccaggccacgcgcagcgacaagaacgccgccgccacgccgctggacagcgtgcagcaggccgccgcgcaactcgaacgcgcggccgaggaaaactcggcccgcgtcgcggcgcgcaaaggcgtggcgcgcgtcatcatcgagcggccgccgttcaacgtgcgcgagtacctgtggagcggcaccgtggggctgctcgccgccgtggggcagctcaccctggtggcctttctcaccttcttcgcgctgtgctcgggcaacacgttccggcgcaagctgatcaagatcaccggcccgagcctggagaagaaaaagatcaccgtgcacgtgctggacgacatcacgcaaaacatcgagcgctatctgctggtgcagatcctgaccagcatacttgtgggcgttgccacggggctggcgttctggtccctcggcctggacaacgcggccgtctggggcatcgtggcggcggtgaccaatctcatgccgtacatcggctcggtgatcgtcatgtccgcggcggggctggtggccttcgtgcaattcaacaccatcgaaatgggcctgctggtggccggcacctcgctggtcatccacaccctcgtcggcaacctgctggtgccctggctcaccagccgcaccagccgcatgaaccccgtggccgtgttcgtcggcgtgatcttctggggctggctgtggggcgtctgggggctgctgctcggcattcccatcaccatggtgatcaagtcgatctgcgaccgggtcgaagacctgcagccgatcggcgagttgctgggggagtagccgaggcgggcgccttactcggccgacgaagcagccagtgccgccgcgccaccgcgtgcgcggcccagcgtgccgacgatgagcgcggcaatcagcaccagcacgccgctgagcaccatcgcgctcgagatgccgtagttgtcgaccgtgacgccgccgatcagtgcgccggaagcaatcgccacctggaagccgctcacgagcagggcctggccggcttcgggtgcatcgggcacggcttccatcatccagcccgtgagcgccacagggatcaggccaaaggccacgccccagatgaagaccacgaccgcgccggccacgaagccgctgccgatcaccgtggacagcaagagcgcggtcgcgagcatcagcgccgccagcagggtggtgccgcgcacgctgcgcgccaccaggctgccgccgatgaaggtgccgatgaatcccaccgcgccgtagaccagcagcagcgtggagaccgagttcggcgccagcccgaatacctgctgcagcagcggcttcaggtaggtgtaggccgcgaagtggccggcaatgaagaacagcaccgcgagcaggccgacctgggccatgcgccgcgtcaacggcgtgagcaggtcgcgcgcaccgatggcgcgcaccggcggtatcgcaggcagcagccacagctgcaccaccagcaccagcgccgcgagcgcgcccgtcaccgcgaaggaagcgcgccagccgaacagcgtgccgaggaacgagcccgcgggtacgccgagcaccgtggcggcggacacgcccgccagcaccagcgacatggcccgcgctttggaggcgtccggcaccagctgcgtggccgcggccggcgcaaaggtccagaagccgccgacgcacaggccgagcatcagccgcgcgaccagcatggtggcaaagttgggcgcaaaggcggcgagcaggttcgaggcgatcagaagcgtggtgagcgcgatcagcacggtgcgccggtcgaggcggcccgacgcgacgatcagcgccggcccggcgaaggcggccagcacgccgggcatggtgatcatcaggccggccgtgccgtcggacacgtggaggccgcgggcgatgtcggtcagaaggccgatgggcatgaactcggtcgacaccatcgcgaaggtgcccacggcaatcgagccgacggccaaccagtcggaacgggtggagcgggcgaccttggccggctcgtgcacgagatcgtcgacgcaggggttgctgctgggtgaattcatcatgggaaggaggtcctgggatcgcatcggcgaagcgcgtgccgacacgttgttgcgaaaggccacccagtgtccaggcgcaagcgcccttcacaaaggggctcgccagcagttgtcagtttccccagagcgaacaatcgacccttttgcttgtcgcgctcttctctcgatccgctagatgcgggctgcgtgcagctgcagcacgcggccgtcggcaatgaaagagtcgcccaccagcacacgaaaggcctcaccttcggggaagtgcgcctttgccgtgtccggcgtcagcaattcgacgtcgatcgcatgcggcgtgccccgctcgagcacttcgccctgcggcacgaaccatcgcgcggagaagccctggttgcccaccaccagcgccgagcggtattccccggcggaaagcggcacgttgtgcgaaagcagcgctgtcggccgcagcgtgagttcgatgcgaaggtgcggcgtgaacgcgccagccgcatcgaagctcacgggctcggccggcggcgtgcgccgcggcagcttgccgatgagccagccgattacgttgccgatgatgggcacccaaagcaccatcagaagcgtgccgatgtcgcgcgtggtcgacccgcgctcggcgtagtgccgcacgagcgctcctcctatcgccacgcacagaaggatgatgacgatgagtttgcggcgagactggatggtgctcatgaacgagcgcttaccgatggattcactcgcatcagcccgtgttgcgcaagcccgccgcgaccccgttgatggagatgtggatgccgcgctgcagccgctcaccgccttcgcccgcccgatagcgccgcatcagttcgacctgcaggtgatgcagcgggtcgatgtacggaaagcggtggcgcaccgagcgctgcatctcggcattgccttcgagccgctgcttggcgccggtgatgagggtgagcgcgtcggaggtgcggtgccattcggtgtcgatcatcgagaacaccttctggcgcagcttgcggtcggtcacgagttcggcgtagcgcgaggccagtgcgaggtcgctcttggcaagcaccatgtccatgttggagagcagggtgcgaaagaacggccactgcgcatacatgcggcgcagcagcgcgacgcgttccttgcgcgcggccggcgtttcggccgacgccaggaactgctccacgcccgagccgaagccgaaccagccgggaatggtgagccggcattggccccagctgaagctccacggcacggcgcgcaggtcgtcgatcttgtggctcgggttgcgcgaggcaggacgcgagccgatgttgagttcggcaatctcgcggatcggcgtggagccgaagaagtagtcgccgaagcccggggtttcatagaccagcttgcggtaggccgccatgctcgcggtcgaaagctccccggctgccgaaaggaatgtggcgggcgccgacttggcctggggcagcagcgtggcttcgagcgtggcggccaccagcgtctcgaggttgcgccggccgatctcgcgattcgcgtacttcgagccgatgacttcgccctgctcggtgaggcggatctgtccgcgcaccgtgcccgggggctgcgcgaggatcgcctggtagctcgggccgccgccgcgtcccaccgtgccgccgcggccgtggaacatgcgcagacggatcgggttggttttcttcttcttgttgagctcgtcgaacagcgccaccagcgcgatgccggcacggtagagctcccagttgctggtgaagatgccgccgtccttgttgctgtcgctgtagccgagcatcacgtcctgctcggcgcccgagcgctcgatcagcgcctggatgttcggcagtgcatagaaggcgcgcacgatgggcgcggcgttgcgcaggtcttcgatggtttcgaacagcggcaccacgatcaggtcgcaggtggcgttgccgttcatcgcgccgcgcaacaggcccacttccttttgcagcagcagcgcttcgagcaggtcgctcaccgtttcggtgtggctgatgatgtagtggcggatggccgccacgccgtatcgcgcacgcgatgtgcgcgcggccgcgaagatcgcgagttcgctcttcgcgagcggcgagtattcggcatcgggcacgcgcagcggacgggcatcgtcgagcagcttgagcagcagcgtctgcttggcctcttcggccagcgaggcgtaggcgggctcgatgcgcgcggtggacagcagctcggcgatcacggcctcgtgcttgtccgaactctggcgcaggtcgaccgtggccaggtggaagccgaacacctccaccgcgcggatcagcggccgcaggcgcggtgcggccagcacgctgccgtgcttctcggcgagcgactgttccacggtgtgaagatcggccagaaaatcctcggcccgggtgtaggggttttgcggcggcacggcatggcgcgcggcctccccgccagtcaggtcgcgcagcgtggccgcaaggcgcgcatacaccccggtgagtgcgcggcggtagggctcgtccttgcggtgttcgctggtgtccggcgagcgttcggcgagcgcctgcatctcgaccgacacgtccaccagcgtggcggaaagcgagagttcgctaccgaggtagtgcacttcggtgaggtagtggcgcaaggccagttcggcctggcggcgcagagcgtattcgagcgtttcggccgtgacgttgggattgccgtcgcggtcgccgccgatccactggcccatgcgcaggaaggtcgccaccgaaggcacggtgccgccctggcccagcgccttttcaaggtcggcatagacgcgcggaatttcgcgcaggaacgtggcttcgtagtagctcagcgcgttctcgatctcgtcggccacggtgagcttggagaagcgcaacaggcgcgtctgccagatctgcgtgacgcggatgcgcatctgcgtttcgttctcggcaaattcgagcggggagagcgcgtcttttccgcccgcgtaggcgttctggcgcagcttgatctcgtcgcgcgtggtgagcagcagggcaatggcgcgctcggcatcgaggatgctcttgcgctgcacttcggtcgggtgtgcggtcagcaccggcgacacgtagctgtgggccagcgaagccaccacctcgtcaggcttgacgcccgccttgcggatgcgcgcgagggccgtttgcagatcgccgtcggcgctttcgccggcgcgctcggcctcggtgcggcggcggatcaggtgccggtcttccgccaggttggccaggtggctgaaataggtgaaggcgcgaatcacgcgcaccgtctcggccgcgctgagccccttgagcaggttcttgagcgcgcggtcggcggcatggtcggcatcgcggcggaaggacaccgacagcgtgcgaatcttctcgaccagcgcatagctctcctcaccctcctgttcgcggatcacgtcgccgaggattcggcccagaagccggatgtcgtcgatcagcggctggtcttcggcttggcggcgcttgggcgcggcaggggtcgtgctggctttcattcgatgttgttcctggggacttgaatggacgcgccgcctgcgttgctgcggcgcaacatgctagcattccggaggtctgaaacttgtactttttggggacggtcttgagcaatatcgtgatcgccacgcgcgaaagccggctggccttgtggcaggccgagcacgtgcaggcgctgttgcaagaaaaaggccactcggtgagcctgctgggcatgaccacgcgtggcgaccagatcctcgacaagtcgctcagcaaggtgggcggcaagggcctcttcgtgaaggagctcgagctcgcgctcgaggaaggccgcgccgacatcgcggtgcattcgctcaaggacgtgccgatggatctgcccgaaggctttgtgctggcctgcgtgctggagcgcgaagatccgcgcgacgcgctggtgtcgccgcgctatgcctcgctcgacgaactgccccagggcgcggtcgtcggcacctccagcctgcggcgcgtggtgctgttgcgtgccctgcggcccgacctgcgcatcgagccgctgcgcggcaatctcgacacccgcctgcgcaagctcgacgaaggccagtacgacgccatcgtgctcgcggcggccgggctcaagcggctcggcctcgaagagcgcatccgtgtcgcgttcgagcccgacaccatgctgccggccgcggggcagggcgcactcggcatcgagatgcgggccgaccgcgccgacctgatcgcgctgcttgcgtccctaaatcacaggggcgattggctggccaccgccgccgagcgcgcggtcagccggtcgatgggcggaagctgctccatgccgctggcggcccatgcgcgctggcaggccgacggcgcattgcgcatcgatgccgcgtggggcgatcccgagggcaacgcgccgctggtgcgggttcatgcagaggctgaagcggccgattttgcgcaggccggcgtgctgggtgagcaggccgccgcgctgctgcgcgccgctggcgctcattgaagcaggcgacccaagagacatggctgccgccaagcccgtgatcgtgacgcggccggcgcgcgaggccgtgcagtgggtggacgaatttcgcgccgcggggctcgaggcggccccgctgccgttgatcgccatcgagcccgccgtcgacgccgagccgctgcgggcctcctggaagcgcctgtcggactacgcggcgctgatgttcgtgagcgccgcggccgtcgagcatttctttcttcacgcggaaggcgcacaagcaaaagccgcgattgcggcgggcctgcgtttctgggccaccggtccgggcaccgcgcgcgcgctgctgcgtgcgggcgtgcccaaagaggccatcgatgcacctctgcccgatgccgcgcgcttcgactccgaagcgctgtgggaacgggtgcgaacccaggtctcggcgggcgtgcgcgtgctgatcgttcgtggcggcgacgcggccggccatccgagcgggcgcgactggctcgccaacgaaatcgaagccgcgcagggttgccgcgacaccgtggtcgcctatcggcgcctgccgccgtccttcgatgacgcggcgcgcgcgctggcgctcgagggcgccgcgggccgtgcgatctggctgttcagcagctccgaagccatcgcgaacctgtgcgatgcgatgcccggcaccaagtggcatgcggccggcgccgtggctacccatgcccgcatcgccgaggccgcgcgggccgcgggattcggcgtggtgcgggtgtgcaagccgctgcgtgaggcactgatcgcgtcgatagaatccttcacatgagtgccgcgtccccgtccgacgacttctccccccatccgccaccgcaccggtgcctgcaccgctggcggcatcgcagtcgccggagtcgctggcggccgccgcgaccacgctgtcacgcatcgggctcggcctcttggccctggtgtcgctcgcgtcgctggtgattgccatttccctgtggcagaaggtcagcggtatgcaggagcagctggcgcgccagagcgcagatgcacaagcccagtcgctcgaagcgcgaacgctcgcacggcaggccatcgagaccgtgcgcgacaccgcggcgcgtgccgccctcaccgaaacccgcgtcgccgaggtcgcgctccagcgatcgcagctcgaagaactgatgcagagcctctcgcgctcgcgcgacgagaacctggtggtcgacatcgagtcggccgtgcgccttgctctgcagcaggcccaggtcacgggcagcgtggagccactgcttgcggccctcaaggccggcgatcagcgcattgcgcgcgcggcgcaaccccggcttgcgccgctgcagcgcgccatgcagcgcgatgccgaccgcttgcgcagcagcgccagcctcgacagcggcgaagccctgcagaagatcgacgagctgacgcgcggcgtggacgatctgccgccgctcaatgcggtggccatgcgcgggaacggactcaacgcctggcaggccgaacccattccggccgacgcgccatggtgggagcgggcgcttctcacggtgcgcgccgaggcgcggtcgctggtgcgggtcgggcgcatcgatcgcccggaggccgtgctgctggcgcccgaccagacttttttcctgcgtgagaacctcaagctcaagctgctcaatgcgcgcctctcgctgctgtcgcggcaggtggatgtcgcacgcagcgagctcgccacggtttcggcaacgctgaaccgttatttcgatccggcgtcgcggcgcacacaggccgccgcaacactgctgcagcaactccaggcccaggtgaagacctccgaagctccgcgcatcgacgacacgctggccgcgctggcaaccgcggccgcggggcgctgatatgagcccccacgttcctcacttcgtgtattcgctgccccccgagggggcgcaggcctgccttggggcggcccggcgggaggactgacatgagggcagcactctggctcctggcgctgttcgccattgcggcggcggtggccctgttcgccggcaacaaccagggcacgatcacggtgttctggccgccatggcgggtcgatctttcgctcaacctggtgctggtgatcctgctcggcgcttttgtcctgctgcaccttgcgctgcgcggcctggcggcgctgttctcgctgccgacccaggcccgccaatggcggctgcagcagaaggaacgcatgctgcattcggccttgctcgattcgatggtgcaactgctgtcggggcgcttctcgcgcgcgcgcaaggccgcgcaagcggcgctggtccaggaaaggacgctggcggccctcgatgccagcctgccgcaggctcatcaggttcgcgtgctgtcgcacctgctggccgccgagagcgcacaggcgctgcaggaccggccggcgcgcgatgcccacctgcagcaagccctcaacgaaagcgccgatcgcaccatgctggccacgccggaaacgcgtgaaggcgtgcagttgcgcgccgcgcgctgggcgctcgaagaccgcgatcctgcggcggcgctggcccggctcgaagagcttccccaaggcgtgcaacggcgaaccctcgcgctccgcattcgcctgaaggcagcgcgccaggatcggcgcacgctcgaagcgctggaaaccgcgcgcctgctcgccaagcaccgcgcgttctcggacgctgcggcgcagagcatcgtgcgcggcctcgcgaccgagctgttgtccggcgcgcacgacccggcgcaactgcttcgtgcctggaccgaactcgacatggccgagcgtcaaatgcccgaggtggcgattcatgccgcccatcgcatggtggccttgcgcggcgacctggcactggcgcgcgaatggctgctgcccgcctgggagcgcatggtgtcgcagcctcgcgcgctgggcgacgccctgcgcgtcaagctggcgcgggcgctcgaagcggggctcgattcagtggacgcggagtggctcgcccgcatcgaatcggcccagcgaaacaatccgcgcgaccccaacctgcagtacctcgcgggcatggcgtgcatgaagcgacagctctggggcaaggcccagcagttgctcacccaggccggcctgggcctgcaggacacggacctctatcgccgtgcatggctcgcgctcgcagaactggccgaagcgcgcggggatgcagagcacgcggccgaggcctggaagcgcgccgcgcagaccgagaaggtctgaaggggctggcagcccctgacgctgcccgcggtgcaccagacagtggccgctcctgcggttcagcggtttcgttccccataaaaaaacggcgccgaattggcgccgttttttattgttctcgggccgtcgggcccgggatgcttcagttcacgccttgtgcgtcggacggcgccttttcgaaaggcagcgtcatcgaaccgagttcgcggcgggtttcgaccagtaccagcggaccggcgtcgagcacgatggcgggcgggcgttcgcgcggcacatgcaccggctttggctcggccgcgatggctgcacgggcctgcgcaatgcgctcggcgtcggagttcacccactgcagacccgaagtctcggcgatctgcgccagttcgctcagcggcagttcgaaaggctgaaccttcggcaaggcgcggccgttggcggcaggcttgctgctgctgacgctgctctcgaccacgacgggagcgacggtgggcgctgcggcaacggcaacgggagcgactgctgcgggcgccggtgccgctgcaggacggtcgaagtagctccgcggtgcgggtgtgtaggcttcttcgggcactgcggcgcgggcttcggcgtgttccggctgctgtcgcacgggcgcttcgttcgcctcggccgatgcgccggccacattggcttcgctctcgtcgcgcggaccgcgttcgcggcggtcgcggccataacggtcgcgtgaacgaccgcggcgctgctcttcgccttcgcggcgcggcgcttgctgctcgttgccaccgatctcgccttcgttgccgggcgcgacgtcagccggctcggcgccgcgcagacccgcttcgtcggcaggtgctggtgcttcgccgttggcgaaacgcggttggccttcaccgcggcgctcgcggcggccgtcgctgcgttcaccacgcgggccgcgctcttcacggccgccgcgcggggcgcgttcggcttgcgtgccgtcctgggcgtcggcgttgtcgccaccgaacgcgtcgcgcggtgcctcggcggcattgcgctggtcgccgcggtcactgcgttcgccacgctcagcacgttcaccgcgctcgccacgttcccggcgttcgccgcgggcgcggggcgcgcgttctgccggtgcattgccttcgtcgccagccggcgcgttgggcgccagttgctgtgcttcgagattgccgtcgaattcggcagccactggccgggcctcgcggccttcgccttcgcggcgttcgccacggccgccgcggcgttgttcgccttcacgcggaccacgtgcttcacggggttcgcgctgctcgcggggttcgcgttgttcgcgaggctcacgctgctcgcgcggttgggcggcttcgctgcgcagttcgctgctgcggccttcgcgtccttcaccacggcgctcgccaccacgtccgccacggcgttcgccgtcgcggccaccggagcggccagcgttttcgctgcggccttcgccaccgcggccaccgcggcgctgctcgccatcgcgggcgccgcgcgcttcaccgtcgcggccggagcggccgccatcacggcgcgcgggcttcggtgcctcgaccggaatcacggccggtgcgggagccggtgccggcgtgccgccgaaccagctcttgaggcgcgcgaagaagcccatttcggccggagccggtgcacttgccacgggcggtgcgaccggtgccggggccacggcgggtgcgcgcacggcttcgggcttgggcggcaccacgggcgccggtgcgtcgggcagtacgcccttgatgaccggcgtctgcttgttggtgggttcctgcgaacggcgtgtcacggccgtcgggtcttcgatctcgtcggccatcctgtagctggcttcgatgtggtcgaggcgcggatcgtcgtgcttcaggcgttcgagcttgtagttcggcgtttcgagcgtcttgttgggcaccatcagcacggtgacgcgctgcttgagctcgatcttggcgatttcggggcgcttttcgttcagcaggaatgacgccacttcgaccggcacctggacgtgcacggcggccgtgttgtccttcaggcactcttcctgaatgatgcgcaggatctgcagcgcgctcgattcggtgtcgcggatgtggcccgagccgccgcagcgggggcaggggatcgacgagccttccgagagcgccggcttcaggcgctggcggctcatttccatcaggccgaacttgctgatcgagccgaactgcacgcgggcgcggtcctggcgcagcgcgtcgcgcaggcggctttcgacttcgcggcggttcttcgactcgtccatgtcgatgaagtcgatgacgatcaggccgcccaggtcgcgcaggcgcatctggcgggccacttcgtcggcggcttcgaggttggtgcgggtggcggtttcttcgatgtcgccgcccttgatggcgcgggccgagttcacgtcgaccgacacgagcgcttcggtgtggtcgatcacgatggcgccgcccgagggcagctgcacggtgcgcgcataggccgactcgatctggtgctcgatctggaagcggctgaacagcgcggcgtcgtcgcggtagcgcttcacgcgggcggcatgctcgggcatgacgtgcgccatgaactgctgcgcctggtcgtagatgtcgtcggtgtcgatcaggatgtcgccgatgtcgtgattgaaatagtcacgaatggcgcgaatgacgagcgacgattcctgatagatcaggaaggcgcccttgccgcccttggccgcgccgtcgatggcgctccagagcttgagcaggtagttcaggtcccactggagttcgggcgccgagcggccgatgccggcggtgcgcgcgatgatgctcatgcccttcgggtactcgagctggtccatcgcctccttgagttcggcgcggtcgtcgccctcgatgcgccggctcacgccgccgccgcgcgggttgttgggcatcagcacgacgtagcggccggccagcgagatgaaggtggtgagggccgcgcccttgttgccgcgttcttccttttcgacctggacgaccagttcctggccttcgcggatgacgtcctggatgcgtgcctggttggcggaaacgccttcggcaaagtattgcttggagatttccttgaacggcaggaagccgtggcggtcttcaccgtagtcgacgaaacaggcttcgagcgagggctcgacgcgcgtcacgacggctttgtagatgttgcccttgcgctgttcgcgcccttcgatctcgatttcgtagtcgaggagcttttgcccgtcgacgatggccaggcggcgttcttcggcctgcgtggcgttgatcagcatccgcttcatgatgcgttgtccttatatgtatcgttcttgcggcccatgacgggccaacgatgcacggacgacgcccgcgaaacgaggggaattgccgcttggccccggttgctgtcactgccgcggcaagcgcgaacaggcctcttgagcgtcagctcaagaagacagccggggtgggggcgcgtggatgggcgcgagccagattcggtgttgagcagctatcttattgatagctggttgcgcaatggtggcgcgcggtgcggatgactcgatgcctgaggccgctggcagaagccaggtgggccagcgcaggcacatttgaatcagcagcatcaacacaagggactcgcttcgatccgcctgcagcttggaagctgcaggctgggtattccgtatcggtgtttcgtgggtgtcggcttaacttgggtgcagggtctgccactttgcgccattgcgcggggtttgcagtctcggcgccaaagcggcatcgacctcgcagcgttgtcctgggcgtttgactgcagtgatctaaacttctgtctaatcaagcacttacacgaccgcgctggtgaaaaacattataggtgcgaagcaaagccctgcggccgctccaaatcccgcagatcaaaaagccgcggccgatgccggggcgccgcacgcgtccatcaaattcattactgtggacgcggaatccgctgggcagcggctggacaacttcctgttccgccatctgaagggcgtccccaagacgcatgtctaccggatcatccggtcgggcgaggtgcgcatcaacaagggtcgggcgcaggccgattcccgcatcgagaccggcgacgtgctgcggctgccgccggtgcggatttcgccgcgtgccgaagagggcgccacggcacccgcgcccgcgcgcgaatttccggtgctgctggaagacgacgcgctgattgccatcgacaagcccgccggcgtggcggtgcatggcggcagcggggtgagttttggtgtgatcgaacagctgcgcacggcacggccgggcgcgaaattcctggagctggtgcaccggctcgaccgcgagacctcgggcatcctgctggtggcgaagaagcgcagcgcgctggtggcgctgcaggaccagttccgcgagcgcgagacgggcaagacctacctcgcgctggtcgaaggtgcctggcccgccaacaagaaggtgctcgacgcgccactcgccaagtacctgctgccgggcgacggtgccggcgccggcgagcgccgcgtgcgcgtggtcgccaaggaccatcccgacgccatgcgcgcggtgacgctggtgcgcgtgctggcgcggctcacgctgcccggcgatgccgcgccgctgtccctgctggcggtcaccatcaagaccggccgcacacaccagatccgcgtgcaccttgcatcggccggccatgcgattgcgggcgatgacaagtacggcgacttcgaacgccagcgcgtgctccataaactcggcctccggcgcatgttcctgcatgcctggcggttgcagttcaaccaccccgcgaccggcgagcgtgtggcgctgcaggccggcctgccgcccgaactgcacgcgttgatgccgtcccatgcgctcgaggcgcttgcccaacacccgactcccacggccaatgactgaatcttccagacccctgcgtttcgacctgatcgccttcgattgggacggcaccctttacgactccacgcggctcatcgtgcgctgcatccaggcggccgtgattgacgtcggcggcgccaagccaagcgagaacgatgccgcatgggtcatcggcctgggcctggcggaggccctggcgcgcgcggcgcccgacgtgccgaaggaaaaatacgccgagctcggcgcacgctaccgctatcactatctgcagcaccaggacgacctcgtgctgttcgacggcgtgctgcagatgatcgacgccttgcgcgcgcgcgggcacaagctcgcggtggccaccggcaaatcgcgccgcggcctgaacgaggcgctgaagtcgatggcgctgcgcgaccgcttcgatgcctcacgcacggccgacgaaactttcggcaagccgcatccgcgcatgctgcttgagctgatggaagagctcgacattccggccgagcgcacgctgatgatcggcgacaccacgcacgacctgcagctggcgctcaatgccggctgcgccagcgtgggcgtgagctacggcgcgcacgagcccgagagcttcgacgtgctgaagccgttgttcgtcgcgcactcggtggccagcctcgaagcatggcttctggacaacgcctgaaaatctcgcgatgagcgaagaagagcccatccccctttgcaacgcctcggacctggtcgaaggcgaccgggccgtgccattcgatgtggtctacggcggtgaaacctgccgcgcctttgcggtgcgcttcgaagggcagccgcatgcctatctgaaccgatgcagccacgtggcgatggaactcgatttccagcccgaccgtttcttcgacgacagcgggcagtggctgctctgcgccacgcatggcgcggtctacaggccggacaccggcgagtgcgccggcggcccgtgccgcggcggcctcgtgaagatcgccctcagcgaacgtgacggcgtggtgcactggcatactgcctggaacctccaccccctgactttttgacaatgaccgacccgaaccgcacggaacccgaaggttttgatccttttgagccggccactcccattgcgtcctcgcagggcgcgccaagaaacatggccaaagacccgacgcagcgcccagggtgggagcgcgcaacgctcgagaaacttgccttcgcctccctgaacgagcagagggccgcgcgccgctggaagaccttcacgcgtctttcgtggctcgccttcttcatcttcctggtctggctcgcgatgtcgcgcaacgcgccgagcgcggccaagaccacggcccacaccgcggtcgtcgaaatcaagggcgagatcgccaacggcggcgacgcgagcgcggaattcgtcatagccgcaatgaagaccgctttcgaggacgagggcgccaagggcatcgtgctgctgatcaactcgcccggcggcagccccgtgcaggccggcatcatcagcgacgagatcaagcgcctgaaggccaagcacaagaagccggtgtacgcggtggtcgaagaaacctgcgcctcggccgcctattacattgccgcggcgaccgacaagatcttcgtcgacaaggccagcatcgtcggcagcatcggcgtgctgatggatggcttcggcttcaccggcgtcatggacaaggtcggcgtggagcgccgcttgctcacggccggcgagaacaagggcttcctcgacccgttcagcccgatgagcgacgcgcagcgcgctcatgcacagaccatgctgaaccagatccacacgcagttcatcaacgtggtgaaggccgggcgcggcgaccggctcaagctcgacaccccggggcttttcagcggcctgttctggagcggcgaacaagccgtcgcgttcggcctggccgaccagctcggcaacgtggactacgtggcacgcgaagtgatcaaggccgaagaggtcaccgactacacgcggcgcgacaacgtggcagaaaagcttgccaagaaattcggcgccgcgatgggcgatgccaccgtgcgttcgctgcagttcgccacgccggcgctgcgctgaggccggcggccggctcagcttgggttgccgctgtccgtgaaacgggcggaggcggccagcgccaccgcgaaaaccacgaccacatagagcgcggctgtcagcgaactggcccgcgccagcaggccgatcacggccggtccggccatgaagcccaggtaggcgatggccgagacggccgcgatgcccgttgcggcttcgacgccgggcacgcgggccgatgcgccgaacaggatcggcaccacgttcgcgaagcccacgcccacacccgcgaagccgatcagcgcgagccagggcaggtcggtcagcagaaccagggtcatggccgccgccgcgagcaggccgctgccgagcagcagtgcagccggcgagaagcgcgcacgcatcgcatcgccagcgaaacgcgcggcggccatggcggccgagaagctcgcgtaggccagtgcggcctgcttctgcgggctgccgagttcctgctgcatgtagagcacgctccagtcgtagatcgcgccttcggcaatcaggcccagcgcggcaagcaagcccagcactgcgagtacgccgcgaggcagccggaatgcgtggtcggccggggatgcgtcgcttgcggcaggtggcttggggagcatgtgccacgaagacacggccaccaccagcaccatggccgccgccacccacagcagatgggcctgggccccgagcccggccgccagtgccgcgctgccactcgcggcgccggccatgccgcccaggctgaacatgccgtgcatgccgctcatcagcggtttgccgccatgcagctcgagttgcgccgcttcggcgttgatggccacgtcgaacacgctggtgacaagaccgaagactgccagcagcgccaaaaggaagaggtagcccggcatggcaatcaacccggccagcagcagcgcgtagacgcagccgcagagggcggccatgcgccgcgggccgtggcggccgatccagcgccccgcgctggtcaggccgaacatcgccccggcgccggccgcgagcatggccagccccagctcggcttcgtcgatcccgtagtgcgacttgaccgttggaacgtgcacgccccaggtcgcgaagatgaagccggaagaaaagaactgcgcgcgcgtggcccagcgggcgccggcagtcaccaccatcgtcagcgcccgatcgcgaataccgcgggcaggcgttcgtccgtcgggctttgcgccttggagcgccaggccttcacggtttcgctgcgcacctgggctgttgcaagcgtcagcccgcgcgccacggccagccgggtgttgtgctgcagcgtttgcaccagcgcttgaagcagcgcggcattgcggtagggggtttcgatgaacagctgcgtctggccggtcttgagggccagcgcctcgagctccctgattcgaacctggcgctcgctcgaatcctgcggcaggtagccgacgaaggcaaagttctgtccgttgaggccgctggccgccaacgcgagcagcagcgatacgggcccggtgagcgggaccacggcaatgccaagctcgtgggcggcgcgcgccaccgaggagccggggtcggccaccgccggcatgccggcttcgctgagcaggccgatgtcgtggccttcgagtgcggcggccagcaatggcttggcatcgaactggccggcgtggtcgccttttttgtgcacttctcgcggcagttcgcgaatgtcttgtgcctgcaggggcgctgcgagcggaacgacggcgtcgatgcgcttcaggtaggcgcgtgccgacttggcgttctcgcagatccagtgggtgatgccggcggccgcttgcagcgtgcccaagggcagggcgtcctgcaggggcgcctgtgtatcgcagccgaagtccagcggcgcgggcaccaggtagagtttgccccgggtcacagcagatcgaccccggcggaacgcagcatccggcaggtgcggattaacggcaggccgaccagggcggtcgggtcgtcgctgtcgatcgcgctcagcaaggcgatcccgaggccttcgctcttggcgctgcccgcgcagtcgtaaggttgctcggcctgcaggtagtgctcgatggccgcatcgctgagttcgcggaacaccacccgaaccggcgccaggtcgcgctggacgaagcccgtggcctggcagacgacggccacggcggtctggaacaccagtgtctggccgcgcatccggcgcagctgggccgtggcgcgtgcgtggtcgcccggcttgccgagcgcctcgccggcgaggtcggccacctgatccgagccgattaccaccgcctcggggaatcgcgcggcgacggcctgggccttttccagcgccaggcgctcggccagttcgcgcggggtctctccgctctgggcggtttcgtcgacttcggggggctgcacgtcgaagggtaggtggaggcgagccagcagttcgcggcggtagcgcgaggtcgaggcaaggatcagggggcgttgcatggcgacgattgtgcgtgagctgccaaaaagcctttggcggcgctccgccaattcccgcggccggcgcgctagactggagcggatgaagagagaatttgttcccgaacggctcgacgtggccgcctttgccgccgaagccgcggcgctttcagccgacgatcccgttcccaactatccccgcctggcgcaggaactggcctcgccggcgctcgatgccgtggtccactgggaagccgtgggcgagcagcgcaccggcgccttgggcaaggccgagccctggctgcacctgatggccgaaaccacggtgccgctggtttgccagcggtgcctggcaccggtggatacgcttgttgcatcggaccgctggttccgcttcgtggccgacgaggccacggccgacgccgaggacgacgaatcggaagaagacctgcttgtcgtgagtcgcgatttcgaccttcacgccttgatcgaggacgagctcctgatggaaattcccgtcatgccagtgcacgaggtctgccccacgccgatccagctgtcgtccagcgacgaagacttccaggcggcggaagaggccaagcccaacccctttgcggtgctcggcgcgttgcgttcgcgcaagccggaagagggcaagtagcccttttcctcaggctaggctataatcatgggcttcgcgcgcgccgccgtgagcagcaagacagaccaaggcattccatacatgcccctgtattgccaccgccagagagcgcatccaatcactcacctaacagtccaggagccatcatggccgtccagcaaaacaagaagtcgccttccaagcgcggcatgcaccgttcccacaatgcgctggtcgtgcccggcatcgccgtggaaccgaccaccggcgaaacgcacctgcgccaccacatcagccccaacggtttctaccgtggccgccaggtgctcaagaacaagtccgaagcctgatctcgcatcccaaggccaaggcccgaagctacttttgccgtagcgtcgggcctttgttttgatggctacgccttcttcccccgaattcaccgctgcgccttccgcaatcacgctcgccgtcgattgcatgggaggtgaccatgggccgcgcgtcacgctcgcggcctgccgcgcgtttctcgaacggcacagcgaagcttcgctgctgctggtcggcgcgcctgccgccttggccgggtttgccgcgcatccgcgtgcccgcatcgttgccgccagcgaagtggtgggcatggacgatccggtcgaaatcgccttgcgcaagaagaaagactcttcgatgcgcgtcgcgatccagcaggtcaaggatggtgccgctcaagcagccatctcggccggcaataccggcgccctgatggccattgcgcgctatctcctgaagacgctcgacggcatcgaccgtcccgcgattgcgcctcagctcccgaacgccaagggcggcgccaccacggtgctggacctgggcgccaacgtcgattgcgatgccgaagacctgcttcagtttgccgtgctcggctcggccctggtctccgcgctcaccggcaacgaagccccgtcggtcgggctgctcaatattggcgaggaagccatcaagggcagcgaaacgatcaaaaaagcgagtcaactgctgcgtacggctgccaactcgaaggatctgaacttctacggcaacgtggaaggcaacgatatcttcaagggtacgaccgacatcgtggtctgtgacggcttcgtgggcaacgtcgccctgaaggccagcgaaggcgtggcctcgatgatcggcgaattcatccgtgtcgagttttcgcggaacatcttgaccaaagcggcggcaattgttgcttacccggtgctaaaagcgtttaaaaaccgcttggaccatcgccggtacaacggcgctgccctgttgggcctgcgcgggctggttttcaagagccatggctcggctgacgaagtggctttcggccatgcgctggatcgcgcttatgatgccgctcgcaacaacctgctcgaccgcgtccgggcccgtattgctcacgccgcgccattgctcgcgcggcaggagcccgcggtgcccgccgacgcggcggcccttcacgtttgatgagccctttttcacgcatcaccggcacaggcagttacctgcctccgcgccgggtgaccaacgacgaccttgccaaggaattggcatcgcgcggcatcgagacctcgaaccagtggatcgtcgagcgtaccggcatccacgcgcggcacttcgcggcgcctgaagtcacgagcagcgatctcggcttcgaagccgcgcggcacgccctcgaggcggcggggcgcaaggccgaagaggtcgacctgatcatcgtcgccacgtcgacgccggacatggtgtttccgtcgtcggccgccattctgcagaacaagctcggcattgccggctgcccggcattcgatgtgcaggcggtctgcagcggctttgtctatgcgctgaccgtggccgacgcgatgattcgcaccggcagcgcgcgctgcgcgctggtgatcggcgccgaagtgttctcgcgcatcctcgatttcaacgatcgcaccacctgcgtgctgttcggcgacggcgccggcgccgtggtgctcgaggccagcgacgagcccggcatcctcgcgagcgacctgcatgcggatggcaagcacgtcggcattctttgcgtaccgggccacgtctcgggcggcaacgtgctgggcacgccgctgctgcacatggacggccaggccgtgttcaagctggcggtgcgcgtgctcgaagacgcggcccgcgccacgcttgcaaaggcaggcaagaccgaagccgacatcgactggctgattccgcaccaggccaacatccgcatcatggaaggcacggccaagaagctgaagcttccgcgcgagaaactcatcgtgacggtgaacgagcatggcaacacctcggccgcctcgattccgctggctctcgacgaggctgtgcggtccggcaaggtgaagaagggcgaaaccgtcatgctcgaaggcgtgggcggcgggttcacctggggcgcggtgctattgaacctgtagccattgcaacgccctcgcagggcgcggcagtgcgacatgacgcttgaaacaatgaaatcctttgcttttgtctttccgggccagggctcgcaggcggtcggcatgctcgacgcctggggcgaccacccggccgtggccgaaaccctgcgtgaagcctccgaggcgctgggcgaagacgtcgcggcgctgatcaagaacggccccaaggaagaactggcgctcaccaccaacacccagccggtgatgctggtggccggcgttgccgcctggcgcgcatggctggccgaaggtggcgcggccccttccgtcgtcgcgggacattcgctcggcgagtactccgcgctggtggcgtctggtgtgctcaccttggcgcaggccgcgccgctggtgcgttttcgggcgcgggccatgcagcaggccgtgccggtcggggtgggagccatggcggccgtcctcggcatggaagcggccaaggtggtggcgagctgcgcggaagcgaccgcgtccttcggcgccggaagcgcagagatcgtcgaggcggtgaatttcaatgacccgatgcagaccgtgattgcgggcagcaaggcagccgtcgacaaggcctgcgagctggtcaaggccaacggtgccaagcgcgcactgctgctgcccgtgtcggcacccttccattcgagcctgatgaagcccgccgccgaggcgctgcgcgaaaagctgaccacgatcacgctcgctgcgccgcagattccggtgctgaacaacatcgacgtggccgttgaaaccgatcccgaacgcatccgcgacgccctggtgcgccaggcggccgggccggttcgctgggttgaaagcgtgcaagccttgaaactgcgcggtgtagccgccatcatcgagtgcgggccgggcaaagtgctggccggcatggtcaagcgcatcgcccccgaactcgaagccgcgtcggtgtacgacccggcgactctcgcggacacccgacaactgctcgccggctgaacggcgcaaggcctccgatacttttatgagcattcccaaattcgaagggcaagtcgccctggtcaccggcgcgtcacgcggcatcggcgcagcgattgcgctcgaactggcgcaccgcggcctcaaggtggtcggcaccggcaccaccgaagacagcgcagcgaagatcacctcggccctgagcgccttcgacggccgcggccgtgcgctcaacgtgaacgacgccgcagccgtcgaagcgctgatcgacgaaatcgtgcaggcctacggtgccatccacgtgctggtcaacaatgccggcatcacgcgcgacacgctcgccatgcgcatgaaggacgacgactgggatgcggtgctcgacaccaatctcaaggcggtgtttcgcctgtcgcgcgcggtcattcgcccgatgatgaagcagcgctatggccgcatcatcagcatcacgagcgtggtcggcgcctccggcaatgccggccaggccaactacgcagccgccaaggccggcgtcgcgggcatgacccgcgcgctggcccgcgaactcggcagccgcaacatcacggtcaactgcgtcgcgccgggcttcatcgagaccgatatgaccgccagcctgccggaagcccagcaacaggcgctgctccagcagatcccgctgggccacctgggcaagccggcagacatcgcgcatgccgtgtcgtatcttgcatcgccccaggcgtcttacgtgacggggcaggaactgcacgtcaacggcggcatgcacatgtaattgccgcaaggcgcaaactttccccgtaccgggtgcacggcaaatgccacaatgcgcccggctaaaatccaccgattacctacaaccctcagagggaaccaaatgagcgatatcgaagcacgtgtcaagaaaatcatcgccgagcaactcggcgtggaagagtcccaagtaacgaacgaaaaggctttcgtggccgacctcggtgcggactcgctcgacacggtcgaactggtgatggcactcgaagacgagttcggcatcgagattcccgatgaagacgccgagaagatcaccacggtgcaaaacgccgtcgactacgccaccaagaatcaaaaggcctgatcgggccagctggaactgccacggccggccgcgctcttcatcgagcccgtacgcgccgcctgcagttgttcagcgcttccagaaaggtttgccggcatgaccaaacgccgcgtcgtcgtgaccggactcggttgcatcgctcctgtcggaaacaccgcaaccgaatcctgggccaacctgttggccgggaagtcgggcattgcgaacatcaccgcgttcgatgcaagcgccttcgcctgcaagttcgctggtgaggtgaagggtttcgacatcacccaatacatctcggagaaggaagcgcgccacatggaccgcttcattcatctggggcttgccgccgccatgcaggcggtgcaggacagcggactgccgaccggcgaagcgctgccctatgaagaagccgtgcgcatcggctgcaacatcggctccggcatcggcggcctgccgatgatcgaagaaacgcacggcgaatacgcgagccgcggcccgcgccgcatttcgccgttcttcgtgccggcttccatcatcaacatgatctcgggccacgtctcgatcaagtacggcttcaagggcccgaacatcgcggtcgtgaccgcctgtaccacgggcctgcatgccatcggcacgtcggcacgcatgatcgagtacggcgatgccgacgtcatgatcgcgggcggcgccgagtcgaccatttctccgctcggcatcggcggcttcaccgcgccgcgtgcactcagcacgcgcaacgacgatcccgccacggcctcgcgtccgtgggacaaggaccgcgacggcttcgtgctgggcgagggcgccggcgtgctggtgctcgaagaatacgagcacgccaaggcgcgcggtgccaagatctacgcggaagtggcgggcttcggcctgaccggcgacgcgtaccacatgaccgcacccgacgtcgacggcccccgccgctcgatggccatggcgctggccaatgcgggcgtcaacgccgacgaagtgcagtacctcaatgcacacggcacctcgacgcagatcggcgacgtcaacgagaccaatgcggtcaagaaggcctttggcgaccatgcgaagaagctggttgtgaattcgaccaagtcgatgaccggccacttgctgggcggcgccggtggcatcgagtcggtgttcacggtgctcgcactgcatcaccagaagagcccgccgaccatcaacatcttcaaccaggatccggagtgcgacctcgactactgcgccaacgtggcgcgcgatctcaagatcgatgtcgcggtcaagaacaacttcggcttcggcggcaccaacggcacgctggtgttcaagcgcgcttgagcattgctctttcatgcacagcgcaccgtcggtgacatacccggtggggcgctcgcgcggtgccacccggattctgatcgccacatgggccttgggcgcagcgtgcgcgggactgtcgtgctatctgttcgatagtgccggctggcgccagctgctgctggtcctgagtgtgctgttgtcgggcctcgcggccggactcgggctgcgaagcgacggtgcgggggtgctgcacttcgacggactgggctggacgctcacgggcgcccatccgggccgtgccgtccatgcggcccgcgccgccgtcgcactcgatctccagtcgctgctgctggtccggctgacccagccgggccgtgcgagccgctggatctggatcgagcagcgcgccatgccggaacgctggcgcgacctgcgccgtgcggtatattcgcgcgccccgaccgcgtcgcctgccggcgagccttggcgagcaaccgctcctgccgatgcgccctgaacctcctcgatgaccacttctccgccgccagtgccaccggactccggcttgcccgatgtgtccgccgaggcgccgcgccccggtgaagtcgacctgcagctggtccagcgcacggtcgcgggtgaccagaaggcattcgaactgctggtcatcaagtaccagcgccggatcgagcgcctgatcgggcgcatggtgcgcgatgtcgacctggtcgaagacatcgcgcaggaaacattcattcgcgcctaccgcgcgctccatcagttccgcggcgacgcgcagttctacacctggctttaccggatcgcggtgaacaccgccaagaaggcgctggtcgacatgaagcgcgacccgaccatttccgaaagcgccatgcggccgtcttctgaagaggacgatgaaacttaccggcccggaaacgaaccaatcagcgacgaaacccccgaatcggtcttggcggcaaatgaaattgcccgcgtggtcgaggcggccatggaagcgctgccgtccgagttgcgccaggctgtcaccctgcgcgagatcgagggcatgagttacgaagagattgccgaggtcatgaattgcccaatcggcaccgtgcgctcgcgtattttccgggcgcgcgaggccatttcggccagggtcaaaccgctgctggacaaccagtccggcaagcgttggtaggtaagcaggtgaatgaaatgaatcagacaatgacggttcgtgagcaggtgtccgcactggcggatggtcatttgcagggcgaggacttcgcgcgggccatcgaggctgtctgtgcggacgacgaggcccatcgggcttggcgtgcctatcacatggtgggcgacgtgttgcgcgcgggtgcgcattcgccgtgcagcgatagcaatgcgttcctggcccgctttcaacaacgcctggcggcggagcccgccgcagccgccccggttgtggcgcccgccccagcagcagttcacgcggtgcggcacaaagccgacgcggccaatgagccggtctttcgctggaagctcgtggccggcgccgcttcgctggtggccgtggctgcgatcagctggacgctggtcggaaacggcgccgccgttccgtcgcagggtgcacagatggcagtccagcagcaaccggcagccaactcggtgctggccgccgctgccactggcaaccagcagcccgccgctgcgccgctgacgccgacccgcgtggtggtcggcaatggaagcccgcaggtcatgctgcgcgatccgcggctcgaccagttgctcgaagcgcaccagcaagccggcggcgcctcgcaaatgccctcaggtttcctgcgcaacgcgaccttcgaaggcccgacgcgctgacgcgcgcctgccgtccttccaatgaccgttcagatgccgatttctgcacgcgcgttcgcgctggtattcgctgctttttgtctggtgcagatcgcggcggcgcagacccggccgggttcggccaacgccaggagcccggcctcggtgcagggcggcgatgcgccgcccgcgatgggcgtggtcgagtggctgcagcgcatgcacacgggcgcgcggcagcgaaactacgtcggcaccttcgtggtatcggcggcgggcggcgatctgtcgagcgcacgcatctggcatgtacgcgacggcgatatgcagatcgaacgcatcgaggccctgtcgggcccgccgcgctccacgttcaggcgcaaccaccacgtgatgaccttcctgcccgaggcgaaggtcgtgaaggtcgagaagcgcgagaacctcgatctctttcccaatctccccgacaagcccgattcgtcgatcggcgacttttacgatgtccgtgccattggcaaggaccgcgtagccggtttcgatgccgacgtggtgcagctggtgccgcatgacgggcttcgcttcggatatcgcatctggagcgagcgccgctccggcctggtgataaagctgcagacgatcgacggcgactctcgcgtggtcgagcagtcggcgttttccgagctgcagctcgatgcaccggtcaaggcgcaggcactcgcgcagatgatggccaataccggcggctatcgcatcgagaagctggaactggagcgcaccagcgcgcaggacgagggctgggtgctcaagtcgcccgtggccggtttcaagccgcgcagcttctaccgccgcccggctggcagcgacaagagcgggcaggatcgaaccgttcagtggaccttttccgatggccttgcctcggtgtcgcttttcatcgagcgatacgatgagaaacgcgcgccccgggacggcgtgctcacaatcggtgcaaccaacgccattcgtcggcgattgcccgagccggcgaacgattggtggctcaccgccgtgggcgaggtgccgcagcagacgctgaacgcatttgcgcaaagcctcgcgcgcacgcgctgatcggccagtctgcgcgcagctgcgctgaaccaactccgcaccaccgactcatagctcttcttttggccgctctgcacttttgaaagaaaaccgatgatgttcaaagtcgagggacacaagcttcgttcctatctcttcgcattcggcgtggcctgcgcggctgccacgggtttcctgccggcaacgcccgccatggcgcagacgccgcaagcgcgcggattgcccgatttcgccgatctggtggagcaggtcggccccgcggtggtcggtattcgcaccgtcgagaaggtttccgcgcgcagcggcagcggcggcggggaaatggacgaggagatgcaggagttcttccgccgcttcttcggccagccgctgcccggcaatccgcgtccgggcccgcgcccgaaccgcccgcagcagccgcaggaggaagagcgtccgcgcggcgtgggctcgggtttcatcctgaccgccgacggctacgtcatgaccaatgctcacgtgatcgaggatgcctccgaaatcctcgtcacgctgaccgacaagcgcgagttcaaggccaagctgatcggcgccgacaagcgcagcgacgtcgccgtggtgaagatcgaggcgtccagcctgccggtggtgaaggtcggcgacatctcgaagctgcgtgtcggcgaatgggtgatggcgatcgggtcgcccttcggcctcgagaacaccgtgaccgcgggcatcgtgagcgcgaagcagcgcgacaccggcgacctggtgccgctgatccagaccgacgttgcaatcaatcccggcaactcgggcggtccgctgatcaacctgcgcggcgaagtggtcggcatcaacagccagatctattcgcgctcgggcggctacatgggcatctcgttctcgatcccgatcgatgaagcgatccgtgtcagcgagcagctgcgtgccaccgggcgcgtgtcgcgcggcctcattggcgtgaccatcggtacggtctccaaggacgtggccgagtcgatcggcctgggcaaggcccgcggcgcgctcgtgaacagcgtggtgccgggttctgcggccgacaaggccggcgtgaaggaaggcgacatcatcaccaagtacggcgacaaggcgatcgagacaccgagcgacctgtcgcgctcggtggccagcaccaagcccggcgccaagagcacgctgaccctgttccgcaacggcgcttcgcgcgaacttgcgatcaccgtggccgagggcgatcccgaagccaagccgtccggcaagcgccagcaggatcgcgaggagccccaggccaagccgtcgtccgcggccagcaagtcgctcggcctggtggttggcgacctcaccgacgcccagaagaaggaactcaaggtgcgcggcgtgcgcatcgaggcagccaccgaagcggccgccaaggccgggttgcgcgagggcgacgtgattctttcggtcggcaacatcgaagtctcgagcgtcaaggagttcgagtccgcgattgccaaggccgacaagaacaagccgctcagcgtgctgttccgccgcggcgagtgggcgcaatatgccctgatccgacccgcacgctgatctggcgctgccgtcaagtggccccacccgtcagtcgggtttggggcctttttttgaggtgtttgcgacgccggagcgcccggtttcaaaaaaatttctggacccaaagtgcgccggttttgtttgtgctcactaacttattgcgaggcttaggacggttttcggtagaatagcgttcattgggcgctgagtccgtgcataaggaggggggtttcctccaccatgcgagatgtcagacagcagtccaccgatgctccacagatcgcccacaagttgttcatagagtgctccaccgatcctgtggataagttgtttatatctttgatgttgtggacctgcaacggcccgtttcgaccctgtccccggatgtacgtgcctccctttttgcctacaatgaagttccaactactgcagttgccattgcttgttggttcagggcgcgtctccagaagacgcgcccttttttcttgcctgtcgcactctgcgcacgagccaattcaagtacttaagcgttcccgttgatgaatcacatcagaaatttttcgatcattgcgcacatcgatcacggcaaatcgacgctcgcagaccgtttgatccagcgttgcggcggcctcgcagaacgcgagatggaagcgcaggtgctcgactcgatggacatcgaaaaagagcgtgggataaccatcaaggcacagaccgctgcgctgcactacaaggcgctcgatggacaggtctacaacctcaatctgatcgacacgccgggccacgtcgacttctcttatgaagtgagccgctcgttgtcggcatgcgaaggcgcgctgctcgtcgtcgatgcatcgcaaggcgtcgaagcgcagacggtggccaactgctacaccgcactcgacctcggcgttgaagtggtgcccgtgctcaacaagatggatttgccgaatgcggatcccgacaacgcgcgcaccgaaatcgaagacgtgatcggcatcgacgcgaccgacgcgattccgtgttccgccaagacgggcatgggcattgacgagatcctcgaagccgtcgttcacaagatgcctgcgccgcgcggcaatcccgacggcccgctgcgcgcgatgatcgtcgacagctggttcgacgcctacgtcggcgtggtgatgctggtgcgcgtggtcgacgggcggctggtgaagggcgagcgcatcaagatgatggcgtccggcgccatgtacaacgcagacaacgttggtgtcttcacgcccgccaacgaaccgcgtgcgtcgctcgaggcgggcgaggtgggctacatcatcgcgggcatcaaggagctgcaggctgccaaggtcggcgacaccgtgacgctgatcaagccgggcacgggcggcgcggccgccaccgccacggaagcgctgccgggcttcaaggaaatccagccgcaggtgtttgccggcctctacccgaccgaagcgagcgagtacgactcgctgcgcgacgcgctcgaaaagctcaagctcaacgattcgtcgctgcgctacgagcccgaggtgagccaggcgctcggcttcggctttcgctgcggctttctcggcctcttgcacatggagatcgtgcaggagcgcctggaacgcgagttcgaccaggacctgatcacgaccgcgccgagcgtggtctaccaggtggtgcgcaacgacggcgaagtcatcatggtcgaaaacccgtccaagatgcccgacgtcggcaagatgagcgagattcgcgagccgatcgtgactgtgcacctctacatgccgcaggaatacgtcggcgccgtcatgacgctggccaatcaaaagcgcggcgtgcagatgaacatggcctaccacggccgccaggtcatgctgacctacgagatgccgctcggcgagatcgtgctcgacttcttcgacaagctgaaatcggtcagccgcggctacgcctccatggactacgagttcaaggagtaccgcgcgtccgacgtggtcaaggtcgacatcctgctgaacggcgagaaggtcgatgcgctctccatcatcgtgcaccgcagccagtcgcagtaccgcggccgggccgtggtgtcgaagatgcgcgagatcatttcgcgccagatgttcgacgttgcgatccaggcggccatcggggtcaacatcatcgcgcgtgagacaatcaaagcgctgcgcaagaacgttcttgccaagtgctacggcggcgacatcacccgcaagaagaagctgctcgagaagcagaaagcgggcaagaaaagaatgaagcagatcggctcggtcgaggtcccgcaagaggccttcctcgcgattctgcaagtcgaagactgatctcaaaaatggcattcatcactactttggtcctcgcggcctttgccggctacgtcggtgcctggtactttggcgccatcgaaggcaacttcgcactgctgctgttcctggccaccgtggtcaccgggctctactggctggccgagcgcttctacttccagccccgccgcgagcgcgccgccgccgcactcgaaacgtcgctcagcgaacgcaacgcgcgcctggccggccagggcatcacgcaggtcgacacggccgatgccaaggccagcgaccgcctgctcatgcagccgtggtggctcgactggacggccgggctgttcccggtcatcctggtggtgttcctgctgcgctcgttcctctatgagcccttcaagattccgtcgggttcgatgatgccgacgctgctcaccggcgacctgatcctggtcaacaagttcacctacggcctgcgcctgccggtcatcaacaccaagatcaccgacggcacgccgctggcgcgcggcgacgtggtggtgttccgctacccgcccaagccgagcatggactacatcaagcgcgtggtcggcattcccggcgacgaggtggcctacctgaacaagaagctcaccatcaacgggcagccggtctccaagtcctcgatgcccgactacctcgacagtgattcgatgcgcctgctcaagcagttcaacgaagacctcggcggcaagcagcacaggctgctcaacgacgatgccggcccggccttcgttcagggcgccgccgactttccgtttcgcgaaaactgccgctactccgtcgaaggcgtggtttgcaaggtgcccgccggcaattacttcatgatgggcgacaaccgcgataattcggcggactcgcgtttctggggtttcgtgccggacaagaacatcgtaggcagggcgttcttcgtctggatgaacttcggcgacctgggtcgcatcggtccattccaataagcagtcagcattgttcgaggggtaagagggcatgagagctaatcggtccatccgcagcagggccgcgcaccagcgcggcatctcgttcatcggcctggtgtttgtcgccgcggtgctgggttgcctgggcgtcgtcgtcgcgcaggtcatcccgacactgatcgaataccaggcgatcgacaaggccgccaacaaggccaaggaaggcaccaccgtgcccgaagtgcgcgccatcttcgatcgggcgcaggccatcgacgacttcaagtcggtctccggcaaggatctcgacatcaagaaggtcggcgacaaggtcgtcgtgtcgtatgcctacgagcgggagattcccctgttcggcccggcctttctggtgctcaagtacaaaggcgagacccgctgaacgcggcgacacgcaaggtggacggcggcctcgcggcgctgcaggagcgcctcaagcattcgttctccgacgcgcggctgcttcagctcgcgctcacgcaccgcagtttttcggctgaccacaacgagcgcctcgagtttctcggcgactcagtgctcaatctcgcggtttcgcacttgctctacacccgcctctcggccctgcccgaaggcgacctgtcgcgcgtgcgagccaacctggtcaagcaggacaccctgcatcgcctggcgctggaacttcagctgtcgccgctgctgcggctcggcgagggcgaggcgcgctcgggcgggcccaaccggccttcgatcctggccgatgcgctcgaagcgctgatcggcgcggtctatctcgacgcgggctttgcggccgcggaggcgctggtgcgccggctctacgagtcggtcgagatcaatccgcgcatggatgcggtcgccaaggacccgaagaccgaattgcaggaatggctccagggccacaaaatgaagttgccggtgtatcgcgtggcggccacgctcggtgccgcgcacaaacagactttcgatgtcgagtgcgaggtgcccgagctgggcctgcgcgaacgcggcatcggtggctcgcgacgcgccggcgagcaggctgccgcggcagccatgttgatccggctcaaggcacgcggagccgcgtgaaaccagaaatgaacgacgctataaattcagcagcaaacccggaagacgcagcgggcgatacgggcacgaccgggccccagcactgcggcctggtggccatcgtcggcaagcccaacgtgggcaagtcgacgctgctcaacgcgctggtgggccagaagatcagcatcacctcgcgcaaggcgcagaccacgcggcatcgcatcacgggcatgcgcaccatcggcgcgacgcagttcgtgttcgtcgatacgccgggtttccagaccctgcatgccaacgcgctgaacaagtcgctcaacaagaccgtgcagggcgcggtcggcgacgtggacctgattcttttcgtggtcgaggcgggcagcttcacgccggccgacgagcgggtgctcaagctgctcggtaagggcattccgaccgtgctgctggccaacaagctcgacaacgtgcaccgccgtggcgacatcgcgccctggctgcagaccatgcaggcgaagcaccccttcgccgagttcgtgccgatgtcggccaagaaccccaaggacgtcgagcgcctgttcggcatctgcgaaaaatacctgcccgagcagccctggttctatgccgaggacgagctcaccgaccgcagcgagaaatttctggccggcgaactggtgcgcgaaaagctgttccgcctgaccggcgacgaactgccctatacctcgaccgtcatcatcgacaagttcgaggaagagccgccgcagaaaaagggccagaagcgcctgctgcgcattgcggccaccatcgtggtcgagcgcgacggccacaaggccatggtgatcggcgacaagggcgagcgcatcaagcgcatcggcatggaaacccgcgtcgaactcgaaaagctggccgacgccaaggtttttctcgagctgtgggtgaaggtgcgctccggctgggccgacgacgaggcccgcgtgcgctcgttcggttacgaataagcaggcaaacccccaggcttgctcgcttcgcgtagcctccaacccccttgcagggggcaacgccagcggctcggtaaagccggttccgcggcgtttgctggcctcaagcctcgatgctccttagcgtactgacatggccatccatcgcgtttcgcacgaaccggcgtatgtgctccatcgctacgactggagcgaatcgagcctgattctcgaggtcttcacccggcaccacgggcgcatcgcgctggtggccaagggggcgaagcggccgagttccaatttcaggccggtgctgctgccgctgcagccgctgcaactcaactacggcggcgatgccgagatccgcacgctcaagggcgccgagtggatgggcggccacgtcatgccgaccggcgaggcgctgctctcaggctattacgtcaacgaactgctgctgcgccttctggcgcgggacgatgcgcatgaagccctgttcgatgcctatgcgggcgtggtgcaggtgctggccagcgaacacgccggcgcgcaggcggccacccacgccgccgcgctgcgcgccttcgagctgctgctgctgcgcgaagtgggccttttgccgtcgctcgacgtgcagaccctcacgctcgagccgctggcggccgacgcccgctacagcctggtgccggaagccggcttgcggctggcgggtgaggacgaggccgcgctggcgggcgcagactggcagtcgctgcagggcgtgctggacgaccgcgcgcctttcaccgccacactgcgcgagatcgcgaccatgaacgccggcagcaacagtgccctcaggaaccagctgcgcaccttgctcaactaccattgcggtgtgtccacgctgcgcacgcggcagatgatgagagatttgcaagccctatgagcacaacatccggccattccgccaccacctcgctgtcggtcaatctgaacaaggtggccctggtgcgcaacacgcgcgccctcggcattccgagcgtgcttgtcgccgccaacgcctgcctcgctgccggggcgcaaggcatcaccgtgcatccgcggccggacgcgcgccatatccgcgcgcacgacgtgagcgacctgtccatgctgctggccagggactggccggcgatcgaattcaacatcgaaggcaatccgttccacaacctgatggacttcgtgcgcgagctgaagccgcaccaggccaccttcgtgcccgacagcgagacccagtcgaccagcgaccacggctggagcttccccgaagacgccgagcgcctgcgccccctgattgccgaggccaaggccctgggcgtgcgcgtgagcctgttcatggaccccattccggaaatgatggctgcggccaaggaagtgggcgcggaccgcgtcgagctgtacaccgagggctatgccgcatcgcgcggcacgccgaacgagcaggccgtgctcgcgcgctatgtcgaatcggcgcgtgcggcagaggccgtgggccttggcgtgaatgcaggccacgacctgagccgcgacaacctcggcgcattcctgcgtgccgtgcgcggcgtccgggaagtctcgatcggccatgccttcattgccgatgcgcttgaactcggctacgccgccacgacgcgggagtatctgcgctgcatcgaagaggcgcagtgaacgcgcaagcggaatgatctacggcatcggtaccgacatctgcgacctccggcgtattgccgcgacgttcgagcggcagggcgagcgttttgcccagcgggtgttgagcgacgccgaattcgccgtttggaaggcccgcagcgagcgctggcccaagcgcggcctgagctatcttgcgacgcgtttctccgccaaggaggccttcagcaaggccatcggcctgggcatgcgcatgccgatgagttggcggctctgcgagatcgccaacctgcgcagcggcaagcccgtcatcgtgctgcacggcgagctgaaagagtggttcgaggccaagggcctcacggcacacgtcacggtgaccgacgaaaccgaatatgccgcgagtttcgtggtggtcgaatacaagaacgaggcatgaccctggcaacgacaagcattcacgcgccattgatcatcgacgtggcgggtccggaactcggcgatgcggatcgccgccgcatcgccaaccccctggtcgggggggtgatccatttcgcccgcaactggcaggaccgcgcccagatgacggcgctcaatgctgagctgaaggccatccgccccgacctgctgatctgtgtcgaccacgaaggcggtcgcgtgcagcggtttcgcaccgacggcttcacgcgcttgccctcgatgcgcgcactgggcgagttgtggatgcgcgacgccatgcgcgccacgcaggctgcgacggcgactggccaggtgcttgccgccgagctgcgcgcctgcggcatcgacttcagttttgcaccggtgctcgacctcgactacggcggcagcagcgtgatcggagaccgcagcttccaccgcgacccgcgcgtggtggcgctgcttgccaagagcgtgatgcacggcatgctgcagatgggcatgcgccattgcggcaagcactttcccgggcatggcttcgtgaccgccgattcgcacgtggaaattccggtcgaccggcgcagcctcaaggccatcctcgccgacgatgcgcagccttacgactggctcgcgggcacgctcacggcggtgatgccggcacacgtgatctatccgaaagtcgacaagcggcccgcgggtttttcgcccaggtggttgaaagagatcctgcgcagccggctttcattcgacggcgcgatcttcagcgacgacctgagcatggaagcggggcgctacatcgatggcgaactgctgagctatgccgatgccgccctggccgcgctcgacgcgggctgcgacctcgcgatgctgtgcaaccagagcatcggcgatggacggccgctggacgaactgctcgacggcgttgccggggcagccagggcagggcgctggcaacctgacgcagcaagcgagatccggcggcgggcactgctgccggaagcgccgtcggctcgctggagcgagctcgtcgaatccgcagggtacaaaggcgcacggcaagtgctggcgaaggccaagctcgcgccggcgcacggcagcgtctgaccacttgctagggcgcgctccccggcgccgcagcgttcggcagcgggttcgtccacagccgctcgccacccgaatccaggtgcgtcaggtacagccgcacgtcgaactccagccggtggtagctcggctccatgtgctcgcacagcgcataaaagctcttgtcatgatcccgctccttcatgtgcgccagttcatggaccacgatcatgcgcagccactccaacggcacctccctgaacaggctcgccacccggatttcgcgcttggccttgagcttgctgccctgcacgcgcgagacggtggtgtgcgtacccagcgcattgcggatcacatgcagcttgctgtcgaatgccaccttggacagcggtggcgccttgcgcatgaaatcgctcttgagttcgctcacgtagtcgtagagcgcgcggtccgtctgcacctcgtgcacggcgccgggatagcggctctgcagcaagggtgcgagtccttcggtcgcgaccagctgctgaacctgcgccagcaaggcgggtggatagcccgcgaggtatttcatgcaaccggcctcgcgcaggccagcccggtggccacgcccccgaacaggtcgccttcgacgaggttgacgcccgcgaagctcctgcgcaaggcctgctgaaacggccgcagcgccgaggagccgcccgtcaggtagatggcgtcgaggtcgccgctgcgcagcccggcgcgtttgacgcaggcgtgcgcgcaggcaatcacgttctcgagcagcggagaaagctgctgcgccatgtcggcgggcgagagcgacgcggccaggcccggctctgcacacgaaaggtcgatggcggtgggcgcatcgctcaccgaggcttcgatcttcgcctgctcgacctcgctggcaatgcgatggccgtgccgctcttcgagcaccgccatcagccggtcgtgcagccgcgtgtcgctgtagctcgtgcgcagatccttggcctgccgcaccgccttggcggcatagagccagttgatcaggtgccaggacgagagctcgaagaagaccttgctcggcacttcgcgcccctgtgcgcccgtgtgccgaaagccgaattccggcatgacgcgatcgaggttcaggcgctggtcgaagtcggtcccgccgatgtgcacgccgctggtggccagcacgtcgtcgctgcggtcttcgcgcgcggcgcggtccgggccgacgcgcacgacggtgaagtcggaggtgccgcccccgacgtcgacgatcagcaccagcgattccttcgtgatgcgctgctcatagtcgaaggccgcggcaatcggctccagctgaaaagcgatgtcgcgaaacccggccgcgcgcgccgcgtggcgcaggctctcttccgcgcgctcgtcgcgcttggaatcgtcatccacgaaatgaaccggccggccgatgaccacgcgctccggcacccggcccagctcgcggcccgcccgtgcggcgagttcgcgcagaaatcgcgcgatgatgtcctcgaagctcacgagcccgtcgtagacggccgttttctcctgcatcagcgcgctgccgagcaggctcttcagggagcgcatcaggcggccttcgacgcctgaaagatagagcgcaatggcctcgcggccgaagtgcgtggtacggtcttcggcgttgaagaagatcgcggtgggcagggtggtggccgagccctcgatgggcagcagacgggccacgccgtcgacccggcaggccacggcggaattggaggtgccgaagtcgatgccgatcgtcggcagcgacgacggtagatgcacgctcaagattccctgcgaagcgccgggaacaggatcacgtcgcgaatgcttggcgaatccgtcagcagcatcatcagccggtcgatgccgatgccgcagccgccggtgggcggcatgccgtattcgagcgcacgcacgaagtcgtggtcgtagaacatggcttcgtcgtcgccgctgtccttggcggccacttgcgcgttgaagcgcgcggcctggtcctcggcgtcgttcaactcgctgaagccgttgccgaactcgcggcccgtgatgtagagctcgaagcgctcggtcacttccgggcgttcgtcgttggcgcgcgccagtggcgaaatctcggtcgggtgctccatgatgaaggtcggctgccagagcttctcttccaccgtctcttcgaaatacatcacctgcaggctcgcaaggctgcgctgcgagagcttgtctttttcttcgctgaggccgatcttgcgcagcgcattgatgagccaggcgctgtcgtcgacgccatcgccggcctcggtgtgcttgaggatggcttcgcggatcgtcaggcgctcgaagggctgggtcaggtcgaccggcttgccctggtaggtgagctgctgcgtgcccacggccttgtcggcaatggtgcggatcagcgtctcggtgaagtccatcaggtcgcggtagttccagtaggccgcgtagaactccatcatcgtgaactcggggttgtgccgcaccgagatgccctcgttgcggtagctccggttgatttcgaacacgcgctcgaagccgccgacgatcagccgcttgaggtagagctcgggcgcgatgcgcaggaacatctcctggtcgagcgcgttgtgatgcgtcttgaagggcttggcgttggcaccgcccggaatcgggtgcagcatcggcgtctcgacttcgaggaagtcgttggacaccatgaaattgcgcagggcgctcacggccttgctgcgcgcggtgaagcgcacgcgcgccgcttcatcggtgatcaggtcgacgtagcgctggcggtacttctgctcctggtcggccatgccatagaagtcaccaggcagtgggcgcagactcttggtgagcaggcgcagcctggtcaccttgactgacagttcgccggtcttggtcttcatcagcgtgccttcggcgccgaggatgtcaccgaggtcccagcgcttgaattcggcgtaggtatcctcgccgaccgcgtcgcgcgtgacgtagagctgaatgcgaccggtggcgtcctgcagggtcgcgaagctggccttgcccatcacgcgcttgagcatcatgcggcccgccacgctcacggaaacggcctgcgcttcgagtgcatcggcttcggtggcgccatgcgcctcgaccagtgcggcggcgcggtgacccggcttgaagtcgttcgggaacgcaacgcctttgccctcggcctgcgcggtgcgcagcagcttgagcttttcgcgtcgttcggcgatgagcttgttgtcgtcgacggcgggcgccgcggctggagccgcagcgggcgtgggaatggaaggaatcaggtgatcggacatggagagcggatgggcgcatcgggagcgtgcgcaacccgccattttagccgatcgggttcgaatgaaaccggcctccagcgcccgccaatcctgtatgaaatgctattgaaaaagtagcaacctattcagtgatgcccgcgcgtgcgagcagatcgctgaccaattcgagccgcatcagcgggctgtcgagctccatcagccgttgccggagttcgagttgcatgggcaccagttcgcaccagcggttggccacccagccgcaatcgtcgaaccgatagggctcgccgacgggcaggcgcacgctttcggcaccctgggcgcggcggcgttcttcaagggcgtcgaccaggcgccgcagcgccgtggcggtgtgcaggaggtcgcccgggatctcgatggccgcatcctcgagcacagcctccacctcggccacccaaagaccgtatttctgaagttcggcgctgcgaatccgaaagcgctgcgtgccgacgcattcgatctgcagcaggccgctttggggcgaatcgaattcgcggatgacggccagcgtgccgacggcggcgaagctttccgcatcggcgcctgccttgcgcacctcgctgccgctcgtgaggctgacgacgccgaaaggcgcattggccttgcggcatttgccgatcatgtcgagataacgtacctcgaaaatacgcagtggaagcacgccgtccgggaacaggaccgtgccgagcgggaacaatggcagtgaatgaagaaggggctgtgtcgtcatcgaagaaccttgcatggctatcatcgcattccgctcacgaccgcgccccatgctctatcagatcccctcgttccttctcgacgtgatcgtcggcctgctcggcggcgcctgcctgctgcgcctctacatgcagtaccaccgtgtgccgttcggcaatccgctcggccgcttcgtgtttgcaattaccgactggatcgtgctgccgctgcgccgcatcgtgcccgcggtcaagcgctgggacctggcgagcctgattgccgcatggctgctggtgctcgcgaagttcctgttgctgtggctgctgatgggcaacctggggcgtatcgcggccttgccgctggtctccctggtggggctgctgcagctggcggtttcaggcctgaccgcgctgctggtggtctatgccgtgctgtcgtggataccgggtgcgtcgccgatgctgctcgacctgatctcccggctggccgaaccgctggtgcggccgtttcggcgcttcattccgctgatcggcggcgtggacctgtcgcccctggccgccatcgtggtgctgcaggtgattgcgatcgtgctgggcaacctgctggtctgggcttatcgactcggcgcttgaacccagcgccgactggggcttgttcgcgcaagggcgctctgattcgagaaacaccgcggaaccggcttcgccgggccgcaggtgttgcccccggtagggggagggcgaagcggacacgaagtgccgcgcagcctgggggcgagcctagctcaccgcgtcggcgggctggcgcagcagcatcgccagcgtgctcgcaatggtcttgcgcagttcgcggcggtcgctgatgaagtcgatcgcgcccttggtctgcaggaattcggcgcgctggaagccttcgggcagcgtcacgcgcacggtcgactcgatcacgcgcgggccggcaaagccgatcagcgccttgggctcggcaatgaccacgtcgcccacgaaggcgaagccggccgagacgccgcccatggtcgggtcggtcagcacgctgatgtagggcaggccctttttcgcgaggcgcgtgagcgcggcattggtcttggccatctgcatcagcgagagcaggccttcctgcatgcgcgcaccgcccgtggcggtgaagcagatgaacggcaccttctgctcgatggccgtctcgacgccgcgcacgaagcgctcgccgaccacgctgcccatgctgccgcccatgaactcgaattcgaagcaggccacgaccacgctgatgctgtggaccgagccgcccatgacgatcagcgcgtcggtttcgccggtgttctccagggcttccttgagccgctcggggtacttgcggctgtccttgaacttgagtgcgtccacggggagcacttcctgcccgacctcgtagcggccttcggcatcgaggaaggcgtcgagccgcgcacgtgcaccgatgcggtgatggtggttgcagctcgggcagacgttctggttgtgctcgagatcggtcttgtagagaacggtctcgcaggcggggcatttgatccacaggccctcgggcacctggcggcgctccgacgggtcggtttgtgcgatcttggcgggtagcagtttttcaagccagctcataggactccggatttagctcccctctcccgcatgcggaagaggggcttgggggtgaggggcacccgcgattatcggccagccgcgttcttgggggtagcggccggcagcgcatcgagcgcctcgcggattccggcgaggaattcgcgcacggcgggcacgaccttttcgcgcggctgtccgtcgatcagctggatgatcttcgtcccgatcacgaccgcatcggcggccgaacccacggcctgcgccgtgcgcgcgtcgcggataccgaagcccacgcccacggggatgttcacgtgctcgcggatgcgcgggatcatctggccgaccgcctcggtgtcgaggtggccggcgcccgtcacgcccttgagcgaaacgtagtagacataaccgctcgcgatgcgcgcgacctgcgccatgcgctcgctggtgctggtgggcgccaggaggaagatcaggtcgatgttcgcggccttgagctcggcggcaaagccttcgcattcctcgggcgggtagtcgaccaccaggaggccatccacacccgccgccgacgcgtcgcgaatgaaggccttcttgccatgcacgaggtcatagcgctcgaccggattcgcataacccatcagcaccaccggcgtggccgtgtcctgctggcgaaacgcggccaccatggtgagcacctgcttcatgccgatgcccatggccagcgcgtcttcgccggccttctggatcaccggcccgtcggccatggggtcggaaaacggcacgccgagctcgatcacgtcggcgcccgccgcgaccatgccgtgcatcagctcgggcgtgatgtccgcgtaggggaatcctgcggtcacgtaaggaatgagggcgcggcggccgtctcttttcagcgcgtcgaaggttgcagcaatgcggctcatcacttgcctcccttcacgctcagcccgcgcatcgagggccggtcgtagaagtcgacgcccgacaggtcggccacggtgccgatgtccttgtcgccgcggcccgagaggtttaccagaatcgactggtccggccgcatggtctttgcgagtttcatggcataggccacggcgtggctcgattcgagggccggaatgatgccttcggtgcggcacaggtagtgaaaggcttcgagcgcctcggtatcggtgatgcccacgtactcggcccggccgatgtcggccaggtaggcatgctcggggcccacgcccgggtagtcgaggcccgcgctgatgctgtgggtctcggtgatctggccgtcttcggtctgcagcaggtaggtgcggttgccatgcaacacgcccgggctgccgcgcaggatcgaggccgcgtgcttgccgctgtcgagcccttcgcccgccgcttcgacgcccaccaggcgggtgcccgcgaacggaatgtaggggtggaagatgcccatggcattgctgccgccgcccacgcaggccaccaccacgtccggctgccggccttcggcctcgccggtgatgccttgggccgcgagcatggcgggcatctggtcgatgcactcggtgccgatcacgctctgaaagtcgcgcaccatcgtcggataggggtgcgggccggccacggtgccgatgatgtagaaggtgttttccacgttcgtcacccagtcgcgcatcgcctcgttgagtgcgtccttcagcgtcttgctgcccgattcgaccggcaccacggtggcgccgagcaggttcatgcgatagacgttggggctctggcgtttcacgtcctggctgcccatgtagaccacgcattcgaggccgtagcgcgcgcagatggtggcggtggccacgccatgctggccggcgccggtttcggcgatcacgcggggcttgcccatgcggcgcgcgagcatcgcctggccgatcacgttgttgatcttgtgcgcgcccgtgtggttgaggtcttcgcgcttgaggtagatctgcgcgccgcccatttcgcggctggtgcgggccgcgtggtagaccggcgagggccggccgacgaagtgcttcagctcgtaatggaattcggcgagaaacgccggatcgtccttgaacctggcgtaggcgtcacgcagctcattgatggcgtgggtgagcgtttcgctcgcgaaagtgccgccgtagttgccgaaatggccggtggcgtcgggttgctggtagtcctggaattggctttgcatggttctcgatcgttgggccgcagccccaaatcacgatcggggtgcggcggctaactggagaaggacgcgtcggcggctctgaccgctgcgacgaattgccggatttttgcggcgtccttcaggcccttgttcccgggtccgtcgatttcgacgcccgagctcacatcaacggacagcgttttgcagcgcgtccgcaggatgcgaatgccatcgctcacgtttgcaggtgtgagcccaccactcaagacgaggtgagcgtcgacggcgggtggaagaagtgaccaatcgaatgccttgccgccaccgccataaccttcgacatgggcgtcgagcaggatggcctgggcgtgggagtaatcggacgcgtattttacgaggtcgaagcccgctccggcagccccgagcggaatgcgcgcggcgcgcatgtagcgaaaacggcccgggccggtggattcctcgcactgttccggcgtttcttcgccgtgaaactgcgcgatggcgcccttcacgcgagcaagcgatgctatgacttcaagagcatcctcgttgacgaacagcagcaccggggtgataaaagggggcaggcgggacgccagctcggcggcgcgctcggccgtcacggcgcgggggctcgcggggtagagcacgaagcccacggcatcggcgcccgcctcgaccgcggcatccacgtcggcctcacgcgtgaggccacagatcttgatgcgggtgcggggaagcgtcatggcggcccatcataaggagcgccgccggcctgaagcgtggcctccgccggcagaccccacttggcgtcgtacaacggcccgagaaaatacagcccattggcggagaaggtgggcgccgccaccttgcggctgcgggcttcgagcacttcgctgatccattcgggccgctcgtcgccgcgtccgatgcgcacgaggcagcccatcaggttgcggatcatgtggtgcaggaaggcatcggcctcgaattcgaaatgccagcggcagcggtcgcccgcgccgacacgcgtgatctcgatgcggcgcagatccttgaccggcgaacgcgcctggcaggcggaggcgcgaaaggagctgaagtcgtgcttgcccaccagcaaggcggctgcggcgcgcatcgcgtcgccgtccagcgcatgcatcgaccagccgacccgtcccgattcgaggctgggccgtacgggagactgcgacagcacgtagaggtagcggcgcgccaatgcactggcgcggcaatggaattcggccggcaccggctgcgcccactgcaccgcgatgtcgtcgggcaggaaacggttggtgccgcgcatccaggagaagggttcgcgctcgacggtggtgtcgaagtgcaccacctgcatcagcgcgtgcacgcccgcgtcggtgcggccggcgcacagcgtgccgatcggctgtgcggcgaacttggctagcgcggcttccagcttgtcctgcaccgtgcggcccgagcgctggctctgccagccctcgtacgcctggccgttgtagcggatgcctagcgccagcctcacgaattcaaaaagacgggaaaaagccgctcagcgcagctcggcgagcaattgcttcgcctgcgacttgaggtcgccagcgctttcagcctcgacttcttccaccagcgagcgggcgccttcgacgtcgccgatggcttgcagttcgcgcgccagcgacaacttgaccgcatgggggctgtcgtcgccatcgtcgtcctcgggcatggtggccgcgggcctcgtcgcttcggcggtgccggccaccggacgggcgggaaggccagccagtgcgctcatgtcgaactcgataaagcccgaatccgcgggaaggccgccgcgcagcgctgccggacgggtgttgtcatcggcttcgtcgagtcccgcggggcgcgagaccggtgccagggcgccgggcgccgtgtcgaaatcgttctcgagatcgaccgatgcggcgggcgcgtgcgcatggccgttggagaagggggttgctgctgcgggtgctgcatacgctgccttcggcaggctggcgctcaccggggccgggctgggcgcaggcggctggctcaggtccaggtcgaaatccagcggtgcgaccgagggcacgaaagccggagcgggcgccactgcgacgggaggagcgacaggtgcgggggcgggcggaaccgcggcagcgggtctggctgccgaggcaagagcgcctgcaaaggcggcgctttcggcctggctcacgccgcggggcgagcccgattcgtacaacgggttgcccggatcgaggtccttgcccatttcggcgacgcggttccagtcggagccggtgccgttggtcagcttgtgcacctcggttgccaggccctcgaaggcccgcacgtcgcggcgcttggcatggatctcgagcagcttgaggtggatggccgtgcggtcggggctcacgcgcagggcttcgcgaaggatctcctcggcctgcaggtcgcggccataggccaggtacacgtccgcttcggccacggggtcgacatcgcccgcgtcgagctggctcggcgagtacgacagcgacgagacgctggagtcgccgcggtgcttggtgtcgaccgattcgccgccgctggcaccgaagaaagaatccttcgggatgcggctttcgaggaacacgctttcgctcatttcctcgcgccggcggcccagcacgcggtacagcaggaagccgaccagcaatgcgatcagcgccgcgccggcaagcatcagcgggttgtcgagcaaatcttcgaagaagccgcgttccaccggaggcggcggcggtgccgccttgaccaccggcttgggtgccggtgcgggggctgctgctgcggcgcttgctgctgcagcgggagcggccggtgcggcttcggaaggtgcggcagcggcgtcgggcgctgggttggcgggagcagcggctgctgctggtgccgctgccacggccgttgcggccggtgctgcgggagtcgacgtggcggccggtgtcgcggcgggcacgacaggcgcggctggtgccacggtcgcggcaggcgcgggcgctaccggtgcgggcgccgtcgccggcggcgacgtggtggcagccacgcccggattgggtaccgaaatgcccggcgctgcaggcgccggtgccgaacccgctgccggtgccgctgtgccagtggccgccttgagcttggcgagttcgttgatgttcttggaaagctccgccacgcggttgctgctgtcctgggcctggcgggtctgcgcaaccttttcctcggcggcgcgggccgtcgcgccgccttgcgagatcgtcagcttgtcgggcgcgcttgccgccgcattgcggtcttccacgttggcttgcagcttgcccgtggccttgcggctggcggcggccacgttcgaggtgggcgcgttctcggccaggcgctggcggtaggcgccgaaatcgcggctttgcgcggtgatggtgcgtcgcgcttccgacggcaggatggcgccggcttcagcggcgctcggcaggtcgagcacggcgcccgccttcatccgattgatgttgccgccaacgaaggcatcgggattggagagcaacagcgccaccagcatctggtcgagcgagatgtcggcgggcttgtaggcaccggcgatcttgctggcggtatcgccgcgctgcaccgtgacctgctcgccgctgctcgcgggacgagccgttgccgcggcaccgggagcttgcggtgcggccgacgcgggcgccggggctgccgcgggagcggtgaccggtgctgccggtgcaacggccgcacgctcgcggcgtgcacgggctgctgcggcggcgggacgttccaccggggtgctgacctggggcgtggcgggcgcgatcggtgcggccggcgcagcctggcgggtcgcgggcggatcgagcagcacggtgtagtcgcgcaccatgcggccggtcgaaccattggcttcgaccagcaaatcgatgaaggggtcgttgagcggacgggtgccggtcaatcggacgacgtactggccgccggcgcggcgttgcagcgttgccttgacgtcgctcaaggcggcgttgtacggaacgcctgctttcttgaaggcgtccgcgttggcgacgttgatcttcaggctgtccgcgtcggcggcagccatctcggtcacgtcgatctcggcgcgaagcggttcgcccagcgccgattgcaccttcaactgccccagcgcaaaagcgctggcgtcggtgcttgcaatgcccagaaccaccgcaacggctgctcccagaacggaaaggcgaagaccgttcaagggtagggaagggcgagcggccgatgggcgggccgcgggcaacagatgtcttgtcatgctgataggggcggctcaggcccagaaattgtaagaggacgttagcatcatcaccgggtgctgacaaggcggtgcgcccgttctacccagtgcgcgcatacttacgcacacatttaatgttgccataaggcaacactttccggctgggaagagccttggcgccccatcaggcctcaagcaggatgcgcagcatgcggcgcagcggttccgccgcgccccacagcaactggtcgccgatggtgaatgcaccgacgtattcagggcccattgccagcttgcgaatgcggcccacgggaatgtccatggtacccgtcacggccactggcgtcaggtccttgagggtggcttcgcgggtgttcggcaccaccttcgcccatgggttgtcggccgcgatcatggcttcgatgtcggccagcggcacgtccttcttgagcttgaaggtcagcgcctggctgtggcagcgcatggcgccaacgcgcacgcagaagccgtcgaccggcaccgcggcgccgccgaagcccgcgccctggcccagaatcttgttggtctcggcgccggccttccattcttccttggacatgccgtcgcccagatccttgtcgatccaggggatcagcgagccgccgagcggggcgccgaagttggctgtttcagcggcactcaggttttgctgcttgtgcagcaccttgcgatcgatttcgagaatggccgacttcgggtcgtccagcagggcgcgcacttcggcgttgagcgtgccgaactgcgtcagcagttcgcgcatgtgctgcgcaccgccgcccgaagccgcctggtaggtcatgctggtcatccactcgaccaggccggccttgtagagggcgcccacgcccatgagcatgcagctcacggtgcagttgccgccgatccagttcttgccgccattggcaagcgcgttctggatcaccggcaggttgacggggtcgagcacgatgatggcgtcgtcctgcatgcgcagggtggaggcggcatcgatccagtggccggtccagcccgcggcgcgcagcttggggaacacctcgctggtgtagtcgccgccctggcaggtgatgacgatgtcgcacttcttcagcgcttcgatgtcgttcgcatccctgagcgcggtctcgttcttcgccatggccggggccttgccgccggcgttggaggtcgagaagaacagcggctcgatgagaccgaagtcgccttcggcctgcatgcggtccatcaggaccgagccgaccatgccgcgccagcccacgaggccgaccagaggttgagatgcgttcgccatttcagtttgccctattaaaagaaagaaaaaagttgtcttttcttgcccccgactcgtcgagccggggaggggcgtgacgaagcgggctgcggttagccggtaatcgtctttttggtgattgctgcaacgaccgcgtcgcccatctcacgggtgccgacgcgcttcgtaccttctgaccagatgtcacccgtgcgcagcccggaggcgagcacgtgcttgaccgccgactcgatacggtcggcagcttcggcttggttgagtgaaaagcggagcatcatggcagcggacagtattgtagccaaaggattggcaaccccttttccggcaatgtcgggcgcgctgccgtggctgggctcgtacaggccctggttgctcgaattgagcgacgccgagggcagcatgccgatggagccggtgagcatggcggcctcgtccgaaagaatgtcgccgaacatgttgccggtgacgatcacgtcgaacttcttgggtgccttcacgagctgcatggccgcgttgtcgacgtacatgtggtcgagctcgatgtccggatagtccttgtgcacctcggtgaccacgtccttccagaactggaaggtctcgagcacgttggccttgtcgacgctggtcacgcgcttgttgcgcttgcgggccgcctcgaaggccacgcgggcgatgcgctcgacctcggggcgcgaatagcgcatggtgtcgaaagcctcttcggctcccggaaagtggccgtccaccgccgtgcggcggccgcgcggctggccgaagtagatgtcgccggtcagctcgcggatgatgaggatgtccaggcccgaaatcagctcgggcttgaggctcgatgcgcctaccagctgctcgtagcagatggcgggacggaagttcgcgaacaggccgaggttcttgcgcagccccaggatcgcctgctccgggcgccgcgggcggtcgagcttgtcgtatttccagtcgccgacggcaccgaacagcaccgcgtcggcttccttcgcgagcttgagcgtcgcttcgggcagcggatggccgtgcgcctcgtaggctgcgccgccgaccagcgcggattccatttcgaaagagaggtcgagcacgtcgagcaccctgatggcctcggccacgatttcagtgccgatgccgtcacccgggagaactgcgattttcatgatttggtctgaagtttgaaaacggaaatgcgaagggcgatcaggcgatcatcgtgtgcgcgagccagggcttctgtgccaggcgctcggcttcgaaagccttgatcttgtcctggtggcgcagcgtcaggccgatgtcgtccagcccgttgatgaggcaatacttgcggaaggcctgcacgtcgaacgcgaactcgccgccgtcgggcttcaccaccacctggcgttccaggtcgatggtcagcgtgtagccggggaaggcaagggtctcgtcgaacagctgcgccacttgcgcctcgggcagcacgatgggcaagaggccgttcttgaagctgttgttgaagaagatgtcggcatagctcggcgcaatgatcgcgcgaaagccgtactggtcgagcgcccacggcgcatgttcgcgcgacgaaccgcagccgaagttcttgcgcgccaggaggatcgacgcgcccgcgtagcgcggctggttcagcacgaagtcggggttcggcttgcggctggccgggtcctggcccggaaagccggcgtccaggtagcgccattcgtcgaacaggttctggccgaagcccgtcttgcggatcgacttcaggaactgcttcggaatgatcgcgtcggtgtcgacgttctcgcggtccatcggggccacgaggcccttgtgcacggtgaatttctgcatgtgtgtctccagatcaggcgaaggtgcgcacgtcgacgaagtggccgtgtacggctgcggccgcggccatggccgggctcacgagatgggtgcggccaccggcgccctggcggccttcgaagttgcggttgctggtcgatgcgcagcgctcgccgggctccaggcggtcggcgttcattgcgaggcacatcgagcagccgggctcgcgccattcgaagcccgcggccttgaagatcacgtcgaggccttcgcgctcggcctgttccttcaccacgcccgaacccggcaccaccagtgcgagcttcacgttcttcgcgaccttctggccgagcttcttcaccacggcggcggcttcgcgcatgtcttcgatgcggctgttggtgcacgagccgatgaacaccttgtcgatgaagatgtcgttcatcgccttgttgggctccaggcccatgtagaccagtgcgcgctcgatggcgccgcgcttgctggcgtctttttccttctcgggatcgggcacgcggccgttgatgtccaccaccatctcgggcgaggtgccccaggtcacctgcggctggatctgggttgcgtcgagttcgaccacggcgtcgaacttcgctccggggtccgactgcagcgtgcgccagtagctcacggcctggtcccactccacgcccgtgggtgcgagcgggcgacccttgacgtagctgatggttttttcgtccaccgccacgaggccagcgcgtgcgccggcctcgatggccatgttgcagaccgtcatgcggccttccatgctcaggtcgcgaatggccgagcccgcgaattcgatggtgtagcccgtgccgccggcggtgccgatcttgccgatgatcgccagcacgatgtccttggccgtgcagccgagcggcagcttgccctcgaccttcaccagcatgttcttcgccttcttgccgagcagcgtctgcgtggccatcacgtgctcgacctcgctggtgccgatgccgtgcgccagcgcgccgaaggcgccgtgcgtggaggtgtgcgagtcgccgcagaccacggtcatgccgggcagcgtggcgcccgattcgggcccgatcacgtgcacgatgccctggcgcttgctcaggaacggaaagaacgcggcggcgccgaattccgcgatgttcttgtccagcgtggtgacctgctccttgctggtcgggtcggcaatgccttcatagccgcgctcccagccggtggtgggcgtgttgtggtcggccgtggccaccaccgagctgatgcgccacagcttgcggccggccacgcgcaggccctcgaaggcctgcgggctggtgacttcgtgcaccaggtggcggtcgatgtagaggatcgcggtgccgtcttcctcggtgtggacgacgtgttcgtcccagatcttgtcgtagagcgtgcgtgccatgtcggtctcttgctttcgtggggaggtgaattgtcttgttttccagccgctatgcggcgagcggctcggcggcatcgcgagcggccgccgcagtcgtgtgcaaatggttgaccagcgtgcgcgcggccaccggcagggtcgaaaagtcgcgcgccaccaggcggatctcgcgtgcggcccaggcgtcgttcagcgccacgctgcgaaggcggctgccgatgcccgcctgcagcagctcgaaggcgcgctgcggcatcacgccgatgcccagcccgttgtcgatcatgcggcacatggcgtcgagcccggtcacgtggatgcgcagcttgacgctgcggcccgcttccagggcggcctggtgcatggccacgtagatcgagctgttggtgtgcagcccgacatggtcgaaatccagcgaggcgacgaaatcgagcggcccctgcgcggccagagggtgcccggcgggcacgatcagcgccagccggtcgtggcggtagggcagcgtctgcagctcgtgggtgccgcccggaacgtggcagatgccgaggtcggcggcgccttcctgcaccgcgcgcaccacctcgttgctgaggtgctcttccaggtcgatcttgatcgcgtcgtgctcgcgcgtgaaggcgcccagatcctcggggagaaactgcacgatggccgagatgttggcgtgcacccgcacgtggccgcgcacgccctcggcgtattcgctgagttcgccctgcatcttctcgaggctgtagagcaccgagcgcgcatggtgcagcaggctttcgcccgcgggcgacagatcgaccccgcgcgcatgtcggtagaggagggtggtgcccagggtcgcttccaggtccgacagccgcttgctgacggccgaggcggcgatgaattcgcgttccgccgcccgcccgatactgccgagttcgcaaacggccacgaacagctgcagcgacgtgaggtcgatgcgccgggcgaaattgcgttcggaagtgctcatggggctttggacatcgcgtctggcgatgagttttcccattttcccagggttttggcgaggctgccatcgtcatgtgcgatgggttggttgccctggggcgacgagtcccggccgccctgcacgacaaaacgccccgcgcctcgctttgcagcgaggggcggggcgtgcgtgggtttgcgccggaaggcccggtgcctactggcgcttcttggcggcgtcttcgaccttttcgccacccttctggatgtcttggccggcacccctgaaggtgttgcagccacccagcgggacggcgagtgcgaaagcgacggcgatcagcgcgacaatttgcttcatgacgggtctcctgaaggcgttgaaaaaggcgacccgaagccgggcctccgatgcacaacgtaccgacaccgcgccgcgggccctgtcagccaagacgcaaaaaagctgcccgagggcagctttccaggttgagcggcagggcgccttcagcgttggccgatgggcttcacgtcgcgcttgggcgagccttcgaacagctggcgcgggcggccgatcttgtactcggggtcgccgatcatctcgttcagctgggcgatccagccgaccgtgcgggccagcgcgaagatcgcggtgaacagcggcaccgggatgccgatggcgcgctgcacgatgcccgaatagaagtcgacgttcgggtagagcttgcgcgatacgaagtactcgtcttccagggcgatcttttccagttccttggccagcttgaagagcggatcctgttccaggcccagttcggtcagcacttcgttgcaggtttcctgcatcagcttggcgcgcgggtcgtagttcttgtacacgcggtggccaaagcccatgagcttgacgttcgagttcttgtccttgaccttcttgatgaactcgccgatcttctccacgccgccttccttctggatgtcgtagagcatgttgagcgccgcttcgttggcgccgccgtgggccgggccccagaggcaggccacgccggccgcaatggccgcgaaggggttggtgcccgacgagccgcacaggcgcacggtcgaggtggaggcgttctgctcgtggtcggcgtgcaggatgaagatgcggtcgagcgcgcgctcgagcaccgggttcaccttgtactcctcgcacggcgtcgcgaacatcatgtgcaggaagttgcctgcgtagctgagttcgttcttcgggtacatgtagggctggcccacggtgtacttgtaggccatggccacgagcgtgggcatcttcgcgatcaggcggatcgcggcgatctcgcggtgttcgggattgttgatgtccgtgctgtcgtgatagaaggccgacagcgcgcccaccaggccggtcatgatggccatcgggtgcgcgtcgcggcggaagccgcgcaggaagaactgcatctgctcgttgaccatcgtgtggttggtcacgagcttggtgaagttggtcttcttggcctggtccggcagctcgccgtagagcagcaggtggcaggtttcgaggaagtcgcagttggttgcgagctgctcgatggggtagccgcggtacagcagttcgcccttgtccccgtcgatgtacgtgatggccgactggcacgcggccgtcgacatgaaacccgggtcgtaggtgaacatgccggtctgcgcatacagcttgcggatgtcgatcacgtcggggccgacggtgcccttgtagatcggcagttcgacgctgtcaccaccgttgctgaacgacagcgtggccttgatatcggaagctttcatttcgggtttctttcagaggagtattcaggagggcgaagaggaaacggaggttgcgggacgctgcgcgccgtcggtgcgcatcagctgcagcagttcgaccacctcggccccggcccatgcgggctcgggctcctttcttcgcagcagaagatcgaggaggtcgttgtccgacaggtccatcaatgtctccatcgctcccgcctgaccgttggtcatgtgggattcgtgccgctcgaagaagcgggcgatgaacaggtcgttctctagcaagccgcgccggcagcgccatttcagcttgctcagcgctcgttcgctgatcggctgtgcgagttcggcggcggtttgcatggtttctctggcaaaagttcagatggcgcggcgcaccatcaattccttgatcttgccgatcgccttggtcggattcaggttcttggggcacacgtcgacgcagttcatgatcgtgtggcagcggaacaggcggtacgggtcttcgaggttgtccaggcgctcggcggtggcttcgtcgcggctgtcggcgatgaagcggtaggcctgcagcaggccggccgggcccacgaacttgtcggggttccaccagaagctcgggcagctggtggagcagctcgcgcacaggatgcactcgtacaggccgttgagctcgtcgcgctcctcgggcgactgcaggcgctccttctcgggcggcacgttgtcgttctgcaggtacggcttgatcgagttgtactgcttgaagaactgcgtcatgtccacgatcaggtcgcggatcaccggcaggcccggcagcggcttcaacacgatcgtgcccttgagcgtgagcatgttggtcaggcaggcgaggccgttcttgccgttgatgttcatcgcgtcggaaccgcagacgccttcgcggcacgagcggcggaacgacagcgtgggatcttgcgccttgagcttcatcagggcgtcgagcagcatgcgctcatggccgtcgagttcgatctcgatcgtctgcatgtagggcttggcgtccttgtccgggtcgtagcggtagatctggaatgtgcgcttcatcgtgaaaccttgtgatgttgttcttgtttagaacgtacggaccttgggaggaacggagtccaccgtcagcggcttgaggttgacgggcttgtaggagaggcggttgtcctggctgtaccagagcgtgtgcttcatccagttggcgtcgtcgcggccgagcggtgcgaccgggtcgtcggccgggcgctcgtagtcttcgaccgtgtgcgcgccgcggcattccttgcgggcggctgccgaaaccatcgtggcctgcgccacttcgatcaggttgtcgacttcgagcgcttcgatgcgcgcggtgttgaacaccttggacttgtcctggaggccgatggcgttgacgcgctcgcgcacggcggcgatcttgaccacgccttcatccatggaggcttgcttgcggaacacggcagcgtgctgctgcatgacggcgcggatctcgcccgccacgtcttgcgcgtactcgccgccggtggctgcctcgagccggttcaggcgctccagcgtgcggtcggctgcatcggccggcagcggcttgtgttctttcagcttgtcgttgaattcgacgatgtggttgccggccgcgcggccgaacaccagcaggtcgagcagcgagttggtgcccaggcggttggcgccatgcacgctcacgcaggagcattcgcccacggcatagaggccgttcaccacggcgctgttctgttcgccctgctggatcacgacctggccgttgatgttggtcgggatgccgcccatctggtagtggatggtcggcacgaccggaatcggctccttggtgatgtcgacgttggcgaagttcacgccgatttcgtacaccgagggcaggcgcttgtggatggtctcggcaccgaggtggtcgagcttcagcagcacgtagtccttgttgggaccgcagccgcggccttccttgatttcctggtccatcgagcgcgacacgaagtcgcgcggtgccaggtctttcagcgtgggcgcatagcgctccatgaagcgttcgccgttgctgttgagcaagatggcgccctcgccgcggcagccttcggtcagcagcacgcccgcgccggccacgccggtcgggtggaactgccagaactccatgtcctgcagcggaatgcccgagcgcgcggccatgcccaggccgtcgccggtgttgatgaaggcattggtcgaggcctggaagatgcggcctgcgccgccggtggccagcagcacggtcttggcctgcaggatgtgcaggtcgccggtttccatttcgagcgccgtgacgccgaccacgtcgccttcggcgtcgcgaatcaggtcgagggccatccactcgacgaagaactgggtgcgggcttccacgttcttctggtagagcgtgtgcagcatcgcgtggccggtgcggtcggccgcggcgcaggcacgctgcacgggcttctcgccgtagttggccgtgtggccgccgaacggacgctggtagatcgtgccgtccgggttgcggtcgaagggcatgccgaagtgctcgagctcgtacacgaccttgggggcttcgcggcacatgaactcgatcgcgtcctggtcgccgagccagtcggaacccttgatcgtgtcgtagaagtggtagtgccagttgtcctcgctcatgttgccgagcgatgcgcccacgccgccttgggcagccacggtgtgcgaacgcgtcgggaacaccttggagagcaccgccacgttcaggcccgcgcgggccagttgcagcgaggcgcgcatgccggagccgccggcgccgacgatgacgacgtcgaacttgcgcttggtgatttgttcttttgtgtaggtcatggtggggtcagatcttccaaagcacttgaatggcccaacccgcacaaccgacaagccagacgatggtgaaaatttgcagggcgaggcgaatgccgacgggctggacgtagtccatccacacgtcgcgcatgccaacccacacgtgatagagcagggaaacgatcacggagaaggtcagcaccttcatccactgcgcggcgaagatgccggcccagaggtcgtagccgatggggccacgcgtgaagatcagctgtgcgagcaggatgatcgtgaagagcgccatcaggccgcccgtgatgcgctggctgagccagtcgcgcaaaccgtaatgtgcgccgacgacgatgcgcttggagccgtaattcacagacatggttggctccttctcagtacaggccgaacagcttggcgcccagcaccacggtgagcaaaacgctcaggaccagcgtgaccagggcggagctgtgtccgaactccttggtgacggcggcgtggctcacgtccatccagaggtggcgcaggccggcgatgaagtggtgcaggtaggcccagatcagcgcgagaaccaccagcttcaagaaccagcccggagcgaaaccaaggccgctgttgaatgcggccttgaacctggcgaacgaatagtcggacgaaagcgaggtgtcgaacatccagatgacgaacggcagcagcaggaacatgatcacaccgctcacgcggtgcaggatcgacacgatgccggccggcggcaaccggtaggtcgtgagatcggtgaaggcgttgatgtttcggaattcgcggcgcggtggccggggaggggttgcaagctctgacattgggggaaggctttcgtggcttggtggcttgttctgatgttctgagagcgaacgcttttgtttcttctgcggaatgcaaacaacgcaaaattctattgcaatgcaccattgtccggcggaggtgcccgtgtcggggcagcgctgcagtcggatgctatggagttcgtagcgtgctgcgcacgggtcgcgggcgcttcgatgcgggtcggtcgtgaggccatctggatgcgatctcagccgagctggttgcggtagtggtgcgtgtcggtgcgatagaggccgcggcgcaattccatcggcatgtcgtgatacgtatgcgccaggcgctccacgctgagcaagggcatctgcaacgacacgtcgagcagcgccgcctgctcggcatcgggcagcacggcgcggattttttcttcggcgcgcaccatgcgcacgccgaattcggtttcgaacatcgcgtacatcgggcccggccaggcccgcagccgctcggcggtcaggcccttgaagggcgcgccgggcagccagagatcctcgaggatggtgggcacgcccccataggcgagcacgcgccgcacctgcagcaccgcgtcgcccgtgcgcaggcccagtgcacgcgccacgtcggccgaggcgcgctggcggcggcaatcgacgatggtgcgctcggcagggccttcggtgctcggggtgccgacatcgggcacgagcttgagaaagcggtactgcacatgctgctcggcatgcgtggcgacgaaggtgcccttgccctggcgccgcaccacgaggttttcggccgcgagctcgtcgatggccttgcgcaccgtgccctggctcacgcgatagcgcactgccaggtccatctcgctcggaatgggctcgcccggcttccactcgccggcctgcaggctctgcaggatcagtgtcttgatctgctggtagagcggactgaaggagggcgtcgcagattcttcgaggacggagggggcattcatggcagcggtgggtgcgccgtggcggaacctccgagcatatcttatataagacataagacgacgctcatcgaatcggcttaaaatgcgggccggcctgcgccgcgggaaggattcccgccctgcaggaccatcggcgctccgcgcgcccgccgataccgtttcactaccttctggagtcttcccatgagcaaaaagcccgtccgcgttgccgtcaccggtgccgccggtcaaatcggttacgccctgttgttccgtattgcgtccggcgaaatgctcggcaaagaccagccggtcatccttcagctgctcgaaatccccgacgagaaggcccagaaggccctcaagggcgtgatgatggagctcgacgattgcgccttcccgctgctggccggcatggaagcccacggcgacccgatgaccgccttcaaggatgccgactacgccctcttggtcggttcgcgtccgcgcggcccgggcatggagcgtgccgagctgctggccgtcaacggcgccatcttcacggcccagggcaaggcgctgaatgccgtcgccagccgcaacgtcaaggtgctggtggtcggcaacccggccaacaccaatgcctacatcgcgatgaagagcgcccccgacctgccgcgcaagaacttcaccgccatgctgcgcctggaccacaaccgcgccgcgagccagatcgccgccaagaccggcaagccggtggccgacatcgaaaagctcgtcgtgtggggcaaccactcgcccacgatgtacgccgactaccgctttgccaccatcaacggcgacagcgttgccaagatgatcaacgaccaggaatggaacgccaacaccttcctgccgaccgtcggcaagcgcggcgcggccatcatcgaagcgcgtggcctatcttcggctgcctcggccgccaacgcggccatcgaccacatgcgtgactgggccctgggcaccaacggcaagtgggtcaccatgggcattccgtcggacggccagtacggcattccgaaggacacgatgttcggcttcccggtcacctgcgagaacggcgagtacaagctcgtcgaaggcctcgagatcgacgccttcagccaggaacgcatcaacaagaccctggaagagctgcaaggcgaacaagccggcgttgcgcacctgatctaagcaggctggccggcatgctcgactggaaccccgcgctctaccgtcgctacgaggacgagcgcacccgacccgcacaggaactcctggcgcgggtgccgttgccggaggccgcccgcgtggtcgacctcggctgcgggccgggcaattccaccgagctgctggtccatcggttcccgacggcgcaagtcgccgggaccgacaactccgaagccatgctggccagtgcgcgcgagcgcctgccgcaggcgcgcttcgagttgagcgacatcgcgacctgggcgccgcaagaagcgcccgacctcatttatgccaacgcagccctgcaatgggtgccggaccacgaaaagctgatcccgcgcctgttcgctgcgctggccccgggtggcgtgctcgccatccagatgcccgacaaccgcgaggagcccacgcaccgcctgatgcgcgccgtggcggccgaggcgccctgggccgagcccatcggcgatgccgaccggctgcgcaccttgctgctgccgcttggcggctactacgacctgctggcgcccgatgctgccaaggtcgatgtgtggcacaccatctaccagcaccccatggccgatgccgcggccatcgtcgaatgggtgcgcggcacgggcctcaagcctttcgtcgaccggctgccggccgacctgcaggtcagctatctcgccgcctacgagcgccgcgtgaacgaagcctatcccgcacgcaccgacggcaagcgattgctggcctttccgcgcatgttcatcgtggcgcagagaaaagcatgacccagagcatccatcccgccgaagtgctgcttggcgcgcaagccggcgccgtgacgctgccggtgtgcgaccactacagcggcgttgaagcgcgcatgaagaagagcctggcgctgcaggccgaaatggccgatgaattcggcgcctgcgtgttcgacgtcacgctcgattgcgaagacggcgccccggtgggcggcgaggcggaacatgccgcgctcgtgaccgaactcgcgctggcagccaggcccggcatgcgggtgggcgtgcgcgtccatccggtcgatcacccggcctttgccggcgacgtgatcaccattgcgggccgcgccggccacaggctcagccacctgatggtgcccaaggtcgagtccgtggccgacgtggtgcaggcggtggcggcgctcgaggccgcggatgccgacgcgctgccgctgcacgtgctcatcgaatcgccgctggccgtgcacaacgcgttcgagatcgcggcgcatccgcgcgtgcaatcgctcagtttcggcctgatggacttcgtttccgcccatgcgggcgccattcccgccgatggcatgggggctgccggccagttcacgcatcctctggtggtgcgtgccaagctggccatcgcatccgcggcgcacgcatacggcaaggtgccgtcgcattgcgtggtcaccgagttcaacgacaccggcgccatgcgcatggcagcccgcaaggcggccaccgaattcggctacacacgcatgtggagcattcatccgaaccagatccggcccatcctcgaggcttttgcgccggacgaggcgcagattcaaattgccacaaaaatcattacaaatgcggccctcgcaaattgggctccgacccaaatcgatggcacattgcacgaccgcgcgagctatcgccatttctggcaagtgctgacgcgtgcccacgcaacagggcgcgtgttgcctccagaggccaaagcctggtttgcactcgcggcctcctgaaactcctgaatccagcctcaaggaaacacccatgaagaaaattgttctgatcgcagccctggccctggcggtcccgtttgccgccacggcgcagaccaccgcccccaaggccgaagccaagaaggcgccccccaagaagcaggtcacccgcaaggccgccaaggccgtcgaggaagtcacgcctatcgccgatgaaaccaatatcgtgctgaccgacgccgacctcgaagtcgccaagcgcgtttcgctcggcagggcccagtgcgaactcggcgccgacgtgaccgtggcggccgacgagaagaagcctggcttcttcaatgtgtcgaccaagggcctgaagtaccgcatgcacccggtcgaaagccgcaccggcgccatccgcctcgaagacccccgcgctggcgccatgtggctgcagctcggcaacaagtcgatgctgatgaaccagaaggcgggcctgcgcattgccgacgaatgccagacggcggagcaggttgcgtttgccgaagaaatgaagaagaacccgccgaagagcctgttcgaaggcgctgacgcagccaagaagtaagagtccccacacggggtgcggcgcggctcttgcttgccgtaccgcacgcccgccagcccagtttccggagaaaagaagatgttgcaagcctacgttgaccatgttgccgaacgcgccgcgctcggtattccgccgctgccattgagcgcgaagcaaaccgccgaagccatcgagctcctcaagagcgcgaatgccaaggacggtgctttcctgctcgatctgctcacctatcgcgtgcccgccggcgtcgatgacgcggccaaggtcaaggcgagctacctggcggccgtggcccacggtaccgagaagaacgcgttcatttcgcgtgcccgtgccaccgaattgctcggcaccatgctcggcggctacaacatcagcccgatgatcgacctgctcgacgacgccgaagtaggcgccgcggcggccgaaggcctgaagaaaaccctgttgatgttcgaccagttccacgacgtcaaggaaaaggccgacaagggcaacgcccacgccaagggcgtgctgcaaagctgggccgatgccgagtggttcaccagccgccccgaagtgccgcaaagcatcaccgtcagcatcttcaaggtggccggtgaaatcaacaccgacgacctgtcgcccgcacccgatgcgacgacgcgtcccgacattccgatgcacgccctggcgatgcacaagaacgcccgccccggcatcgtccctgaagaagacggcaagcgcggccctgtgaagttcatcgaagacctgcgcgcgcgcggccacctcgtggcctacgccggcgacgtggtcggcacgggctcttcgcgcaagagcgccaccaactcggtgctgtggttcaccggcgaagacattcccttcgtgccgaacaagcgcttcggcggcgtctgcctcggcggcaagatcgctcccatcttctacaacacgatggaagactcgggcgcactgcccatcgagctcgacgtgacgcagatgaacatgggcgacgtggtcgagctgcgtccctacgaaggcaaggccttgaaagacggcaaggtcatcgccgaattccaggtcaagagcgacgtgctgttcgacgaagtgcgcgccggcggccgcattccgctgatcatcggccgcggcctcacggccaaggcgcgcgaagcgctgggcctgcccgtctccacgctgttccgtctgccgcaaagcccggtcgacaccaagaagggcttctcgctcgcacagaagatggtcggccgcgcctgcggcctgcctgaaggccagggcgttcgcccgggcacgtattgcgaacccaagatgacctcggtcggctcgcaggacaccaccggcccgatgacgcgcgacgagctgaaagacctggcctgcctgggcttctcggccgacctcgtgatgcagtcgttctgccacacggcagcgtacccgaagaaggtcgacgtcaagatgcaccatgaactccccgatttcatggccaaccgcggcggcgtttcgctgcgtccgggtgacggcgtgatccacagctggctcaaccgcctgctgacgcccgacaccgtgggcaccggcggcgacagccacacccgcttccccatcggtatcagcttcccggccggttcgggcctcgtggccttcgcggccgccaccggcgtgatgccgctggacatgcccgagtcggtgctcgtgcgcttcaagggcaagatgcagcccggcgtcacgctgcgtgacctggtcaacgccattccgctgtacgccatcaagtcgggcctgctgacggtggccaagcaaggcaagaagaacatcttctcgggccgcatcctcgagatcgaaggcctgcctgacctgaaggtggagcaagccttcgagctgagcgacgcctcggccgaacgctcggccgccggctgcacggtgcacctgaacaaggaaccgattcaggagtacatcaacagcaacatcacgctgatgaagtggatgattgccgaaggctacgccgacgcccgtacgctggcacgccgcatcgctgcgcaggaagcctggcttgcggacccgcaactgctcaagggcgatgccgacgccgactacgctgccatcatcgagatcgacctggccgagatccacgaacccatcgtggcctgcccgaacgaccctgacgacgtgaagacgctgagcgacgtggccggcgccgtgatcgacgaagtgttcatcggctcgtgcatgaccaacatcggccactttcgcgccgcgtcgaagctgctcgaaggcaagcgcgacatcccggtcaagctgtggatcgcgccacccaccaagatggacgcccagcagctcaccgaagaaggccactacggcgtgttcggcaatgccggtgcgcgcaccgaaatgccgggctgctcgctgtgcatgggcaaccaggcacaggtgcgcgaaggcgccacggtcatgtcgaccagcacccgcaacttccccaaccgcctgggcaagaacaccaacgtgtacctgggctcggccgagctggccgcgatctgctcgcgcctgggccgcatcccgacgcgggaagagtacatggccgcaaccggcgtgctcgatgcgtcgagcgcccagatctaccagtatctgaacttcgacaagatcgacgactacaagaccgaagcggctgccgtggcctgatccacgcgctccgtcgcaacctgaagagccccgcttgcgcggggcttttttacgtgcggcgcaagtttgctttcttcagccggccgccaatgcggtcagcgccgcggccgtctgcgcatcggccggaaagaacgactccaccgccagctcctgcagcgtgacatcgaccggcgtgccgaagatggtggtggtgctgatgaagctcagcacgccgttcggcgtggccaactgaaacggcaccaccaggcctgagaattcggtgtccacggcgggcgtatcgtggcttacctggggcgtggggtaggcctcgagttcgtcgtgcagggcctgcagcgccgtgtcgcccgtggctgcgatctgctgctgcaatcgctcgagcagatgggagcgccactgcgccagattggcaatgcgcgaggccaggccgtcgggatgcaggctcagccgaagcacgttgatgggcggcttcaccagttcgggtgcggcgccggccatcagcatcggcaccagcgcgttgtgcgccaccagattccagtggcgatcgaccgccaatgcgggaaaaggctcatggcccttgagcaccaggtccaccgcgcgccgtgccgacgccatggcggggtcgtcgagcgagcgttgcctgtacatcggcgcaaatcccgccgccaccaggagcgcattgcgttcgcgcaggggcacttcgagccgctcggccagacgaagcaccatttcgcggctgggtgcggcgcggccggtttccacgtagctcaggtggcgggtcgagacctcggcttcctgagccaggtcgagctggctcagccggcggcgggtgcgccaatgccgcaggtggacgccgaacgggtcgcgcgcgccgggctggctggccttggacgagtgggtgcgggaagtgttcatggccccgattctggcgtggcgccgcgaccgcgccatgacctcacaggttatcgaccgtgtgcgcacccttcggaatcattggctccaacgcggcaggacaggcttgcggcgtaaccacccaaaggagattctcatgtccgtctttgcatccccccgcttcctgcccaacgtgatgtgggccgacgcggcctcctgtgccgcgaccggtgcgctgcaggttgcgttcaccggcgcgctcgcgcggctgatcggattgccggcgccgctgctcctgggaacgggcgtgttcctgctggcctacgcggccgccgccggtttcatggccagccgccgcacgccgcctcgcatgctgatcggcctcgtggtggccggcaacttcggctgggccgcggggtgcatcgcgcttctgatgagcggcgtgttcgcagtcaccgcgctgggcatggcgtgggtgctggcgcaggccctctgcgtggtggtgctggccgaactgcaatggaccggtttgcgccgcagtgcgcgaagcccggggacggacttagtccccgactacagcaattgacattgatccccgctatccttgaggcgcttccacgaaccaacaggagttcctcaatggccaaagcaccggcacacgcctttgcgtccaccctcaagaccttcaagaccgcatcggggaaagccggcaaatactggtcgctcaaggagctggccaggcaatatcccaccgtcgaacgcctgccggtgtcgattcgtatcgtgctcgaatcggtgctgcgcaattgtgacgggcagaaggtctcgcccaagcacgtggaagagctggcccattggtcgcccaacgcagaacgcaccgacgaaattccgtttgtcgtgacccgggtggtgctgcaggacttcaccggcgtgccgctcctggccgacctggccgcgatgcgcagcgtggccgccaagctcggcaagtcgcccaagaccatcgagccgctggtgccggtcgatctggtggtcgaccactcggtgatggtcgactactacggcacgcccaaggcgctcgacctgaacatgaagctggagttccagcgcaacaacgagcgctaccagttcatgaagtggggcatgcaggccttcgacaccttccgcgtcgtgccgccgggcttcggcatcgtgcaccaggtcaacctcgaatactttgcgcgcggcgtctacaagagctcgagcgacaacgccgaagttcccacctactaccccgactcgctggtgggcaccgacagccacaccaccatgatcaacggcgtgggcgtggtcgggtggggcgtgggcggcatcgaggccgaggccgccatgctgggccagccggtgtacatgctgacgcccgacgtggtgggcttcgaactcaccggcaaactgcgcgaaggcgtcacggccaccgacctggtgctgtttgtcaccgcgatcctgcgggccgaaaaagtggtgggcaagttcgtcgaattcttcggccccggcgccgcctccatcgccgtgcccgaccgtgccaccatcggcaacatggcgcccgaatacggcgccaccatgggcttcttcccggtcgatgaaatgaccgtggcgtatttcgaaggcaccggccgcaccaaggaagaggtcgagcgcttcgaggcctactacaaggcgcagggcctgttcggcatgccggcgcccggcgacatcgactacaccaagatcgtcaagctcgacctcggcaccgtgtcgccgagcctcgcgggaccgaagcggccgcaggaccgcatcgacctgggccacctgtcgaccaagttctccgaactcttcagcaagcccaacgatgccaacggcttcaaccagccgcccgagcggctgaagctgcgctatccgctgaccacgaacggccagggcgacgacgaggaaaccgcccctccgccgccgggcgcaccgcgcgacgtggtcgagatggtggccaaccggtcgaccaaggcggctgcccacgtgagcgccaccgcgccctcgtcgcccaagggcggagtgaccatcggcaacggcgacgtgctgatcgcggccatcacctcgtgcaccaatacctccaacccgagcgtgatgctcgcggccggcctgctggccaagaaggcggtcgaggcgggcctcacggtcaagccgcacgtcaagacctcgctcgcgcccggctcccgcatcgtcaccgagtacctcgagaaggccggcctgctgccgtatctcgaaaagctcggcttctacctggccggctacggttgcaccacctgcatcggcaatgcgggcgacctcacgcccgagatcaacgatgccatcgtcaagaacgatcttgtcggcgcggctgtgctctctggcaaccgcaatttcgaggcgcgcatccatccgaacctgaaggccaacttcctggcttcgccgccgttggtggtggcttttgccattgccggcaacgtgatggtcgacctcatgaccgagcccgtgggcaagggcaagaacggcaagaacatatacctgggcgacatctggccgacgccgaaggagatcgacgacaacctgcgctatgcgatgaacgccaagtcgtttcgcgagaactacgacaaggtcaagagcgatccgggcaagttctggagcagcatcgaaggcacggcgggccaggtctacgattggcccacgtcgacctacatcgccgagccgccgttcttctcagacttcaagatggcgccgcacgcgtccgacgcaggcttcaagggcgcgcgcgtcatggccctgttcggcgactcgatcaccaccgaccacatctcgccggccggctccatcaaggaaagctcgcccgcgggcatctggctcaaggcgcatggcgtggccaaggccgacttcaacagctacggctcgcgccgcggcaaccacgacgtgatgatgcgcggcacctttgccaacgtgcgcatcaagaacctgatgattccgcccgacatcaacggcacgcaggaagagggcggcgtcacgctgttccagcccggcaaccagaagatgttcatctatgacgccgccatgaaatacatggaacagggcgtgccgacggtggtcttcggcggcgaggaatacggcaccggctcgtcgcgcgactgggccgccaagggcacgcagctgctgggcatcaaggccgtggtggcgcgcagcttcgagcgcatccaccgcgccaacctggtcggcatgggcgtgctgccgctgcagttccgcggcgccgattcgtggcagacgctggccctcaagggcgacgaaaaaatcgatgtggtgatcggcgggcagctcaagccgcagatggacgtgaagctggtcgtgcaccgcgccgacggctcgcatcaagaggtgacggtgcgcctgcgcatcgacacgccgatcgaggtcgattactacaagcatggcggcatcctgccgtttgtgctcaggcaactgctcgcggcttgattcgcgtcggcctcatctccgatacgcacggcctgctgcgcccgcaggccgtggcggccctgcagggcagcgacttcatcgtccatggcggcgacatcggcgatgcgggcatcctcgacgcgcttcgggccatcgcgcctctgacggtggtgcggggcaacaacgaccgcgagccatgggcatcccggatcccggaaacggagttcctgcgggtcgccggggtgctcgtctatgcgatacacgacctgtcgcagatcgacatcgaccctgcggctacgggcgtgcgggtggtggtgtccggccattcccacaagccgaaggtcgaggagcgcggcggcgtgctctacgtcaatccgggcagcgccgggccgcgccgcttcaaactgccgattgcggtcgccgagctgatcgtggtggacgacgcagtcacggcgcgcatcgtcgaactggcctgagcagcgagaaaagggcagaaccaagctggtcgtgcaccgtgcgacggctcgcgccaggaggtgacggtgcggctgcgcatcgacacgccgatcgaggcgactactacaagcatggcggcatcctgccgttcgtgctcaggcaattgctggccagctgacggtgcaagggcgccggtctcagatcgacaagacagggatcggcaccttttctttcagccgctgcgtgaagtagcggtcctggtagtagcggatcttgtcgcacttgaccggatgcggaatgccttcgtagaggaagacctctgtgtccggccccatggccttgagctcctgcggcagcatcagggcgcggcgctcttcggactcgctgcggctggtctccctgcctctggtcacgttctgtttgcgcacggtggtgtagcccagcatgtcggagtagtcgttggcgtcttgctgctcgcgcggcgcgtagatgatctgcaaagcgtggttggtgatcagggtgcgcgccacttccttgccataggtggcgtccaattgggccatgctctggatgatgggcagcagccgcatgttgtagcccgccatgtagctcacggcgttggcgatgatgtttaccttgccgatgctggtgaactcgtccatcagcagcaggcactggtgcttgagctccggattgttctgcggcagctccttggtgttcacgttgatgagctggctgaagaacagattgacgatcaaccggctctcggcgagcttgttgggctggatgccgatgtagatcgtcatcttcttcttgcgcacatcggtgagcaggaagtcgtcggcactggtggccgcgtcgagcaccgggttgatccaggcattgagcggttctttgaaggtgcccaggatcgaggcgaaggtttccgccgcttgtgagagcaggttcgagaaagcggattgcgcattgccgctcaggaagggcgattgcgccagttgctcgtagaacttgcgcaggtcggtgccgttaccggaagacagttgatagatttgcccgagcgtgcgtgcgacgcggagcggttcggagatgtcccggcctttttcgtcatcccacctttcgaacagataaagcgaaaacgccatgaatgcgttgcgcgcctggctgacccagaacttctggtcgtccgcgccgtccgggtacagcatggcggcaatgctcatcaggtcagacacgcgaaacgccggatcgctggagacgtaggtcaacggattccagcgatgcgaccgtctgtcttccgcgaaggggttgaaaagatagacatcctgcccctgtctcgcgcgccatccgctggtgagttggtagttctcctgtttgatgtcgagcaccaccatcgactccccgtactcgagcagattgggaatgacaatgccgacgcccttgcccgagcgcgtgggggccgcaagaatgacgaactgctggcccggcaggcgcaccagcttgccgtcgaacttgcccaccagaattccgttgtccgcaggcttgaacatgccgaacttgccgaggtcagcacccgtagcgaagcgggcgtctccatggatcgaaggcgccttggtcctggcgagcagcgccagcaggccgagccagagcaacagtggcacgccaaagccaacgtagccagccagatggatttgctgcgagtaggcgtggtaagcgggcagttccaacgcttgccagtaagccggatatgtattccaggccagcgttcgcgtgtccagtttgagcagaaggagggcgagccaacccgacaggtaaagccccgctggaatcgccgcaagaagggtcaaggctgcagcagcccacttggccttggtcatttgaatatcacttgtagttcgcgagtgcccagcactcgatgcgcagatggctgcggcgaatcgaagacgcttggatctgccatgcgtcttgaggcaagctgcctcacttgaatgtcaccgcccgaaggaatcagtgttcgaacggcgtgctgcccagtactcacgcgtgaggtcaactcaatgcagaaccggcgaagtttgcgtctgggcaggctgattcatctgctgcgaacgtaggttctgttgctggttgtgggcatcggcgaaggcttgcgaactctgcgcaagaggcgtgttcagtgccaccatcgtgtcgacatcgatcacctttgaatgagcggtccccggtcggccctgtatggcgatgaacttggcgccactgtcgttcggcgctatatcgtcgatgcgcttgagcccgcgatgctgcgcttcggtagctattgctgcggcggcattcttggtgccctgatcggatgggatgtcgtgctcgcgattccacttttccaaacctgccaaggcttgcttgtacagcgcgttgcctgggtggccttcttcagtgagagagctcatcgccgctgccttgacggcgcgctgcatcgttggaccgtggtagacagcagccaactgcttggcgtagtgtggatcggttgcgtagccagccttttgcagcgcagcggcttctttctcaagatttcccttggtgcccggatcgaacagtcccgacttggtatagcgcgaattttcctggagaaacttcacgcggtcgttcagcgcatcttcggtggaagcatagacacggaactccgcattcaccatcactttcttgccgtccaggaactccggaacagcgaaggtcttggtagggccgcgccagtctggcgatgccttgatattgaagatgttgttggtgccggacagcaccttctcgccccagcccgtttccagtgcggcctgcgccaggatcaattccttggacatgcccgtctgctgcgagaccttggccgctgccgggtatagatctgcgatgaattgctctttgccattttgttgcgcgggtgtggctactgccaatcggtccttgtcactcatggtttgctcccttggggttctagatcgttgttcaaacgcacggtgaatttctgcacgcgctcatgatctgaagccaaacgcacattgccggtgatgacgaggcgattgccgctccagacaaagcgagtcgcacccttgttcacccaggcagagtaggtggcgggtatttcgacatcctgcagaagctgcacggcacccgtgaaggcattgagctttacaacgcgcaatcgcgtttgcgaaaggctttgcgacgcttgcgtatcggactgcaacagcacatagagtgcatcgccacgtccggcgcaatgcgtggcccggctttggtacatgtctgcaggcaagtcaagccgtgcaatccacagcacacgcttgccagaagcgttcgttgcgtagacctcaggcctttgattcatgccatcctcgtcggcgctcatgccggagacgcagcgccggctatggccaatggatgcggacgcataagctgtgaaatggtccggcaatttcagcgcggcgctagatgttccagccgcattgtgttgaaccggcttggcctgtgtgggctgagcatgagccgataccgagtgcgtgctccaggcgaggaatagcgagcacaaggcgagaaggtgacttgaatggatgcgcttcatgatgctatgaaattaatggcgatctgcgcccatcccataggcgcaaagggatgatttgcctggaagtcagtctgtggttcaggccaacatgaccggctgcgccagctgctgggtttgggactgcgacgcaggttgctgtggcgtggccttgttcattgcctggaggtagcccctggagctgtcttcaagcgatgtgttcatggcttgtaccgtcggcacatcgatcaccttggaatgcgccgttcccggagtaccttgcaccgcaatgagcttgctgccgttgctgccgagtgccacatgatcgatctgctcgaacctggattcacaagccgatgcggccaacgtgccggcggcattgcgggtacgttgatcggtggggatgccgcgctcgacgttgatcttctccagcccggccaaggcctgcttgtagaacccgttgccaggatgctggccatcgttcaacaacggcaccggtcctgtctggctgctgaaccacgaccccggatgagtgagcttgtcaattgcgcgggaagcgccctcatgcagcgcttcaccggtccgctccagcgcttcacctgcctgccgagcacctgtctccaccgtgtcgcgcgctgcatcgtaggcccgctcggccgcgtggctggccgcctgtgcgcccgaaacgacagccttgccagtcgttttggcagcgtcgacgaccgcggtgcttgttgcgtcgtaggcctgccccgcggcatggccgactgcctgggcgccgtgcacggccgtctgcgcacccgacaccatggcttgcgtggccttctctgccaccgccgtgctggccgcatcggccacttgcacaccgaggcgtacgccgttcacggcggaggccatcgggatggcgttgttggcgaccttgttcaaatcgacgcgcccccgcaccacgtcattcttgtaatgctcgatggccgaagcataggcgcggccccgtgcttcgttgttcgcgctgagcaccgaatcgccgatcacctcgttgtccggcaggaagttggtgatcgtgtgcgcacccacatccgccgccagcagcgggttggccggcaagggcgaagcgccgatgtagcggccacgcttcaggttctcgatgtcctgcggtgccgcataggtgcgtgtgctgcccaggtgcgggccgcccgcgcccaccacatcggtggcgcgcacatggttgacgatatttgggtgcggggtgtgcacatcgacgccgtagcggtcgaggttcttcagcgcaccggggccgtacgcattgaaggtctcggcgtgcaagccggttctggctgccgtaatctcggccagcgtgcctcccagggagtggccggtgagggagatgttgaggggagtgttgttgtccttggcgtttttcctggcaagcgcgatcgcctgctcggtgaacgccaccgcatcgtcgagctggttgttgcgccctgtgaagaccatgcttgcatcggtcaggccatctttggccgactccgtgccgcgatgcgcgatgatgacttccttggtgtccacgcgctggtagaccgtgccctgatagtccgtcttggggttgttggcgacggcaaggacggtgtactcgatgctgctgcccctgagggtgaatgacttgtcagagcccgccaacttggagcggtcctcgtaggagtcagcggacaggcgtgcatattcggcggcatcgatgctcattcgaagtgctccttggcagccagggtggtggagaagaagtcggcttgaatgcgagtcgcaacgtagttcgtgcccaagctggaaatgggcgccgtccgaatcgtgaggccggaggggagggtgacagtggagggggtggagttgtctccgtaagctctcttggcgaaatactcagtctttgactgctgcgcaacgacatccctgtcccacatgctggccccaaagctcacctcgccagccgtcatcacagcgctgaaggacgaaaaccgccatcgacagacccccaacccgtagtagtcctcgtcctcgggccagtccatgtacatcgtgccttggtagatgttcgcgctcaaggcacgcagcaccactggcacggagtggcccagcggatacttcgcgccatagttggctgcggtgatcggcgcctccggcacgcagttggtgtcggtctcgaaattcgcataccccgccaccgactcgaacggccctggcgcgtcttcaatggtcaacgtgatttcatagcgcatcttcggatgcggattgagtttgatgtcgggttgtttcatggactgtccgcaggcggttgtagtgagagcaagaaggacggtgagagcggggatgaggcgcttcatggccatctaaccccgcaacgcgcgtgagctgtgcgcgagtcgctcgaattggcggcaactgatgaagtgcatggcatctaccgaattcgtaccggcaggctgcaggcggtgtaaagagtgcggcaatcagtgtcaccaccaacgggacagagttgctgatttgctcgttgaatggcggcgttctgtgagtcgccgacatagatcccataacccttggcccctaccaccatcgccacgcattcgttggcatatgaggcttcaaccttgcagggcgatccaccattggttgcgcaatcggacaatgctgcttgctctgcctctcttttgcttgtcttgtcgacggcagtcccaagaattcctttgggcttatcgcctgcaatcgctccccacctgcgctcccactgctgaggcggaggctggggtgctcgttgctgtccatagcccgggatcggggagcaaacaatcgctgctgcccggccgttgttgtggtcgatggtgcccggtggacaaaacccaccctcggcatgcgcggcgctggcacacagcagccacaaacccacgatcagcagcctgtacaagagatgtgctggcatggtcacgccccatccacgttgagcgctcgcgctggtggtgccgtcgtcctggtggtatctatggaatcagtaacgggtggtgtgttgcccgcaatgcgggttgcagcactgccagggttgcctccatacccaccacgatcagcttgatttccagcatccactcctcgccccgcattcgtctgctgcggccccccaaaagtccccggcgcctgcccccccggcccctgctgcgcaccggccccgccaccgagcaccgagctcgtatagaactgccccagcgtccccccaaagaactgcgccgccgccgcaggcgcggtcaccagcagcaccgtcagcagcagcccgatgcccccttgcagcatcgcctggctggtcaggcccgtgcttccacccacgcccagaaagctggtgatcgccttgctagcccacagccccgcggcaatgcgcaggttcaactccagcaccagcgacaccatgaagctgagcaccgccatcgagaacagcagcccgatgccgtacagcagccacttgtgaaacagcgactcggtctgcttgaaaatcaggcacaggatgaacagcggccccaggctgatgaacagcgccaaccccacctggtaggtcagcagtagcgccccggccgttatcgccgggctggacacgcccagcgcacccacgagcgaggagacgcccacgctggtgacattggagccgctggtgctcacgtccaggccctgcgcgttgtcgatggccgacatgaccacctgggtgagcaccaggttcttgtcaatggccgagaccggtgattccttctcgccggtgaccatgtagttgatctccttgagcagaccatccgtgaagatcgaatgcaggtccgagcccccaagggccatggtgcttgcggcgatcacgatcaaagcgttgcggctcatacatgactggacgcttgcaatccatgcgccgaacattttgtttgctatcggatggatagccggggtcgcggtattcatgggcgttagcagtgattcgacttgtgaatggggatctcagcgagacatcgcaggcgccgcttgctgcgcggcctgctggttgttgtgctgaggggcttgctgctgcgcctgctgtacgactgtgaacgcctgtgagctttgcgctactggcgtgttcagtgccaccatcgtgtccactacgaccacctttgagtgcaccgctcccggtttgccctgcacggcgatgagcttgtcgccaggttcgttgggctccacatggtcaatccgcgtgagccggtgctgatgagcttccacagccaacgcagcggcggtattcctggtgctctggggatccaccttgatgtggtgatcgtgattccacttctgcaacttgtgcaacgcctgctcgtagagcccatgcccggggtgaccggcagacgtgatcgtcgctgcgctcgaacctgtcgaactcagcgccaagccgcccttcgattggagttcgcctaggtacttgttgctgtcgtccctcaactgaccaagaaatttgttgtactcggcagggttggtgttccatgccttgtagatactggcaacgtcaccggatttggccgttgcttttttatccagataaatggcaatgccgtgttctatgttggagttcaaatcaaagcgattgaactcgcccaacttgtgcccgttgatcctggaggttccatccaagcgctgatgcgcatccttggccgttgagtcggtaatctgaaaaacgccggatgccgacgactgatgcccgggcgttgctgcatccggattgaacctcgactcgaccttggcgatggcgatgaggtttgccgtgtcgcgatccggcagcccatacgtatgagccttgctgacgatcatgtcaatcaccttttgcttgacctcgtcggacgcgcctcctgcctcgcgggagaagcctccgacgcgaccgacggccgtgtcgatcggatccttgtagtggctgtggttggtcatgatcctctcctatttggttgaagtgactctgtcgatcgaaattgatttgtcctcttgagagtcgttgagcaggcgctcaagctcttttgagagtttcttgtgtggcaattgcagcgagcgcgtggcagactgggtagagccgatcagccttccgcgcgtcgtgtagacatccatccattcgcaggtcgagcaactgccaaagttagagctgtatgcaatgacatagaagtcgctttttactggattgcaactcaattggttaacaaacgactcatccatatttttaagaggcttcggagcgtatttgatagagatactgactcgggaatcagcctctttgaagatcagcttctgggtgcaatgaggtggagcgccgtcgctgctggcggaacaggcggtttgaatcaaaacctccgattcaccacaaaccagagcattcgcccttgaaggaggggaagtcgtttcccctgccaagctggataccgagaagcacgcgatcgtgatcagcgaaaagatcagagtggatcgaaggaggagcgagcgaacgaggtttgatgccccaatcgctcgtaagttggtaggtgggatcaaagcatccatggcgtggtccgagtttggctcgctattgaatccgaaccggcaggctgcaatcggtgtagtcaacctgacagctggcgtcaccagagcgttgacacttttgcatgccttcctggatggcgtcatctagttttggtttctgaatcgctacatacgaatggtcagaaactacgtaagcgatgcaaccattcccataccaagcttccatcttgcagttgatcccacccttcgcttggcagccgttcagtgcagcttgctccgccgtagcacggcttggcatttttgaagatgtgcctattgcgccttttgaagcatcaagataaatcgccccatatcgatccctccaaacctcggcgggctgctgaggtgctcgctgttgcctgttatccggcccgcacatgttgagaccgggacccgagccataagcaatctgcccgggagggcattgctgggcaagcgcggtgccgccccagaacatccagagacttgccaccagcagtctgtacaagagatgtgctgacatgggttacgccccatccgcattgagggcccttgaaggtggtggtgcagaagcagccctgatttcatcgtgtcggggttctgtcgaggtgcggggaggtgggagggatgtagttgtgggaacctgactcgattgcccagggatattcgccggctgctgcgcccccgccccataaggcccaggagctcccccacccggtgccaccgcgctctgaccgctgcttccgccaccgagcaccgactggtgataaaactgccccagcgtccccccaaagaactgcgccgccgccgcaggcgcggtcaccagcagcaccgtcagcagcagcccgatgcctccctgcagcatcgcctggctggtcaggcccgtgctgccgcccacgcccagaaagctggtgatcgccttgctcgcccacagccccgcggcaatgcgcaggttcaactccagcaccagcgacaccatgaagctgagcaccgccatcgaaaacagcagcccgatgccatacagcagccacttgtgaaacagcgactcggtctgcttgaagatcaggcacaagatgaacaagggacccaggctgatgaacagcgccaaccccacctggtaggtcagcagcagcgccccggccgttatcgccgggctggacacgcccagcgcaccgacgagcgaggagacgcccacgctggtgacgttggagccgctggtgctcacgtccaggccctgcgcgttgtcgatggccgacatgaccacctgggtgagcaccaggttcttgtcgatggccgagacgggcgattccttctcgccggtgaccatgtagttgacctccttgagcagaccgtccgtgaagatcgaatgcaggtccgagcccccaagggccatggtgcttgcggcgatcacgatcaaggcgttgcggctcatgctggccaccagagcaatcatcggctcgcgcgactggccggtgaggatgcggaagccctgaatcagaatccacaacgtgagcagcaccagggcgacggtgctgacccaggtcgtggtgaggacactgcgcacgcgcgccttgacccgtgcggccatctcgtcgtgcacgcgaaacaactcggctgcgatcaaatcgaaggctgatggtgtggtattcatggtcggtgagaggcgttggggctatgaaccaaagcgctgatgcgcgtgctcaactcacgccagagccggcccggtttgtgcctggactggccgattcacctgctgggactgctggttctgctgcaggctgtgcgcctcgacgaaggcttgcgagctttgcgcaaggggcgtattcagcgccaccgtcgtgtccacaccgatcaccttggaaagcgcggagcccggcgtaccttgcaccgcaatgagcttctcgccgttgtcgctcacggccacatgatcgatctgcctgaatctggattcacaagctgaagtggccaacgtgcctgcggcattgcaggtgcgtggatcggaggggatgccgcgctcgacgttgatcttctccagcccagccaaggcctgcttgtagagtccgttgccaggatgctggccatcgtccagcaacaacggcaccggtcctgtctggctgctgatgaaccacgaccctggacggatgcgcctctcgatcgcgcgggacgcgccttcgcgcagcgtttcaccggtccgctccaacgcctcgcctgcctgccgggcgcccgtttccagggagccgcgtactgcatcgtaggcctgccccgcagcatggccgacggccttcacgccgtggccggccatttgcccggcctgcatcccgctttgcagcggaacagacgcgatggcacgggcgccgtatacgtcgttgcggtagcgatcgatcatgccttgatgggcgtgataatgcgtttcgttctcgcgcgagatgatcgagcgacccagcgtctttccgtcgggcacgaagttgtcgatgaaatgcgcgctgaaatcggttgccttggcgggattgcgagcactcagagcgccgccgtcgtcgcggtacccggccttgcccagcgtgtcgatatcctgctggaccgcgtagacccgcacctcgccaaaatgcgcactggctgcgcttaccgcatcgcctgcgcgaacatggttgatgacttggtggccgcctttcggaacgccatgcaccagccccgcagcgccaaaggcgttgaaggtctcgcccttgaggccgaacttgtgggcgtgaagttcggccagagtgccgcccagtgagtggccggtgacagtgacattgagaggctgattgctcttttctgcatcggcctttgccttgtccagcaccttttgcgtgaaggcgttcgcgtcaagtgcctgggcattgacgcccgccaatgccatgccagcatcgacgaggccgtcttgcatcggctcgcggccaaattcggtaccgcgaaaagcaatgaccacctcgcccgtatcgacccgccggtaggccgttgcttgaaatcccgtcctcgggttgtcggcatggtccaggacttgataagccacatctcccagggtgacatcctttttttggagctcgcgatccttgtacgaatcctgtgccagcagtgcgtaatccgtggacgtgatcgtcattggaatttctccttggcagtgagcgtcatcgagaaggtgctcttcggctctttgaaatcagatcgctgcgcattgccgctgttgacccatggtcgctctccgtctttcaatggagtgctttcgcggtacgacaacgtggagaaataacgcgtggcggacttgttcgccaagatgtcattcagggcgatggagtggccgaacaccaagttgccgatccgcaggctgaagttggcgaagggcatggaccagcggcaaaggcccagcccgaagtagtcctcgtccgtcaacagatcgacatagagttcacccttgtagaccttatcgctcacgcggctcagggccatccagacatccttctcgggagtcagcgtggcgccgctgaaaggggcgagcggtacgcaaccaccattcgctacttcatagccagcggacccctccacggcatcgaacggcccaggcgcatcctcgatggtcagggtgatttcgtagcgcatcttgggatgcgggttgagcttgatatcgggttgtttcatggactgtccgcaagcggagaaagtgagggtcaagagaatgaagagggagatagcaaaaaagcgcttcatggctatctaaccctgcaacgcgcatgagctgcgcgcgagtcgctcgaattggtggcaattgatggggtgcatggcaactaccgaatacgcacgggcaggctgcaggcggagtagtagacgtggcagttggtgcgcccagcatcacgacatgtcttcatgcccaactcaacggccctgtctactgtggcggcactaggtacgttgtagccaccatcgcctacaacaaccgcggcacactggttgtaatacgcagtgtcaatcttgcaattcaccccgcctttagatcggcaatcctgcattgccacttgcgaggcttcctgcttgctccgtttgtcggtggttgcgcccaaagcgccatttggcccgtccgttgcaatcgctccccatcgacgttcccattgctcgacgggttgctgaggcgcttgttgctgcccataccccgggagcggcgagcaaacaatcgctgctgcccggccgttgttatggtcgatggtgcccggtgggcagaacccgccctcggcatgtaccccaaagctgaccatcagcaaacccagccacagggccgccgtacgtagcgcggccctcatcgcgcttctccgtcgatattgagagccttggctggaatagacgcgggtctgatctcatccgccgggggctgtgatggcgtggacgctcgagcgccactgagtggaccattgacgccagtttgatttggattcgccgtatccgtcctgctgggggcaggagcccccgcctcaaaagtccccggcgcctgcccccccggcccctgctgcgcaccggccccgccaccgagcaccgagctcgtatagaactgccccagcgtccccccaaagaactgcgccgccgccgcaggcgcggtcaccagcagcaccgtcagcagcagcccgatgcccccttgcagcatcgcctggctggtcaggcccgtgcttccacccacgcccagaaagctggtgatcgccttgctagcccacagccccgcggcaatgcgcaggttcaactccagcaccagcgacaccatgaagctgagcaccgccatcgaaaacaacagcccgatgccatacagcagccacttgtgaaacagcgactcggtctgcttgaaaatcaggcacaggatgaacagggggcccagactgatgaacagcgccaaccccacctggtaggtcagcagcagcgccccggccgttatcgccgggctggacacacccagcgcaccgacgagcgaggagacgcccacgctggtgacgttggagccgctggtgctcacgtccaggccctgcgcattgtcgatggccgacatgaccacctgagtgagcaccaggttcttgtcgatggccgagacgggcgattccttctcgccggtgaccatgtagttgacctccttgagcagaccgtccgtgaagatcgaatgcaggtccgagcccccaagggccatggtgctcgcggcgatcacgatcaaggcgttgcggctcatgctggccaccagggcaatcatcggctcgcgcgactggccggtgaggatgcggaagcccttggtcgggatgatgagcgaacggaccggtgttggggtattcatgggcgctggcggtgacttggctgatgaatgagaggctcagcgagccatcgcaggcgccgtctgctgtgcggcctgctggttgttgtgctgagaagcttgctgctgcgactgctgtacgactgtgaacgcctgcgagctttgagcgaccggcgtgtgcatcgattccgccgtcggcacatcgaccaccttggagagcgccgctccaggcttgccttgaatcgcgaagatcgtgctgttgtcgttgccgcccagcgtcatgtgatcgatgcgggtcaggccgccgcgcaaagcggccaccgcgatggcggcagcggcgttgtcggtcaactgatcgggctttcggccgaactgggcatcgattttttcgaggccggacttggcctgcttgaacagcgggctgtcctgcagcgactggccgggctctggatcgccaggcttgtagccgtgggcgagctttgtttcccactgcgtggcggcggccttgcgttctttaagggagttttggccgccgttgatgtcctcagtggcacgggtgatgtcgtgctgatggccatgggccaccacgcgttccttccaatactgcactgcgatcttggccgagttcgcgggctctgaagccaaatcggggtgattcacgaggtccaggccaagcgccttgccatagcgctcgtagttgtagcggcccgtcaattgaacaaagccgcgaccgtgatacttccacccatcgcccggttcattgttgccaagatcgcggcgacccccatagatggcttcagccaccttctccgagccacccgcggcaatggcgctggcgtcttcctgggtcatccctgggtgccgtttgtgcagagccttgaacacgttttggcccgaatagcgcaggttttcatgcgctttagtaaagccatgcgattccacctgcatctggcccatgaagttggccagctccttcgcatttgtgatgcccgccccgtgcgcggcctgcaacacgaagtcgccgttttctttggaatacggggctgcgtggtgtgcgttgtgtggatgcgatgcgtgacgagttggacgttgtgacatggtgagttctccctggatgaatcgaacttcagcgcgtgcttggcaagccgtgggcttcgatgtctgcgtcgaccttccattcggatgtgatgcgtaccagctcggtgtctttcgtctccaccagagtcgacggccggcacgccatctcccgggctgcacctagctgaccctcgcgctgtaccaacaagcccgagcggtcgttggcgccttcaatcgaatagaggatgtacttgtagtcctcgtttctgagcgagtgggcatagccaaacgtgccaccggcatagaacaggcgcgtgaacgtgaaggcctcatggctattgccgctagccggatatctcagttcgatttttgaaggtcgcccatacaggtaatggaagtgcctttcaccctgcgtcgatgcaggcgatgcgcacagcgaaaccatcttgcggctggagccttgcagcgtgcaagagaacaccggctcttcgttggccgcgcacaagctgggtgcctgcgtctgtgcccgcgcgctctgcgcaaaggcatgaaggcaaaccagaccgagagtggcgccggtgagaaatgaggcgatgcggttcatgaagtatttgctatgaaaaattgctagttcgtcgccgctttatccatgggtgttggcagcatgcagcagtggcaattgcaagaaaaatgaagcgcactgcgatagggcgcctcatggtggctattgaatgcgcactggcgggctgcaagcggtgtagtaggagcggcagttggtgaatccaccgccacggcatgtctttacgcccgaggcgacagcttgatccactgtcggggcattgcctacgttgtaggcgccgtcgcctacgacaacggcaacacattggttgtcataggtaatgtcaatcttgcagttcacgccgccttttgactggcagtcccgcatggctacttgtgacgcttctcgtttgctccgcttgtcgatggctacccccaaagcgtcattgggtccgtctgtcgcaatcgcgccccaccggctttcccattgcggtgctgattgctgcggcgcttgttgctgtccataccccgcgatcggcgagcaaacaatggcggccgccctgccgttgttatggtcgatagtgcccggtgggcagaacccaccttcggcatgcaagaggccattccaaagcaaccccgccactatcatcaagaacgctcgtgccaacgtcttcatcatgcttctcctcaaccttgagtggctttggtggcgggggtaacggatgcggctctgatttcatcagcaggtggatgcgccgaggtgcgattgagactgccaccgagcccgccggtgctgcctgtttgattcgatgttgtttgcggcgcttgcccggccgtcggcgaaaaagtccccggcgcctgcccccccggcccctggtgcgcaccagccccgccaccgagcaccgagctcgtatagaactgccccagcgtccccccaaagaactgcgccgccgccgcaggcgcggtcaccagcagcaccgtcagcagcagcccgatacctccctgcagcatcgcctggctggtcaggcccgtgctgccgcccacgcccagaaagctggtgatcgccttgctcgcccacagccccgcggcaatgcgcaggttcaactccagcaccagcgacaccatgaagctgagcaccgccatcgaaaacagcagcccgatgccatacagcagccacttgtgaaacagcgactcggtctgcttgaagatcaggcacaagatgaacaagggacccaggctgatgaacagcgccaaccccacctggtaggtcagcagcagcgccccggccgttatcgccgggctggacacgcccagcgcaccgacgagcgaggagacgcccacgctggtgacgttggagccgctggtgctcacgtccaggccctgtgcgttgtcgatggccgacatgaccacctgggtgagcaccaggttcttgtcgatggccgagacgggcgattccttctcgccggtgaccatgtagttgacctccttgagcagaccgtccgtgaagatcgaatgcaggtccgagcccccaagggccatggtgcttgcggcgatcacgatcaaagcgttgcggctcatgctggccaccagggcaatcatcggctcgcgcgactggccggtgaggatgcgaaagccctgaatcagaatccacaacgtgagcagcactagtgcgaccgtgctgacccactgcatggccctgcccatgaaatccgtgccgaagtcgctgattcggctggacagccacttgtagatcagaccgaaaacaaaggcgccgccgctggcatcaggcacttgcgcatgggcgacgcccatcggcatcagggcgaccatggccaaggctgagcggagagtaccgcgcgacaggtgtggatgggcttcaatgtgttgcgacatggggttccctgagggcaggttgtgctcggtgcaatggggcaacggctacttgacggccagggccgcggcaatggcggcggcctgaacgagctggcctgcattcatgcggccgaagctgtcggcactggcacccccgctcccactgcccttcatggcggtcttggtgagggtgttctgctggccttcgtggaatttgatggccgcgtcgtaggcatcgatacgggtgcgccaaaagcccatttcggcttgcagcttggccgtggtgcgggtggcttcgttggtgagggcttgcacgtcgccatgggtgttgctggaagtgcgcttgttgtcgatggcggtgagctgctggccgtattgctcgaagcggttggccatgtcgatggtttcgttgaaggactgcacgcgaagctgaatgagttcctggcagattttttgtgacatgtcgctgccgccggttgcgctgatggtggtcaggctggtgaggggctggctgccgactcccgcactggccccggcgacactgccgctggaactggggcaggcttgggagatgtagccggagacgtcgccgattttctgaagcttgttgttgggcgtcagggtggcggtaaagccgaggttttgggtgctgttcttgagctgaccgaggatgtcggaggcagattttttgatgtcgccagtggtcgagtcgatcttgtccagggatttttcggcgtccgcgtctttgacatccacttgcgcatgggcggcacccatcagcacccaggcagcgacgactagagcgcaacggattgcacggcgtggcaggaatgggcaggcttcaatgtgttgtgacatggtggattccctttgggcaaagttgtcgtggtgcggcagttggtgcgggcctgaattcaatgctcggtgcacttgtggttttcgtggtttgccggttttttgaccggcagtgcgagcaagaagcgaaagaatctgctgctgacacgccaccacagccagagcatcaggactgcgaacactgccaagccaagcatcatcagaattcgaccgagtgaatccgcggcaaattgagaaagagtctcgggatggatgaagagctggtagatcaccgagcagcaaaggacggcaacgatttctgctcgccagctcagcaggtaggggcgtagcttgttgttcagtggggctagcatcgcgcgtgtccagatgggttcggatggttgttcggggtgggtgtgtttttggtgcccgcgcttactcgacccggccccattggttcatgatggtgtcggaaatattgctgttgttctgggtgttggtggcgccagagcagctgttcatgtactgcttgcggtactcgtaggactggtcgggccagaatttggtaacggggtagtaggtccagatggccaggccaccgggggccggtatgtgccaataggcaatggcggacgagcagttgccgggaggtgtgccttggccggagatgctcgccatgcagaggtacagggtgcaggcgtctggaacctgggcttgtgcggatgtgctgaggctggcgatcccgagcgcaagggaaaagccggccaaatgggtgcgtagcctcattgaaaacctccgaaatattgaagcgatcgtcgaaagggtgtgggggccggtcatgcaatgaggcgcggacgcgccgagcgctggccgggctgttcggtggacgcggaggcgcgcttgccgctgcccttgcgctggtcgtagaagtcctgcaaccattgctcgggccggaggtcgttgacggagatgccttcggctctggcgctcccgtccagcacgccgtgcaggatctcgatgttgtcggtggaggctgaaatgacggccagcgcgtcgtccatgccgcgcaggtcgagctggcacaccgaggacatgtggccctgcttgacgagaaagcggcgcgagcgctcgtcgaggctgaccaccacctggtattcagactcggtgagcttcaggccctcgatgtagtccttgcggctggcgttggggttgggcagcaggatcatggtggcggtctgctcgatgagcgcagccgagatgtcgctgcccagcgcgtcttcggggctctgggtggcgaagatgcccatgccgttctgtttgcggatggtcttctgtttgttcttggcaaagtccttgagggcgccgccgccgtcgagaattttccagaattcgtccatcacgtaaatgagtcgacggccatcgatcagggcgtcgagccggtgcagcaggtagttgatgaccgggacgcgcacctcggggttgtcgatgacatcggtgtagtcgaagccgatgatgttggctttttgcaggtcgatggtgtctttggggttgtcgaacacccagcccagcgagttgcccgcggtccacttgcgcatgcggatgaagaggccgtcgtcgcccatgttgggcaggctcttctggaagttggtcatgttgcgcagatgctcgggggtgtcgagcatggcttcgacggcgcggaagatgtcgtcttcctcgcgcgaggtatagaccggcttggcggccagcaccttgacgaggtcgctcaggaactggacgttggcctcggtgcgcgcgcaatgaaaagggttgaatccggtgggctggccgttttccagcgagaggtagttgccgccgcacgcgcgcacgaagatctcggcgccgcggtccttgtcgaagaagaagatggtgggcgacgggtcgagcttctggatctggctgagcaggaagttgatgagcgccgttttgccggttccggacttgccgatgacgatggtgttggcaatggccttctcgcccagggaattctcgcccggtagcgtggcgtgaaagttgaagaaataaggctggccgttgacggtctgcagcgtggtgacgcacgggccccaagggttgttgtcgcgcttgccgctggcaaagttgtggaggggcgacatgcccaaaaagttgagcgagctgacgttggccagccgggtgcggtatttccaattgccgggaaattgcgcgtagaacgcggcggtgacggccaggtcttccttgatcgagacgaagcccgcgttggagagctcggcgcgcgtagtggcgatgtgctgggaaagcgtcgcctggtcgggcgcgtagacggcgatggtgaagtgatactggcccagcacaaagttgccggacgaaatctggtccatggcctgatcgagctcgacgatttggctgacggccttgtcgcctgacgaaatcatcatgcccttggtgcgctcgagcgccttgagcgcgtcgtgccgccccatggggctgaaggaatgggtgacgacgtattcgaagtcgaggtacttgagcccgttgaggatgccgggatgggtaccgtcgggatattccttgacattgaggatggcgccaaagtggttgacgccgttgggtgtggtcagcacgaagtcaccggtcttggccgagaagcgctggcggctgacggccaggtagcggtagacgggcgccttcagcaccggcacgggctcgtcgacgcggttgagcagatagccgaagaattcgagggtttcagaaaagacgatgccgttggtggcttcgtacatgcgaaggcgcgtaggcgcgtagtccttgagcacggcctccatgttgccggcgagttcaagtaccttgtcgatggcttgttgttgttcggaggtcagccgagagacatcggcggacttttcgacgaaacgtttgcccgagaccacggggcggtacagcatcgtcacgtagagctcgttctgcatgagcttttgcgccgagagccctttgaagtacgcgtcggacagcgattggttgaaggcttccttgaaccggctgctgtccttgacgtgccggcggcggcgcaggtcgtgcacccagaaggccacattggtgaagtccggcgcgcgcatcgtttgcagcatgcggttgaaggtgttgtgccgatgctcgagttcccattcttcgcggccgacgaagggcaacccttccagtcgccaggtcaggaggtagtcgccacccgtggtcttgagcacggtaggagacacgtgcgtggacagcgggatgaattcgctgatgggcgtgtcagggctgaagggcggcgtggacatggttgtggaacccggcttcttctagacgttgtctctggactgcccgcggtacacgttgggcgtgaacacccacatgccctcatgctgtccgatgttgcgcgtgcggatacggaactgcaggcgcagcccgagcagccggaagatcatttcgtcgcgcttggccatcatgcgcatgatgaaaatgaccggcgggatcagcagcaaatagaacaggttgaagtacatggccagcaacatgcatccgcccgcgcccacaaaaaagggtacatagggcacgcccatgaacatgggcgggcgggtgcagccgcggaacatcgcgtttttatgcatagtgggccagcgactgcacgatgccggcgagttgggtcaagggatcgaccgtgatgctggccgagcagctggtaccgccgccgacggtggagctgccgccgagaaacagtttggcgatctgggtggccgcgccaatcagcagggcaccgatgaagactggggcaacgtcgctgatgcgcttgtgggcgaatgcaatctggtagcccgagaaaatgatggcgacggtgaccaccacgatggacacggcgttgagcacgccgacgatggttttgacaaaaccgcaggcggtttccccgagcccgccgtctgccgacccctgagccatggccaggcaaggcaagacgatcagcgcggcaatggcgagattgcgaagcgctcgcgcgtgcgtgctgctggcgaacgatggagcggcggtgttgttgtgttggcggtgcatggtgagttcctctctggttgaataaaagtgaagggccgggttagaaaacaaaggcgccgtcgccgccaggtcggtcggtcggagcggcttgtaccgctgcggctggcacgtggcccgcgcctggatagtgaatctggggcacgaagacatcgggggcgcccgcaggtgcgcccattggcgaggcgggggcatgggtagctgcagctgacaaggcaacaggtgccgccgctgcgctttggggaacaacgggcgcggcagtggttgcaggggtggtaactggttgcgtggcagcacctagcggaaccacgcgcatcgagatgcgcgatgccgcggtggtggattgcgctgccgcggcggatcgggcgccgccaggggcaggcatggatgccggtgcgagggcgtccggcggcgcgccggccggacgcagggggatcgcggcgcgcggctcggccggtgtttgtgagagggtgacgccgcggctgatcgagtcgtagactttctggacgtagccgcttcgaaacccgcccacaaaattgccggagtagtagcagctgaaggccttgccccagtcgccgccggctcgggcatggcagttggccaggatgctggcaccggcggccagattggcgcaaagatcgaaggctttctcgtgggtgtctaacccgtacttgcgaaagttgacctgattgacttgcgctgcgccaagcgaatagttgtagcccttggacttgagcatttgcgccgtggccactgcttcttcaagcgttttgggctggcgcacgagttggcctccgacgacgccgatggcgaacggattggcgccggactcgacatgaaccacgtgtcgcatcacctgtgccggaacggcgaggttggggcaagcgatggcttccattcccgggaacacgatgtttgctccttttgcttaggaggcgccggcggttgccaggcgaccagggtcgaaatcgatacccgtgatgtaccgccgccccgcatgggccttgatgtgcacgatgatgtcgatggtcatcatgagcagtcgcttgatggtggcgaattcgagcccagcgccttcgctcgaggccttgaccatgagtgccagctggtcccaggtttgctcggtgctgcccgagtggcagctcgtgatggagcccgggtggcccgaggcgcagttgcggatgaaatagaacgcctcgtcgccgcgcaattcggccaggatgatccggtcgggcttcatgcgcaggcacgcttccatgcacgtcttggcgctgatgttggcggtgctctggccgcccttggagtaaagcaggtgcaccacgttgggctgctcgatgaagagttcgcgcgcgtcttcgatggtgaccaggcgctcatcggacgggatgtgatgcacgagcgacttcatgaaggtcgtcttgccgctgccggtagcacccgagaccacgatgtttttcttgtggaggacggcttgcttgaaaaagtccgcgtagcgccctgcggcgcgcagttcgagcagttccctgtcgtgcgcgttgaggcctgatgtttcttcgagcagcttgtcgaaaaatccgtcctcgtggtactggcccagggtgcgggtctgcctggacgggagccggatggtgatggaaacctggctcgcttcgacggcagggggaatgacgaactgggcgcgctggccggtgggaaaggtcagcgagacgaccgggttgacgtcggtgatgcgctgacccgtgttgctttcattgaccacggtggtgcagaactgcagcgcacgtgcggcggtgaggcccggcacctcgacgcgttgccagccggaacggttttcgaggtagatctcgccgggccggttgatgcagatttcggtgacgtcgggcgagtgcatgaaatcccggatgcccagcacctggtattggtaatccagaaattcgttcgagacggcggcaacgagttcttcggtcatgtaaagctatgccgtgtcagaagttcgccaccacagcgctgaagtcgacatctttggcgacgtagacgttgacgacggtgccctggttgatggtgactgtgtcgggccggttggcgttgcggcgcacggcctggctggccaggctctgcaacgtctgcgccgtggtgctctcgtaaggcgactggactgcgagcccgcccgctgcaacggtggtcgactgcgggccttgctttgccagttgatatttgaaggcgtcggcgaacatgctgatcagcagggccgaagtgatgcgttggccccagtgctgatcgaggtggcccggatgacccgagccaccgaggttgtcgacgccgggactggccatgttcacatcgatcccgttcggggtgacgatgcgatcccagatcacggcgatgcgatcgccattgggttcggtgtcgtactttccaagtaccttggagcccttcggcagcagcaggcgcttgccggtgacggagtagaccggctcggtgacgacgcaggatgtgaagcccggaatgtcgctgacgatatgcgtctccagcacgcagcggatgtaggtgccgcgcagcatgagcacgttcggatggacaagggcttgtgcgctcgatacggccgacagcggcttcatgcgataggcgctgttcggcgcgatgccctggtcgccgcccgcgccgggcatgccggccatgcctggcgccatgccgggatattgaccttgtccgggctggccaccatccgtgggacccactgcgatcgtgcccgcgctcgatgccatccggcgctccatgagcgtcggaccgtgcggtccttgtgggccttgcggtgcgggcggaatcggcggcagcgatggctgggccaacgggatgggtggggttggtggtgtggcaacccgtggcaggggtggcggtgccggcagttggggcgctgcagggaccgtaaccacttcttccttggctttttgtggcttgtcggggcgcatcacgttgccgatcagccagatggcagccaacccgagcagaagcacgatgcccgcgaggaacccgagggcgcggcgattcatgcgctgcatttcgctggatttaagctccggcgcgtgcgcgtctaggttgggtgcggcggtcgctcccatgccctcgaattgcctcgaatagggattggcttgaaaagcaggctggctattgccgtccgtgggatcttgccgatcgtggtcaggcacggcgtctcctggtcgggaaggaggatgttggttcactggacggtgttcctgcgaagacccacgacgttgtcgccgtggcggatgaccaggtagggataggtcccatggacgatgagggtgctgccttcgacggtggtgttcaccacggagtcttcgtcgcgctccttctgacgcatgtagacggtcgggaagttgcccgtcgggaactgcttgaggtcgctcatcttgatgtaggtgaagcggctgtcgtcgtagacattgatcggaaccagccaggctgcgccggcgctgctggtggcaaagtcgtactcgaagttgtagctccggtccttgagcagcgctgtattgagcgcgggcgcctcggcgacgctttttgcttccttgccgaacgtcatgtcggcgggataggtgaacttgatccggtactggacacctgcattgcgcgcctgctccagggttcgccagtcggtggccacgaccttgagttcgaagatgtacgaattgatcgcagtgcggatcatcatgttggtgtccacgtcgacgttcttcggcttcaggtagaagacgttgtcgcgacgactaaggtcccagccactgctgaagccggtgctgtagtcgaggattttttcttcggggctcagctcgatctgggtgctgattcccaagccgacacgcaccgggtagatgcggtcgggctggtactcgtacatctggacggtttgcgcaaaggcgcagggcatggcgctggcgacgactgcccatgctgcggacatcagcgcccgtcggcggtagttggactgttgtgatttcatcggcggcgcgttccctgattggcacttgtcggcgcgacggctggagcgacgggcgcgggagcgcctggggccccgaaaccgggtggaagagggggggggtggcatggcggtttgcgcagacggagccaccgcttgggcactacctaccgcgccggcaagggcatcggtgcccggcgggagcgccgcgccgggcatcgcgggcatgctttcggcgggcttgagattgcttgggacttcttcgggcggcgatgacgcgtagtcggtatccacgcgatagtcggtaacctggaagccgagtggattttcgatccgctgctgctcgtccatcgtgaggttcgacttgtaggtgaacgccatcgtcacgatcttgctgtccagaggcgccgaggagccgttctgcttgttgtagacgctgcgctggaagcgcactgtggcgcccttgggaacttcgccgcctccgccaccgatcagggtgatgctcaggatgcggacccggatggctttgtccttgccgtatatggtgtacgggttgatgggatttcccgacgaatacaagttggtatagccgccggagacgttgcccgacgacatggtcagtaccgtggtccagtcgcgcaagttggtgatcgcgaggtcgtaggactcgcgggccagcacgaagtgggcaacgttgctgcgattgatcgcttcgctcgtggtgatgcgctgcaaagccgcgtcatcggtcaggcgtgcggcggtgctggtgcctgtgtacgcatcggcgatgaccagatacggcactttctccttgagcggcagcacgtagaagtagccgcccagcagcaccagcgacatgactacggcagagcccgcaacccaccaggcgcgccgttcgctgcgtcgcgcgatgtccgcaacagtgagttcgaagttgaccgattgactgatcgtttggtcgatcttcgaggtcgacgcgttgttcttgaacatcagcgcggcccggttgtggccggcgcagcggcgcttgtggcctgaaccaggatttgtttgccgtccgccgaaatggacacaccctgcggcgagtagatggcgctcagctcacccatggctgactggaggtcggtggtgcgaaccttcgctacaggttggtggagggtgaagtcggaacctatttgataggacaactgcagtccgttgtccgacgcccagcgcttcagcatggtcctgagcgtcgcgtccatgggcgaagcgtagaacgtataggcgggcgagagcgggatctcggtaatcgcactctggaaccggttcaccggcgcccaggagccaccatactccttgggtgcaggcgcaccgcacccgatgagcgtgaccgccagaatggacaaggccgtacccgccgaaaggcggtttgtagcgcgcgcacgagcgccccacgcaatagcctgcgtttggttaaacactgcgactccctgaagtcttttttatgtccgcctatcttaggtagatgaggcggccgtgacagcacggcgctgtgcaggagtgcacgaatcggcgggatttagtgccgcatatcgttgaggcggcgaaacaccggcttgtccgcggagagggtgggttcctcgtcctcgtggattcggccgggttgagacctcggagcagaggcgcaattcgtcgacgtcgggcggggcagtgatggcccaccgagaccagggatgagtccgtttcaatgataatagttctcattgctgagatgaacgagttccaacccgcatgaccatccctctttccgtggccgctacccctgtctctatccgtctggacgaattacccagccatcagtgggcgacggtattggacgtcgtgcggtcggccgatgccgaggggcaagagttggcactgcgcctgaccgagatcggcttcgtgcccggcgaagccgtgcgcatcgtagctagcggcctccctgggcgagagcctctggcggtgcggctgggccacaccacttttgcattgcgccgccacgaggccgcgctgattcacgtggcaccgggcgtgccggaaggcgcacgccatggttgaagccgtcatccagaggccggggcgccttgcggccaccgcacagccggggcgcattgcgctgctgggcaatcccaactgcggcaaaacggcgctcttcaacctgctcaccggcagccgtcaaaaagttgccaactacgccggcgtaacagtcgagcgcaaggaagggctgctgcgcaccgcatcgggccgccgcgtgttcgtgctcgacctgccgggcgcctacagcctcaacgcgctcagcgcggacgaagccgtgacgcgcgacgtggtcaccggcaagagcagcgagccattgcccgatctgctcgtgtgcgtgaccgacgccaccaatctgcggctcaacctgcggctcgtgctcgaggccaagcgcctcgggctgccgatggtggtggcgctcaacatgaccgacatggcgaagaagcagggcatcgccgtcgacacggcggtgctctcgcgcgaactgggcgtgccggtcgtggagacggtcggcgtgcattcgggcggcgcacagggcctgctcgaggcgctcgattcgccggtggccgccgccgcgccgcagcagccctggcaggcgccggggctcgacgacgtgctggccacgcagcgcgaagtgcgccgcatcctcggcatcgccgtgcgcgagccggtcggcagcctggccaccagcgaccgcatcgaccgcgtggtgatgcacccggtgtggggcatgctggtgctcgcggtcacgatgttcctgatgttccaggccgtgttcagctgggccaacgtgccgatggacgccatcaaggccggcaccgaggggctcggcgacctgctcaaggcccacatgcccgaaggcatgctgcaaagcctgctggtcgatggcgtcattgccggcgtgggcggcgtgatcgtgttcctgccgcagatcctgatcctgttcctgttcatcctggcgctcgaagactcgggctacctgccgcgcgccgcattcctgctcgaccgcgtgatgggcacggtcgggctttcgggccgctccttcattccgctgctgtcgagctttgcctgcgccattcccggcgtgatggccacgcgcaccatcagcaactggcgcgaccgcatcaccaccatcatgattgcgccgctcatgacctgctcggcgcgcctgccggtctacgcgctgctgatcgcggccttcattccggcgcgcaccgtgggcggcgtgttcaacctgcagggggtggtgctgttcgcgctgtacgtcttcggcatcgtctcggcgatggcggtggcctgggtgatgaagcgcttccgcgacaaccagcagcattcgccgctgatgatggagctgccggcgtaccgctggcccagtcttcgcaaccttgctgtgggtttgtatgaacgagcctggatcttcctccagcgcgtgggcacgatcatcctcacgctcaccatcctgctgtggttcctgtcgacctttccgtcgccgcccgaaggcgccacggggcccgccatccagtacagcctggccggcatgatcggccgcgggctcgaacacatctttgcgcccatcggcttcaactggcagatttccatcgcgctggtgccgggcatggcggcgcgcgaagtggcggtgggtgcgctcggcacggtgtatgcgctctcggccaccggcgacgacgtggcgagccagctcgaaccgctgatcgcgggcagctggtcgctcgccaccgcgctctcgctgctggtctggtacgtgtttgcgccgcagtgcatctcgacgctggcggcggtcaagcgcgaaaccggatcatggaagtacgtctggatcatggccggctacctgttcgcgctggcctatctggcgtgcttcattacctaccgcgtggcggtggcgttgggcgccggatgatctgccgcaagtcttgcacgatgtttctgggttagtctcgaacgcgcgtcggagtaaacggatatgacacagcaactgatcgtcggattgattgtcgcggccgccgcgttctacgcggtctggcgctggatgcccgcgggctggcggcgcagcgcggcgcgcaagctcgcgacgggcacgcaccgtgccgggctggtcgaccaggagcgcgccgaccagctggcggcctcgctggccaagacctcgggctgcggctcctgcgacagctgtggcagctgcggccccaaggcagccgacaagaaggaatccgacgaagccggccgcggcgcgctgtccacgcacagccgctgaggccgatgcccgcacacatcctcgtcgtcgggggcggcatcggggggcttgccagcgcgctggcgctctccaggagccgccaccgggtcgatgtcttcgagcaggcggccgcgttcggcgagatcggcgccggcatccagatcggccccaacgtcacgcggcgtctccatcaactgggcctggccgatggccttgcggccgttgccgcatgccccgaggcattggtggtccggagcgctggcagcggcgccgagctggcccgcctgccgctgggcgatgccatgcgacagcgctatggcgccccctatctttgcgtgcatcgcgccgatctgcattcgctgctgctcgaagccgtgcgcgcgcgtggcaccggcaccctggtgaccgatgcgcacatcgcggaggtcgaggtcggtgacgatctcgtctgcgtatcgagcagcggcgcacgggcctgggagggcgaggcgctggtcggtgccgacggcctgtggagcgtggcgcgccagcggctcgaatcgccatcggcggccgagccgccccgcgtcaccggccacacggcctggcgcgggatcgtcgcacaggccgccttgccgcaagcattgcggcgccaacggatcgacgtgtggctcggcccgcgcttgcacgcggtggcatacccggtgcgcggcggcgcctggctcaacgtggtcgtcatcgccgaagccgcaccggccggcgatgcgcgcgactgggaccaggccagcagtctggccgcgctgcagcaggccacgggacgcagcggcggcggcctgcaagccttgctcgaagccatgcccggctggcgcgcctggacgctcagcgaccgtcctccggtggcttctgcagccgacatggcgcacgagcgcgtggcgttggtgggcgatgccgcgcatccgatggtgccctaccttgcgcagggcgccggcatggccatcgaggacgcggtggccttggccgaagcgctcggcgaaggcgcggcggccgaagtgcctgccgcctttgcccgctatgccgaggcacgctggcagcgcaacgcgatggtgcaggcaagggctcaccgcaatgggcaggtctttcatgccaccggtcccatgcgcctgggccgcgatctggccatgcgcgccttgggcgcacggctgctcgaccagccctggctctacggcggctgacggagctgcgccgggggttctcagagcctgaacgtctgcaggtgctcgatgcgctcggccaggccctcggcaccgaggtagtggccgtgggagccatcgcgaacctcgagcagcgtcgcctcgagttcggtcagcattgcatcgcgctcggcagcgaatgcgggctgcacgtcgatgcccgcctgcgtgcatgcatcggcaatcaggtgcgcgcttgccggcgcaccgcaggccgcacaatggacgatggcggccacgctgggctccgccccgttggcgagcagtgcgctcgtgagttcgggcgaaatctggccgtcgatgttgcgcaaggcatcggccgccaccggcgcgcccgcgcgcaccagcgccatggccgcggcgaaggcgtccttgccgatggccacgtcggtggccagcgcgctgccttgcagggggccgtcgaagctcacgcccgcggccgcgagctcggccaccaggtccgcatcgtcggtggctatggcatggtgcagcgccgcgcgtgccgtggctggcaaccggcgcagcgttccgtcggccagcggtgtgcgccagtcgatcatggcctggcaatagaagctcaccagcttgtccatcaggtcgagatccaggccgtggtcctggtgcctgtcgtcgaggtactgcagcagggcctggcccgagaaatagtcgctcgtgggggccagcgggttttcgtcgaggtgcagggccgcaaaagcgccgcgcagatcgggtgcgatggtgctcacgccgtcttcgtgcagcgcatgcgtccaggccggcggcagtccttgtttccatgcggtgatgtgcccgtgctgcgggccgggctcgaccaccgcgtagacgcggtcgaggtactcgaagccgccgaagggcaggtgcgtgagcttgccgctccaggggcggctttcttcttcggcggcctctttggccaactcctgttcatggccgatccagccctgcagatcgcgatagccgtcgctgccatcccagaacagctccgaccagctgacggattccacgttgccgttcatcagcagcgacaggtcgtagtcgagccggccgccggccgtttgccgccacagcgtggccagcgcctcgggaatcggccccgcgcattgcgcttcgatcgcggcaaggcgcgactcggccatgggcggttgcgcatcgaagatcacgcggtccgcgaacaggaccacaccgtgttcgcgcaggtttgcaagctcttcgagcgtgaactggacatcgttcatggcagtgcctccgttgttgccaatgtagcggtttgtgcaaacgaggcaacaacccgcatcaaagatcggtgcggagcttccagatttcggggaacagcaccacgtcgagcatcttgcgcaggtagctcacgccgcccgtgccgccggtgccgcgcttgaagccgatcacacgctcgaccgtggtcacatggcgaaagcgccagagacgaaaagcgtcttcgaggtcggtgagtttttcgccgagctggtacaggtcccagtggtcgtgcgggttgcggtacacggtgagccacgccgcctcgacgccgtcgctggcctcgtagggctgggtccagtcgcgctccaggtggtcggcgggcaccggaaggccacggcgcgcgagcagcttcaatgactcgtcatagagcgaaggcgaccggtaggccgcgtcgacctgcgccagcagatcgacccggtgcgcatgcggcttgagcatcgcggcgttcttgttgccgagcgcgaattcgatgcagcgatattgcgcgctctggaagccgctggagttggccaggtacgggcgcattgccgtgtattcgggcggcgtcatggtcgagagcacggtccatgcgctcaccagctgttccatgatgcggctcacgcgcgcgagcatcttgaaggcgtcggacagcttctcttcggcgatgtggcgggtggcggcgcgcagttcgtgcagcatgagcttcatccagagctcgctggtctggtgctgcacgatgaacagcatctcgtcgtgcgcgggcgagagcggatgctgcgcgttgaggatctcgtcgaggtgcaggtagtcgccgtagctcatcgacttgctgaagtccagctgcgccttctcttcgtgaacgattttttcggtgctcatgatgcttgctggccggttatcgcgagactacggcggtgtaggaggggcgacccgggatcgagtctttccgggggtagacgaagcgcacgacatcgttcttgcgcttgaactcctgataggtctcgccgccgggaatccggcccttttcagccggcgcgtagcccgcggcgcgaacctccttgaccagccggtcgaaggcggccttgtcggtcagcgagagctcgacgctgttctcgctggcgcggctttcggcatgggtggatttcatgaggcggatgttctggtcgtcgaccatcttttcgtactcgatcatgctgacctcgtcggtcaccgtcttgtcggcgtaggagaagccctgggccttgacctgctgccggaacgcatcgggcgtgagcgcggcgaaggctttgagttgctccagcgtgaagctggcctgctgtgcgaaggccggtgcggccagcatcaggagcgatgcgaagagggcgatcaatcgatgtttcatgggaaggttctgctcaggtcactgcgttcttgcggttgaattcttcgcgcttccactcgccggattcgagcacctgcaccaggtgctcgaccgcgttccacacgtcctcgaagccgatgtaaagcggcgtgaagccgaagcgcaggatgtcgggcatctgcgaatcgccggcgcggtagtcgccgatcacatcgcgcgcgatcagcgcctgcacgatggcgtaggcgccttcaccgcggctgaggcacacctgcgagccgcgctgtgcgtgttcgcgcggcgtgaccagcgcaaggccctggcccgcgcagcgctcttcgacgagttcgatgaagaggtcggtgagcgcgagcgacttggcgcgcagcgcggccatggcgccttggtccttgtcgaatgcttcggcggcaagcacggtgtccaggccgcattccagccccgccagcgcgatgatcggctgcgtgccgcagaggtagcggccaacgcccggcgccgggcggtaatgcggcgtgaactcgaacggcgccgcgtggccccaccagcccgacagcggctgctcgaaccggcccgcatgccgcgtatgaacccatgcgaaggcgggcgcgcccggcccgccgttcaggtatttgtagccgcagccgatggcgtagtcggcgttgctttcgttcaatgccactggcacggcgccggcgctgtgcgccaggtcccacacggtgagcgcgccggcggcatgcgctgcggcggtgatggccttcatgtcgtgcatggcgccggtgcggtagttgacgtgcgtgagcatcagcacggccacttcgtcggtcagcaccgaacccgggccttgcagttcgtccgcctcgatcagcttgagcgtgaagccgcgctcgcggcacagcgattcggcgatgtagagatcggtcgggaagttgctgcgctcgctgaccaccagcttgcgcccggtgtccttttgctgcgagagcgctgcgaacagcaccttgtaaaggttaacggaggtactgtcggtgcacaccacttcgcccggcgcggcgccgatcagccgcgccaccttgtcgcccaggcgctgcggcaggtcgaaccagctcgcggtgttccacgagcggatcaggccctggccccactccagggtgacgacttcggcgatgcgcgccggcgcggccgtgggcagcacgccgagtgaattgccgtcgaggtagatcacgccttccggcagtgtgaattggtcgcgcagcgggcgcagcgggtcttgcgcgtcgagcgcgcggcagtcttcaagagtcgtcatggggcggatttcagcgtgaaagttcgcgcagcacggcgcggacgggggaggcatcggcgctgaccagcttgagcggcagcgcgatgagttcgtagtcgccctcgggcacctcgtcgagcacgaggttctcgagcacgcgcaggtcgaggcggcgaatgcgttggtggctttccagcgtcttgctgtcggccgggtcgatgctggcggtgtcgatgccgatgagcttcacgcccatggccgccaggcgctcgatggtggccggtgcgtaggccgcgagctgcgggtcccagcggtcgatgggcatggcgctgtaggtgcgcaccagcacgcgcggcggcagctggctggtgatggcatgcgcgatgtgctcccattcgaccagcgggcccttggcgatggcatggatcacgcggcaggggccgatgaagggcgccaggtccaccaggccgatggtctggccttcggggtcgtagtgcaggggcgcatcggcatgcgcgccgacatgcggggagagcttgatttcgctgacattgaccgggcaatccggcgaaatggttgccgcccagcgctgctggtagggcgtgtcgccgggaaacaccggcgtgccttcatgcacgggcggtgaaatgtcccagatgcgttgcggatgagatgaagccatggcgcgaagttagcgcccggcgaggggtcgtggtgtcggttatttccaacaccatgcgtgacgagatgaaccggctcagtgatcgagcggcggcagcccgtgccgcgagcgcgcccgctcgcaggcgtcgctgccggcctgcagctcgtggcacgggttggggcgccattcgtagatgccgcagcccacggcgtggccgatcttgccggtcagcgccgcgcagcgcatcggggtgtggtcggtgccgcgcatgcggcaaagcgcatcgttcacctcgaccgcgaggcccgagggcacacgcccgccgttgtcgtcgagttcatgcacgctgaagtcgacgcggtagctggcgcagcaggcgccgcattgctggcaatcggacacgcggccgcgccttcagctgttcagagcctgcccaggagcaagaactccatcagcgccttctgcgcatggagccggttctcggcctcgtcccacaccaccgactgcgggccgtcgatgacctcggcctgcacttcctcgccgcggtgcgcgggcaggcagtgcatgaagagggcgtcgggctgggcgatgcgcatcatgtcttcgtcgacgcaccagtcggcaaaggccttgcggcgcgcctcgttctcggactcgtagcccatgctggtccagacgtcggtggtcaccaggtcggcgccgcggcaggcttccatcgggtccttgaagacctggtagctgtcggccgagcgcaggcccgccaccgactggtccacctcgtagccgctgggcgtgctcacgtgcaccttgaagccgaggatctcgctggcttgcagccaggtgttggccatgttgttgccgtcgcccacccaggccacggtcttgccctggatcgagccgcgatgctcgatgtaggtgaagatgtccgcaaggatctggcaggggtggaactcgttggtcaggccgttgatcaccggcacgcgcgaatgcgcggcgaaggtgtcgatcttggtctgttcgtaggtgcggatcatcacgatgtcgaccatgcggctgatgaccttggcgctgtcctcgatgggctcggcgcggccgagctggctgtcgccggtggtcaggtgcaccacgctgccgccgagctggtacatgcccgcctcgaagctcacgcgggtgcgcgtgctggccttctcgaagatcatggccagcgtgcggtcggtcagcggctggtgcttctcgtaggtcttgaacttcttcttgatgatcgccatgcgatcgaagaggtaggcgtattcgtcggccgtgaagtccgagaactgcaggtagtggcggatggcgttgggcgtggtggcggtcgtcattgcgctacaggctccgacagaaaggttttcaccaggggcgcgaggatggcgacgatctcgtcggcctcggcaatgctcaggatgagcggcggcacgaggcggatgaccttgtctgccgtgacgctcagcagcaggccggcgtcgcaggcgcggttcaggatcacgccgcagggccggtccagctcgatgcccagcatcaggccctggccacggatttccgtcacgcccgggaggccgccgatttcgcgctccagcgcgctcttgaggtgctcgcccaccgcggcggcgttctcgagcagcttgtgctcttccatgatgcggatggtctcgatgccggcacgcattgcgagcggattgccaccgaaggtggtgccatggttgcccgggccgaagatgttggcggccttggggcccgccaccacggcgccgatcggcacgcccgagcccaggcccttggccagcggcatcacgtcgggcttgatatcggcccactggtgcgcgaaccacttgccggtgcggcccatgccgcattgcacttcgtcgatcatcatgagccagtcgcgcgcgtcgcacagggcgcgcacctgcttcaggtattcccagcgcatcgggttgatgccgccttcgccctggatggtttcgaagaacaccgcgaccacgttgggattgccctcggtggctttcttgagcgcctcgatgtcgttcagcggcacgcggatgaagccctcgaccagggggccgaagccggcctgcaccttcgggttgccggtggccgacagggtggcgatgctgcggccgtggaacgcggcttcgtacaccacgatctcgggccgctcgatgcccttgtcgtggccgaacttgcgcgcgagcttcagggcggcttcgttggcttccagtccggtacagcagaagaaggcgttggtcaggcccgacagctcggtcagcttggcggccagttgctcctggcccggcacgtggtagtagttggagctgtggatcagcttgctgatctggtcctgcagcgcgggcaccagctcggggtggttgtggcccagcgtgttcacggcaatgcccccgaggccgtcgaggtaggccttgcccgtggtgtcccagactcggcagccctggccgtgcgacagcgcgatcggcaggcgaccgtaggtgttcatgacgtggggcgaggtgggctgggcggtagcgctcattcgggttctccagaaagggaaccgcggattctaggcgtgcgccatggcggcttcattgaggattccgcatcacagcaatgccccctgcccgggaggcaaaagtagggcggatagaatctcttgttgcaccgcagcacccgctccgggcgcctcattcaacgatgatttcccccactgccaaagaaatcttcatccagggcatcacccatgatggccggacatttcgaccgagcgactgggccgagcggctggccggcgtgatgtgctctttccggcccggcggcgcgtatccggggagccatttgagctattcgccctggtgcgttccaaccaccatcaacggggtcaagtgcgtggtcgtgaaccgggccctgcgcgatgccgaacccatggcctgggacttctgcgtcaattttgcgcgggacaacgatctgcaggtggccgaagcctgcctggtgcccgacgcgccggccgcgccacccaagacctgagccagaccttccagtttcaggaagcgaacggacatgaaaaaaccgcccgaaggcggttttttacactttgctgcagcgcaccccgatcaaacggcggaccggagaattccgatccgggcttgcctgacaggtgtcaggcggcggccttttcaggcgcgagggcgagggccttgaccttcgccgacaggcggctcttgtcgcgagctgccttgttcttgtggaagatgcccttgtcggcgacgatgtcgacgatgctctgggccttcgcgaagagttcgcttgccttggtcttgtcgccggccaggacggccttttcgacattcttcacggcggtgcggtatttggagcgcagcgaggtgttcgcagcgttgagcttggtgtcctggcggacgcgcttacggccggaggcgaggcgcgggttctttttcttgggcttggcggatgccatgatttagttccttaggtgtctgaggatgatgcagcaaagccctccattataggccgggttgcctttttcgccgaatcggggccttggccggccctacactcgccccgtgtccctgctcaaatccgcttccaccgtttccctcttgacgctcgcatcgcggatcacgggcctcgtgcgcgacgtgctctttgcctcggtattcggcgtcagtgccctgaccgacgccttcaacgtcgcgttccgcattcccaacctgttccgccgggttttcggcgaaggcgccttcagccaggccttcgtgccggtgctcgcggcgcgcaagaccgaagccggcgaagagggcgccaaggcgctgatcgaccacgtcgctacgctgctcacgtgggcgctggtggtgctgtgcgtggctggcgtggtgggcgctccgtggcttgtgtgggccatggcgagcggcctggcggggttcgacgctgctgtggtcatgacgcgctggatgtttccctacatcggcttcatgtcgctcgtggcgctggcgggcggcgtgctcaatacctggcgcaagttcgcggtgccggccgcttcgccggtcttgttgaacctttcgctcattcttgccatcgtggtgggcgcgccgctgttcaggcgctacggcatcgagcccatctatgcccagtgcgccggcgtgctggttggcggggtgctgcaactggcgctgcaagtgccggcccttcgtgccctcggcctcatgccgcgcatcggtgccagctggacggcgctgcgcaccgcctggaccgatcccactacgcgcaaggtcatgcggctgatgctgcccgcgctgctgggggtgagcgtggcgcagatctcgctgctcatcaatacccagatcgcctcgcaccttgccacgggcagcgtgacctgggtggtcaacgccgaccgcctgatggagtttccgaccgccatgctgggcgttgcgctcggcgtggtgctgatgccgcaactggccggcgcgcgcgccgccaaggacgacgagcggtactcggccctgctcgactgggggctccggctggtggtgctgctctcggcgccctgtgccattgccctgttgctgttctcgcagccgctggtggccgtgctgtttcacaacggcgcctacggcgacgaggacgtgaagcgcaccacgctggcgctcatgggctacggcgtcgggctggtgggcatcgtggccatcaaggtgctggcgccgggctactacgccaggcacgacatgcgcacgccggtcatcattgccgtctcggtgctggtgctgatccaggtgctcaacgtcttcctggtgccagtgctgcagcacgccgcgctcacgctgaccatcggcatcggcgcggtggtcaatgccctctggctcctggccgggctggtccgccggggcagctacaagcccgaaccgggctggggcaagttcatcctccaggtggctgcgggcacgctggtgctggcggccttgctcgcctggggctcgtactatttcgactggatcggcctgcgcgcccacaggctccagcgcatcggtctgctggcggcgctcatcgcgggagcggggctgctgtatttcgccgtgctggcggccgtgggcgttcggctgcgcagtttcatgcgccggtagggccccgagacattgcccggtcggggcttgggcaacagggttgttttcaaattgtgcaagctgaaaacaccgccttgacgctccccgaatgctcctctacaaagacacatgacgttcagcttccaggttcccaccgcactcgcgtatttcgaatcgctggtgcagagcgacgaccactttccgctgctcgaggcggccgccagccttgcgcaggacgaataccccgacctggacgtgcagcaggtgctcggcgacgttgaccagctgctggcccgcctgaagcgccggctgccggccgatgcggcgccgctggcccggctgcgcgcgctcaaccagttcttcttcaacgacctgaacttcggcggcaacgtcaacgactactacgaccccgacaacagctacctgaacgccgtcttgcgcacgcgccgcggcattccgatctcgctggcggtgctgtggatggagctggcgcagggcctggggctgcaggcgcgcggcgtcggttttccgggccacttcatgctcaaggtcacgctgcccaaggggcaggtggtcatcgaccccttcaccggcaaatcgctctcgcgcgaagaactgggcgagcggctcgagccgtacaagcgcagcaacgggctggtcggcgacttcgacgtgccgctgggcctgtacctgcagccgtccagttcgcgcgaaatcattgcgcgcatgctgcgcaacctgaaggaagtgcaccgtgcccaggaagactggcagcgtgccatcgccgtgcaagaccgcctgattgcgctgctgcccaccgcctggggcgaataccgcgaccgcggcatcgcgcacgccgagcagggcaacaccgcggccgcggtgcgcgacctcgaaacctacctggcgcacgcggaagacgcgctcgacgtcgacgccattgccgagcgcgtagccgcattgcggcgcgcggccaattgatggacgccacggacggcgtggccgccgcgcccgatctcggcacgctgcacgaattccacggtgtgcagccggtgctgccggtgtccgacgtcacgcgcgccgcgcgctggtttcgcgacgtgctgggcttcgagctcgacttcatcgccggcgagccgcccagctatgcgcgggtcaagaagggcgaccgcagctacggcgatccggtctacctgcgcctgtggcagtgcaacacgcgcggcacgccgccctggcgcggcgaaatcgtcatccacgtgggcaaggacgtggacggcctgcacgccgcctacgtcaagcgcggagtgacggtggtggagcccccggcctcccagccctggggcctgcgcgaattcgcgatccgcgagccggatggacacatcctgcgcttctgcggctatttgccctgagtttctgatacaaataattacaaatggatcgacgcggaggtgtcgatccgtctttcgctcgtccgacgtgtgaacaggagcacgtggtttttgcggctccaacctcatcaaaccttcaggagaaacgacatgcgattcatggttctggtcaaggccaacaaggattccgaagccggcgtgatgcccagcaccgaggtgctcaccgccatgggcaagttcaacgaggaactggtcaaggccggcgtgctgctggcgggcgaagggctgcatccatcgtccaggggcgcccgcgtgcgctgcgaagggctgaagcgcaccgtcatcgatggccccttcgccgagacgaaggaactgctcgcgggtttctggctgctccaggtcaagtcgaaggaagaagccatcgagtggatcaagcgcagcccattccaggagggcgagatcgagatccgccaggtcttcgaagcctccgatttcggcgactcgatgacgcccgaactgctggcacaggaagaccgcctgcgcgcggagaccgaggcccgcggcaaggccggcaactgagccggccgcacacccaaggagacccaccatgcgattcatgctgctgatgattccccacggctatgaaacggccgcgcccggcaccattcccgacgacgtcgatgcggtggcggccatgatggcctacaacgagtcgatgcagaaggccggcatcctgatcaattgcgacggcctgcatccgccctcgatgggcgcgcgcgtgagctttccgggccgcaagcccaaggtggtcgatggtccttttgccgaagccaaggaagtgctcggcggctactggatcatcgacgtgccttcgcgtgccgacgccatcgaatgggccacgcgttgcccgggcagcgagaacgaggtcatcgaggtccggcagatccaggagattgccgactacccgcccgaggtgcaggccttgaccaccgaatttccgtcgatgcaggcggtcaagaaaacttgatcatgggcgctgcgcctcgcgacgaggctgccatccaccgcagcatcgaggcggtgtggcgcatcgagtccgcgaagatcatcgccactgtggcgcggatggtgcgcgacgtgggcctggcggaggagctggcccaggacgcgctggtttccgccctcgagcaatggcccgaatcgggcgtgcccgacaaccccgcggcctggctcaccgcggttgccaagcgccgcgccctcgaccgtctgcggcatggccagctggcggagcgcaaggcacccgagatcggccgcgagctcgatgcgcagcacgaaatggcgcaagccgacttcgccgaagcggtggatgcggccatcgacgacgacatcggcgacgacctgctgcggctggtgttcaccgcctgccacccggtgctttcgaccgaggcgcgcgtggcgctcacgctgcggctgatgggcggcctcacgaccgatgagatcgcccgtgccttccttgtgcccgaagccaccgtggcgcagcgcatcgtgcgggccaagcgcacgcttctcgaagcgcgcgtgcccttcgaggtgccgcgccggcacgagctcgaggcgcggctcgcgtcggtgctcgaggtgctctacctgatcttcaacgaaggctactcggccaccgccggcgacgactggatgcgccccgcgctgtgcgacgaagcgatgcgcctgggccgcatcgtggccgagctgatgccggatgcggcggaggtgcacggcctcgtggcgctgatggaaatccaggcctcgcgcacggccgcgcgcatgggcccctcgggcgagccggtgctgctgctcgagcagaaccgcgcgcgctgggaccagatgctgattcgccgcggcctggctggactggcgcgcgcggaagcgctggtcggcgctcacggcccctatgcgctgcaggccgccattgccgcctgccatggccgagcgcgcaccgcggaagaaaccgactggccgcgcatcgccgcgctgtacgacgcgttggcggagctgtcgccttcacccatcgtcgaactgaaccgcgccgtcgcgctctcgatggccttcggcccggccgcagggctcgaagtggtggatgcgctcgtgggcgagccggcattgcagaactatcacctgctgccggcggtgcgcggcgaccttctgttcaagctcggccgccgtgtcgaggcgcgcaaggaattcgaccgcgccgcctcgctcacgcgcaacacgcgcgagaagacattgctgctggcgcgcgcccgggcctgcaccgtgccggaaagctgattctcggagcctctgcggcgctaggctttcgacagcgatgtggaagcggatggcgagccgggcagcccgaactgatgccatgcgcgccgcagctgcgtgtccgatccgaagcccgagatttccgccgcccgcgtcacgctcgcacccgaggccagcgcgagctgcgccgccgccagccgcagccggcgcaagtaggccagcggcgccacgcccgcatgctcgacgaacagccgcgtgaggtgacgcgccgaggtgtgggccacttccgccatccggggcacgctccagtcggcttgcggctgctcgctgacggcgtcctgcacccggtgcagcgcggcatgcaaatggttgcggtaggccaggaagggcgaaagctccgggtcgtgcgggccgcgccgctgggccaccaccatggtctgcgccacctgggcggccagcggctcgccgcacacctccgcgatgcggtgtagcaccaggtcgatgccggtcgtgacgcccgcgctgctgtagaccggcggatcgatgacgaacacgcggttggccaccacgtcgcagcgcggctctacggcgcgcagttcgtccaggtggtggtggtgcgtagtgacacgccggcctgcaagcgcccccgcgtgcgcggcgagcagggcgccggcgcagaccgtgaccagttcgagatggccgcgctcgaagcgctgcccgcgcagccagtgcagaagatcctgggtctcggcgttgtcgacggggatggagtcgccgggcagcccgaccagcacgatccaggccgggccgttccattgcgccggcaacggcgcgagattggcaagcgcaacccccacggaaccgatcgacgtggggcgcgggcttgcgaattcgatctcgaagcgctcgggctggcctgcggcgcgcagccgctggttcgcgatgcgcagcgcctcggcggggccggcccagtcgagcaccaggctgcccggcagcagcacgaacactacgcggatgggttgctgcaggaggtccatgcgtagtccatctggcgcgcggtgcgttcggccagcgcgcggccagccagccgttcgactaggtacaggctcatgtcgatgccggcgctgatgcccgcggagctgacgacgcggccgctgtcgatccagcgctcgccttcgcgcacgtcgagcgagggaaactgctcgcgcagatccgcgatgtcttcccagtgggtggtgacggcttcgcgcgtgaccacgccgcttttcgcgagtaggaagacgccggtgcagaccgaggcgaccaactgcgcgccggtcgcgcagtcggcgatccagcgcagcgtggcagggctcgccatcggcgcatcgaccacaccgccgggcacgatcagcacgtcggcacccgggttggtggccaggtcatggtcggccaagaggcgcaggccggctcgggcctgcacgggttggccgttgttcgacagcgcgacggacgcgacttcgaacggggctttcacgccgggattcatccgctggcagacgcggctcgcggtggtgaacacctcgaaggggcccgcgaaatcgagtgcctcgacaccgtcgtaagccaggatccgaacgcgcaaggtcatgccgccatgctttcgccggtcttggcgccggcacgttgcagcgcctgcgccacgctgcagacgctggcaaagcggccgtccagcacggcggcagtgcgtgccttgatgtcggccgcggccagcggccggccgtcgggctgcaccatgtcgaaagtcagcgtggcgtcggtcacgtagtcgacctcccagcccaggtcggaagcatggcgcgtggtggtttcgcagcattgctcggtgcggatgccgctcacgatcagccggccgatgccttgctgcgtgagccagacgtcgaggccgctgttgaccagcgcgctgtggcggtgcttggtgaaggtggccgcggcctcgaacgatgccacgccttcgatcggccgcacgaagcccgactcgatggcgaacgggttggccgccgttgcggggctgtcgacatggaagacgcgcacgatcggaagaccggcggctgagcagccttcgatcagcgcgttctgcgcggcgaagtagggttgcgcaatatcctcggaccagtacgggcgctggcgaaacgattcctgcgcatcgatcactatcagacaggatttcatgggggtcggctcgaagggcggagtgaatgatgccgcctattcttcggagttgccagcccgcggtccgcgccaaagcagaccagaatcgatcaaatcaggacatgagcgctagacgagctcggcagcctgcagctctttcttgaggtacgcgtagaaaagcggcgccgccaccaggccggccgggccgaaggccgcttccgccacgaacatgacggccagcagttcccacacccgcatctgcgtgcggctacccaccaccttggcgttgatcacgtactcggccttgtggataaggataagaaaaacaaggcaggcgagtgccgtgaccggcgacaccgagagcgccaccagcgtgatgaccgaattgcagaccaggttgcccacgatcggcaccaggcccgccacgaaggtcagcgtgatcagcgccggcgtgtagggcaggtgggggccccagagcggcatcaggaacagcaggaagatggcggtcagcaaggtgttgaaggccgcgatccagaactgcgcggcaacgatctggcgaaaggcctcgccgaagatggtgatgcgccgatacaactgcgcggcaagcgggcggcgctgcagcggcgttggcgcgatggcggccaggccgcccacgataaggccgacataggcgaacagcagtccccccagccatgcgcgtccggccagggccagcgaaccggcctgcgcccgcaggtagttggccaccacgcgctgcacttcggccgcgccttcgggcaggtagaccgcaatttcaggaggcagcttgagccgcagctcgagcaccgtgcgcgccgtgtagtcgagcaactcgcggtattggtcgggcgcatcgaggatgtactcgcgcgcctgggacaggcccagcgaaatcagtgcaatgggggccagcagcaccagcgtgaccgccaggacccgggccagcacgctggcacggaccagcggcagcctcagccgcaccaggccattgccgatcaggcgtgcgaaccagcgcgtggccagaaaaccgatgcacacgcacaagaggccgggcagcaggtgctcccacatcaccagcagcagggcggccggcatcaggaggtagctggccagcaccacgttgcgggaagctggcttgggcttggtgtcgatggtgacgagggtgggtttggacatcagggtccgggtgctgcgcgcgcttcggagggaaaaatcagccgaccaccacggcggcacccgcgccgcgctcggcgatgatgccgatttcatacaccgactcgccggccgcgcgcagcgtggcggcacaggcggcggcttcggtcgcctcgatcaccaccaccatgccgatgccgttgttgaaggtgcggttcatctcgatgtcgtcgatgcccgccaccttctgcagccaggcgaagagctcggtttgcggccaactgcccttcttgaggtgggcggccgtgccttcgggcagcacgcgcggaatgttctcgagcaggccgccacccgtgatgtgggccagcgccttgatcgggtgcttggccagcgcttcgagcaccggcttcacgtagaggtgggtgggctccatcacggcttcgcggaaaggcttgccgtcgagcgtggcgggcaggtctgcacccgcgcgctcgatcaccttgcgcaccaggctgaagccgttggaatgcacgccggccgaggccaggcccagcaccacgtcgccgggcttcacgttctggccggtgaggatcttcgacttttcgaccgcgccgaccgcaaagcccgccaggtcgtactcgccggccgggtacatgcccggcatttcggcggtttcgccgccgatcagcgcgcagccggagatttcgcagccgcgtgcgatgccgccgatcacggccgcggccgtgtccacgtcgagcttgccgcaggcgaagtagtcgagaaagaagaggggctcggcgccctgcaccagcacgtcgttgacgctcatggccaccaggtcgatgcccacggcgtcatgcatgttccattcgaaggccagcttgagcttggtgcccacgccgtcggtgccgctcaccagcaccggctccttgtagcgcttgggcacctcgaacagcgcgccgaagccgccgatgccggccagcactccttcgcgtagggtcttcttggcgaggggcttgatgcggtcgaccagggcgtcgccggcatcgatatcgacaccggcatccttgtagctgagcggggtgggcgtaggggaagtcatggtcggacggtgtcgagaaaggagcgggaaggagacgaagaggtaggggcgccggtaaccgaagcggccgggccgatagaattcctcacgattttaagggccctccgggccccctccatgaaccttcccgggatgaaacagctcgcgctcgatatcggcattgcgacgggccccagcttcgacgctttttttgccggcccgaacgaggcggcgctgcggcacctgcaactgtgggtgggcggcgccggcacatcggtgcctcactctcccgtgcccacctatctgtggggcgaaagcggcagcggcaagagccatctgctcgaatcggtgcgtgtcgcactgcgcgagcagggcgcgagcgtgggctggctgcatgccggcctgctggagccgcccgagttcgacgagcgctggggcgccgtgctgctcgacgacgtgcacctgtacaccgcggtgcagcagcacgcggccttcaactggttcgtcaacgcgcagaccctgcagcgcggcgtggtggcggcgggtgcgctgccgccggccgacctgccgctgcgcgaagaccttcgcacccggctgggctggggccacgtgttccacctgcaggtgctgagcgaaagcgaacgccgcgcggtgctgcggcaggcggccgacgcgcgcggcgtcatgctgtcggacgacgtgctcgactacatgctgcaccgcttcagccgcgacctgggcagcctcatggagctgctcacgcagctcgatggctatgccctgcagacacagcgagcgatcacgatcccgctgatccgatccatgctcgaaaacgaataaagaagagcttcaaccaacaatgatcaagaaattcatcgacaagctgctcggcaaatccgccggcggcacgcagggcaagagccgttttggcaagcgccaggaggtgccggccgaggttcacaagatcgatccagccctggtcgacgaacgcgcgaagaacgtggtcaccacgctccagcaagccggctacgaggcctacgtggtgggcggcgcggtgcgcgacctgctgctgggcctgcgtccgaaagacttcgacgtggccaccaacgccacgcccgagcaggtcaagtcgctcttcaggcgcgccttcatcatcgggcggcgctttcgcatcgtgcacgtggtgtacgggcgtggccgcgagcacgaggtgatcgaagtctcgaccttccgcgcctacatggacaacgccgccgccgagcaggttgccggcaacgagcgcaccagcaagggcgagcttgcaagcatgaagcacgcggtggacgccagcggccgcgtgctgcgcgacaacgtctggggcccgcaggaagaagacgcggcacgccgcgacttcaccgtgaacgccatgtactacgacccggccaaccagatcgtggtcgactatcacaatggcatcaaggacgcgcagaagctcacgctgcgcatgatcggcgacccggccacgcgctaccgcgaagacccggtgcgcatcatccgcgccatccgtttctcggccaagctcgcggccctgggtttcaagatggaaaccaagaccgccgcgccgctgatcgagtcgagcaagctgctggccgacgtgccgcagagccgcctgttcgacgagatgctcaagctgctgcagaccggccatgccattgccacggtcgagcagctgcgcaagctggacctggtcacgggcatctatccgctgctcgacgtggtggtggagcgcgccgactcgccgttcgtgaaggcggccctgcaggacaccgatcgccgcgtgggcgaaggcaagcccgtggcgcccagcttcctgttggcctgcgtgctgtgggccgacgtgcgcgacggttgggcccagcgcatcgagggccggcatggccagcgcccgcagccgccgttcccggccttgcaggacgccatcgacgacgtgttcaacgcccgcatcggcgacgtgtcggggcgcggcaagctggccgccgacatgcgcgagatctggatgatgcagccgcgcttcgacaagcgcacgggctccacgccctacagcctggtcgatcaggcgcgtttccgcgccgccttcgacttcatgcgcctgcgcgccgacgtgggcgaagtcagcgaggccattgccgagtggtggcaagagttcagcacggccgacgatgtgcgccagcaagacctgctggagcaggtgcgcgacgagcagaagacccgccagcgcgtgcgcacgcgcgatccggtggcgcccaagccccgcggcgaaccgccagcgcgccagcgccaggatggccaggagccggcgcagcaggacgacgatgagctggaaaccgaagccgcgggcgtctcggccgatggcgaggccgcggcgccgcgcaagcgccggcgtcgccggaagccccgcaccggtggtggcggcggtgcaggcgagggcggcgggagcgccgcaggcgaatgagcgcgcccaaccggccgaaggacggcaagagcggcggcaggagccagcccccgccgcgcggcggtgccgccaagccgaagagcggcgcggcaccggcacgccgcgcacccagccggccctcgggcaaggtggcgcccggcagccccgccgcgcgccgcacgcgcgaggactacccgactgtgcaggccttcgtcgccatcggcgccaacctgggcgacgcacaggcggcggtcaaggcggccatggatgccatcggcaccatcgaacgcaccgtggtcacggcacgctcgtcgctttaccgcagcgcaccggtcgatgcggccgggcccgatttcatcaatgccgtggtggccgtccggaccgggctcacggccgaggcgttcctggccgagctgcatctgctcgaagagcaggccggtcgcgagcggccgtttcccaatgcgccgcgcacgctcgatctcgacctgctgatgcacggcaatgcgatcaaggacacgcccgcgctgagcctgccgcatccccgcatgcgggaccgtgccttcgtgctcaagccgctggccgagatcgcgcccgacaaggtgccgcgcgcggcgatcgcccgcgtttcctcgcaggtcatcgagcgaattcgcgactgaaccgggcaggggctggagccgtgccggaccggccggcttcgcttcgcccattacacttgcgcggtttttcatgatgctgtcacacatttgtggcagtcgcgaacccaggagagagcgccatgttcggcaagctgctgccccgcgaggggaattttttcgagatgttcaaccagcacgccgagcgcatcgtcgaagcggcgcgggcgttcgagcaactcgtggccaattacagcgacgtgcacctgcgggagcagtacaaccgcgacgtcgacaatgccgagcgtgcggccgaccgcgtgacgcatgacgtcaaccggctgatccacaagaccttcatcacgcccatcgaccgcgagcagatccacaagctcatcaacacgatggacgacgtggccgacctgatccaggattcggccgagaccatggcgctgtacgacgtgcgccacatgaccgacgagatcgtgcgcctcacggccctgagcgtgaagtgctgcgatcgcctcaaggacgccgtcaagttcctcggcaagatcgccgacccggccgtggccgaggccacgctcaagacctgcgaggaaatcgaccgcctcgagtcggacgccgaccgcgtgatgcgcagcgccatgagcaagctgttccgcgaggagcccgatgtgcgcgaagtgatcaagctcaaggcaatctacgagttgctcgagacgatcaccgacaaatgcgaggacgtggccaatgtgatcgagggcatcgtcctcgagaattcctgagcgggtagcgattgatggcaacggttcaggtcgccctgtgggtggtgatattgctggtcgcgctcgcgatcgccttcgatttcatgaacggcttccacgatgcggccaactcgatcgccaccgtggtgtcgaccggcgtgctcaagccggggcacgcggtgctgttcgccgccttcttcaacctgatcgcgatcttcatctttcacctgagcgtggcggccacggtgggcaagggcatcgctcagcccggggtggtggatgtgcacgtggtgttcggcgcgctcatcggcgccatcagctggaacctggtgacctggtactacggcatcccgagcagctcgtcgcacgcgctgatcgggggcatcgtgggggccgtgatcgcgaagaccggtaccggcggcctggtggccaccggcatctggaagaccgtggccttcattttcgtttcgccgtttctcggttttctgctgggctcgatgatgatggtgttggtggcctggggtttccggcgcgccacgccgtcccgcgtcgaccgctggttccggcggctgcagctggcgtctgccggggcctacagcctcggccacggcggcaacgacgcgcagaagaccatcggcatcatctggatgctgctgatcgccaccggctacgcctcgtccggcgacgcggcgccgccgacctgggtcatcgtgagctgctatgccgcgatcgcgctgggcaccatgttcggcggctggcgcatcgtgaagaccatgggccagaagatcaccaagctgaagcccgtgggcggcttctgcgcggaaacgggcggcgcgctcacgttgttcctggccaccgggctgggaattcccgtctcgaccacccacaccatcaccggcgccatcgtcggcgtcggctccgcgcaacgcgcgagcgccgtgcgctggggcgtggcgggcaacatcgtctgggcctggatcttcacgatcccggcatcggccttcgttgcggccattgcctactggctcagcctgcagattttctgaggcgcgcggccctcgggcgctcagcagctactgtgagatcttccggccttcctcgacctggtgttcgaagtagcgctggaagctgaacacgatgctggccatcagcaccgtggtgccgaagaggagtgccagcaccacggcgccaatggtggcccagttcgtgcggcccggggcggcgtccggcggcgcaccggcgttgaagcgggcattccacttctcgggcgtcatgaggccgtagatgatggccatcagcgcgcacccggcgatggtgaagcccaggagcggaatcagcacccagctccagccgtcgtccaggccgtacattcgcgtgcgctcgatgccgtagaggccgagcgccgtgggaatgggcagcagccagccgagccagtcgcccatgccgcgaagatagaagcggtgcaggcccagcgggccgcccaggaaggagagccaggcggcaatggtcttgtttttcattcgggtttggtggtgctgccttcgccgagcaccttttccatcaggaccacgtcgcgccattggccgaacttccagccgcagtccttgagcacgcccacgtgcgtgaagccctggctgcgatgaacgcccaccgagccggcgttggccgagtcgccgatcactgcgatgagcttgcgcacgcccaccgcctctgcggcctgcgagagggctgcgagcaactggccgccgaggccccggccgcgtgcggcttcggagatgtagatcgagtcttcggccgaaaagcggtaggccgggcgtggcttgaaccagttgcagtaggcaaaacccaacacttcgccattttcttcggcaacgaggtagggcaggttcttgccgagcacgtcggcgcgccgcgcggccatgtcggcggccgagggaggctcggtttcgaaagtgccggtgccgttcagcacgtgatgggcatagatggccgtgagggccgcgacatcttcgtcgcggctggggcggatggtgagggtcatgcaggtggaaatcgaagcgcgccaagcgctaaattcggagaaaacgcgggtcgggctataatcgcaggcttttcagcgtgtcgctggccgggtggccatgtcgcgtgtctcgacgttgaaagaacactgtgagcgggcctcctgtttagaaaacgggcttgctgcaccacccaaggataaatcatggtcgtcattcgactctcccgcggcggctccaaaggccgtccgttcttcaacatcgtcgtgtcggacaagcgcgttcgccgcgatggccgcttcatcgagcgcctgggtttctacaacccgatcgccaaggaaaacgaagaaagcatccgtattgcccaggaccgcctggcctactggaagagcgtcggcgcacaagcttcgcccacggttctgcgcctgatcaagcaagctgcagccgcagcgcccaaggcagctgcctaagctgtccggcacgacgatgctgcctacactcgaaaccgccgaattgccggcggatgcgatcgaggtaggacgcatcgccgatgcatggggcatcaagggctggttcaaggtcctgccccacagcgcccaaccagaggcgcttttttcttctaagcgctggttcctgcaggctcccggagcctccgcaaccgcagctttccggctcgcgatccgcgaagccaaagaacattccgactgcatcgtcgcttcgtccgaagaggtgcccgaccgcaatgcggccgaggcactgcgcggcgcgcgtgttttcgtgccgcgctcgagctttccgaccgcgggtgacgacgagtattactgggtcgacctgatcggcctttcggtggtcaaccgcgaaggtgtggcgctcggcacggtgcgcgagctgctcgccaccggcccgcagaccacgctggtgctcgcggccgaagaagacggcaaggccatcgaacgcatggtgcccttcgtctctgtcttcgtcgacaaagtcgacctcgccggccggctcatcacggtcgactggcagcctgaatactgaccaggcgccgcgcgcatgcgcttcgacgtccttacgctgtttcccgaactgttcgcgcctttcatggccagcggcgtgacgcgccgtgcctatgagtcgaagcaggtcgaggtcgtgctctggaatccgcgcgatttcgcgcagggcaattacaagcgcgtggacgaccggcccttcggaggcggtcccggcatggtgatgatggccgagccgctctcggcctgcctcgatgcggcactggccgcgcgcggatcgccggcgccggtcgtgctgttttctcccatcggcgaggcgctgcgccacgaggcggtcgagcgctggtctgcgagcgaaggcgcggtgctggtctgcggccgctatgaaggcattgaccagcgcttcatcgacacgcgcgtcacgcaccagatcagcctcggcgacttcgttctctccggcggtgagattccggccatggcgctgctcgatgccgtggcccggctgcagcccggtgtgctgggcgacgaagccagccatgtgcaggacagcttcaatccctctctcgacggcttgctcgactgcccgcactacacgcggcccgagcaatggaacgggcagggcgtgccggcgccgctgctctccgggcatcacgtgcagatcgagcgctggcggcgcgaccagcggctggccattaccgccgcgcggcgtcccgacctgattgccgccgctcgcgctgcgggccgcctgagcaaggccgatgagacggcgctgaaaaaaaagctataatcctcggttccccgatcctctgcccggccgcgcctggctttgttgcagtcccttgttgtgttccttgtcgccttcggcgatcaaggagcgacgaaagagcaacgaaaccaaaggcgccttttgtgtagcgcgagcacgatcgaatatcaggaaatcatgaacctcatcgaaaccctcgagcaggaagaaatcgcccgcctcggcaagaagatccccgatttcatgcccggtgacacggtcatcgtcagcgtgagcgtcgtcgaaggcacccgcaagcgcgtgcaggcctacgaaggcgtcgtgatcgccaagcgcaatcgcggcctcaacagcggcttcacggtgcgcaagatctccagcggcgaaggcgtggagcgtacgttccagacctacagcccgctgatcgccggcatcgaaatcaagcgccgcggcgatgtccgccgcgccaagctgtactacctgcgcgaccgcagcggccgttcggcacgtatcaaggaaaagctgccgggcaagtcgcaggctgccaagtaagctgcttcctgccgtgcaaaaagccgccactctggcggctttttgcgttgtgcgccgcgcacgtttcttgcaaaaagacagcacggcttttttacgctctactccttcactgaaactccctcacttgaccgattccgccgcccccatgccatttgctcccgtcgaacccgtcaatgccgtggtgccgcccacgctgctggcgatcgacccgcgcaaggcgccggtggtcggcggccccgacggcctgcccgccgtcgcacccgcgcagttgaccaccgaggcgctgcgcagccgctttgccaccccgccggcgtggatgcccgagttgcgccgcgagccgcgcctgaccgaccgtgtgccggcgcaggcagccgtgctggtgcccatcgtgcagcggccgcagggcgccaccgtgctgttgaccgagcgcaccgcgcacctgtccactcattcgggccaggtcgcgtttccgggcggccgtgtcgaccccgaggacgcgaacaccgcggcggccgcgttgcgcgaagcctgggaagaagtgggcctgtccgcccggttcatcgaagtgcttggtagccttccgacctacacgaccgtcacttcgttcatcgtgacgcccgtggtcgcgctggtgaagcccgacttcgagctcaccatcaatccctacgaagtggcgctggccttcgaggtgccgctggcctggctcatggacccggccaaccaccgccgccataccgtgcccgcgcccgatggcacccaccgcgagtggtactcgatgccctaccaggacggcgccgaagagcgcttcgtctggggcgccaccgcgggcatgctgcgcaacctctatcgctttctcagcgcctgacctcgggccgggccaagccttcgcaagctctctcgctatcatcgaaggatgagcttctttgccatcctgtgtgcgttgctgatcgagcaggtgcggccgctcgccccccacaacccggtgtacggcggcgtgctggcgtggacgcgctggaccagccgcaacttcgatgccggcaagccgcatcacggatgggttgcgtgggcccttgcggtgttcgtgcccaccttgctgacgctgggcattcactggctgctggtgctcacgctggggcttccgttcgccgtgctctggagcattgcggtgctctacgtcaccctcggcttccggcagttcagccaccacttcacggacattcgcgatgcgctcgacgaaggcgacgagccgctcgcgcgttcgctgctggcgcactggcagggtgtcgatgcggccgacctgccgcgcagcgaaatcgtccgccacgtgatcgagcattcggtgatcgcggcgcatcgccacgtgttcggcgtgctggcgtggttctcgatacttgccgccctgggcctggggccggccggtgcggcgttctatcgcatgagcgaattcgtctcgcgctactggatgcacaagaacggcgccgcaatacagccttcgagtgtctcggtgcagcgggccgcggagcgcgcctggcacgcgatcgactggctgcccgcgcgcatcaccgcactgggcttcgccgttgtcgggagcttcgaagaggccatcgattgctggcgcaacgacgcgcggcgctttccgagcgagaacgacggcgtgatcctcgcggcaacctcgggcgcggtcaacgtgcgccttgggggcggtgcattgagcccgattccggtcaccgatccgctgccgcgcgcgcaggccggcgattcagtggacgacggccgccggctcgacagcggcagcacgccgggccgcgagcccgagcccggccacctgcgcagcgtggtcggcctggtctggcgctcggtcgtgatgtggatggtgctgctggccctgctcacgctggcccggctgctcggctgaacgacatgaccacctcgctaccggctttctggagcccgcgcatcggcgcgctcgaaccctatgtgcccggcgagcagccacgcatcgccaacctcgtcaagctcaacaccaacgagaacccgtacccgccgtcgccgcgcgccgtcgacgccatccagcaagcggcagcgagcggcctggagcgctatcccgacccgacttcgcttgcagtgcgcgaagcggtggcccggcgccacggcctgcaagccgaccaggtgtttgcgggcaacggttcggacgaggtgctggcgcacgccttcttcgccttcttccagcaggccgagccgttgctgatgcccgacgtgagctacagcttctatcgggtctatgcgcagctctatggcattgcatgcgaactgttgccggtcgatgagggtctgcgcatcgacgtcgatgccatggcggcccgtgcccgcggcggctgtgccggcctggtgatcgccaatccgaacgcacctacgggcatcgggctgccgcttgcgcgcatcgagcaactgctcgcggcgtgccctgggcgcgtggtgctggtggacgaggcgtatgtcgatttcggcggcgagagcgcgctgccgctggtcggcaaatatccgaacctgctggtggtgcagaccttgtccaagtcgcgctcgctggccggcttgagagtcggctttgcctgcggccaggcgcacctgatcgatgcgctggtgcgcgtcaaggacagcttcaattcctatccgctcgaccggctcgccacggcgggcacggtggcggccctcgaggacgaggactggttcaagaccacgcgcgacaaggtcgtcgatacccgcgaagggctcagcctgcagctcgaagacctgggcttcgaggtgctgccgtcgcacgccaacttcgtgtttgcgcgtcatccgaagcgcgatgcggctgaactcgcggcgcagctgcgcgagcgtgcggtgctggtgcggcatttcaagcagccgcgcattgcgcagtacctgcgcatcagcatcggcacgcgggagcaatgtggggcactggtgcgggcgctcgaatcgatcctgggcgttcagtagttcagtagcgggactggctcagttcggcaaagagctcgccgtagatcttgtagcgcgacgcgctgatcggccccggcctggcgggcgaatccacgttcgcgatcacgccgcatccgggctcgtgcagatgggtgcagttgtagaacttgcagtcgttcgcgtgctcggcaatgtcgggcatcagcttcgcgagctgcatcggctggatgtggttgagcccgaattcctggaagcccggcgagtcgatcaggccggtggtgcgtgcctcgtcgatccagtaccaggtggtgctggtggtcgtgtgcttgcctgagttcagcgcctgcgaaatctcttgcgtcagcacggtcgcgcccggcaccagcaggttggtcagggtgctcttgcccgagccggagggtccgagcacgagggtcgacttgccggcaagcagcttcatcagcgacgcatagtctgcttcgcccgatgccttcagcgacagcggcagcacgccgtgatgcatgcggcgatagggcgccagcttgttccatgcgcgcccgaagggctcgaccaggtcgctcttgttgagcgcgatgatcggcgtgatgcgctcggcctccgccgcaatcaatgcgcgcgccaactggtgctcggaaaactccggctcggccgcgatcaggatcagcacgtggtcaaggttggccgcaaacgacttggtgcggatctcgtcctgtcgatagaagaggttgcggcgcggcagcacctcttcgatggtgccctcgtcctccgtggcctgccagtgcacacggtcgccgaccacggcctggctcttcttgccgcgcgggtggcagatcagccgctcgccggtgggtgtttcgacgaggcaatgacgtccatggctggcaacaacgagaccgtcgtgtagcgtcttcgcagcagaggcggcggaggcagcggcgcggcccggcttagccacgggcgtgatccgtcatgcggtggggcccgcaaccagcgcatccgcctggcgtgcgcattcgaagtcggtgaccgaaagtccgcccacgtcgtgcgtgttgaagcgcacggcgcagcggttgtagtgcaccgacaagtccggatgatggtcttgcgtgtgggcgatgaaggccagcgcattcacgaaagcgatggtctcgaagtagttggcaaaggtgaaggtcttctcgatggcgacgttggcaccgtcgccgctgagcttccatccgtcgagcttggcgaggccggacacgatctcggtggcgctcaatgcgtggcggggaggaatgtttttccagtctttgggcttgaacatgctgctcatggtctcggcttccggggcaagtattttttcaggccgccgccatgcgcgcgaggcgctcggaggccggagggtgggaatagtagaacttgacgaacaccgggtcgggcgtgagcgtcgacgcgttgtcctggtagagcttgagcagcgccgtcgacaggtcggcgccgctggtctgcgcaatggcatacgcatcggcctcgaactcgtgcttgcgcgacagccgggcgggcaggggcgcgacgaagaagccgaacaccggaaccgccagcatgaacagcagcagcgcgagcgcattgttcggcgccgtcgccgtcatgctgggctgcacgcccagccccgtgtagaaccagacctgggtcgacacccagcccagcagcgcgaagcccgccaggctcagcgcgaacatggccacgagccgcttcacgatgtggcggtgcttgaagtggccgagttcgtgcgcgagcacggcttccacttcgcttgcgctgagctggcgcagcagcgtgtcgtagaacaccacgcgcttgctcgcaccaaagcccgtgaagtacgcgttggcatgggcgctgcgggtgctgccgtccatcacgaacaggcccttggcggcaaagccgcagcgcttcatcaaggccgtcacgcgatccttgaggtcgggatcgtcgagcggcttgaacttgttgaacagcggcgcaatgaacgtggggtagatcagcatccccagcaggttgaagcccatccacacggcccaggcccagagccaccacatggtgccggcggcgcccatgagccagaggatcagcgccgcgatcggcagaccgattgccgcgccgagcagcgtcgacttgagggtgtctgcaagccagaggcgaagggtcatcttgttgaagccgaaacgctcttcgagcctgaaggtctgccagagcgtgaatggcagctcgagcaggccgccgatggccgcgaacgccgccagcagggccaactgctgcaccatgccgccgctgagccaggccagcagcagcttgttgagcacgtcgagcccgcccaaaagcgtccagcccagcagcaaagcggtgctccatgccatctcgaccaggccgaaacgcgccttggcaatggtgtagtcggctgccttctggtgcgcggcgaggctgatggtgtgttcgaaagcggccggcaccgcgccgcggtgctgcgccacgtggcgcacctgccgcgaggcgagccagaacttcacgagcaggcccgcgaccagtgcagaggcgaaggcaatggtgaagatgagcgaataggacatgagcgtcgagtttagccctcgggtccggccggtgcagaccttcgacgacaatccagcgatgcccgaatcccttgaccccacgaccgccacagccacgcccgtcctgaagaaaagcgaccagaacctggtctggctcgactgcgaaatgagcggcctcgacccggagaaggagcgcctgctcgagattgccgtggtcgtcaccggccccgacctcacgccccgcatcgacggccccgtgctggtcatccaccagagcgacgcggtgctcgacgccatggacgcctggaacaaaggcacgcacggccgcagcggcctgatcgacaaggtgaaggcttccaccctggacgaagcggcggccgagcagcaactgctggaattcatcgccaagtacattccgcgcagcggttcgccgatgtgcggcaacaccatcgggcaggaccggcgcttcctggtcaagttcatgcccaagctcgaggcgtacttccactaccgcaatctcgacgtcagcaccttgaaggagctggccaagcgctggaagccggcggcatacaacgccttcaagaagcagcaggcgcacaccgcgctggccgacgtgcacgaatccatcgaggagctcgcgcactaccgtgaaacctttctaaaactcacggattaggtaaaaaccccgacccgtgccataatcgaaggcttcgctgatccgggttaccggtatttttggtttttctggtcggcgtctcttgcatctccctatcttgcacaccgcgcccgatcgcatccgctgatcaaaaagggccgcagcctccggcgtaagccagaagctgaatgtcgttggatggttgatgtttttaaccaccaacggggcgccgccttcggcagcgctcgcgtttgagattgatatctacatgaccgacgcttttgaagcgcagggcgagttcgcgcctgtgcaatccaccaacaacaacgaattcatcgccgccgtggacaccgtgtccgaggcaccgattctcgaggcgctcgacgcagcagcccccgaagcggccgtggccgaagagccccgcctgcccaacggcttcgtcaagctcggcctcgcgcccgaactgatcgccgccgtggccgacctgggctttacccagcccaccaccgtgcaagacaaggtgatcccgctcgccatgggcggtgaagccggccaggacggcaaggcccgtttcgtcgacctgatggtctccagccagaccggctccggcaagaccgcggccttcctgctgcccgtgctgcacacgctgctcaagcgccaggccgaagccgaagctgaagccaaggccgaattccagcgcctggccgccgaagccgctgcccgcggcgaagccgtgccgaagaagccgaagcgcaaggacccgaccaatgcgcgtcatttcaaggccgccacccctggcgccctgatcctgtgcccgacgcgcgaactcgcgcagcaggtggcgcacgacgccatcgaactggttcgccattgccggggcctccgcgttgccaacgtggtgggcggcatgccctaccagttgcagatcgccaagctgcagaacgccgacctcgtggtggccacccccggccgcctgctcgacctgcagcgctcgtcgcagctcaagctcgaccaggtcaagttcctggtggtcgacgaagccgaccgcatgctcgacctcggcttctccgacgacctggccgaagtgaaccagctcaccatcgagcgccagcaaaccatgatgttcagcgccaccttcgcgccgcgcatccagcagctggcccagcgcgtcatgcgcgagccgcagcgcatcaccatcgacagcccgcaggaaaagcacgccaacatcaagcaatcgctgtactgggccgacaacagccagcacaagcgcaagctgctcgaccactggctgcgcgacaccagcatcaaccaggcgatcgtgttcgccagcacgcaagtcgaatgcgacggcctcgccggcgatctgcagcaagaaggcttcagcgccgtggcgctgcacggcgccctgagccagggcctgcgcaaccgccgcctgatggcgctgcgccagggccaggtgcagatcctggtggccaccgacgttgccgcccgcggcatcgacgtgccgaccatcacccacgtcttcaacttcggcctgccgatgaaggccgaggactacacccaccgcatcggccgcaccggccgtgcaggccgcgacggcctggccatcacgtttgccgaattccgcgatcgccgcaagatcatggacatcgagcagtacagccgccagcagttcaaggccgaagtggtcgccggcctcgagccgcaacaacgcatgccgcaatcgcgtcccccaatgggcgagtaccgcggtggccgtggtgacaaccaatcgcgcgaccgcaagttcggcaatggcggtgcaggcggcggcggtggttaccgcggcggcaacagcggcggctacgccggtgccagcggcttcaacgaccgcaacgcacgcggtccggccccgagccaaggtcaccagggcccgcgcggcttccagggcggcaacaacgccggcttcggcggcagccgcgacgacggcggcaacggtggtggctacggccgcaagccgggctggggcgacagcgccccgcgcggcggccatggtcatggcggtggccgtggcgacggtggcttcgccccgcgtgaaggctttgcaccccgcgaaggcttcgcaccgcgcggcaatggcgcaggccatggcggcccgggcaaggtgttcgtgccccgcgacgcacaaaagcgtgcgttcaagcccacgcgctgatccattccgaagcggccagccggccgtctcgccccaaaagaaagcccgcgcttcgcaagaagcgcgggctttttcattgcgggtttccgaggggctccctgcagcggattttgattgacacatgaatcgatgaaaagtaatgtaatagcgcattgcttccccggtccgcatcgcggccgccggttcatcgatatctgcttttcaaatttcgaccatgaaaatcgcgattcttgggggtggccacggcgcctatgcggccgccgcggacctgtccgaagccggccatgaggtgcgcctctggcgtcgcgacgcggccgcgctcgagccggtcgtgcaagccggggccatcacgctgaaggatgccgatggcgcgcgcgaggtgccgcttgcgctggccaccgccgacatcgccgcggcgctgaagggtgcagaactcatcgtcgttcccacgcccgccattgcgcagcacgacatcgcgcttgccatggcgccgcacctggtcgacggccaggtcgtcttcctgccgccgggcaccttcggcagctacgtgatggcaagaacggtgcggcaggccggcaaccgcgccgacgtggcctgggccgagaccggcaccttgccgtaccttgcacgcaagcacggcgagcgcgaagtgaatgtcacgatccgcgccatccgcctgcccaccggcgtgtacccggcccgcaaggaggccgaagccatcgaggtgatccgcagggcctacccggccgtgcatgcctgcggcaatgcgctctcgggcgcgctcatgaacgccggcccggtcatccacccgcctctgatggtgatgaacgccgccccgctgcagcacttcgaacgctgggacatccacaacgaaggcacgcagctcgccgtgcgcgacgtgaccgaccggctcgaccgcgagcgcatcgcggtgcgcgaggccttcgggcagggcgcgccgcactatccgctggccgaccactacgacaacgaccggtggatgtacggcgatgcgcacaagcagctcgtcaagtcgggcgactggcgcgagaacatcgacctgcacacgcatcgctacatcaccgaagacaccgagctcggcctcgcgttcctggcctcggccgcgcgccatgccggtgtggatgcgcctattgcgcacggcttgctcgccatcgtcggcggctttctcggccgcgagctgcgctacggtccgcgcaccttcgaaagcctgggccttgccgagctgagcgcggcgcagctcgagcaaaggctgcacgatggcgaatgagccattgctgccccgcttcgccgccgtcggtgccggccgcatggggcgcggcatcgcgattgcgttcgcctatgccggccaccgcatttccctggtcgacctgcgccagcgcagcgacgaagcctggcaacgcctgcagggcgaagccaaggccgagatcgaaaacagcctcgagagcctggcgcagctcggcgtgatcgatgcggcgcagatccagcgcatcgccgagcgggtgagcttcgtgaatgccgaggcggcgccgcaggcactggccgccgccgagctggtgttcgaaggcgtgcccgagaccatggaggccaagcgcgaggccttcgagcagctcaaccgccattgccgcgacgacgccatcctgacctcgaccaccagcagcatcctcgtgacgcagctcgcggcgctggtgcgattgcccgggcgttttctcaacatgcactggctcaacccggcctacgtgattccggtggtcgagctcagctgccatccgggcaccgacaccgccgtgctcgcgcgcaccaaggcgctgatggaagccatcggcaagctgcccgtggtctgcggcgcatcgccgggctacatcgtgccgcggctgcaggcactggtgatgaacgaggctgcgcgaatgatcgaggagggcgccgccaccgccgaagaaatcgacaaggccacgcgctatggcctgggcttgcgcttcgccgcgctcggcgtggtcgagttcatcgacttcggcggctgcgacatcctgcaccatgcgagccgcgagatgtcggcctcgatcgacaagggccgttacaccgcgccggccatcgtcgatcgcatggtcgaggaagggcggctcggcctcaagagcggcagcggcttctacgactaccaaggccgcgacatcgcagcctaccggcgcgacgtgctctcgcgcacgctgggtgaactgaagcacgccgggctgtggcgcgcgcccgccgacgagacgcgttcatgacgatccgccgcgcctttgccgacctgtcggtggggcaggtgcactacgcggcgtgcggcgatgcggatgcgccagccgtgctgctgctgcatcagtcgccgcgcagctgggccgagtaccgtgcggtgctgccgctgctcggcgcgcgataccgggccattgccatggacaccgcgggcttcggcgattcgtcggacggcggcgtgccggccagcattgcgcaatgggcgcgcgtggcgtgcgaactgctcgatgcgctgaacatccggcaggccgatgtggtgggccatcacaccggcggcgtcgtggcgatcgagctggccgcggcctttcctgatcgcgtgcgcggcctcgtgctgtcgtccacgccgtacaccggcgaagccttccgcatcgccagggcccagaggccgcccatcgacgaggtggcgccaagcgacgatggaagccatctggccgcactctggcaaaagcgccagggcttctacccgccgggccgccccgatctgctcgaggccttcgtgctcgatgcgttgaaggtcggccatcgtgtggaggagggccatcgcgccgtcgcgtcctaccgcatggaagagcgcatcggccgcgtgacgcagcccgcgctcgtcatccgcgccaccggcgatccgtttgccgcaccgcatgccgaggagctgcggcaccatctgccggatgcgcgcatcgtcgacatcgaaggcggcatggtgccgttgcccgaccagatgcccgaagcctttgcgcaagcggtgctcgactttctttcggccttgccatgaaagccatccgcatccacggcttcgacgcggcgccggtgctcgaagaggtgcccgatccggtgcgacgggccggccgcaccatcgttcgcatgcatgcggccactgtcggccatatcgaccgcaccgtttggcgcggcagctttctgcgccatccgccgctgccctacacgccgggcgtggaggccgcgggcgtcgtcgtcgagagcgaccgttacgctgcggggcagcgcgtgtggctgcgcggcagcggcctgggcacgctgttcgacggcacctggtgcgagcagatcgatgcacccgatgaagcgcttggcctcttgcccgacgcattgccgatgacgctcggtgccgcattcttctcgcccaccacatcggcatgggtggcactgcatgaagtcgccaggctgcaggccggcgagcaggtgctggtgacaggcgcgagcggcgccgtgggctcgctcgccgtgcaactggcacgcgagcttggctgcaccgtggcggcggtcgatccggaggccgaggccccggccatcgcgagtgcggacctgctgatcgacgcggtcggtggcagcgtgctttcggcggccttgcctgccgtgcggcccggcgggcgcgccgtgctcatcggctacacggcggggccctcgctgcagctcgacattgcgcacttcctgcagcgtgacgtcgcgctgctgccgctcaacatgttcaggcgcgaagccgccggccgcgccgcagcgccggagttgctcgcgcgcctggccgatggccgcctgcatctcgacgtgcggagcttcgcgctcgccgatgccgccgtggcgctcgaatggatcgcgcagcgtggccatcgcggccgcgcggtgctggttccctagtcttcttccggctccccgaccggcacatgcacgtgcaggtcgatcatctgccgcagggtctgcttcagctcttcggcgcgccgcaggccaaagggctcgagcacgcgccgctcgtggtcgcgcgcgagttccatcaggtgctccaccgccttcagccccttgcgcgtgatgcgcaccagcgtgatgcggcgatcactctcatggggcagccgctcgacctgtccgcgtgcttccatgcggtccagcaagcgtgtcacggtcggctgcttggtcacggtcacctgcgcgagctgcccgatgctgatcggctcgctgcccgcgagcgacgccatcacgcgccactccgacacggaaaaaccctgctgccgcgccacctcgtggaactccgaggagatcagctggctggcctgcgccagcagtgcgggcaggtagtcatcgacgaagcgatgcggttcgggcggctgctcagccatgaaggcacctcacggccacgagcctcacgccagccgcgggcacgctgcttgcatgtctagggtaattcatgattgtggatacattcatttgtcaacattataggaaccacggtgcggcagcttgctcgcatcgtcccacgagagagaacaaggacccacatggctgagcgttcgttcgtcgaagaagtcaagaagctgcggctttccggtggcgaggtatttcgcggtgaaggcattctggcggtcaccaaggccctgcttgaatcgggggtttcctatgtggccggctaccagggcgcacccatctcgcatttgatggatgtgctggccgatgcgcaggacattcttgcggagcagggcatccgcttcgagaacagcgcgagcgaagccaccgcggccgccacgctggccgcatcggtcaactacccgctgcgcggcgccgtcaccttcaaggccaccgtgggcaccaacgtggcatccgatgcactggccaacctcgcctccggtggcgtgaccggcggtgcgctgatcatcgtgggcgaagactacggcgaaggctcatcgatcatgcaggaacgcagccatgcgttcgcgatgaagtcgcagatctggctgctcgatccgcgccccaacctgccgagcatcgtcgacgcggtgaagcagggtttcgacctgtccgaggccagcaacacgcccgtgatgctgcagctgcgcatccgcgcctgccacgtgcacggccacttcatcgccggtgacaacaagcgcgccaagttcacgctgaaagatgcgctcgagaacccgcagcgcgacgtcggccgcatcgtgctgccgccagcgagcttcattcacgagcaggaaaaggtgaaggaccgctggcccgccgcggtgcgcttcatcgaggagcgcgagctcaacgagttcttctcggaggatgccgacgacatcggcatcatcgtgcagggcggcagctacaacacgctgctgcgcgcgctggagcggctcggcctggccgatgtgtacggcaacacgcaggtcccgctctatgtgatgaacgtggcctaccccgtcatcgagagcgaggtgatccgcttctgcgaaggcaagcgcgcggtgctgatcgtggaagaagggcagcccaacttcgtcgagcagaacctcgccaccatcctgcgccaggccggttcggccaccgcgctgcacggcaaggacatgctgccggtggcgggtgagtacaccgcgtccgaactgctgaagggcgcgcgcaccttctgcgagcgctatgagcgcctggcgccgctgccagcgcccgtcgcgcagcgcaaggtgatcccgctcaaggaagtggccgccatcggcgtcgatggcgcgcccgagcccgcgctgccatccacgtcgctcagcgaagtggtgcatgcgcgtcccccgggcttctgcaccggctgccccgagcgcccgatcttcagcgccatgaagctggtcgagcgcgagctcggcgcgcaccacgtcagcgccgacatcggctgccacctgttctccatcctgccgcccttcaacatcggcaacaccaccatgggctacggccttggcggagccggcgcggcggcgctcaatgcgccggcgggcaaacgcgccatctcgatgatgggcgacggcggcttctggcacaacggcctcaccagcggcgtggccaacgcggtcttcaacaagagcgacaacctcaccatcgtcgtcgacaacaactacacctcggccacgggcgggcaggacatcctttcgtcgaacgccgtcaacaagacgcgcagcaccggccacgagatcgaacgcgcagtgcgcggcgtgggcgtggagtgggtgaagacgctgcgccgcacctacgacgtggccggcatgcgcgatgcgctgaaagacgcgctcaccacgacgaaaaaaggccccaaggtcctgatcgcccagtcggaatgcatgctcaacaagcagcgccgcgaaaagccgctggtgcgcaaagccattgccgacggcaagcgcatggtgcgtgaaaagttcggcgtcgattccgacacctgcaccggcgaccactcgtgcatccgcctctcgggctgcccctcgctttcgatcaagcccaaccccgatccgctgcgcaccgacccggtcgcgaccgtgctcgacagctgcgtgggttgcggcgtgtgcggcgaggtctcgcatgccgcggtgctgtgcccctcgttctacaaagcgcagatcgtcagcaacccgagccgctgggatcgggtgcgtgaccgggcgcgcgccgccgtcatcggctggctgcaacgcggcgaagcacgccgccgcgaagcccatgcgttctgaagcgatgatgaacaaggttcaacctatcaagatcgcgatcctcgccatgggtggggaaggtggcggcgtgctcgccgactggatcgtcgacatgggcgaggccaatggctatgtcgcccagaccacgtcggtgccgggcgtggcgcagcgaaccggcgccaccatctactacgtcgagctgtaccccgcgtcgcaggccagggcggacggcggacagcccgtgctggcactgatgccgttgccgggtgacgtcgacgtggtgctggcgtccgaactcatggaagcgggccgcgcggtgcagcgcggtctggtcacggccgaccgcaccacgctcatcgcctcgacgcaccgcgtgttctccatcgcggagaagagcgcgctcggcgatggccgcgttgacagcgcccagctgctcgcgcacaccgcaagagccgccaagcgtttcatccgcttcgacatggcgcaggcggccgaggcttcgggcagcgtgatcagcgccgtgctgttcggcgcgctggcgggctcgggcgtgctgccgttcagccgtgcgcagttcgaggccaccatcgagcgcggcggcgtgggcgtcaaacccagcctcaaggcctttggcgcggcgtttgcgcgcgcccagggtggcgacgatggcgagacgccgccggaggcggttgtcgccatgccggcgccccagcctcgccaccccgcggtgcgcgcgctggtcgaacgcgtgcagcacagtttcccgctcgccgcacaagactttctgctcgaaggcgtgcgccgcctcatcgactaccaggatccggcctacgccggcctgtacctcgaccgcatggccgccatcgccacgctgcccggcagcggcgatcaccgcctgccgcgtgaaaccgcacgccaccttgcactgtggatgtcctacgaagacaccgcccgcgtcgccgcgctcaagacccgcgccacccgcttcgagcgcgtgcgcggcgaagcccgcgtgcagccgggccaggtgctcgccatcaacgaatacatgcatccgcggctgcaggaaatctgcgagacgctgccgggcggcatcggccgctggctgatgaattccacgctgccgaagaagctcgtcgagcgcttcacgcagcacggccgcgtgatccagaccagttcgcttcgcggctacctgatgctgcgcaccgtggcggcgtgcaagcgctggcgccgctccacgatgcgctatgcggaagaaaaccgccgcatcgaagaatggctgcagcgcattgccgccaccgcacagcgcaaccccgaactcgccgtcgagctcgcgcagtgccagcgcctcgtcaagggctacagcgacacgcacgagcgcggcatccgcaactacgacaccgtgatgcgcgccgtcgagcgcgcgggtacggcgctggcgcccgccaccttgcgcgagttgcgcgatgccgcgcttgccgacgaacacggccacaagctgcaggccgcgctggcgcagcacgcgctggcctgacgaagagacacagatgaccgcccaacccgtcacccttgaactgcgcattgccgaggtgcgcgaactgaatccgctgatccgcatgctgcggctgcgtgccgaagacggccgcgcgttgcccggcttcgcggccggggcccacatccgcgtcaaggtgtcgctgccgggcggcaaggccgactggcgtcattactcgctcatcaactttgcgaccgagcgaaatgccaccaacgcgccagccgaatacgtgattgccgtgcgcaaggaggccgaaggccgcggcggctcgcgcttcatgcacgagcagctcaagcagggcgacacgctcatcatcgaatcgcccaagaacgacttcccgctgcacacggggcccggcggttcggtgctcgtcgcgggcggcatcggggtcacgccgctgacgagcatggcggcgcggcgccgcgcggaaggcgccccggtgcgcatgcactacgcgggccgaagccgcgacctgatggccttcctgcccgagctgcaagcgctgctgggcgccgacctgcgtgtgcatgcggatgccgaggccggcgcgccgctcgacatcgatgcgctgctcgacgacgtgcccgccggcgaccgcctctatgtttgcgggcccaaggtcatgctcgacgccgtgctcgcccgcacccaggcgcgtggctgggaacacgaccgcgtgcacttcgagctctttaccgagcccgtcgcggaggagggcgaccagcccttcgaggtggagctggcgcaatcgggccggcgcttcacggtgccggccgaccagagcatcctcgattgcctgatcgacaacggctgcgatccgatgttcgactgcaagcgcggcgaatgcggtgtgtgcgccacgcccgtgctcgaaggcgagatcgaccaccgcgactatgtgctgaccgcacgagagaaggcggaaggcaacgtcatgcagatctgcatctcgcgcgcaaagggcgcgcgcctggtgctcgacatctgaagcaaggagccacgagaaccatgacctcgtaccgagacaatcccgaagcggtccgcgcgctggtccagaacgaccgcgtgcatcgcgacctgtacatcagccaggaactgttcgagctcgagcaggagcatttcttcgccaacacatggaactacgtgggccacgagagccagctgcccaagccgggcgactggatcagcaacgagattgccggccgcccgctgatcgtggtgcgccacaccgacggcagcgtgcgcgcgatgatgaaccgctgcgcccacaagggctcgcggctggtgaacgggccctgcggcagcaccggaaaattcttccgctgcccctaccacgcctggaccttcaagaccgacggctcgctgctggccattccgctcaagaccggctacgagaacacggcgctgcacgaatgcgagtcggccaaggggttgaccacgctgaagcacgtgcgcagctaccgcggcttcatcttcgtgaagatcaacgacgcggggcccggcttcgaggagtacttcggcgattcgctgagctccatcgacaacatggccgaccggtcgcccgagggcgaactcgagatcgcgggcgggtgcctgcggttcatgcaccagtgcaactggaagatgttcgtggagaacctcaacgacaccatgcatccgatggtggcgcacgaatcgtcggccggcaccgccaagcgcatgtgggccgacaagcccgaggacgagcccaagcccatggcggtggagcagttcgtgcccttcatgtcggactacaagttcttcgaggacatgggcattcgcacctacgaccacggccacagcttcacgggggtgcacttcagcatccacagcaagtacaaggcgattcccgcgtacgacgacgccatgaaggcgcgctacggcgaggagaagacggcgcagatcctcggcatggcgcggcacaacacggtgtattacccgaacctcaccatcaagggcgcgatccaggcgatccgcgtggtgaagccgatctccgccgacaagacgctgatcgagagctggacctttcgcctgaagggcgcgccgccggagcttctgcagcgcaccaccatgtacaaccggctcatcaactcgccgttctcggtggtggggcacgacgacctgcaggcgtatcgcggcatgcaggccgggctgcacgcgagcggcaacgactgggtcagcctgcaccgcaactacgaaccttcggagctgaagggcggcgagatcacgactggcggcaccagcgagctgccgatgcgcaaccaatatcgcagctgggtgcagcgcatgacggagaccatgtgatggccggcacctcggaagtcacccgccaggacctgatcgacttcgtcgtgaacgaagtgcacctgctcgacacgcgccgctacgaggagtggaacgcgctcttcaccgacgacgccttctactgggtgccgctcgtgcccgaccaggaagacggcatcaaccacacgtcgcatctttacgaggacaagctgttgcgcgacctgcgcatcgagcgcctcaagagcccgcgtgccttctcccagcagccggcgagccgttgccaccacctgcttcagatgccggtggtcgagcagttcgacgccgagggcaatcgtcatgtggtgcgcaccgaattccattacaccgaatcgcagggcgatgagctccagttttacgtcggcaccttcttccatcacctcacggtgcaggacggcgcgctgcgcatgacgctcaagcgcgtcaacctgctcaactgcgacgcggccttgccggccgtgcagcttttcatctagggacgcgatgccacacgtcaccgtccatcaagtcttttcggccactgctgcgcgcacgccgcaggccgagtttctgttcaccgagtcggtgaccgccgcggcttacggcattccggccggcgccatccgctggggtgaggcggcggcggaagtcgagcggctgcgcgcggcttatgcgcaggccgggtacgggcacggccatcgcgtcggcctgctgctggagaaccggccggcctttctctttcattggttcgcactcaatgccctgggcgtgagcgtggtgccgatcaatgccgagatgcgctcggccgagttgacctacctgatcggccacagcgagatcggcttggccgtgacgctgcccgagcgtgcgaacgacctgagcgcagcggcgaaacaggccggtgtgcccttcgagaccatggggcccgacgacgcggtgccgaaagcgaagaccgccgcaccgcgcgcgcatgagccgattggcgccgacaccgaatgcggcctgctctatacctcaggcaccaccgggcgtcccaagggctgtatcttgagcaacgcctacttcctgcgcgccggcgagtggtacgccgcgctcgacggcgtgtgcagcatccggcccgatgccgagcgcgtcatcacgccgctgccgctcaaccacatgaacgcgatggcgttttccaccatggtggtgctggtcgcgggtggctgcctggtgcagctcgatcgcttccacccgaagacctggctcgcgagcgcgcgcgaaagcggcgcgaccatcgcgcactaccttggcgtgatgcccgcgatgctgctgtcggcgcccgcttccgcggccgaccgggatcatgcgatccgctggggcttcggtgctggcgtggaccgcaagaaccacgcaccgttcgaagagcgcttcggctttccgctggtcgaggcctgggccatgaccgagactggcgcggccgcctgcatcatggccaaccgcgaaccgcgcctggtgggcaccagctgcttcgggcggcaggaagacttcgtcgagattcgcctcgtggccgaagacggcggcgaggccggcgtcgatgcaccgggcgagttgctcgtgcggtccgccggcgacgatccgaagcgctatttcttttcgggctatctcaaggacgaggaagccacgcgcgaggcctgggcggacggatggttccacaccggcgacctggtgcggcgcgatgccgagggcaacttcttcttcgtcgaccgcaagaagaacgtgatccgccgcagcggcgagaacatctcggccgtggaggtcgagagcgtgctcaaccagcacccggctgtgaagacctcggcggtcgctgccacgcccgacgcggtgcgcggcgacgaagtgctggcctgcatcgtgatgcgcgaaggtgcggatgcctccgcgcgggaagcgatcgccgccagcatcgtcgagcacgcactttcgcagttggcctactacaaggccccgggctacgtggcttttgtcgatgcgctgccgcttacgccttcgcaaaagatccagcgtggccagttgcgcgagatggcgcagacgctgcctgggcagggccattgcatcgacacccgttcgatgaagaagaggcaggcatgacgaagcgacgactctcctacgaaggcgtcgcggtggccgtgccggtcaccgtgccctacgtgcgctactccacgcgcaccgcgcactggttcatcgggcaggccatcgaggcgctggtgcagaccagcggcgtcgccaaggaacagatcgacggcctctgcctcagcagtttctcgctcgcgcccgacacggccgtgggcgtgacgcagcacctgggtctgtcgccgcgctggctcgaccatgtgcccaccggcggtgcctcgggcgtgatgtgcctgcgccgcgccgcgcgggccgtgcaggcgggcgatgccgacatcgtggcctgcgttggtgccgataccaaccatgtcgattcctttcgccagacgctcggcagcttcagcaactttgcgcgcgatgcgagctacccctacggctccggcgggcccaactcgatcttcgccttcatcaccgccaactacatgcgcacctacggcgcgaagcgcgaagacttcggccgcatttgcgtggaccagcgcaccaatgcgctcggtaatccgaacgcgatgttcaagaagcccctgacgctggaggagtacatggccgcacggccgatctccgacccgatccatctgttcgactgcgtgatgccctgcgcgggcgccgacgccttcctcgtgatgagcgaggagcgggcgcgcgacctgggcttggcgcacgtcgtgatccgcggcgccatcgaacgccacaacgcctatgccgaagacccggtgatggtgcagggcggctggcgcaaggaccgtgacgacctgtacgcgcaggccggcgtgcagccccaagcactcgacttcgtgcagacctacgacgactaccccgtcatcgtgatgatgcagttcgaggacctgggcttctgcgagaagggcgagggctcggccttcgtgcagtcgcacaccatgaccttcgacgggagctttccgaacaacacgagcggcgggcagctgtccgcagggcaggcgggcgcggcgggcggcttcctcggcatggtcgaggcgatccgccagctgaccgatcaggccgggcaacgcaccgtacccggcgcacaactgggcctcgtcgccggcttcggcatggtgacctacgaccgctgcctgtgcacaggcgccgtcatcctcgggagatcggcatgaccatgcccctgatgcgccccccgcgcaagaacccggtgctgcgcacccggcagatgaacctgccgcccggcgcgcgcggccgcgtggcgctcggcctcaccgcggctgctgccgaaggccgcttcgagctgcagacctgcgaggactgcggcacggtgcagtacccgccgcgcgaggtttgccacaagtgcctctccgccgcgctgcgttggcgcgcgcaaagcggcgagggcgaactgctcggcagcaccacgctgcaccacagcaacgacctgttctttcgtgagcggctgccctggcggctgggcctcgtgcatctggacgccggacccacgctcatggtccacctgcacggcgaggttggcgatgcgccccagcgggtgcgggtcggtgcccggctcgatcgtgcgggccaggccgtcctcattggttttccgaacgaagggagtgcccacatggccgacgacaagatgctccgtgaaatgaccagcgaccccaagttccgcaaggcgctggtgaccgacggcaagaccgagaccggccaggccatcgtgcgcgcgctggtgaaggccggcgccgacatcgtctgggtcggccatgccgagccctggaagaagatgggcgacgggctcgacgacatctcggcgctgccgcaggtcacgctggtgccgctcgacctgaccaacggccgccaggtgaccgagctcgcgggctcgattggcggcaaggtcgacatcgtgatcaacaacgccgaggtgcaccgtaccttcggcatcggcgcgcgccgtggcaccgacgtggccaaggccgagatggacatcaactacttcggcctgctgcgcctcgcgcaggagttcggccccgcgctcaagggccgctcggccgacggtgcgacgggcgcgacggcctgggtcaacctgctgtcgatctacgcgctcagcaactttccgccgcacggcaccttcagcgcctcgaaggcggcggcgcattcgctcgcgcagtgcctgcgcgccgagatgcggccggccggcatccgcgtgatcaacgtgttcccgggccccatcgacgacgaatggaaccagcacacgccgccgcccaagctggcacccaccgcactggccaatgccatcgtcaaggcgctgcgcgacggcgtggaagacgtgtaccccggcgacgtggcgcaggagtggctggaacgctggcgtgacaacccgaaggtgctcgagcgcgaactagcggcaggcggctgagaacaggagccacacgatgacgacaaccactgaactgatgtccgccgccgaaatcctcggcggcctggtgaccgccatggcgagcggccgcatccgcgtgatcgatctcacgcagacgctcacgcccgagtttccgcagatcgcattgccgcccgagatgggccaatgctggcccttccggatcgaggaagtgtcgaagtacgacgagcgcggccccggctggtactggaacaacttctcctgcggcgaacacacgggcacgcacttcgacgcaccgatccactggatctcgggtcgcgacctgccgaacaactcggtcgacacgattcccgtgcagcacttcgtggcgccggcctgcgtgatcgactgctcggccgacgtgcaggcgaacgacgactacctgttgagcgtggccgacatcgagcgctacgaagccgcgcacggccgcattccgaagggtgcgtgggtgctgatgcgcaccgactggtccaagcgcagcgacccggcggcctatcagaacttcgacgagaccggccagcacacgcccggcccgagcaccgaggccgtgcgcttcctggtggagcagcgcgacgtgctgggcttcggctccgaagccatcggtaccgatgcggggcagggttatcacctgcggccgccgtacccgtgccattactacatgcacggtgcggggcgctatggcctgcagtgcctgagcaacctcgacctgctgccgccgtctggcgcggtgctgatctgcccgccgctcaagatcgagaagggcagcggcagcccgctgcgcgtgctggcactcgtgggagcgtcgctatgaatcgttgccccggtatcggctttggctccttctcccgcttgcgggagaaggcgggggatgagggctcggcatcttgcgcgcacccacaccccaaccctctcccgcgtgcgggagagggggcaagacagggagcgcgcgcatgaacaaggtagcagccgtcaccggcggcagcgccggcatcggcaaggcgatctgcgaagacctgctcgcgcagggctacgaggtggtctcgctcgcgcgccgcaagaccgagatcgaccatccgaagctgcacggcatcgaggtcgacctgagcgaccgcgccgccaccggcgaagcggtacgcgaactggtcgatcgctttgcgccgaccaccatcgtccacaacgcgggcgtgatccgcgccgcgctgctgcccgaagtgaagctcgacgatctcgacgcgctggtcgacctgcacctgggttgcgcgatccagctcgtgcaaggcgcattgcctgcgatgcgcgcgcagcatttcggccgcgtggtactgctgtcgtcgcgcgccgcgctcggcctggccacgcgcaccagctattccgccaccaaggccggcatgctgggcatggcgcgcacctgggcgctggagcttgccgccgacggcatcacggtgaacgtggtggcgcccggcccgattcggaccgacatgttctacgacgtggtcgaggccggcagcgagaaggagcgcgcgctcgcggcctccgtgcccgtcaagcgccttggcgaatcggccgacgtggcacgtgccgtgcgtttttttgccgatccggccagcagcttcatcaccggacaggtcctctacgtttgcggcggcaccagtgtcggcagcctcgccctctagtcattcagcgttcttctcgttcatcccttacttctggagcatcgccatgaaagtcctgaaccgattccgtgccctcgcaggcattgctgccgcctttggtgcgctgggcgccgcgggcgcgtgggccgccgatctcaaggtcggtttcatcacctcgctgtcggggccggtgtcgtcgctcggcattccctatgagaagggcatgaaggcggccatcgcctacaagtcggaagtaggtggccggaagatccagctggtgcagctcgacgatgcgtccgatccgtccacggccgcgcgcaacgcccgcaagatgatcgacgaggacaaggtcgacgtcatcatcggcacggcaggatcgcccggcgcgctggccattgccggcgtggcgcgcgaaaccaagacgccgctgatctcgatcgccaacgccaaccttccgggtgaagagggcgcctggatggtgacgctgccgcagcctgcaccattgatggtgagcgcggtggtcgatcgcatgaagaagtcgggcgtgaagacggtcggctacatcggcttttccgatgcctggggcgacctggtgtacgacgcgctgcagaagagcgcggagccggccggcatcaagatcgtgtcgaacgagcgctatgcgcgcgcagattcgtcggtgacgggccaggtgctgaagatcgtcgcactgcgccccgacgccgtgatcaccggcacctcgggcacgcccggtgcgctgccttacctggcgctcgcggagcgcggctacaagggccagatctacggcatgcatgcgctcatcaaccccgacttcgtgcgcgtgggcggagcctcggtcgaagggctgctcgcacccaccggtccggtgatcgtggctgagcagctgccgggagagaacccgatccgcaaggtgtcgatggacttccgcgctgcctaccagaaggccaatggcgcgccgcccaccgatgccttctcggcctacagcttcgacgcctggctgctgtacctggacgccgcgcagcgtgcgcttgccaccaaggccgagcccggcacgccgcagttccgcctcgccttgcgcgacgccatcgtgagcaccaaggagctggtgggcacgcacagcgtctacaacttcaagccaaacgatcggtatgggtcggacgagcgttcgcgcgttgtcgtcaagcttgaaaagggccaatggaagctggttccctgaaatgaaaaaacttactcgcatcctcggcgccaccgccgtggcactggcagccgcgcaggccgtggcggccgacctcaagatcggcttcatcagctcgctctcgggcccggttgccgcattgggcgttccgtacgaaaagggcattcgcgcagccattgccgagcatccggagatcggcggccggaaggtccagctcatcgtgctggacgacgcctccgaccccaccaccgccggtcgcaatgcgcgcaagctggtgacggaggacaaggtcgacgtgctcatcggcacctcgggcgtgccgggcgcgatggccattgcctcggtggcgcgcgaactcagcacaccgctgatctcgcccacgccggtgaccatagccgggcctgaaggtgcgtggaccgtgacggtgtcgcagccgttcccgctcatggttgcgggcgtggtcgaccggatgcagaagtccggcgtgaagacggtggccttcatcggattctcggatgcgctcggcgacctggcctatgactcgctggtgaagagcgccgacaaggccggcatcaaagtggtggcgaacgagcgctacgcgcgcagcgattcgtcggtggccgggcaggtgctgaagatcgtcgccacccggccggacgcggtgtttgccggcaactcgggcacaccgggcgcgctgccctacatcgcgctggccgagcgcggctacaagggcaagatctacggcacacatggactcatcaacgccgacttcgtgcgcgtgggcggcaactcgatcgaaggcctccaggtgcccagtggcccggtgctggtggccgaccaactgcccgacagcaacccgatcaagaaggtgtcgatgggctttcgcaacgcctaccagaaggtgaatggcgcagcgccgaccgatgccttctcgtcgtacacctacgacgcctacctgctgttggccgacgccgcctcgcgcaccaagggcgaaccgggcacgccccagtaccgcaccgcgctgcgcgacgccatcgtggctacgcgcgagctggtgggcacgcatggcatctacaccttcaagcccgacgaccgctacggctccgaccagcgcggcgtggtgatcgtgcagatgaacaagggccagtggaagctggtgccctgaagacagcccgagcacgccgatgaccagctaccgccatcatcccgaacggatcgccgccctggtgcaggacgaccgcgtgcaccgcgacctgtacctgagcgatgagatcttcgcgctcgaacaggaacatctgttcgcgaacacctgggtctacctcggccatgcgagccaggtgccggagcccggcgacttcgtgacgcaggacattgcgggtcggccgctcctgatggtgcggcagcccgacggcgcggtgcacgtgatgtacaaccgctgcgcccacaagggtacgcagctggtgacggacgagtgcggcaacaccggtcgcttctttcgatgcccgtaccacgcctggacctacaagctcgacggcgcgccgctcggcctgccgctgaagaacggttacgagggcacgcagctcaaggcctgcgagtcggggcagggactttcggtggtcaagcacgtgaaggtgtatcgcgacttcgtgttcgtgcggctgtccgattcgggtccgtccttcgaggactacttcggcgaagtgctgggcgccatcgacaacatggtcgaccgctcgcccgagggcaagctcactgtcggtggcggcgtgcttcgcaatatcgtgcactgcaactggaagatgtacctcgagaacatcaacgacacggtgcatccgatgtcgacgcacgagtcggccaccaaggcggccgaggcgctgtgggaggggcgtgcgcccaccgatcccaagccgatggcgatggagcagatgctgcccttcggttcgggctatgaattcttcgacaagatgggcgggcgagtgttcgccaacgggcacagcgtgttgggcgtgaacttcagcatccattccaattacgcgcagctgcccgagtacgaggctgcgatgcgcgccgcgcacggcgaagagcgcgcggccgagatcctgcagcgctcgccgcagaactcggtcttgtatccgagcctgtcggtcaagggctcgccgcaggccattcgcgtgatccggccgctggccgcgaaccgcacactcatcgaggcctggagctttcgtgcggcgggtgcgcccgtcctgcttttcgagcgcgcgatgagctacaaccggctcgtgttctcgcccatgtcggtggtcgcgcacgacgacgtgcatctcttcgagagcatccagcagggccttcgcgccggtggcaacgaatgggtgagcctgcaccgcaactacgaccctgccgaactcgcgcaagagacgatcaccaccaacggaaccaacgagctgctcatgcgcaaccagttccgcgcctgggcgaagtcgatggcggccggcatggaggccgcggcatgaacggcgacccgcgcgattttgccgctcacgaggcagccctgctcgacgagcggcgcctcgacgactggctggcgctgttcgccgaagacggtcactactgggtgccgctgctcggtgcggcgcaggccgatccgttctcgcacaactcgctcgcctatgaagaccggttgctgctgcagcttcgagtcgatcgcctgaagaacccgcgtgcgcattcgcagcatccggcaagccacagccagcatgtgctgcagccttcgcgcatcgagcacgaatcggccggcgaagtgcggttgcgcacacccttcatctacatcgaggcgcgcggcgaagggcaggttttgctggccggcaccgcccgtcaccacctcgtgcgcacgcccgcaggaggctgggccatccgcgagaagcgcatcgacctgctcgacgccggccgcgcgttgcctgcgatccagttgttcatctgagttttcctttcatccatccttcctcactggagctacgacatgaagagcctgatgcagaccttgacgcgcggtgccctcgccgcggcgctgaccgcctgtggtgttgcgagcgcgttcgcggccgacctgaaggtcggcctgagcgtgtcgctgtcggggcccaattcctcgctgggcgtgccctatgccaagggcatgcaggccgcgctcgcctacaagccggagatcaacggccgcaaggtgcagctcatcgtgctggacgacggctccgacccgaccaccgccgggcgcaatgcacgcaagctcatcgaggaagacaaggtcgacgtgctcatgggcacctcgggcgtgcctgccgccatcgcaatggcccaggtgggcaaggaggccaaggtgccgatgatcggcctcacgcccatcctgctcgatccgaacgagaacccctgggtcatgacggtggcccagcccacgcagctgatgatcgatgcggtggtcgagcgcatgaagcgcaacaacgtgaagaccgtcggctacatcggcttcaccgacgcatggggcgacctggtctacaacgcgctcatgaaggccgcgcccgaggccggcatcaaggtggtgagcaacgagcgctacgcgcgcgccgacgcctcggtgaccggacaggtgctgaagatcgtggcgctgcggcccgacgcggtgatgaccggcggtgccggcacgccgggcgcgctgccgttccttgcgctgcaggagcgcggctacaagggcggggtgtacggccagcacggcttgatcaacccggacttcgtgcgcgtggtgagtgcttccgggcagaacgcgctgatgcccaccggtccggtgatcgtggccgagcagctgcccgacagctacccgaccaagaagatcgcgactgaattccgcgccgcgttccagaaggtcaacaacgcacccaccagcgacgccttctcggcctattccttcgacggctggctggtgtttgcggacgccgcctcgcgcgccatgaagaaggcggagccgggtacggcggagttccgcgtcgcattgcgcgatgccatcttcagcaccaaggaagtggtgggcacgcacggcgtgtacagcttcaagcccggcagcctctacggcgtggacgaacgtgcccgcgtgatcgtcaagctggacaacggccaatggaagctcgcaccttgaaccgcttgatgccaacgacgacgattctccgaggggcttttctatgacatgggacgtggcgctgatcctcgtcaccgatggccttgccaacggtgccgtctatctgctggccggactcgggctggtcttgatcttttccgtcacgcgggtggtgttcgtgccgttcggcgacatcgcggccttcgcggccctgtcgctcgcagccttcgaaaccggccgcgtcccgccgaccattggcatggtggccgtgctcgcggcgctggccctggccacggaaatcggcagcctgctgcggcgcggggaggccaagcgcattcccaaggcggtgctgatgtggggcgtgctgcccgccatcccgtgcctcctggcatggctggcggcacggcccggtgtgccggtggcggtgcacatcgcggtggccgtgttgctggtggtgcccattgcgccgctgctcgcgcgggtggttttccagccgatcgccgatgcctcggtgctggtgctcctgatcgtgtcgctggcgctgcactttctgctgtcgggcctgggccttctgttcttcgggcccgagggctcgcgcaccacgccgctcacgagtgcggtgttcacgctgggcgacggcttcacggtcagcggccaggtggtgctgatggtgggtgcggccatcgtgctgagcgggctcttcttcctggtgttcgagcgcacggtggcgggcaaggccttgcgcgccacggcggtgaaccgcgtcggcgcgcggctggtcggcatccggccagtgcgcacggcgctgctcgcctacggctgcgcctcgctgctggccgggctcatcggcgtgttgattgcgccggtgaccaccatgtattacgactcgggtttcatcatcggcctgaaggccttcgtggccgcgatcatcggcgggctcgtgagctacccgatgacggccctgggtgcgctggcggtcggcgtggtcgagagctttgcctcgttctggagcggcgcgctgaaagacgtgatcgtgttcagcctgctgataccggtgctcatgctgcggtcctttcttgcggcccatgccgaagaggaagaagaggaggtggaccagtgatcgacaacaacaacagaaacggcaagcgcatggcctggatcgccgcggtggtcgccgtgctggcgctggtgccggccgtggcgggcagcttcacggtctcgctgctcaacgacatcggtatcggcgcactggtggcgctcgggctggttctgctcaccggcgtgggcggtgccacgtcgttcggccaggccgccttcgtgggcattgccgcctatgccacggcatggctcactaccacgcagggcatgtcgccatggatcgggctgctgttcgcgctgctgctcacgggcttgtcggcgctggccatcggcatgctcacgctgcggctcggcgggcactttctgccgctcagcaccatcgcgtgggggctgtcgattgcgatgctgttcggcaacgtcgatgcgctcgggcggcacacggggctgtcgaacattccggcgttgcgcatcgcgggctggtcgctggccgatccgcgcgcgatgtattacctgatctgggtggtggtcgggctggcctgcctgttcagccacaacctgctgcagtcgcggccgggccgcgcgattcgcggcttgcgcggcggcgccacgctgctggcgagcgtgggggccgatgcctaccgtgtgcggctcacgctgtttgttacggccgcgctcttcgcggggctggcgggctggctctatgcccacatgaaccgcttcgtgagcccgtcgcccttcgacgtgcgcgccagcattgaatacctgctgatggcggtggccggcgggctcgggcagctggcgggcgcgctggtgggtgcggccctggtgctggtgctgaagaacggcctgcaagacgtgctgccgatgctcacacagcgtgcggggcaactggaggccgtggcgttcgcaacgctcttcatcctgctgctgcactttgcgcgtggcggactcatgggcctgctgcggcgctggacgcgccggcgtgccggtgcaccaggtgcttcgcgctaccaggcgcccacggtcgatcccctgccgcacaggcagctgccacagcgcggcacgcaggtgctgtcggtgaagggcgcggtcaagcgattcggcggattggtggcggtcaacgacgtgagctttgaagtgaacgcgggcgagatcgtcggcctgatcggacccaacggcgcgggcaagtcgaccatgttcaacctgctgacctgcacgctgccgatgagcgcagggcaggtgcgctttctggaacacgacattgccggcatgccgcagcggcaggtggcgcggctgggcctggcgcgcactttccagcacgtgaagctcaggccgcacatgagcctgctcgacaacgtggcgctgggcgcgcattcgcgcacgcgctcgggcatcctcaaggcgggcctccggctcgaccgcaccgaagaaaagcagatcctgcaggaagcgcagcgccagctcgaccgcatcggcttgggcgaccgcgcgcacgagttggcgggcagcctgccgctgggcacgcagcgcatcctggaaattgcgcgcgcgctggccgccgacccggtgctgctggtgctcgacgagcccgcggctggccttcgccgcaaggaaaagatggcgctcggcgacctgctgcgcaagctgcgcgaggagggcgtgaccatcctcatcgtcgaacatgacatggacttcgtgatgaaactggtggaccgtctggtggtgatgaacttcggctccaagctcgtggaaggcgtgccctcggccgtgcgtgccgacgagcgcgtgcaggcggcttacctcgggagcgtcgtatgagcgccgcacggccgcccgaaggcgcgggcccccttgagggggtgggcgtcgtacacgaagtgacaagcctgggggtgatgcaatgaccgcaatgctggagatcggcgacctgcacgtgtcctatgggcaggtcgaggcggtgcgcggggtttcgctcgagctgcagccgggccagatcatctcggtgatcggccccaacggcgcgggcaagaccacgctgcttgcggccgcgatgggcctgctgccctgcaagggcacgctccgcttcgagggcgaagacctgcaggggctcgacgtggaggcgcgcgtggagcgcggcctgtgcctcgtgcccgaaaagcgcgagctgttcggcgagctcacggtgctcgacaacctgcagctcggcgcctatgccaagcggctgcgcagcgatgcgatgaagcggcagctgcagtcggtgtacgaccgctttccgcgcctggccgaacgccgctcgcagcgcgccgacacgctctcgggcggcgagcggcagatgcttgctgtgggccgggcactcatgtccgcgccgcgcctgttgatgctcgacgaaccgagcctcggcctggcgccgctcatcgtgcgcgacattctttccatcgtccgcaagctgcgcgaagacggcgtctcgatcctgctggtggagcagaacgcgcgtgccgcgctcgaaacgtcggaccacggctacgtgctcgaaaccggcgagatcgcgctctcgagtgcttcagccgaactcgcgagcgatccacgggtgcaggccacctatctcggcggaggcacgcacgatgacgaatgacccgcgcgcggtgccggccgctcagcgcacgttgcccgacatgctgcgccgacaggcggcgctgttcggctcgcgtccgctgctgcgcatcgcgggccgccaatggtcgcattccgatgcggccgaagcggcgggcgttcgagcggccgtgctggcgcaagcaggcgtcgcgcaaggcgaccgcgtcgccgtgatgtgcggcaatcgcatcgagtttctcgaaacctttctgggagccggctggctcggcgcttccacggtgccggtcaacaccgcctccatggggcctcagatcgggtacttcctggcacacagcgaggcaaagctgctggtcatcgaggccggctttctggaccgcctgcagaccgcgaacctggcgcaggcgaagctcgaagaaatctgggtcgtcggcgatgcgccggcggccggcggtgccgcatggcagccgccggccggcgtgcggattcgggcctatccaccgggcgggatgcccgctattccgcccgccaatgtgcagcccggcgattcgctggccatcctgtatacctctggcaccaccggcccggccaagggcgtgatctgcccgcacgcgcagtatttctggtggggcgtgaacagcgcggaggtgcttggcgtgggcgcggacgacgtgctgtgcacgaccttgccgctctttcacatcaatgcgctcaacacctttgcgcaggcggcgctcacgggttccgaggtcgtcttcgaaacgcgtttctcggcgtcgggcttctggccttcgatgcgtgcgaacggcgccaccgtggtctacctgctgggcgccatggttccgatactgcttgcgcagcccgcgggcgatgcagaacgccatcaccgcgtgcgcaccgggctcggccccggcgtgcccgaggccgcgggcaagatttttttcgaacgcactggtgtgcgcctgctcgaaggttatggttccacagaaaccaactttgccattgccaccgcgcctgattccccgcgcggcggcgtgatgggctggcttcggcccggctttcaggcgcgcgtggccgacgaaagcgatgtggaactgcccgccggagaggccggcgaactgctgctgcgcgccgacgagccgcacgccttcgcgagcggctacttcaacatgcccgagaaaacggtcgaggcctggcgcaacctctggttccacaccggcgaccgcgtggtgcgcgatgccgacggggcctttcggtttgtcgaccgcatcaaggacgcgatccgcaggcgcggcgaaaacatctcgtcgttcgaggtcgagcaggtgctgctgagccactcctcggtcgcctcctgcgccgtgtacccggtgcaatccgaactggccgaagacgaggtgatggctgcgctggtgccgcgcgacggggagcgcatcgaccccggcgaactggttcgcttctgcgagagccggctgccttacttcgcggtgccccgctacatcgacgtgctgcaagacctgccgcgcaccgagaacggcaaggtgcagaagttcaagctgcgcgagcgcggcgtcagtgcacagacctgggacgggcggccttccgctcgcgcccccgccaagacggcatgaattccgcgccgccaccgcttcaaggccaggccgccttcgttactggagcggggcagggcctgggggcagccattgcgcgcggccttgccgaagcgggtgcgcgcgtggtgcttgcggacatcgacgcggacaacgccgagtcggctgccgcgagcttgcgcaacgcgggcgccgactgcatcgccatgaagctcgacgtgcgcagcgaagccgatttttctcgctgcttcgatgcggcgacggctcgttatggcgccatcgacgtgctggtcaacaatgcggcgcgcacgcccttcagctccatctgggacatcacgcagggcgaatgggacgacgtgctggccgtcaacttgcggggcagcttcttcggctgccgcattgccggccggcacatgcgccagcgcgggtccgggcgcatcgtcaacctggcgtcgatggccggccagcaagccagtgccaccaccggcgcgcactatgcggccagcaaggcggcgctgcttgccctgacgcgtagctttgcgcaagaactcgcaccgcatggcgtcacggtgaatgcgttggccccggcggcggttgaaaccccagccctcgacacgctggcccccgcacggcagcaggcgctgaaagctggcattccgctgggccgtttcggccgcccggaagaagtggcagccgccgtggtctacctggcatcgccagcagcggccttcatgaccggtgcaacgctggatctcaacggcggccgcttcatgcgctgaacaggcgatgagccggccacacgcgctaaaatcgttcagaactaaataattcaggtatgcacgcaaattcattgattggccgccacgctctcgttactggcgccgcgcgcggcattggcgccgaaattgcccgcacactggctgcggagggcgcaacgctgaccttgctcgggcgcgaccccgatgcgctccaacgcgtggccgccacgctcgcgggccagggccacggcgttgcttctgccgacgtggccgatccacaagctgtgcagtcggcctttgcgctggcgcgcgccgagcgaggcccggtcgccatcctcgtcaacaacgccggggctgccgagagcgcgccgcttctcaagacctcggtcgagctctggcagcgcatgctgtcggtgaacctgaccggcagtttcctgtgcgcgcaggcggcgctgcccgacatgctcgaagccggctggggccggatcgtcaacattgccagcaccgcgggccagaagggctatgcctacgtcgcggcctattcggcggccaagcatggcgtgatcgggctcacgcgatcgctcgcgctcgaagtggcgcgtaagggcatcaccgtgaacgcggtgtgcccaggctacaccgataccgacatcctgcgggcaagcgtcgccaacgtggtgggcaagaccgggcgcagcgaggtcgacgcgctggccgagttctccagcgtcaatccgcagcggcgcatcgtgcagcctgccgaggtggccgacgcggtgcgctggctctgcggcaacggcgctgcatccgtcaccgggcagtcggtctcggtgtcgggcggggaggtgatgtgatgcgcaacgatgcctcgcacgccgcactcagcgatgcagaagaacttggccacgaggcccgggcgggccgcgaagaccacgccatgctcaggctctggctgcgcatgctcgccagcaccacgcagatcgaagccgagatccggcgccggctgcgcgagcgcttcggcatctcgctggcacgcttcgactacatggcccagctctaccgctatgaagaaggcctcaagatgcgcgtgctgtcgcgctacctgatggtgaccggcggcaacgtcacgggcctgaccgacgaactggagcgcgacggcctggtggcgcgcgcgcacagccccgacgaccgccgctcgtggatcgtgagcctgacgcccaagggccgcgcgagcttcgagaccatggccaaggaacacgagcagtggattctcgaaatgttctcgggcctcgacatgaagaccgtcaagcagatgcacacgcagctcggccagctgcgcgtgcacgtgatgcgcagcgagccttcgggcgaggagggctgacgatgacgagcgcagcagcagaagccgaggcgcaagaagaagcccccatggccgagttccagcgaccgcggatgatccgtttttcggactgcgaccctgcgggcatcgtcttctatccgcagtacttcgtcatgctcaacggcctggtggaagactgggtgagcgaggggttgggcattgactaccacgcgctcatcagcgagcggcgcatcggattgccgacggtgcgactcgaggccgattttcgcgccgtgagccgcatgggcgacaaggttacgctcggcctctcggtggagcggctgggctcgcgctccatgacgctcgtgctgcgctgcttcgaccccgccagcggcgaactgcgcatgcaggtgaagcaggtgctcgtgaccacctcgctcgaaagccaccgggccgtcgaaatcccgcaggatatgcgcacggccatcttgcgcggggcgccgtcactcgcttgaatgcatggtgctggcttccgttgcgcagtgcctcggcggtgcgccggcgggcagacggagcgtgcgagagctttcgcttgcgctatcggacatgggccttgaatatctcgacttggactggcgcgcgaggagccgaggactggtagtacctcaaccatcgatacagatatgaaagagtcccggatggacaagcaaacaatcatcgaaagcctggagcgggctttggaaagctggatccgccatgctgtcgctgcccaactgtggcaggttcagcagcaaggcggtttgggtgcgtccatcgtggtggaggaagacctcgtgcacatccgcgtcgaactcggcggtccacgcaacccgctgtcggagttgggccaaaccgatggacgcttgcccgtaacggaggcctttctcggccgcggagtcgcatcttggggcaccccacctccacagggagaagacgaggcgcgcgaggcatggttcttgtcgagcgagctcgcccaagagcacgcgcggcaatacctgctggcggaggtgagagaaaagcgggacgtcctgtcgcggtttgtcgagggctggttgaccggtgagtcgtagccgttgagccaataaaaaagcccgctaccgatgaggtagcaggcttttcagcgtttccgcgatgttggttggtgggccctgagtgactcgaacactcgacctacggattaagagtccgctgctctaccaactgagctaagagcccttgcactggaaaacgttttgcgttttttggcaagaccgcaagtatagcgtaaaaattcctgggttcaacgattttgtgcggggcggcgttagcattggccatcatccgacgggtcccggggggccctccaccaggagaatctttcatgacagatacaaccaccatgcctcatgttgtgatcacgggggccgcgggcgcgctggggcgcgcagtggcgcagcactttctggagcagggcgcacgccttgcgctggtcgaccaccatgcggatcgcctgtccgaggtctttccgggtctggacaattcgcagcacctgctgctggcgggcgacgtgacctcggcgtcggacatgtcggagctcgcgggccaggcactcaaggctttcggccgcatcgatgcgctggtccacattgcgggcggcttcgagatgggcgaggcaacccatgcgctcacgcgggccagctgggaccgcatgatgaatctcaacgcctggtctttcgtggcggttacacaagcggtgctgccttcgatgatcgagcacggcaccggccgcatcgtggcggtcacggccaaggtggcggcgcgcggcctgccggccatggcggcgtatatcgcatcgaagagcgcgttgcagcgcctggtggaagccatggcggccgaggcggcgccgcatggcgtggccgtcaacagcgtggcccccagcgtgctcgacacgccagccaaccggcaggccatgcccgacgcgaatcccgcggaatgggtgtcgacggcggtcgcggcgcagaccatcggctttcttgcatcgcccgcagcggcggcgctgcatggccagcatctgacgctcgacacctgagcccagatcgctaccagcaagctggctcgatagatcagtagctacacagggccctggcgcaacgccagggcccttttttgtcctcttccgccgcaatggcgcgccgactctggggcaggcgctttgtcatggatgcggccagggtgggcggggcgcttgtctcgcttcagaaggggcgcaccgctcatgtgcccaggcggcgcaatttctacagtgaccccacggcgaaacgtttgagcccgatgagggcaacaagcagcgccggccgaccacatcactggggacacgcatggaaccgcactacttgccgccaagaaatttcatgaacctgctgcgggaagacgctggcatgtcgttcatggaattcgcgttgctcggttccctcgtggtgttcgtgagtttgttgctgctgcttgcagcacggcgcggcgcctgaatgcgcaacagcagatcaataacaacgccatacggagctgtccatgcgtgaattcgatgccttcctcgagctgctggcgatgctggcaacggatttccgcatggttgcgctgcttgtcctgctggtgacggccgcggtcagcgacttgcgcacctatcgcattcccaactggctgacgttcggcggcatggtcttcgcggtgatctacggaaccttcgcggcgcgcacgccgctggtgggcgcgacgcaggcactgggggggctgggaacaggccttttgatcatgctgccgctctatgcgctgggaatcatgggcgcgggcgacgtcaagctgatggcgatggtcggcgcctttgtcggcccctatcaaacgctgtgggccattctcctcacctgcattgcgggcggtgcggccgcgctgattgttgccatgcaccggcgccgcctcggccacatgctggccaacgtgaaggacaccgtgaacggcatggcgatgtcgggcattgcgggcctgcggcccaacggaaccatcgacatgcagcaatccgtcggaaagctgccttacggaatctgcatttgcgtggggacggttgcacaggtcctggcgcatcaactgggctacgtgtagtccgccactttcattccaccgcactcggagattcgcatgaaaaacatcaaggcactcgggctgctgctgctggccctcctcactggtctggccgccgcagtctacgcggcgggatgggtctcacgacaagggggaatcgcttccaacaaggtggtagtggccgcggtcgacatcgagttgggcagcagggtcaacccgcagatgctgtcgctggtcgactggccgagcggctcgctgccggcggggtcgttcaaggacgccaaggcgctcgaagaccgggtggtcaaggtcggggtgctgcgcggcgaagccattctggagggcaagctcgcgcctgtcggcaccaagggcggcctctccgccgtcattgccagcggcaagcgcgccatgaccgtgcgggtgaacgacgtggtgggcgtggcgggctttgcactgccgggcaactacgtcgatgtgatggtcaacgcccagcaggacaagaaccgtggcgaggagaaccgccagatcagcaagacagtgcttgaaaaggtgctggtgctggcggtggcgcaagaggccaaccgcgacgagacaaaaccgaaggtggtcagcgccgtgacgctggagctgtcgctcgaagactccgaaaagctcgacctggcacgcagcgtgggaaccctctcgctggtgcttcgcaaccagatggacaagaccacggtcgccaccgccggtattaccaagggccagttgttcggcgagaaggaaatcctgccgatctccaccaccgtggcagcgcggccggcccccgcgcgagtgccgcgggccgccccagtggcgctgcggcaacccgagtgcgtggaagtgatccagcacgcagcccgctcgctcacctgcttctgatctcaatcccgccaggaggaaccacaagtgcaacatctctcttcttcatccgcctggctgctggcggcgctcacgaccttggcagcgccggggtttgcagcggagcctgcagccccggctccgaccctgaccccggtcgccgcgccatcggcacccgcgccagccgccgcacccgccatgcgccgatgcacggccatcatcccggacgaccagccgacctacgccgtgctcggcaagtcggtggtgattccgctcaaggcgcgtgttgcacgcatcgtggtcagcggtcagccgccaagcggtgcgccagcggccgcaccggccgctgcaggcgctccggcacaggcgcccgccgcgatgcgaaatgcaggtgaaggcgttgcggatgtcgacgtcatgctgctcagccccaccgatcttttcttccgcggccgccaggccggctcgatgaacgtggtgctgcagaacgccgaaggcacctgctacatcaaggacgtcatcgtcacgattgatccgggcgcgctgcagtccaagctggccgagctgatgcccgaagagagccggatccgcgtgcgcagcgcggaaagatccattgtcctcacgggtgaggtgagcgacgcgctcaagctcgacgacgtgatgagtcttgcgcaggcctacggtgccgatggcaagaaggtggtgaacctgctgcgcatctccacgccgcagcaagtgatgctcgaagtgaagatcgcagaggtcagcaagacgctgctggaccgcctgggtgcgcgcgttggcctgacccgcacagccagcggcgggctcaacacctattcgctgatttcagacttcctgagcggcggcgcgggccttgccgaggcgttccggatcggccgtgcatccatcgccatcgacggccagaaggacgacggcctggtgcgcatcctggccgagcccaacatcatgtccatcagcgggcagcaggccagcttcctgtcgggcggaaagattttcatccccgtttcgcagaactccaacggccgcagcggctcgaccatcacgctggaagaaaaagagttcggcatcggcgtgaagttcacgcccaccgtgctcaacggcggacggatcaatctcaagatggtctcggaagtgtcggacctgtcgcagacgggctctcccttcaccaccgtcggcggcgtcacagccgtgctgccctcgctcacggtccgccgcgcagacaccaccgtgcagctcaacgacgggcagagctttgtcatcgcggggctcatcaagagcaactcgaccgaaaccgtgaagcgctacccgggcctgggcgaggtgccagtgatgggggcgctgttccgcagcaccgagttccagaacgaccagaccgagctgatgttcgtgatcacaccgcgtctcgttcggccgctgggcgaatcgcctcgcgttccgaccgacaaccacgtggttccaagccgcgccgagaggtacctgaacggaagtctcgaaagcagcacccctgccccggtcgcaccggccagcaaccccctgtaaggagcaccaccatgttcttcaagtcgaccattctcgcgctgagcctgctcgtgggcaccggctgctcccacgtcacaccccactacgacgcgcgctttggcgatgccgtgcgcgacgccaaaagaaagatgacgctcaaccccgatgccggcaaggacgggaatccggtggtgggcatggacggccgcgcagcacgcgagtcgatgctgcagtaccagaaatcctacaagtcgccgcccccggcggtgaacgtcatcaacatcggcggcgcgatcggcggcgaaaagtagcgcattcgttcatcgaccgattgcacttcttctcatcgctcgctttttcatcaaccagctttgtatgaaaggagagtcacgaccaaagtcatcactcttatgcaacgcagttcactcattcagtaaatcttgttttctcatttgaaccttgaaaggaaattctcatgtccaacattcttcaatccattggccaatttacccgcagcttcctccgtgacgaagagggcgcccaggtcgtcgagtacgcactgatcatcgctgtcgtttcgatcgcgctggttgttgcattgcaagcgctcacggcagatgacggcggctttgcagatttcatcactcgcgtcacgacctgtctgaccacggctacgtgcgcgtaagcggcagtgaagcggatcgggccttgcccgaaccgcttccctttcgacaccactcctcggtcttcccaagcaaagaggtagccatcatgtgcaagtcattcctgcaggacgagagcggcgctcaagttgtggagtacgcgttgatcattgccgtcatttcgatcgcgttggtgctcgcgcttcaaccgttgtcgattgccagcagcttcggcagttttattgaccgcgtaaccgcttgcctgagcggcggggactgcgcctgagtcgaccccattcgaaccgccgtcattccaccggagccgatcatgcaagttcgccgccctcagcgccgccaacgtggcgcaatgatcatcacagccgcactggtgctgctgtttctcttgggcttcatgggcgttgctctggacttcggccgcctgttcgtcgtcaagaccgaactccagaccgccgtggacagctgcgcattggccgccgctcgcgagctcgacaaacagggcacggccatcgagcgcgctcagagcgccggccagacggccggcaacgcgaaccgcgtgaacatgcagtcggccacctggagcggagagggccagatcgttctcgccgacatcacctttcgagatgccgcctatgcgcccacgaccaatcctctcgtggccacttatgcgcaatgcgtgcacacccagcccaacatcgaggtctggctcatgaaagccatgggggccttctctggcgacaccgctggcaatcccgcaacccgcagcgttgcggccagcgcggtcgccacccgtgccagtgcacagacgacctgtcccattccggtcggcgtgaaacccaaggcgggcggcgtggcgcccaactacggcttcgtcgtcggcgaatgggtgaagctgatccaggcccagaacggggccgccggcggcgagatcggctgggccaatctcgatggaagcaacagcgcctcggagaccgagtccgagatgaacaaccactgcggaaccaaggtgggtgacgtgctcggcacgcccggcgtccaggcctcgatcgtcgacgtctggaaccagcgcttcggcatctacaagaacagtggcaatccgagcacgcagcggcccgactacaccggctatgcctacacggccctcaactggcccgcgcagttcaatgcctacgacggcccggctcctggatcgcctgcaagcgcccagaactacgtggccaagcgagcggtctttgcttcctgcgccgataccggcaccaacgtgaagggcgcaaacggctgcgaagcgatcaccgggctgtcgctcaacggctttcagaaactggcagcgccaggcgacgtcgcaggcggccacaagcaatacgggttcgatcggcgcatcgtcacggcgccgattctcgacggcgccgggcatgtgatggactacgcctgtttgctgatgctgcagccgctgagcattccaatgaccgatacgtggctggagtttcgcggcaatgcaggcgccgtgggcagcccctgcacgacgagcgggctccccggcggtgctgcggggccgctggtcccggtcctggtgaggtgacgcacatgaaaaaagcatccaaccacagccagcgcggcgcagcgctgatcgagttggcgctcattacgcctctcttgctgcttctcactttcatcacgaccgagttcggccgggccatgtacgagtacaacatcgtcgtgaaggccagccgggatgcggttcgctacctgtcggtgcagacgccgggcacgaacatcaccgaggcgcgcaacctgatggtgtacggcaacaccgccggcacaggcacgccgctggcccccggcctgagcttgctgaacgtgcccgcagacagctgctgcacctggcagtcggcgggggcgaacccgctcatcaacacggtgtcggtgcgcatcagcagctacaccttccattcgatgtttccgtcggtgatgggcatcgtgtttgccgatgcaaacggcaacatcgtcttcagcgacatcactgccaccatgaggtctccatcatgaaacgccagatggccggtgccaccaccgtcgagtttgcgttgggcctgctcgtctttctcatgctggtcctgggcatcgtggacttcgcgcgcatgctgttcacctggagcgcggccaacgaggccacgcgtgcgggcgcgcgctatgcggtggtctgcgacgacaccgcccagcaggcactggtgcttgcccgcatgcaagctttgctaccgcagatcaccacggtgagcgtggcctggatgccggcgggctgcaacgcagccacctgccagggtgtcacggtgggcatcaccgggctcaactaccaatggatctcgcccatcgtgggcgcggcggcgccgctgatcccgatgccgagtttttcgaccttcctgccgcgcgaagtgatgcggaacgaccctcacagcccaaccatctgctcgtaaagacgaaacggaccctgccatgaagatctccctcatctcgcccaacccggcccacttgcaggaaatgcgcaagatactcgaggcgcgctcccacgtcgtctcggtgtttgaaggaggcaagagccgcatgcaatgggttgtcgagcgatcggctcccgacctgatgctggtggacggcatgtgctgcgacccccacgagctggagatggtcgagcagctgaccatgcgccaccccgccatcgcagtggtgctgctttgtgccatgcaaacgcccgagttcctgattcttgccatgcgttcgggcgtgcgagaggtgcttccttcgccgccccaacccgcggcgctcgaggccgccgtggagcgcattgcgctcaagatggccggcacgctggcacgcgagccggcgcaagtggtcgcgttcatgccgtgcaagggcggcagcggcgcaacctttctcgctaccaacatcggccaccaattgtcgatgcggcgctcggttctgctcatcgacctgaacctgcagttcggcgacgcgctttcctatgtgagcgacctgcggccgacgtccacggtggccgacgtggcccgcgacatcggcaggctcgatgcttccctgctcgccgcaagcgtggtgaaggtggcgccaggcttcagcattcttgccgcgccggatgatctttcgcgtgcgttggaggtcaaggccgagcacatcgacgcgattctccaggtggcctcggcgcagtacgacttcgtgctgttcgacctcggcctgcgcatggatccgctcaccatccgcgtgctggaccgtgccgaccgcatcttccccgtgctccagccgagcctgccgcacgtgcgcaacgtgacgcgcctgatacaggtgttcaagtcgctgggctacgcggccggcaaggtcgagctgctggtcaaccgcagtgccggaggcacggagatcgggctgtccgacatgcggcgttcgctcggcggggccacgctggtcagcgtgcccgacggcggcaaggacgtggatgcatcgatcaaccgcggcgtaccgctggcggacatgtcccgaagcagcccgctctgcaagcggcttgcggaaatcgctcacacgctcagtccgcgtcccaaggaagcagcgggcttcatcggccggcttttccgccgcgcctgagcgcctggttgtttgctgcagatgttttcttccctatcccttcttccatagcaaggcaggttccccatgtcatttcgagaacagctcaatgcgatcgaagccgagccggtcgtgcagtcggcggggcggccctcggccgagacgacgctttcatctttcgcctcggacacctacaagctcttgaaggagcgaatgcacctgaagctgctggaccgcttcgacctgacggcgcttgaaaccctgaagcccgagctgctgcggcaggagatctccaccatggtcacgcggctgctgcaggaagagcctgaggcgctgaacgacatcgagcggcgcacgctgatacgcgacatccagcacgagatgctcggcttcggccccatcgagctgttgatggcagacccgacggtctcggacatcctgatcaactctcacgagcagatctacgtcgaacgcaagggccggctggagctgacggacgtgagcttcaccgatgagaagcacctcctgcgcatcatcgacaagatcgtctcgctcgtcggtcggcgcatcgatgagtccagccccatggtcgacgcgcggctgcccgacggatcgcgcgtcaacgcggtgattgcaccggtggcactggacggcccgatgatgtcgattcggcggttcgcaaagattccgctgaagatggaaaacctggtgaacgacctgaagacgctcacgccgcagatggcgcagatgctcgaagggctctcccagtcgaaggtcaacatgctgatctccggcgggaccggtgcgggcaagacgacgctgctgaacattctttcagggttcatccccgcaaccgaacgcatcatcaccatcgaggatgcggccgaactccagctccagcagccgcacgtggcgcgaatggaaacgcggccgatgaacatcgaaggcaagggcgagatcacgcaacgtgcgctggtgcgcaacgcgctgcgcatgcggcccgaccggatcgtcatcggcgaggtgcgcggcgccgaagcagtcgacatgctgcaggccatgaacactggccatgaagggtcgctgaccaccattcacgccaacacgccccgggatgcgctggcgcggctggaaaacatgatcggcatggccaacctgaatctgccgcaccgcaccgtgcgccagcagatcgcatcggccattaccgtggtgatccaggtcctgcggatgatcgatggccggcgcaaggtcaccagcatccaggagatcacgggcatggaaggggaggtcgtcacgatgcaggagatctttgcctaccgccagaccggcatgggcccggatggtcagctgcgcggctatttccacgcgacgggcgtgcggccgaaattcgttgaacggctgcagtcctttggcgtcacgctgcccgacaacatgttcgatcccgacaagcactacgaataggaggccatcatgttcgacaacctgattggcgacaccctcatcattctgaccgtgctggtcttcgtcacagtgctgatggtcatcgagggcttgtacctgctgtggaagtcctaccggggggccgatgccaagaagatcgagaagcgcctccaggcgctttcggcaagttccgatcacaccgtgcaggcgcggctcgtcaaagaccgcatgctcagcgatgcgccgtggatgcagcgcgtgctgctgaagttcccgcgggtccacagcctcgatcgcttcatccttcaggctgggctggagtggacggtgtcgcacgtgcttctcgcctgcgggctcttgggcgcacttgcctttttggcgatggtgtcgttcgcgaatcagcccgcgtggattgccgccttggccggtgccgccggcgcggcggtgcctctgctctatttgaactatcggcgcgcccgccgcctggcccatctcgagaggcagctgccggacgccctggacctggtgacgcgtgcactgcgcgcgggtcattcgttcgcgagcagcgtgcagatgatcggcgacgaaatgtcggaccccattgccagcgaattccgcatggtggccgacgaggtcaacttcggggtctcgctgcaacaggcgctcaccaacctgagcgaacgcgtgccgctcaccgacctgcgctacttcgtggtgtcagtgctgattcagcgtgattccggcggcaacctgacggaggtgctgggcaatctgagccggctcatccgcgagaggctcaagctgctggcccgggtgcgggtgctgtcatcagagggacgcttgtcggcctggatcctgggtttgatgccttttgcgctggcgggcgccatgaacatcttcaacccggcattcatgtcgccgctgtggaccgatccgatggggctgagcgtcatcaagtacatgctggtaacgatgctggtcggcgtggtgctcctgcgcaagatcgtgaagattcgtgtttgaaggagaagaatcatgctgtttcccatactcgtgttcgttaccgtctctcttgcagtcggaggcttcgtggtgtgggtgctgcccacgcgcaccgagcgccgtcttcaggccttagccccctcgacagccaaatcggcctgggccgaaaccgctgtcaagatcgtcggccccttcgcgcaactgtcttcgcccacaggcgatggtgaaaccacgccactgcgcgttaggttcctgaatgcgggaatccggcatccggatgccagcctcttcttctttggattgaagacgctgctgcccttgggcttcgccggcctggccttcctggccatgcgcacggcgggagccgacgacggattgaagaccctgctgtggctcgcagtcgcggcgctggtcggctgctacctgccgaacgccgtgctgtacgtgatggtcagggggcggcagcgcgaaatcttcgataactttccggatgccgccgacttgatgctggtgtgcgtcgaggcggggctcgggctggatgccggccttgtcaaggtcactgaagagatccgcgtcaagagcgtggccctggcgcaggaactgcactggaccaacctggagatgcgtgcaggcgcgacgcgcgagaagtcgctgcgcaacctgtcgctccgtaccggtgtggaagaaattgggaccttcgcgaccatgctgacccaggcagaccggttcggcaccagcatcggcgaatcgctgcgtgtgttctcggacgatcttcgccacaagcggcagatgcgtgcggaagagctggccgcgaaggtacccaccaagatgctgctgccgctggtggtgtgcatcttcccgtgcatctcgctggtcattcttgcgccggcggcgatccgggtcattcgcaccatcatgccgatgctcgctggccactgagccgggcagtcaaagacagtcaggggcagtcaacccggccgggttgactgcttcgcgttcagtgaggcaccacgtccagctggtgcttgatcgcgtagatatacagctcgagccggttcgacacgccaagcttctggtagatcgccgtgaggtgattgcggaacgtgtgctcggtaacgaacagccttgacgcaagcgtcttgttcggagcgccgctgccctcgaccacggcacgaatgacctgccgttccttctgcgtcaggctggccagcttggcttcttcgggattcaccttcaccggcttcttgggagaggtcagctcggagaacacgcggcccatggcctgcgcgtcgatgcacagctcgcccttgtggacgcgttggatcgcatcgagcacctgctccgcggaagcgtccttgcccagcacgcctctggcaccgcgcagcacggcgaggtccagcgtttgctgccggcgctccgccgtgaggacgagggcgcgcgaaatgtcgttcgacagcagcatcggaagaatgtcgagcgagcattggccggccaggtcgagatcgagcacgatgacgtcgggcacgtagtgcacggtgtgttccagcgcctgttcgaagcagtttgcggtggcaacgaccttcatgcgcggttgttctccgtcaatcagcctcgacagcccccacagcatggtttggtggtcgtcgaccagcatgaccccgatgggatggtccgttgtgatgggttgcatttttttcccctttgtcttgttcagatgggtatttcgaccagaaccgccgttgcgccgcccatgccctgggtaacctcagcgcttcctccgagggctgccgcgcgttcgctgatggagcgagggcggaagttcgagaaaatcgtgccgcatgcttcgttttcgatccggatctgcagcttgccgtccgtgcagccgatgcggatgcggccgtgatgggcatgggtgtgcttgcagatgttgttcagcccttcgcgcaccaactggagcacttcggccgtcatccggtcgtccaggtgaacgtcgccgtcaacgacgatctggatatcgattccgtagagcgtcttgatgcgcgccgcctggcggtgcagatgcggaaggatgaactcgcagtggctgtcggcgccgtgcttgacggtgccggcaaagtggcgcagatcggcaaccacgctctcggccatggcggccagcttgtccaggtcgtcgatcagcggattgtcggcgccggccttctttcgaagcgcgctcagtcccagcttgagtccgatgtagggctggatcgcggtgtcgtgcaggtccagcgagagcttcaggcgctctttcgaggcggcctccgaggccatgccgtcgagcacccggatggtctcgatgaccggaaagacctgattcatgaggtgagccagaaacagcgcgtcggacttgcggaattgtccttcgtgcgaagacacgtagatccgtccctcgccctggcgcatcggcagcggtgcagtcatgaagctgcgagcctccagcatcgcggcgaccgccgcgctgtgccgcaagccctgttcatcctggggatgccagcgatgcgtgcgagggtcgcaggcgtgtccgtcggcacgcaccatgctcatcggccagggcaggcggctgctcagcactatctgctcgacgcccagggccatcagcggcgattcggagacgcggtcgatggtctcgacactgacggattcgcccgtatcgctctttccgaccgagcgcagcacccagccgctggtatccgtgtcgcgcatcagcaggatgcagtggcttgcctcgaagaaggccagggtcttctccatcgtgctggcgatggtgcggttgacgccgaaccgcgggttggacagccggctcacctggctcagcagcgcaaggcgccggcgcaactcgaccttcgatccgccccaatggccgatcatgtgtcccagcgccaggaggaacgtggtgcgcatgagcagttgcggcgtgtcgctccccgtgcctgttccgagcccgcaggtggcgaacgacaccaccgcggccatcgtcatgcgggcaccttcttcatagccccaccggaaagacgacgtgagaatgacgaagaagtagaagagaaagtagaggctgctgccgccgccggtcaccaagaccatcagcgtaaaccacaggatgtctagccagtggatggctttgccctgaaaatacggctggcccgttcgggtgcagacgtgaacaccgaggctgtagaccacaaagcccgaaaagacgagccagacggcgctgccgatggtctgttgttctacctcgccggcgtcaaccccgactgccagcagcgccgaaaccgacagcaccaaccgcatccgcgccaccatgagagcgtcggcggtcagagagtcggtcccggaatccgggtcgatggacgtggcaggcatcgctggttttccagtgcatcgagcggctcatatctcgccggttgtcaacagcgacgagacgcccatatccccgggaggggatctgcgggacgtaacacttgggttcacttttgcgccaaaattaatattgtgaagatttcacattactacttttgtagtcgaaagcaatactttttgttaataccctggtccagtgtgtacttttgttaccaactgatgcgagatgcgagggctggccagcagatgtatccgccagtgggaagcggcagaagcgggcaagaaaaagggctcgggaagaatccgagcccttgaatggtggttggtggagaggatgaggatcgaactcacgacctccgcattgcgaacgcggcgctctcccagctgagctacccccccaacacagtccgaattttaaccagaacctgtctcctggcgcagggggccatgccaagattcgcgcctcgcaaaagaaggagcaggaaccgcatggcctcgtacgaacccgcctggctggaaagcatgtacaacaatctcgcgcgcgtgaaggatcacccggcgtacttcgcgcgctgggccggcgattcagcggcggcgcgtgaggcgcttcccagccggatcgatgtgccctacggccgcggagtgaacgaaacgctcgacatctttcccgcacccgtggccgatgcgccggtgctggtgttcattcatggtggctactggcgcgccatggacaagcgggaccattccttcattgcgcccgcgttcaatgatcgcggcgtgtgcgtggtgatgcccaattacgcgttgtgtcccggaacgccggagcagccggtgaccgtgccggacatcgtcatgcagatcgtgcgcgcgctcgaatggacctggcgcaatgccgcgagctttggggcggaccccgcgcgcattaccgtggcaggccactcggcgggcggccacatggcggccgcgctgctcgcctgcgattggaaggccgtgtcacccgggttgccggcgcagctggtgcgcagtgcgctgtcgatctcgggcctttacgaccttcggccattgcagcgcacgccgtttctcgagcacgcgctgaagctcagcgacgcggacgcgctgcgcgcgagcccggcgctgtggccggcgccagcacgcgggcagctccatgcggtggtgggaggcgacgagagcgaggaattcattcgccacaacgcattgattcgcgaagcctggggccgcaacaccgtgccggtgtgcgaaacgctggcaggcttgaatcacttcagcatcgtcgatgcactggccgacccggcccacaggctgcaccggcacgcggtgcagctgctggaagcctgatccggcccggcggcgccgaaagggcgcctacatcagcaggtgttcgcccgcgttgtcgccgcccagcgtgacgtagttgaccttgcgaatgtccatcagcgcgcgcccgcccgcgtagctgatggagctttgcacgtcctgctccatctcgaccagcgtttcggccagcttgcccttgatgggctcgaggatgcgcttgccctcgacgtgcttgtattcgcccttgttgaagtcgctggccgagccgtagtactccttgaagagcgtgccgtcgacttcgaccgtccggcccggcgactcctcgtgccccgcgaagagcgatccgatcatcaccatcgaggcgccgaagcgcacgctcttggcaatgtcgccatggtcgcgaatgccgccgtcggcaatgatcggcttggtggccacgcgcgcgcaccacttgagcgcgctgagctgccagccgccggtgccgaagccggtcttgagtttggtgatgcagaccttgcccgggccgatgccgaccttggtggcatcggcgccccagttctccaggtcgatcacggcttcgggcgtgccgacgttgccggcaatcacgaaggaggccggcagcttctgcttcaggtagccgatcatgttcttcacgctgtcggcgtggccgtgcgcaatgtcgatggtgatgtattcgggcaccaggccctcggccgccagctggtcgaccgtgtcgtagtcgggcttcttcacgccgagcgaaatcgaggcgaacacgcccttgccgtgcatctcccggacgaacttcacgttgtccaggtcgaagcggtgcatcacgtagaagtagccgttctgcgccagccagaggcagatcggctcgtcgaccaccgtcttcatgttggccggcaccaccggcaggcggaagctgcgcgcccccagcgtcacgctggcgtcgcactccgagcggctttccacgcggcatttgcgcggcagcaagaggatgttgtcgtagtcgaaaatctgcatgaccaggctcctggaaggaatcgttgaaaaaaacgaatgagcgcttggtccggccggcctttgcggtgcttctcgaaaagaaaacgcccacaaaaaaccggacgcaagaaacttgggcccggtgattgattttacgcagtctcgccgcggcgggtcttccagttcttcgtataacccgcatacgggttggtttctacaatcgacggatgttgtttaacgaacctgcggctgatgccaacccctcggaactgccattgctgcagaacctgaacccggagcagcgtgccgcggtcaccctgcctgcgggcaatgccctcatcctcgccggcgccggttcgggcaagacgcgggtgctgaccacccgcatcgcctggctgctgcagaccggccaggtctccgccggcggcatcctggccgtgaccttcaccaacaaggccgccaaggaaatgatgacgcggctcacggcgatactgcccgtcaacgtgcgcggcatgtggatcggcaccttccacggcctgtgcaaccgccttctgcgcgcgcactggaagctggccaacctgccttcgaccttccagattctcgacacgcaagaccagctttcggccatcaagcggctcatgaagcagttcaacgtcgacgacgagcgctttcccgccaagcagacgcagtggttcattgcgggggccaaggaagacggcctgcgccccaaggacgtcgagatccgcaccgaggacgaccggaaaaaggtcgagctgtatcagctctacgaggagcagtgccagcgcgaaggcgtggtcgacttcggcgagctcatgctgcgcagctacgaactgctgcgcgacaacgacccggtgcgcgagcactaccagcggcggtttcgccacatcctgatcgacgagttccaggacaccaaccgcctgcagtacgcgtggatcaagatgctctcgggggtcaccgcggccggccagttcacgccgggccagagcagcgtgattgccgtgggcgacgacgaccagagcatctacgcctttcgcggtgcgcgcgtgggcaacatggccgacttcgtgcgcgagttcgacgtgcagcaccagatcaagctggagcagaactaccgcagctacagcaacatcctcgattcggccaacgagctcatcagccacaacaagaagcggctgggcaagaacctgcgtaccgaccagggtccgggcgagccggtgcgcgtgtatgagtcgcccaccgacctggccgaggcgcagtggatggtcgaggaaatgcgccagctcgtgcgcgacggcttcgaccgcaaggaaatggccgtgctctaccgcagcaatgcgcagagccgggtgatcgaaacggcgctcttcaatgcctcggtgccataccgcgtgtacggcgggttgcgcttcttcgagcgcgccgaaatcaagcacgcgctggcctatttgcgcctgctcgagaacaaggacgacgacaccagctttctgcgcgtggtcaactttccgccgcgcggcatcggcgcgcgcacgctggagcagctgcaggacgcggcgcgcacggcggggcgctcgctgcacgacgcggtgcacgcggtgggcggcaaggcgggttcgaacctcacggccttcgttgccaagatcgacgtgctgcgcgagcagacgcagggtgcgagcttgcgcgagatcatcgagctggtgctcgatcacagcggcctggtcgaacattacaaggccgaccgcgaaggcgccgaccggatcgagaatctggaagaactggtgaacgcggccgaaagcttcgtcacgcaggaaggcttcggccgcgacgcggtggcgctgcccatcgacgaactgcgccagtcgcttgcgagccagggcatcgatccgaaccggccgctgatggacgagccgctcgcgcccgatgccgaaaccggtgaaacgctgagcccgctggccgcgtttctcacgcatgcggcgctcgagtcgggcgacaaccaggcgcaggccgggcaggacgcggtgcagttgatgaccgttcacgccgccaagggcctggagttcgactgcgtgttcatcaccggcatggaggagggcctgttcccacacgagaactcgatgagcgacttcgaaagtctcgaggaagagcgccgcctgatgtacgtggcgatcacgcgggcgcgcaagcgcctgtacctgagccattcgcaaacgcgcatgctgcacggccagacgcgctacaacgtcaagagccgcttcttcgaagagctgcccgagggcgcgctcaagtggctcacgccgaagaaccaggccttcacgccgtcggccttcggctatggcggcggctatgcgagcacgcgtggcggcggcggcagttacagcagcggcagcggctacggtggcaacaaggacacctatgcaagcccgccggtgccaccgcagaaaaccgcgccctcgcacggcctgcgctcgggcatgcaggtgttccacaacaagttcggcgaaggcacggtgctgtctctcgagggcacgggcgacgatgcgcgcgcgcaggtcaagttcacgcggcatggcgtgaagtggctcgcgctgtcggtggccaagctcacgccggtgtgagcgctgccatgccctgcccacatttgctattaaacaaatagcttaggccgcaataaccacgggcgtttggggcggttctaaagaagcaatccccgtacactccatgctcgccaaaacaaggggagttagggatgtggtttcttggcatgatcgccggtctcttcataggggccctggccgagtcggttccggccgcgctgattcttgcggtggtcggcgcgtttgggttgccgaaaatcgtcggcaagaaaaccgccgccgagcctgcacgaaccgaggctgagagcgcacagctttccaccggtgcgccggcggcccccgcgggcggcgtgttgaagctgcagcagcgcgtcgccgaactcgaacagcgcgtgagcttgcttgaacagcggctggggcagggcgcagcaggtgcggcggtcgagcctatgccttcgcctgtgaccgtgcctgtgcctgccaagccagacatccgcgtcgcccagcccatgcccgtgccggtggcgcggccggcggcagcggccgctgcagctgcagcaaacgctgcggcgcacgttccggtgccgcccatccagcctgcagcggccaagacggctcccgagcccgcggcgcccgtggccgtcaagccgcccgcggccatgcctgcgccgccccggcgcgtgccaccgccgccgccgcctcccgcggtcccgctgcgcgaccgcctgcctgcgcccatcgccaatttgatcttcggcggcaacatgctggtgaagctcggcgtgctgatcctcttcctggggcttgccttcctgctgcgctacacggccgagcgcgtcaccgtgccggtcgaactgcgctatgcggcggtcgccctcgtgggcgcggggctgctggcgctgggctggtttttgcgccgcaagcgcaccggctacgcgctgatcctgcagggcgccggcatcggcgtcttctacctgacgacgctggcggccatgaaggtgcacgaactgctgccgccgaccgcgggcttcgttttcctgttcggcgtggccgcgctgagcgcggtactggcggtgctgcagaacgcgccggtgctggccatcgtggcggtgctcgagggctttgcggcgccggtgcttgcgtccactgggcagaaccggccggtggggctcttcacctacctgctggtgctcgatgtcggcatcgtgctgatcgcctggttcaaggcctggcgcgtgctgaacctgatcggcttcgtcggcaccttcacgctggccgcgggctgggcgcacaagtactacaccgacgaccagtacggcatcgtgcagcccttcctcttggcgttcttcctgctgttcgttgccatcggcctgctgtttgcgcgccgcacgctgttcgatgcgcccgtgcagcccgcacagccgttggccgcacgcgcgctcgataccctgcgccgcgcgggccgggtcgacagttcgctggtgttcggcacgcccatggtcgcgttcggcatgcaggtgctgctgatgcagccatgggagtacggcgccgcgttctcggcgatggcgctcgcggccttctacctggtgctgggccgcctggttttcgccacgcagccgaagggcctggcgctgctggcggaggcctacgcgatcgtcggcgtgatcttcggcacgctcgccatcccgctcggcctcgaaggccggtggacgggcgcggcctgggccgtggaagcggccggcatgtactggctgggtgcacggcaggggcgcgtgtatgcacgtgccttctctttcctggtgttcgccggcgcggtgtggaagctgctcgaagccacgcagctcgatgccgccgcgggacatccgctgctgcagggctcggtgatcggcccgctgctggtggccgtgagcgccttcgcgatgtggaccattcaccgccgcgccaagctggacgaaggcaatggctgggaagcgctcgtgggcaccgcgttgccgtggctcggcatgggtgcgctcacgctgctgctgtggcagtggttcacgccgccttgggcagcggccgcgacggcggtgctggcatccgccacttttgccgtggcggtgcgcttcaagctgcggccgctggccttcgtgacgtatggaatgcaggcactggcagtggccggtttcattgccacgctgcatcgcgtggccgatgcccgtgccggcgacgaggtgcttgcaaccggctgggagggcgcggtggcggcgagcctgatcgcgctcagcctgctcggcagcgccgcatggtcgatgctgcaggcgcaccgtgccgcattggcgcgcggcatccagcctgtgtggtcgccgggcaatgcggtcgcggtgattgcgggcgtgagcctgctgcatctcgcgatgctgttccaggtgagtctggcgcaggccgcgttgctgtggccgctcacggccacggtcgtgctctgggtggcgctgcgcatggcgcacaagccgctggcggcgctggcgggcgtgctgcaggtcgtctcggcgctgctgcacgtctttggccagatctggatcttctacggcaataccccgccgccggctttcgcgcacctgggtttctggacaccggtggtgctggggctcgcggccttgctggccggcggctggatgagcggcgaggcatggcggcgcgccaccgaaggcaccagcacggccaagcgcacgcgctggatcaacgactggtgcgccaatccggtcgtgctgtgggcgccggtggtctggggcctggcctggtggctcttcggctggctggacgaatccggcgaggtgctgcgccgcaacgggctggccggccatgtggccgcggccgccatggcgatcgtgctcgtgacctccgttctgtcggcggtggtggcgcaccggcgcggctggccgcagctgggccgggccacgctggccaccttgccgggcctggtgctgatcgccgcccatggcgctgcgttggcggcgcccgcggtgtacgtgccgtcgagcgcgctgggctggatcgcctggccgctggcactgctctggcacctgcggctcctgcatgcgcagaagcgctggctggctccgtcggcactggcgaccttgcacgtggcgggcttctggttcttcgtgctgctggcggcgcgcgaatgccaatggcagctcgggcgcgtgggcgcggagtggtcgagctggcaactgctgggctgggccatcgtgcccgcgctcgcgctgtggatgctgcgttcgcgcgcgctgctgcagcgttggccggtgtccgagtaccgggccgcgtacctcgaaatcgcggccatgccggtggcggcctacctgctggcgtgggtctgggtcaccaacggcaccagcccgggcaacgcggcgccgctgccttacgtgccgctgctgaacccgctggaactggcgcaatggctggtgctcttcgcgctggtgctctggtggcgagccttgccgcagggctcgttcgcgcgcgtgcagcccatggttgcgaagggcgtgctcggcctcaccggcctggcgctgctgaccggcatggtgctgcgcagctgccatcactatgcgggcgtcgagtggcggttcgacgcgctctacgcctcgtggctcacgcaggcggcgctctccatcacctgggccatttgcggcgtggtcgcgatggtgctcgggcatgcacgcggggtgcgcaccctgtgggtcggcggcgccgcgctgctcggcgttgtggtgctgaaactgttcttcgtcgaattggcggaccggggcgggttgttccgcatcgtgtcgttcattgcggtgggtgcattgctgctgctggtgggctatttcgcgcccgtgccgccagccaggaaagaaatggagaaggatgtgttgttgcccgaaggaggtgtcgcatgaagcacggtgcaatcccgttgcgccacgtggtgggtgttcgcctggccgcgggtctggctgcggcctggttcggtgtggccggggcgcagccctccaccacggcaacggcccccatcaccgtgcaaggcaacggcccctactaccggctcgcgctgccgctcggcatctacgcccatgctgcatacggcgatctgcgagacctgcgcgtgcgcaatgccgccggcaacgccgtgccctatgcgtggctgcgcaacgaagccgccacgccgcacttcacctcgaaggaggtgccgatcttcgcgctgcccgcgagtgccggaggcgcggcggaagcatcggacgacgacgcatcgctgagcttcaaggtgcggcccgacggctcgctggcgctggcccgcaagccggcgcgcaagccagccgaagcggcacagtggctgatcgatgcgagccagctcaaaggcggcctgctgcaggcgcgcttcgaagtggcaccggaagcgcgcggcctgttcgccttcaggctcgaagccagcgacgacctgcggcattggcggccggttggcggagaagagcaactggtgcggctggcgcatggcggccaaaccatcgaacgcctggcggtcgacctgggcagcgtgcatgcgcgcttcctgcgcttgcgctggagcaatccgcaaaacggcgcgccgctgaccggcgtggcgatcgacagcgtgcaggaggtcgagcccgtggcgcccatcgaatggacgggcgcgctcaagccggaacgttgcggcaccgaccattgcgactacgcgctgccgcgcggccttcctgtggaaagcctgcgcatcgacctggccgatgtcaacacgctcgcgcaggtcggtgtttcgggcctgctcgcggccacgccggcggctgccgccgagccggcacccgtgccgcgcaatccgctgtatgcgctgcggcaccagcaacgccggccggcagcggccacaggcagcccgggtgaagtaccgctgctcgacaccgtggtgtaccgcctcgcacaagcgggcggcgaggcgcgttcgccgttgcttgcgctcgacggcaggagctactcgcacctgcggctgcgcacggccggtccggtgagcgttctgggcccgacgcctccggcgatcgcggtaggcgccacgccgcgcacgctggtgtttctcgcccaaggcgccgcgccgttttcgctgaactggaatacggcgcccgaaaagaacgtggtgcagggcggttcgccgggagcggccttggcactggccacgctggtgccgggctatgccgccaacaagccgattgcggcgggcgaagcctccgtcacgctgccgccggcgccggtggccgctgtcgaagccgtggtcgccgcggccgcgcaattgccccttcccacgcagcccgatgcgtcgcgcaagtggtggttgtggggggcgctgggcatcggcctgctgctgctggccggcatggcatggtcactttttgcgagcctgcgcagggacagggcgctggcagactgaacgcccttcggccgcgagtcagttcgggtcgaagctgtcgcggaaggtgaaccaggtggagctcatcgacatggccgcgagcaccagcgccgtgccgacgatcagcacgttgccgatggccgcggcggcggcgcctccgcccaccgcaccgacgccgatcagcacggtggcgatcaggccgatgccgatgccggcgagcaggaacacgccgagccatgccagcccgaacagcgcataggcgccgaagttgcgaaacagtgcgaccacgctgaagaacacgctcttgaccggctccacgcggtgccagtgcacgagcgcgggcgcatgccacatggcgagcgagagcggcaggttcaggcacatcaggagcatgcgtgccacctggaaatcgctgctcgccatcacctctggcgtcagcacttcgtcgagcaggtaggccttggcaagctggccgccgtcgacgaacgtggtcagcagcacggccaccacgaaatacagcgcggagatcacgcccagcttgaccagcgaacgccactcggcgcgcatggcgccggccacggcaacgaacatggcggagccggtgggacgctgcgcgtgtccctcggtgccgatgccctcggcgttgtcggtgtacgccaccgaagtggccaccatcaggcccagcgtcatgaagggcagcagcaccggcgccagcacgctgccgatgagcggcagcagcgacaccgtcgagatcagcgccatcagcaggaagaacagcgagatgaaggcgagcggctgccgccagaaagtcttgagcccgagacggacccattcggcgccggttcgcgccggcacgaggtggagtttcattttttgagagtcaggcggccagcggttcgagcgactgcgccatggcgtgcggatgggcggcgcgctcgcgcagcacgcgctcgaagtgcgccgggtcgtgcggcttcagcatgctggcttcgcgcggcaggtgaaagtcccagagccgcgaaatccagaagcgcagcgccgccgcgcgcagcatggcgggcagcagggcgcgctcggccgcgttcagcgggcgcacggtttcataggccgacagcaatgcgtcggcgcgttcgacgtcgtgctggccggtcgcaaggtcgatggcccagtcgttcaggcacacggccaggtcgaacagccaggtgtcggtgcccgcaaagtagaagtcgaacacgccggtcaggcgcggtgccgcagcggcgtcttcgccggtggcgaacatcacgttgtcgcggaacatgtcggcatgcacgggcccgcgcggcagcgccgcgtaggccgacgactcgaccacgtggttctggtaggcgagttcggcgcgcagcaacccggcttgcgattcgtcgacgtaaggcagcaccaccgggacggtgtcgttccaccaggccaggccgcgcaggttcggctggatgcgcggaaagtcgcgcgccgccaggtgcatgcgcgccagcagggcgcccagctcggtgcaatgcgacgcgcccggtgcgagttcgctccggcccgagagccgctgcaccagcgccgccggcttgcccgccaccttgagcagcagttcgcacggggcgttcgcggcgatcgtcagggcatgccccgaaggcggctggatggccggatcggccacgggctcgggcaccggcaggccgcggcccgccaggtgcttcatgagacaaaggtagtaaggaagctgctcggcgcccagccgctcgaacagcgtcagcacgaactcaccggtctcggtggtcgcgaagtagttggtgttctcgatgccaccctcgatgccgcgaagctcgcgcagagggcccaggcccaggcgctgcacgagcgcgtcggcctcgccgaattcgacttcggtaaaaactgccatggcggtgctcagcgtgtcgctgccgattgaaagcgcggcacggtcagaacttcatcacgttccagacccgggcgccgttgccgttcgagttcgcttcgcccgaacccgttcgcgcgcctggatcgttcggccgcacctcgtagcccggcacgttggccttgggcttgacgttgatgctctgcgtgcggccgccatagcgcacctcgtcgaccgaggcgccgctgtcttccgtgtggatgtgctcgaccttctggttgcgccggccatcggcctgctcctgattttgtagcggctggggcggcgcggaggctccagcgggtgcgggctgcgcctggacggcggcaaaagggacggcaaaggccagcgccagcaggatgcggcgggcgaccaggagtgtggggctaggcatgcaaggattgtaggctcggggccgcttccagcgtgtcggcgggcggcgcttgccgccgtggttcgggagcccggtccgggcacggcaaaatggcccgatgaccgacaagaaaacgctgctgctcgtcgatggctcgagctatctttaccgcgccttccatgccatgcccgacctgcgggccgtgcccggcgacccgaaaagccccgcgaccggcgccatccgcggcatgatcaacatgatgaccgcgctgcgccgcgaggtccgcgccgactacgcggcctgcatcttcgacgcgcccggcaagacgtttcgagacgacctgtaccccgaatacaaggccaaccgctcccccatgcccgacgatctgcgcagccagatcgaacccatccacgaggtggtgaagctcatgggctggccggtgctctgcgtgcccgacatcgaggccgacgacgtgatcggcacgctcgccaggacggcggcgcgccagggcgtcgaggtcatcgtatccagcggcgacaaggacctgagccagctggtggacgagcacatcaccatcatcgacacgatgaacggcaagcggcgcgacgtggccggggtcacggcggaattcggcgtgccgccttcgttgatgatcgactaccagacgctggtgggcgatgcggtcgacaacgtgcccggcgtcgagaaggtcggtccgaagaccgctgccaaatggctgctcgaatacggctcgctcgacgcgctgatcgaacgcgccgccgaggtgaaaggccaggccggcgagaacctgcgcaaggccctggacaagctgccgttgagcaagaacctcgtcaccattcgcaccgattgcgacctggacgggcacgtcaccggcctgccgtcgctcgaaggcctgccggtgggcgcgccgcaaaccgccgagctcaagcccttctacgagaagttcggtttcaagagcctggtcaagtcgctcgaggcactggaagtgccaccggagctgatcgaggaaaacatcaagaagcagacggcccgcggcgccgcggcaagcagcgatcaaggtgggttgttcgacgaatcggcggacctcggcgcgatggaggcggcatcgcccgcgagcaacctgaagtacgagaccatcacgagctgggagcagttggacgcctggctcgccaggctcgaggccgccgagctggccgccatcgacaccgagaccacctcgctcgacgagatggtcgcgcgcatcgtcggcgtgagcttcagcgtcgagcccggcgaggcggcctacgtgccgctcgcgcacaactatcccgacgcgcccgcgcagctgcccatcgacgaagtgctcgccaggctcaagccctggctcgaaaacccccagaagaaaaagctcggccagcacatcaagtacgaccgccacgtgctcgccaaccacggcatcgaggtgcagggctatgcgcacgacaccatgctgcaaagctacgtgctcgaggcgcaccggccgcacggcctcgcgagcctggccgaacgccacctgggccgcagcggcatctcgtacgaagacctgtgtggcaagggcgcgcaccagattccgttcagccaggtcgacattgccaaggccgccgagtattcgtgcgaggacagcgaccagacgctcgacgtccacctggcgctgtggccccagatcgagcgcgacgaaaagctgcgcttcatctaccagctagagatggattcgagcgaggcgctctaccgcgtcgagcgcaatggcgtgctgatcgacgcgcccacgctcgcggcgcaaagccatgaactcggcacgcgcatcatggcgctggagcaggaggcctacgagatcgcgggccagccgttcaacctcggttcgcccaagcagatcggcgagatctttttcaccaagctgggcctgccggtggtcaagaagacgccgagcggcgcaccgagtacggacgaggaggtgctcgagaaactggctgaagactatccgctgccggccaagatcctggagcaccggggcttgtccaagctcaagggcacgtacaccgacaagctgggccagttggccaacccacgcagcggccgcgtccacacgcactatgcgcaggcggtggcggtcacggggcgcctgtcgagcaacgatcccaacctgcagaacattccgatccgcacgcccgaaggccgccgcgtgcgcgaagccttcattgcgccggctggcagcgtgattgccagcgccgactactcgcagatcgagctgcgcatcatggcgcacatcagcggcgatgagtcgctgctgcgcgccttccgcgaaggcatcgacgtgcaccgcgccaccgcggcggaagtgttcggctccacgcccgaccaggtgtcgagcgagcagcgccgctacgcaaaggtgatcaacttcgggctcatctacggcatgagcagcttcgggctcgcacgcaacctgggcatcgagaccaaggccgcggcctcctacatcgaacgctacttcgcacgctacccgggggtgaaggcgtacatggacgagaccaaggcgctcgccaaggagaagggctatgtcgagaccgtgttcggccgacgcctctacctgcccgagatcaattcgcccaacggcccgcgccgcggcggtgccgagcgcgcggccatcaacgcgccgatgcagggcaccgcggccgacctgatcaagctcagcatgatcaaggtacagaatgtgctcgacgaagagaagcgcgccacccgcatgatcatgcaggtgcacgacgaactggtgttcgaagtgcccgaggccgaggtcgaatgggtgcgcaccgagattccgcgcctgatggccggcgtggcggaactcaaggtgccgctcctggccgagatcggcatcggtcccaactgggacaaggcacactgaccagaatccagacgaagaaagaagaagtacgcccatgaaaatccagcccggcaaattcctcctcgccgccgtctgcgccgcatggctcggcactgcctttgccgcgcccgatgcccgcatcgccgcgctcgccgccaaggaaaagcccgccctgctcgagacgctgaaggaactggtctccatcgaatcgggcagccgcgatctcgaagggctcgagaagatctccgatctgatcgcggccaagttcaaggccatgggcggcgaggtcgagctgatcgacccaagcgccgaggcctaccgcatggaggacacgcccgagaagctcgggcgcgtcgtgcgcgccaccttcaagggcacgggcaagaagaagatcatgctcatcgcgcacatggacacggtctacaccgtgggcatgctcaacaagcagcctttccgcgtcgaaggcgacaaggcctacggcttgggcattgccgacgacaagcagggggtcgcggtcatcacgcacacggtcgcgatgctgcaggcgctcaagttcaaggactacggcacgctcaccgtgctgatcaacggcgacgaggaaatcagttcgccgggttcgcgcacgctcatcacgcggctgggcggcgagcacgacgcggtgctgtcgttcgaaggcgcgtcggtcaaggaagacaagctctcgctcgccaccgcgggcattgcctcggtcacgctgaacgtcacgggcaaggcctcgcatgcgggttcggcgccagagcagggcgtgaatgcgctctacgagctctcgcaccagatcctgcagatgcgcgacctgtccgaccccgccaccggactcaagatgaactggaccatctcgcgctcgggcagcaaccgcaacgtgattccggccagcgccacggcgggcgccgacgtgcgcgtgctcaaggtgagcgactacgaccgcatcgagcagcaggtgcaggagcgcgtgaagaagcagctcgttcccgaggccaaggtcgagatgaagttcgagcgccgccgcccgccgctggaggcaaccgatgcctcgcgcgcgctcgctaagcatgcgcagcggatctacaaggacgagctcggcaggccgctgggcgccgacgacgcggtggccggcggcggcaccgatgccgcctttgccgcgctcaagaccaaggcaccggtggtcgagcgcttcgggctgcagggctttggcgcgcactcggccgatgccgaatacgtgctggtcgattccatcgagccgaggctctatctcgcaacccgcatggtgatggatctctcccgcagcaagctccctggcaactgacccggccatgcgcctgcgccacatcgaggtcttcaacgcgatcatgctcaccggcagcgtgagcgcggcggcgcggctcatcaacatcacgcagccggcggtgagccgcaccttgcagcatgccgagctgcagttgggctttccgctgttccagcgtgccaagggccggctcacgccgaccaccgaggcgctcacgctgtatccgcacatcgagcggctgtttgcgcaactcgacgaggtgcagcgccttgccgccaacctgcgcgcgggcagcgacaccggcgaactgcgcatcctgagcgtgctggcgctgagctacgaggtgctgccgcgcgcgctcaaggccttccgcgaaaggcacccgggctattcgatcaccgtggagtcgctgcactcgccgcagatcatgtcggcgctgctgctgcaggaggccgacgtgggctttgtcttcagccccgcggtgcatccttcgctcacgcaggaaacgctggccgacacgcgcatggtgtgcatcgcgcccaagggaatgctgccgcgcgcgctggtgcgcaacggttcggtggcgctgcacgacctggtcgaccggcccgtcatcgggctcgacagccgcgacccggtgggcaccagcctgagccaggcctgccgccaggcgggggtgggcttccagcaggcggtggtgacggtgcagacctatcacgccgcgctgtcgatggcgcaccacgggctgggcgtggcgctggtcgatgcatgcacggcccgatcggccgacagcgccaaggtcgacgtgctggcgctggagccgcacattcccgtgccggtgcgcgcgctgcgttttgcaggaaagcccgattcggtggcggtgcgcggcatcacgcgctgcatgcgcgaggcgatcgagcaggcggcctgacccgcgtgccggccgctcaggaggccgcaggctccagggcctctgcaatccgccgcgccgagccgaaggccagcgtgaagcccagggcgccatggccggtgttgaacagcatgtttgccggcgcgctcggtagccgaccaatgatcggcagccctgtgggcgtggcgggccgcatgccggtccacgggtgcagctcttccagttggcttgcatgcggaaagacagcgcgcgtggcggccgccagcgtctcgatgcgggtggccggaatgctcgcgtcgtgtcccaccagttccgccatgccggccacgcgaagccgcgagccgatgcgcgcgaacaccaccttgcgcgcgctgtcggtcacgttcacgcgaggtgcggcgcccgccgagggatcgacctccaccgtgatgctgtagcccttgagcggatacaccggcaggtaggcgccgatggcgcgtcccagcttgtgcgaggccgagcccagcgccatcacgaaggcatcggcctcgatgtcttccgcattcgttttcacggcagccacgcggccttcgctgcgggcgaagccgtgcacgtcggtgccgagcagaaagcgcacgccgcgcccgctgagcatgcgcatgagttcggcacagaccttgaggcagtcggccgcgcattcgctcggcgtgtagaccgcgccggccatctggctgcggtagcttgcgagcgcgggctcgatcgcgacgcactcgtcgggcgacacgatgcactgctcgctgcccatggtgcgctggagttcgagttgcgcgcgcgcgccttcgagcgacgccgggctggcatagagcaccagtttgccggtggccgaaaaatcgcagtccggcgcgatgtcggcctgcatcgcctcgaattcggtccggctcagcgcggccagcgcgagcagctgggccgtggtgttgcgggaagtctgtgccttgcaggccgccaggaaagccagcccccagcgccactgcagcggatcgagctgaggccgcagcttgagcggtgaagagggcgagagcagcagcttgggcaactggcgccagatcgacggatcggccagcggctgcacgtacgagtagctgagctgtgcgccgttgccgccgcttgcgcccgcaccgggggctgcgcggtcgattaccgtgacctgatggccctggcgttcgagttgccaggcggtggccaggcccacgatgccggcaccgagcacacagacatgcatggaggcaactttccgggagtgaatgggagacagcatcgactgtaggggcgcaccgcgccggccggaaatgccaaaagcgccgtggcccatagccaaaccgcatgccctgcagcccataacctttgggtatggcccagggttcaattggaattgtcggagtgcgtcactccttcttacactggccgctccgttcaaccatctgaagaaggctcgcatgaaactctccgcattgatggccgccgctgccgtggtgctgttttccgccaccggcgtccaggccgccgacacgctggccaagattgccgagtccggcaagatcacgctcgcctaccgcgagtcgtcggtgcccttcagctacctggacggccccaacaagcccatcggcttctcggtcgaactctccaacgccgtggtcgaggcggtgaagaagaagctcaacaagcccaacctgcaggtgcaactgatgcccgtcacctcgcagaaccgtattccgctgatcaccaacggcaccgtggacctggagtgcggctccaccaccaacaacagcgcgcgcggcaaggacgtggcctttgccgtgaaccatttctatacgggtacgcggctgctggtcaaaaaatcttcgaagatcaagaactacgccgacctggccaagaagacggtggccagcaccaccggcaccaccaacgcgctggtcatgcgcaagtacaacaccgagaagaatctcgacatggacatcgtgctcggcaaggaccacgccgacgcgttcctgctggtggaaagcgaccgtgccctggcgtttgcgatggacgacatcctgctgtatggcctcatcgccaacgccaagaacccggccgactacgaggtggtgggcgacgcgcttcaggtcgagccctacgcctgcatgctgcccaaggacgacccggctttcaagaagctggtggacgacacgttcattggcatgatgaagagcggcgaattcgagaagctctacaccaagtggttcatgtcgccgatcccgccgaagaacgcgccgctgaacctgcccatgagccagcagctcaaggacaacatcaaggcgccttcggacaagccagcgacctgaccgcaatacgtacctgaccgcaatacgtaatacgcaatggcttcgacgaacgtagttggcattctgggcggcatgggccctgcggcgggggccgacttcgttcggctgttcgtgcaggcctgcgcccagcagatgcgctctcgcggggaaccggtgcgggaccagtcttttccggagcactggctggcgcaggtgccggtgcctgaccgcaccgatgcgctgggctcgcccgagagcggcgggcaccagccgctcgaaccgatgctgcaggcgttggggcgccttgccgcgctgggcagccaggcggtggccattgcctgcaacaccgcgcatgcctggcatgaccggctgcaggaacgttttccgcaggtcgagctgctgcacatggcgcgcgaggtggcgcagcatcttgcggcgcaggatgcgggcaacgtggcgctgatggccaccgagggtacctaccgcgtgcggctctacgagcaggcgctggcccaggcggggctcgaatgccatgtgccgctggcggaagaacgccgcctcatcacgcgtggcatcttcgagggggtcaaggcgggcaacatgcggctcgccgaagaatgcttttcgcacgtggcgctgcggctcgccgaacgccatgggccggtcaccatcatcatgggctgcaccgaggtgccgctcgggctgcagggttcggccgctgcggccgggctgagcctggtcgacccggcgcaggtgctggcttcggcattggcccggcgcgcgtatcgcgactagtgcacggcgggcatcaacctgatgacgcacgggccgggctgatttcgcctacattgcggcgtgcgttttggcgcatgcccctttgttcgacgattcaactggagctctacccatgtcccttcgcgacgacagccgttccgatttcgattcgcttcgccccggcgagagcacagagcagggcgccacgcgccgcactgcactcaaggccgccattggcgtgggctacgcggccgccgtcatgccggtcatggcgcagaccgcgatcagcacctcggccgaaggcctgaaggccgggccgatcaagtacaccgtcaacggtttcgaggtgccggcctatgcggccgcgcccgcgggcaagaccggtctgccggtgatcctggtgctccaggaaatcttcggcgtgcacgagtacatcgccgatacctgccgccgcttcgcgcaactgggctatctagccattgcgcccgagctctatgcgcggcagggcgacccgcgcggctacaccgacatccccaagctgcaggccgacatcgtgagcaaggtgcccgatgcgcaggtgctggccgatctcgatggcgcactttcgtatgcatcggccaacggcggcaacgtggccaaggccggcatcaccggcttctgctggggcgggcgcttcgtgtggctctatgccgccaccggcaaggtcaaggccggcgtggcctggtatggccggctggtcggccagcccggcgagttgacgccccggcacccgatcgacgtcgcggccaacctgcaggcgcctgtgctcggcctctacggcggcaaggaccagggcatcccgcttgacacggttgataagatgaaagcagcgttggcaaatggaaccccggctgccaaggcttcgagcttcgtcgtgtatcccgaagcaggccacgcgttccacgccgactatcgcccgagctatgtaaagagcgcggccgaagacggatggcagcgcgccaccgcctggttcaaagccaatggcgtcgtctgacgacagcctgtagccacccaccgccgaaggccgtcccagtgacggccttttctctttttatgaacggtatcgggtatcgatgcccatcgacattgcagctatgaatttgatagtgatcatcctggccaccctggtcgccggcatcggaagcgtgtggctggccgccttgctcctgcgcgtgggtgtgcgcagcgggtcgggcggcgtgaattcgcagcacctgctgagcctggccgcaggcgcgctgctcgccacggccttcatgcacctgctgcccgaagccttcgaaagccgcatcgagcccgcgatgctgttcggcgtgctgctgttcggcctggtgttcttcttcttgctcgacaaggccgagctctggcaccacggacacgagcatcaccacggcgacgctctgccgggaccggtggggcaccaggcggccgggcacgcgcatgatcacgatcacgatcacggccatgcgcatcacgatcacggcgatcacagccacggccacgcaccccgcgcgggcggcggctgggcagtgctcaccggcgacagcgtgcactgcttcggcgatggcatcctgatcgcgtcggccttcatcgcggacatccgcctcgggctggtcgcggccgtcgccgtgctcgcgcacgaaatccctcatcacatcggcgatctggtggtgctgcggcagagttcggccaaccagcgtgcggcgctggtcaaggtgtcgctggccggcaccatgaccatgctcggcggcgtcgtagggtggtggctggtcgatcggctgcacggcctgttgccgtacttcctggtgctggcctccagcagctttgtctacgtggcgctggccgacctgattccccagttgcagaaacgactgcccgcgcggcagaccgcggcgcagatcgcatggctgatcgtcggcattgcgcttgtcacgctggtgagccggctcgcgcacggcgagcacgaccacggccatgcggaacacggccacgcagagcatggccatgcgcacgaaggcgagggcgccccggcgcacaaggactgaccggcaccggatggatactttccgaaacccacacctgtccggggaatggcgcacggcacccgaaagaggtgcaccattgggggtatgacgaatgtctcgcccatgctatcgccgaggaaccgatcatgaacaacgtcgacgccaagaagcgttctgctccgccatcgacagaggatgacgacgactcgcctgtcgatgatttcgaagagtccgaatcggaatccgaagccaccgacgacctgtcggacgaaaccggcatcgacctgaccgatgccagcgaactcgacgccgacaacgttcccgcggacgaagaattcgaccgggtgatgaacgcgcccgattgagccggttcttgatcaaccctgggccacagccgctgcgcgcagacgctgcgggccgagcatttcagccgtgagaccgaagcccgcgatgcgctccggcagcggcaggccgcgcgccagtgcggcgcacgcctcgcccatggccgccgatgtctggatgccgtagccgccctgcgccgccacccagaagaagccgggtgcatcgggttcgaaaccgcccaccaggtcgccatcgcccacgaaggaacgcaggccggcccaggtgcgggtgggccgccggatggcgagcgtggttgcttcctcgatgcggtggatggcgatggcgatgtccagttcctcgggctgcacgtcctgcggttcgacggggtcggcattcgccggggagccgagcagcatgccggcgtcgggcttgatgtaccagccttcgtcggcactgaacaccatgggccagtgcgccacgctgccgccgctgccttcgggcggcgcgaaaatgaaggccgagcgccgccgtggctcgatgccgatgggctgcacgcccgccatttgcgcaatggtgtcgacccacgcgcccgcggcgttgatcaccaccggcgcttcatagacggtgccgccggccgtcacgcgccagcgctcgccgatgcgctcgatggcggtcacgccggcatcgcacaccagcttgccgccggcctgccgcatgccgcgcagatagccctggtgaatggcgtgcacgtccatgtcggccgcctcgggctcgtagacgccgccggccacgtgctcgggccgcagcaccggcaccatcgcgagcgcctcttcgccgctgagccgcttcgcgcccgtgttcatggcgcgcagcacttcccagtgggcgtcgagttcggccacatgctcggcgcctgccaccatcaaggcgccgcgcggcgtgagcagcgggtgctcggcaaagccctcgggcgggtgttcgagaaaagcgcggctcgccatggtgagcgcgcgcacctgcgccgtgccgtagctttccatgaagagcgcggccgaacggccggtggagtgatagcccggctgggcttcgcgctcgagcaggatcacgcgggcgtgcggggcaagccaatgggccaccgaagccccggcaatgccgccgccgatcacgaggtagtcggccgcaacgggcgctggtgtgttggaagtcatgggtgaaaagtgtaggtacaaatttgcgtatacgcaaattaaatcgttatcactacaacgagactcgctgcatcgtgctggtgaaatttgcgtgaatgcaatttgcgcatgcgcaaatttcatgcgcacagaacgaggatctggagcggaaggcccggcatcgggctggcagaatcgcggtgcactacaagagagagccaagcgtgaatccacacacggggaccaagccgggcaccaagccagcggccaagccgaagggcgagcagctcgcgctggaccgcaccaccttcggccaccgcctgcgcagcgcgcgcaagcgtttcggctggacgctggcgcagctggccgagcgttcgggcgtgtcgatcaccaccatctcgcgcgcggaacgcgggcagctcgcgctcggatacgagaacttcaccgcgctcggccgcgcgctggagatggacatgaacgcgatgttcgcgggcgcgggcgtcaagcccgcacagctcgacgggccggtcgtcacccgcgcgggcaagggcgtggtgtaccgcggcctgtcgatcgcctacgagttcctgggcaccacggcagccggcaagcagatgagcccgatcgtcggcaccgtgcatgcgcgccgcattcatggccccgaagacttcgtgcggcacgcgggcgaggagttcgcctatgtgctgtctggcgaaatcgaagtgcacttcgacaatggcaaggtcgtgcggctcgcgcgcggcgactcgctgtacttcgacagccgcatcggccacgcctatgtgagcgtcagccggcaactcgcgaagatcatcggcatgacgatgggcgagagcgggcacatgaaatctgcgcgcgaagcaccgtcgttgaagccagcgcgcaaagttgcggcggcgaagaaaaccgggcgcggcggcaagggctgacgggggggcgactcgcgtcccgggcgcgctctgccggctgcctctgcgcgcccggcccgtcacgccatcggctgttgcgccatggcccacccgcgcttgccgacagcgtcgttactgaagataatgcatttaacgttgagttacatttgcggatgaccgctgtcccttctgcccttcttttcgctctcccgtctcttgccctttttccgctgatcccatcgggcggatcaggcaaggcgcgagcgacgcggttgcgggtccgttcggcttgagtgcgcgccgcgtccgtgccgttggcttgagcctgcttgcggccagcgcgttcggcgtggcccatgcgcaaaatgcgatcaaggcggttgcgggttcgatgcaacagggtgtcgaggtcatccagatcgatctggcacagccgctcgccgccgtacccagcgggttttcggttcagagccccgcgcgtattgcaatcgactttcctggcgccaccaacgatgtggggcgcaccgccatcgaagtggatcaacccaacctgcgctcgatcaacgtggtccaggcaggcgagcgcagccgggtggtactgaatctccggcagccgacgctctacacggcagagatacagggcaggtcgctgcgggtcacccttcaggcggttgcccagacacggcccacagaggctcccgcaccggccagagccgcagcggcgccccgtcgcaccgagccgatcacgctgaacttctacgaagccgacatcgaggccgtggcgcgcaccatggcggtgatcacggggcgtgatgtggtggtcgacccgagcgtcaagggcacgatgagcctcttcaccgaccgcccggtccagccgacgaccgccttcgatcagttcgccgcggccttgcgtctgcagagcttcgcggtggtggaggccgacggcctctacaaggtggtgcccgaggccagcgccaaggtgctgagcaacacggtcaacacgtcgatcggcgccatgtcgtcgtcgggcagcaatcaggtcgtcacgcagatcttcaggctcaactacgagtcgccgggcagcctcctgccggtgctgcgcccgctgatttcatcgaacagcgccgtcaacctgagcccgggcaacaactcgctcgtgatcaccgagtacgccgacaacatgcgccggctcgcgcgcatcatcgcggcgctcgatgtacccaaagcgtccgacgtcgagatcatccagctcaggcacgcgatcgccaccgacctgatcccgctggtgcagcggcttatcgacggcggtggctcgggcgcaacgagtgccgctgcagcaggtgtcgccgacacatcgtttcgcaccacgctgctggccgatccgcgcagcaactcggtgctcatgcgtgcggccaacccggcgcgcgcgcaactcgttcgcacgctggtcgagaagctggaccgcgcacccgccgagagcagcaacggagcggctggcaacatctacgtggtctacctgaagaacgcggatgcggtgcgcctggcggccacgctgcgcgccgcgatggcggcaaaccagcagtccacgacgccgggtgccccgggcgccgccggcaacagtcctgtagcgcagcaggccatgcagaacagcatgaacgggcaaggtggctcggccggcgccaatgcgccgctgaacaacgccaaccagccgtcgaccggcggccagatccaggccgatccgtcgaccaactcgctgatcatcacggcgcccgagccgcagtaccgccagatgcgcgcggtgatcgacaagctcgacggccggcgcgcccaggtcatgatcgaggcgctgatcgtcgaggtgagcgccagcaaggccgcaagcttcggcgtccagtggcaaagcgcgctgggcagcaacggtgtcatcggcaccaactccagcctcaacgggacgaacatcctggcactgacccaggcgctggccacccggaatgccgccggcctggcgtcgtcgattcggccgggactgaacctgggcatcgccggcaagatcggtggccagtacatcctgggcgccatcgccagcttcttcagcagcgacggcgatgccaatgtgctctcgacgcccaacctgctgacgctggacaacgaagaagccaagatcgtcatcggccagaacgtgcccttcgtcaccggccagtacgcgagcacctcgggctcggtgggcatcaacccgttcaccacggtggaacgcaaggacgtcggcctcacgctgcgtgtgcgcccgaccatcaacgagaacggcaccgtgaagatgacgatcttccaggagacctcgaacgtcgatgcggccacgatggccaacgccaacggccccaccaccaacaagcgctccatcgaatcgagcgtgctggtcgaggacggcgggctcatcatgctgggtggcctgctgtcggacacctacaacaccagcatcgagagggtgccgctggccggcgacatcccggtgctcggcaacctgttcaagaacgagaaccgcacgcgcaacaagagcaacctcatgatgtttctgcgccctgcggtgatgcgcgacggtgcctcgaccgaggccttcgcctacgaccgctacgacgagatccgcggtttgcagaagcaggtgcagccgaacaccgacaacatcatgctgcgcaacgtgaacgccgctcccgtgctgcccgaggcaccgctcgcaagctcacccaaccgcggcaacggcagcatcagcatggaaggcacccggctcattcccgctccgcaggaaaccgccacgggcaaccgcaagctcgcgccgccgctgctgcgcggcgccttgccctccaccgccgacccggccagcggacgggagttgccgtagggcgcgagtcgaagcaccggctttggctgccacgcacgcgacgagtacatcgagattcgatcgtgccgcgcatctaccttgtcacgcgcctgctgaccgagaccggcaagcagtaagcagcgccggggcagcacgcctcagggctgttgtcccggtggctcgccggggcggcgcggcggtcgtttggcggcggccgcagcggctgctgctgccgcgtgctgctgggcttgttgctgctgctgctggcgcatctgcgcctggtgtgcctgctgttgctgcatctgctgctggcgttgctgctgctgttgttgcatcgcctgttgttgctgttgcgcgcgcgcggcctgcgcttgctgctgttgctgttgctgttgctgttgctgttgctgttgctgttgctgttgccggcggcgcatctgctcctgttgctgcagggcctcgttctgggcccgttgctgctgcgcctgctgccgttgtatctgctgctgttgagccgcctgctgttgctgggccgcacgcgcttgctgctgcgcctgctgttgctgttgcatctgctggcgccgtgactgttcctgctgggcctgctgctgggtttgctgcgtctgctgctggcgctggcgctcctgcaatgtgtgctgctgctgttgctgggcttgctggctggcggcgcgcgcctgttgctgctgcgccatctgctgccgccgcacctgctcctgttgttgctgctgttggagccgggcctgttgcggctgctgctggttggcggcgcgggcttgttgctgggcctgctgcgcctgttggcgccgcatctgttcttgctgctgttgctgctggcgctgtgcctgccgtgcttgctgttcctgggcttgccgctgttgcgcctgctgttgtcgggcctgttgttgtgcgcgttgctggccttgctgttgctcctgcatcaacgcttgctgctgccgtgcttgtcgctgttgctgctgctgctgtgccagttgggcttgcggctgtggcgcgaagcccgggctgcccgcggcagggggcaagggagcgccggggggcatgccgcggggcgcgccgctgttgtagacgttccgcacgttgttgttgaccacggtggtcgagcgcgagatgtaggtgctgttgttgtagaccaccgccggccgggcgtaggccggctgcgcgatgcgctccggttcgcgaccccgccagcgcggtgcgccccagttcatgttccatgcgttccagccccagtcgtgccgctccagcgcggcgcccacgatcacgccggcaccgaacgccagcgcgcccgccgcggcgacttgcccgcggctgtagcccggcgcgacctcgacgggtcgggcgtacgcatagccgggatagacgggtaccggctcgccgtagatcacctgggggtcatagctcggcacgtacaccacgtcgggctgcaccggctcgatggtgatcagctgccgcggcggttcgatcaccgcggggcccgcatagaccggctgcatgtccggcgccgggacgtagtcccgcggcgtcgcggcgctggcgacccggagcttgctgttgttcttgaggcggcctgcgctcgacgcgcgctgccgcatgacctggatcgcgttcatcacgtcggccgggtcgttgtagtaggcctggccgagtgcctcggtccacgcgatgttcccggccatctggttcagcaccgggcggaatgcggtaagcgacttgacgctcggatcccaaggctgctggttggctgcatcggcgagcgggccgcccttgagtgctgcgttctgtgccagccaaccgtgtgcggcggtgatctggtcgggataggtggagccggccagcacctgcgccaccagcttgtcgggatacagcgcgatgggagcgacgagctggtagagctgctcggccgagggcggcgtataggccgcaggcgctggagcggctggcgcaggtgggggcgcaggcgcgggtgcagcggccactggaggcgcgggtacctgggcgctgggcgcgttgtcggtcttgttgcagccggcgatggcaagcgcgccaatgcacagcgagatcgtcaggagccgcgcgacggacgcgcggcggaatgatgttgtcatctggagttcctatgggcgccgaccttgtcacgccctgaactctttcaacggcgcgtcacgtgccgcgacgacgccagcttgcatcgccgatgcaacggtctgtgtcggtgctgtgccgcctgcgctgtcggcgcagaaccacaggcctccttacttggcgccgcccgcgtacttggtgacgctcgtcgcgttcacgtgatagccgctcacgcccatcatcgaatcgttgcgcagggtctgcagcttgccggtgacccacacggtgtccatggcgcggaacttggcgccctttggcgtgaccacatgcaggatctggttggccggtggcggcggcgtgtggatgcacgcgccgaagtagggcacgagcaggaactcggtcacctcgcccttggcctcttcgagcggcacgatgaagcccgggatcttgatgtcggcgccgttcatggccggattggtcggcgcgttgttcgacacctcctgcatcttcatgagcagttcgttggcgcgcgggtcgccgtcgttgagtgcactcaggtccatgcccttgaattccttggccgggtcccagtccttgggcaccagttcttcccaggtaatctggcgcggctggcccggcgcggccttggccgcagcaggcggtgcagccttgccgccgagcgggttcgatgcggtcgtgtccttgggcgcgggttcggcggcccacgcggcggcagcgaggccggcgccagcgagcagcatcgaaagccgggtgaaagctcggagcgtgggtgtcttctttgcgatgcgcatggtttcaaatcctcggtgagaggccgtcggccaacgagagccggtaagcacggatgccgggcaaaaggcttgcgagccagcccgccaccagcaggcttcccatcagcagccattcgttcagtgtaggttctgaaagactcaatgtcagcccgaactgcgactgcagccatggcgagagcagggcgatgccgagcacggccatgaccacgccgaaggccacgcccagcacggtgaccatggcgccctcgagcgcgagcagcgccagcacatggcgcaggccggcacccacggcgcgcagcacggccagctcgcgccgcctttcgttcaggcctgccatcaccaccgagacaaggcccgcgaggcttacgagcgcaaccagcgccgacatcagcagcagcgcgttctcgccgatgccgatcacgctccacagttcatcgagcgccacgcccggcaggatggccatcagcggctcgccggagtaggtggaaatccagcgctggacgccgaacaccgcagagcggtttttcaggcccacgagagcggccgtcacgttcttcggcgtcaggtcgaacttgcgcacctgctcggccgggatcttcacgcccggcatcggcgcgccgcccacccattcgaggtggatggcttccattgcttcgagcccgatgtgcaccgtgcgatcgaccggcgtgccggtgcgggcgagcacgccgaccaccgtgaagggcttgtcggtatgttcggccgtgttgagctcgccgctgccgtgcgcgagcgtgatcttccggccgacgtggtagccgagcttgtcggccacttcggcccccaccaccgcgtcgaacagttcgctgaagggcttgccttcgcgcagcttcagcagctggcggtcgccatagcgaaagcgcgtgaagtattcgggcgaggtggccagcaccgagaagccgcggtgcgagtcgcccagcgaaagcggcaccacccagtcgacgccctggtgcgcggccagcgcctgcacgcttttccacgagatgttgttggtggccgcgccgatgcggaacaccgaatacagcagcagttgcgtggagcccgtgcgtgcgcccacgatcaggtcggtgcccgagacggacgatgcgaagttctcgcgcagctcggtgcggatgcgttcgacgccgagcagcagaaaggtcgacagcgcgatcgagaacacggtgagcgccagcgtgaagcgccggttccaggcgctgtgccaggcgatcgaaaaaagtgctctcatcggcaggccttcacgcgtccaccgccatcgcaatcgaagccgcgcggttgatttcgggcagcagcacatgccgggcaaagcgctgcgcgatgcgctggtcgtggctcacgaacacgagcgcgctgtggttcaccgcgcatgccgtcagcagcacgtcgagaaacgcttcgcgccggtcttcgtcgagcgcggaggtgggctcgtcggcaatcaccacttcaggctggccgatgagcgcgcgcgccgcggccacgcgctgctgctggccgaccgacaactgcattgcctggcgcttccacaggttgcggtcgagtcccatctggtcgagcaggtgctcggcttcttcgcgggggcttccgctgcgcgcggcctgcgatgcacgccgctgcgagaaacggcagggcagcagcacgttgtcgagcacgctcagatagggcagcaggttgaactgctgaaagatgtagcccacgtgcgccacgcggcagcggtcgcgcgcggcacccgagagctgcgaccagtcgtgccccagcagcgtgacgcggccttcgtcggccaccagcacgcccgccagaagggagagcagcgtgctcttgccgcagccgctcgggccgtgcagaaagaccgactcgccggccgtgatgcgaaaggcctcgatgtcgatgcacggcgccttcatgccgggccacgcaaagcgcagcgcttcgacggcgagcaccacgcgcagtggcgatgcctcgccctggggggcggtgctcacggccttacttgccccagccgaggcgcaccggctgcgcggcctgcgcaccgccggggcgcttgagctggcgcttgaactggccttgcgccgaagcgatctgcgcatcgatctggcgcgtgcccttgaatgcggcgaaaagattcacgtcgatgaactttgccgcggccgcgttggtgcagttgaaagagaaggtggcgtcgaggtccgcgtggccctcgggctcgctcgggtcaggcttgccgaggccaagcgcgccggagcgcaggtcgaccgggccgagcttgcagttggccgccgggtcgatggcaaagagcttgtccgccgcgcgcagctgggcgacggcgtcttcggcggtcttcttctcggcatcggtcttgggggctcgctcgaagccgacgatgttgtcgagcggcgtctccatgttgatcacgacggtggggccgtcgatggccacgtcgagcttgagctggccgtgcacgtgcgcatgctgctgctgtgcctcggcggaaagaaaaggggttgccgcgagcattgccgcggcaaatgcgaagccggatgaaatgcgtcgtcgaagtcggatctgtttcatggttctgcgccttgccgggtcggcagcccaggcgtgttgctccactcgctccagctgccggcatagagcgcggtggtccccagtcccgcgatctgcatggcaagcaggttgggcacggcgctcacgccgctgccgcactggtggacgaccgtcgccggatcgcgtcccgcgagcagcgcttcgaactcggcacgcaattgcgatgccgacttgaacttgccgtcggggccgaggttttcggcgaagggccgattgaaagccccggggatgtgacccgcgatcgggtccagaggttccacctcgccgcgatatcgtgcggcggctcgcgcgtcgatcaggttctggtcaggctggccgagccggcgcaccacggcgtcggtggtcacgagcttcgcaagcggctcgcccggcacgaaatttgactggaagtgcgtcggctcttcgcggttcgtgacttcgccgcccgcggcctgccatgcctgcaggccgccatcgagcacggcaaccgcgtcgtgccccatccacttgagcatccaccagagccggccgcagtagttggcgccgttgcggtcgtacaccacggcctgcatgtcgttggaaaagccgacgctcgacaaccaggccgcgaacttctcgcggctgggcaacggatggcgcccgcccgaggccggcacgccgtcatcccgcgcgacgaccacgtcgccctgtgcgccaggcaggccatgtttcgcgctgaggtcggtgtcgaggttcgcatacacggcgccggggatgtgcgcggcggcatattgcagcgcgcccgcctcgggcttcatgaggtcgaagctgcagtcgatgaccatgagcggcgcgccgccggcctgcagctgctggagttgttcgacgctgacgagggtggtgtacatggtgcggttccttcgttgtcgatgggttcgatgtggttcagtgttcttcggccggcgccttgggcactgcgcgctggcgcagcacggtggctgcgatgccgctcacgatgatgagcgccatgccggcccagccggcgccgtcgatgcggtcgtcgaacagcaccacactgtagaacgccgcaaagacaatgccggaatactgcagattagccaccaccagcgtaccggcctgggtcttggccgtggcgtaggcgcgcgtcatgcagagctggccgagggccgccaaaaggccgatcggcagcagccacagcgcatgctgccacgtccacgaatccccgcccgaaaacccggtggcggccgtggcaaaggcacccgccacggccgagcccaccgcgaaatagaagaccgtacgcagttcgggttcgccgatgcgcgacagcgccaccacctgcatgtaggcaaacgccgccgtgaggcccgaaagcagaccgagcaggcccgcgaaaccttcgttggcgttgaccgagggcttgagcatcagcaccacgcccacgaagcccgcgagcaccgtcagcaccagcggcccctgcagcggcgggcgctgcacgcggccgtcgcggccgggcaccggcacccatgcgagcagcgcgccgcccaccaggaacgccgcgatccagacgctgctcatgtagttgagcgtgaccgcggtggccagcggcatgtgggcgatggcgtagaaccatgcgcccagcgacaccacgccgatggtgctgcgccaggcgtgcatgccggggtagcgggtggccaacgagacaccgcggttgcgcgacagaagccacaggaacacgatgccgatcaggccgcgcccgagcaccatctcgccgctgttgaaccaggccgaggctaccttgacgaccacgctcatggtggcgaacaagaaggcgcccagcaccatccagagtgcttgcactatgtgctcaggcgctctgcattgcgctgcggtaccactcgtggaattgctgcatgccgtcttccatcgggctctggtaggggccgctctcgtcgtcgccgcgcagcatgagggcgcggcggccggcgtccatgcgctcggcgatctcgtcgtcttccacgcaggtttccatgtaggcggcctgctgggcttcgacgaattcgcgctcgaaggccacgatttcctcggggtagaagaactcgaccatgttgagggtcttggtggggcttaccggatgcagcgtcgacaccgtgagcacgtgcggataccactcgaccatcacgtgcgggtagtaggtgagccagatggcgccgtacttgggcggcttgccctctcggtacttgaggagctgctcttgccacttctggtagatggggctgccggcgcggccgagccggttggccacgcccaccgtctggaccgagaagttgcggttgaactcccagcgcaggtcgtcgcaggtgacgaagctgccgaggccggggtggaacgggccgacgtggtagtcctcgagatagacctcgatgaaggtcttccagttgtagttgcactcgtgcagttcgacccggtcgagcgcgtagcccgtgaagtccaggtcggcgcgcgggccgagttcggccatgtcggccgccacgtcgcggcccacgccgttcgggccgccctcgaacagcaggccgttccactcggtgagcggatagttgtgcaggttgaggcaggggtcctggtcgaaatgcggcgcaccaatgagcgtgcccgtggcgcgcgggtcggcggcagcgtaggtccagcgatgcagcgggcagacgatgttgccgccggtctggttgtcgagctgtccgcggccttgcaggatgagcgcctgccggtggcggcacacgttcgaaatgagttcgacgcccttgggcgtgtgcacgagcgcgcggccctggtgctcctgcggcagggtgtggtagttgcccagctcgggcaccgcgagccggtggcccacgtagcgcggcccatgcgcgaacagcgtttgcatttcgcgcgagtaaagcgactcgtcgaagtatgcggaaactggaagttggctcgcggcctgctgcagttgaagacttaaatcagacatggaggacctgaccaagctccccacagggagaaaaaagagaaaaaacggaaggcgccgtctggagtccgaaggggcgacggcccgaagagttgtgccggggtggccggcaagggaagctcggattgtacccaagggggcaccgcagcgcccatggcttttcacatgcctgcgccggacggccgcggtcgacgcccatggtccgttcagccgccatccgccgcatgcttcggggtggtcggcggcactttggttcccccaccctaaaatgcttgatttcacattcgttcgctcgcatgcccaaggtcccttcttccgccacgtccagcccgacagccacgcccgacaccgggccgctgccggccagctacgaagccgggctccaggagttggaacaattggttgcagaactcgagtccggacaactgccgctcgaccagttgcttggcagctatcagcgcggcgccgcactgctcgccttctgccgcgaaaagctgcaggcggtcgaggaccagatcaaggtgctcgatgcggggagcctcaagccctggaccgccgaatgagcgccgcacggccgcccgaaggcgcgagcgcccccttggggggcagcgaagtacacgcagtgacgagcgtgggggcaacaatgagcggggctgtggtcaattgggatgctggccggctggccggttggagcgagccgcacctggcgcgcgtcgaagcagcgctttcgcgctgggttggtgtcgatgcgccggtgctgctcggtgaagcgatgcgctacgccgtgctcgacggcggcaagcggctgcgtccgctcctggtgctcgctgcgagcgaagcggtgggcggcaatgcggccgctgcgttgcgcgcggcttgcgcaacggaactgattcacgcctactcgctggtgcacgacgacctgcccagcatggacaacgacgtgctgcggcgtggcaagcccacggtgcatgtcaagttcggcgaggccgatgcgctcctggccggtgatgccttgcaggcgctggccttcgaactgctgacgcccgacggcgacgaaattccggcttcgacccaggccatgctgtgccgcctgctggcgcgcgccgcgggcagccagggcatggcgggcggccaggccatcgaccttgccagcgtcggcatggccctgaacgaagcgcagttgcgcgaaatgcatcgcctgaagaccggcgcgctactgcagggcagcgtcgagatgggcgccgcctgtgccggtgccgtggcgcctgctgcgctgaatgcattgcgcgactacggcgccgccatcggcctggcgttccaggtggtcgacgacatcctcgacgtcaccgccgattcgcaaaccctcggcaagacggccggcaaggatgcggccgccgacaagccaacctacgtttcgctgtggggcctcgacggtgcgcgtgcacaggcacggcagttgctcgccgaagcgcttgcggcgctcggccgcagtggccttgccgacaccgccgcactgcgcgcgctggcccacatggtcgtcgaccgcgaccgatgaactgttcacagatggacaagaagaaccacgacgattccatggcaccgctgcttcccacgcttcacgatccgtcgccgatccgccactacgaccgcgcccagctcaagcagctgtccgacgaggtgcgcgcctgcgtgctcgacaacgtctcgcgcaccgggggccacctgagctccaatctcggcaccgtcgaactcacggtcgcgctgcaccatgtgttcaacacgccgcacgaccggctggtgtgggacgtgggccaccagacctatccgcacaagattctcacggggcggcgcgagcgcatgcccacgctgcggcagattggcggcatctcgggctttccgcagcgcagcgagagcgaatacgacaccttcggcaccgcgcattcgtccaccagcatctcggccgcgctcggcatggccatggccgccaagcaaaagggcgaagaccgccacaccgtggccatcatcggcgacggcgcgctcacggccggcatggccttcgaggcgctcaacaacgccggcgtgtgcgactgcaagctgctggtgatcctgaacgacaacgacatgtcgatcagcccgcccgtgggcgcgctcaaccgctacctcgcgcaactgatgagcggcaatttctacgccgccgccaagaacgtcggcaagagcgtgctgcgcgccgcgccgccgctgttcgagcttgccaagcgactcgagcagcatgccaagggcatggtcgtgccagccacgctgttcgagcagttcggcttcaactatgtcgggccgatcgacggccacgacatcgattcgctggtgcccacgctcgagaatctcaagcatctcgacggcccgcagttcctgcacgtggtcaccaagaaggggcagggctacaagctcgccgaggccgacccggtggcctaccacgggcctggcaagttcgatccacaggtcgggctggtcaagtccactgcggtggcgaagcagacgttcacgcaggtcttcggccagtggctgtgcgacatggcggcgcacgacggccggctggtgggcatcacgcccgccatgcgcgaaggctcgggcctggtcgaattcgaaaagcgctttcccgaccgctactacgacgtcggcattgccgagcagcatgcggtgaccttcgcggccggcctggcctgcgaaggcctgaagccggtggtcgcgatctactcgacctttctgcagcgcgcctacgaccagctcattcacgacgtcgcgatccagaacctgccggtggtgttcgcactcgaccgcgcgggcctcgtgggcgccgatggcgccacgcacgcgggcgcctacgacatctcgttcctgcgctgcattcccaacatgagcattgcctgcccggccgacgagcgcgagtgccggcagctgctgtcgagcgcctacgagcagagccatccggtcgctgtgcgctatccgcgcggcgcgggtgcgggcgtgacgccgcaccttgcgctcgacgcgctgcctttcggcaagggcgaggtgcgccgggaaggcaagcgcgtcgccatcctcgcattcggcagcttgctgtacccggcgctcaccgccgccgaatcgctcgacgcgacggtggtcaacatgcgctgggccaagccgctcgacgtcgacctgctgctgcaggtggcgggcacccacgatgccatcgtcacgatcgaagaaggtgccgtcatgggcggcgcgggcagtgcggtgctcgaggcgctgcaggctgccgatgtgatgaagcccgtgttgcagctgggcctccccgatcaattcatcgagcacggcgacccgggcaaactgctcgcatcgatcggcctcgacgcagcgggcatcgaagccgcgatcacgcggcgtttcggcgccgtcgcagggtaaaccccggccggccgcgtgtaagcgcgtttttacaatcgttgcgacttacaaaagtcgtcgacgcggccacaagccgcgtttcgttttttccaatgcactcggagtgaattcaatggatcgtcgttccctcatcaaaaacgccggcatcgctggcgttctggccgccggcattgcgcccgcagttcatgcgcaagccgccgtccgctggcgcctggcgtcgagctttccgaagccgctcgacacgatctatggcggtgccgaggttttctccaacgcagtcaaggccatgtcgggcggcaagttcgagatctcggtgcatgcagctggtgagttgatgccggctttcggcgtggtcgacggtgtgcagcagggttcggtcgaagcctgccacacggtgccctactatttctacggcaagaatccggccttcgcgctcggttcggccatccccttcggcatgaacgcgcgccagatgaacgcgtggatgatgcacggcaacggccgcaagctgatggacgagttctacggcacctacgggatgctgagcttcaacggcggcaacaccggcacccagatgggcggctggttccgcaaggaaatcaagacccccgctgacctcaagggcctgaagatgcgcctgggcggtggcctggtgggcgacgtgatgaccaagctcggcgtggtgccgcaaagcatcccgggcggtgagatctaccaggcgctggaaaagggcacgatcgacgctgccgaatgggtgggtccgtatgacgaccagaagctcggcttcaacaaggtggcgccgaactactactaccccggctggtgggaaggcggccccgaggtcgacttcttcatcaacaagaaggccttcgacggcctgtcgcccgagaacaaggccatcattgcggcagcttccgccgtggcctcgcaggacatgctggccaagtacgatgcccgcaaccccaccgcgctcaagcaactgatcggcgccaagaccaagctgctgcctttcagcaaggaaatcctcgacgcatcgttcaaggcttcgctgcaggtctacgaagaaaacggtgccaagagcccggagtggaagaagatctacgccgacttcctgactttccagcgcgaccaggtggcctggttccgcgttgccgaaggccgcttcgacaactacatgcaatccgtgaagctctgagctttcaaggctgcaaaaaaaaccgcgcattgcgcggtttttttatgggcgctacttcatgaaagagcgccggcacgaacgcgcaaatcagagcctgcgtgcctgcttgagctcggccaccagccgctcgaactcggcaatgagttccggcgtggccgcatagaacacggcgaacttgccgaccagcgtgcgcacgtagagccgcggcgcaatcagccagtcgagcccgcgcacgcggatcagcttgccgaatgcgaggtcgtcgaacgccatctgcttgtcccagatccagcgctggtgcaggccctggcggtcgatgcgcgtgcggctggtcatgatgtggaaccaggtccagcccatcagcgcaatgccggcgagaaaccagccgaggccaccggtcttggcggtgccgagggcgcccaccgaccagagctgtgccagccagaaggcgcagccgcccacgatcacggtggccagcagcttgaagggcagcgagaacgcctggccctcgactgcatcgccccccgacggctcgaaacgaaacggtgcgggacccaaggcgcctacttcttctcgggttcggtggccgcaccggcaggtgcttcttccttgggcggatcgccgaagggattttcaccaccgccgccgctgtcagcgccggagttcggggtcatgtcgtcgatcggcacctcgatctggaccttgtcggtatcgatcgtctcttccttgggcaggaacatcgtcaccgtctgcggcacgaagatcacgatcgcgaccaggatcagctgcatcagcacccagggaatcgcgcccatgtagatgtcgttcgacagcaccggcttggctattcgtttctccttgaacagcgtgtccgcaatgcctcgcaagtagaagagggcaaagccgaacggcggatgcatgaagctggtctgcatgttcacgcacagcagcacgccgaaccacaccaggtcgatgccgagcttggccgccaccgggcccagcatcggcaggatgatgaaggcgatctcgaagaagtcgaggaagaaggccaggaagaagatgaacaggttgaccacgatcaggaagccgatctgtccacccggcaggcccgtcagcaggtgttcgacccacttggcgccgtccacgccctggaacaccagcgagaacacgcgtgcgccgatcaggatgaacaccaccatggcggtgagccgcatggtgccgaccatggcttcccagatgagacccagcgtcagccgcttgtggatcgccgcgaggatcagcgcgccgaccacgcccatggcgcccgcttcggtgggcgtggcaatggcggtgtcgatgcctggcaagccgcccatcgaacccagcacggcgaagatcaggatggccgacggaatgatgccgcgcaggcatttggcccacagcttggcgccgctcagcgtgcgtgcgctcttgggaatgcccggaatgtggtgcggcttgatgacgccgagcatgaaggtgtagcccgcgaagatcagcacctgaaggatcgacggaccccacgcgccgcggtacatgtcgcccaccgatcggcccagctggtcagccatgacgatcagcaccagcgaaggcggcaccagctgcgtgatggtgccggacgctgcgagcacgccggtggcgtagcgcatgttgtagccgtagcggatcatcaccggcagcgagatcagcgccatggcgatcacctggcccgccaccgtgccggtgatggcgccgaggatgaagcccacgatgatcaccgagtagccgaggccgcccctgaccgtgccgaacagctggcccatggagtcgagcatgtcttcggcgagcccgcacttttcgaggatggcgcccatgaaggtgaagaacgggatcgccagcaacaggtcgttcgacaaaatgccgaagatgttgatcggcaagttctccatgaacaccgccgggaaccagcccatctggatcgcgaagaagccggaggccatgcccagtgcggccagcgagaacgccaccgggaagccgatcagcatgatcagcaccagcccgccgaacatgatcggcgcaaagttttccatctgcatatctgtgctgtcctgtatttctagtagttcactgcgctacccgtcacgccaggcaagcgaagcgatgcccgttcgggaaacaccgcggagccggctttgccgggccgctggtgttgccccctcgagggggagccggctacacgaagtgagccgcttcgggggtgggtccagttcactggaccggcttttcgtagtgcgtgtccatctcgatcaggcccatcaggtaggccacgcgcttgatcacttccgacactccttgcaggaacatcaaggcaaagcccagcggcagcagcagcatggcgggccagcggatcagcccgcccgaattgttcgacatttcgccggacagcagcatgctgtagaaaagcggccagctgagccaggcgatgatgcccatcaccggcagcagaaagcagagcaggccgaacagatccacgtagactggcccatggcccttcagcttgccgtagatgatgtccacgcgcacatgctcgttgagcttgagcaccactggcgcgcccagcatgaccgtggcggcgaacaggtaccactggatttcgagccaggcgttggagctggtgttgaggccgaagcggacgaaggcgttgccggcggaaatcagcgccgcggagagcaccgtgaacgcggcaaccttgccgagctggctgctgatccagtccatccagaacgaaaacttgagaagtgcggacaagggggtctcccggccagatgacaaaagtgtgatgccttgtgggcaatcggcacaaagcctgcgatgttaacgcggctatgctgagtggccgctgatgcccatcggggggtttccctgagcaccataatgaagcaatggctgcgccgcattccttaccgcactccatcgattcgcccgacatgcagcgcgcaggccgcgagctgctgtctctggccctgatcgatgcgcgcaaccacacgctccatctcctgtcgatgtatgaggaggcgctgggttcggccgcgctccacgtcgcgcgcacggacgacaccggcgtggtgccacccatctggctggccgggcacatcggctggtttgccgaatggtggatagggcgcaacacgcagcgggccttcggcgccgattgtccggtgcgcccaacccggctggccgccatcgatcccaacgccgacgcctggtggaaccccgcccaagcgtcgcacgcgcaactctggtcgcccggcttgccggacctgggccagaccaaggcctacctgctcgaaacgctggagagcacgctcgaactgctcgagcatgcggccgagaccgatccggggctgtacttctaccgccttgcgctgttccacgaagacctgcgcggcgagcagttcatcgtgatggcccagaccctggggctgccgctcggcatcgagccggtccccacctccgtcacgcgcgagccgctgctgctgcccgccacccggtgggagcttggcctgcccgagggctgcggcttcgcatttgcgcaggagcgcggcgcgcaccgtgtcgacgtgcccgagttcgagatcgatgcccagcccgtcacgtggaaccagtacatcgagttcgtcgacgagggcggctacgaccgcgaggagttctggcaccccgaaggatggcgctggctggcttcgcagatcgaggggcggcgcgggccgcgccatgtcgagcagatcggggcggcgcgccacggcacgggtggttcggtgctgcagcagcggttcggcgccaccgtgcgcgcggccggccaccacagcgcggtgcacctgagctggtgggaggccgatgcctgggcgcgctgggccggccggcgcattgcgaccgaggtcgaatgggagattgcggcgctgaccgcggcacggcgcggctttcgctgggccgacgtgcacgaatggaccgccaacacgctgcggccctggcccggctttcgggccgatccgtggagcgcgggcagcgagttcgatcccactacggttttcggcaaggcgcgcgtgctgcgcggcgcctcgttcgcgacccgggcgcgcctgcgctcgccgcggcgccgtggctttgcattgccggaccgcgacgacggctttttcggctttcgaacctgcagtctgtaactcaccctcggcgtcgctagggaatgccgcctgatgagagcggcggcgccacttcctccagcggcttgcactccgcatcggctgcatagcgcagggccagcaatcccgcgacgatgaccagcgtggcgccgatcgcgtagcccaccatcaccgcgccgcggctgccggtttcgatcaacatgccgaacagcacgggcgccgcgaagccgcccgcgcccatgccgatggcgtagaaaatcgcgatcgccatggcccgcatctcgagcgggaacacttcactgacggtgagataggccgagctcgcggcggccgaggccaaaaagaacaccgccgaccagcacagcgcctggctgcgcgcgtcgagccagcccatcatgaaggcccagccggtgagggcgagcccgacgcctgcgagcacgtaggtgagcgcgatcatcttgcgccggcccacgctgtcgaacagcgggcccagcagcagcggcccgagcacattgccgagcgcgaacggaaagatgtagagcgccacgttgccttcggccacgccgtagaagcgcgtgagcaccagcgcataggtgaagaagattgcgttgtagaaaaaagcctgcgagaccatcagcgccacggccaccacgctgcgctcgcggtagcggcgcagcagcacgtgcgccacttcgcgcatcgacgggctgtggtggcgcccgccggcgtaggtcacgcggccttcggccaccgccagcgggccgtgctgcgcgcgaacctgggcctcgatgtcctcgacgatgcgcagtgcctcgtcggcgcggccgtgcgccatcagccagcgcgggctttcgggcacgtcgcgccgcaccagcaggatggccacggccagcaccgcacccagcgcgaagcccgcgcgccagccccacaccggcccgatcacgcgcgcatcgagcagcaccaggctgagcccggcgcccagcgccgcgccgatccagaagctgccgttgatcgccaggttgacgcggccgcgcacacgcgccggaatgagctcgtcgatggcggagttgatggccgcgtattcgccgccgatgcccaggcccgtgacgaagcggcagaacgcgaagaaggcgaagttcggcgagaacgcggtggccagcgtgcccagggtgtagaccaccagcgtgaccaggaacagcttcttgcgcccgagccggtcggtcaggcgtccgaagagcagggcgccgatgactgcgcccgcgatgtagatcgaacccgaccagccgatctctccggcgctgagccccagcgtgtcgggccgctcgagcacggcgccgatcgagccgaccagcgtcacctcgaggccgtcgagcacccaggccacgcccagggcgatcaccacgcgccagtgccagcgagaccagggcaggcggtcgagacgggcaggaatgtcgctgtgcaccgcagctgtcgtcatgggctcaaccttaacccaagtgcctggatggccctttcagcggctgtgcttcttctcgcgcggaaaggtccaccagggcagcagggcgcgcagcgactgcacctcgccgctggccgcggtttcgtagccgggcagcgtgcccagcaggtgctgccaggtctcgctgcgcagtacggccaccagcgcctgcattgccggctgctcgagtgccgacttgaggcaggcgaggtggtagcgctcgtgcaccaggggcacgaagcccaaccccacggcgtgggccgccgattcgagcccgagcccggcatcggcctggcccgacgccacggcctgcgccaccgcggcatgcgaggtttcagagcgttcgtagcccgcgagcgcggtggcatcgagcccggcctgcgccagcagttcctcgagcagcacgcgcgtgccggtgccgatcgcgcggttgacgtagcgcgcccgcagccgtgccacgtcggccagcgagtgcaggcgcagcgggttgcccggcgccacgatgaggccctgcgttcttcgcgcaaagccgatgagcttgtgctgcccgggcttgagcagcggctggtaggtgcgctgggccagcgagccgcgctgcggatgttccagcgtatgaaagcccgccatcacgcagcggccctggttgagcgcgcggatcgcatccacgctgccggtgaaatgaatgtcgaggtgcagctgcgcggtgcccgcggcatgggtgcgcagcagtgccagcgcatcgtcgtggcttgcctgcaggctcagcacgtgggtgcgatcgtcgaaggcgagggcgaaggcgcgttccagctcggcgtgcagcgcctcgatctgcggcgccagccgggcctgcgcctggcgctcggcccacagcagcttgtcgccgaattcggaaagctgcgcgcgttgtccctgctcgccctgtatcagcgggtggccgagcgtctgttcccagtgcttgagctcgccccacacatggcggtaggacaagccgagcgcgcgcgcggcggccgagatggagccgtgctcgcgcaccgcctgcagcatctgcatcagcggattgcggatctgccgcgaaccgctgcggcggggacggatcgcgtaggaaaggtcgatctgatgcacggggctggcgggaggggaatggaggccggcagattatgcagaccgctgtgtcccgggcccagtccagtgcacccgcggaaccggctttgccgggccgccgggtgcgcccccagtgggggaggcgccgaaggcgcttcgggggcgtttgtttacgcggtttccgcgagcgcgtcgcccaaggcgttgatgaggcggtcgatctcagccttctcggtgatgaatggcggcgcgatctggatcgtgtcgccgccgtagcgcacgtagaagcccttcttccagcagttcatcgcaatctcgtacgggcggcgtgccggttcgcccggcagagcggcgatggtgatgccggcagccaggccgtagttgcggatgtcggtgacgtgcttgctgcccttgaggctgtgcaccgcgttctcgaaatgcggcgcaagcgttttcacgcggccgatcatgtcttccttctgcagcacgtcgagcgccgcaatgccggccgcgcaggccaccgggtgtgcgccgtaggtgtagccgtgcggaaactcgagcatgtagtcggggccgcctgccgccatgaaggtgtcgtagatctccttgctggcaaccaccgcgcccatcggctgcgcgccgttggtcacctgcttggcgatgttcatgatgtcgggtgtcacgccgaaggcctcggcgcccgtgagcgccccgcagcggccgaaaccggtgatcacctcgtcaaagatcaggaggatgttgttcgcggtgcagatgtcgcgcagccgcttcaggtagcccttgggcggaatcaccacgccggccgaacccgcgaagggctccacgatcacggccgcgatgttcgatgcatcgtggagcgtgatcaggtcgagcaggcggtcggccagttcggcgccgttttccgacatgccgcgcgtgaaggcgttggccgcaatctgcgtgtgcggcaggtggtcggcttccacgccctggccgaagagcttgcggttggccgcgatgccgcccaccgagatgccgccgaagttgacgccgtggtagcccttctcgcggccgatcaggcgcgtcttgctggcgaggcccttggtgcgccagtaggcgcgcgccatcttgagcgaggtgtcggcggcttcggagcccgagccggtgaagaacacgtagtccaggcccgcgggcgtgagttccttgatcttgttggccagttcgaaagagagcgggtggccgaactggaaggccggcgagtagtcgagcttggcgatctggcggctcaccgcctcggtgatttcggggcggccgtggccgaggcccgagcaccagaggcccgagaggccgtcgaagatcttgcggccgtcgccatcggtgaagtaggcgcccttggcctccacgatcatgcgcggatcggccttgaagttgcgattgccggtgtagggcatccagtgcgcgtcgagccaggcggcgtcggtgcgcagggcgggcgtcggttcgatggcgggtgtggcaagggtcatggcgcttcccgctcggggcgggctccaaaggggtaatgaggtatgcggattgttggcacagccgtcagtgtggagaatggcgcaatatcaatgttcacttgacacttcatgcaagtaaaggccaagacccgaagcgacgtccaaaacggtgcgtcaagcacgcgcaaccgcgccgtgctggggcagctcagcgacatggacctgcgcctgctcaaggtgttcaagagtgtggtcgactgcggcggcatggcggcggccgagctggagctgaacatcggcacctccaccgtgagccggcacgtgaaagacctggaaacgcggctcggcctggtgctgtgccggcgcggccgggcgggctttgcgctcacggccgaaggccagcgcgtgtacgacgagacgctgcggctgctggcttcggtggatgcgtttcgcggcagcatcgacgacatccacaaccgcatgggcgggcagctggaggtggcgctgttcgacaagacggccaccaaccccaaggcgcgcatcggcgaggccattgcgcgcttcacggagatcgcacccgaggtgaacctggcggtgcacgtgggctcgatcaattcgatagaacagggtgtgctggagggcaacttccagatcggcatcattccggcgcaccgcgcgtcgaagagcctggtgtatgcggacctgttcgacgagacgatgctgctttactgcggcgcggggcatccgctcttcggcagcaacaacgcaaagctcacatgggcaaagctgcgcgagcatcacttcgcgggcctgggctaccactcgcccaacatggaactgagccatcgggccaagctgtcgcgcaaggccacggggttcgaccaggaggcgattgccacgctgattctgtcggggcgattcctgggatttttgccggaccactatgcgcaggtgttcgaggagcgtgggctgatgaaggcggtgttgccagcgcgattcaactatgtgtgccgattcgtgagcctgctgcgaaggtcgccgaagccttcacgggctgtgttggcgtttcaggagtgtctggagaaggcgcacaagtaaagcttgtgcgcgacctcggtcttgctccctctcccgcttgcgggagagggctggggtgagggggtcggcgatggcaaagggcgtgcgggtgcgaaggcccgcggccctcaccctaaccctctccccagggggagaggggacaagaaaaacgggttgctctcaactcggccggtcaacgctgcccgctaggcagcaacagatgcttggccccgatatgcgcctccatctcatgcatgtgcgcctcggcatcgaccatgtgctcggccatcaggcggcgcacggtgtcggcgtcttctcggcgataggcatcgagcaactgggtgtgatagtcgacgttggcctcgccgaagtggtgatggtccagcgccttcttgtagacgacgaggtcgcgcagcaggtcgttgagaaagcggcacatgaaggacagcaccggattggggcaggcctcggccagcatggtgtgaaacgcgagctcggcctcgcgctggctgcgcagctcgtcttcggtggtgggctctattgtgcaaaggcgcacgttggcttcgagccgctcgaagtgttcgggcgtgagccggccgaccacgctcacggccaattcgggctccagcaccttgcgcagctggtagatgtggtggccgtccaggtgatgaaagtgcaggaagttgcgcagcggctccgatgcgtggtcgaccgacacctgctgtagataggcgccgccgcccggaccggtgcggatggaaatcagcccgcgcacctcgagcgccttcagtgcctcgcgcaccgtgctcttcgaataaccgaacagctcgatcaattccttctcgttcggcagccggtcgcccggctgcttgcgctcggcaacgatccagcgcttgacgtcctcgacgatgacatcggagagcttttgccgtttggggcggttttgcccaaagctcatggcgtcctgcggcgatttcatgcgtgaagagtcatttcgagagtgatgagggtacttgggagcagatatcgggcccgacctttccggattttggcacggccattgctagcgggtttttaccaacatattaatcctatttatccgcttaaattcgctgccgaccccaggccgcacttttctcttactcccaaccacgtccggagaattccatgcaacgcagacaccttcttcagctcgccgccctgtcggccgctcccgtttcgctcctgggcggccgcgccgcctttgcccagtcggccgacgcgatccgcttcggctgcccggttccgatgtcgggcgccttcgcggccaacggcaagttcgccgacctgggcatgaagctggccatcgagcaatacggcagcgtgctgaagcgcccgctggcctacacggtgctggacaccgagggcaagccggccaccgccgtgcgcaaggtgcaggaagcctcgcagcagcagggcgccaggttcttcgcgggcggcatcctgtcgtccgaagcgctggccatgggcaaggaggccgagaaggccggcggcatcttcatcaccaccgcgggtgcggacgagatcacgggcaaggactgcaaccccgccaccttccgctggtcggtgcccaccttcggcgccgtcgagcagacggtgcgcccgctgatcgccaccatgcccaaggccaagcgctggtacaccatcacgccgcagtacgttttcggcgaaggcctcttgggcgcggccaagaacatcttccaggagaagggcatcgagcacgtgggcaacagctaccactcgctcaacgagaaggagttcagcggctacctcaccaacgccatggccgccaagcccgacgtgctgctgctcctgaacttcggcgcgcagtcgtcggcggcgctgcgccaggcggtgagcttcggcatgcacaagaacatgaccatcctcattgcctgggcctcggggctggagcagttcgacgaactgggcgccgacctgtgcgacggcgtctacttcggtgcgcagtactggcacacggccgacaccacgctgaacaaggacctggtgaagctcacagccgacaagctgaagatcgttcccaactacagcctcgcaggctcgtacgtctgcaccaagatcctcatcgacggcatcgtcaaggccggcaccgtcgaccagaaggccgtgattgcggcgctcgaagggatgaagtacgaaggcctcacgggcgccgaggaaatccgcaaggccgaccaccaggtcatcaaggactactacctgctcaagggcaaggccaagtcgaagatgaagagcgcggccgactatgtggacgtggtgagttccggcaagtccttccttgcagtggacaagaccggctgcaagctggcctgagcacgccgacaaggaatccggcgcacccatccatgaccgtctacctgctccagaccatcaacggaatcggcatcggcatgctgtatttcctgctggccgttggcttgtccatcgtgttcggcctgctgcgcttcgtgaattttgcgcacggggctttctatctgctgggcgcgtacctgtgcttccaggccatgcagtgggggctcgacttctgggccgcactggtgctggtgccgcttctcgtgggcgggctgggctggctcgcggagaagctgctgctgcgccgcgtatacgccaaggcgcacgagttccacatcctcgtgaccgtggggctcgcgctcgcggtgcaagagatcgtcatcgtgttctgggggccgctgggcaacagcgtggcgacccccgacctgctgcagggcgtggtgatgtggggcagcttcatctatcccaagtaccgcctgttcgtgatcggctttacggccgtgctcgcggtgctgctgtggtgggtgctcgaaggcacgcgcctgggcagcgcggtgcgcgcgggcagcgaatcgacggagatggtgtcgctgctcggcatcaacgtcttccgtgtgttcagcctggtgttcgcactgggtgcggccacggcggcgctggcaggtgtgctggcggcgccgatccgcggggccgagcctttcatgggcgtcgaggcactcggcgtcgccttcgtggtggtggtgattggcgggctcggcagttttggcggcgcgctggtcggcggcttgctgatcggcatcgtgcaaagcctcatgagcaccatctggccgccgggggcgagtttgatgatctacatcgcgatggcggccgtactgctgctgcgcccgcatggcctgcttggccggagcacatgaaaaaacaccccatgccaagaaaaatcactttcctcctggcgctgatcgtcgcgctgggcctgccgctggtgctgcgctcgggttcgctcgcgagcgaggtgctcatctacgcacttgctgcgctgggctgcaacctgctgctgggctacacggggcttctttcgttcgggcaaggcatcttcttcggcctcggcagctacaccatcgcgatcctgctcacgcgtttgcagctgccgatgccgctcgcgctgctcgccgccatcgccatgggcgcactgggcgcggcggtggtcggttgggtcgccatccgccagcgcggcacctacttcgtgatgctcacgctggccttcgcgcagatgttctatttcgtcgcgtacaccgcttcggggctcacgggcggggacaacgggctgctcgacgtgccgcgccccgccttcatggacacgccctggaagtactacgccttcgtggccgtgatgttcctcatcgcgttcggcctgttgctgcgcgtgaccgattcggtgttcggccgcacgctgctcgccattcgcgacaacgaggaccgcgccgccgcggtgggctacaacctcaagcgcttcaagctgctggccttcgtgatttccggcgccgtcaccggcctagccggcggcctgcacgcgatgatgaccggcatcgcgccactgtcgaatgccgagtaccacacgagcgaaatgatcctggtcatcaccgtgatcggcggcaccgggaacctgttcgcctcggtgctgggctcggctttctacgtgctgctggccgactggctttccacgctgtggccgcgatggctgctgctgttggggctgttgctgatcggcgtgagcatcggtatgcagcgcggcctctggggcctgggcgaaagcgcgtggcgccgcgtgttccgcaaggcgccgcctttagcgccggccgtgcctcacgtgcatggagaaaaagcatgacccaaccggtactcatcgaagccatcggcgtcaccaagcactacggcaagttcgccgcactcggcggggtcgacctgaagatcaagcgcaacaccgtgcactcggtgatcggccccaacggcgccggcaagaccacgctgttccacatgctcacgggcaccggcaccaccaccggcggccgcatcttgttcgacggccacgacgtgacgcacgagcccgaccacaagcgcgtgcagcgcggcatggcgcgctcgtttcaggtgaccagcctgttcgccagcctttcggtgcgcgagaacctgcgcgtggcggcgcaaggcgttgcgccgcgccaggccatgaactgctggcgcgcgccggtcggcgaacgagcctgcgccgaaacggtggccgaggtgctggagcgagtgggcctccagcggctggccgacgtgcccgccagcgaactctcgcatggccagcaacgccgcctcgaagtgggcatggcgctcgccgcgaaacccaaggccatcttcctggacgaaccgacctcgggcatgggcatcgacgacctggacgacatgaagcggctgattcgcgggctgcgcgacgcgcacaccgtggttctcatcgagcacaacatgaacatcgtgatggacatttccgacaccgtgacggtgatgcagctgggccgcgtgctggccgaggggctgccgggcgacatccgctcggatgcgcgcgtgcgcacggcgtacctgggcaacatgatcaccggaggcaaggcatgaggagcactgcttctttctccctctccccttggggagagggcaggggtgagggccgcggccttcgcacatgcaccgcctttgccatcgccgccggccctcaccccagccctctccccgaggggagagggggcaacagccgggccatgaccggctcggagagaacggaggcgccccgatgagcgcgaacatcctcgaagtcggcggcctgcacgcgcactacggcaagagccacgtgctgcagggcgtgtcgatgacggtgggcgaggccgaactcgtcacgctgctgggccgcaacggcgcgggcaagtcgaccacgctcaagagcattgccggcgcggtcacgcccagcggcggccgtgtgcgcttccagggtgcggacatcgcgggcctgccaccgcaccgcattgccacgcgcggcgtgtgcctggtgcccgaacaccggggcgtcttcaagctgctgacggtggaagagaacctcctgctcggccagcggcgcgactcaccctggcagctcgacgacatctaccgcatctttccgcgcctgaaggagcggcgccgcaatggcggcggccagctttcgggcggcgagcagcagatgctggcgattggccgcgcgctgatgaaccatccgcgattgctgattctcgacgagccggtcgaaggccttgcaccggtgatcgtggaggaaatcgttgcgcagttgaagctcatcaaggcggccggcgtggccatcctgctggtggagcagaacctcgaagtctgcgtgcaactcgccgaccgccactacatcctggagcagggcgtgatcgtgcacgaggccggcaacgccgccttcatggccgaccatgaagtgaaagaccgttatctgggcgtgggccttgcttgaggcctcgcataccttcttctttttgcaaagccatgaactcacagaccccactccgcatcaacggcgagcgcctctggaactcgctgatggaactggcgaagctcggcgcgaccgagaagggcggcgtctgccgcatcgcactgaccgacctcgaccgccagggccgcgacctcttcacccgctgggcgcgtgaagctggctgcgaggtgcgcgtcgaccagatcggcaacatctttgcgcgccgcgccggccgtgacaacgcgctgcccccggtcgttacgggcagccatatcgacacccagcccacgggcggcaagttcgacggcaactacggcgtgctggccgggcttgaggtgatccgcagcctgaacgacgcgaacgtcgtcaccgaggcgccgctggagatcgccgtgtggaccaacgaagagggctcgcgcttcgtgcccgtgatgatgggctctggcgtgttcgccgatgccttcacgctcgaacatgcgctggcgcagcgcgacaacgacggcatcagcgtggccgaggcgctcgcgtcgatcggctatgcgggcgccgcgccggcttcggccgaggcatcgcccgtgggcgcgtatttcgaggcgcacatcgaacagggcccggtgctcgaagccaacgagcgggtcatcggcgtggtcgagggagcgcttggccagcgctggtacgacgtggtgctgcagggcatggaagcgcatgccggccccacgccgatggagctgcgcaaggacgcgctgctcgcggcatccgaactggtgatggaggtcaaccgcatcgcgctggcccacgcgccgcatggccgcggcacggtcggctggatcgaaaactatcccaattcgcgcaacgtgattccgggccgcgtgaagctcagcgtcgacctgcgcgcggcggacgacgtggtgctttcggccatggacgccgagctgaaagcgctggtgcagcgcatcgccgtcaagggcaaggtcgaggccacggtggagcaggtcgtctactttccgccgcagcccttcacgcccacgctggtgtcggccgtgcgcgaggccgcacaggcgcagggcatgacctggatgaacgtgatcagcggtgcggggcacgacgccgtttaccttgcgcgcgtgtgccccgcggcgatgatcttcgtgccctgcctggacggcatcagccacaacgagatcgaggacgcgcagcccggccacctggaggcgggatgcaatgtgctgctgcaggcgatgctgcaaagcgcagggggggcagtgtgaaggcggcgctccggagcatccgccttcgcatcctcgcggcaggcatcgcggtggcagccactgtcactgctgctgtggccgcggaaccccccatcctggtgggtcagtccgccgtactgaccgggccgctcacgcccaacagcctggcgttcatggaaggccagacgctgtttttcgaccagttgaacaaggccggcggcatcggcgggcggcccgtgaaggtgattacctacgacgatgcctatgtggcggagaaggccgcggccaatgcggagaagctgctcggcaccgaccgtgtcgtctgtctcttcggcgccatgggcacgggtatcggcgccgccatggtgcctgtcgcggccaagtacgacagcttcatcttcggcggactgaccggcgcggccgtgctgcgcggcccgaaggtaccgatctatcacatgcgcgagtcgtatgccgacgaagtccggcgcgtgatgacccacctgacgaccatcggcgtgacgcgcatcgccatcgtctcgagcgacgatgcctacggcaagggcatcgagaaagacgcggtggaggcgctcgagaagaacaagcatccggcgctcctctcgctgcgcttcaatcccaaggacgcggatctttccgccatcgcgcaacatgtcaccgcgagcggggcgcaggcggtctacgtcattgcggccggcatgccggcgatcaacgtcatccgggcgctggtggccgcgccggtgcacccgcagatctacaccaactccgtggcgagctccttcctcctgtacaaggaactcggcgagcgaagccgcggcatcgtgctgtcgcaggttgtgccgccgttctggaagacccggtttcccatcgtcgacgagtaccagcgcgcgatcaagagcgcgggcggcggcggcgaaggctcctacctgggcctggagggctacatcacggccaaggccttcgcggaagcgctgcagcgcgtcaaggggccgatcaccaccgaatcgctgaagcgcagcatcgagaactcgccgcccatgaacctgagcggcttccaggtcgctttccggcccgacaaccggaacggctcgagcttcggggacatcacgatgctgggaagcggcggaaagtttgcgcaatgaaagtgctgatcgcgcggctcaaccacgagaccaacaccttctctccggtgcccacgccgctggcggccttcgggcccgacggccccacgttcggagaacaggcctacagggacaacaagggcatgcgcaccgccatgtcggccttcatcgacctggccgagctggcgggcgcgacgctggtcacgcccgtgtcggcctcggccaacccgagcgggccggtcgacgcagcggcgtacaccacgcttacccaatgcatcgtcgatgcggcgccgggctgcgatgccatcctgctcgacctgcacggcgccatggtggcgcagaacagcgcggacggggaaggcgacctgctggtgcggctgcgtgccgcggcgccgggcgtgcccatcggcgtggcgctggacctgcacgccaacgtcacgcccgagatggtcggcaacgcggacgtgatcgtcggcttcaagacctatccgcacatcgacatgtacgaaaccggcgagcatgccggccgcctgctgttcgacttgctcgcgggacgcagcaagcccgcgatgcgctggcacccgctgccgttgatggcgcacacgctgcgcagcgcgtctttcaccggcgcgatgcagcgggccatcgaggctgcacgcaaagccgaagcatcggaatcgctcgcggtgtccatctttgccggcttctcgctgtccgacatcgaggcgccctgcatgagcgtggtggttgtcgatgcgaagttgcacgagcgcgcgcaggccacggccgaccgcatcgcgaagcagatgtgggacgagcgcgaggctttcgtctaccgcagcgagccgcttgccgaatcggtggcgcgtgccaaggccattgcccagggcgcgacgcgtccggtgctgctgctcgaccatggcgacaactgcatgtccggcggcagctgcgacaccatggacgtgctgcaggaggccctggcgcaggggctcgacggcatcggcgtggggccgctgtgcgaccccgaggccgtgggcgaactcatcgcggcgggcgagggcgccacggtcacggtggcgctgggcaacaaggtgtcgctcgaaggcatcggcttgtcgaagaagcccgtcatgctgaccgggacggtgcgcaccgtcggcaacggcgagtacgtgatcaccggtcccacctacaccgggcagcgcagcagcatgggccgcacggtgctgttcgacatcggcgcggcgcgcatcgtggtgaccgagcgcacgcaggagccctgggacatcggtgttttcgaatgcgcggggctcgacccgcagaaggaacgcttcctgctgctcaagtcgcgcatgtactgccggccggtgttcgagccgatctcggccgcgctgatcgagtgcgacagcccgggcgtaaccagttccgactacagcctgttcccgttctccaaggtgcgccggccggtgtttccgctcgacatggtctgatcggcgcgagcagtatggctacctatgcaaaaaattgcataggtaattggaagtacaccgcgatactgcggcgcttccatccatgagacccagcgcgtgaacacctttgcacagagcggcgtcgcggcctggcagctgctcgtgtcgggcgatccggtgctgctggccatcgtcgggcggtcgctcgcggtcagcgccagcgcctgcgtgctggcctgcgggctgggcctgctgctgggggcgtggctgggcgtggcgcgctttcgcggccgtgccggcttgctcacgctgctgaacaccctgttggccctgccgtcggtggtggtcggactggtggtctacctcctgctgtcgcgctccgggccgctcggctttctgggctggcttttttcgttcaaggccatggtgctggcgcagacggtgctggtgctgccggtggtgacggcgctcacgcgccaggccatcgaggatgccgagcgtgcgcacggcgagcaactgcgctccctcggcgccgggccgctgatgcgggcgctgctcctggtgtgggacgagcgctatgcgctgctcacggtgctcatcgcagccttcggccgcgcggtgtcggaagtgggcgcggtgatggtggtgggcggcaacatcgacggcttcacgcgcgtgatgaccaccgccattgcactcgaaaccagcaagggcgacctgccgctggcgctggccctgggcatcgtgttgctgggcgtggtgctggtgctcaaccttgccattgccgcggtccgcggctggcgcgagcgggtcgatggcgggggcggcgaaggcggcggcatggcggcctggtggcggcccgaggtgcgcccatgaacgaacacgtgcaactggcgagcgacgacaccacggtctttgcgctgtacggcgtcgacgtccggctgggacgcgtggcggccctgcagggcgcgaccctgaccattgcggccggcgagcgcgtggcgctgatcggcgccaacggcagcggcaagaccacgctgctgcggctgctgcatggcctggtgccgcatgcggcggggagtttcaccagcgccgcgccgggccgccaccaggccatgctgttccagcgcccgcacatgctgcgcgcgtcggtggcggtcaacgtggcggtggcgctgtggctgcgtggcatgcgctggcgcgatgcccgccgcgccgccattccggcgctggcacgcgtggggctcgaagacttggcaaatcgcaatgcccgtgccttgtcgggcggccagcagcagcgggtggcgctggcacgcgcctgggcgctgcatccggcggtgctgctgctcgacgagcccaccgccagccttgaccctactgccaagcgcgaggtcgagtcgctcatcgccgaagccgccgcgggccgcacgctggtgttcgcgagtcacaacctcgggcaggtgaagcggctggccagccgcgtggtctacctcgagcacggccgcgtgctggccgatctgcccgtgcacgagttctttcatgggccgctgcccgaagaggcccacctgttcgtcaaaggagagttggcatgagtctgtctttcaagcaccgcggcaatgcgggcatccgcgcctcgctggcggtggcggttttcttcctggccgcgggcatcgtgcgggccgagaccatcaccatggcctcgaccacgtccaccgagcaatcgggcctgttttcgcacctgctgccggccttcaagaaggccagcgacatcgacgtcaaggtggtggcggtgggcaccggccaggccattgacatggccaagcgcggcgatgccgacgtgctgttcgtgcacgacaccacggccgaggagaggttcgtggccgaaggcttcagcgccaggcgctacccggtgatgtacaacgacttcgtgctggtggggccgaaggccgacccggtggcggcgaagggcaaggacatcgttgccgggctgaagaagatcgcaaccgccaacgcgcctttcgtctcgcgcggcgacaagagcggcacggacgcggccgagcgccgactctggacgcagaccggcgtgggcgaggcggggcagccggtgcccaacgaccgcaagggcacgggctacaaggaatgcggctgcggcatggggccggcgctgaacatcgcggcctcgtccggcgcgtatgtgctggcggaccgcggcacctggctcagcttcaagaaccgcgccgacctggcagtgctggtcgagggcgacaagcggctcttcaaccagtatggcgtgatggtcgtgagcccggcgaaatttccctcgctcaacagcaagggcgcgcagaagttcgtcgactgggtgatctctccggccggacagcaaaccatcgcggactacaagatcggcggcgagcagctgttctttcccaacgcgctgggcaactgaattgcgcagcggcggcggccgcgctccatgacctgcgaggtcatcgacgccgcgcgcacccggcgcgaccattccttcaccccgcgatgttgcgggccccactcttgaaggaatcgtcatcatgaacatcgccgcacacgacgccgccgccattgcccagcgctacatcgccgtctggaacgaaaccgacgccgcgcgccgggccgcgctgatcgaggctcactggacggccgacgcacgctacgtcgatcccttggcgcaggccagcggccgcgagcagatcagcgcgctggtcggcgccgtgcagcagcgctatccgggttttcgcttcagcctgttcggcaaggccgaggcgcacggcgacaacctgcgcttctcatggaccttgggcccgagcggtgccgaagacttgatccagggcaccgacttcgcccggctcgatgcgggcaagctgcaatcggtgaccggctttctcgacaaggtgccggtgggcgcctgaaggcttcagtccgccgatccggaggcccggccgcgccagagcttgcggtagaccgtggcgcggctgatgccgagggtgcgcgcggcttcggccacgttgccgcgggcgtcggtcacggccttgcggatgagcgcggtctcgaggtcgcgcagccgcggctgtcgggcttcggttgccgcgcccggcgaaaccttgccgccgcgccggggccgcacctcgatgcgcaagcccgaccagagcggcgcctcgagcacggcgtcgccgcgccgggcggcatcgaacagcatgctcagtggcagcgcgaacaggtcgttgcagtgcaggccatgcgggctgcgcgttgccaggggctggtgcagcatttgccgcgctgcagcattggcgcccgtgaccttgccgcccgcgtcgatgcacagcaggccctcggtggcgtcgttgcccgggggacagccgggccatgagagatgcagccgcagttcgcatggcgtgttcagcaccagcatgttctcgatgctgcgcgccgacagcgtggccaggtgacgcagctcgggccgctcgaccacctggacgccggtcaggtcgagcatgccgatgcagtcgccttgcgggccgaagagcggcgcgccggcgcaactgtagacgctggtgtcctcgaagaaatgctcgccgcggtgcagccacaccgattcctgctcggtcagcgcggtgctgatggcgctggtgccgatggcgcgctccgacaggtcgacgcctacccgggcgatgttgcgcgcatagcggctggcggcgtcggtgccatcgggcagggggcccacgtcgaccacgatgccggcggcgtcggtcagtacggcgaaatactgcgtgtcggcaatggcgcgggacagccgctcgatcaccggccgggccgccaccactagcgcccggttgcgctcggccacgtcgcgcacggccgacctccccacgggttcgaaggccacgcgctgctgcggctgccgcccggcttcgaggcaacgctcccaggagcgggcgatccatggctcgatgcgcacgctgcttcgggagcgcgagccttcaccatgaatcagctcccggcgggcctgcgcaatggcgagcgagcgctcgggcgggggcagaacgggggaggcgggcatcgggtcagggggctcggacgggaggtctttttgttgaaacttgcgggtcggcaagttgtttcattttgagaatttcgcgacggctgcgcaagcggcgagggttttgcctaggatagtgcacgggaccggcatccaagatgccattcgctgaaccagccatcaccttcaacggagacagccaaatgcaggtagctttcacggtcaacggccgaccggccacggtcgacgcaccccccaatactttcctggtgcacgccatccgcgagcatcttcatctcaccggcacccacgtgggctgcgacaccgcccagtgcggcgcatgcaccgttcacctgaacggccgcgcggtcaaatcgtgcaacatactcgtggggcaggtggccggtgcgcaaatcaccaccatcgagggcgtcgcccagcccgacggcaccatgcaccccatgcaagcggccttcaaggagtgccacggcctgcagtgtggtttctgcacccccggcatggtcatgagcgccatcgacctgtgcacccaccatcccaagtcgagcgaagccgagattcgcgagctgctcgacggcaacctgtgccgatgcacgggctaccagaacatcgtcaaggccgtgaagatgggcggcgaggccatggcctcgggcaccccggtcaagaccacggccaccgtttaagggagccacatcatgggtgcctccgacttctcgaacctgccccacatcggcgaagcgctgcggcgcaaggaagactaccgcttcctgaccggcgcgggcaactacaccgacgacatcacgctggccaatcagagccatgcggtcttcgtgcgctcgccgcacgcccacgcggtcatcaagtcggtcgacattgccgaggcgctcaagatgcccggcgtggtcggcatcttcagcggcaaggacatcgagggcaagatgggcgggctgccttgcggctggctcatcaacaaccccgacggcacccccatgaaggagccgatgcacccgatccttgcgatcaacaaggtgcgctacgtgggcgaccacgtggccatggtggtggccgagacggtcgaacaggccaagaacgccgccgaggccgtggtggtcgactacgacgtgctgcccgccctggtgagcgtggccgacgtggcaaagaaagccagcggcgtcacgctgcacgatgaagcgcccgacaaccagtgctacaagtgggcgctgggcgacaaggctgcggtcgatgcggtgttcaccatggccgcgcacgtcaccaagctcgacctggtcaacaaccggctgattcccaacccgatcgagccgcgcgtggccatcggcagctacgcccgcggcaccgacgactacaccctctatgtgtccaaccagaacccgcacgtcgagcgcctgctgatgacggcctttgtgctgggcctgcccgagcacaaggtgcgcgtgatcgcgcccgacgtgggcggcggcttcggctccaagatcttcctgtacgccgaagacgtgtgcctgacctgggccgccaagcagctcaaccgcaacatcaagtggacggcggagcgctcggagtgcttcctgtccgacgcgcatggccgcgaccacgtgagccatgccgagatggcgctggacaaggacggcaagttcctcgcgatgcgggtgcacaccgacgccaacctgggcgcctacttgtcgacctttgcgaccgcggtacccaccatcctctacgccacgctgctcgcgggccagtacaccacgccgcagatctacgtcgaggtcgatgcctggttcaccaacaccgcgccggtcgatgcctatcgcggcgccgggcggcccgaggccacctacctgctggagcgcctggtctcgcgctgcgcctgggaaatgaacctgggccaggacgagatccgcaagcgcaacttcatcagcacctttccgtaccagacgccggtggcgctgcagtacgacaccggcgacttccatgcctgcatggacaaggcccgggtgctcgccgatgtcgggggctacgcccagcgcaagtcggccagcgaggcccagggcaagctgcgcggcatcggctactcgagctatatcgaggcctgcggcatcgcgccgtcgaacatcgcgggggcgctgggcgcgcgcgcgggcttgttcgaatgcggcgaaatccgcgtgcacccgaccggcagcgtgacggtgttcaccggctcgcacagccacggccagggccacgagaccacctttgcgcaggtggtggcggcgcggctgggcattccggtcgacaacgtcgacgtggtgcatggcgacacgggccgcgtgcccttcggcatgggcacctacggctcgcgttcgatctcggtcggcggcgcggccatcatgaaggcgctcgacaagatcgagaccaaggccaagaagattgccgcgcacctgatggaggcgagcgacgccgacatcgagtttgcgaacggcgaattcacggtcaagggcaccgacaggaagatcccgttcggccaggtggcgctcacggcctacgtgccgcacaactatccgctcgacaagctcgagcccggcctgaacgaaaccgccttctacgacccgacgaacttcaccttcccgggcggcacctacatctgcgaggtcgaggtcgacaaagagaccggcgaggtccgggtcgaccgcttcaccgcggtggacgacttcggcaccatcatcaacccgatgatcgtcgagggccaggtgcacggcggcctggtgcagggcatcggccaggcgctgctcgaaaactgcgtctacgacaacgagaccggccagctgctcaccggcagcttcatggactacgccatgcccagggccgcagattttccgcagttcaatctcgacaccgtgtgcacgccgtgcacgcacaacccgctcggcaccaagggctgcggcgaggcgggcgccatcggttcgccgccagccgtgatcaatgccgtgctcgacgcgctcgcgccgctcggcgtcaaggatctcgacatgcccgcatcggccagccgcgtctgggaggcgatgcaaaagggcagcggaagcgcggcgcaagctgcgccaccgcaagcgccctcgctcgccgccagcacccaaggccgtcccgccccctgaacctggaaggaaccacacaccatgtacgccttcacactcgaacggccctccaccgtggccgatgccgccaagctggtcaccgccggcgccaagccgctggccggcggccagactctgctcgcctccatgaagctcaggctgtccgcgcccgagcgactggtggaccttggcggcatcaaggaactcaccggcatcaagaaagacggcagcgcaatcaccatcggtgccatgtcgagccacctcgacgtggccaacaaccccgacgtgaaagccgccttccccgcgctggccgacctggcctcgcgcatcggcgaccggcaggtgcgcgcgatgggcaccatcggcggctccgtggccaacaacgacccggccgcgtgctatcccagcgcggtgctgggttccggtgccaccgtcatcacctcgaggcgcgagatcgcggccgacgatttcttccttggcctcttcaccacggcgctggaagaagacgagttgatcaccgcgatccgctttccgattcccaagcgcgccgtgtatgaaaagctgcgccagaaggcgtcgaactttccgctcgtcggcgtgttcctcgcgcagtacgacagcggcgtgcgggtggccatcaccggcgccggcaacggcgtgttccgccacgccgagctggaagatgcgctcaacaagagcttcacggcggcagccgcggcggccgtgaagatcgatgcgagcgacctcaacagcgacctgcatgcatcggccgcctaccgtgccaacctgatcagcgtgctgacgcagcgcgcggtgaccaaggcgctgggctgaagcagccgggcgctgattcggaaggcgcgacatcctcgcgtcttccgctacgctttgccatgatcttcccgaccatcgattcccttgccggcggtttgatgcaggccggctacttcgccgaccggcgcctggccacggccgtgttcctcgcgctcaagctgcagcgcccgctgctgctcgagggcgagcctggcgtcggcaagaccgagctggccaaggcgctgtcggccgcgctgaaccgcgaactgctgcgcctgcagtgctacgacgggctggagcagcgcgaagcgctttatgaatggaactacgcggcgcagctgctccacatgcgcgccgcagaggcgaccggcgcggcacgcgacgtcgaagccgaggtctaccagccgcactacctgatccgccggccgctgctgcaggccctgcagacgcccgcgcccggcgccgtgctgctgatcgatgaagtggatcgcgccgacgaacccttcgaggccttcctgctcgaatacctcggcgaataccaggtcagcattcccgaactcggcaccgtgcgcgccgtggtgccgcccgtcaccatcctcaccagcaaccgcacgcgcgaactcaacgatgcggtcaagcggcgctgcctctatcactggctcgactaccctgagcgcgaacgcgagctggccatcgtgcgcgcgcaggtgccagaggcgggcgaaaagctctcggcccaggtggccgctttcgtcgcgcggctgcgcgatgcgcctttcgtcaacgcattccagcgcgcgcccggcatcgccgagagcgtcgaatgggcgagggcgctgattgcgctcgacaccgtcgagctcgaccccgaagtggtggtcgacaccgcgggcatcctgttcaagcagcgcgacgacgtggccgcactcacgcgtgaactggcgtcggacctgctgaagcccgaagagccggttgcgccctgagcgcggccgaaggtagcggccgcccatgaccggcatccagcaactcggcgacgtacgcagcggcaagctggccggcaacatcacggcctttggccgcgcgctgcgccgcgctggcgtgcgcaccgatgccatgcgaatctcgctcgccgccgaagcggccacgctggtgggcgtggagaacaagctcgacctgggcgccgcgatggaagccgtcatggtgagccgcgagcaggaccgcatggtgtttcgcgaactcttcgatgcctggtttcgcgaccccgaactggccaacaagctgcttgcgcagatgctgccgagcgcggagggcaaggccgagccctccaagcggcgcccgcgtgtgcgcgaggcgctcactgcgcctcgcgatccagcaaaaccggccgcgcaggccaagcccgacaaggaggtcgagttcgatgcggccatgacgtcgagcgatcgccatcgcctgcagcatgcggacttcaacgcgctcggtgcgtccgaataccgcctggtcgagcggctggcgcgcgacgtgaccttgcccatcccttcgctgccctcgcgccggctgcgcgtggcgggcgatgcggggcagcagcatgcgcgcatgcactggcccggcgtgctgcacgaggcggcgcgcacgggcggcgagatcctgcgcctgccgcggctggcccggcgcgagcagccgctgccgcttctggtgctggtcgacgtgtcgggctcgatggaacgctatgcgcggctgctgcttgcgtttctgcatgcatccacccggcgggccggccggcgtgatgtgttcgcgttcggcacccggctgaccgacctgacgcccgccttcaagttggccgataccgacgccatgctgggcgcggccagcctcgccatcgacgatttcgcgggcggcacgcggctcggcagttcgctggccgaactccgccgcgcccatgcccgccgcctgacgggccgccgcacgctggtgctggtgatcagcgacgggctcgacaccggcgagcccgcgctgctcgaaaacgagctgctctggctcaagcgccattcacgccgtctgctgtggctcaacccgctgctgcgcttcgagggctacgcccctttggcgcgtggggccagcgtgctgcaccgccatgcagacgcgatgctggcggtccacaatctcggtgctctcgaacagttggccaccagcctcgccgcgctcatgcgatccggccgctagcggctcacagaaaagacaaaaggaaactccaccatggaaatgctcggtaaccgccgcctcggcatctcgcaacaacaggcctgggaagcgctcaatgatcccgagacgctcaagaagtgcattcccggctgcgacaagttcgagctcacgggcgacaaccagtacagcgtggcgctggcggtcaagatcggtcccgtgtcggccaagttcaacggcaaggtggcgctgtcggacatcgtcgcgcccgacggctacaagctcaccttcgaggggcagggcggtgtggcggggtttgccaagggttcgtccagcgtgacgctcaggccgctggacggcgctgccgccgcgccgccggcaagcgacggtgccgaggccgtacctgcggcggccggctgcgaactcgactacaccgtgcaggcgcaggtcggcggcaagatcgcccagctgggccagcgcctcatcgacggcgccgccaagtccaccgccgacgatttcttcaagcgcttcgaggccgaaatgcaaagccgctacggcccgccgccggttgccgccgaagaaacagcggaggctcccgcggagaaggcgggcgtcatgtccggcttcatgaagaagatcggcctcggcaaaaaggacgacaaggatgcgtccgccgcatcggacgacgcaagctgaggacacggaacaaacacgccatggaaaatctcgacgtcatggtgctgcgcacgctacgcgactggcggcatgccggcaagcgcgcgctgctgaccacggtggtgcgcacctggggctcgtcgccgcggccgatcggctcgatcatggcgctggcggacgacggcgcggtggtgggctcggtctccggcggctgcatcgaggacgacctgatcgcccgctacagccacgcccacgcgaaaaacggccagggcgaagaggtgccgctgggcgcgccgcccgcgctggtgaaatacggcattacggccgacgaagcgcatcgcttcgggctcccctgcggcggcacgctggagctgctgctcgaatacgaccccgatgcggcctcgctcgacacgctggtggccgagctcgagcaaggcaagctgatgcagcgcacggtcacgctcgcgaccggcgccgcgcggctggccgaggcaaccgcgcccgacgcgctcaaggtgaacgacaccgagctcaccaacaccttcggccccgagtaccgcatgctgctgatcggcgcggggcaactggccgaatacctcgcgacgatggccaagttcagcggctttgccgtgacgctgtgcgatccgcgcgccgagtaccgcaccgcgtggtccctgccgggcgtggaaatcaccaccgagatgcccgacgacgcggtgctggccttcaagcccgaccggcgcagctgcgtggtcgcgctcacccacgatcccaagcttgacgacctggcgctgctcgaagccttgcagagcgaggccttctacgtgggcgccatcggctcgcgccgcaatgccgaggcgcggcgcgaccgcatgatcgagcacttcgaccagaccgctgaatcgctcgcgcgcttgcgtggacccatcggcatctacatcggcagcaagacgccgccggaaatcgcagtgagcgtgatggccgagattcttgcggtgaaaaacgcggtgacgctgccgcgcgaaatggaagtggcgcgcgccaagggcatgcagcagctcgcaatgagctgaatgaatcgccggcccggtgatgtcggccaggtcagtcggccgacttcgccgccggcggcacgtcgccgcctttttgccgttcgcgaaaaagcgcggcacgcatcaggaagatggtggtgatgggcgccgtgagcgcgatgaagagaacgatcagcacggcgtgcaggaacaggctgaagccctgcaccgagaaatagacgatggtggcgatcgtcatgcaccacacgcccaccgtggcaccgagcgtcggcgcatggatgcggcggaagaaggtgggcaggcgcacgaggccgaaggagccgatggccgcaaaggccgcgcccagaacggcgaacgcggcggtgacgatttccgcccacaggggcagcggccccacgatgaagtcgttcactcgatcacctccccgcgcaagagaaacttcgccatggcggtcgacccgacgaagccgaacagcgccgtgagcatggccgcctcgaagtacacgttgctcgcatagacgatgccgagcaccagcatcatcagcatgccgttgatgtagaggcagtccagcgccatcacgcggtcttgcgcgctcgggccgatcagcaggcgggcgagtgcgcagagcatggccacggccagcagcagcagcgcgagtttcaaggcccagaaaagcacaggcgtcatgattcgaagatctccatcaaggggtgctcgtagcgctctttgatcgtggcgatgaaagcggcttcgtcttcgacgtcgaacacatggatcagcagcgtactgctgtcgaacgagatttcgccccaggctgtgccgggcgtgaggcacatgatcatggccagcaccgcgagcccgttcgggtcgcgcagctcgagcggcacgttcacgaacttcgatgcgatgcgcgaggtgcggcgcgtgagcagccggcgcgccacgaagagcgcggaatgcagcatgtcggccgaggcccggcccgcgagccgcagcgcaacccagggcttgcgcatgcgaacggtggcgggccgcaggccctcggtgagcagcggaaccgcaatggccagcaccagcgcggatgccagcgtggcagcctccagcgactggttgagcaggagccacacggcgaacagcgcgatcgacagcggcggcgaaggaatccagcgcttcatggggcagggccttttgccggagccaccggattgggaacctgccgcgcattcatcactgcattgcgatacgccgcgggcgcgtgcagcccttcggcggtgatgagcgcgtggcgcatgacggggccggcccacaccgtcaatgccacgcaggccgcgagcagcccggccacgggcagcacctcgagcgcgggcagggcgggcatggtgggatgcggctgggtccagaagtggcgcatgccggtgcggctcagcgcaatcagcgccaggaagcccgaggcgatcagcagcgccaggaagatccatgccgccgtggaggtgccgctggtcacgaaggcacccgacagcatcgcgaacttgcccacgaagcccgagagcggcggcaggcccgcgagcaacaaggtgcagcctatgaagctcaggcccaggaacgccacgccggccggaatggcgcggccgtagagcgcctgcgcttcgtcgtcgagattcacgtcgtcgagcacgcgcaggtcttccgccaggaacggcgcattgcctgcctgctcatgcggcgcgacgctcaggccggcgttgcgccagcgctcgatcatgtcgatcaagaggaagaaggcgctgaccgcgagcgtggaactcagcaggtagtagagcgcgcccgcccacacggccggttccccgaggccgatggccgcgatcagcgtcccggccgacaccagcacgctgaagccggcaagattggagagccgctgcgtgcccacgatgccgagggcacccgcgaacagcgtggccaggccgatcgcgatgagtaccgattgcccgaaggcggccgaggcgcccgcatcaggcgcgaagagcagtgtccacaagcgcagcagcgtgtagatgccgagcttggtcagcagcgcgaagacggcgcccacgggcgacaccgccgcgctgtacgccggcaccagccagaagttgagcggccaggcgccggccttggcgaagaaggcggtcgcgagaatggcggcggccgcatgcacgaggccgcgatcggccggcgcgagctcggcgatgcgcatgccaaggtcggccatgttgagcgtgccggtcacgccatagagcagcgccgcgccaatcaggaagagagacgaggcggccaggttgatggcgatgtagtgcagcccggcctgcacgcgcagcctccccgagccatgcagcagcaggccataggatgcggcgagcatcacctcgaagaagacgaacaggttgaacaggtcgcccgtcaggaaggcgccgttcaggcccatgagctgcagctgcaagagcggatggaaatgcacgccggcacggtcccatcgcgaggtggaatagatcgaggccgcgaaggcgacgacgccggtgagcgccaccatcatggtcgacaggcggtcggccaccagcacgatgccgaagggcgcttgccagttgccgggcaggtagacgccgatcgacccgggaccgctgccggtgtgaggtgcgtttacccagcgcagcaacgccagcgccgccagcaggcccaccagccccgagaccacgctcagggccgacttggtgcggcggcgcctttcgccgagcaggagcatcaatgcggccgtgagcagcggcacgaggatcggcactgccacgagatgcggcatgctgaagtcgagcagccggtcgaggagttggaccagtgccgtcactccgccgcccccttccgctcttcgccgtccacgtggtcggtgccggcgaggccgcgcgaggccagcagcacgacgaggaacagcgcggtcatcgcaaagccgatgacgatggccgtcagcaccagggcctgcggcatcgggtcggcggtgttctccagcgtggcggtgaagcccttgaccagcacgggttcgctgtctagcttgagccggcccatgctgaagatgaacaggttgacggcgtaggagatgagcgtgaggcccatgatcacctggaaggtgcggggacgcagcagcaggtacacacccgagccggtgagcacgccgatggcgagtgcgagcacgatttccatcagtgcactccctccacggcctcggcctgtgcaattgcctctttctcgcgctgctcgtcggcccagcggtggctgcgaatggattggtgggccagcgcggtgaggatcagcatggtggcgccgagcaccagcgcgaacacgccgatgtcgaagaaaagcgcgctcggcacgtgcagctcgcccaggatgggaaggtgcaggtgtgcggtgtgcgtggtcatgaacggatagccgaacatcaccgcgccgcttccggtggccagcgcaagcagcaggccgacggcgatccagcggcgcgggtagatgcgcagatgttcctccacccactcggtgcccgagacgatgaactgcagcagcagcgccaccgacatcaccagccccgcgacgaagccgccgcccggcgcgttgtgcccgcgcatgaagaagtagaccgacaccagcaccgcgagcggcagcagcagccgcaccagcacggccggcaccatcaggtagcccacggccgtgtccttggcgaggcgcgggttcagcaggtcgctgcttccatcgtcggcctgcgcgcgttgctgcaccggcagcgccatcgattcgcgcgccggccggaagcgtcgcagcagcgcatagaccgtgagcgccaccacgccgagcacggtgatttcgccgaaggtgtcgaaagcgcggaagtcgaccagcatcacgttgaccacgttggtgccgccaccctcggtaagcgcgcgctccagaaagaacggcgagatgctttgcgggaacgggcgcgtcatcatcatccaggccagcgccgccatgccgctgccagcggccgtggccaccagcaggtcgcgcccgcgccggccccaggggcgcagccgggtgcgcgcggactgcacggcgtccttgctgcgcatcggcagccagcgaaggcccagcaggatcagcaccgtggtcacggcctcgaccacgagctgcgtcagcgcgaggtcgggcgccgagaaccagatgtaggtcacgcagcacaccaagcccgcgcccgcggcgagcatcagcgcggcaagccggtggaacttggcctgccacgccgcggccagtgcgcagacgccgccgatgagccaggtcatcgcgaacatggtcgagaacggcagcagttcgcgggtgccgcgcgtggcgggtgcggtccagagcgaaaccgcggcgcccaagccggccaccgcgatcaagagcagcaactgcacctgcagccgccgggtgcccagcacgcggcggctgcgccggccggcttcgctgagttgcgcaagcaggtgctcgaagatggcctggccgtcgaagcggtgcagcagcggcgtgcgttcgagctcgccgcgcgcgcggcggcggcgctgcgacaggtacagcaccacgccgcccgccagtgccacgaagctcattgcgagcggcaggttgaagccgtgccatacggccaggctgtactccggcagcacaccgcccaccacgggcatggcggcggccgccagcagcgggccgatggaccaggccggcgctacgccgaccaccaggcagaccagcaccagcagctcgaccggcacgcgcatccagtgcggcggctcgtgcggctgcctgggcaggtcgggcccgcacggcggaccgaagaacacgtcgaacacgaaacgcgccgagtacgccacgctgaagatgcccgcgacggtggcgatgatcggcaggctcacgttgacccagggcgtcgcctggatgaacaccgtctcggcaaagaacatctccttcgagagaaagccgttgagcagcggcacgccggccatcgaggcgctggcgatgatggccagcgtgccggtgatcggcatcagccgcagcagcccgctgagcttgcgaatgtcgcgtgtgccgctctcgtggtcgatgatgccggcggccatgaagagcgacgccttgaaggtcgcgtggttcatgacgtggaacacggccgccaccgcggccagcgggctgttgaggccgagcagcagggtgatgagcccgagatgggagatcgtcgagtacgcgagcagcgccttcaggtcgcgctggaacatggccacgaagccgccaagcagcagcgtgatcgcgcccgcgccgccaaccagccagaaccattgctcggtgcccgagagtaccggccacagccgcgccatcaggaacacgccgagcttcaccatggtggccgaatgcaggtaggccgagacgggggtcggtgccgccatggcgcgcggcagccagaagtggaacggaaactgcgcgctcttggtgaaggcgcccagcagtatcagcaccagtgcggcgggatacagcgcatgcgcgcggatggcgtcgcccgaggccagcaccacgtcgaggtcgtagctgccggcaatgcggcccagcaccagcgtgcccgccagcaggcagagcccgccggcaccggtgacggtgagcgccatgcgcgcgccgcgccgcgcgtcgcgacggtgatgccagtagccgatcaagaggaacgagaacaggctggtgagctcccagaacagcaccatctggatcaggttgcccgagagcaccacgcccaccatcgcgcccatgaacgcgagaaagaacgagaagaagcgcggcaccgggtcggaggccgacatgtagtagcgcgcgtacagcaccaccagcgcgccgatgccaagcaccagcatgcagaacagccatgcaaatccgtccatgcggaacacgaggttgaggccgagctctggcagccactcgatttcctggcgcagcacgttgccgtgcgcgatctgcggaaagagccatgcggcctgcaacgcgcagcccagtgcgacgaatcccgccagggtcgattcccgattgcgcgcgttcgacggcatcaacgcggccagcacgctggcaatgaagggaagagcgacgagaaagaccaggggcattgcgatcgattctatcgaccagccctgcggctgacgctgttcatggccccatgggaggggccggtttccggtgtgcccggaagccgaaaattcaggccagcgcgaactgcaccgtgcggatgccgaaccacgtcagcaccagcgaaccgcccagatgcagcatgctggtagccagcgccaacaggggtcttgcgtcgagcagcagcgtgacgacttcggccgagaaactcgagaaggtggtgaggccgccgagaaagcccgtgatgagcagcaggcgccacatcggatcgagctgcggcatggcctggaacacgccgacggccacacccaccagatagccgccgatcaggttggccgccagcgtgccgtagggaacggggccgccggtgttgagccacaggccgagaccccacctggccaccgcgccaaacgaggcgccggcgcaaatcgctacgaccgggagcaggggcatccgtttcttctcgctatttctcgatgcccatcaccgtgttgggcaggaccgtgacgatactcgggaacagcgtgatcagcacgatgcacagcaccaggcagaagaagaacggaatcgcagccttggcgatcacgttgctgtctttgccggtcaagttctgcagcacgaagaggttgaagcccaccggcggcgtgacctcggcgatctcgaccagaagcacgatgaagatgccgaaccagatcaggtcgaagccggccttctggatcatcggcagcaccaccgcgctggtcagcacgatcatcgagatgccgtcgagcgccgtgcccagcaccaggtacaccaccaccagcgcgccgatgagcgcatagggcgagagatgcatgctgtcgacccactcggccagctcgcggggaatgccggtgaaggccatggtcttcgtgaggaaggcggcgccggccaggatgaacatgatcatgcaactggtgcgcgtggcacccatgatcccctccttgaaattcttccaggtgaggctcttgccccacgccgcgatgcccagcgagcccagcacgccgaaggccgcgcattcggtggccgtggcccagcccgccaccagcacccagacgatgaagacgatcagcagcgcgcacggaatgaggttgcccgagagccggatcttttccatgaaggtggtcggcgggtcggcgggcggcacctgctcggggtggcgcaggctccaccagccgatgtagcccgaaaacagcagcatcagcaggaagcccggcaggaagccggccaggaagatgcggatgatcgaggcatcggccgccacggcgtacaccaccatcgtgatcgacggcggaatcaggatgcccagcgtgccggcggtggcgagcgagccgatggccagcttctcgttgtagccgcggcgcttgagttcgggcagcgccaccttcgcgatggtggcgcaggtggcggccgacgagcccgagaccgagccgaacacgccgcagccgagaatggtggtgtgcatcagccggccgggcacgcggttgagccagggccgcaggccttcgaacatctcctcgctgagcttggtgcgaaagagtatttcgcccatccagatgaagaggggcagcgccgcgagctcccagctcgcattgctttcccagaaggccgaaaacaggttcttccccggcagcgtgttggtgaagaaggcttgcccgacccagcccacgatggccagcgtcatggcgatccacacgccccccgccagcaacagcagcatgatggcgagcagcagggcgcccatccagagattttcgaacatcggtgtctttgtcgctgttgttcagacgtcggaggagaaatcgcccgcggcgtgccgctcttcgatggcgcgctggtagctgggcttctcgccgcgtaccacgcccaccagttcgtcgatcatggcgatcagcagcaaccagcagccgatcacgaaggtcgattgcggaatccagatcgggatgacgacgaggccggtcgccatttcggcgaactcgtagctctcgtaggtgaagctggtggcccagtaagtgagataggcgaccgacaccgaggcgatcagcaggcagaccacgtcgagcacgcgtcgaaccttggccggcaccgcatcgagcagcagcgtcacacgcacgaaatcgccgtgccggaaggcttgcgccatcgcgaagaacgcggcagcggcgcacagccaggagacgacgtcgttcagcccgctcacgtgccaattcatctgccggcccacaccggccaggatcatcagcacgaagatgaggaacacgcagaaggcgccgagtgcgccggcgccgttgtacaaatgatcgaggaaacggcgcacggctcagacctcccgcgatgagcgtggaggcttcatcacttcttcttgtaggcgtcgatgatcgcggcgccctctgcaccggtggccttgagccagtcggcctgcatgatgccgccgacctggcgcatgtcggcgtcgagcttggccgagggcttgtgaaccttcatgccgcgctcggcgagcaggcgcttgtattcgtcgttcttctcctgcgcgattttccagccgcgggcttccgcatcggccgcggccttggtgacggcggccttggtggtggcgtcgagcgcgtcgaaggccttggcgttgacgaggatcgcgttcttcgggatccaggcctgcgtgtcgtagaagttcttgatgtgctcgtaggtcttggtgtcgtagccggtggagcccgagctcatgtagctttcgatcacgccggtggccatggcggcgctgagttcggcctgctggatctgcaccggctgcgcgccgatcagctcggcgatctttgcggtggccgggctgtaggcgcgccacttgatgccgcgcaggtcggccaccgagctgatctccttcttggaatagatgccctgcggcgcccatggcaccatgaacagcaccttgatgccttgtgctgcgagcagcttttccatggcgggcttggaggcctcgtagagcttctttgcgtcgggataggtggtggcgagaaagggaacgccgtcgagcgcgtaaatcgggttctcgttcgcgtagttcgccagcaggatttcgccggcctgggcctggccgctttgcacggcgcgcttgatttcaggggccttgaacagggacgcgttggcatgcaccgtgatcttgaccttgccgccggtggcggcgtccacgtcttttgcaaactgcgtgatgttttcggtgtggtagttggtcgccggataggcggtgggcagatcccacttggtttgcgcgaaagccgcggcaccgagggtgaggccggccagggcaataccgaacttgtgattcatgagcgctccggaacgaatgagagtgaaagcgaaagcgagcatacgtgcaaattccgggccactcctgaggcatttccctgccacgccgcgctgcgcggcagcagggccttgtgctgcggcggacgcaaaaaaaccgcctcgagggcggttttgctttgggctgccgtcagtccgcgcatgcgggactgggcacctggcttgtggcttttcgatcagggcttggctggcttcgcatcggcagcaacggcggctgccttgacgggctttgcggtcttgtctgccttggcggctgccggtgcgctggcttggccaccgaaggcctggccgttgatcgtgagcccttcggccgacagcttttcggccttcttttccttcacgcccttgatgcgctgcatgaagtcgggccagtccttgaactcgcctgcctttcgcgcgtcgaggatgcgcttggacatggccgggccgatgcccttgatgccatcgagatcggccgcggtgcccttgttgacgtcgacggcggcgaacgaagcagccgcaaacagcatggccagcgtggccaggattttcttcagcatgatttcaaactccctgatttgttgatttctgtccgccggcgcagccgccggctcgcgttcaacgagttcagggaaagaggcgttgacggcctcgtgccgtgcaagggttcagatcaccattgttccgaaacatgttcggaacgttgctcagagttcttcgacgcggcgtggcgggtagctgtcccaggcctggcatccggggcagtgccagaaatgctggtgcgcctcgaagccgcaggcggcgcagcggtagcgcatcagcggccgcgtggcctggtcgagcgcgcgctgcacttgcggatggaactgctcgtgctcgaagcgctcgctggccagccagcgcgaagcggccaccagcgaaggctgctgcgcgagatgcgcgatgtagccgtcgcgcggtgcgagcggcgagccttccgcggctgccatggcatgggcgggcgaaccgccaagcgccatcagtgcctcgagcacgtcgatggacggcgattcggcatagcggcgctgcagcaactgcagcgcttcgccttcgcggtgcgcagccaccgcggcctgctgcagcgcagccgcatacagcggcagcgcgagtggagcggtattgctcaacgcgacgagggtttcgaatgccgtggcggactcgccattgcgcaactgcagcgtggccgagtcgatggcggggcgcggcgcctgcggggccagtgccacggcttccgagagcagccggttggccgcggccaggtcgccggcggccacctgttcggccgcctgttcgcagagatgatgggcccggcgcgtgctgtagctcgcctggtcggactcatcgagtttctgcgccacgtcggcggcctgggtccattcgcgcgagcgctcgtagatggccaggagcgaaagccgcgcctcgttttcgtagcgcgtgccctcgagcttttgcaacgcggcttcggcgcggtcgagcaggccggcgcgcaggaaatcctgcgctagcgcatgctgggcccgctcccggtcgctgcggctcagatcgccgcggcccagcagatgttcgtgcacgcgcactgcgcgctggtattcgccgcgccggcgaaacaggttgccgagggcgaagtgcagttcctgcgtgtcggggtcgttctgcacggcctcgatgaacgcatcgatggcctggtcctgctgctcgttgagcaagaagttgaggccgcggaaataggccttgggggcttgcctgttttcgagcttgagctggcggatgtcgaagcgcgaggcgagccagccaaggacaaaggcgacgggcaggctgatcagcagccagctgggatcaaagtccatgttggcgtacggcgggtaggtcggtggcggagatggacggtgccggtgcaggcgccggtgaggccggcaatccggtcgtggccggggtttgtgggcggggcgcggaaggcgcctgggccgcggcggcggcgcggtgcttccaccatcccggcagcatgccgagcgcacccacgaccaagccgccggcaaaggctgcgagcaccacgagcaccagcggcgcgcgccagtgggtgccaaagaagaaatagacggtcgcgtcgtgctggttgttcagcgcgaaagcaaaaagcgtaaaaaaaatggctgccttgagcagccacaggaggtatttcatagccgttcccgttggcgggagcattctacgtttgcatcatcatccatgcggatcaggccttgcggcccttggcttccttgcctgcgtccagctcggcggtcttggcgtcgacggcttcgcgcagcgccttgcccggcttgaagtgcggcacccgtttttcgggaatctgaacgctttcgcccgaacgcggattgcggccgatgcgcggcggacgccggttgaccgagaagctgccgaaaccgcggatctcgatgcggtgcccgcgcaccagtgcgtcgctcatcgcgtcgaggatggtcttgacggcgtattcggcatcgcggtgcgtcaactgcgcaaagcgcgctgcgagttcttcgacgaggtcagagcgggtcataggccaaacaaaaacgtggacgaaaaaaaagacagagcggccccagggcctgctctgtcttcggacgcagcttacttgctgtcgttgttgtcgagcttggcgcggagcagggcgcccaggctggtcgtgcccgcgttttcgcgtgccgactgctggctcaggttggccatggcgccttgttcgtcgaccatgtccttctgcttgatcgacagctggatgttgcgggtcttgcgatccacgttcacgacgatggcggtgacttcgtcgccttccttcagcacgttgcgtgcatcttccacgcggtcgcgggagatttcgctggcgcggaggtagccgatgatgtcttcgccgaggtcgatttcagcgccgcgggcgtccacggtcttgaccttgccggtcacgatctggcccttgtcgttcacggtggtgaacgtggtgaacgggtcgctgtcgagctgcttgatgccgaggctgatgcgctcgcggtcgacgtccacagccagcacgatcgcttcgacttcctggcccttcttgtagttgcgaacggcggtttcgccggcttcgttccacgagaggtccgagaggtgcaccaggccgtcgatgccggcagccaggcccacgaacacgccgaagtcggtgatcgacttgatcgggcccttgacgcggtcgccgcgcttggtgttctgcgcgaactcttgccacgggttggccttgcactgcttcatgcccaggctgatgcggcgcttgtcttcgtcgatttcgaggaccatgacttcgacttcgtcgcccagggagacgatcttgttcggagcgatgttcttgttggtccagtccatttcggagacgtgcaccaggccttcgatgccgggttcgagttcgacgaacgcgccgtagtcggcaatgttcgtgaccttgccgaacaggcgggtcgattgcgggtagcggcgcgaaacgcccatccacgggtcgtcgcccatttgcttcagacccagcgagacacggttcttctcggtgtcgaacttgaggatcttggcggtgatttcctggccggcctgcaccacttcgctcggatggcgaacgcggcgccatgccatgtcggtgatgtgcagcagaccgtcgatgccgccgaggtcgacgaacgcaccgtattcggtgatgttcttgaccacgccacggacaacggcgccttccttcagggtctccatcagcttggcgcgttcttcgcccatgctggcttcgaccacggcacggcgcgacaacacgacgttgttgcgcttgcggtcgagcttgatgaccttgaattccatggtcttgttttcgtacggcgtcagatccttgatcggacgcgtatcgatcagcgaacccggcaggaacgcgcggatgccgttgacgagcacggtaaggccgcccttgaccttgccgctggtggtgccggtgacgaagtcgccggattccagtgccttctcgagcgcgagccacgaggccagacgcttggcggtgtcgcgcgagaggatggtgtcgccgtagccgttttcaacgctgccgatggcaacggaaacgaagtcgccggcctggacttcgagttcgcccttgtcgttcttgaactcctcgatcggcacgtacgcttcggacttgaggccggcgttcacgacgacgtggttgtgttcgacacgcacgacttcggccgtgatgacctcgccggtgcgcatttcggaacgcttcagggactcttcgaataggtcggcaaaagattcagacatttatggttccttccgtcaggcagggttggcaggcgctcttgcgaaattgcgtgcggctgctgtgggtctggagacggcggttttgtgggctggtgcccggttggttgaacaaccagcaggccggtgcgctgtcgcgcgagaggagcctgccggagcggtatgcgctaccccggaatccggttggcgcgagcctttcgggcggacctgaaaggctgtgacttcaaaccatccaagcggacttgaacggctgtaacttcaaaccgctcaagcgggcttgaacggccgaatctcctgccaccagttcaacacctggtcgatcgattgctcgatggacagctgggagttgtcgagatgacgggcatcctgcgccggcttgaggggagcgacgctgcgggaagagtccctggcgtcgcgcgcttccaagtcggagcgaagactgtcaagtgtagtcgaaataccctttgaaatcaactgcttatgccggcgttcggccctctgggcggcgctggccgtcaggaagaccttcagcgccgcgtcggggaagatcacggtgcccatgtcgcggccgtcggccaccaggcccggaagctgccgaaaacgctgctgcagcgccaggagcgccgcgcgcaccgcgggcagggtggagacgcgggaggcgtccatgccggcggcttcggtgcggatgtcgtcactcacgtcttcgccggcaagcagcaccttgccttcggtgaagtgcagcggcagggacgctgccagggtggcaatctgcgcctcgtgctgggggtcggcgctgagcccggcgcgccgcatggccaagccggtcacgcggtagagcgagcccgaatcgaggtagtggtagccgagcaggcgggccacttcggctgcgagcgtgcccttgcccgaggcggtggggccgtcgatgcagatcaccggaacgtcgaaggcctcggccaccgagaacagggtttcgaagtagtccggaaaggtcttggcgacgcagtggggttcgaggatgcgcaccggcacccgggccggattgaatgccgcgagcgaaaaacacatcgccacgcggtggtcgtcatacgtgcggatgctcgccggccgccagtcggccggcgcaagcgggtgcacccggatgaaatcggggccggactcgacggtggcgccgagctttcgcagctcattggccatggcgtcgatgcggtcggtttccttgacgcgccagctggcgatgttgcgcagggtgctcgggccgtcggcatacagcgccatgacggccagcgtcatcgcggcatcggggatgtggttggcgtcgaggtcgatggccttgagcggccaggcgccccggcgcacttcgagccagttcggcccgctgtcgacccgcgcgcccatttgctgcgccgcgtcgatgaagcggatgtcgccctggatcgaatccgcgcccacgccctcgatgcgaacgccgttctggccggcaatacccgttgcgatggcgcccagcgcgatgaaatagctcgcagaggaggcgtcggcctcgacatggatgtcgcccggcgagctgtagctgctgccggcgggaatggtgaagcgctcccagccatcgcgccgcacgctgatgccgaagcgtgccagcaggttcagcgtgatctcgatgtagggcttggagatgagctcgcctactacctcgatgacgatgtctttgcgggctgccagcggcaaggccagcagcagcgcggtcaggaactggctcgacacgtcgccgcgcacacggatgggcgcatcgagcgccagcgcgccgtgatcggccgggcggatgcgcagcggcggatagccggggttgcccagatagtcgatgtggcagccgagctgggtcagcgcatcgaccagatcgccgatcggccgctcgtgcatgcgcggcacgccgctcagctcgaattcgccgcccagcagcgacagggcggcggtcagcggacgcatcgcagtgccggcattgccgaggaagagcggcagcaacggcccgcccggcttcaactggccgcccaggccggtgatgcgcagcgtgttgaccgccgcatcgatgccgcagccgagcgcgcgcagcgcgtcgagcatcacgcgggtgtcgtccgagtcgagcaggtcgtgaatggtggtggtgccgctcgccagcgccgccagcagcagcacgcggttcgagatgctcttggagcccggcagccgcacggtgcccgaagccgccgcgagcgggggaatgtccaggaaggccgtcgaaaacatgtcaggcgtcctgcgaggcgtcggtgttgggctgccaggcggcgcggaccttgctggcggccgcaatcgcatgctccagcgcctgcgcgtcggtggcggccatcagtgtctcgagttccagcagcgccttgcgaaaggcctgcgattgcagcagcacctgctcgcggttggcaagcagcacgtcgcgccacatcactgggtcgctggccgcaatgcgagaaaaatcgcggaagcccggccccgcgaggcccaggaagcggtcgccctgcggctgcgcgacaagggcgttgatgtaggcgaaggccagcaggtgcggcaggtggctcacggccgcaaaggcgctgtcgtgctcctcgtgcgtcatggtgaccacgttggcgccaatgccgctccagacttgcgaggcccgctgcacattggagcgcagcgtcgccttgaccggcgtcagcacgaccttgcggccggcatagagcgaggcgtcggcgtgctcgatacccgacacctccttgccggcgatcggatgggccggaacgaagctggcgaactggttctgcaggccgttgcgtgcggcttcgatcacgtcgcctttggtcgaacccacgtccatcaccagcgtgtcgttcgaaatgccgtggcgaatggccttgaaggtggcttccgaagctgcgaccggcaccgccagcagcaccaggtcggaacccgagaccgccagcagcgcggaaggcgccaccacgtcgatcacgccgagctggcgcgcccgctccgtggtggagggcgacttgctgtagccgaccacgcgcttcacgagttttgcgcgcttgagcgcaagcgcaaaggagccgcccatgaggccgcagccgatcaatcccaattgctcgaacatggtgcttgtccggctcaggctttgacggggtaggcgccaagcaccttgtagaacgcgcagaggccgcgaagctcggccagggccgccgccacgttgggctgcgagggatggccgtccaggtcgatgtagaagtagtactcccactggccggtgcgcgcgggccgcgactcgaaacgggtcatggaaacgttgttgaccttcagcggcaccagcaggtcgtgcacggcgccggggcggttgggcacggagacgatcaggctcgtgcaatcgcgcccggatgccggcggcatggccagcgtctggggcaggcagatgaccgagaagcgggtgcggttgtaggagtcgtcctggatggcgtgcgcaacgatgtgcaggccgaatcgggtggcggcgcgttcgccggccagcgcggcccaggccgggttggtggccgcgagccgtgcgccttcggcgttgctcgagacggcgcgccgctcggcgttgggcagatgcttcgaaagccaggtctggcactgggccagcgcttgcgggtgggccagcaccgcctcgacgccgtcgagcgtattgctgctgcgcagcagatggtggcgtaccaggaggctgacttcgccgaccacgtgggtgggcgaatgcaggaacaggtcgagcgaacgcgtgaccacgccctcggtcgagttttcgacgcccaccacgccgtactgggcgctgcccgccgccgtggcgtgaaacacctcgtcgaagctggcgcagtagatcaggtcggcggcgccgccgaagtattcgatggcggcttgttcgcagaaggtgccctcggggcccagcacggccacgcgctggggcgattcgagcgccaggcaggccgacatgatctcgcgccagatggccgccacgtgcaggtccttgagcgggcccgcattgctcttttgcatcttttcgatgacttgggccacgcggtcggggcggaaatacggcgtaccttcgcgcttcttgacctcgccgaccagttccgccacgtgggcccgctcattgagcaggctgagcagttgctggtcgagcgaatcgatctgcacgcgcagaccggcaaggctctcggagttgtcgggggaggagggcggagttggagcggaggcggtcatcggtgcgagcaacagggcatgcgcctaggcatgcgatcgctcgaattctcgcatgtagctcacaagtgctcgcacaccttccagcggcatggcgttgtagatgctcgcgcgcatgcctccgaccgacttgtggcccttgagctgcagcagcccggcctcgcgcgcgccggccaggaaggcgtcgttccggctctcgtcgcacaggaagaacggcacgttcatgcgcgagcggcagcccgggtcgatcttgttgacgtagaacgaagagccgtcgatgaagtcgtacagcagcttcgccttggcgatgttgcgctgctccatggcggccacgcccgtgaggggaccttcggtctgctgcagcagccattggaacgtgagcccggccatgtagatgccccaggtcggcggggtgttgtacatggacttgttgtcagcaacgatcttgtagttgaacgcgctggggcagatctcgagcgcatgaccgagcaggtcgtcgcgcacgatcacgagcgtgaggccggccgggccgaggttcttctgcgctccgccgaatgccaggccgacgcggcgccagtcgatggtgcgcgaggccacgtgcgacgaaaagtcgatgaccagaggcgcattgctgccaagggccgccaggtcgggcagttgatgaaactcgatgccgttgatggtctcgttggtgcacaggtgcacgtacgaggcgtcttgcgtcagctgccaggtcgacggggcgggcagccgcgtgtgatggtcggcggcgttgctggcggcgatgttcgccgtgcaatagcgctgcgcttccttttgcgacttgatgctccagctgccggtgatgacgaagtcggcggatttgccgcgcgacaggttcatcggcacgatggcgttctcaccgagcccgccaccctgcatgaagaggatgtggaaattctcgggcacagccagcagcgtgcggatgtcggcttcggcctgggtgcagatggcgccgaattccttgccgcgatggctcatttccatcacgctcattccgctgccttgccagtcgagcatttcggaggcggcgcgttgcagcaccacctccggcatggcggccggacctgcggaaaagttgtacgggcgcgtgccggcgggcttgggctgctgctgttgtgtcacgtcacttcttggcgggagccttggccggggccttggcgggagcggcgccttgctgcgaaccgccggtcggagcgcccagcgccttggccacgttttcgtcgagtgcgcgcatcttgggttcgatggttccgcgcgtttcggccacgagcttttcagtcagcgcggtctgcatcttcggattcaggtcctggtacttcttgctgagcggcgagttgatccaggccagcaattgcttgagctcttcttcgctgaagttctgctcgagcagcggggtgagggcgcccggtgccagctgcacggccttgtcgcgcacgatcgggtaggcatcgtcgaagtacttcttcagttcggcgtcggcggccttggcagccgactcgcgcttggcttcgggcacttgcgtttgcaggtactgcgaaccggcctgcgcgatgggcgcgctcgattgctcgaccaggccgcgtgccagggattcgatgccggggcgttgcacgtccacgaactgcttgataagcgcggctttgtcctgtgccatggcggccatcgagctgccagccagggcgacagtcagaagtgcgagcttgaattttttcactgagggttctccgttgaagatgtggaagtatcgtctgcgcctggctcggtctcgccgttggcgtcgttttcgacgattcgctgtagcccgctgagtttggcgccttcgtcgagcccgatcagcgtgacgccttgcgtcgcgcgacctagttcacgaatctcggcaacccgggtgcgcacgagcacgcccttgtcggtgatgagcatgatctcatcgtccgcatgcacgagggtggcggcaacgactttgccgttgcgctcgctctgttgaatcgcaatcatgcctttggttccccggccatgacgggtgtactcggtaatgcttgtgcgctttccgtaaccattttcggtggcggtgagcacgctctgctgctcgtcctcggccaccagcatggcgatcacgccctgtcccggatcgagcgacatgccgcgcacgccgcgtgcattgcggcccagcggacgcacgtcttcttcgtcaaagcgaaccgccttgccgccatcgctgaacagcatcacgtcgtgcttgccgtcggtgagggcggcgccgatgaggtagtcgccctcatcgaggttaaccgcgatgatgccgcccttgcgggggttgttgaactcgtcgagcgtggtcttcttgaccgtgcccatggaggttgccatgaacacgtattgatcggccggaaaattgcgcttctcgccggtcagggcgagcgcgacgttgatcttctcgccttcctgcagcgggaacatgttgacgatcgggcggccacgcgatccgcgcgaacccgccggcacttcccacaccttgagccagtagagccggccgcggttggaaaagcacaggatgtagtcgtgcgtgttggcaatgaagagctggtcgatccagtcgtcttccttggtgaccgtggcctgcttgccgcgcccaccgcgtttttgcgcgcggtattcgtggagcggctggctcttgatgtagccgctgtgcgagagcgtcaccaccatgtcggtcggggtgatcaggtcttcggtcgagagatcgaaggcgctgtgctcgaccaggctgcggcgcgcgccgagcttcgattggccgaactcctgcctgatggtgccgagttcgtcgccgatgatgaccgagacccgctcgggcttggccaggatgtcgagcaggtcgtcgatctctgccatcacctctttgtactcggcaacgatcttgtcctgctcgaggccggtcaggcgctgcaggcgcatctgcaggatttcttgggcctgggtttccgacaggcgatagaggccgtcagagcccatgccgaactcgcgctccaggccctcggggcggtagtcgtcggcattgaccgcgccgccgtcggcgcgtgaacgcgtgagcatttcgcgcaccagcttgctgtcccagctgcgggtcatcagctcggccttggcgaccggcggcgtcggggcgttgcggatgatcgaaatgaattcgtcgatgttggccagcgccaccgccaggccctcgagcacgtggccgcgttcgcgggccttgcgcagggtgaagacggtgcggcgcgtgaccacttcgcggcggtgctgcaggaagacctcgatcaggtccttcaggttgcacagcttgggctggccatcgaccagcgccaccatgttgatgccgaaggtgtcctgcagctgcgtctgcttgtagaggttgttgagcaccacctcgggcacttcgccgcgcttgagttcgatcaccaggcgcatgcccgacttgtcggattcgtcctggatgtggctgatgccttcgatcttcttctcgtgcaccagctcggccatgcgctcctgcagcgtcttcttgttgacctggtaggggagctcgtcgacgatgatcgcctggcgctggccgcggtcgatgtcctcgaagtggcacttggcgcgcatcacgaccttgccgcggccggtacggtagccgtcccggacgccgttgatgccatagatgatgccggcggtggggaagtcgggcgccggcacgatttccatcaactcgtcgatggaggcctgtggattgcgcagcaagtgcaggcaggcatccaccacctcattgaggttgtgcggcggaatattggtggccatgccaaccgcaataccgccggagccattcaccagcaaattgggcagtttgctcggcaaaaccttgggttctttttccgagccgtcgtaattgtcttggaaatcgacagtttccttgtcgatatcgccgagcatttcgtgcgcaattttggcgagccggatttccgtataccgcattgcggctgcgttgtctccgtcgaccgacccgaagttgccctgaccgtcgaccagcatatggcgcatggaaaagtcctgcgccagccgcacgatggtgtcgtagaccgactggtcgccgtgcgggtggtacttgccgatcacgtcgcccacgatacgggcggacttcttgtaggcccggttccagtcgttgttgagctcgtgcatggcaaacagcacgcgccggtgcacgggcttgaggccatcgcgtgcatcgggaagcgcccggccaacgatcacgctcatggcgtaatcgagatagctgctgcgcatttcctcttcgagactgatgggcagggtttctttggcgaaggaggtcattgagcgagaggctggcggcaggaaggcgaaattttacgctgtgaggggtgtcgcaccgccgcaacacaaggcggctattccgcctccgtcctacgcttccgggccgtccagcggcctgtttgccaaagaccctatggcacaatcgcctcaacgttttgggtggtggtcacttaaagcgtccttgattcgcagcgcggctgcggctttttccccaagaggagaaccatgaagaaactgaataaagtggcgatgatgtttgcagtcgctgcgctcgccactgccgccggcgcgcagacccgtgtcaccgctgcgaatggcggtcctacgatcgacaactggcaaaacggcaccggcgaactggtttggaagaacggcacgaatgaactgtgctggcgcgatgccaactggacgccggctactgccgccgctggttgcgacggtgctctggttgcagcagctccggctgcagtcgctcccgttccgggcgcaccggccgctcctgcgcccgcaccgcaagtcgctgcttcgaaggtgaccttcgctgctgacgcattcttcgacttcgacaagtcggttctgaagcctgaaggtcgcgcaaagctgaccgacctggtctcgaagatccgtgacgtcaacctcgaagtgatcatcgctgtgggccacaccgactcgatcggttcggacacctacaaccagcgtctgtcggtgcgccgcgccgaagccgtcaaggccttcctggtctcgaagggcatcgaacgcaatcgcgtctacaccgaaggcaagggcgagaagcagcctgtggctgacaacaagaccaaggaaggccgcgccaagaaccgccgcgtggaaatcgaagtggtcggcacccgcgccaacaagtgattcgattgaatcgctaaaagaaaaccccgcctcggcggggtttttttatgcctgtcgaattccttctgatacgcgtcgagtgtccactcgtgttcgccggcgcattctccgtttcataatcgtggcatgacagataacgtgaatgccgatccggcggaactcgccaagttttcggaactggcccatcgctggtgggatttggacagtgaattccgtccgctccatgaaatcaatccgttgcgactggaatggattgacggtattgcgcccatttcacagcgcaaggtgctcgatatcggctgcggcggaggcatcctcgccgattcgatggcccgaaaaggcgccgaggtgctcggcatcgatctggcgagcaaggcgctcaaggtggcgaggctgcatgcactcgaagccggcacgagcggcgtcaaataccgtgaaatcagtgccgaggcgctcgctgcggagcagcctggcagtttcgacgtcgtgacctgcatggaaatgctcgagcatgtgcccgagcccgcttccatcgtccaggcttgcgcaacgctggtgaagccgggcggctgggtcttcttctccacgatcaaccgcaatctcaagtcgttcatgctggccatcgtcggtgccgaatacgttctgggcatgctgccccgcggcacccacgaatacgccaagctgatccgacccagcgagctggcggcccactgccgcgcagcgggcctcgacttgcggcacacgcgggggatggaacacaacccgttgacgcgccgctactggctcagcgccgacaccagcgtcaactacatgttcgccacgcagaagccggcctcgacgacgggttcgcaaacgtgacggccgcagcagtggaagccgtgctgttcgatctggacggcacgctgatcgacagcgcgcccgatctcggcgccgcagccgacaagatgcgtaccgaccgcgggctcgagtcgtatccgctggagcgctatcggttcatggccggagctggcgcaaggggcatgctcggcgtggcgttcggcatcatgcccgatgcaccggagttccccgcattgcgcgaagaattcttcgtggcctacgagaaccgcatgttgctcaatacgcacgtgttcgacggggtgcaggcgctcatcgacaccatctgcgcacgtgggctggcctggggtgtggtcaccaacaagtcggcgcgcttcaccgatccgttgacgcgcgccattccgcttttcggcagtgcgggcgccatcgtgagcggcgatacgacgccgtattccaagccgcaccccgagcccttgcacgaagcagcgcgacggatgggcgtgccgtccagcgcgtgcatctacgtgggagacgacgaacgcgacatcatcgccggccgtgccgcgggcatgcgaaccatcgcggcgacctatggctacatgggcccgcaggccgatgtgacgctctggaacgcagatgcttcgatcgcagcgcccctggagctcttgcaattgctgaataaggcctaaaatgcttggcttggggctgcactggtttcgacgtgggttcggaatcgcagcggggcatgtcgagctgaatgcgctcgtaaaacagattcaaacaaactaactgcaaacgacgaacgtttcgcactcgctgcttaattgccagtgagccttgcaacagttggccgatgggctgggcaagggggtctggagcaatcctgacctcccggctgcaaggataattacatgggctggctccgatccgggtaccttgggtcggggcgagaaaatagggtgctggcgtccggtttagcgtgtgactgcgcgactccggaagcgagactcaaatcagatcactaaacatgtagaactgcgcgaagaaggcttgcggacgggggttcaaatccccccagctccaccaacacaacgtccaagggcgttcactgaagttcagtgaacgccctttttcattggagaaacagctgttggtcgtacgaggaggtgtggctcagttctgccgtgcggctggctgtctcctcattaccgctgcgcaaggtgatctgctgcgcctgcgggccgccccttcgccacgcacgaaaaaaggggagctctttgccttcaggccggctctggccaagtcgcctggggtgggcggaccaactcgtagaagtgcgcgatctgcagcacccccaggtcgtcgaatcggcgccccgcgatctgcagccctatgggcaagccgccgtgcgaatagccgcagttgatcgaggccgcgggctgctccgactgattgaacacggaagtgaagtgcgaatccgtcagtggattctccgagccgctgcgaatcgcttccgctgcgaatggcaacaccggcgagacaggcgacagcacatagtcgtacggctgcgtagcggtcacggtcgcggcgcgcagcatctgaaggcgggtgaaggcacggaaggtgtcctcgggcgtcagcgaagctgcgaactccgcggcttcgtggatatagctggcggtaagcttcgcgcgcgctgccggcatcgcagccagatcgacacggcagcgcatggtgaagaaatgggctatgcccatgcgcatctcttgggttgtccagtcggcgatgggctcgacgatggccccagctttcgcgaagacgtgagctgcggccagtacggcttccttcacttcggggtcaatcggccacccccccgcagtgtcggtccacaggccgatgcgtaggccgcggatatcacgatcgagacgctcccacgggatgtcctgcggcggcaggctcatgtagtcgcgcgggtcgggacgcgagaccactttcatcagcagcgcggcatccgccaccgtacgggttatggggccgatgacgcgggcgttggccggtggatcgaccgggatgcgtccctggctgggcttgaggccgaagacgccgcaaaaattggcgggaatgcgtaccgagccgccaatgtcggagcccaggtgcagcgggccatagccggcggcggcagcggcaccggcgcccgagctagagccgccggtgttcttgctgaagtcccacggattgcgcgtaagaggatggaagctcgatggcgctgcgcccaggaagccgaaatcgggcatcgtcgtcttggtgacgatgatcgcgccggcctcgcgcacacgcgcggcagcgggggcgtcgtgcgcggcgggtgtgagcacggtcgcggcgctgcccagcggcatcggcgtcccgcgcgtggcgatgttctccttgagcgtgatcggcacgccatcaagttcgccctggggcgcgttgcgcgtccaccgcgcctcggaggcccgtgccgccgccagcgcggcattggcgtcgagcccgtacgtggcacggatgtgcggctcccagcgctcgatgcgtgcgagtaccgcctgcgttacatcgaccggggacaggacgcgatcccgatagcgttccaacagttgcgtcgcgctgagttcgtgcaaggggcgtgttgttgccatgacgggcggaactcctgggatagctggaaagcgactagcgtcctccaactgccctcctgtgaaaacgagaggctcgccgtcggcggcgacgaagtccactagagcaagggcgcagcgccgcgccatccaggatgaccagaattctaattaaaaatgaattctaaagtactaaaaatggatggaaagatttccggctattccggacttatttcacgagggatgcacattcatcggcactttgtctcttttgagtatcgagtgttaaccgttttgatgcaatgacgcaataaacttgtatccattgttttcaatggttttcatactaataccaaagagttattggagggatatgcacgcggatttggcattgaagatgatgtcagacctgttctggacggggctgctggtctgccttccgctgttggggctcactatgctcgtcggcatcgtgatcagcgtgctgcaggtcgtcacgcaggtccaggaaatgtcactgacgttcgttccgaagcttgtgactgctgccgcagtgatgatcgtggcgggcccctggatgcttcgcaagttgactcagttcaccgtccagctctggggcggcattccctcgatgttctgaggcaagggctcccgtgaatgctctccagctgcatgcagcgcttgcgttgcctgaggtcgtgacgtctggaatcagcacgtccggaatggttgtcgtcggcttgctggcgttgcgcgttgccgcaacctttgcgatgacgcctgtgctctatgcggtgccgctgcctgcatcggtgcgagtgctgctcgtcgttggactctcggtggcattggcgtcgggtttggccgttccggctggcacagcgattgggtggggcgcgttgctttctgcggcgatggcggagcttgcgcttggagccgtgctcggtcttggcattctgctggcgtttggtgcctttgccgttgcaggccagttgcttgatgttcagttgggctttggcattgcgcaagtcatcgatccggtgacgcagcgtcccattccggtgcttacttcggcattcaactatctcgcagtactggtgttcttccttctcaacgggcatcacgcgctgctgcgcggcatcagctatagcgtggagcgctttcctgtgggcgcatcttggtctgtcggacatgcagttgccccggtgctgaagcaggcggcgggtctcttcagccttggttttgcgctggcggccccggtggtgttttgcatattgctcgtggagttcgcactgggcgtggttggtcgcaatctgccgcagatgaacatgttcaccatgggcattccggtaaagatcctggtcggcctgatcgcactctcattctggtttgccggcatcggccctgtcatgacgcgcgcctatgccggtatagcgtcgacatgggacggcatcttcgtcgccgcgccggcaccgagggagcagaggcgctgatggcagagcaggaccttgaccgcaacgaggcggccacaccttacaagctgcagcgtgcacgcgagcgtggacaggccgcgaaaagcactgatgtcgtggctgcgctcgtgttcggtgtggcggtggtctacctgacctggcgcgggtttggcgctgtggcgagccagttccgattcgaccaggcgcttctgatccacgcgggccggatggatccctcgggcgtgggcctctggccgctgatcgagcgtgccttgcgctccgcattgacgcttgcggcgcctttcttcgcggccatcatgctggctgcgatcgtcggcaacatgatgcagaccggcccgatactttcgttcgagcccgtgaagatcgacttcgaccgaatcaatccggtcaacggcctcaagaaactgttttcgatgcgcgtgctgttcgacacggctcgcgccatcgtcaagttgagcttgctggcactggtcgcttttctagcgctcaaggccctgacaagtcagttctatgcgctggcctctctttcggccgtcggctatctgcgcgcgctgctgggcgatcttgcgagcgtcgggctgaagatggccctggtgctcacgctcattgcactgctggatctgatgtacacccggcgcgagttcgcaaaaaaaatgcggatgagccagcgtgaactcaaggacgaagccaagcaccgcgaaggcgatcctcgcatccgcgcccgattgcgtgaactacggcgggagacgctgaagcgaagccttgcattgcgccagacccgaaacgcggatgtgctgatcaccaaccccacccatcttgcagttgcgctcaagtacgagcacggccgcatggcgtcgcctcagttgctggcgaagggagcagggcacatggcggccgccatgcgcgagattgccgcacgccaccgcattccggtggttcgtaatcccgcgctggctcgccgcctctacaaggagctgccggtggatcactcggtaccccccgaactctacgcgcaggtggcacgcatcatcgtgtgggtgtttgccatgcgcgaacagcggcatggccgaggtgcggcctcggctgcagagggccgggcatgaactcgcttggacgcgtccttggcaagcacagcgacatagcgctggttgtgctggtgctcggcgtgctggtggttctctttgcgcccattcccagcggcttgctcgattttctgatcctgagcaatttcggcttcgcattccttgttctgctgttgaccttctacatggcgcggccggtcgagttctcgaccttcccttcgctgctcctgatcgcgaccctgttccggctgtcgctcaacgtggccgccacgcgtctcatcctttccgacggggatgcgggccgggtgatcggcgccatcggtgcattcgtggtcggcggcaactatgtcatcggcttgatcgtgttcctgattctcatcgtggtgcagtacgtggtggtgaccagcggcgcgcaacgggtttccgaggttgcggcgcgtttcacgctggacagcatgccgggccagcagatgagcatcgacgccgatctcaacatgggcttcatcgatcaggccgaggctcagcgaaggcgcaagaacatcgagaaggaagccggcttctacggtgcaatggatggggcgagcaagttcgtcaagggcgatgcgatcgccggcatcatcatcctgttgatcaacatcatcggcgggctggtgattggtgtcatgcagcacggcatgccgtggggccaggcgctgcagacctacaccttgctgaccatcggcgacggcatcgtcacccaggtgcccgcgcttgtgatcgccgtgggcaccggcatcatcgtgacgcgctcttcctccgacgtcaatctgagccgcgaagcactgcggcaggtgagttcgtttccaaagacgttgcttctcgttgcgatggctcttggaggattgctcttgctgcccggcattccggtgttgccgacgcttgttctcgccatgttctttctgctggctgcaacgatgctctaccgggccgccaaggcaaaggactcgaatgccgcttcggcctcgcctgatggcgcagaaggttcgcagcaagctgccgatggctcgttgacgcaggcgagcgacgatgcctacgcgcagctgcaggtcgagcccatcgaagtccatctgggaagcaactgggtcccggtggtcaaccagccgggcagcgtattcatggagcgggttgccgcctttcgcaagcagcatgcgcaggagttcggcctggtgctgccgcgcgtccgtttcaaggactccgcgcgtctgtccgccgatcggtacgaaatacatctggacggcgtcatcgtgggcaagggcgaggcacgtgcggaccggctccttgcaattcatccagcgggcgacacgaaatcggtgcctggcgagcccacgcgcgatccgacctatggactgccggcgttgtggatcgaagaaagccagcgcagtgctgcgagccaggctaggtacacgctggtggatgcgcccacggtgttcatgacgcatctcaccgaaatgcttcgtcgcgaatcggcggcgctgctgacgcgcgccgaagtcgacagattgcttgcccgcgtacggcagagccagcccggtctcgttgaagagctgatcccgaccgttctttcctccagcgacgtacagaaggtgctgcaaaacctgttgcgggagaaagtttccatccgccatatcgaagccattctggagacccttgccgacgccggccgcaccacccgcgatgccaaccagctcacggagatcgtgcgccagcggcttggtcatgccatctgccaagggttgctgggcgactcgacctcgctgcaggtgctcacgctggacccagcggtcgaaagccagttcctgcaaagcattcacgcggccactgaggcgggcggggcgcagcctttcgccctggacccgcgcatgtccgagcagctgatgaagcggttgatccagcaggccgaaagaatgatgaagagcaatcttcttccggtacttctgtgcgcgccagaactgcgccgccatgtgcgagcgctgtcggagcgcgtgatgccgcacctgcgggtgctgtcgatggccgaggttcctcacaccatcgagctgaagtccttcagcatcgtccaactttgagacacaagaaagcacccatgagcgacgtactcgccatcagtttgaacagcatgcagcaggatatggcgcgcctggagcgcatcagcatgaacatggccaatgccaccacgcccggctacaagcgcgaggtcgctagctcgctgccggcgggcgcgggggcgttttcggacgcgttacgcgatgcccgggcgagagccttgagcggtagggcggcaggttctgcggcagcgggcacgttgctcgttcagaccgatgccagaccgggtagcctcaagtcgactggccagagcctcgacgtggctttgaccgcagctgggttcttcgaggtttcgaccgattctggcttggcctacacgcggcaaggcagctggcagctcgatgcacgcgggcgccttgtcaccgcgcagggccatcctgtcatgggcgtgggcggcgagatcgtgttgacacggcccaaccccgttatcgatgcgagcggccaggtgttcgagagcaggctcggtggtggagcggagccaacgccggtcggccagctcaaggtggttcgtttcgagaacaccaatgacttccagcgcatgggcgacggactgatgcgcacggagcagcagcccgcgcaagtggcagaggccgatgtccagcttcgccaggggttcgttgagaactccaacgtgagctccatgcaggaaatggcacagctgatccagtcgatgcggcatttcgaatcgatgcagcgggttgcgctgggttacgacgaaatgatcggtggggcggtacgcaagctcggcgaactttcgtaagagctgccgccagccatcttcaatcttcaacggaatacaaccatgttcgatgccctctacatcagtgccaccgggatgcaggcccagcaactcaacgtcgacaccattgccaacaacctggccaacgtcaacaccacggggttcaagaagagcaaggtcgggttttccgacctgatggttcgtgaggctggccgcctcgcgcagacgcaagaagaggctggcatcctgggggccgagagtcgcctgggagcgggtgtcgggatcgcatcggtatcgaagctcttcgacatgggcgatctgaagaagacggagtcggcgttcgatattgccattcggggcgaaggctttctggaagtgaccatgcccgatgggtcgagcgcgtacacgcgcggcggcactttcaaggttaaccgcgatgggctgcttgcaacttccggcgggtttccactgaagtccaatctcgccatcccggacaacgcccagaacctgcagatcgacggcgatggccgtgtgcgtgtgcaggtgggtgggcagagcaccccggtcgaggtcggtcaactcgatctcgtgcgctttaccagcccgtcagcattgctgccccagggcgacaacctctaccgatcgagcacgggctcgggagaagcgattgccggaaaggcttcggaagatggcatgggcagctttgcgcaagggtttctcgaaggctcgaatgtcaagctgacagaggaaatggtcaacctgatggtggcgcaacgcgtgtatgaggccaacgtgaaggtcatgcaggcgtcggacgagatgttgggaatgatcaatggccttcgcaagtagtttgtccgtgcgcatcgcctcgatcctgggatttgcggccatgtcgacgctggccttcgccggaacctcgcccgacagaggcaccgggttgacgagtggtccttcggtctccatcgagctgcggccattggtccgggtcgaacgctccagtgtgcggctgggcgacatcgcgtttcttacggcgcgcgacttgtcgacgctgcgtcgcttgatggctctgcccatcgggacggcccctcggccgggatcaccggtcagcctcgatcgtgacaccattgcgcgctgggtcgaggcccgaagcggcctgcagttcgtggatggcgaccccggcatcctttggggcggtgcgagcgagacttccatcgaaactgcggctcaggaagtgcctggcgaaactgttgtcgaggcggcgcgctctgcgctgctgggctggctgtcgcagcgtagcgtgcgagccgaagtgcaggcggtgtcttcggcccgcgatctgattctgcccgcgggtgtgcctgtgctgcgcgtgcggccccttgcaagtcagtcgcagccttccaggcgcatgatggtgtgggtcgatgcctgggtagatgaccgttttgtgcgcacgacggccgtgaccttcgaagtcaatgcctggacgccactttcggtcgctacggcaagcataagtagcggctctcaggtcgatgcagttttgctgcggggagccaccgagtcgcgcgaagtcgacctcacgagcgtcaagcagggaatgccggtgtctgccggcgccgaactcgacgcgggccggcagcgtttgcgcaagccgctgaaatccggcgaagtgctcaccgatgcccatcttgaatcagcgcctgcggtagtgcgtgggaactgggcgcatcttcaagcccgcagcggtgacgtatcggtcgagagccgcgtccaagtgctgcaggacggtcgcaccggccaacttgttcgcgtgaaggttcctggatcgagcggcgaggtgatcgcccgagtcaccggccccggacaggtcgaggtgcaaccatgacgggcagtccgctccagttctcgcgcgccgtcttagtcgcgctggtttccggcacggcgttgctttgcgcagcgccagctgtcgccgaaagcctcttccaggaaaacagcttccgaccgctgacggcggacaacaaggcgtttcgggtgggcgattcgctcactgtccaggtgttcgagaactcgtctgccacgaccagcgccaacaccggcacgcggcgcgccaacgacatcagcggctcggtcactcagacgggcaatcgggtcgtggggcagctgggcatcggcgtgaccggtgaattcgacggcggtgggcgcacccagcgcgccaacaagctgctggcgacgctgaccgtgactgtcaaggaggtgctggcgaacaacgagctgcgcgttgccggcgagcaattgctcacggtgaacgacgaactgcaaaaggtcaatctggaaggccgtgtgcgtcctcaggacatttccgacggaaacgtcgtgctctccacgagactcgccgacgcccgcatcacctacgtgggcgagggcgatgtggccgaccgcgcacgccgcagcgcatggcggcggatcttcgactggctgggattgtgatgaccccgatgacttctttggcgctgatccgcctgcttcgctgcgcgctggtggttgttctgctcggcgctggctggccggtggttcatgcggcgtcctccgacgttgttcgcgtcaaggatctcggcaagctcaagggctggcgagacaacgctcttttcggtaccggcatcgtgaccggccttgccggaacgggcgactcgccttcgaaccgcacgacgcgccaatctctggccaacgtgctgtcgcagttcaacctgacgatcgcaccggaggccgtgcaaagccgaaacgtcgctgtggtgatggtgagcgccgcattgccgacctttgcccgagagggggacacgctcgacgttaccgtgagctccgccggggacgcgcgcagcctggtgggcggcaccctgttgatcacggcgcttaagggcgccaacggtcgtgtttatgccctggcccagggcggcctttcggtgggggggtaccgctacgacgccaacggcaacgtggttcagaagaaccatcccacggccggctcgatccccaacggtgccacggtggaagtcggcctgaacgccgagatgctcgatgaacggcagagcgtgaccttcgtcttgtccgagcccgactacaccactgcgagccgggttgctgcggccatcaacacccagctgggcagcggcatggcgaaggctcgcgatgcttcgggcatcgagattgcggtgtcgccggcgcagcgtgatgaactggtcagcctgttcacccgcatcgagaacgtgaccgtcgaacccgatcggcgggccaaggtggtgatcaacgaacgcaccggcactgtggtttcgggcggcgatgtgcggatatcgaaggtggccatttcgcacggcgacatcaagatcgcgatatcgagccagaacacggcttcgcagcccttcaatatctggaatggcgggccggacatccgaacggccatcgtcaccaatacgcgcgtcgacgtcgacgaatcgaacgggaccggtttcgtgaccggaagcaacaccgtctccgatctcgtgcagtcgcttgcccgcctgaagaccagcacgcgcgacgtcatttccatcctgcgtgccgtcaaggccgcgggcgcattgcacggcgaactcgtcgtgcaatgagcctcggcgctgcatcgcttttactaccccattcatcaagcatccggagacgaggcatgacagacggaatcgaagccgtgacccgatcggcgctggcaatggcgctggacgccgcaagcctgcgccagcaggcgatcgcgaccaatatcgcgaatgcaaatgccgttggctacgtgccgcagcgcgtgagtttcgaagaccaactcgccgatgcacgacggggcctggcgcaatccggccggctcgacgcattcgcgttgagccaggttagcccgcgcatcgagccggccgcggacaacctgggcgccccggcgcaggtgcagctcgacgccgaagctgcggacatggcacgcaacgccgtgcactaccaggcactggtcaaaggcctttcgcgccactttgcaattctttcaatggctgccggcgacggcaggagatagccatggactacacccaatcctttgccatcagcgccatcggcatgaacatcgagcgcgcccgcgtcgatgtcgcagcgctcaacctggccaacgccaacaccgtgcaaggcgttggcggcaccagctatcaaccgctccgcgtggttgccgaagctcaggccccagggagcgagaacgctgctgcattcagcgcgctcgtcagccaggggctggacgcggcggatactccgcaggggagcccgctcgtgcgcatcgtgccgacgaacgcgccgccgaggctcgtctacgaacccgggcatccgctggccaacgatcgcggatacgtctcgtacgcagccgtcgatacggccaccgaaatggtcagcatgatgagtgcgacgcgcgcctacgaggcgaacgtttcggctatgaacaccacgcgcgtgctggcgctcagggcgctcgatatcgggagcaacgcgtgatggccttcttgcccatcgaggccttgtcctcattgtcgacgcaggcgcaatccctggcggtggcggcccaatcgcaatcgctctcgggcgccgtgccgggcacattgccaagtgccttgacccccgcaggggcatccgtcgcaggctcgttcgggcagatggtgtccgacggcatctcgcaagtgaatagcaagctcatctcgaatcaggtcgacctccagaagcttgcgctcggtgatacgcagaacctgcaccaactgatgatcaatctcgaggaaagccgcgtttccttccagatgatgatgcaggtgcgcagccgcttgcttgaagcctaccaagacatcatgaagatgccgatatgaacttctggcaaggattgacgcagcgcgcgcgcatcggcctggtcgggggagtactggccattctgctggccatgtcggccgcggcatggtgggtattccatactgagtaccaagtcctatttgcggacctgaagcctcaggacgcgcaggcaatgaccacggaactcgatcggctcaagattccctaccgcctgggcgacagtggtacgtccatcctggtggacaagaccaccgtgcatgccacccgcatcaagctgatgggcaaggagcttccgttgcaaggcacggtcggcctcgagttgttcaacaacaccgatttcgggatgaccgaatttgcgcagaagatcaactatcagcgcgcgctgcagggagaactcactcgcacgatccagtctctctcacaggtgcgcgaggtgcgcgtgctgctggccttgcccgagcagggcttgttcaagcaggcgacttcgaaggccaaggcgtcgatcacgctgacgttgcgccaagggcagacgctgcggcccgagcaggtgaccggcgtgcagcgcctcgttgcagctgccgtgccgggcatggccacgcaggacgtgacaattgtcgacagccatggcgtcgcgcttacgcgagcggaaggcggcagcggtgacctcgaaatgagcagcgcgcggctcgatctgaagcgcgacaccgaggcatacctgtcgcgcaaggtcgcagccgtgctcgatcgcagcttcggcgtcggacaggcactcgcgagcgtcgatgtgacgctgaacatggaccagatccgcaccaccacggaagacgtgctgcctgcagcatcgcgctcgggcctgcagtcgaccggggtcgtggtacgcgagcgggaagtgctgcgtgatactggcgcggtgctagatgccagggcgggcgacgctggcgggccgcgcagcggcagcgcgcagcgggacatcgaatatgcggtaggccgccgtgtcgagcaggtggtcagccagccagggtcgattcggcgcgtccaggtggttgcagtggtgcgcaagatgctggactcggggcaggaagatcaactgcgaaaggtgattgccgccgcggtcggggcgtcgatcgaacgcggagacacggtcatcgtgcaatccctcgctggcggcgccatcctggcgcctgatgccgccgtcggcgcagcggccggatcgcgcgcagccctggcgcccgatgaggccagcgaagcgccggtttcagcgaattccctggaaaagtccagtccaacgccattgcagtggttgctgggcggcgcattgattgcaatgctggccgtgtggctgcttcgaaccggacgacgcggtgcggctgtgcgtgaaacggctcaaggagcggcttctctttcggaggccgagcgcgcggcggcgttgcgccgcgtgcgcgattggatgcgtgaaccggtctccgcaccagctggaaccccctcggcatccagctcggccggagcgaggaggccccattgatgatgtcccggcatggttcgtcgctgaacggggaagagggcacgggtttgtctgaaaccggcggtgcgcgtcatgcggcactgctgctgcacgccatggcgcccgccgatcgggcctggatgctcgatgccttggacccctcggagcgagaaggcctcctgaggcttctggcggaactggaggccctgggcatggagcgggatgccacgctgatcgccgaggccacggcgagtgcgtcgcagccgccaccgttgccggacgaggcgatacttctggcactcgacggatcgcagttgcatgagttggttcagtgcttgcgcgccgagtccgctggtctgatcgcacgctggctgcatctggccgactggccgtggcgggaggaattgctggccgcgttggagccggcgcagcggcgacgcgtcgatgccgccttgtcggcaatgagtgccgaagattcgacgccgccagccatgcgcgctgccttgatcgaagcggtagcaacccaagtttgcaggccagtcgccgcgcgcgagcattcaggaaagccgtggcgaaagctgaagccttcgttcgatcggctgttccgcggccgctgggcgcattggagggccggcacgtgaccgagaagatgccgcagccggcttcggccagagagcctatttccggcgcgcctgcgcgcccgagcgtggtgttgcgcgacgtcgtcatgcaggggcacgtcgcattgacgcggccccgcagccgcggaccgaacgtgcagccgttgcaggcacggactcaagcgacgaatctggtgccggtccggccggggcgcaaaccggaagaggaaggcgcgaccgttgcagccagtgcattcgtccgggccaacgtccccgcggcgacggctcaacccgacgaggaagcccggcgaggctatgaagaaggccttgccaagggcatcgccgagggacgtgcccgcagcgcggaagaggctcggcagctggccgtgcagacggccgaaaaggcagagcgggaactgcgtgagcacgccgatcgcctggcgcaggaactgaagcagcaagcccagtcggcctaccaggcacgtgttcaaacgctggacaacctgatcgccgcggcaccgccgcagatcgagtcgcgtttggctgctgcgcaagaagacatgctggcgctctgcttcgaggtcgtctgccggatactgggcgaacgcgccgcaatgcccgaagcggtgcaggcgcacctggagtacgctgtcaacggtctgcgcagccgccggctggtggcggtgcatctgcaccctgacgatctcgcggcgcttcagaaagcgcagagcgatgtgccgtctgcccgctggggcggagaggatgtgcaatggatcgcaagcccggacatcgcgctgggcggatgcgtgctgcagtcgcccgaaggcggactcgatgccaggttcgaaactcagctcaatgcgctgcgggacctgctgcttcaatcgcgcgcgtccctgcgttcgcggaactcttgagatgaacctgctcgccgtcagccgcaaggcactccagggtaccgatctgcgtcgtcgaatcggttgggtgcgcgagatgcaggggttggccatcgatgcgctcgggcccgatgccgccgtgggcgagctgtgccggatcatggtgcgctcgcatggcggcccggcagcaggcggcgcagtgtcggccagtgtgctggccgaggtcgtcggcctgaagcccggccgggtcacgctgatgccctacgggtcggtggagggcattgcagcagggtgcgaagtgcatgcgctcggtgccgattcgcagatgggcgtgggccccgccatgctcggtcgcgtgatcgacggttttggtgaaccgctcgatggtttgcccaagccaattgcaatccagcgtcggccgctcaaggcgccgccgatcaatccgatgcagcgcccgccgatccgcaacatcctggaaacagggattcgagccatcgacggactcttgacgctcgggcaggggcagcgcatcggcatctttgccggaagcggcgtcggcaagagcacgctgctgggcctgctggcgcgtcacgtcaaggcgcagggcggtgcggacgggaacggtggcatcaacgtgattgcgctcattggcgaacgtggccgggaggtgcgcgagttcatcgagaagcagctcggaccggaaggcctcgcgcgttcggtcgttgtggtagcaacctccgatcaacccgcgttggccaggttgcgcgctgcctatgcggcgctctccatcgcggagtactttcgcgatgagggccaaaacgtgctgctcacgatggattcgatcacccgctttgccatggcacggcgcgaagtgggactctcggctggcgagccgccgaccgcacgcggctatacgccctcggtgttcgccgagctgccggagctttgcgaacgctgcggcatggcgccaggcggcggatcgatcaccgcactgctcaccgtgctggtcgagggtgacgacctcaatgaaccggtatcggatgcgttgcgcgccattctcgatggacacatcgtgctgtctcggcagctcgcgcaccgcgggcactatccggccatcgacgtgctcaaaagcgtgagccgcctcatgcctgagctggcggatgaaagccaacgctcactggcagtggcggcgacgcagcacttggctgtgctggagcgcaaccgccagatgatcgacatcggcgcctacgaaaagggctccaatgccgaactggaccgggccatcgataccgagcccgggcttcaggcatggttgcggcaaagcgtgggtggtgttggccgcatggaatcgatccacgacttgcgcgccatcctggctccggctgctgaaggcagaaaaccatgagtgccgggaccacggttctttccgcggcggtgcgcgacgtcgacgtacgcggctttgtctatccgctcgagcctgttcgccagcggcaacagtggaggctcgacaagtcgatggcagaactcgcgcaggctcagcaggtgctggccgacacggaggcgcggatggcgcagatgctgaaggcacatgacgagcaggctcgaacggtcggccaggcaatgctcgagcgcctcgaccccctggcccacaggcgaaccctggtgtatctgacccacctgcgcagccaatgggcacaacttgatgcgcagcgcgaggaacagcgccttgcccgtgaccgcctgcgccaagagtgcttgaagcagcagatgcgcctagagggactgaccaggcataaggagaatgcattgaccgaatacgcggacgaagttcgccagcgcgccagcaacgaacaggaccgcgactggctcgcacggtcggcttttgcgcacgctgcaactggagcaggccaatgactcccggcgacaacatcgcagcgccatccggcatggcttcgccggtgcggcgaaacatgccacaggcgacaactgccggcgagacagcgcagcggcagctggcatggcagcgcgagatggaacgagcccagatggctggctggttcaagccgggcgccgtggacacgcaggaggcctcggcacctgccagccagaggccgcagcaaagtccccaaggccagggccccgaacagcaccgcgaaagccgtggtcctgcacagggaaaaaggctgccgccaaccctcggcgtatcggtggccaccctgcgaccgggtttgcagggcagcccccggatgtccctgaacggcgaaacggctgcaggcattccggcgccgcgcacggcggcaagcgctcttgtggaacgacaacccgtgtccgagttcgattcaaccgcggaaagcaaattgcgccccgaaattcgaacgttcgaacgtctcgggccgcgtgcagtcggggcttctgcgccggaggccgccgcttcacaggacgaggcgacggatgttgcggcagtaccccagtcgaaccccgaaatttcgctcgcgccacttcggctgcatgaagaaacaaggcggcacgggcaggccgtctggatcgccatgcgggcggacgaccagacgctggtctcgatgttgccgcgactcgtttccgatctcgagcgcggcatgcgcgaacgaggacagcggctgcatcaggtggtgtgcaacggccgcctggtctggcgcgatggcgtcgagatgctaggcggtagccactcaaatacgttcgattcaattgaccccaaggaggcgtgatggccatcgatgcaattagcggttccactgcaaccaacctccaggccagcagcctgggcatggaggatttcctcaagatcctgctcacgcagctcacctaccaggatcccctgaagcccatggacaaccaggagttcatggcgcagatggcgcagttcacgagcctggagcagacacagcagctcaacaacaagatcgagaccctgatcaccaaccaagccgcgctccagtcggtggggctgatcggcaagacggtcgacgtcaacacgtcgaccggcgccgtcaccggcacggtgagcgcgctttcgctctccggcgacgcgcctcttttgactgttcgcacggccgcaggcgccatgctggaaaacatttcgctgagccaactcgcggcagtgcgctgagcgcagcagcctcaaacttcgaagggacgacccatgcttgaatccatctatgtcggaatgactggactgctgggctactcgcgcggactgcgcgtcatcgccaacaacacggccaacatcaacacgcctggcttcaagagttccagcctccagttcgccgacatgttctacagcggcggcaatcttggcggcggcggtgcgggccagaaccgggaccaggttggctttggcctcagtacggccgggacatcgctgtcgttcaagcagggcgaactgcgccagaccggcaacgacctcgacatggccgtcgacggccagggcttgtttgccctgcaggacgcgaacgggaagaccacctatacgcgggccggccagttcaagttcgatgccgacggtacgttggtgagccgggtcaatggcgagaaggtcatgggtcttgacgatcgcggcggcctcgtggccatcaccttggcgggccagatgatgagcctgggccgtcccacttcccgtgtggagttttcaggcaacctgtcgaacacggtcaccgagcagaccatcggcggcataacggtcgtggatgctggtggtgccagccacacgctgaccatgaagttctcggtcgtcagtgcggccgagagcggcaccacgatgaaggtcgagctgatggatggaaccacggtcgtgagtaccggccagatggtgttcgtcggcggaaagccgactcccgagaccgcgatcatgcaagcgacatacgctcccgcggggcaggcgccagtggcgttgacgctggatttcagttccgacgtcgttctttttgcggggcagacctcgctcaaagtcgattcgcaggacggcattggcccaggcgcactgagcgggacgaccttcgatgccagcggcactctcacgctgaactattcgaacggttcgaccgtcaagggtgcccgcctggcccttgcgcgcttcgactcgcccgatgccgtgggatccttgggcgacaaccagttcgaacagctggacgagaacgcgtggcacttcggcacggcgggcgaaggcgcttttggcaatgtcagctccgggcgggtcgagatctcgaacgtcgacctgtcacaggaattcagcgatctggtgatcatgcagcgcggctatcaggcaagttcacaaatcatttcgactgccaacgacatgctgcaggaactgttctcgatgaagagcaaatgaacgactcctcacttctcgatcttgccgagtcgatgcgcagggcgcggcccttgcgaagctggcaaggcgcttcaaaggagacactgcgtctgcgtcttgccgcgcttcatcgggcgtggagcgacgagtggcttcccgcgcgccaggattcgttggcggacccggagatccacgtggacgagcccggtagcaccacgggcccggcgtcggaagacatcgcctgctgggcgttcaccgcggcggaacgccgcgtaccttcaagcttgacgggcttcgagtcggcacccgctgccgcaaaggaggcatcagccgcgccgttgcgcgccatcgccggctgcatgttcggatccgatgcagccgtatcggcacaaggccccgccaaaatcgcggccgtcgtcgcgcgggcagcctgggccgactggttgcgccgcaacgaagtcttgctggccggtttcgggctcgagccccaacagtccgaaggctcacgcggcgccagccccctctcgaatccctggtccggtgcgctcagcgtgcgctggccatggtgcggcggtgtctggcagctcagcttgccgcatggtgccgttgcggcgctgcttggaagcgagtctgcggccaagccgccatcgcgccccagcgaacacctgttgccgaaagagcctctggaccaggccctggcccatcggcccgtggcgttgcgcgtcatgctcaagggggcggagctcaatctgggccaactgcagcaactgcgggtcgacgacgtggttccgctcgagcacctgctcgatgcaccggcacaagtggttggcgcagatggtgggcgggtatgcgatggctggcttgggcaaagcgacggccgaattgccatcgaattggccgcacctgcgtcttccgcggcaggcatggacctgcgcatcaacactcaacaatcgaaggaaggaaaacaatgaccaaagccttggaaggaatcgccaccgacaaccgtgttggcgcatccggtgccgcagtcgagacgcgcggcgagagcagggcgcgcgccgcgcagggtccgggcagcttgccgaccgcgcagatcatcgcgctgccggatctccatgccggtgccgagggggatgccgccaaccaaggcggcgatgcgtcgatcctcaaggactggaatccgcttcaccagatcaaggccagactgcaggtctgcgtgggcgaggtcagcctttccgtcggcgagctgctcggtgccaaggagcaccaggtgttgcggctcgaccgggagatcgatcacccggtggacttgaccatcgagggcaaggtggtcgcacgcggccaactggtcgcggtcgacgggcactttgcggttcgcatcaccgaactgccggtggcgctgggcctgacttcgggaagctgacggatgaatcaagcgcagccgcggttggccgtggtcaatcgagccgccacgtgcaggtgggtcctggcgtgtttcgccatcgcggcgggactgctgtgcgctgtgccggccagtgcgcaggaagcacagagcggtgcagttgcatcgagcggcaacaccagcttgccctccagcatcccggtcaagcgggatccgccgggcgcgctggaatctgacgtgggcgaccgttggtggatcgccattcttgtggcgggcggactgctggcgtacggcgtggttgccatgcgccgaaaggcaaggtcgtcaggaaagcgagccggcacctggtggccggggctcggcggcctgctcgataccgggtcgtcccatgagatccaccgtgtgtcgagcacgcacctgtcgccgcgccacggcctccacgtcgtggtgtggaacggcaagcgcctgctgctgggatgcaccgatcaatccatccaggtgcttgcggagtctgcgtcatccgtgaccggcgatgaggccgcgccgttggcgccgggggccgttcgatgatgcgcgcggcacctgcagtcggtcatcgcacgccgcggccgtggggtttgattcttgccgtggtcctgctggtgattggcctgatcggctggcccaccggtgatgccagggcgcagatgcccggcgagacgagttcctcggagcccgcgaacgtgccggcacctggaactgcgccggagattgcccccgcggcaacggcaccctcgacaaccgcgccctccgtctcggcgccgcccccttccgcgccgaaggctgcgctgcccgccgccacgtcaactcggcctcggtctgcggccccggccgcgccgccggtcgtgggcgccgcaacgccggctaccgaaaccgcccaggccctgcgcgtggtgctcggcctcaccgtgctggcgatcctgcccgcgctgttggtctgcctcaccagctttctgcgcatcatcgtcgtgctgtcgatgcttcgccatgccatcggcatgaacgagacgccgcccaacaccgtgctcatcggcttggcgctttttttgacgctgttcaccatgtccccggtgctgcagaagcttaaccaggatgcattcgagccgttcatggcgggcaagctctcgatggaggacggctacagcaagggtattgcgcctttgcgcgagttcatggtccgccagacccgcgaggccgatctggcgctgatggtcgagctgtcgaaggcgcctacgcccaagtcgatggaagacatcagcaacgttcagctcattccttcgttcatgctgtcggagctgcgcgcggcgttccagatcggcttcgtgatcttcctgccgttcctcctgatcgatctgatcgtatcgagcattctcatggcgcttggcatgatgatgatgccgccgaccaccatcgccctgccactcaagatactgatgttcatcttggtcgatgggtggagtctccttctcaaggccctggttggcagctttcactgacacacgccaccccaagcctcaccgtatcgcgcaatgtcacgcctgagtcccacgctgccgcccactgccccgccgttcttcggcctggcggcggatgcggtcgcgtccgtcgaggccgtgcccgaggcgcccgacctcgccggcactctctgggagcgctggcgcaaggatcgagacgacgccgtgcgcaacgacctggttcgacactatctgccctatgcgcgaatgatggccgccactctctacggacggcgcacccacgatgacgtcgagtttgccgactacctgcagcttgcacgcattggcctcatcgaggcagtggaccgcttcgacccgacccagggtgcgcagttcaagaccttcgcaaccaaacgcgtgcaaggctcgatgctcaacgggctgatccgcctcaccgagaagaaccagcagatcagcatcagcatgcgcttgcgccaggagcggatggacgcaatcaaggaagcggctgcgagcgaggtcctgggaaccagcgagaagggagaggccggtgcggccgcgtcgccgcgcaacccggacaagctgttcaagtacctcgctgaagtcggcattggcattgcgctgggagtgctgctcgagggcaccggcatggtcgatgccgaggctttcgacgaccacgcccacgcaccttcccccgaagtgagctacttccggaagactgagatccttcaactgcgcactgtgctgcatggtttggtggatcaactcagcgaacagcagaaaaccgtgatccgccaccactacctgcaagaaattccgttcgacgaaatcgcaacgctcatgaaagtcacgcgtggccgcgtttcgcagttgcaccgccaggggctgctgcgcctgcgcgagttgctgagcaaagatgggcgcctggacgtctcgtggtgacacgagcgccccggcctggacaaccaaattcattcctctccatgacagacaccaccgcaaccactgctgctcccccttcactgcgggacgatccacgcatcgtggccgcgctccggcgcctcgaccggctcgatggctttctgcgcgaagacccgtcgaacaattcgctgctcatcgatgctttcgagactgcgctgtcctgcggggaatgggagcgcgcggaatttcatctgcggcatgcccaatcactgcagtccgacccgctggcgtggcgcctgcgcgaaggcgatttctggctcgcccaacagcgctacgacgaggccctggccgtgctcgaggccttggccgacacgccccagccgccgccaggctttgcggacgtgctgctgcacaacctggccttcatcgaactgaggcgaggtcgccatgcggagtgcgtcactcgccttgcgacggcactcgaagcgcaggctgcgccgtcgacgagcgacgcccccgttgcggcacgcgccctgcagcagctctggctgcgatcgctgcatcacgacggccagctcgaacgtgctatggcctggaccgctggcgccgagcaacaaggccgactcgatccccaggcggctggcattgcgagcctgatcgccatcgacgcctcggactttgccgccgccgagcgctggtcgaatgccagccttgccgcgggaacgcctgccgagcagccggtggaggcctttgtcaccaaggcttcgctggcactggccgcacgcgatgctgccgacgccagccagttcgccgatgccgccctgcagcgtcatccgggcgatggccgtgcctggtccacgcgcggctttgccgccttgctggcgggtgacctgaacggcgcacacagcgctttccggcaggcgctggccgttatggcgcagcacatcggcacctggcatggcctggggtggacgcagatcctgcaaggcgatctggcgggggcgcgcgagagctttgagaccgcgctggcgctcgaccgcaactttgcggaaagccacggtggcctcgcagtcgtgctggccatgcagtcgctgcgcacggaagcgcaagagcacgccgagttcgcattgcggctcgacaaggccaacctgtcggggcgctatgcccaggcgctgttgagcggcgaggtcaaggatgcgaaggacgtgcagcgctttgcgcggcgcttgatggggggaaggcccggcccgcttggcggggacatgggcgacatattcgcatcgcctgatgcaccaccggaagcgaacgattaattgattgactcgcgcgcgcagttgcgccggccggaacgttagcgcgaggggctcggcccaggttgcgcatccgcgagcagaagatcgcccgcttcgcgcaaggcggcgtgcagttcggcatcgccttccatccgctccagaaccgcgtcgaccatctggtcgaaccccctgtcgtcgagccgttcgcggccaaacgcctgcatcagcaccgattcgaggaacagccggaaggccttgcgctgtcgctgcggatcgtcgggggacagcgcacgcacgcgcagggccaccatctgctggatctctgcgtcggtgctgttcgacgcgggggagggcgactgcggctgcttgccgccggccgttgtccgcgcaccgtggggggcttcgcgcccggccacgccgcgctccctggcctgggcctgcgcccgaaactgcgcgccgaactgcgcacgaatcatcgcggcgagttgcgtcgttggatcgatcatagccaaggcgtgcagatgcgttgcgaatcaatcaatgcgcgcggccttgctgatggtagttggccagcagcacgtggttcgaggcttcgtcatcggccatcccgacctccggcgccgcggcagcggagctctcagtcagggctttgatgccagtcactaccttttcgatatcgtccgacagtgcttcgttcgtggtgttgagcgccagcccctgtgcgtaatgccgcagggcttcgtcaaaatggtcttgcgcaagggccgcaaagccgttgacgaaatgcggcaggggatcggtggccggcagatcgagcagcggctgccaggtgagcagggcgatggccgcgcggccggagctgaactgcagaaggccgagctggtagcgtgccatcgggaagccaggggccagccgcgttgcgttggcgaaggcggcctcggcctgagtcatgtcgcccagcgccgcaaactccgcacccagaaggaactggggcagggcggcgcctggatcggcggcgctggcctgctcaaacaaatcgatggcttgggggccgtcgttggcctggcttgctgccatgccgctggacatcagggcatcgaacgaattgggttctgagctttgcatcgatcggtctttggtgggttgttgtgcatcgagtctttacggctggtgaggtgtcgaggcaacaaattcgcaagcggtgctgtcgccgcaggttggattgtcgcgcggagttgggtgtgagcaaagcctcggtcgatggagggcgatgcgggtgcagggctggtgatattggccgaaacgcacagcgcaagaaacatctgacattggactaagtcgatcagaccaaatactgccaggggcttgcgccagacgcttgctgaattcacgtggctctacaacaccgtgcgagtccaccacaacctcaagggctgaccccgatagaggcatggcacggccggacgctggccgactacgttcgatgtagatagagacgcaatgagagcacgaacgaaccggtcaacgagtcagcgtcgggacgggagccagagatttcagccttgcatcgactccaaatgtttgcgccactcatcgagcaagccaacttgcaaggtcgtgtcgacttcgccatccacgatctcgcccacgaatatatccccgtacatgaactcgaacgtgatgccagttcgttcggatagctcgcgcactgcttcaaccacatcgctgacctcggcgtagaagacggcttccacatctttgggaacgaggccaggaaccttcgaagagcaaacttccatctcggctcctaaggtttcagttggctcgtcgccttcttgtgtagccaggtcctcgatgacttcaaccaactcaggcgcaccaagaagccaacttcggcgctcgcgcagagtggggacgaacactctaatttgttctcgaatctcgggggtaatcagctgcgcaacgtagaacagcagcttctctctcggcaaggaacgaatcacttcgggtgtcatgggctacctacttttcctgtttggccggatagaacggaaccgcggcaccgggaccgccaggattgaatttgaagcctcccggcatgtgggcttgcatatggcgagtctttggcagaggcactgtgacgggcaaacctgcaatatggtgcggggagatcagctcgcccataagaccagcgtcctcggggaagaccttgacccatgcgtcatccactttcggccttaagctctgtttgatcaacgttctgtttgcgtcactaagaatctcgccatagccaagatcgtcccacagatctcgcaagttgcgcatgtcagccgcgttatttcggcgtatccccgcgcgagtggtgttcgatgatgagccgaccggctcggctacaggctccgctgccgcagctcttctcagcgttgagtaaatgccaacccctggaacaggcgccggcaatcctccaatttcggccgtgcgcagcgctacggacatgatcgcggctcgaccggtggtagtgcccaacgtggcctgagcaaggaagttgacgccgttgaccagcgctgtgcccgctgcaagagcaatccggccggccaacgtgacagccctggttgcgccggcaccaacggggaaggcgagcacactcgcaacgtccattgcgttggacttgacgccgccgaactggaagccgttgtatggcttgccgtcgtattcgacagaggagcgcgccatcgaatccaggttggccgtgatccgatcagagtcgttggccagagcaagcatgcccagcaacccgcccatagcctccgggcttgtacgaatgccgtgcgaaccactcatcgccatcgagagcgccacagcactttcaggcgatggattgctcagcagcgttcccagcgcaacccccgcgttctggatcatcggcggcttgagccagccgccctcaatggtccacgcctcgtagcgcgagatcagggcatcgcgtagcttcgggttctgggcggtgtactccaccacttccttaaacgcacccaagctctcttggtaaagctctgaggactgctgctgctggacgggagtcgcgtattccggcgcacccgtctgcgtggcagtcaagatgcccgaccaagccgaagtaaagcgggtcgtcggactcggccggctctgcaccggtcctgcgacgagcgagacttcctccaagtcgagcaacgtaggcggctgactggaggcaccagctctccccgcacccattactcgggttgggctgtccgtcatcgcctccgccaggcttgaccccaatgcattgccaaacgcgtcagttgcgacttgcgtgacgctgaccttgccgccccggagcgccgtcgttgtcagcccggcggcaaagcccgccaccgttcctcgcgccaagttggtcgcaaagccgccgcccaagctgctgaacgcttcaccatccctcagagcaccaccgacggctgcgcccatcccagcgccggctgcagtagctgcgacgctcttccagttgaagctttgctgcagacctgtcgcgactgcaatgccctgggtcagcgagctcccaacggctgatcgaatgattgcatttccgaccagcgcatccttacccagagggctccaggcacccaagccgcccgatacaccgccgctaattgcggccagtgccacgcctttccaactgaaggagtcctgcgccccgatcgcgatgccaacgccttggctagcaatggagccgactgcagcaccaaccgcgcccgctacaacggcgccggcgccaccggccgtcaagacagcagttcctgcagccatggtggctccgatgctgccagccccggcagcagtggcagcacttgctgccgttgctgcagttccagccgcagcacttcccgcgccaccaacagctgcaaatgcccccgccgtatagatggtcaccaccacggcgataacgatcatgatcagctgaccgatcccgccgcacccaccgccttccttggcctgcggcatcggcatgttgggattggtatccccaaccaccttgctcgggtcataaggcttgaagctgttcgcgttgttcgccgctcccaccttggtgggaatcgtcagcacctggcccgacttcagatccgcattgcccgacagcccgttggcgtccgcgatcaggtaccacagcccctcgtcgccataagccccgcgcgcaatgctctgcagcgtgtcacccgcgctcaccgcatacgtgcccgggctggccgacggatagctgccgtcgatcggccggtacccaaaattgaactccgccttggtctggaacagcggcaccccgttgggcgcgctcgggttgttcgcatcgcggatgcgcccgtactgccccagcacctggccattgaccaccagctggcgctgctcctcgcccgaggccaggtagcgggacgacaggatattgccctccatgtcgctcacgaacgtgcggttgttcagcggctgcgtcacgtcgcccacgcccgtgagctcgttgccattgccgtagtaccagttcgtgcccccgggtaggttcacgttgctcgtgcccaccgtggccgtctggcggtagccctcggcgcgcccgtaggtgttggcgtagttcgtcacgctgggctggcccaggaaattccacaccgtgtagcccatcaggttgcccgcgccgtcgtagccgccggccgttcccatgcccggcagggtgggaggcgtgccgtagccgatggtgtacttgcgcccgttctggctgtcgaacacgtcctggcgcgtgatctggccgttggcgttgtaggcgctgatgcgcgtctcgctgccggtgcccgccagggtctggccgttccaggtcgtgcccagcagggcgttgacatagcccacgggcagggtgcccgccgggccggtctgcaccacgcggctggcgccgtcgtacaggcgcgcatcggtctgcacgccgtcgcgcaccacgctggccaggcgagcgagcgcgtcgtagcggtagtcctcggtggtgtagccctggctggtcacgtactgcttggtggccgtgctatagatggccgcgccggtcatcgggtcgtagccggtgatctggctctggccgtccaccgtgagcacgcggttgccccaccaggtgtcgctggtgcggttgccgttctggtcgtagacgatgcggtggccctggccgcccaggttgccggccgcatcgaccgcgttgaccaccgtctggcggttcatcgcgtcgtactggaagtacaggtcgctgtccaggctggtgtcctggttcagcacgtgggtcttgatgcgggtgcggttgccaaccttgtcgtactcgatgttcacgaacgcgcggccgtcggccacccagcgcatgcgccccagggcgtcgtaggcgatgtggttgtccttgtagaccacgccgccctggccgaaccattcgcgcacgcggttgccggccaggtcgtactcgtagcgggcgtcctggcccgtggtgcggtcgtaggtgcgtgccagcaggccttcgatgttgtaggtgtactcgcggttggtgccgctgtcgaaggtgagctggccggccttgtcgtaggtgtaggcgtaggcacggccgccgtagtcggtatgcgtgagcaccttgccgaagtagctgtagctccaggtggccatgtagccgttgccatcgacctcggcgatcttgttgcccagggcgtcgtaggccacctgggtgctctggcccatgggctggatggtgcgcaccacgcggccctgcaggtcgtaggcgtagcggatggtctcgccgttgccattggtctggctgagcttgcggccggcctggtcccaggtgctggattcgacgatggcccgcgtgtcgaccagctgcgggaggttgttggccgtgttggcattgaagacctgcaccacgccgcgcgtggtcgtgagcaggcggcccaggttgtcgtaggtgaagcgggtgagcgtggggttgctcacgagcgcatcggtggccgagaccttgtcgccgaagacgttgtagctgttgcggatcaccccgccgtcggcatgcagttcctgcgcgaggttgccgcgcgcatcgtagacctggccctgcaccttgccattggcgtccttgatggccacctggcggcccatcttgtcgtagaacagctgggtcacggcggcacccgatgtgccctggatgccgttggcatcggtctgcttctgctcgatgagctggttgttggcgttgtagcggtaggtggtcacccatccggccgagcgcggatcgctgatggaaatcacgttgccccagcggtctgtgttctggttcaccacagggcgcggcgaactgctggtgccctgcgtgaccggggtttgcaccgcgttggcgccgtcggtgttgttctcgctgaccgccgagctgcccgctaccgtggtggtgctcgaggcaaagagcgcggggatgagcggcgtccagtagcccggtgtgtagggcggggtgctgtcctggaccgagggcgtcgttgtacccacctgcacctggtagctgtaaggcacgtactggtagcgggtttcatacaccggctgatagccgaggatgacgggcctctgcaccgcaacctggaccgggtaggtcacgttctgccagccggtgattaccaggtagttgtcgtacacggtccgatagcgtgtctcgtagaccgttgtgtactggatgttgccccatgcatcccgcacgacggtgacgttgccctgctcgtcctgggtcgtctggggcggaccctgcaccgccacctggtacgcctcggtgcgcggcacctgcacccatccgtagaccggatcggttcgggtctggtactgcgtttcgtagacggtctcgtagatgatgttgccgttctcgtcgcgcgagtagacgggctcggacccgatctggaccaggtacggcaccgcgctcacgcccgagcgcgtttccatgatgggcgttttctggttgtcgagaatgcccgtcgcctggcccaccgactgcgtggttccgcccgaggtgagcgttgccaggatctggtattcgtaacgcccggcggcaaggttggtgatgtcgacctgctgcgagccgatcggaaagctcgactcgttgctgccggccaggttgaccacgggcagcgaactccaggcgctgccgcccacgagccggtactggaaagtcacgccattgccggcgttgaggacggacgagtaaggccactcgatcatcgtgagcggcgtgccgatgggggcgcccgactcgtcattgccaccggtgccgacgatgcgtatcgcggtgccggtgatcactggcagattgaccggcggaacccattgcgggaaggtgattccgctcgaggcgatctggcctgttgcgtgggcgtatggcacgccttcgcccgaatgcgtccagagcagctcgtagtcgtacgtgcccgcagccagcagggtgacgtccacgccatctctgccgttgccgcgggccgtgacgggctgggatatccaggcgcccgtgctgccggccgcccggtagcgaaagacctgttccacggatgttccgggcgatgaccacgtgaacaggccgctgctggttgggcccatctggtagaaggccagcggaacgctgatgagggacagcggcggcgaggccagggtcacggtgccgctggcggtcacgctggccacgccggctgtcgtggtctgcgtcacgcggtactcgtagctgcccggtggcagggcggtggcgttgtagcgcagcaggtcgccaaagttcaccagcggggcatcgacccagccggtctcgccggtgctgcctgccgggcggatctgcatccgcatgctggttgtgaggtcgtccggcgcatcgacgtcgatgacctggccgctgtagcccagcgatccctcgctgatgacgggctgccagttgccgtagacgtccttcttgtagatggtcagccgcgacacgcgcccgatgccgccgtttgcgtcgttccagccgtcctcccaggtcatggtgaggctgttggtgttctccgccgcattggtcacgatccgggtttgcgtacgggtctccccacctgccatcggcaacgggttacccgattcgtcggtcatgatcggattgccgttggggtccagcaccggcggagtcaacgaataaacctgggtcgtgtactccatcacgaccttgatgtcgccgctgccaaggttgcgcaccggcgaccaggccagatggacggtattcgtaccggaccgcccgttgactgttccggtctcttcgcgggtcgggttgctcgacccggcgacggagccctggctgaacaggcggctgatctgggcgccgcccgtccattcgctgcgccgaggggcgatggtcgaggtgacgcggcccagcgcgtcgtagatcgtgtcggtgcggcgaaggtcggccacggcgaccgagtcggggttggtgaaggcccgcagatccgcgttgcccgatgccgtgccgtagctcgtgatctgggcggtttggttgcccagaaggttgtagagcgcaaccttgtcgacgccgtcacccgaattggtgcgccagacgcggccggcgttgtcgtagtcgaagtattcctggcgcccgccgcccacacccttggctgtcatttcgccaaaggcgttgtactccattgcggtgtcgatcaggccagcctgcgcttgcgagacgatggcgaccgatccgccgctgacttggctcctggaagcggggtcgatgacgtgcgtctgctgtccgagcttgtcgtactggtaggcgcgaaagagggtgctcgagacgttgtcaccgtcggtgaccagttgccattccttggcgacgttgcccagggcgtcgtaggagctgtagtgattgaagccggccgcgtcggtgttctgcgtggcgtggccgagcttgtcgtactgggtgtacgtgatgcggtctgggttgatctgcgagttgtcgtcgatattgccgctccagacggcaccaccgctggcggtgtagagcacgaggttgccatcgccctgcatgaccaggttcgtaccgcccttcgcataggtatcagaactccagacgaccccgttcgggccgtacagaaccatgttgccgtcagtctggaaggcgaaattgttcgcaccgctcccggcagtctgcgaattccacagcgcctgcatgttgtcgtggcggtcgtagacgaccagattgccatcggtctgcagggtgaagtagtagcggccgtcaggcgaatagatgccctggccgggtgcaaggttctgcccgggggcgagagtgctggccgttggcgcactgagtgcatcggtagcggctgtggccttgtagacgtgcgtctcggtcttgacgactacgttgccgtaggcgtcgcgttggtatttggtaacggccgtcaggagcccgttgctcgtcgaaggcgctgccgtggcgcgcacgcggccgagggcgtcgtagtagctgtacgtggcggcgcccaatgcgtcggtcgtccgcgtcaggttgccgaccgcgtcgtacgcgtagctggtgacgagattggcgcgcgcgctggtaccgttgctgctcgcgctgaattccacgctgacgcgggtttcgctggtcttgcggcctccgcgatcgaacgcaaagattgtctggcggtcattggtggcatccaccgttgtcgtcggcactgcgatgggcgcactggccgggttccatgccgcgacggccttggcaaactcggtgcggacggtcacgttgcccgcgccatcgaaagcctgggtcgtcaggtagcccagtgcgtcgacgctcgcaacctgctggcccttctggttgtagtagttgttcgtgtaggcccaggtgttctgcccggcattcttgagcaagccgacgcgcgtgaggtcgccaaaggcgttgtaaacgttgacggtcgtgcggcctgccgtggcgtactgcgcgcccagcgctgcggacgagtcgtacgtataggtcgaggactcgatgactttggtggcgcggcccgctcggtcgtaggaggtggtaagcgtgcgatcagcgccgtgattcacgcccgcggcattgaccgcagcgctgacctgggcggtgctcaggcttgccggattgccgctggtgagcgtggttccgacgccaaagcgcttgagttcggtgacttggctccatgggttgtactggtagctcgtgacgaaccccaatgcatcgacctcgtagccgatccggccaagcagatcgtaggtcttgtagctgaagctgcccgccacgtcgcgattggcaatggcgtcgccgaagacgttgtaggtcgtcaaggtgtcgagcgtcttggtcagctcggtgcggctggccaggccgccggccccattggtcgtgagagcgtcgcccgccgggtcgtagacgctgacgggtgggtagatcacccggacctggtggccgacggcatcgtattcgtagctggtggtgcgctgctcggcgcgtccgaccgcctcggtgcgcgacgtcaggttgcccagcgcgtcgtaggtcatctgggtcacgatgctcgcgctgcccgaacgagtcgcgtcgaccacgagcttgccgctggcatcggggacgacggtggtcacctcgacggccggtgccgtctccttcgtcatccgtccgcccgcatcgtaggcgtaggtccagacggagcccttcttgttggtaaaggtgaccttctgccccaggccgttgtagccatagctttcggtgaaaccaagggcgtcgacgctgctcagcagccggcttgcggcatcgtaggtgaagctgttggtgcggtcctgcgccgcctgcaacacgatggccagggctatggcttcggcggtgttggctgtggcggcgggaatcgacagcgagtactgcgtggtctgaacgatacggctcaggccgtcataggtcgtacgcgtgacgaagcccattggatcgacgctgtatgccagacggttggcagcgtcgaagttgcgtttcacggtccggtcgatggccgtgtttgcggtgatcagggcccgtagtgtcgtggcgctggctgtccagttgccctgcaacgatgcgagattggccggcgttccatagctggtgatgcgaaccgcattgccgtttgcgtcaaagctcgtttcggtaacagcgccggtggcatcgacaccgaggatcttgcggttcgccgcgtcgaatgcggcgcgatccacgcggtcggcgcctgcatagtcatagacgcgtgctgcctttgcctgtgtttcggtcagcttgctggctgccgtgggcaccgcgatgcgcgtggcatagctgtagcgcgtggtgacgttgccgttcttgtcgtagaccgcttcggtgagcgcacccgtggcgtcgatcacaaaggtctggcggttggcctggtcgtacacccggtcggtgatgcggtcgctggccgaggctgcaacggaagaggggaccatgccgcctgagaccgcagtggcgtactggatcgtcttgagcaggttgccgttcttgtcgtagacctgtttcgttacggcacccacaccgtcggcagcccaagtgagccggtccgcgcgatcgtagatgaatcgttcgcgcgtgccgcccgccacataggcgatcggtgacgtggtggtcggggtgtagcggctggcgacatcggcctgctcgagctggtagccgctcacgcggaaagccctggtgtcgttcgcggtgtatttgacaaccccgaaagccggtgccgttgacgcaggcgccacgccggtcatcgacacacgatagcgcccgccgccaaggtcctgcacgacatacttgagaggattggtcgcgccagtgaacagcaccaaaccaaacgagttcgccgcagtggcaacgctcgcattgctgaaagacggcggcaatccgtcttccatctccacgatcacggacagcgtgtacgcgacgccggcgatcggcgtgaacgacttgtaggcataggtgctgaccgtgtcggacgcaagcctgatcgcgcctgagaatccggtcattgtggtcgccgtggcggcgccgcctctgtacggcgcgtcgctgaggccattggcgaactcgctctgcgtgagcaggttggtgcccgcttgctgcgggttggttgccagtgtgattgccgcggccagggcggtggcagtggcggcagtggccacgggcacggtcgcagcgtaggcgatccgctcgaccacgttgccgttgccgtcgtagatcgtgcgcctgaccgcacctacgccgtcgatggtgtaggtggcgcggttgagctggtcgtagaccgagcgcaggcgcaggtcgcgcgcggcatccgcagtgggcgcaggcaccgtgcccacggtccagctggccagggcgatgcgattggcatacgccatgcgctcgatcacgttgccattggcgtcgtaggtgtacttgaccacctcgccgaggccgttgacggtggccacctgtcggccgtccttgtcgagcacacggtgctcgacgctatcgcgcgcagcgttgacaaccaccttggcatcaagctgcgcaatggtcggtgccgccggcaagccggtcatgtcaacggcggttgcgtatccgatggtctgtacgacgcggccttcggcatcgtagcgggtgcgctgcaggttgccggccggatcgagcgtgtacgcaagccggttctcggcgtcgtaggcgtagcgggtaacctggccgtttccgtcggtgctgctggtgaggttaccgtccttgtcgtaggcgtagctgcgggtgatgttcagcccagacggatcgatgcgctcctgagtacgccggcccagcttgtcgtagatgtactgggtggtggcgccattcgggttgacgaccgtgagagcgttgccgacaccgtcgtaggtgtagcgcgtgacaagattcaggcccgtgggatcgatggcctggctggtcacctgtcctttgaggtcatagacgatgagcgtgagcgttccgttgggatcggtgacttcgatctgctggcccttggcgtcgtacttgtaggtggtgatcagggcgaggccagtggggtcgaccgtgcgcgtgagcagcctgttggctgcgtcataggcgagcgtcacgatgttgccgttcgcgtccttcgtttgcgacagacggcccgaccggtcataggtgttggtggcagtcgtcagcgccgtggcggtgctcagcaggttgccgttcttgtcatagctgtagcttgtcgtgttgccgttgccatcgaccacgctttgcttctggccgaggcgtgtgtacaccgtggtaacgctgatgttctcgggtgtcttgatcacgacgcggcgcagcgtcttgtcgtaggtgtaggtcgtaacccgcccgagcgcgtcggtctgggtcatgacgcgatcgaaagcgtcgtaactggtggaacggacggccgagagcgcatcggtcgtcgtgacaatgcgacccaaccggtcgaagctttgctggcgaacgttgccgttcgcgtcggtgctgcgcgtgagtcgtccgaacgcgtcgtagatggcactcgtgacggcgttgatgcccgacgcgtcttgcaccgtgccggttacgaggccgcggcggtccaccgacattgactgaaccagttgcgtcccattaccgagcgcctgcgtgcgaccggtcaggtcgccgaaggcgttgtagctggactgggtgaggttgccaagttcgtcggtgctgccgttgagctttccggtcaccgcatacgtgaagctctgtttgctgtcgagcccgacattcttgattccgtcgatggcggtcgtcagctcagcgttaaccagcccgccggccaggccggccacgctgccaagacgagtgccgtagcggatggtcgcgctgagctggcccagggtgtcgtactgctgctcggtcacttcgccgagcgcgttgacgctgtgggtgaggcggctgttcaggtcgtagaagaacagcgttttgttgccgtacgcgtctgtggtgccgaggcgccggcccgccgcgtcatacgcatgcgtgagcccatactgcgaccagatggcatcgatctgtgcctgggtctggccggctacgaggagtgcgccgccttcggcggtgagttcgccggtgaggcgcccctggatgtcgtagcgcgcgttgatcgtctggatttcggtcgtgccgaaggcattggtggtctttaccaggttgccagcgctgtcgtattcgtaccgggagacagttccttcatagttggtgcgctgggtgacgcggttgagtttgtcgtagacaagcgttgtcgtacgaaacccggcgctggaagatggacgcaaagccgccacagtggttgccgtcgtcatctgcgagagcagggtggcatcgactcgaacgacatagcgcgtggaggtcgtgacgttgccattggcgtcgtacacgctctcggtcatgaagccttcggcgtcaatctgcgccaggactcgaccttgggcgtcgtagagccagcgcgacgtctggtcctgcgcatcgcctgtcggaatcaattgcgcgagcgtgccgctgtcgcgcatcgcggcgatcgtgggcgtcgcgtaggaaatctgggtaacgaggcggccttcggcgtcgtaacgcgactccgtcagatagccttcggcgtccagggtgcccagcagcaatccgtcgttgtcgtagaaacggcgcgtgacccggtcgttggcggcatctgccgttggggtcgttgcggcgagagttggcgccgcgccgaaggagttcgtggcgatgactgcccagtattgcttggtgcctacgagtcgcgacgcaccgtcatagcgcaggtcggtgaccgcgcccgccgcgtcgatcgttcggacgagccgtccggcgccgtcgtagatgcgccaggacttctggtcgaacgggctgttggcaggccggatggcacccaaccggttgacgggcgcgctgttcgggtcagagaggtatgccgtgaccgctggcgcgttggccggagtggcatagacgatcttgtgggtgagctggttgttcttgtcgtagacatactcggtcacccggttgttgccgtcgatctcggcaaccagtcgtcccgcctcatcatagaggcgtcccgtgcgcgctcccgtcgggtcgacctgctggtagagacgcccgttcttgtcgtagtaattggtggtggtgccgaggttcgcgttcagtgcggagctctgcgtcacgctgaccatgcggccgttcttgtcgtaggcgctggtcgtgacaagcccgttggccagtgtgacgacggtcttgttgttcgcgtcgtcgtagctggtgagcgttgtctggttcagcgcgtccagtgtcgagagctgccggcccatgccgtcataggtgtactgggttgtcccggtcgtggcactgatggtactgagcagcaacccggctcggtcatagacgtactgggtgaccgactggctgccatcggcaatgccgttgccgctggcatcgacccggctgaagacggtgtttttctggacctggccccgggcgtcgtagaccgtgtcggtccggctggcctgggtgcggtcctgcgctgcgccccatgtgaccagctcggcctcgctcggcgtggcggtggcgccaagcgccgagacatcgtacttgccggcggcgtattggagcgtggacgtgcgttggccgtagctgtcgtagcggtactcggtgacacggccctccgaactgagcacgaatctcagctggttcttgcccgtgttgtcgtagacatagcgcgtcgtgaccggcaggctcggctgcgcagcgccggcaccatccggatccggagcaaggtagaccgtctcggtgagcagttggttgcgtgcgtcgtaggtgcgggtgatcgtgttgcccgcggcgtcgcgctgcagtgtctgattgccataagcgtcgtactgcatcgtcaccgcgaagccttgcgggtccgtgacgagagtgacgttgccgctggcgtcgtagttgaacagcgtgagctgcgatacgccgcccaccggcggagcctggatctgggtcagttgtccggcggtgtcgtagctgtagacgctgacgaggcccagcgggtcggtgaccgtcgtactgcgggtcgtggtgttgtacgtatagctggtggtctggcccaacccgtccttgacggtcgcaacgcggtagtcgggtccgaccagcacgtacgtgaaggccaggctcgtgccatctttttgcgtgaccgaggcaacgcgtttgctcgtgtcatcgtacgtataggtggtgacgtatgtctggccgtcggcaatgctgttgtcttcggggctgaggtcgaccgttactgtcgacagccgattggcgccatcgtacgcatagcgcacgcgcgtcagcgcggcaccgccgttggcggggctggcaacggtccggatctgcgtcaggtttgtgccggtgtagtcgaagtaggtcgtctcgccgttggcgtcgaccatgctttgcagcgtaccgttggtgttgtaggcgtaggtcagcgtgttgccggcggggtcgctggccagcagaagtcggccctggccggtggactcgtagcgctccagcaagcccgtgctgccgtcggtccaaatgaactgcagcgctgcggaatcgtaggcgatggtgtcgaacgcgccagcaccggccgggctgacgtagaggccgcgtgccacgtcccacgtgtaggtggcgctggcgccatcgcgatcggtgcgcgtcagggtactgccagccgttgcgaccgtccccgtaagctggatgcgctggccataagcgcccacgatccagttgtccgcgttgtcgtcgttgagcaggccctggctgttgtaggtccgcacggcatggatgtccaggcctcgcccgacaagcttgtcgtcgaagtcctgcagcaccagattgccgttggcaatgttgacgaaggcctgttcgccgtttcggccctggctggcagttccctgggtgcctcgctgtccgagggtggccaaggaggccaaactcaatccaagactgttgccgctgacgatcgctaccattttttgtgcccgtctgtctaaatatgtagaagcgaaccgcacacgctcggcctgctcgagtcggcgttttcacgcagccgactcggactccggggttgttccccagaaggccgccaactctcctcctggtggttggcgcacggttcttgggcaatacatccagggatttggaattttgtttagtggtcggacgctctttttcttcttgaccccgagcggctaaacaaatcttttctgggctggatatattggtcgaatggtcgtcatggccgacatggaccggatctcttgtgtcttacatcgctctcaccctgaaccactttcgggctcttcaagaatgggctctccagcatcaggcagaggtacgcctggatgtgccgaccttccgcgtggaagtccggcgcggggcagcgcgtttcaatcttcatcctcggtttctgaacacgacggaaatgggtctgagctattcgtctgcgctcactcagagcgccacgggtttcatcggctggctcccatatcgtccgatccgatggcagctttcgagcgacaagctggacttcaaggacttcgtgcggcgctgcggcatgcgtgctccgcaaatttggaccgcagacggtgcaatcgatcaggactatgtgctgaagctcccgtcgggctcgtttgggcaggcggtgtttggcccttatcacaagggctttgatgcgagatcacttcccgaacaccagaatcgcgtgaaggacaggatcttcgcggagcaattcgtcaccggtcgcaacgtgaaggtctggttttggggtggggtgccgtttcacgcgcacattgatccgtatccagtgatccgaggcgacggcgtctcgaggattcaggagttgattgctcgaaagctggggcgccccgatggatgtgtcccggagaacgccgacaagccatggctcatatcttcgttggcctatcaaggttggagcctgtcggacatgctgcccgcagatcaggaggcctggatcgagtatcgctatggccgaagatatgcgagttctcccgctcaagcccaatcggacagcatgctgtcggagctctctcgatcagccgcacagcaggtcaaggccatgggagccttgctgcacgaggagttgatgaaggagttccatgttcctgtgctattcgcgctggatggggtcctggactcgagcgaccagatctggtggctcgaagcgaattcgaaccctatcctgcctccctcgggatatccggtggtcttagggacgctgtttgacatggacgatcccaaggtgatggacgttcgtcaggaactgccccaagcagtcgctacagacatatagaccgatgacggtaccggaacaggggacctcgagtccgccgcagctacccctcgcggtaggaaaatggacctaccaacggaacggtggggtgctttgcagtctcccattgagaagactgcgtgtttcggcacccacggactttcttcgagctgtagagcgtacttgcgacgggaaatcgccctggagcaaggtccgtgacggactgagcgcaaggtggcctgtgcgggacgtggacgcgtgcctttcaactctcgtcgaacaaggcttgctggtggaggcggggcatgcgctggcgctccaggcgcagattggctggaccccgcagccgcttggcgcgccgctcaatagcgtcgaggaccttcgcgtgttgagcgagacggctcgcctccggttgaaggtctccactcccgaagcggaaaaattgcggccgcatggaacgccgatgctcgatgcgcttcttgaccgaggcagcgcgagaacattcgaggatcaggcgctgtccctgcagtcgacggtcaatattctgtggtcgatctatggggtactgcgcgaaggggccgagcatgtgcaccgaacggtgccctcaggaggcgccctgtatggtctgcgatggttcatggctttgctgcgccccatggacggctacgccgccggcttgtacgaagtcaggtaccacgcgaccgaacacgaaggcggtgagctttcgttgcatccgcaacagggggcggttgacgatgcctggtgcacgcttctggtggcctccgtcctgagcttcgcacatgccgtgatctatccggttgccgatctgcgcttcatcagcaaaaagtatgggaatcgggcgttgacccttgcgctcatggaggcggggcatgcactgcaaaatggggcgctggcagcgcgccacgagggggctgcaaccatcgtacgcgcagacactgtagagatggaggtgctgtctctcctggcattggatccgtcgttctatcccttgcccgcgctggtgctgggtgcgaagccgacgcaggcgcaggaggttcaggcgcaattggcgcatcgaatggttccggtctgctcggtgccgcagcattctcagatgctgcacctggcttcgcgaatggcggtggcggggccgattcaggtcgggagccgggtcgcgcaatcgatgtgggcgggagggcgttcggagagcgcccgcgtcgccgtgatcaaggcggaagcagaggcatgggagcggatcggatggtcgaccccaccggcatcgttgccgcgggcgagattcgatgaacttgccagtgctgtcgacccgcgttgcctggttggctattcgccggaacagtacgcgcgcgacgccttcccatacgctcctttttcttcccgcagacgctatccttggactaagggtgttcgcgccgaagacggcgcagaagttctcgtcatggcgcagtgcgtttatgcattgagttcgctggatgccgccgatgtgcggttgccatataccaacgcgagcacttctggcgttgccgcttacacagacatgcaagaagcccgatatcgggcgctcgtcgaactcgtggaacgagatgctttctcacgcacgtggctggcgcgcgctgcacctgatctgatcgaggagtcggctctccctgcggggcttcggcaacggttgcgccaattgcggcaggccgggtacacggtgtctcttcatgccttggagtcaaagtacctgccggttgcaggcgtttttgtgcagcaccaggatgcggtattcaccgcgctgaccaccggggcagggttcgaactcgaggaggcgctggcgtcggccctctctgaagcggaaagtcgtgtgcagcagcagcacggacagacacatccagttgttcatatgaagccaaaagaaattcggctggccaagcatcacggcgactattttcaaacgcggcgcggttcacggaaggctgactggttttccaccggtgcgaggcagactctgagaggagcggcaagccgttttcctgcatccgggcgagcattgctcgacggtttcgtgaatcggggacagcaggtctatttctgcgacttgacgccgcccggagcttcgataaatcaggggcgtacgccgctgtatgtggcaagagcatttgcgcctggcctgatccctctctggtttggctatggcaccgagccgctgggatcgtggggcgctaacgcaaccggcaaagcgtcccccgaagttggcagcctggaactcatccatccttgcacctaatccaatggggagatcgccatcgaacgttctgcctaagtgtcgaagcccaagtaattttgtttgatagaaggagttcatatgaagaatggtcaaagcaagcaggcatccagccgtcgttccaacgcaggaattacgctgaactgcaacgtggtggtggagccttccagcatcgatttcctcaacgagggagcggttttcgtagcgggttcgcaacaagattgcggttgcggcatctcgcccatgcctgaactcagaaaagggcatcgccgcggcccgacgggaaacaagcgctgatgcctggccggtgacggagcacttcggatgttcatccttcattgcactgatacagcgggggtgcccgtcagcctgcggtatgcaccgcattccagtgcgttgacaaaccttgacggcacgccggttctcgcaaatcggcaagtcgcggagcaacgcgcctgggaagacgccgtgcgcatcaacccggagcagccaggcctcaaagtcgccaatccgtctgtactcaagatacagctcggtcttggctgcaactacacctgctcgtactgcaatcaggcaagtcaggtcgagtccatggcgatgacgaagaccgcggatgcgctggcttttctgcatgatctcgaaaagtggcttgaaggtgttccttcccggatcgaattgtggggaggagagccgctcctgtatttccggaagcttcaggtcctggttcctgagcttgatcgcaagtttcctgatgcagagatctcgatggtgaccaatggaagcctcttgacgcaggaaattctggacttcatcgccttctacgacattcaaataaccgtgtctcatgatgggccaggccagtacctgcgcggcgaggaccccttcgaaaatcctgcacgggccgctttcctgacggcactttggaaggagcgcaaggcaaaggggcgcatgatattcagttccgtcttgacccccggaaacagcgatccagcagcgatcaggcaatggttcgtcaatcgactggccgatgattcggtgatcacctccctggagggtattgttgcgactcatgatgacaacgcactggcggggccgggggtctggagccccgcgcagtatcaggagatgagggcatcggtcgcaagatccttcgagacgggggaggctctcaggattcccgccttagcggaaaaggcaaaaagtttcttccaggctgtgatgctgggtatgccgtccacttccatggggcaaaaatgtggaatggatcgcagtgaccatgtcgccgttgatctgcattcgaatgtgctgacatgccagaacaccggggcgaacgccgagcatggcctgggttccgcattggagatggatgccattcgcatgacgacttccacgcattgggcctaccgcgaatgctgcaatcattgcccggttcttcagttgtgcggaggctcctgcatgtatctcgaaggggagcagttcgcccagtcgtgcgagaacgaataccagttcggcatgggggtactcgacggtacgctgcgccgggctttaggattgaaactggaaagcatcgaaggtgatattcgccgcccgatccgccgaaagacgatcccgatcattgcccgtcagtagcttcgacgcacggtggcgcagcgctgtgcagcgaaacaagaagtccggcaaccatgagggttccggcgcatcgttcagtaggccccggcccaccatccatcacaaaaagccaatctgcggcaggttggcttttttttgcccggacgcacggctatagtcagcgggcgctgtcacgccatcaccgttctgccttctcgcaaaggacgcggctggccacctagatccgcccaaaaaggacgccgtgcccgattcactgacctcgacgctcacgcgctactacgatgcggtgccctatgaatcgcacccgttcccgcaaacggccgtcgagcatctggaggccattgcgttcttgttcggtctccaagcaccggcaccggcccgggcgagggtgctggagcttggttgcgcggctggaggcaacctgattccattcgccgcccgccacccggaggccagcgccctgggcatcgatttgtcgaaggtgcaggtggagcagggcgccggagccatcgcccgcgcggcgctgcccaacgtggaactgcgggtgttcgaccttgcggaggtcgatgcatcgttcgggcagttcgactacatcgtctgccatggggtctacagctgggtgccgggcccggtgcaggatgcgatcctccgcatctgttccgagaaccttgcgccggacggcgttgcctatgtcagctacaacgtgtacccgggctggaaggcgagggagatcgtgcgcgacgcgatgatcctgcggggcggtccgcgcgacacgccggaagaacagctgtcgtatgcgcgcggcatgctcgaatttctggagcagtcggcccggtccgacagcgttctcaagaaaacgctcgaggaaacgatgcctatcgtgcgtggtgccagcagctactacctgctgcacgaattcctcgagccctgcaacgcaccttgctatttcaaggagtttgcggcgcgcgccgaggcgaagggcctcgcctacctggccgatgcggagccctcgacgatgttcgtgcagaactatggcgacaaggttcgcgaaccgctgctgcgcgagtgcggcggcagccaggtcctgatggagcagtatctcgactttctggtcaaccgcacctttcggcagacgctgctggtgaagcagcatcgtggcggcgacatccgctaccggctcgatcatgcccgcatccgcggtcttgaattcgccggcatgttcacggcggcggacggcggcgcgttgacgctcgatgcacgcgagcagccgtgcaaggcgctgcgcaatctcacggtgacgctgcgcctgccggtgcacaaggccttggcacaggtgctcgattcccgctatccggccagcacgtcgttcgaggcgctggtcgcggcggtgctggctgtcacgggtgaaccgcgcacttcggtcgagccgctcgtgctgtcgatgctcgaggagctgctcatcctcggcgccgtgcgtatgcggcgcgcgccggtgcaggtcgccgccgagatatcggcgtggccgcgtgccctgccgtcggtgcgaacggcatccggcctcgcgttgtcggccggaaattcggcgagcgtctgcaaccaatggcacgattccgtgggactcaccgcgctcgagcgttgcctgttgccgctgctcgatggcgcgcattcgcacgagatgctggcggaccacctggtggacgaggtgcgtgccgatcgcctgcgcttcgtccacgacgacaagccgctcgccgaaacctcagccttgaaggaattcgcgctgaaacaagtggcgattggcttgaacgacttgcggcgcagggcgctgctggttgcgtgacactatccatcgcctcccaccatccaactcaacgagggactttctccatgcagcaactccactggactccaacattgcgcgccgcggtagcggccgcactcgtactggcgggcgcaagcgcttccaacgccgcctcgcaggcacctgtcgcggccgagcacggcatggtcgtgagcgcgcagcacctggccaccaaggtcggtgtcgacgtgctcaagcgcggcggcaacgcggtcgatgcggcggtggccgtgggctatgcgctggcagtggtgtacccggcggcgggcaacctcggcggcggcggcttcatgaccgtgcaactggccgacggccgcaagacttttctcgacttccgcgagaaggcacccctggccgcgacggccaacatgtacctcgacaaggacggcaacgtcatcaagggcctgagcaccaacggccacctggccgtgggcgtgcccggctccgtgtcgggcatggaatacgcgcgcgagaagtacggcaccatgaagcgcgccgacctcatcgccccctcgatccagctggccgagaagggctttgcgctggagcagggcgacatcgacatgctgcgcaccgccaccaacgatttcaagaaggactcggtctccggcgccatcttcctgaacaagggcgagcccttcgcggtcggccagaagctggtgcagaaagaccttgccaagacgctgcgcgccgtcagcgccaagggtgtcgacggcttctacaagggctgggtcgggcaggccatcgtggcgtccagccaggccggcaagggcatcatcacccaggccgacctcgaccaatacaagacgcgcgaaatggcgccggtcgaatgcgactaccgcggctatcgcgtggtgtcggcgccgccgccgagttcgggcggcgtgatcatctgcgagatgctcaacatcctcgaaggctatccgctcaaggacctgggcttccgctcggccgagtccgtgcattaccagatcgaggccatgcgccacgcttacgtcgaccgcaacagctacctgggcgacccggacttcgtgaagaacccgctcgaccgcctcctcgacaagggctatgccgagaagatccgcgccgtcatcgaccccaagaaggccggtgtctccaaggacatcaagcccggcgtcgcgccgcacgaaggcagcaacaccacccactactcgatcaccgaccagcagggcaatgctgtctcggtcacttacacgctcaacgactggttcggcgccaaggtcacggccgacaagaccggcgtgctgctgaacaacgagatggacgacttcaccgccaagatcggcgtgcccaacatgtacggcctggtgcagggcgaggccaacgccatcgccccgggcaagcgcccgctgagctcgatgagcccgaccatcgtctcgaaggacggcaagccggtgttcgtggttggtacgcccggcggcagccgcatcatcacagccgtgctgcacaccatcctgaacgtggtcgactacggcatgaacgtgcaggaagccgtcgatgcgccgcgcttccaccagcaatggctgcccgatgtcaccaacgtcgagacctttgcgctgagccccgacacccgcaagatcctgaccgacatgggccacaacctgggcgtgccgcagccggccaaccaccttgcggcgatcatcgtcggcgcgccatcgctgggcggcaagcccgtcggcgccaaccgtttctacggcgcgaacgaccctcgccgcaacaccggactggccgccgggtactgatccggcaaactcgggcggtcgtgccactttggcgcggccgcctttttcatttccatgcatctgcaagacattctttattcccagggcttcggcacgcggcgcgtgtgcgcggggctgatccagcagggcctcgtgacgatcgcgggcaaggtcgtgaacgacccgttcgccgacctcgatcccgaaggcctccttttcacggtccagggcaccgagtgggcgtaccacgaaaaggcctacctgatgctccacaagccggcgggtaccgagtgctcgcaaaagccctcgacctacccgagcatctacacgctgctgccgtccccgctgcggctgcggcccaacaagggcgcggtgcagggcgtgcaggccatcggccggctcgaccaggacacgaccgggctgctgttgctgaccgacgacggccagttcatccaccggatgggctcccccaagcaccacgtgcccaaggtgtacgaggtcacggccaagcatccggtggacgaagcggagattgccaagctgctggccggcgtggtgctcgacgacgatccgaagcccgtgcgcgcggccgcctgcgaatcggacagcccgctgcacttgcggctgaccctcaccgagggcaaataccaccaggtcaagcgcatgctggccgcggttggcaaccgggtcgagggcttgcaccgctcgcgcatcggccagctggcgctgcccgcagagcttgcgcccggccaatggcgctggctcgacgccggacaagttgctgcgctccgtgaaaaaacaccgggataagggcaccgcgaacgggggcggtcagccagccgtcgggtccggacgttgataatcgacagcactcttccggaacttctcccttgcgattccttgcccgaccgaatggccgcttgccggccttcctgctttcctgcctgacggtctgggtggcacaagccgccactgctgcaccgcccgaagccccgccgatcttcgtgctcaattcgctggatgccagcgtcagcgtgatcaacccggccgactggaccgaaaagcagcgcatcgccaccggcaaggagccgcaccacatctacatgacgccggacgaaaagtcggtcatcgtggccaattcggcgggcgattcactgacttttctcaaccccaaaaccgccgaagtgcagcgcgtggtctacggcatcatcgatccgtaccagctgcagttctcgcgcgacatgaagtggttcgtcaccgccggaaaccggctcaaccacgtcgacgtctaccgctgggacggcaaggacctgaagctcgccaagcgcattgccaccggcaagacgcccagccacatctggatcgacgccaccagcaccattgcctacgtgaccatgcaggacagcgacgaactcatcgccgtcgacctgcccacgcagaccatccgctggcgcatggccaccggccccatgccggccgacatttttggcacgcacggcgacaagaccctgctggtgggcctgaccggcagcgacggggtgcaggtgttcgacgtggcgggcgccgagcccaagctcgtcggcaagatcccgaccggcaagggcgcgcacgccttccgttcggccggcgacggcaagagcgtcttcgtgagcaaccgggtggccaacaccatcagccggatcgacctggcgacgctcaaggtcagcgcaacataccccgtgccgggcggccccgactgcatggacgtttccgccgacggcaagaccttgtacgttacttcgcgctgggccaagaagctcagcgtggtcgacctggcaagccagaaggtcgtgcgccagatcaatgtcggccggtcgccgcacggcgtctggaccctggaacatgcaaaaagaatctgagcgggtcccggtggcaatccggcagatccggcttcgcagcgtttccggggccgtttttgccatcgcctgcgccgcgatgccggccgcgtgggcgcaaggcgcttcctgcgaaaagccggtctacctgaccttcgacaccggccacatgggcgtcgctccgctggtggccgacgtgctcaagcgccagaacatacgcgtcaccttctttgccgccgccgaacgcacccagaccgacggcgacagcctcgacagccactgggccccatggtggaaggcgagggcggccgaaggccacgaattcgcctcccacacctacgaccatgcgtactggcgcggcgacctcaaaggggtggagccgagctttcgcatcaagccctcggcgggcgcgttcgctgggcgtgagttcacctggaccgcggccgagtactgcgccaacatcggcaaggcctccgagcggctggccctcatcaccggcaagaagccgctgccgctgtaccgcgcgccgggcggcaagacctcgacccggctgctcgccgcagccaaggcctgcggcttcgaacacgtgggctggtcgcccgccgggttcctgggcgacgagttgccgagcgagaaattcagcaacgaaaagctcctggcgcaggcgctggagaccatccgccccggcgacatcctgctcgcgcacctgggcatctggtcgcgcaaggacccgtgggcgccggccaacctcgagccgctgatcgtcgggctcaaggccaagggtttctgcttcgaaaccctgcgccagcaccccgattaccgcgcctggatcgcgtcccacccctgaggcccctgccgtgatcgattggttgacggacgccttttccgcgctgcagggctggtttttcgagacggtgatccagcccctggtctatgccgtcggcctcggcggctggaccgaagatgccttcgacgccaccggctggctgctggtcggcctgatccaggtcctggtgctgctcgcggtcatcggtccgctgcagcgctggcgggccgccgagccggtcaccgaccgccgcgccattcgcatcgacgttctctacacgctgatccatcgcctcggcgtgttccgcctggccatgttcttcacgctcgagccgctcttcgacgaagccatcgggagcctgcgcaccgcgggctggggcaccttccacctcgacgaggcctggcccggcgtcaccgacgtgccgtgggtcgcgtttgcaatctacctcgtggtgctcgattttgtcggctactggatccatcgcggccagcaccagttcaactggtggtggggcctgcattcgctgcaccattcgcagcgccagatgaccatgtggagcgacgaccgcaaccatctgctcgacgacatcgtgcacgacaccctgatcgtcatcgtggcgcagctgatcggcgtcgcgcccggccagttcattgccttcgtggccttcacgcagctcagcgaaagcctgcagcatgccaacctgaagctcggtttcggcgccattggcgagcggctgtggatcagcccgcgctttcacaggctgcaccacagcatcggcctgggccatgaatcgcgtggcgcccacacgctgggcgggcacaacttcggcgtgctgctgccctggtgggacatgctctttcgcaccgtcaacttcgagccgcgctacgacccgaccggcatccgcgaccaggtcgagcccggcgccgacggacggctgcgcgactacgggagcggcttctgggcgcagcaatggctcggcctgaagcggatggtcggccgcggctgagcgccggcccgaaccgagccggttatccttcgcacccaatgcgcctgctcctcgactctttctggcgcgcggtcgcctattgcatgctgccgcgcgtgatcgtgctgtcgctgctgcccctgggcctgatggtgctgctggccgcagggttcggctatttcttctgggacgccaccgtggcatggacccgcgaggcgctcgacgcctggcccctgctgtcgagcttctggggctggatcgggcggctcttttcgggtgacgtcacggccgtgctggcgccgctggtggtcgtggtggccgccaccccgctgatcgtggtcgtctcgctcctgatcgtggccggcctcatggcgccgccgctcacggcactggtggcgcaccgccgctttcccgcgctggagcgcaagaagggcgcctctttcttcggcagcgtggcgcgctcgctcggcgtgactgtgctggcgctggtggcgctcgtggtttccatgccgctctggctcattcccccgctggtgctcgtcctgccaccgctgatctggggctggctcacctaccgcgtgatgagcttcgatgcgctggccgagcactcaagccccgaagagcgggccaccatcctgcgcgcgcaccggctgccgcttttatgcatcggcgtgctgtgcgggtacctgggggccgcgcccagcatcgtctgggcctcgggcctgctgtttgccgccgccttcttcgtgctggtgccgctcgccatctggatctacacgctggtatttgccttttcggcgctctggttcggccactattgcctcgatgccctggcgcagttgcgtgcccagcgcggagccgccgccgcttcggccgaaagcgccccagccctcgaagccgaccaggccgttctttctcagtggaaatccccatgacccgtgcattcggactgatcgtcgtcggcgacgaaattctttcgggcaagcgtgccgacaagcacatgcccaaggtcatcgagctgctcgccgcgcgcggcctgcagcttggctgggccgaatacgtgggcgacgtgccggcgcgcatcacggcggcgctcggccgggcctttgcctcgggtgacatcgtcttttcgaccggcggcatcggcgccacgccggacgaccacacgcggcaatgcgccgccctggccctgcggctgccgctcgaactgcatcccgaggccgagctgctgatccgcgagcgcatgcaggacaccgcgcgcgaacagggcattgcctacgagccggatcggccggacaacatccaccgcctcaacatgggcgtgtttcccaagggcgccacgatcatccgcaacccgtacaacaagattccgggcttcagcgtcgatcacgtccacttcgtacctggctttcccgtcatggcgtggccgatgatcgaatcggtgctcgacagccgctacgcgcacatgttcaccagcgggcaggcggccgaaaaatcggtcatcgtctttggcgccatggaagcaacgctcacgcctctgatggaggccatcgaagcggcgcacgcgggcatcaaggtgttcagcctgcccagcgtcgaccatcccgagtacggccgccacatcgaactcggggtcaagggcgatcccgttcgccttgaagccgcctacgcgcagctgatcgagggcctgcacgcctatgatgcgaagcttggcccggaattggtgcgctagttttgaatgcaccaaattagtgatttctcgcctttttttggggtttgcggcccttgccggcgcctcttccgaagaggcgacaatggcacagaaactgcatccttcgtccctgtattcctaaccaccatccaactcaggagaaactgatggcaaagaccgtcgccgatgtactcaagctcgtcaaggaaaacgaggtcaagttcatcgacttccgcttcaccgacacccgtggcaaagagcagcacgtgaccgtgcccgtctcggctttcgatgaagacaaattcacctcgggccacgctttcgacggctcgtccatcgctggctggaagggaatcgaagcctcggacatgcagctcatgcccgaccccaacaccgccaacatcgatcccttcttcgaagaaacgacgctgatcctgacctgcgacgtgatcgaccccgccgacggcaaggcctacgagcgcgatccgcgttcgctcgccaagcgcgcagaggcctacatgaaggcttcgggcctgggcgacaccgcctacttcggtccggaacccgaattcttcgtgttcgacggcgttcgctggaagaacgacatgtcgggctgcttcgtcaagatcgactccgaagaagcctcctggaacaccgacaaggaatacgagcacggcaacaccggccaccgtcccgcggtcaagggcggctacttcccggttcccccggtcgacagcttccaggacatgcgctcggaaatgtgcctggtgctcgaatcgctcggcatcccggtcgaagtgcatcaccatgaagtggccaatgccggccagatggaactcggcaccaagttcagcacgctcgtgcaacgcgccgactgggtccagctgcagaagtacgtgatccacaacgtggcccacgcctacggcaagaccgccaccttcatgcccaagcccatcgtcggcgacaacggctccggcatgcacgtgcaccagtcggtctggaaggacggcaagaacctgttcgcaggcgacggctatgcgggcctctcggacttcgcgctgcactacatcggcggcatcatcaagcacgcccgtgccctgaacgccatcacgaaccccggcaccaacagctacaagcgcctggtgcccggcttcgaagccccggtgaagctggcctactcggccaagaaccgctcggcctcgatccgcatcccgttcgtggccaacccgaagggccgccgcgtcgaagcgcgcttccccgatccgctgatgaacccgtacctcggctttgctgcattgctgatggccggtctcgacggcgtggaaaacaagatccatccgggcgaagccgccagcaaggacttgtaccacctgccgccggaagaagacgcgctgatcccgaccgtctgccacagcctcgaccaggctctggaatacctcgataaggaccgtgcgttcctgaccaagggcggcgtgttcaccgacgcgtacatcgatgcgtacatcgatctcaagatgcaggaagtcacgcgcttccgcatggcgacgcacccggtcgaattcgacatgtactactcactctaaatcggtgggcgcaagcccctgatggttaagtaagacaaaaaggacggctgcggccgtcctttttcgttgacgcggaacatcttgtcaccgatggggtcgaattgcaggaaaatgcacctttgtcgcgccatccaccgattctcatgaagactgcttccctcattttcctggctggttcattgttcgccgtcgccttgccggcgtcggctcaggagcgcgtgtggcgctgcggcaatgaatacaccaacaatgcaaccgtggcgcagcaaaagggctgcaaggttctcgaaggcggcaacgtcaccgtcgtgcagggcaccaagccttcgggcggcggttcggcgagcagcggttccgggccggccgcggcgcgtgcgccggccggcagcccgcgcgtcgagggcgtcgaccagcgcgcccgcgacggcgaagcacgctcggtgctcgaggccgaactgaagaaggccgaggcccgccaggcggaactgcagaaggaatacaacaacggcgagcccgaaaagcagggcagcgaaggccgcaactaccagaaatacctcgatcgcgtggctggaatgaaagccgagctggcgcgcaacgagagcgacatcgcgggcatccgccgcgaactcggccgtctgccggccaagcagtaaaccatggtgttcgggaagaaggcgactggcgccggcctgcgctttcagtccttcgacctgctgtccacgctgattgcggtggtcagcaccaacggctcggtgctgttcgccaatgcggcgctcgaagacgcgctgggcacgtcgcgccgcacgctcgaaggttctcagttcggtgcctgctttcacgagccgcacgttctgcgcaccgccatcgacggtgcgcgcagcaacgactttgccacgctgcgctacgaggcgtttctgcgccgcgtcaaccacgaactgatgccggtgcaggtcacgctggcgcaaggcgacaagacgggcgaactcatcatcgagatgtcgccgctcgagcagcaggtgcgccaggaccgcgaagagcgcttgatcgaccaggcgcaggccaacaaggaactcatccgcaacctcgcgcacgaaatcaagaacccgctgggcggcattcgcggcgcggcgcaattgctgcagatggaggtcgagtcgcgcgacctcatcgagtacacgcaagtcatcatccacgaagccgaccggctgcagacgctggtcgaccggctgctggcgccgcaccggcgcccgcacgtggtgggcgacgtgaacatccacgaagtgtgcgagcgcgtgcgctccgtcatcctggcggagtttccgcgcgacctgcacatcgagcgcgacttcgatccctcgattcccgagttccgcggcgaccgcgagcagctgatccaggccacgctcaacatcgtccacaacgccgcgcaggccctggccgagcgccgcgccgccggcgatgcgcagatcactttcaggacgcgaatcgcccggcaggtgatattcaacaagcagtggtatcgattggcactggaattgcatgtcatcgacaatggaccgggtgtgccggacacgatcaaggaccgcatcttctatccgctcgtatcgggccgggaaggcggtacagggctcggattgacgctcgcgcaaacctttgtgcaacagcatcacggcgtgatcgagtgcgacagcgtcccgggccgaaccgatttcaagatattgataccgctgccctagcagccacggcaacaaggagatgcatgaagccgatctggatagttgatgacgaccaatcgatccgcttcgtgctcgagaaggccttgctgcgcgaagacttgcccacgcgcagtttcaccaacacgcgcgaggtgctcgccgccctcgaactcgccgaagacgacgagcagcagggcccccaggtcctggtgagcgacatccgcatgcccggcggctccggcctcgatctgctcgacaagatcaaggccaagcaccccggcctgccggtcatcatcatgacggcgttctccgacctcgacagcgccgtgtcggcgttccagggcggtgccttcgaatacctgcccaagcccttcgacctgccgcgcgcggtcgaactcatccgccgcgccgtcgacgaaagccaacgcgaggaagtggccgaggagcgcatggtggccgcgcccgaaatgctgggccaggcgccggccatgcaggacgtgttccgcgccatcggccggctctcgcaaagcaacgtcacggtgctcatcaccggcgaatcgggctcgggcaaggagctggtggcgcgcgcgctgcacaagcattcgccgcgcgccaacggtcccttcgtggccatcaacaccgcggccatccccaaggacctgctcgagagcgaactgttcggccatgagcgcggcgccttcaccggcgcccagaccatgcggcgcggccgcttcgaacaagccgagggcggcacgctctttctcgacgaaatcggcgacatgccgttcgacctgcagacgcgcctgctgcgcgtgctgagcgacgggcacttctaccgcgtgggcggccacaactcggtcaaggccaacgtgcgcgtcatcgcggccacccaccaggacctcgagcagcgcgtcaagctcggcggcttccgcgaggacctgttccaccgcctcaacgtgatccgcctgcggctgccggccctgcgcgagcgcggcgaagacgtgcccgcgctcacgcgccacttcctgcaggtgagcgcgcgccagctcggcgtcgaacccaagcgaatttccgacgccgcattggccaggctcgccgccttcggcttcccgggcaacgtgcgccagctggaaaacatctgccactggctgaccgtgatggccccggcgcagctgatcgaagccaaggatctgccgcctgaagtcatggccgccgccgccagcccgcaggtccaggccaccgacgcagcccccgccgcagcagcagcaccggctcaagccgcgccgcagttgtcatcgagccccgagcgcgaaacggcgccggcaagcaccgcgcccgaagccgccgaaggcctggtcggcgcaagcagctgggaaagcggcctcgagatcgaagcccaggcactgctcgcagccggccgcaccgacgtctgggacgtgctctcgcgccgcttcgaatcgcgcctgatcctcaccgccctcgccaacacccgcggccgccgtatcgaagccgctcaaaagctgggcatcggccgcaacaccatcacccggaagatccaggaactgggcattgagtaaggcaaagccggctcgcaagcgagcggcgggctcccttccagggataccgcggaaccggctttgccgggccgctggtatcgcccccggtagggggttggcgtagcgacacgaagtgcgcggagactgggggcgagccagttatctgcttcgttggcccagcgtcagcgagtcgagctggaagtttccgctcttgtcccagagccaggtgtcgacgtaggtatggctgccaaggcgccccgggctcggcagcggcgacgccgccttgatgagttccgcgatcttgggcgggacttcgggtgcatggctcggtacgcggctgaacgtcacgttcttcacgttgccgctggcgtccaggtcggtttcgaccaccaccaccgcatagaccagcgggggaatcttccccttgtagatgcgctgcggataggcgttgtagatctgccgcgccccggacttgcgatacgcccgcacggcgggtgtttgcgcggtgatcaggcgcacggtcggtacgtcgcttcttgggcttgcgacttcgtcgggtgcggaagcggtcggcttgccgtcgccggccttttctgtcggcttgagagccgaacagcctgcgagcgccagtgccgccgcaaggattgcgagagtgcgtatgttcgtggtcataaggtgccttggtcgagttcgagcaccacgggcgcgtggtcacttggtttttcccacttgcgtggcacgcgatcgatgatgcagcccttggcgcgcggcaccagcggctcgctcaccaggatgtgatcgatccgcaagccgcggttcttctggtagccgagcatccggtagtcccaccacgagtagcttttctcgggttgctcgaagaggcggaagctgtcggccaggcccagctggagcagcgccttgaaatggtcgcgctcctcggtcgtgtgatgaatcgtctccttcagtcccaccggatcgaaactgtcgcggtcttccggcgtgatgttgaagtcgcccagcaggaccaggttcggatgtgccgccatttcggcgcgcagccattcgcgcaaggcgcggagccagcccatcttgtattcgaacttgtcggtaccgggcgcctggccgttgacgaagtagccgttcaccacgcgcagcggacccgccggtgtctcgatcgtggcggcaatcacgcgcgactggtcgtcggtaaaaccgccgatgttcctggccacgtcgcgcatcggcgccaggctcaggatggccacgccgttataggttttctggccgaacacggccgcctcgtaaccggccgacttgagcacgtcgagaggaaacttgtcgtcgctcatcttgagctcctgcaggcagagcacgtccacgggattggcaatcagccagtcgagcacatgctgcaggcgggcagtgagggagttgacgttccaggtggctattttcatgaagttgcgaagtgatggcgatctgccgcgaagggacgccagcttagcaaaagcagtcgaaaaacctgcttacatcaacgccaggcagcctggcgaagcgtgcacgttaccgcttcctttgttcatcgcgcccagcgcagcaccagcgggtcgagccgccgcgcggtctcgatcaggctcttgcgggtctccgggtgcatctctggccagggatggcgcggcgcttcgcaggcgatcacgccgccttccttcatcagcgccttggccgcgaggaagcccgactgccggttctcgtggttgatcagcggcagccagcgctggtagagcgcaaaggcctgatcgcggtcgcctgcgcggtgcgcctcgatgatcgggcggatgccatccgggtagccgccgccggtcatcgagccggtggcgccggcgtccagatcgggcagcagcgtgatcgcttcttcgccgtcccacgggccctcgaccgcatcgccgccgagccggatcagctcgcgcagtttggatgccgcaccggccgtttcgatcttgaagtacgcgacatgctcgatctcgcgcgccatcttcgcgaggaacgcggccgacagcggagtgcccgcggccggcgcatcctggaccatgatgggaatgtccaccgcgtccgacaggcgcgcatagaacgcatggatctgcggctcggtcacgcggaaggtggcgccgtgatacggcggcatcaccatgagcatggcggcgcccatggcctgtgcgcggcggctgcgctcggcgcacaccttggtgctgaagtgcgtggtggtcacgatcaccggcacgcggcccgccacgtgctcgagcacggtgcgcgtgagcacctcgcgctcgtcgtccgacagcagaaactgctcggagaaattggccaggatgcaaagcccgtcggagccggcatcgatcatgaagtcgacgcagcgcttctggcttgccagatcgagttctccgctttcggtgaacggcgtcggaacgacggggaagatgccacggaagcgggcagggcgagtggttgtcatggtgtggagaaagaagttgcgggtcaggtgaccacgctgatttgccagggcacaaactcctgctggccgtagccgtggagttcgctgcgcgagggctggcccgaggcggtgtcgagcagcatctggaacagccggacaccgagttccttgatgctgcgcgtgccgtcgagcacctcgccgcagttcaggtccatgtcgtccgactgccgctcccacagcgcggtgttggtcgcgagcttgaaagagggggagggcgcgcagccgtaggccgagccgcgtcccgtggtgaagcaaatgaggttggcgccgcccgccacctggccggtggccgagatcgggtcgtagccgggcgtgtccatgaacacgaggccctgggcccgcaccggttgcgcgtactcgtacacgtcgacgaggttggtcgagcccgccttggcgatcccgcccagcgacttctcgagcacggtggtcaggcctccggccttgttgccggccgatgggttgttgtccatcgccgcgccgttgcgcgcgcaataggcctcccaccagcggatgcggtcgaccagcttgcggccgacgtcgggcgtctgcgcgcggcgcgtgagcaggtgctcggcgccgtagatctcgggcgtttccgacaggatggccgtgccaccgtgcgcaaccagcaggtccaccgccgcgccgagcaccgggttcgccgaaatgcccgagtagccgtcggagccgccgcactggaggccgacgaccaggtggctcgcgggcacggtctgccgccgcaccgcgttggcctgcggcagcatctgctggatcagctcgatgccccgcgcaatggttttggtcgtaccgccggtgtcctggatcgtgaagctttgcaggcgggcgctgtccgccaggccctgcgtggccagcagcgtggacacctgattcgtttcgcagcccaggccgataaccagcacgctcgcaaagttgggatggcatgcgtagccgcccagcgtgcgctgaagaatcgcgagcccttcgccgtcagggtcgaccgcgcagcccgcaccgtgcgtgagcgccaccacgccgtcgatgttcgggaacggcgccagcatctcgggatggatgtcgcgcctgaagcggtccgcgatggcgcgcgccaccgtggccgagcagttcaccgaggtcaggatgccgatgtagttgcgcgtggcgacgcgcccgtcttcccgcacgatgccttcgaaggttgcgggctctgccgtgcgcaccgttgggcgtgcatcggccgaatgcgcatggtcgcgcgtgaagtcgcccatcgcgaggttgtgggtgtgcacgtgctggcccgcgcgaatcggccggctcgcaaagccgatgatctgcccgtagcggcgcaccgcggcgcccggctcgatggcgcgcgtggccatcttgtggcccggcggaatcagcccggccacggccacgttttcgctttcgatgtgggttcccgcgaccagttggtcgagcgagatgacgacatcgtcttcggcatgcagccggatcacgcgcgcgtatgacatggcggggtgcaccgtcactcgacgatgttgaagtccttgaggtactcggtcttcagcgtaaggcccaggcccggcttgttgtcgtccagctgcaggaagccgttctcggccaccggctcgccgtcgaagatgtaatagaacagctcgttgcccacttcgacgtcgtgcatcgggaagtactcgctcatcggcgaagccagcgtgctcatcgtcaggtggtagttgtgcatctggcccgcatgcggaatgaccggcacgctgtaggcctcgcacagcgcgttgatcttgtgtgccgccgtgatgccgcccacgcggttggtgtcgtactgcaccaccgacaccgccttgcggtccaggagctgcttgaagccgtagagcgagaactcgtgctcgccgcccgagatcggaatgctggtcagctggttcagctcggcgtagccatcgatgtcgtcggcgatcaccggttcttcgagccagcgcggctcgaacttctcgagcttgggcagcatgcgcttggcgtactcgaggttccagcccatgtagcactcgagcatcaggtcgttgtcgtagccgatgacttcgcgcacggcctccaccgacttgaggttttccgccacgcccttctgcaggtgcgccgggccatagccgaagcgcatcttgaacgcggtgaagccctggtcgagaaacttctgcgcctcggcctgcatttccgcgaggtcggtgcgatacagcttcgagtagtagcagggaatcttttctttcgtgcggccgccgagcagcttgaacaccggcttgttgaccgacttgcccaggatgtcccagatcgcgaggtcgactgccgagatggcggccatcgtcacgcccttgcggccccaggcgtgcgtggcgcggtacatgcgctgccacaggtactcgtagtcccacgggtcctgcccgatgaccagcggcgcgaggtactggtcgatgatggccttggcaatggccggcgcaagcgccacgttgcccaggcccacgatgccgtcgtcagtctcgatctcgaccacggtccacgaatggaagcggaaggtgctcatcgtttcctgcggcgcatacagcaggtccatcgcgttggagcagaagttgccctgcggtggaacggtcttgcccttccattcgaagactcgggcgcgcacggatttgatcttcatcttctcgatctttctaaggtgataggtaggtgttgaatgggaccgtcaggccgcgaccgcggccttgccgaggaggcgcgcggcgcccatgcggccggcgatccggaaggcctgccacatggcctcggcgctggccttgccctggcccgcgatgtcgtaggcggtgccgtgcgcgggcgtggtgatcggaatcggcagcccgccctgcaccgtgacgccgcggctgaaacccaggagcttgatcgcgatctggccctggtcgtggtacatggtcacgatcgcctggtactcgccggcctgggccttgagaaagatggtgtcggccgggaacgggccgtggaagggcgcttcggtgggccagctgcgcgcctgcagggccttgacggccggctcgatgatgtcgatctcttcgcgtccgcacacgccgccgtcgccgccgtgcggattgaaggccgcgatcgcgaccttgggctcggccacaccgttggccagcagcgagcggtagatcagctcggccgcctgttcgatgcgctccacgctcaggtagccggccacgtccttcagcggcacgtgcgaggagatgcgcgaggtccagagctcgccgagcgtgttgaactcgcagaagtagccggtcacgcccaggtgctccgcaaagtggtgcagctcgtcttcgtgctgcatgccgccgatcttcatggcctgcttgttgagcggcgcgaagcagatcgcatcgacgtcgccggccagcgttgcgtccatgcactggtcgagcacctgcagcaccgcgcgcccgcccggcgcagcggcccggccgcgctgcaccagcgccggatcgatgctctgcaccgccaggaaggccggacgcgccgtgctcgcgcggcttcgcacttcggccagagtcttcacctcgtcggtggcgaccgagacgcccgcgatgcgttggccgtcttcccacagccagcggtcgccgatcagcacgacgttcgcgtccgcggtggcgtcgggccgggccagcagccgcgcgatcagttcggcgccgatgccggcggggtcgcccagggtgagggcgacgacggggagggtttgcatgttcatcgagagatgcctagtccagcttgatgtggttcttcttgatgacctcgccaaagcgcttgtattcggcggcatggaattgcgcgaactgcgcctgggtcatcggcgtgatctcggcgccgatggcgtcgaggcgggtcttggtttcgggcatggccagcacctggttcacggcgtcgtgcaccttgtcttgcaccgccttgggcgttgcggccggcatgtagatgccgtaccaggcgctcatctctatgccgggcacgccggcctcggccagcgtcggcacgttgggcagttgcgggttgcgctttggcgtggtcacggcgagcgcgcggaccttgttgttccggatctgcccgatcaccgaaggcatggtgtcgaagctcagctgcacctggccgccgacgaggtcgatcagcgcggggccgctgcccttgtacggcacatggacgaggtcgactgcggccgcatccttgaacatctcggccgcgatgtgctgcgtgctgcccgcgccgctggtggcgtagttgagcttgcccggctcctgcttcgccagcttgaccagcccctgcaccgagtcggcgggcacgctgttgctcaccaccagcacgttgggcaccgcgccgacgaaagccaccggcacgaggtcgcggttgctgtcgtagttgagcttgagcaggtgcggcgcaatcgcatgggccgtgaccacgcccatcaccatcgtgtggccgtcggtggacttggccgtggcgtccgccgcgagcgtgttcgatgcgccgggccggttgtcgaccacgaccggctgcttgagcaagggcccgagccggtcggccaccgcgcgggccatggcatcggtgccgccgcccggcgccgagccgacatagatcttgatcgggcgtgcgggccagtcctgggcctgtgcggtgccggcgccaagtgccagcaaaccggcggccatggccgccatgagcgttcgtttcatctgctttgtctccgactgattttcgaaatcctcggcgcccatcgtaggcaggcgattgatcctcgtaaactgaaagatcttgatcgatcaataaccggaggtgatcaaaaaatgggctccatcgacaagcaggacaccacgccccagttgctcaaccggctgcgcatgcggcagatcgccctcatcctggcaatcgaggaccggcgcaccctgcgcgccgcggcgggccagctcggcctgacgcagccggcggccaccaagatgctccatgaactcgaaagcgcgctcggccagtcgctgttcgaccgcgtcggccggggcctgcagctcaacccggccggcgagcgcgtgaccggctacttccgcagcattcgcggcagcatggaggcgctgaatcgcgaactcggcgaactgcggctcggcagcgcgggcaggttctcggtcggcagcatcatggccgcctcacccggacacctgaccgaggcgctgctcggcctgaaggcgctgttcccgctgctgtcggtggagatcgcggtcgacacaagcgaccgcctgctggcgcagctgcgcgagggcgtgctcgaagtggtgatcggccggctggtgagccagccgggcttcgactgcgtgttcagggccatcgaggacgagggacttgcggtggtggtgggcaacgaccatccgctggcgcgcaagcgcaaggtggagttcgagatgctgctggactacccctggatactgcagccggccggcagcccgatgcgcgacctgatcgagcacgagtttcgcgatcatcacgcgccgctgcccaaggggctgatcgagacgggctccattctcaccaccgtcaacctgatccggcgctcgcagatgatcgcggtggtccccgaggccatggcgcaccgggacgccgagcacgggctgcttcacatcgtgcgctaccgcatccgccagaagctcgaagcctacggcagcctggtgcgcaaggaccgcccgctgaccaagcccgcggagcattttctcgaactggtgcatgccaggccgaaggccggccgcgcggagtagccgcagggcgcgtgtagaaattgtcctgcatcgacgatggcattcgtccggcccggcgacattttccggctgcgaaactgccgtctcccaaccacttggagaccccgatgccggacgacatggagatccgcgttccgcagaacgatgagcgaatcgacatcaccgacctgaaagaggtcgactactggacgaagtggttcggcgtcagcgaggcgcggctgcgcatggccgtcgcgtccgccggcaccatcagggacgatctgcgggtctaccttggccttccctgaagcgcgaagcgcgcgggtgcccgtcggccttcgctgaccatgacacccgcctttgcctgagcgctgcgctacggcgcccgcaccaccatcggggctccttcaggagattgccccatgaacacaccatccccgtcgccttcgccgcgcccgaagcgttcccccgacgaacctgaaatcacccaggaagagtccgtgcccacggacggaaccgaccccgagggcgaggcaatgatgaaaaaggtcgagaacaggaagctcgaggatcgtggcgacgccgagcgcaagacgcccgacaagtcctgatccgcaacccggcgcagtggctttgtcttcttgcgaagaacggcgattccctacaaccgccgccgcagcgccttgatagaaccctcgggtggcagaggcggcttggcctgcggagccttttcgccgcggttggcggggagaacagggcagaaaagttcgcctgtccgtacgacggaggaagaaatgaaactcgacggcgcggccgggtcggtcatgcaggaaagcctgatgcaggtgggcgtgccggggctcgacgatgttcttggcggcgggctcacgtccaatcgcctctacctcgtcgaaggtacgcccggcgccggcaagaccaccatcgcacttcaattcctgatcgaaggggcgaagcggggcgaatcggtgctgtacgtcaccctttcggaaacgggacgcgaactgcgcggcgtggcgcattcccatggatgggacctcggtggcatcgaagtgcgcgagatgcttccaacggaagccgcgctcgaacccgacgagcagtacacgatgttccatccctccgaggtcgagctcagcgagacgacgttgaggatcctgtcggacgtcgacgtgctcaagccgtcccgggtggtgttcgattcgctctccgagttgcgcctcctggcgggcagttccctgcgctacaggcggcagattcttgcgctcaagcaattctttgcgggccgccaatgcaccgtgctgctgctcgacgacatgaccgccatgaagcacgacctgcaggtgcagagcattgcccacgccgtcttgcgcctggagcagatcagctccgactacggcgccgcgcggcgccggctggtcgtcaccaaataccggggccagcagtttcggggtggctatcacgactaccgcatcgagcgtggcgggctgcgtgtgttccctcgcctggtggcggccgaacatgcgtcggagctgtcgcaggcgcgaattcccagcggtatcgattcactcgatgccttgctgggcggcggcatcgagcggggcacgagcacgctgttcgtcggcgcgccgggcaccggcaagtcgacggtcgcggtccagtttgcgctggctgcggcgcagcgcggcgaatgcgcggccctcttcatcttcgacgagagcattcatacgctgcgcacgcgctgcgaaagcatgggcatggacctggcgccgcacatcgaagccgggcgcatcaaggtgcggcaggtcgaccctgcggagctgtctccgggcgagttcgtgcacctgatccggctggcggtggtcgagtcgggtgcggcggtggtggtgatcgacagcctcaacggctatctcaacgccatgcccgacgagcgctttttgatcgcgcagctccacgagctgctttcctatctggggcaggccggcgtcgccacgctgctggtgggcgcgcagcacggcctcatcggcatgcagatgcagacgcccgtggatgcgagctacctggcggacgccgtggtgctgctgcgctacttcgagctcgacggcgaagtgcgccaggcgatctcggtgctgaagaagcgcggcggtgcgcacgagcggaccatccgcgatttctccatgacatccacgggcctgcacgtaggcgagccgctgcgcaatttccgaggcatcctgacgggtatccccattcccatcgacggcgtgcatcccgcatcgtgagctcgctacccgcatccgtcgagcagcgcatcctgttgcgcaccgcgacctccagggatgctttcatggcgagcgccgtgctgggacgtgcgcaggtcaccgcgcatatctgcgcaaacttgtgcgaactggtgcgtgggctccaggaaggtgccggtgccatcatgctggcggaagaagtgctgtccgatccggctgccgccgcgttgaccgaagcgctggccgcgcagcccccctggtccgatctgccggtgctcatcctggcccgccagggcgccgactcgccggtcatcgccgcggccatggaccggctcgcgaacgttacggtgatcgaacggccgatgcgcgtggcctcgctgatcagcacggttcgcacggctctgcgggcgcgcaaccggcagtaccagctgcgcgacctgctcgatggcctgcgcgagtcggaccagcgcaagaccgagttccttgccacactggcgcacgaactgcgcaacccgctcgcccccatgagcaccgcgctgaccctcttgatgcgaaagccgcacgagcatgcggaggcccagcgctactacgagctcatgggccggcagatcgagcacatggtgcggctcgtgaacgacctgatggaggtctcgcgcatcacgcgcggaaagatcgagctgcgcatggaagccgtcgcgctcgaagcggtgatcaaggatgccatcgagctgagccgccctttgctcgaaggctccagccacacattgagcgtggagctgtgccgccagccgctggtggtgcggggcgacggcgttcgcctcacgcaggttttttcgaacctgctgaacaacgccgcaaagtacaccgcgcccggtggaaagatccgcatcgttcttcgcgaggaagggcgcagcgccgtggtcgaagtgtgggacaacggcacgggcattgcgcccgagatgctgaagtcgatcttcgagatgttcgtgcaggtgagcggcacctccaaggcggcgcaaggggggctgggcatcgggctgaccctggtcaagagcctggtcgaactccatggcggcagcgtggaggcgaagagcgacgggctcggctgcggcgcgatgttctgcgtgcgcctgccgctcacgcggctcgaggcgggcgtgccccaggcgccattgccagccattcgcggctggcctacatcgttgccgggcacggtgctgatcgtcgacgacaaccgggatgcggccgatgcgctcggcgatctgctgcgctcgcttggcgcttcgacgcgtgtggcctacagcggcgatgccgcgctgcgcatgatcgccgacggcccgcggcccgggcttgccattctggacatcggcatgccgggcatggacggctgcgaactggccgagaagctgcgcgccgatcccgcacttgccgggctggtcctcgtcgcattgaccggttggggacagcgcggcgacagagagcgcatcgcaagggcgggcttcgaccatcacctgctcaagccgctcgatctggcggcgctgttctcgattctgcggggccggtcatgaaccacgatgcgtccacgctctctgcggccgcccgctcggcccacaggccttcgctctggcgacgctgccgccgatgggtgctgccgctggtgggggttgcggtgctcgggctgctgctgtcgcatgcgcacaaggtcgactgggcgggcgcatgggaggcgctgcagcgctatccggcgacgctgctgctcggggtgctcgggattgcaaccgcaagccatgcgctctacggctgctacgacctgatcggccggcagcacacccgccaccgggtgccgcgctggcgcacctgggccatcgccgtcgccagctatgccttcaatctcaacctgggttcgctggtcggtggcgttgcgctgcgcgcgcggctctacgcgcgcgccggcctcgatgaaaccgtggtggcgcagatcgtgggtgtcagcctggcgaccaactggctcggctacgggctcctggccggcggcctgttcgcggccggcgtcatcgcgccgccgcgccaggcgagcatcggggcggacgcactgcgcgccctgggcgtggtgatgatccttctcgcggcggcctacgtgttggcctgcgctttttcgcgcgggcggcaatggcaggtgcgagggcggcggctgaggctgccttccgccaagctcgcgctcatgcagctcacgctctccaccgccaactgggcgctgatgggctgcgccatgtacctgctgctcggccgccaggtgccgtatgcaaccacgctgagcgttctgctggccgcggccatcgtcggcgtgatcacgccgattcccgccgggctcggcgtcctggaggccgtgtacctggcgctgctctcgggcagcgtgcgccagggtgcgctgatgggcgccgtgctggcctaccgcgcgctttactacctgctgccgctgggcgggggcatcgtgctctacctgcttctcgaacgccatgcggcaagccatccgcaaggcggtgcggaggccgacgcaccatggcgcgcgcaaacccgctgaagcgctacaaggagaagcgcaacttcggcgtcacgcccgagccggaggaagggggcgcatcggcgcctggcacgctgcagttcgtggtgcagaagcactgggcgacccggctgcactacgactttcgcatcgagctcgatggcgccatgaaaagctgggcggtgcccaaggggccgagctacgacacgcacgacaagcggatggccgtgcacgtcgaggaccacccgatctcctacaaccagttcgaaggcgagataccgcccaaacagtacggcgcgggcaaggtgatcatctgggacaagggcacctggaccccgctcggcgatgcgcgcaagggctacaaggaagggcacctgaagttcgaactgcacggctacaagctgcgcggcaaatgggcgctggtgcgcatgcataagaaagacgacaagcaggatgcgtggctcctgatcaaggagcacgacggctatgcccgtccggcggccgagttcagcgtggtggaccagtttccggacagcgtggccaagctgccgatgcccgagccggttgccgcggcgcctgctgctgttgctgttgctgctgcgacttcgccggcaaaacgcggcaaggcggctgtgcgaggcatgcccgccgatgcggtgaaagctgccatgccggccaggctctcgccgctcctcgccacgctggtcgatggcccgccgcccgatccgcagaactggatcttcgagatcaagttcgacggctacaggctgctcgcccgcgtcgatgcgaaaggcgtgcagctcttcacgcgcaacggccacgactggagcagccgcatgccgcacctggtgcacgccatcgaacgcatgaagctcaagccgggctggctcgatggcgaggtggtggtgctcaacgaatccggcggcaccgactttcaggcgctgcagaacgcgttcgacaccgacaagacacgcaacatcgtcttttttcttttcgacctgccgtactacggcggcttcgatctcacccgcgtgccgctggtcgagcgccgcgcgctgctcgagacgctgcttgccaaggcgccgccggaaatccgcttcagcgacatcttcgatgcgccgccccaggacatcgtcgcctcggcctgcaagatcgggctcgagggcgtcatcggcaagagaaagaacagcggttatgcatcgcggcgctcgcccgactggatcaagctcaagtgctcgttgcggcaggagttcgtcatcggcggctataccgatcccaagggctcgcgggtgggcattggggcgttgctgatcggcgtgcacgacgagaagggcgacctcatctacgcgggtgcggtgggcgccggcttcaatggccgcacgctggtcgacatgctcgaaaggctgaagccgcttggcatcggcaagcggccgttcaagaaccccaccgagaacgatcgccgcgcgcactgggtcaagccggcgctgctggccgaggttactttttccgaatggaccaaggacggccatgtgcgccacccggtgttccacagcgtgcgcaccgacaagccggcaaaggccatcatccgcgagaagccggttcaccaggcgggtgcggaccgcgaacccgaggccggacccgcacccgccgccacgatgcccgccaacttcaaggtctcgcatgccgatcgcgtcgtcgatccgtccaccggcatcacgaaggtggaggtggtgcgcttctacggactggtcgcgccgctgatgatggagcacctcaagggccggccggtgtccttcgtgcgcgcgccgcagggcatcaagggccagcttttcttccagaagcatctcgaagaggggcagatggcgggcgtgcgtcaactcgatccggcgctgtggcccgcgcatcccgagctgatcgaagtggcgggcccgctcggcctcttgagcgctgcgcagatgaacgtcatcgagttccacacctggaacggcgtgaagacactcatcggaaaacccgaccgcatgaccttcgacctcgatccgggcgagggcgtcggctggcccaccgtgcaacaggcggccgagctgatgcgcgtggtgctcgacgagctcggcctgccttccttctgcaagacgagcgggggcaaaggcctccacgtggtggtgccgctgaagcggcagtacgactgggacaccgtgaaggatttttcgcaggccatcgtgcagcacatggcccgcaccttgccgcagatgttcgtggcgaagagcgggccgagcaatcgcgtcggccgcatcttcatcgactacttgcgcaatggtttcggcgcgaccaccgtctgcgcgtggtcggtgagggctcggcccggaatgggcgtgtcggtgccggtggagtggcaggaggttcccacgctcgcgagcggcgcgcagtggacgctgcgaaacatccatgcccggctcgatcggggcaacgagccgtgggccggctatgcaaaggcggcgaagagtccgggcgccgcaatgaagatgctggggttcgaagcaagcagtgcgcgtgcacgcaagcgctgacgccgcgccccaatcgaagcgcttggcgatgcgccgaagtcaggtcagagttcgatgaaggccgaggtggctttgttcagcgccagcttgcccttggcagtgatcgattccacctgggcgagatgacggatcgcacgatcgtcgggcgcgtggctggtggtgggaggaatgaaagcggtcaccagctcggcggcccgcagcacgcgcagcctgtcgatgtcggctggcgtatggacgacgtatggcaatctctgctcggcgaggacccgaagaaactccatggacatgagccgtctccttgtctagatatggacgtgcattttgcggaaaaattcgcagttgtgcctagtccctgcagtgcacattacctttgcatgtgtaccgaagtgttgtcctgccgctgcggccgaaaacgaaggtgccaattttcagggcaggccgattgcggggtcttcgctggttaccggtatcgggtgccgccgatgcgatcgagggcgcgctacgccgcgttaccgctcatgctttgatgaaccgactcgttcgtacgtcacgaagctgtaatcgaggccttccttggccgagacgtgcgattcgcgactcgtctcgcgccactcggaggcagagagttccggcgcatgcgcatcgccttcgtagtcgcgcgcaatctcggtgacgacagcttgctgtgccagcggctcggcctcggcatagatctgcgcaccgccgatgatccatacgtcgggcacctgcgattcttcgcacagcgagagcgcctcttgaagattgcccgcgcgctgcgcgccttcggctttccagtcgtcctgccgcgtgacgacgatgttgcgccggcctggcaagggacggaaccgcggcggaagcgagtcccaggtcttgcggcccatgatgacgggcgcgccgccggtcgtccgcttgaagtgcgccaggtcttcgggcaggtgccagggcatggtgccgttggcaccgatcacgccattggcggcgcgggcgaagatgagattgatgcgcggtgatgtgttcatgaggccgaacggtccgctcacaccgccacgggcgccttgatggcctcgtggtgcttgtagtcgagcacttcgaagtcttcgtactggtagtcgaagatcgaagccggcttgcgcttgatgtggagcgtgggatacgggtagggcgcacggctcagttgcagcgccacctgttcggcgtggttgctgtagatgtggcagtcgccgccggtccagatgaagtcgcccacgtcgagatcgcactgctgcgccatcatgtgcgtgagcagcgcgtagctcgcgatgttgaagggcacgccaaggaagatgtcggcgctgcgctgatagagctggcagctgagcttgccgcgctcgcccggtgcctgcggcggcgccacgtagaactggaagaacgcatggcagggcatgagcgccatcttcgagagctcggccacgttccatgcactgacgatgatgcggcgcgaatcggggttggtcttcagggtcttgatgacttcggagatctggtcgatgtggccgccatcgggcgtgggccagctgcgccattgcacgccgtacaccgggcccaggtcgccgtcctcgcgcgcccattcgtcccagatggtgacgccgcgctccttgagccagttgttgttgctggagccggtcaagaaccacagcagctcctgaatgatggaccgcaggtgcaccttcttggtggtgaccagcggaaaaccttcgttcaggtcgaagcgcatctggtggccgaacacgctcttggtgcccgtgcccgtgcggtcgctcttgtggacgccatgggtgtccacgtggcgcatgaagtcttcgtactgggagcggatggggcgggcaggcgtggaggtcatggggagaggtgtcgggaccggggtgttcgaattttacggactgattgctttcttgctccttccccctttgggggaaggttgggatgggggcggctgccgtcgtgcccccaccccgaccctcccccggaaggggagggagaaagagcgaagctacacgcggatcacgcggcccgggttcaggatgttctgcggatcgagcccgcgcttgatcgcgcgcatcatttccagcgccacaggcgacttgtgtttttcgagcttgtcgaccttgagcgaacccacgccgtgctcggccgagaacgagccgccgaacttctcgacggcgtcgtacaccagcgtgttgatccgctcttcctcgttcttcaggaaagccttggtgtcgatgttctcgggcgcctgcacgttgtagtgcaggttgccgtcgcccaggtggccgaagttcaccagccgcacgccggcgatctcgcgtgccagcagggcgtcggtctcggccacgaaggcggggatgctggagacgggaatcgagatgtcgtgcttgatgttcaagccctcttcggcctgcgcgaggggaatgctctcgcggatgtgccagagctgatgcgcctgcgcaaggttctcggccaccactgcatcggtcacgcagccgtcttcgaatgcggtttcgagcagcgcctcgaagcgcgcgcgcgcatggtcttcggactcgctgtcggagttctccagcaaaacgcaatagggcacggcctcgtcgccgatgaagggaacgcgcagttgcggcatgtgcttgtcgaccaggctcaatgcaaacctgcccatcacttcgaagcccgtgaggcccgagcccaggtgcttgtgcgcaaggcccagcagcgtgaccgcgtgatcgagcgagggcaccgcggcccaggctgtgagctgcgccgcgggcagcgggtagagcttcatcgtcgccgcggtgatgatgccgagcgtgccttcgctgccgatcatcaggtcgcgcaggtcgtagccggtgttgtccttgcgcaggccgctggtgccctcccagatctcgccctgcggcgtgaccacttcgaggcccaggcacagctcgcgcgtgttgccgtagcggaccacctgcgtgccgccggcgttggtggccaggttgccgccgatggtgcagctgccttcggccgcaaggctcagcggaaacaggtagccctgcttctcggccgtctcttgcagggtctgcaggatgcagccggcttccacggtcatcgtgaggttggccgcatcgacggtgcgaatcgcgttcagccgctgcaggctcagcaccacctgcgtgccgctgtcgtcgggaatggagccgaccgccaggccggtgttgccgccttgcggcacgatggccgtgccggccgcggcgcaggccttgaccacgtcggccacctgttgcgcattggcgggccgcaccacggccagcgacttgccgcgtgcgcgcttgcgccagtcctgttcgtaggcggtgagatcgccttcgttcagcacgtgttgcgcacccacgatggcgcgcagctggtcgatcaagggagaagaagtcatggggtggaagcctccagttggcgggcagccttggcgttgcgcaggcgcagccggacgtgcaatgcgcaggccgtgaagagcgcaaggcacagcagcacctcgatgagcgcgagcacttggcccacgccgttggtgtcgctccaggcgcgcaccacgccctcggtgaaatagagccagaccatcaggctgacccagcggtaggtgtacatgcggttcttgtagagccccgcgagtggaatgaccagcggcagcaccttgagcgccagcagcgagccgcccggccgcagcggcgccagccacagctcccaggccaggcccagcacgatgagtccggcgaggctgcccacggcaagccatcgggtggtgctgacggaagaagaggcgtgcggtgtgatggtttgcatggattggacaccgcggaactggcgacacgaagcgtgcgaagacgagaagagggttcgggttcttatgataccggccatgaatcgtcagcagctctggagggatctttcgcgctttccgtggggcaacaccgcggcggtgctgggtgagcgtttccgggaagaccggctcggcctgacggccagcagccttaccttcaccaccaccattgccatggtgccgttctttacggtggcgctggcgctttttaccgtgttcccgatgttcgccaagctgcagggacggctgcagcgctggctcatcgagagcctgattcccgacaacatcgcgcgccaggtgctgggctacctgaaccagttctccagcaaggccggcggcctgggcatcgcgggcctggtggtgctcctgatcaccgccattgcgctgatcctcaccatcgacaagacgctcaacaacatctggcgcgtgcgttcgccccggccttttgcgcagcgcgtgctgatctactgggccgccatcacgctcggcccgctgatcctggcggtgagcctctcgaccacttcatacgtgttcgccgcgtcgcgcgacgtgatgggcggcagcatcctcaagctgttcttcgacaccttcgaagtcgtgctgctcgcgggcggcatggcgtcgctctaccactatgtgcccaacaccaatgtgcgctgggcgcacgcctgggccggcggcatcttcgtggcggccgccatcgaaattgccaagcgcgtgctgggctactacctgagcctggtgccgacctattcggtgctctacggcgcctttgccacggtgccgatcctgctcgtgtggatctacgtggcctgggtcatcgtgctgctgggcgccgtgatcgcggcctatctgccgagcctcttgaccggcgttgcgcgccgcggcggccgggccggatggccgctgcaattggcgatggaggtgctgcagcacctggcgcgggctcgcgccacgccggccaagggcatgggggccgccgagcttgtcgcccacatgcgcgtcgacacgctgcagctggtgccggtgctcgaaacgctggtgatgctcgactggattgcgccgcttgccgaagagaccgccgacgaagacccgcgctacgtgctgctggccgacccgtccacgcccatcgagccgcttctcaaggagttgctgatgccgcgcgccgaaccgctcgaagacctgtggcaaaaaggcccgctgcactcgctgcgcctgggcgatgtgctattgatttaatagcggtcagatcttcaccttgcccagccagatgtcgcggtacatcgcccagtcgcccatgaagctgtagagcgggcgcttgaacgacgcgggcctgttcttctcgaagccgaagtgcccgacccaggcaaagccgtagcccgcgaccagcccggccaggagccagagcgggttgagcgtgacgatcagcgccaccaggcacagcagcgaaatcgtcgagccaatgaagtgcaggcgccggcaggtgcggttggcgtgctcggtcaggtagaacggatagaactccgcaaagctcttgaaacgtcgcggatcgacggcagattccggggcagtcgtggtgttcatcgggcgagcctcctgagcgccgggagcgctttgtccataatagccacgaccctcccgccgggccatcccggctccgtattcacaccttcaccgcatcagctttgagcgctcttcccgccgcccccgattccgccgagccggcccgcgatgcgccatgggtcgtgtgcctgtgcgccgaatggtgcggcacctgccgcgactaccggccgctgctcgagcaggtggcgcgggcgcatccgcagttccgctttgcctgggtcgacatcgaagaccacgccgagattgccgatgccttcgacgtcgagacctttccgacattgctgatcgccggtgtcgacggcacgcgctttctgggccctttgctgccgcatgccgagacgctctcgcgcatgctcggcgcgctgcaggcgccgcagccttccagcctcgacgtcgacctgctgctggcagtgctcgagaagcgccccgctgaattcgcggtctgaaccgcgcgctccctgccatgaacatcctgatctttggcgccaccggcatggtggggcagggcgtgctgcgcgaatgcctgcttgcgcccgacgtggcgcgcgtggtcgcggtcggccgaagagccaccgggcagcagcacccgaagctgcaggacctggtcatcccaaacatggccgactacagcggcttcgagccgcagctgcagggcttcgatgcctgtttcttctgccttggcgtgtcgtcggtcggcatgaaagaggccgactacaagcgcatcacctacgacctcacgatggccgcggccacggtgctcgcgcggctcaacccgggcatgaccttcacctacgtgacgggtgcgggcaccgacagcagcgagcgcggcagcagcatgtgggcgcgcgtgaagggcgccaccgaaaacgccttgctgaagttgccgttcaaggccgcctacatgttccgtcccggcatgatccagccgctgcacggcgtgcgttcgaagacgccgctctaccaggccgcgatcatggtgctcaagccggtcctcgggctcgcgtaccggctgtggcccgacaaggtgacgacgaccgagaaggtgggccgggcgatgctggccgtggcgcggcacggtgcgccgaaggtgctgctcgacccggcggacatcaacgccctgggccgctgaagctcacgcggcctcggccgcgctggaacgcgcgcggcccagcttgcgcctgcccgcgctggcaatggcatgcaccaggtgttgtacgaactcttgcgccagcggcgtgagcgtgcggccttcgagcgccagcacctgcagttgccgctgctgcagcggcgcctcggcaaacgggcgtgccaccaccgtgcccgcatcgatgaggtgcgtgaccgtgaggtgccccgaaagcatcacgtccggcgtgcgcaagagcggcagcagcacggatgaaaagttgctcacgaagatcgcgcggtactgcagcccctgcaggctgcatgcttggtcgaaaagctgccgcgcggtcacgcccttgtcgcccacggccagcggatagcgcacggcgtccgccaccgacaccacgcgctgccgcgccagcggatggtcggggcgcagcacggcaaacaccggcgcattggccgagtgctcgatcttcagtccgggctccggcgcaacgacgtacttcagcgcgatgtcggcctcgccgcgcgcaagcaacgcgctcacgccgtcgggcgagcccacgtggagttcgagctgcgtgcccggatgcgccgactcgaagctgcgcatgacctgcggcatgaagtgcgccgcgaacccttcggtgcacgccatgcggatgcggtgcgcgctgcggccgccgaggtcgcgcacctgctcgatgacttgctcgatgtcgagctgggcattgcgcaagtgcgccgcgagccgctcgcccgccgcggtgagcgccatgcccctggcgtggcgctcgaacagcggcgtgcccaggctgtcttcgagcttggcgatctggcggctgaccgccgacgaagccacgaacagccgcgccgccgcctggctgaccgagccgctgcgtgccacttccaggaaatggcgcatcggaatgctgaggagcggtggtgtcatgaccattcaagcgttgccttgaaggcaatggtagcttgcaaaaacggtgctggaagcattgcccttcaggccttgtacttgctgcacccgatggaaacaggaaatcccttcatgcaacgtaccgaaagccttgccgctgccgccgcctatttcgacgacggcagcttctttgccgacctgaagcggcgcgtcgcctttcggaccgagagcgataccggcgccgccacgcccgcgctcggcgcctacctgcgcgatgagctggtgccgccgctggccgcgctgggtttcgcgtgcgaaatcgtcgagaaccccgtggccggcggcgggcccttcctgatcgcgcgccgcatcgaagaccctgcactgcccaccgtgctgagctatggccacggcgacgtggtgagcgggcaggatgcgcagtgggacgaagggctcgggccctgggcgctcaccgtgcgcggcgaccgctggtacgggcgcggcaccgccgacaacaagggccagcacaccattgcgctcggcggactggcggccacgctgcgcgcgcggggcgggcgcctgggctacaacatcacctggctcatcgagaccggcgaagaggccgcgtcgccgggccttcatgcggtgtgcgagcagcagcgcgacaggctgcgtgccgacctgttcatcgccagcgacgggccgcgcgtgagcgccgcgcggccgacgctgttcctcggctcgcgaggtgccgtcaacttcagcttgcggttgcgtgcccgggcgcggggctaccactcgggcaactggggcggcgtgctggccaatccggccacggtgctgagccacgccgtggcatcgctggtggatgcgcgcgggcgcatcctggtcgaggccttgcggccgcctgaaattccgcagggcgtgcgcgaggcgctggccgacatcgccatcggcggcggtgccgacgatcccgcgctcgacgagggttggggcgagccgggcctccgcccggccgagcggctggtggcgtggaacaccatcgaggtgctcgcgctcggcgccggctcgccgcagcggccggtgaatgcgattccgtccgaggcggtggcgcattgccagctgcgcttcgtggtcggaacgccgtggcgcgatctggcgaagctcgtgcgtgcgcatctcgatgcgcacggcttcggccaggtggaagtgcaggtcacgctcgaaggcgcggcgacgcggctcgacgtggagaacccgtgggtcgactgggcccggcgctccatcgaagagagcagcggccagcgcgtcgacctgctgcccaacctcgcgggctcgctgcccaacgatgtctttgccgacctgctgggcctgcccacgctgtgggtgccgcattcgtacccggcctgcgcccaacacgcgcccaacgaacacctgctggcgccgctggcgcgcgagggcctgcagatcatggccggcctctactgggacctgggggagccggggctggctccctgggccgccggaaaaacgcagcacgccgccgcctgatttctcttcctggaccgaacccatgaaaactgctctcttccaacgccttggcggcctgctggcttgcgcttcggccctcatcgccttccccaatgctcccgcgcttgcgcaggacacctggcccgacaggcccgtgaagctggtcgtgccatttccgcccggcggcggcaccgacatcgtcgcgcgcgccatgggccagggcctgtcggagcggctcggccaaccggtggtcatcgacaacaagcccggtgccgccaccatcatcggcaccgacgcggtcgccaaggccgcgcccgacggctacacgctgctgctctcgggctccaccagctacagcgtgaatcccgcgctgcgcgccaggctgccgtacgacccggtgcgcgacctggcgcccattgccatcgtcgcgcgcacgccgctggtgctggtggtgggcgccggcacgccgtggcgctcgctgcccgagctcatcgccgccgccaaggccaagccgaagagcatccgctacgccaccttcggctccggctcggggccgcacctggcgggcgagctgtttgcgctggccgcgggcatccaactgcaggacattccgtacaagggcagcagccagggttcgatggcggtgatcggcggagagatcgaaatcggcctggacactgtggccgccgtggcaccgcacgtgcgctcaggcaagctgcgcgcgctgggtatcgtgggcgcgacgcggtccagcatgctgcccgaggtgcgcactctggccgagcaggggctgcccgatgccaccttcgatgcctggtacggctttgccgcgccggcgcgcacgccggcaccggtgctcgacaagctggcccgcgcggtcacggccacgatgggcagcccggccctgcaggcgcagctgcgcgcgcagggcatggagcccgtcgccatcggcggcgcggcgttccgcagccagatggagggcgagatttcgcgctaccgcgcgctggcgcatcgcgcggggatcgcggcggagtagccggcgattggctcaggcaggcgttccgacgaagtcgcgcagcgcgaacagcacttcgtcgggggcctcgttcatcagcgagtggcccgcatgcacggtcaccaccttggccttcttcgccttgccgaccagcgccttggtggcgcgcggtggcgtcatctggtcggcatcgccaagcaggaaaagcacggggcactgcacggcctcgatcgctttttcgccattggcgtagtcgttgcaggccttgaagccgacgtgaaagacgttgacgtcgcggttgctcgcgagcacgcggcgcatcagcgcgcgcgaactgccgtagagccaggtgcccgggccaagcgccgagggcggcggcgcgagcagcgaatgcgagaaggtgttgaccatcgcgatggcgcgttgcggatcgttgagcgcaccatcgagcagcgcgggcgacacggtcatcggataggcggtgcccaccaacgccagatgggtcacccgttcgggcgcgcgtgaagcggcctcgagcgcaatcagcgagccgaagctgtggcccacgagcgcggccttctgcacgccggccgcgtcgagcagcgcgatgacgaactgcgcggcgtcttccacgctggcgggtggtgggccttcgctcttgcagtggccgggcaggtcgagcgcgagcacgttccagccgtggttggcgaaccagcggctctgcaggatccacacgctgtggtcattgagcacgccgtggatgaaaaccacggtcggcttggttgcatcgaaagttttgccgccggtgtagcagtaggtggtgtggccgttgactttgtagttcatgtcagttgctccgtcctgagatgcgtcgctgttgttcagggcgcgtgcacaggctaccgggtactcccctccgcgaatgtcccccgccttcggctcccgcagctcctcctttgtttcgctgcggggtgcacccggcgccctgtgcacaccaggcgctgcggttgttccgcctgatcaacgaccgctctgcataacgagcacgctgatggggtgccttgcgcagcgaaataaagggggaggccgcaggccggaggacattcgcggagcaaggtaccccgtcggcgggatcgcgccccgaacacaacgcgccaaactcgacacgacgaacaaagaaacaagcgttcattcctagacccccgccttttccgcagccttcagcgcacgcttcaggtcgtcgatcaggtccgccgggtcttccagcccgatggaaagccggatcgtcccttgggaaatgcccgcacccgccagcgcctcgtcggtcatgcggaagtgcgtggtgctggccgggtggatcaccaggctgcggcaatcgcccacattggccaggtggctgaagagcttcagcgcctcgatgaaagccttgccctgcgcgcggctgcccttgatgtcgaagctgaacaccgcgccggcgccgcgtgcgccatggcgcagcagcttctgggctagtgcatggctcggatgcgattcgatcagcgggtgacccacgcgcgacacgaacgggtggctcacaaggaattcgaccaccttctgcgtgttgtcgatatgccgttccatgcgcagcggcagcgtctcgataccctgcaagatcagccacgccgtgtgggggctcatcgacgcgccgaagtcgcgcagcccttcgcgccgggcgcgcagcaagaacgcgccgaccgtgctttcctcgctgaagaccatgttgtggaagccgtcgtaggcctgcgtgagctcggcgaattttcccgatttctcccagtcgaagctgccgccgtcgaccaccacgccgccaatcaccgtgccgtggcccgagaggaacttggtcgccgagtggtagaccaggtcggcaccgtggtcgaagggcttgatgaggtagggcgaggtcagcgtggaatcgaccagcagcgggacgcccgccgcgtgcgcgatgtcgctcaccgccggaatgtcgagcacgtcgagcccggggttgcccacggtttcgccgaacagcagcttggtttcgggccggatcgcggccttccagccatccaggtcgccgggcttcacgaacgtggtgtcgatgccgaagcgccgcatcgtgtagtgcagcaggttctgcgagccgccgtagagcgcggtgctcgccacgatgtgggagccagcacccatgagcgtggcgatcgacaggtgaagcgcggcctggccgctagcggtggcgatggcgccgatgccgccttcgagcgccgagacgcgctgctcgagcaccgcgttggtcgggttgctgatgcgcgagtagacatggcccgcgcgttcgaggttgaagagcgccgccgcgtggtcgctcgactcgaagacgaaagaggtggtgaggtggatcggcaccgcccgcgcgccggtggcggggtcgggtgcggcgccggcgtgcagcgcgagggtgtcgaatccggggtcggaatagccgggcatgaggacctttctgggttcgttcgcaatgccccgttacgtctgctaatcatgcgcgcgcatcatgggcgtgagagtcggcgccgattgtgggctatattcaaatcggcacgccgccgagaacgatttccgagaggagcacacgatgaaagtcagcgacatccttcgcgtcaagggcaacacgctcttcaccatcacgcctgacgacctgctggccgaagccgtcaacaccatggcggaaaaggacattggctccctggtggtcatggaacacggcgacctggtcggcatgctcaccttcagggaagtgatcctggccattgtcggcaacggcggtcaggtaggcggcatgcaggtgcgcaaggccatggacgacgcgcccgtgacctgcacgctcgaaaccgacctcgacgagatccgccgcatcatgctggagcgccatgcgcgctacatgcccgtgatggacaagcgcatgctgatgggcgtgatcagtttctacgacgtggccaaggcggtggtggacagccagaacttcgagaacaagatgctgaaagcgtatatccgcgactggcctgaagaacagtaactaccgcccctgcgctgggcgcctggcttattccttgatattggccgactgcacgatcttctgattccgggcgtattcggcctggacgaactggccgaattgctcgggcgtgccgctgccgggcagggcgccttgttcgttgagcttgctgcgcacctgttcctcggcgagcaccgcgttcagctcctggttgaggcgggccacgatcgctggcggggtcctggcgggggcgaagatgccggtccagctcaccatgtcgtaacccttgaggccgggcatctcgttgaaggtgggcacgttgggcagggcggcgaggcgctggctgccggtaatgcccagcgccttcaggcggttgccgttcacgtgcggaatggcgctggtgctgaccagcatggccagatcgacctggttgccgatcacgtcggtggcaatctgggcgccgccgcggtagggcacgtgggtcacgaagatgccgctgcgctgcttgagaagctccatggccaattgcagcaccgtgcccacgcccgaggtggcgtagttgtaggcgccgggcttggccttggcgagtttcacgaagtcggcataggtctgggcctcgaggccgggccgtgccaccagcaccatcggcgcggtgttgagcatgccgaccggggccagttccttgagcggatcgaacttgaaggccgaggggttgaccagccggccgatggcgatggcgctgtcgggtccgaccaccagcgtgtagccgtccggcgaggcgttcacggccttggccacgccgatggcgccgcccgcgccgctcacgttctcgatgaccaccgactgcttcagccgttcgcccagccgcgtggcgacgaggcgggcgttgacgtccacgctgccgcccgcggtgtagggaacgatcagcgtgatcggcctggcggcgggccatgcactctgcgcgagcgccgcggcaggcagtgccgaacagagggtggcggcaagaagaaggcggcgggagcggttcatggcgtgggtcattcctggtgggcgggatggggctatggcgcaaggcgcgcgcgcagcgcgtcgaactcgtggctccactgcgtgcgccatgcgcggcgctgcgtgtcgtcgatccatgcgccgtcgagcccgttgtgcatgaagccgcgcaggtcgtccagcccgaagccgaagtcgcgcgccatcatcagccaggcctctgtgggcgtgaccttgtgcagcgtcgggtcgtcggtgttggggtggatacgcaggcccagggcgggcatgcggcgaatggggtggtcgagcgcccagcgctcgggcggcagggtgcgcaggtagtacgagttggtgggcaccacggtaaagatcacgccgcgctcggcgcactggcgcgcgaagtcgggctggtcgaccacggtgtagccgtggtcgatgcggtccacctgcagcacgtcgagcgcggtgcgcacgttggtccacggcatgccgaactcgcccgcgtgcgcggtggccttgagccccgcgcgccgggcctcggcataggcctctacgaacagttcgggcggccggtcgacctcgcggtagtcgatgccgatgccgatcacctcgtcgcagcggtgggccttgacccactccaccatctccacggcggcctcggggctcgcctcgcggtcgatggcggcaatgagccggcccgtgatgccgaactcccgctgtgcgtcatggatcgcgcggacgatcgcgctttgcgccatcggatacgaaatgccggagccgtgcacggtgccggtcgggttccagaagaactcggcgtagcgcacgttgtgggccgccgcgtcttccaggtattcgcgggtcagctgatagaggtcatcggcgctgcgcaccagctgcgcgtcgagcgcgcgcagcacgcgcagcacgccgaccggtttttccccgcgcgtatagaagccttcgatttcctcggccgcaagcggcgaaccggcgcgacggttgagttgcttgaaggtttcgtggcgcaccgtgccgaacaggtggcagtgcagctccaccttcggaatcccatgcagcatggattccagcgtgaggggcggtggggcggagctggtcatgcctgccagtctagggagcggaacgccataagcaaaattttgaatttctataatttgattcattgaatcgataacgggatcgccatggcttccttgccgcttcgggcgctcaccttgcgccagcttcagttcttctcggtgctggtggaagaagggcacttcggccgcgcggcgcgccggctggccattacccagcccgccctgagcaacgccatcaagcaaatggaaaaactgctcggcgccgaactgctgacccgttccacccatcgcctgcagctcacctccgtgggcgccgaagtgcttgcgcgcaccgatttcctggtcaacaccttcgaggtggcgctgcgcgacatcgaaagcacggtgcagcgcgggcgggctttcgtgcgcgtgggcgtgatcccgtcggccagcgcgcgcgtgacggccgcggccagcgagtttctggaggccggcgatcgcgaggtcgagatcgcctggcgcgacgcgccttccaccatcctgctggccgaactgcgcagcggccagctcgacatggcggtggctgcgatcaccgagccgccgggcggcctggcctgcatcgacctgttccgcgatccgctggtgctggtggtgcgtcgcgaccatgcgctggccgcggctgcagacacgagctgggaggccatcggcaaggagcggctggtgctgttcgaaagcggcagcatgccggcactcggcaacccggcgcgcgcgcagttcgaacagggggccgagccctatcgcgtgagctattccgaaacgctctatgcgctggtgcgcagcggccaggcgctgggactgatgccgcggctttatacctcgtcgctgcgcgaccccgagctggtggtgctgccgctgctgaagccgcgtgtcgagcggcgcgtggtactggcctacctgccggggccgatgcgcaacgtggtggcgcaggagctgattgctttcttgcgcgaacggctcccgcaggccggtgaggccgcggtgcggcgtgtggcggcgaagggaaagcgcagccggcgctgacgccggacagcaggttcagtacagctcggccgcggcgtggatggtttcgcgcacgcgcggatagatctgcgcgttccacttgctgccgctgaaaacgccgtaatgccccacgccggcttggagatgatgaaccttgaggtacggccggatgccggtgcagaggtcttgcgccgccaccgtctgcccgaccgagcagatgtcgtcgcgctcgccttccaccgtgagcagcgcggtgcggcggatggccgcggggttcaccgtgcggttgcccacggtgagcacgccgcgcggaaggtcgtaggtctggaacacgcgctccaccgtctccaggtagaactcggccggcaggtcgttcaccgccaggtattcgtcgtagaagaggccgatggtgcgggccttctcgatgtcgccctcgaccaggtggtggaccatgtcctggaactgcttcttgtggcgctcggggttcatgctcaggaaggccgagagctgcaggaagccggggtacacgcgccgcatcatgccggcatggggccacggcacgtggctgatgaggttgcggcgaaaccactcgatgggcttgctgttcgcgagctcgttcacgccggtggggttgacgcggcaatcgaccgggccggccatgagcgtgaggctgcgcggcgtggcggggttgtcgtcttcggccatcagcgccgtggcggccagcgcggccacgcagggctggcagaccgcgaccatgtgcacgcccgggccgatggcttcgaggaaccggatgacctgcagcgtatagtcgtcgaggctgaagccgccatgccacagcggcacgtcgcgcgcgttgtgccaatcggtcaggtagacgtcgtggtcgcgcagcagggtgcgcacggtttcgcgcagcagcgtcgcgaaatggcccgacagtggtgcaaccagcagcacgggcggatgcacggcctgcgtgtccttgcggaaatgcagcagggtgccgaagggcgaaaccagcgttatctcttcgtgcaccacggtttccacgccgtcgaccggcacgctggcaatggcgtagtcggggcgcgaatgggtcagccgcatgcgcgaaagcacgtcgaactgtgcggccatgcgccgcaacatggtgcgttcggtgccgtccttccaaagcgcctggccgaggtactgggctgcgagccgggagggcgagagcaggtcggcttggttctggtaggcccggtacaacatgaaagtagtacaggcaagttgcgggccaagcggtggcacaggccttgcacggccatgggagccaaccggcagcaagcaccgtcaaggagatccacgatggccaaacccgttctcacgatcagcagcaggaactacggcgcctgggcgttgcggggctggctgatgtgcaggctggccggactcgacttcagcgaaaagatcatcccgcccgacgacccggccatgaaggccgagatgctgctgctctcttcgtcgatgctggtgccctcgctgcagcacggcaatgtcaaggtgtgggacacgctggccatcggcgaatacctgaacgagatcaagcccaagggcgcgctgctgccggccgacatccaggcccgcgcgcactgccgcgccatctgcggcgagatgcattcgggcttcgcctccatgcgcggcgcattgccgatgaacatcaaggctcagttccgcggcttcaagatctggtcgcgcgcgcaggccgacatcgaccgcatcgtcgccatctggcgcgaatgcctgaagacctacggcgggccctttctcttcggcaagcagccgggcatggccgatgccatgtatgcgccggtggtcacgcgcttcctgagctacgacgtgccgctggacagcgcctgcgccgcgtactgcaagcgcgtgatggacttgcccgccatgaaggagtgggtggccgccgcgaaggaagagcccgaggaaatcgacgagctggatgcggagttctgacctgcccgcgtggggtgccggctagtgccggaacatccgcaggtcgagcgggctttcctcgccgagccacatggcatgcgccgtgtggtcggcaaagtcgtcgcccgtgacgccgtgcacgaagatgtcgaggccgtcgcgatgggcctcgagccattcgatgacctggtcgaactcggcggcgtcgaaggccagttggcagctccaatgcgtgtgcgggccgaccagccgctcgtgcacccgcccgaccaccaccatcagctcccggcccgcctgctcgcacagctgcctggcctgcgccaccgtggcggggccgaagtagacgtgggcgtggtattgcggatagaggttctcggggcggcgcggcatgatgcggtcattgtgaacccaaccggaagcgcccgctgtagcggaacacgtcgccgaaccagcggtggcgcagcaccatcttcatggtgaagcggtcggcgtcgtccgggtcgggccgctcctcgacgtaggcggttcccatcaacaggccgagcggcagcggcaggtgcagccggcccaggcgccagacgtagccgaggtcgcgaaacaccagcgcgccttcttccgcgctcaccgccaggcgcatgccgaggccgaatcgcacgtactcgatcacctcgccgccgcccgctggcgcgcgcgccatgtgtgagcgaaagtggaacggcgcgcggccctcgaagctgaagacgcggtcccagtacaggagcgcgtcgccgggccggcagcggtagtgcacttcgatggggacacgggtgccggtgtagggaacgagcgcaccgaacaggcggccgaagggcatcagcacgcgcgcccagggcgcatggtgcacctcgtccatcgtgccgcgcacgcacacgtgggcattcgagaacggggccatggtgtagtgccggcggatcacgtcgcccaactgctcccagcccgggccgagcgcctgctggaagacggggcgcatgtccttcatgcggccgccacggcggtttcgctgcgcgccttgtagaagcgcaggatgtgctcggagaagtcgcccagcagaaactgcgccacgcggtcggcataccagttgaagcgcgtgctcacgcgccaggaaacatcgatgcgaagctccgtgccgccctcgcgcggcgtgagcgtgtaggccgaatcgcgcaggtcgaaatagtggccgccgatcaccacgtggtcgtccagcgcgccagcgggaaaggaatcgggcgaaaagcggtagcgccagctcacgcgctgcagcggctgccactcggtgatgacctcctcgaagtgcacgtccttctgccactgcaccttgcgcacgcggccttcggcggtgtcttcggtcagggcgcccaccggcatcggcaccccgatgcgataggcccaggcatcgccgacttcgctcggccggatgtcacgcacttcgttgagttcatgccatacgcgctcggcaggcgcggcgatgaagagcgtgcgcgaggtgttcgagatctgttccgggttgggccagtgcggctcgaccgcacccagcgccagcggcagcaccgcgaagccgtagagcgcaggcttgggccaattggtgatgcggcagacgatgcccatcgcgaggccgccgaggctccccatgacgctgaacaggggcacgatgacgacggcgcagatcatcccttcgatgaacaccagcagcgtgccgacgacgaacaacgcggtcgagacccacggcgcccagatgtagtagccccagctgcgccgctcgatgcgctcggccatgtagaccgtgacagcgccgcacaccgcgggcgcaagatagatgaaggagcccagcatggccgagaagcgctggcccggcaggccgctgaaggcgatgcgaagcaccagcgctgccgcggcgccgacgatcagcggccagaaccatgcgaagggcatgcggcgcacgggcatgtcgcgcatctgcgcggcgtcggcctcgatgggtgccagttcccgggggctggcttcggcgggttcggtgctcatgaaagtttcttctcctcgtgtgttgttctggatccgacaggcgttcagccgctgcgcttcgcagtcaccatgcagtagtcgaagtcgcgccagaaaaagcccagcaccagcgcgcaataactggccacgatgtgcttgcggcgccaggggctcagcctgccgcgcgccttccagagttcggccagcgcaaagcgcgtggcaagcgccggaatgtgcagcgcgctgggcgccacgcgccatcgcagcgactgcacctcgatatcttcgaatccgtggtggcgcagcgcctcgacgaaatcgccgcgcacggccagcgtgggcacggcccagctgtcggcccacaggcggtgcagccagccggcaagccggcccggccgttgccgcagcaggaagccgtcgaccaccgcaagccgcgcacccggcttcagcaggcgggccgcctcgcgcacgaaatcggccttggacgtgccgctggcgtagcaggcgctttccacggcccaggcgccgtcggcctttgcggtgggcaggccggtgcgcgtgtagtcggcctcgatgtgcgccatgcggtcggccacgccggcacccgcgtcgagccgcacggcgatgctgttctgcaccggcacgttggtgaccgtgacggcatacagcgaagggttgtcgcccaccagcgtgcgtgcggtggcgccggcgccgcagccgaggtcgatcacgcagcggcgttgcggcgcctcctgcgtggaccggggctcgtcgagcttcagcgcgcggccgaccgcgcggttcatttccaccagcatgccttcgcgccgcagcgggttcagcccgagccgccagaagccgaagtgcatgttgtagctggggctccaggcgcggtagtcgtccgccacctcggtgaaatagtcctgcgtgtcggccttggtgatgggctgcgcggtttcgggcgagggcgcgtcggccgcaccggccattcgaggcacgcggaaatcgggctggaagacattcggcatgaaagctccttttttcagatccggcagttgccgctggcgcaggtgcgggacgaccgcgccgccttgccggcaagcagggccaccagccagcgcggcagccggtagcggttgcgcgcaagcacgccataggcgcggtcggcgaacggcgcgacccatggcaggtcgagcaggaagctgccactcggcaacccgacggcatcgcggcaagcccggatggcgggaacgccgacgaacacccggcccgccgcgtcgaccacgtggatggccgtcatcaaggcctcgcgcggcgccggcccggcatcgaacccggggggcgagcagtcgacgagttccagccgggcggctgaatcccgcgtcttcattgcgctcatttccgccgtgcagaggatgcaggtggcgtcgaaatacacggtgagcgggtaggcggcggtgaggtgcatgttgggtttttcgttgtttctgtcaaaacagaaataatcaggcaaaaaaaaggactcagatcatgggcaggctggcgtgatgggcgtcggggtcgtcgtcgtccttcttcgaggccggagtcgtcggcgccggggcatccccgcgaacgaacttctgcacgctggcgccgagcgtcagcaccttgtcgagtgtgccgggcgagagccgcagcatctcgtcggcccaggtggcgagcttgctcatcaggtccatggtggagcggatgcggtcttgcgcatcggccggctccttcaggaagtcggggctggagacgatctcgcgcagcacgcggatggtggggtcgaattcgcgctccttgcgctcgcgcaccacggtgcggaacagttcccacacgtcgacactggtctcgaaatagtcgcgccggtcgcccaggatgtgggtgacgcgcaccaggttccacgcctgcagttctttcaggctgttgctcacgttggagcgggccacgccaagcgtctcggagagttcttccgcgtgcatgggcttgccgcgtgcgaacagcagcgcatggatttgcgagaccgtgcggttgacgccccacatcgagcccatttccccccagtggagaacgaacttgcgttggatgtcggtgagttccatgcctcgaagtctaggattttagaaatttctgtcaagagagaaatgaaaattcgtttgctcggcaggtgcaattggaatactgtacaaataaacagtattcaaagagaaaggatctgccatgcccgccgcccacattcccatccacgccatcaagggccgcggcgccgccacgcgcctggcgcaccgtttttcgcgcgacgagcgcaacgctttcgacgacggctggggcacgctcgaagaaggcgctgccgaagccgaagagctgccgccgctcgccaccgaggtgcgcttcgaggacgtgaagtcggtgctgaacgaaaacgactcccccgatatttccttcgatcgttcgctcaacccgtaccgcggttgcgagcatggctgcatctactgctttgcccggcccacgcacagctatctcaatctctcgccggggctcgacttcgaaaccaagctcatcgccaagcgcaacatcgtggaggtgctgcgcagcgaactcgaccgcaagagctacaagccgagccacgtcgccatcggcaccgccaccgactgctaccaaccgatcgaacgcgagctgcggctcacccgttcggtgatcgagctgctgaaggaaacacggcatccgtttgcgctggtcaccaaatcgagcgcggtggagcgcgacctcgacctgatcgcacccatggccgccgagcacctggccgccgtgtacatcaccgtgaccacgctcgacggcgaactggcccgcaagctggagccgcgcgccgccgcgccgcaccggcggctgcgcaccatccgcacgttggccgaggcgggcgtgccggtgggggtgagcgtggcgccgcagattcccttcgtcaacgaagacatggaacaggtgctcgaggccgcatgggaggccggtgcgcgcagtgccttctacaccgtcatccggctgccgtgggaggtggcgccgctcttcaaggaatggctccagctgcactacccgcagcgcgcggaccgcatcatggcccgcatccacgagatgcgcggcggcaaggactacgacgctgactttgccacgcgcatgaagggctccgggttgtgggccgacctgattcgccagcgcttcgagaaggcggcgaaccgcatcggcttcaaccgcgagcgcattgcgctcgacctcagtgcgttccggccacctggcgcggcggggcagggcatcctgttctagggccggtcaatgccgatgccgttcgccatcggaactccctgctttcggcggaaaaagttttgcctcatgaagaggtcgatttggaagtagattcaagttcggccgatgcacggggaatgccccgtggttgcgccagaaaaggtatctatgaacggggtatggctggtcgtgatgggggtttcgggctgcggcaaatccagcctcggggctgcgctggcggtcgggttcgggctgccgctgatcgagggcgacgactaccacccgccggccaacgtcgagaagatgagccgaggcatcgcgctgaccgacgccgaccgcgccggctggctcgcgacgctggcgcatacgttggccaatgcgtcgcagggtgcggtgctcacctgttcggcgctcaagcagagctaccgggaccagttgcgcgcgggcgtgccgggactgcgcttcgtgttcatggagatcgagcgcgccgaagccgaaagccgcgtggccgcgcgggccggtgcgggcgagcacacgtttccggcgagcctggtcgccaaccagttcgcgacgctcgaatcaccggtcggcgagccgggtgtgctcgcgctcgatgcgaccgcgccattgggccagttggtcgcgcaggtgaaggcctggctgcccgccgattagtccttgctgccggcgcgcagcgcctcgagcaccacggacacgcggtccatcgtgtcggcgactgttttcagctcttcctcggtggccggcgccaccatcgccgtgaccaactcggcctggaccgccaggcccttctgtgccatggccatgccgtcaggcgtgagcgtgagccgccggatgcgcgcatcggcgctgtcgctttcgcgccgcacccagcccctggcttccatctgcgtgagcagcatgctgacgccgctcttggcgacgaagcagcgcgccgcgagcgcctgctgcgtgatgcccggcgtggtggcgatggtggccagcacctcgtgttcgccgacgcgcagcccgatggcagcgagccgcgaggtcatgaccgcatcgcagaggttgtaggcccgcaccaccgccagccaggcgagcgtgccgtggggcgacgagggagctctgtcgggttttccggacttcgggggttttgcggtggccattcgatatcgttcagtattgaacatatactgttcattgtcgaaccaattctagtcgcgccatgaacctctacctccgcctgctgatgaccctgctgcgggcctggcgcgcaccgcgcctggctccgggcgacacgctggagcggcggctgcgcgtgctgcccaatgacctcgacatcaacggccacatgaacaacggccgctacctgacgatcatcgacctgatgctggtcgaatacttcgtgcgcaccggctttgccgccaccatgctgcgccagggctggcggccgatgtcgggcggttcgctcatcagctaccggcgcggcctgaaccccttcgacgtgtacacgctgcgtttccggctcgacgcgaccgaccagcaatggaactacatgcgcttcgagttcgtcaaggacgacaaggtctgcgccgccggctacatgaagggcgccgcggtgggacacggcgggctggtgtccaacctcgagtcgtacgccgccatggggctggtgccgccagcgcatgcgctgccgccgccggtgcgcgactggatcgccgccgagcagggcgtgatgagcgccgcttggtaagccgcgccggcggcaagcccttggatcagccgatgacttcaggccagtcggtgtggaagaactggccttcgggcttgtcgacgcgctcgtacgtgtgggcaccgaagaagtcgcgctgcgcctgcagcaggttggccggcaagcgctccgtgcggtagctgtcgtagtaggccagcgaggcgctgaacgccggcaccggaatgccattgctcactgccagcgccaccacttcgcgccagttctgctgcgtgcggttgagcaggtccttgaagaaggggtcgagcatgaggttgccgagggcggggtcggtgcggtaggcgtcggtgatgcggttcaggaagcgggcgcgaatgatgcagccgccgcgccagatggccgcgatgcggccgaggtcgagcttccactccttcttctcgcccatggtctggacgaggtcgaagccctgcgtgtagctgatgaccttcgacgcatagagcgcgtcgtgcaccttggccaccagcgccttcttgtcgagcgagagctcgatcttcggcccctgcaacaccttgctggccgccacccgcgcttttttctgcgacgacagcacgcgcgcctcgaccgcggcgttgatggtgctgatgaccaccgcgttctcggccgcgttgaggagcgtccactggcctgtgcccttctggccggccttgtcgaggatgagatcgacgatcggctggccggtttccgggtctttctgctccagcgccttggcggtgatctggatcaggtagctctgcagctcgccctcgttccattcgttgaagatggcggccatctcgtcggtggtgaagcctgcggccttgaacaggctgtaggcctcgcagatcagctgcatgtcgccgtactcgatgccgttgtgcaccatcttcacgtagtggcccgcgccgccggggccgatgtggatcacgcagggctcgccgtccaccttggccgcaatgctctcgaaaatcggcttcatcacttcccaggtggaaagcggcccgcccggcatgatcgacggacccttgcgcgcgccttcttcgccgcccgacacgcccgcaccgatgaagcgcaggcccttggcttggaggtaggcgtcgcggcgttcggtgtcggtgtagaggctgttgccgccgtcgatgacgatgtcgtccttgtcgagcagcggaatcagctgctcgatgacctggtcgaccggtgcgccggccttcaccatgatctggatcttgcgcggccgggcgaggctctgcacaaactcctcgagcgtcctggcgccgaccagcttcttgccggggttctccgccacgaaggcttcggtggtggcttgggtgcggttgtacacactgacctggaagccgcggctttccacgttcagcaccaggttctggcccatcacggccaggccgatcaatccgaaatcgcttttgtccttgctcatggctcttctttcgtctgcggtaaatgtgacgggcattgtgccgggggtgccccggggctgccatcggagggcgtctatacccgcttggcaagcgctcgcggcttgggtatgttggcgcgatgaacggaaatgcctcgcccgcgattgcctccccagcgatccacacctggtccaccgacgccgtgccgccgccgcagcggctcgactactggatcggcgccgtctgcgaaggcttcctcgagatggacgtgaccagttcctgtgccggcagcttcggggccacgctcgaatccgcgccgctcggcgccatcggcgtgaaccgggtgcgcggcagcgcgcaggacgtgtaccgcacacggcatgccattgcccacagccgcagcaactattactacctgttgtgcaagaccgattcgccctgggtcgccgtgcaggacggccgctcggcgcgcatgctgccgggcgacgtggtgctggtcgactcccggcgctgctacgaattgcacctgctccagtccgccgatacgctgtcgctcgaactgcccaccgcgtgggtggagtcgtggcttccggatgccggcgaccaggtggcgcggcgcatcgacgggcaatcgggctggggccgcgtgctgagctgttttgcccaggagctttcgccgcagggcgcgctgaagccgccgctgcctgtggcgttgctgaccgaccaactcggcgggttgctcgcgctcgccaccggcgccgcggccgatgcgggcggcccggccgcaccgggcgaaggcgcccgtgccgcgctgcgccgccgcgtgctcgacgccacgcgcgaacggcatgccgagcccggcctgacggctgccagcgtggcgcgcggactgggcatctcggagcgcagcctgcaccgcagcctgagcgacggggcgaccaccttcgcggccgcgctgaccggctttcgcatgcaggtggcgcggcgcatgcttggcgaccctcgcttcgatcgcctgggcattgcggacatcggctttcgcgtcgggttgaccgacgcatcgcacttcgttcgccaatgccgccggcatctgggcctgacccctggcgccttgcgacgccagcgttgagaaaagcggggcaggcggcgggcgtcaatcggccacaaggctggcagccagcggccattcgcgccgcatcgtgtttcctaaagtcgtctttattcaatgacgacgaagaaggagatacacatgtccgacacctatgttctgatccacggcgcctggcacaccggcggcgagatggaggccgtggccgccggcctgcgcgaggccggccacgtggtgcattgccccacgctcgtgggcaaccgcgcgggcgacgaccgctcgcgcatcggcctggatgaagcgatcgactcggccgtccgcttcatcgaggaccaagacctggccgaggttcgcctggtgggccacagctacggcggcatggtgatctcgggcgtggcggatcgcattgcgcctcggctcaggcgcctggtctacgtcaacgccttcgtgccgctcgatggcgaatcgctcaacgacatggcgccgccgcactacgtcgcgatgttcgacgccgtggctgcggccaacggcaacgcggtgagcctgccgttcgaagtctggcgcgaggcgttcatcaacgacgccgacctgccgctggcgcaggccagctacgagcagctgaacccgcatccctaccgcaccttcaccgacaagatccggctgcgcgagccgctggcggcgctgcagatcggcaagtcctacgtcaactgccagcaggacacggccatgccgcacagcctgccgtggcatccgcgcctgtcggagcggctcggcctcttcaggctggtggagtgccccggcagccacgagatgttcttctccaacccgaagcggctggcgcaggcgatcctggaggcggggcgggactaggcgaacagcgcatcgaacacgcggatcgacgcataggcgtcgttggccgcatagcggatctgcgcttccgtcagttgcctgttggcccagttcgacgtggtggccttgcgcgacttgacgaagcgccggttgaacaccagcgccacggccgccttcacgcccaccgacttgcggtagccgcggcggcggaactcgctgtcgatgtcgaacaccgccttgggctcgatgttgaggcggttgcgtatcagcgtgaggtcggtcgaaaggccgaagccgaccttcctgagttcggtggaagcaatcagcgcggccaccaccggattgcattcggtgcggtgcagctgaaagagccaggcggtttcgcgcgtggagaactgcaccacgtgcgggccgctggacacttcgttctttgcgaaggtgggcttggattcggtgtcgaagccggcaacgccggcggccagcaacgcagcggcagcgcgctcggcctcggccagcgtggaaacgaccacgatgtctttcagtcccaggccttcgaaggcttcgagcagcgcgatctgctcgcgctcgggaaggggcggcaaagcgagtgtgtcgtcgctcaaggggaggctgctttctttgtcttcactggggctttccttgcgggttttttctttggcgggtggcccgaacgcagggccgcctcgtaggcgcgccggccccagagcgcggcttcttcgcggtcttcgaagagatcggcgggcgcttgccggtacgacatcggcatcgtcttgcctttgcgttcgtaggtgaagggcggcaggttctgcttgtcgaaatgctcggcgctggtggcgtccgacttgaggtagagcgtgtccttgacgatgatcgcgatcatccgtccctcatgaaagatgccgtggcctccgaacatgcggcgcgcctcgatgcggccgaagcgctcgaaaatctcgtgcaggctttcgacgaattcactcatcgcaagcggctcatgcggtgatctcgatgcggttgccgtccgggtcgagcaccacgctctcgtagtagccgtcgccggtgcggcggggcccgtcgagcagcgggtagccgtcggctttcaggcgttgcgtgagcgcgtccaccgccgcatcggaacccacgctgatggccaggtgcgtccagcccatgcgctgggcgccgggttcggcgggcacgggcgagagcgtgcgggtggtcatggcttcgatccgggcaccgtcgcccaggctcaggaagcaggacgcaaagcccttggccggattgacatagccagcgccggccgtggcgccaaagtagtcgatgtagaagcgcttgcagcgttcgaggtcggtggtccagagggcgatgtgatcgatgcgcatggagaaacagaaaggaagagcgctcagccgatgcgtcttgattggcgtggcgggctcgtcggataccaatggtaggcgacccgttcgcgtccgctggacgggtgccggtcgacggcgccgcgctccaggccgtaacgctcgtagaagcgctgagccgcggtgttgctggtggccacgtgcagcttccagccgaacggcatgcgcacgctggcttcgtcgagcagcgcctgcccgagaccctggttgcgcagatggggttcgacaaagagctgtgccacgtattcgcgacgcgccagcagcaccataaaggcgagtacctggccgtcgcgctcggccagcaccacgtcggcgggcggcacgaattcggtttgcacgcgccgcagccaatgcgtgatgggctcgatgacggtggcccggcggttggccgcgatccaggcccggcgccagatgccggcgagcaccaggttctcttcggcggcgccatcgcgggagcgcaaatggaaggcaggaatctgtgctgcggacatgcgctccatgatacggcgcccgtacgccgaggtcgatcagccgttcagtgtttgtgcgtggtgcgcgatgtggtccgccatgaaagtctggatgaagtagtagccgtggtcgtagcccgcgtgccggcgcagcgtgacgggctggctggcggcaaagcaggcggcctcgaaggcctccgggtagagctgctcggcaaggaatttgtcggagagcccctggtcgatcaggatgccctgggggtagggcgcggcgatctgcgatttcatcagtgcgctggcgtcgtgcgcaagccactgcgcccggtcgccgcccggctcgcccaggtagccgctgaacgccttttcgccccacgggcattgcgtgggtgcgcagatgggcgcgaacgccgacagcgacttgaagcgcccggggtgccgcagcgcgagcgtgagcgcgccatggccgcccatcgaatggccgcagatgcccaggcgctggtcgtcgatggcgaagtgccgcgccacgaagggcagcagctcgtgcacgatccagctttccatacgccagtgggcggaccagggcgcttcggtggcgtcgaggtagaaacccgcgccaatgccgaagtcccagttggcggtggcgccgggcaggctttcgacggcgcttccgcgcgggctggtgtcgggcgcgatcagcgcgaggcccaggctggccgccatgcgctgcgcgccggcctttaccgcgaaggtttcctcgttgcaggtcagccccgccaggtagagcagggccggcacgcgctggttcgcggcttgcggtggcaggtagaccgagaagcgcatcggcaggccgatttcgtgcgaagcgtgctcgtgaaagctttgcacgccgccgaaggcatggtgctcggaaagggtcttgaggatgtcggtcatcgggcgatgtcgttgttgtggcgtgcgggcacgagttcgagcacggcgtcggcaaagatgcgcggcgcctcctggggcatgttgtggccgacgccgggcaccagccggtgcgatcgcagcccgctgaagcggtgcgcatgggccgaggcgttggctggcgggcgcaccccgtcgtcgacgccgtcgaaggtgatgatgggcacggcgatcgtcggctgcgcggccaggcggcgctcgatgtatgtataggccgggtcgcccgggaccaggccgaagcgatgccggtaggagtggatcaccacgtcgacgaagtcgggatggtcgaaggcggcggcgctgcgctcgaaggtggcgtcgtcgaacttccaggtaggcgaccacagctgccacagcaggcgggtgattgcgcggcggtccttagcgaggccggcgcggccgcgctcgctgtgaaagtagtactggtaccagaggctgtgctcgttcgcgggcgtgtccggctccatcgccttcgcgatgtcctggatgttgtagctgttgaacgagaccagccccgtgcagcgctccggccacagcgccgccaccacgcaggcggcgcgcccgccccagtcgtagccagcgagcaccgcgcgcggaatggcgagggcatcgagcagcgcgagcaggtcggcgccgagggccgcctgttcgccggagcgcggcgtggcgtcgctcaggaagcgcgtggcgccgtagccgcgcaggtagggcacgatgacgcggcagccctggccggcgagcattggcgccacctcggcgtaggtgtggatgtcgtaggggaagccgtgcatcagcagcacgggcgggccgtccgcagggccggcttcgaagtacgcaacttccagaacgcccgcttcgatcttgcgcaagggttccatgcggttcatggcgggcgttctcttcagggggtcagtacagaaccacgccgcggatggattcgccgcgtttcatgaggtcgaagcccttgttgatgtcttcgagcggcatggtgtgcgtgatcaggtcgtcgatgttgatcttgccttccatgtaccagtcgacgatcttgggcacgtcggtgcggccacgcgcgccgccgaaggccgagccttcccacttgcggccggtaaccagctggaacggacgcgtgctgatctcggcgcccgcctcggccacgccgatgatgatgctgcggccccagcccttgtgcgtgcattcgagcgcctggcgcatcaccttggtgttgccgatgcactcgaagctgtagtcggcgccgccgtcggtcagctgcacgatcgcgtcgaccacgttctcggtgtctttggggttgatgaagtgcgtcatgccgaacttgcgtgccatggcctcgcgctcggggttcaggtcgacgccgatgatcttgtcggcgcccaccattttcgcgccctggatcacgttcaggccgatgccgcccaggccgaacaccaccacgttggcaccggcttccaccttggcggtgaagatcacggcgccgatgcccgtggtgacgccgcagccgatgtagcagaccttgtcgaagggagcgtcctcgcggatcttggccagagagatctcgggggcgaccgtgtaattgctgaaggtcgaagtgcccatgtagtggaagatcggcttgccgtccaggctgaagcgcgaggtcgaatcaggcatcaggcccttgccctgtgtgccgcggatcagctggcagaggttggtcttgcgcgacaggcagaacttgcactggcggcattcgggcgtgtacagcggaatgacgtggtcgccctttttcagcgtggtgacgccggggccgacgtcgaccacgatgcccgcgccttcatggccgaggatggcggggaagatgccttccgggtcggcgccagagagcgtgtagtagtcggtgtggcagatgccggtggccttgatctcgaccagcacttcgccgaacttcgggccctcgaggtcgacggtttcgatggtgagcgggtctccggacttccaggcgacggcagctttggttttcatggggcttcagggcaaagaggggatgagaccggcaaggatacccagaccgcgttcaggctggacccgcggcaaagatacccgacattccgatgaaaccgggcaggtggcgaaagtcccaggcccagcgtcgcaacgccggatattcgtcaagggatattccgccttcgccggccagcgccacgtacggaaagcaggccaggtcggccacggtggcgtgcggaccggccagccattggagcccgtcgctcgcgcgctcggccaggtggtcgtcgagccgtcgaaagaccgcgtgcgcgccgcggcggcaggcctcgatgtcgaaatgctcgtagccgaaaacatcgtgcagtcgcgccgccgacgcggtgcgggtgatttcgtcggccgtggcgaaccacattgcgatctggccgcgcaactgcggatcgtccgggtaccagcggccttgcgtgtcgtgcctgctcgcgaggtagacgaggatggcctgggcgtcgcgcagcacgaagccgtcgtcgtcgatcaccggcaactgcccgagcggattgacgtgtgccaggaacgcggccgacttgtgctcgcggcccggatgaaagtcgaccggcacgctctggtagtccgcgccgagccaggcgagcatctgccgcaccttgaagcagttgcccgacagcgggtagtcgtagagccggatcatgcggcctgcctcacgccaaagcgcatgccgcgctcgcgcagccagcgccggtaggcaaccgaagaggtgtcgccgcgtgtcggcgtttcggcgcggccttcgagcggcatgcgcttgaaggcgtggttttcgagaatcggcttgtcctggccgaagatcgtgtgctggaacgcgatgagctcggcatcggtcgatgtgtcgtcgtagcaggcaaggagcgtgtgggcggtcacgtgttcgtcgtccagcggctgcaggaacaggccgatggcgtcgagcttgccggcccggtggctcgacttgtagagcatggcggtgagcggctgcatcacccggtacttgtagagcacctcgctgccgctgtcgtgggccgctgaggcgcgcggctgccagaagcggcaatcggtggcccagatttctccagtgccgggttcgatgcgcacctggtacgcggccacctcggtgtgcggcaccttgcccagcacgtcggcgtgcacgaagggaaagtgcgccatgtccagaaagttctcgatcacgcgcagccccgacacggccacgccgatgccgccgcaatcgacgatgcggcgcccggtttcgccatattccggaaaatcgaacagcggccgcgcgggcttgccgctggggcagacccagagatagccatggcgcgactggacggccagcgcctgcgaacccagccggcattgcggcttgccggccgcatcgctccaaagctgcagcgtttcgccgagcaggcgtgctgcgcggggctttgcttcggagctgccggccagcgcggcggcggagccggcgaccagccagtcgtcgagcatgttggggtcgtcggtgatgaagggcatgggtctttttctttcgctcaggcggccggctgccgtgcctcgatctcgccgcgcagtatgcgtgcggcgacgtgcagcgccttcatcgcatgggtgccgggcgcggcatcggtccagaggtggatgaaggccagccgcggccgggcgtcgagcaccagcgccgcggcatcgatgcaatcgagtgcgccgcgcatggcgggcgcagacgcatcggccctgaagtcgcgtgccgccagtgcatcgcgcacacccgccgcatcggctcgaacggagagcgtgcggcagaacgaccaccccgggggaacggcgtcgtcccgcggcagaggcggcggctccgcgtccgcgagatggacccacagcatgccggccgcatcgaccgcgctgaacaccttcgcgcagacgttgcgcggcggcggcatgtcggggtgcgcgggaatgcggatgcactgaccgctgcccgcggcgtactgccagccgtggtaggcgcaggagaggcggtcttccatcacgtggcccagcgtgaagcgcacgctgcggtgcgggcagcggttttcccatgcctgcggtgcgccgtcggccgaccgccagagcgcgagctcctggccctccgcaaagccggcgacgatgttggcgccggggctcagctcggccgagcgagccaccgggtgccaggttgaaatgctgctgtctgcgctcatgattcgcgttaccttatcgcaagtcattgcgagggcgctcgcccataatggcggctcgcttcgaccgccatcatcatgaagaaaatactcgtcctcaacggccccaatctcaacctgctcggcacgcgcgaaccagagcaatacgggcgcgacacgctggccgacgtcgagcgcctgtgcgcagaggcgggcgcgaagcacggtgtcgagatcgaatgccgccagtcgaaccacgaaggcgtcctgatcgactggatccacgaggcgggccgcgaggtggccgcaggcaacatgctcggcgtggtgatgaacccgggtgcctacacccacacctcgatcgcgctgcatgacgccatcaagggcgcgagcgtgcccttgatcgagctgcacatttcgaacgtgcacgcgcgcgaggagtttcgccaccgctcgtacatttcgccggcggcgcgcggcatcatcgtgggtcttggcgtgaaaggctacgcactggccatcgcggccctggtgccctgagcctgcggggaaccggccaaccagtcagtcggtttgcctgggcgctgaggccttccagctgcggctgatgtggccttgcgcatcgacgctctccaggtgaacgtcgaagccccacagccgcgcgacgtgcttcagcacttcttccgcatcgtcgtgcagcggcaggttgttgcgctgggtgtggcgcagcgtcagggcgcggtcgccgcgcatgttgacgttccacacctggatgtcgggctccctgctgccgatgtcgtactggcgtgacagcgattcgcgcagcagctgatagccgctgtcgtcgtgaatggcggacacctcgagctcgggctcgctctggtggtcgcggatcgcgaacagcctgaaatcgcgcatggtcttcgggctcaggaactggccgacaaagctctcgtccttgaagttgcgcatcgcatagtcgagcgtcttgacccagtcggtgcccgcgaaatcgggaaaccagcggcggtcttcctcggtcgggttctggcagatgcgccgcagctcggtgaacatcgagaagcccagcgcataggggttgatgccgctgtaggcgcgatgcccgacgggcggctgaaagatcacaccggtgtgcgagctgagccattccatcatgaagccgtcggcgagctggccgcggtcgtacatggtgttcagcagggtgtagtgccagaaggtggcccagccctcgttcatgacctgcgtctggcgctgcggatagaaatactgtgcgatcttgcgcacgatgcgcaccacctcgcgttgccagggctccagcagcgcggcattcttctcgaagaaatagagcaggttctcctgcggttccgaaggaaaacggcgggacgcgtcggactccgcggcctgctcgctcttgcggggcagggtgcgccagagatcgttgacctgctgctgcatgtggcgctcgcgttcggcgcgctgcgcgccttccctcgccagcgagcgcttctgcggacggcgatagcggtcgacgccgtagttcatgagcgcgtggcacgagtcgagcagttgctccaccgcgtcgagtccgtggcgctcttcgcattcggcgatgtagtgccgcgcgtagacgaggtagtcgatgatcgaggacgcgtcggtccacatccggaacaggtagttgcccttgaagaagctgttgtggccgtaggccgcatgggcgatcaccagggcctgcatggccatggtgttttcttccatcaggtaggcaatgcacgggtcggagttgatgacgatctcgtaggccagccccatgtggccgcggcgatagttcttctcggtggcgatgaactgcttgccgtacgaccagtgccggtagatcatgggcatgccgacgctggcataggcgtccatcatctgctcggcggtgatcacctcgagctggttcggatacacgtcgagcccgaagcccctggccgttttcgcaatctcggtgtggtaggtctcgatgaggtcgaaggtccagtccgaagggctgggcaggcgctccaggcgttcgaggggagggtgctcggaagtcatgcgggcactccttccttcttgaagaggtcgcggaacacggggtagatgtcccgtgcgtcagacaccttgcgcatcgcgaagttgggctgtatgccttcgagctgcgcgtattcctgccacaggttctgctcggtttccgcgacctgcacgtaggcgtagtagcgcaccacgggcaggatgtggtcgaccagcagttcgcggcagcggccgctgtcctggtgccagttgtcgccgtcgctggcctgcgcaccgtagacgttccattcgccgctcgggtagcgtgccttgatgatctcgtccatgagcaccagcgcgctcgacaccacggtgccgccggtttccgtggcgtggaagaactcttcctcggtcacttcctgcgcctgcgtgtggtggcgcaggaacacgaggtcgatcctctcgtagtggcgcgtgaggaacatgtacagcagcataaagaagcgcttggccatgtccttgcgcgcctcgtccatcgagccagaaacgtccatgaggcagaacatcacggccttggcgctgggcacgggggtcttcacgcggttgcggtagcgcaggtcgatggggtcgatgtagggcacatgccgcatggtgcggcggatctcgtcgatctgctcttcggtttcgcggatctcgttcttgatcaggccctgcgccgcctgcgggtgcgacctcagcgtcagcaggtgggcctcgaggcgcttgagctccttgcgcggctcgccgcccagtgcaatgcgccgggcgagggcgccgcgcatcgagcgcaccacgtgcaggttgttgggcgagccgtcgttcgtgaagcccgcccggtggctcttccattcgggcacctcggcgatctgcgtgcggatgaggtgcggcagcgcaaggtcgtcgaagaagacgcgcatgaattcttcgcgcgtgaggcggaacacgaagtcgtcttcgccttcgccgctgtccccggcctcgccgctgcccgagccgccgccggcctgcccttcgggccgcgcaatgcggtcgcccttcaggtattcctggttgccggggtgcacgtattcgcggtctccgccgcgcgcatggccgaacacgggctcggacacgtcgtggcgcggcagggtgacatcttcgccttgctccagttcgcggatgttgcgcccgctgaccgcgcgccgcacggcctcctggatctgccccttgtagcgccggagaaagcgctcgcggttgccaatggacttgttcttgcccgaaagccggcggtcgatgatctgctgcaggatggccacgatgatgtcaaagctccttgcaaaaaagggggcgaagcctgtgcctcgccgctatgaactgtcgctatgaactcttgcgcacccggaggtaccactcgcagagcagccggacctgcttggccgtatagcccttctcgaccatgcgggtcacgaagtcctcgtgcttcttctgctcgtcggcactgctcttggtgttgaaactgatcaccgggaggagttcctcggtgttggagaacatcttcttctcgatgaccgcgcgcagcttctcgtagctggtccaggcggggttgcgcccggcgttgccggcgcgcgcgcgcagcacgaagttgacgatctcgttgcggaagtcctttggattgccgatgcccgcgggccgctcgatcttctcgagttcggcgttgagcgaggcgcggtcgaacacttcgccggtgtccacgtcgcggaactcctggtcctggatccagtagtcggcgtaggtcacgtagcgatcgaagatgttctggccgtattcgctgtagctctcgaggtaggcggtctggatctccttgccgatgaactcggcatagcgcggcgccagcagctccttgatgtaactgatgtacttctgctcggtttccggcggaaactgctcgcgctcgatctgctgctcgagcacgtacatcaggtgcaccgggttggcggccacctcggagctgtcgaagttgaacaccttcgagatgatcttgaaggcaaagcgcgtggagacgccgctcatgccttcgtcgacaccggcgtagtcgcggtattcctggatcgacttggccttggggtcggtgtccttgaggttttcgccgtcgtacacctgcagcttgctgtagatgctggagttctctggctccttcaggcgcgtgagcaccgacagctgggccatcatgcgcagcgtgccgggcgcgcatggcgccttggcgagcgaggagttgcgcaccagcttctcgtagatcttgatttcttccgaggcgcgcaggcagtagggcaccttgacgatgtagatccggtcgaggaaagcctcgttgttcttgttgttgcggaaggccttccattcgctctcgttgctgtgcgcgagaacgatgccgtcgaacggaatggcgccgaagccctcggtgcccttgaagttgccctcctgcgtggccgtgagcagcgggtgcagcaccttgatgggcgccttgaacatttccacgaactccagcaggccctggttggccaggcacaggccacccgaataggcgtaggcgtcgggatcgtcctgggcataggtctcgagcttgcggatgtcgatcttgccgaccagcgaagaaatgtcctggttgttctcgtcgcccggctcggtcttggcaactgcgatctgccgcagcaccgaggggtagcgcttgacgaccttgaactggcggatgtcgccgccgtactcctcgagccgcttgacggcccagggcgaaagaatgcggttgagatagcggatgggaatgccgtattccttctcgaggatctcaccatcctcgacggcgtcgaacaggcccagcggcgtttcgttgaccggcgaaccctggatggcatagaacggcacgtgctccatgagctgcttcaggcgctcggcgatcgaactcttgccgccgccgacgggaccgagcaggtagaggatctgcttcttctcctcgagcccctgggcggcatgcctgaagtacgacaccacctgctcgatggcgtcctccatgccgtagaactccttgaacgccgggtagatcttgatgaccttgttcgcgaagattcgcgacagccgggaatcgttgcgcgtgtcgaccagctcgggttcgccgatggccttgagcatccgctcggaagcagtggcatacgcagtggggtcgcgtttgcaaatatccaggtagtcctgcagcgacaggacctcctcgcgggtgcgctcgtaacgggcggcaaagttgctgatcacatccatggtcacgcctccatcaggtctgcgggtttatcggccccgaaggcctgcagccccaacgcgtcgcaactttttaaaggtgtgccccgcccatggctgcaagccgtggaaaactcccttaatcacatcttcacaaacagcataaagcaaagagtgcacccgggaaattctttgttaaatcagaaccacagtgccgagtaaagttcctgagaaaaacccgcagcatttggcaattccagctaaatttcagggttcggcaatcgagcttcgcgcgacccctccgcccagtgaaaatacctatggcgatcggcatatgtagtcattgcatcttttcccgggaacgcacctcctaaagagcatcgagcggctcaaagctgttacataaccaataacgcgccgcatcctgtttgggtttattgctcaatcgaaaaaaatataaaagcaatccccgcgccatcttttgatgagcatgtcgcgcatgtgagcgtgggaaagcgcgccaacccgcggtcagcgtggttccgaggagagggtgcgatggtgcgcgcaccgaactaggtcggcaggcaccgttcgcgtgcgcgaaggcgggcagcgccgaagcagcgccgtgcggccgcttctaactgcttgaaaaatctggggaatcggtgcgccggccgctgaagagcgccgggcagaaggcaaggcagcagggcgcagcgaagtgcgcctgccgcattccggtgcctcctgtcagctgagtcagctgaagaattccttggccttgtcgaaccatcccttgtcggtcgggctgtgcttgtcgccgcccttcttgagggagtcgtcgagctccttcagcagcttgcgctggtgctcggtgagcttgaccggcgtttcgacgcgcacgtggcagtacaggtcgcccggatagctcgagcgcacgcccttgatgcccttgccgcgcaggcggaactgcttgccgctctgggtgccgtcgggaatgtcgatggccgcggcacccttgagcgtgggcacgctgatctcgccgcccagcgctgcagtggtcatgctgacgggcaccacgcagtgcaggtcgtcgccgtcgcgctcgaacagctcgtgcttcttgaggcggatctcgatgtacaggtcgccgggcggcccgccattggtgccaggttcgccgttgccggtgctgcgaatgcgcatgccgtcgtcgatgccggccgggatcttgacctcgagcgtcttgttgttcttgatctttccctggccatggcacaccgtgcagggctcgggaatgatcttgccgctgccgtggcaggtggggcaggtctgttgcacgctgaaaaagccctggcgcatctgcactgctccggcaccgtgacaggttgtgcaggtaatgggcttggtgccgggcttggcgccggagccgtggcaggtgccgcagtcgtcccagctcgggatgcggatctgcgcttccttgccgtcggccgcttcttccagcgtgacttccatggcatagctcaggtcgctgccgcggaacacctggcggccgccgctggtgcggccgcggccgccgccgaacacgtcgccgaagatgtcgccaaaggcctcggcaaagccgccgaagccgtcggcgccggggccgccgcgcatgttcgggtcgacaccggcgtggccgtactggtcgtaggccgcgcgcttctgcccgtcggacagcatttcgtaggcttccttgacctccttgaacttggcctcggcgtccttgctggtgtcgccgtggttgcggtccgggtggtgcttcatcgcaagcttgcgataagccttcttgatttcctcctcgctcgcgttcttgggaacgccgagggtctcgtagtagtcgcgttttgtggccatggctgattcggtcggggcgggcgggaagccgtaacttgaagcgagaaaggctggaccacccgatcaggtgatccagccttgttcgaagggctgaaggtcagcctttcttgacttccttgacttcggcgtcgaccacgttgtcatcggccggtgcactcgcagcttccgggccagcagcggcacccgggccgccggcggcgcctgtcgcggcctgcgcatcggcatacatcttctcgccgagcttctggcttgcggtcatcagcgtgttggtcttttcctcgatcgaggccttgtcctcacccttcagggcttcttccaggtccttgatcgcggcttcgatcttttccttctcgccggcgtccaggctcgcgccgtgttcgccgagcgacttcttcacgctgtgcaccatggcttcgccctggttgcgggcctgcacgatctcgagcttcttcttgtcgtcggccgcgttgagttcggcgtccttcaccatcttctggatctcttcctcggaaaggcccgagttcgccttgatggtgatcttgttttccttgccggtgcccttgtccttcgcgcccacgtgcaggatgccgttggcgtcgatgtcgaagctcacctcgatctgcggcgtgccgcgcgatgccggcggaatgccctcgagattgaactcgccgagcagcttgttgcccgaggcaatgtcgcgttcgccctggaacaccttgatggtcacggccggctggttgtcttcggcggtggagaaggtctgcgcgaacttcgtcgggatcgtggtgttcttcgtgatcatcttggtcatcacgccgcccatggtctcgatgcccagcgacagcggggtcacgtccagcagcagcacgtccttgcggtcgccggagagcacctggccctggatggcggcgccgacggccacggcttcgtcggggttcacgtccttgcgcggctccttgccgaagaaggccttcaccttttcctgcaccttgggcatgcgggtcatgccgccgaccaggatcacgtcgttgatgtcggacacgctgatgccggcgtccttgatggccaggcggcagggggcgatggtgcgctcgaccagctcgtcgaccaggctctcgagcttggcgcgcgtgagcttgatgttcaggtgcttcggacccgtggcatcggccgtgatgtagggcaggttgatgtcggtctgcgcgctgttcgacagctcgatcttggccttttcggcggcttccttcaggcgctgcagcgcgagcacgtccttgctcaggtcgacgccttgttccttcttgaactcggcaatgatgtagtcgatgatgcgctggtcgaagtcttcgccgcccaggaaggtgtcgccgttggtcgacagcacttcgaactgcttctcgccgtcgacgtctgcaatttcgatgatcgagatgtcgaaggtaccgccgccgaggtcatacacggcaatcttgcggtcggccttgtcctgcttgtcgaggccgaaggccagggctgcagcggtgggctcgttgatgatgcgcttgacgtccaggcccgcgatgcggccggcgtccttggtggcctggcgctgggcgtcgttgaagtaggccggcaccgtgatcacggcttcggtcacgggctcgccgagatagtcttcggcggtcttcttcatcttgcgcaggatgtcggcgctgacctgctggggcgcgatcttcttgccgcgcacttcgacccatgcgtcgccgttgtcggctttcgcaatggtgtagggcatcaggtcgatgtccttctggacttctttttcttcgaacttgcggccgatcaggcgcttgatcgcgtacagcgtgttgcggggattggtcacggcctggcgcttggccgaggcaccgaccagcacttcgccgtcttcctggtaagccacgatcgacggcgtggtgcgcgcaccttccgagttctcgatcacacgcgtggtgttgccttccatgatcgacacgcacgagttggtggtgccgaggtcgatgccgatgatctttgccatgttctttactcctgaaagcctgaaaaatatgttgttatgaacttgtggataacccggcgcgattcaaggtatgaagcggggatttcctgtgggaatcttgtgtgcggggtcggccgtggctgactattacttcggcgcgctgaccgtgaccagcgccgggcgcagcacgcgctcgttgatggtgtagcccttctggagcacgctcaccacggtgttgggttcctgctcgggagcgggcaccaccgagatggcctggtgctggtgcgggtcgaacttggtgccgggggcgggagccacctcgatcaccttgttgcgttcgagtgcgctcttcagctggcgcagcgtggcttcggcgccctcgcggatctgctccggtgtggcgtccttgatggccaggccggcttcgaggctgtccgtcacgggcagcaggctctcggcaaaggcctcgaccgcgaacttgcgggccttggtgatttcgtcgtcggcgcggcggcgggcgttctggacgtcggcctgggcgcgcaggtattggtcggccagttcggcgttcttgctctgcagggcggcgagttcaccttgggctgcggccagggcgtcttgcgcctcggcttcgttggcagcctgcgcggcttccagttcttcggggcttggctcgccttgcagcatttgcgaattctgtgcggattgttgcgggtcagacatttttcaaggaaccggcgtgtgccggaaaacaagcgatagccagccacttggggctggctcaaggcatttcaagcgaaaaaatgcggcaaaagaggccgcggaggcatgaaaaaggcccgcaatcgggccttcgtgccagtcctggctcgggaacgatcagtgcgcgtcgagcagttcgacgtcgaacttcagggtggcgttcgggggaatcacgccgccggcgccgcgtgcgccatagccgagcgatgcgggaatgatcagcgtgcgcttgccgccgatcttcatgccggcgacgccttcgtcccagcccttgatgacctggcccgcgcccagcgagaaagcgaacgggtcgttgcggtcgcggctcgaatcgaacttggcgccttgcacgccgtcgttgtagagccagccggtgtagtgcacgtgcacgtgctggccagctttggcttcagcgccgtcgcccacggtggtgtcttcgtattgcagtccggagggggtggtaggcatgtcgaacgctccttgcgtcaatgagatggatgtgagtggataagcagagaccgaaggcgcgaagtttaccgacgcccggagctcgccggccggcccgctcaattgccagtgtcaagaggcggggtggaggacggcgccgaaggagaggaagaagagggcggtgccaccggggaagaggacggcgctgggggagaagaagacgagggagacggtgacggcgatggcgaagaaggaggcgcagtcgcggcagtcgcggcagccgcaggcgccgcggccttcttgatctgccccagctgccacttgcccgcgaaggcctgcaggtccgaaagccgcttgagcaggtcttgcccgctcacggtcaggctgtagccgtcgccgccatggctgacgagaccggcctcgcgcaattccttgatgcgggtgttgagcgtgttgggagtgatgccgccgacgctgtcctgcagcaggcgaaaggtctgggcgtggccgtcgcgcaaggcccagagcaccctcatggcgtagcgggcctcgagaagtgcgagcagctggctgacggctgcgttttccttggtactcatcgacatcatctcctcggggctggtcgggcatcgatccttgggggcagggccggtgccgcgcgttcttgtggcttgtagcctgctatggcgctcgttggccggcgactatagcgcaaggatcaggatgctactagttttatagctacgagggcatgctgcgcgcggcccctgagacaaagcttcacaaattagcgaaatttgccatggcttcgcccaaccggaccgcgcgggcgggcgaccattccggattgaagcccagcgcgggcggcgggaacagcatgaccacggtggatccgagcaggaaacggcccatctcctcgccttgcttgagcacgatctgctggtcgccgtagtgccactcgcgcagctcgccgccgcgcggcggattgaccacgccgtgccacacggtttccatgctgccgacgatggtggcgcccaccagcaccagcacgaagggcccgcgcgcggattcgaagacgcagaccacgcgctcgttgcgcgcgaacaggccgggcacgccgcgcgccgtggccggattgaccgagaacaggtcgccgggcacgtagatcatgcgcagcagccgcccttcgcagggcatgtgaatgcggtggtagtccttcgggctcaggtacagcgttgcaaagctgccgtgggcgaactggtgtgcgagcgccgcatcgccgccgaccagcgcggtggtcgtgtagttgtggcccttggcctggaagatctggtggccttcgatggcgccgaactggctgatggcaccatccaccggacatacgagatcggcctttgcgagaggccgggcgccgggcttgagcgcacgcgtgaagaactggttgaagctcttgtagtagttgatgtcggattcgagcgcttcgcccatgtcgacgccgtacttggccacgaagcgccggatgatccacgtggtgacggcgccgcgctccttgcctgcgacccagccggcgaagttcgtcagggcctgcttcgggaacaggtattgatgcagtacggcagagcggtcggacacgagtgaaaggcgtggagcgcctggaatgcgaatcggaggggcattctataaagggctccgcgcgccggacgtaggaagcttcccttgtatgcggggcccctcgttcgcacgcgaggccccgtgcacgcacgcaggcacaccgcccggcgtcagtcggccttgatgccggccgccttgatcacttgcgcccacttctccacttcggccttctggaaggcggcgatcttgggcggggtcaggtgggcgggctccatgccgaagcccttgagcttgtcctgcatttcgggcgttgcaaggatcttgcggatctcggtgtgcagcctgtcgacgacgggcgcgggcgtgccggcgggcacgaagatcgcctgccacgacagcacctcgaaatcctgcaggcctgcgattccggactccgcaaccgtcggcacgtcgggcatcgaagccaggcgcttggccgaggtcacggcaatggcacgcagcttgccgctctgcacgtgcgggccggccaccacgctggtgtcgaacatcatgtcgacctggccgccgatcacgtcctggatggcagggccgctgcccttgtagggaatgtgcgtgaacttcacgcccgacctgaacgccagcagttccagcgacaggtgctgcgacgtgccggtgccggccgatgccgacgacagcccacccgacttggtcttgctggcttccagcacgtccttcaacgtcttgtaggggctggcctggttcaccaccagcaccagcgggttggtgccgatgagcgtcaccggcgcaaacgacttctgcgggtcgtagccgagcttggggtacaggctcacgttgatggcgtgcgagctgatggtgccgccgacgatcgtgaagccatcgggcgccgcgcgcgcgccgatctccgagcccacgctgccgcccgcgccgcccttgttgtcgatgatcacgctcgtgcccagcaccgtgccgagcttctggccgatcaggcgcgccagcacgtcggtggtgccgcccgcgggaaagggcacgaggtaggtgatggccttgcccgtgggccagttgccggggccttgcgcgaaagcgggcaggcccacggcgatcgaagaggcgagggcggtgcggatgagtgtgcggcgttgcatggcgaagtctcctttgatgatgttgcgggtcgtcgtcacggcgtatcgacgatttcgatccagttcgggttcttgcccacgctgatgcgcgcgggcttgtccaatgcgccggtcgcgggatcgatggcgtacagcgcaacgctgtgcgactcctgcccggcggcgatcaggtagcggccgctcgaatcgatggcaaagccgcgcggcgttttctcggtcggcgtctggccgagcggcttcagctgtccggtggacgcgtccaccctgaaggccgacagcgtgctcgacgtgcgctccgaggcatacagaaagcgcccgtcgggcgtcaggtgcaaatcggctgcccagggcttgccggtgaaaccgggcggcagcgtgctggtgctctgctcgtgcttgagcgttccgcgcgcggcgtcccagccgtacacgtgcaagctcgcatcgagttcgttcagcaggtagacgcgtcgctgcgccttgtcccacacgaagtggcgcggccctgactttgcggtgccctgtgtcagcggcggatcgttggccgacagcagccccttctccgcatcgaagcgccaggtcgaaacgttgtcgccgcccaggctggtggccagcacgaagcggttgctcgcatccgcgtggatcgcatgcgcattcggcgcggtctggaccagttgctggatcgcacccgctgcaccgtccttgccaatggcgttgaccgagatcttgccgccctggtaggaggcggcaaagagccacttgccgctcgcgtcgaggtcgatgttggccatgctgtcggccagcggcgcttcgccgagcttctgcagcttgccggtggcggcgtcgatcgaaagcgacaccacgcggaacggctgcgagcgaagcgccgcatacagcacgcgcttgtcgtggctcaccgccatcggcatgaccgtgccgccgacgttgagcgtctgcaccggcttgagcacgccctggccgcggtccagttcgagcaccgagatttcctggctgtccgcattggacacatagacccatgtggccgccgacgcgtggcctgcaacgatcgacagcagctgcgcggcggcgaaccggagcgctcggggcgcacgaaggaatgtgttgttgcttttcatgaaggtgttgtctctgttgttgtcgatccgatgctgcaaactggaagggaggtcgttcccgtgtcagggcatgtactgcccgccgttcacctcgatcacctgccccgtcacatagcccgagagctgctccgaggccaggtagagaaaagcgcccacgcattcgtcggccgtgccaatgcggcccattggaatgccggcgcggaacgattcgagcatcgcgggcgtcgagaagcggtcctggaacggtgtctggatgacgccgggcgccaccgcgttcacgcggatcttgtcgccgacgagttccctggcaagcccgtgcgtggccgtgctcacgaagcccttggagcccgcatacaggtacgcgcccggtccgccgccggtgcgtgccgcgaccgaggtcacgttgatgatgttgcctccgccatgggtgcgcatcagcggcaccacctcgcgggcaaacgcaagcaccgagcgtgcattgatatgcatcacttcgtcgaacagcgcatcgtcgaattccgcgatggggacgcgcttcaccaggctgccggcgttgttcaccagcacgtcgatgcggccgaaccgcgcggccgtctgcttcacgcattcgcggatggctgcggtgtcgagcacgtcgccctgcagcgcaaaggcatcgccgccggccgatcgaatggtctcgaccacctggttggcggcatcggccgagctgttgtagtgcaccgccacgcgcatgccgcgcgccgcgaacgcaatggccaccgcggcgccgatgccggtgctggcgccggtgacgagcgcggtcttgcctttgaggtcttccatggatgtttcctttcgaggtcgggtgaagtcaggtcacgggagcgggattgaacagcaccagcgcgttgtgcagcttccactgttcggcccaggttttcttcctgccgctggccacgtccagcatcagccggaacatctcccagcccacgtcttcgatggtggcgtcgccgtcggcgatgcggcctgcgttcacgtccatcaggtcgtgccagcggcgcgccaggtcgctgcgcgtggccaccttgatgaccggcacctcggccagcccgtagggcgtgccgcggccggtggtgaacacgtgcaggttcatgcccgcggccagctgcagcgtgccgcagatgaagtcgctggcgggcgtggcggcatagagcagtcccttctgcctggccttctcgcccggcggaaccacgccggagatcggcgcgctgccgctcttgacgatcgagcccatggccttctcgacgatgttcgagagcccgcctttcttgttgcccggcgtggtgttggcactgcggtcgacgcggccgcggtccaggtaggcgtcgtaccaggccatctcgcggatcatggcgtcggccacctcgggcgtggtcgcgcgcgaggtgagctggtcgatgccgtcgcgcacctcggtcacttccgagaacatcacggtggcgccggcgcgcaccagcaggtcggtgcaaaagcccacggccgggttggccgtgacgcccgagaaggcgtcgctgccgccgcactgcacgcccaccaccagctcgctcgcgggcacggtctcgcgctggcgcgcgttgagccgctccaggtgttcctcggcctgccgcatgatcgaatcgatcatcgacatgaagccgacgtgggcgtcgtcctgcaggcacaccacgtcgagcttggcgttggccgtctcgccgatgtcggccacgttgcgttcgtccaccagcgcaatgctgcccggcggcagcaagcgctcgggctgcagcttctcgcagcccaggctgatgaccatcacctcgccgccgaagttcgggttgaggctgatgttgcgcagcgtgcggatcggaatgatcgcgtcgggcgcgtcaatggccacgccgcagccgtagctgtgtgagaggcccaccacgtcgtcgacgtgggggtacttgggcagcagctcggccttgatgcgctgcaccgcgaaatcgaccacgcccgccacgcactgcacggtctgcgtgatggcgaggatgttgcgcgtgccgaccgatccgtccaggttgcgatagccctcgaaggtgtagccctccagcggcggctgtgcgggcggcttcacggtggcgatcggcaggccttcgagctcgcgcgcggcgggcatcttcagcagccgctcgtgcacccagctgccgcgcggaatggccttcagcgcgtagccgatcaccacgttgtagcggacgaccgcatcgccttcggccaagtcggtcagcgagaccttgtggccctgcggcacgttgtcgaccagcacgaggccgtcggaaaacgccgtgccggccttcaggccgccgtcattggcaacgatggcgacgttgtccgccgcgtgcatgtggatgcggtgcggcgggcgcaccggcggggaagagggtagtgatgagtcggccatcggatcgaactccgcgttgcttgtctttggtgtcacttgaccgcgttgacgaggtccggcagccacatcgagaacgccggaacataggtcacgagcatcaggcagatcaggagggcaccatagaacggccagatcgaccgcatcacctgcccgacggatacccctccgatcgcgcagcctatgaactgcgtggtgcctaccggcggcgtgttgaggcccagggcgcaattgatcagcatgacgatgccgaactgcaccgggctcatgccgaactgcatggcaatcggcaggaagatgggcgtgcagatcaggatggtcgcggccatgtccaggaaggtgccgagcacgaacagcagcacgttgatcatcagaaagatgacccacggatcgctcgagacgctggtcatgagctcgccggtcttctgcggcacttcgtacagggccatgaagtagccgaaggccgaagagatgccgatcagcagcagcaccacgccggtcgtcttgcaggccttggcgcaggccttgaaaaagtccttgcggctgagcgagcggtacacgaacacggtcacgcccaatgcccagagcaccgccgtcgccgccgactcggtggcggtgaacacgcccgacaggatgccgaccaggatgatcgccacgatcatcaagccgggcagtgcgccgatgaacgccgcaagcacttcgccccagccggggaaagcgccgcgaatcggatagccgcggcggatggccacgtagtaggcggcggccaggttgcacagcgtgagcagcagcgccggaatgaggcccgccagaatcaggctcagcacgctgaccgacgcaatgcccgtggtcgccagcgtgaagatgatcaggttgtgcgacgtgggcatcagcgcacccaccagggccgcgtgcgtcgtgacgttgaccgcgtagtcggcgtcgtagccttccttcttcatcagcggaatcatcaccgagcccatggccgagacgtcggccaccggcgagccggccacgccgccgaacagcgtgcagccgatcacgttgctcatgcccaggccgccgcgcacgtggcccaccaggctgttggcaaagcggacgatgcgctgcgcgatgccgccgtaaagcatgagctcaccggcaaacacgaagaacggaatcgccaggaacgagaagacctgcatgccgccgaccatcttctggaacaccacggcaacgggcaggcccgcatagagcacggtggcaacggaggccaggccgatcgagaacgcgaccggcacgcccagcaccagcagcaccaggaaaacgagggataggacagtcagttccacgcgggcaccacttcttcatcgcgcagcagggcgacgatatgttcaatcgaaaagaggacgatcaggagacccgcgatcaccagcgcgagatagtcgagacccaccggaacgcccatcatgggcttgatgtcgctccacttgagcgtggtccagacccagccgctccaggtcatgattgcgccgaagagcgcgaccagcgcgtgaatcagtatttcgatcttcaggcggagcgattcggggagcagcaccaccagcgagtcgagcccgatgtggccggcatcgcgcacgccgacggcaacgcccagcgccgtgacatacagcaccagctgcagcgcgaggccttcggcccaggtcggcgtgtcgttgaacacatagcggccgacgacctggtactggacgcacacgatgatggtgatgagcatcgccaccgcgagcatcaggctggccttggagaggaacgcgcagaagcgcgaataggcgtggttggacggagggcgtccgttcggatcgaccaggtcttcgagctcgacgggcgcgccggtcgccagcttgtctaccgcggggacggtaagtgtcatgggaacttccctgaatatgggtgaggggccctccccggaaagcgggagggccgaggcacgtcacttgttgtcttgaacggccttgacgaggcgctgcagatcgggcgtcgagatgaacttggtgtagaccggggccatggctgcgcggaacgatgccttgtccacgtcggcaatgatctgggcgccgcccttggtcacgacctcgagcgacttggcttcctgctcgtcccacttcttgcgctggaaggcgaccgattccttggccgtggcgcggaacaggtcctggtcggccttgggcagcttgtcgtagatggccttggacatcacgagcatttcaggcgccatggagtgttcggtgcgcgaatagaacttcaccgcttcgtagtgcttgaaaccgtcgtatgaaggaatgttgttttccgccgcgtcgatgagtccggtcttgagtgcggtgaacacttcgccggtgggcattggcgtggcgttggcgcccatggcgctcaccagtgcgacccacaggtcggactgctgcacgcggatcttgagccccttcgcgtcggccagcgtcttcaccggcttcttggcgtagatcgaacgcgcgccgctgtcgtagaaggccaggccgaccaggccttcatgttcgcagcccttcaggatctcgtcgccgatggggccgtcgagcgacttgcgcatgtgcgcgatggagtcgaacaggaagggcatcgtcggcaccagcgtcttggggcagatcgaattcagcgcgctgatgttgacgcggttcatttcgagcgcgccgatcttcacctggtcgagcgtttccttctcgctgccgagtgcgctcttgttgaacaccttgatcttgtacttgccgttgctgcgcttgtcgagcagttcgctcatgtgcttgaccgccgcgacggtggggtagtcgtcgctgttgtgcacgtcggccgagcggaactcgaccgcgttggctgccatggccaaggcgcctacggccagggcgatgaggtggcgggtgtatttcatttgtcttcctcttggggttggtggttaaaaacaatcagaaacggcattcgggttccggcaacccctggacgccgggacgcagcgcaaaaacgccgcccgccagcggttggtcggacaggtcgccgccggggcggatcgacgtcacgtagagcgtgtcgagcgctggcccgccaaaggcgcacatcgcgggcttcttcaccggcacggcaagggagcggtcgagccgtccctcgggcgtgaatcggtgaacgagcccggcgtcgttgccgcagatccaatagcaaccgtcggcgtcgacggcggcgccgtcggggcggcccggcagcggcttcatgtcgacgaacacgcggcggccatgtggcgtgccggtgtcggtgtcgtagtcgaaagcccagatggtctgcaccgccggatgcgaatcggagaggtacatggtcctgccgtcggggctgaaggcgaggccgttgggaacgatcatgcggtcgaactgggcgcgcagcgccacttccgcattcacgtcgccctggtagcggtacacgcggccgacctcatgcgctgccgccatgtccatctgcatggtgccggcccagaagcggccctggcggtcgcagcggccatcgttgaagcgcatgccgcgttccgcgtggacggcgctcgcaacggggctcgcggccagggtgccgtcggcgcgcgtggcgatggcgaacagtccgctttccatgccggcgatccactcgcccggatggccggcgcgcggtgcgatgcaggccagcatctcgtcgccggtccagcagctgtgcgcgccggtcggggcgtgccagcggtgcagttgtttcgccggaatgtcgacccagtagagcgcctgctcatcggcgcgccagaccgggctttcgccggtcgcgcatcgcgcatcgagaacgagttcggcttgcatgccggtcgtcattggtcgccgaacgggccctgcgccgtgaacgcgccgccctggtagatcgcgttggggtcggtaggcgccacgggaggctgggcctcgaccttgtcgcggaacacttcggaggtgtcctgcggcacgaagcccaggtgcgctgccgcgctgttgtcccaccagacatcgcggttggccgacatgccgtagacgatggtgtgcttcacgtcgggcgtgaagatcgacttctcgatcagcgaggtgaggtcgcggtagctgagccaggtgctcatcatccggcggttgagcggctccgggaacgacgagccgatgcggatgctcaccgactcgatgccatagcggtcgaagtagaactgagcgacgtcttcgccgaacgacttcgacaggccgtagtagccgtcgggccggcgctgggcgctggcgtccagccgatcgctctgcttgtgaaagccgatcacatggttcgaactcgcgaacaccacgcgcttcacgccgtgccggcgggcggcttcgtagacattgaacacgcccttgatgttggcttcgagaatttcctcgaacgggcgctcgaccgagacgccgcccaagtgcacgatggcgtcgcagccctcgaccagcgcatggacggccgtcttgtccgacaggtcgcagggcaccacttcttcgtgcgcaccctcggagggggcgattgcggcaatgtcggaaaggcgcaggatctcggcaaaggggcgcaggcgttcgcgcaataccttgcccaggccgccggccgcgccggtcagcagaatccggtggagcttgctgttggtagtttgtgaggacgtcgacatgtgtggtggcgtgtgaatgggttgaggtccagggcgatggagcagtcaccgaaagctagccagaaagcggcttcatctcccatgccgcgccagttcgaataaccggtcgatggatggacgacacttgccgcaaactgagtgataagttatctgttgtcgtacaactaattggggattattatcttgaccatggtccaaacggctacgggtaatccctcaatttcggatgcggcggcagacgccgctgccggcgcctcctttgtgggggtggggcgcccgcgcccgcgcggcctggcccacgggctggtggaagacctgggcgaaaagatccgcagccagtcgctgcgccccggcgacaagctgcccaccgaatcggccatcatgaagtccttcggcgtaagccggacggtcgtgcgcgaggcactgtcgaagctgcaggccgccgggctggtcgaaacgcaccatggcgtcggcaccttcgtgctgcagccgcgtgcggcgggcatgttccggctcgattccgccgacatcgccacctcggtggacgtgctggcggtgctcgagctgcgcatcagcctggagaccgaatccgcgggcctcgcggccacgcgccgcaccgaggagcacctgcttgccatgcgccaggcgctcgacgatttcgagcgcaacgtggcggtggcgggggatacggtggcgcccgatttccgctttcacctgcagatcgcccaggccaccggcaacccgtatttcgcggacatcatgagccacctgggcaccacgatcattccgcgcacgcgcatcaccgccattcgcaactacgaccggcgcggcgaatacctgagccgcgtgaaccgcgagcacgaagagatctatgcagccattgcgcgccgcgatccggagtcggcccgtgcggccatgcgcatccacctgaccaacagccgcgagcggctgcgcgtggcgcaggaagcggcgcaacaagccacggccaacacgccgccagccgcttcctgagcgaaattttcttgccgacgctggacaagcgtcatttgtggttgtacgatgactgacaacacaacctgacaggagacctgaatgagcttgaaaagacgtgacctgatgctcggcgccctgggcggcggcgtgcttgccgccggtggtgtgcatgcggccgacgcctggccctccaagccactgcgcatcgtggtgccgtacccaccgggcggttcgtccgacatcattgcccgctccatcagccagccgttgtcggaagcgctcggccagccggtcatcgtcgagaacaagccgggtgccaacggcaaccttggcgctgatttcgtcgccaagtcgaagcccgatggctacacgctgctgttgtgcgacgtcggcgcgctcgccatcagcccctcggtctacacgcggctgcctttcgatccctccaaggacctgcgcggcgtgaccatgctggcctattcgccgcacctgctggtggtgcatccgtcggtccaggccaacagcctgaaggaattgatcgccctgtcgaagaagtcggacatcaacttcgccgtgaccgccaccggcagtgcgccgcatctggccggcgtggcgctcgagcgcgccagcggtgcgcgctggcaatacgtgccctacaagggcggcgtgcaggcggtgcaggacacggtcgccggccagacccagattctcatgaacggcatgctggccaccttgccgcacgtgcaaagcggcaagctcaaggtgctcggcgtttcgaagtcgacgcgcatgccgctgatcggtgacgtgcccaccatcgcagagcagggcgtggccggtttcgagtcgggcacctggcaaggcgtgcgggttgccaagggtacgcccgacgccatcgtccagcgcctcaacaaggaactgatcacggtcattcgcgcggccgacatccgctcgcgccttgcagggcagggcgctgaggtcgtgaccatggcgccggccgaggaagagcagttcttcggcaaggaacgcacgcgctgggccaaggtggtggccgacgccggcatcaagctggattgataggctcacccccagtctgcgcgcacttcgtgtcgcgcgcgccaacccccttccgggggcactgccagcggcccggcaaagccggttccgcggcagtccacgaaaagaacggatccatttttaacccactctcattggtgtctcgatgaaccctcaagaacttaaatccatcatgggctccggcctgctctcgttcccgctgaccgacttcgatgcgaacggcgacttcaaccgcaagggctacgagaggcgtctcgaatggctcgccccctacggcgcgagcgcgctgttcgcggccggcggcacgggcgagttcttctcgctgaccggcgaggagtaccccggcatcatccagagcgcggtcgacacctgccgcggcgtggtgcccatcattgccggcgccggcggcccgacgcgctttgcgatccagtgcgcgcaagccgcggagaaggcgggcgcacacggcatcctgctgctgccgcactacctgaccgaagccggccaggaaggcctggccgcgcacgtcgaagcggtgtgcaagagcgtgaagttcggcgtcatcgtctacaaccgcgccaccagccgcctcaagcccgacacgctcgccggcctggccgagcgcaatccgaacctggtcggtttcaaggacggcatcggcgacatcgaagccatggtggccatctaccagaagatgggcgatcgcttcgcctacctgggcggcctgcccacggccgaggtctatgccgcggcctacaaggccatgggcacgccggtgtattcgtcggccgttttcaacttcattccgaagaccgcggtgcagttctatgaagccgtgcgcgacgacgacatggccacccagcatcgcctgctgaagaacttcttcatgccttacctcgaactgcgcaacctcacgcctggctatgcggtgagcatcgtcaaggccggcgccaagatcgtcggccacgacgctggcccggtgcgcgcgccactcaccgacctgaagcccgccgagatggaacagctcaaggccctgatcgacgcgctcggcccgcagtaagcggccgggtcgataaaaccgacaacggagacaacaaggcatgctgatgaaaaagcttcttctcatcgcggcgggccccgcgcttgccgccactgcgctgctgcctccgcatgccttggcccaagccgatgcatggccgcagcagaagccggtgaccatcgtggtgccgttccccgccggtggctccaccgacatggtggcgcgcgcactggcgctgcaattgcaggcaaagctcggcgggagcttcgtcgtcgacaaccggccgggcgccacgggcaccatcggcacgggacaggtcaagcgcgcggcacccgacggctacacgctgctggtgtcgtcgctcggagccttcgtcgtcacgccgcacctgcaaaagagcgtgccctacgacgccaccaaggacttcgactacatcagcgttcccgtgcaggcgcccaatgtgctggtgaccaatgccgcgcggcccgagcgcaccgtggccgacctgctggaattgctgcgcaagaccccgggcaaggtctcgttcgcgagctcgggcaacggttcgtccgaccatctgtcggccgaactgttctggcagcagagcaagaccgaaggcgtgcatgtgccctacaagggcggtgcgccggcagtcaacgatctgctcggcaaccaggtcgatttctcgttccagaacgtgaatgccgtgctgcctcatatccgcgcgggcaagctgcgcgcccttgccgtcaccggcgacaagcgttcgcccgtgctgcccgatgtgcccacgctggccgaggccggcgtgaagggtgcggaggtctactcgtggcaaggcatggctgcaccgaagggcttgccgcccgccaccaagaagaagctgagcgacgcggtgattgccgccatgcaggacccggagacgaagaagcgcatgctcgaccagggcctggaaatcgtcgccagcacccccgaggaattcaccgccttccagttgcgcgagtggacgcgctggaagacattgatcgacactcgccacatcaccgcagattgaggcaccgagcccgaaaatgacaagtcctgaatccctttccaaagccgtgtcgggcgcccctgtcgtcaccggcatgcgcgtggtgcccgttgcgggccacgacagcatgttgatgaacctgagcggcgcgcacggcccgttcttcacgcgcaacctgctgatcctgaccgacagcgcgggccacaccggcgtcggcgaagtgccgggcggcgagaagatccgccagacgcttgaagatgcacgcgacctcatcgtgggccagcccctcggcaagcacaacgcggtgctcaacagcatgcgcagtgcgttcgccaaccgcgacagcggcgggcgcggccagcagaccttcgacttgcgcgtgaccatccatgcggtcaccgccgtcgaggcggccatgctcgacctgctcggccagcacctcgaagtgccggtggctgcattgctcggcgaaggccagcagcgcgatgcggtgcagatgctcggctacctgttctacgttggcgaccgcaccaagaccgacctgccgtacgagagcgaccccggcgccgacaacgactggttccgccttcgccatgaagaagcgatgacgcccgaagccatcgtgcgcctggccgaggccacgcatgcgcgctacggcttcaccgacttcaagctcaagggcggcgtgctgcgcggcgaagaagaagtcgaggccatccgtgcactgcacgagcgcttcccgaaggcgcgcgtcacgctcgacccgaacggcggctggctgctgcaggacgcgatccgcctctgccgcgacctgcacggcgtcatggcctatgccgaagacccgtgcggtgccgaaggcgttttttccgggcgcgaagtgatggccgagttccggcgtgcgaccggcctgcccacagccaccaacatggtcgccaccgactggcgcgagatggtgcacagcctctcgctgcagtcggtcgacattccgctggccgacccgcatttctggaccctgcagggctcggtgcgcgtggcgcagctgtgccaggcctggggcctgacctggggctcgcattccaacaaccatttcgatgtgtcgcttgccatgttcacgcacgtggcggccgcggcgccgggcaaggtcaccgccatcgacacgcactggatctggcaggacggccagcgcctgacgaaggcgccgctgcagatcgaaggcggcttcgtgaaggtgccgacgcgcggcgggctgggcgtggaactcgacatgaacgaggtcgagaaggcgcatcagctttacctcaagcatggactcggtgcgcgcaacgacgcgcaggcgatgcaatacctgatcccggggtggactttcgacaacaagaaaccctgtatggttcgttgaaggtttagtctctctcccgttttggttttccgcagccggacacgcagtgctccggcttctttctttccatcgagcagcaaggaatcctcatgcaaaacttcgacaacctgatcggcggcgaatggcgagccggcgccagctacagccccaacgtcaaccccagcaacctgaccgacgtgctgggccagtacgcccagggcaccgccgctgacgtgcaggccgccgtggccgccgccaccgccgcctttcccgcctgggccaccggcagcatccaggcgcgctccgatgccctggacaagatcggcaccgagatcctggcgcgcaaggaagagctcggcaccctgctggcccgcgaagaaggcaagacccgcgccgaaggcatcggcgaagccacccgcgccggccagatcttcaagttcttcgctggcgaatgcctgcgcctgtccggcgagctgctgccctcggtgcgcccgaacatcggcgtggagatcacccgcgagcccgtcggcgtggtcggcctcatcaccccctggaacttccccatcgccattccggcctggaagatcgcccctgcgctcgccttcggcaactgcgtggtcctcaagcccgccgacctggtgcccggctgcgcctgggcgctgtccgagatcatccaccgctcgggcattccggcgggcgtgttcaacctcgtgatgggccgcggcagcgtgatcggcgaagccctggtcagccaccccggcatccatgccatcagcttcaccggctcggtcggcgtgggccgcaacatcgccgtgcagtgcgtcaccaaccacaagaaggtgcagctggagatgggcggcaagaacccgcaggtgatcctggacgacgccgacctggcccaggccgtggaactgagcgtgcaaagcgccttctactccaccggccagcgctgcacggcctccagccgcctgatcgtgaccgaaggcatctaccccaagttcatcgaggcgatgaaggcccgcatggccaagatcaaggtgggcgatgcactggcccagggcaccgacatcggcccggtctcgtccaagtcgcagctcgaccaggacctggaatacgtggccatcggcaagggcgagggcgccacgctggccgcgggcggcgagctcctgaagctggagaccgacggctattacatgtcgccggcgctcttcagcgaatcggcagccgccatgcgcatcaacaaggaagagatcttcgggccggtcgccagcgtgatccgggtgaagaactacgaagaggcgctggccacggccaacgacacggagttcggcctgtcggcgggcattgcgaccacgagcctgaagtacgccacgcacttcaagcgccacagccaggcgggcatggtgatggtgaacctgcccacggcgggggtggactaccacgtgccctttggtgggcgcaagggttcgagctacggcccgcgcgagcagggcaagtatgcgcaggagttcttcaccacggtgaagacggcgtacacgctggcttgagtctctgcaggccgggtgcagcgcgcccggccattcggctcatcggacatggctgctgcgcgacggcctcatggcggcggcgaagacggctgcggcgcctggcgccggcggcgcatcagcatctcgacgagctcgaaaaagccctcgctcagcagcgccagtgccgcggccggcagcgcgcccgccacgagcagctcgcggtcgttgagcgccagccccgtgacgatgcgttcgccgaatccacccgcgccgatgaaggccgcaatggtcgcggtgccaatggcaatggccgtggccgttcgaatgcccgccagcagcgttgggagcgcgagcggcagcagcaccagccgaaggctctgcggcggcgtcatgcccagcgcggtgcccgccatgcgcaggccgctcggcacttcggccaggccggtcaccgtgttgcgcatgatcggcagcagcgaatagagcgtgagcgcaatcaatgcgggcagcgccccgatggcgccgagcagggagatcagcaccgccagcaatgcgagcgagggcacggtctgcaggatgctcgccatgcccagcaccagcgcgcgcagccgcacatgcgcaaacaccaggatcgcaatcggcacgccgatcaggatcgcaatgcccacggacaccgccaccagcagcaggtgctgccgtgccagctgccagagatcggggccgaacagcttggcgatgaagccgcgccggggctcccggggctgctgtgcctttccacttgtgctggccaggaagtcgcgcgcaatcgcgtcgaagggcacgctctgcagttcggcacgcgcattcatcgcgatcatcgcgcgctcgtcgatgcggccttccagcgcctgcagcgcggcccaggccttcggcagccgcgccggcaggtcgagcttgtagagcaccaccgcgtcgtagcgcggaaagtatttcttgtcgtcttccagtacgcgcaggccgagatggtcgatcttggcgtcggtggtgtagatgtcgatcgcgtcgatctgcttcgcggccacggcttcataggccaggccatggtcgaggccggtcggcgtctgcgtgaagccgtagcgcgcggccaggcccttccagccatcggcgcggccgatgaactcgttcgacaggccgagcttgagttcggggtgtcttgcgaggtcgctcagcgtgcgcaggccgagccgctcggcatcggctgcccgcaccgccagcgcatagccgtcgttgaagccgagcggaatggccacgcccaggcccagcggtgccagcgccgcattcatggcctcgcgcgtttcagctggcgagcccttgaggatctcgagtgcgatggtgccggtgtattcggcatagaggtcgatggcgcccgaacgcagcgcctcgtagacgatggccgtgttgcccagcccctgccgcaccaccggtggggatgcggtgtgcggcgccgccgtctgcgccagcagctcggccaggatgtacgactcggtgaagcgcttggaaccgacgcgcagcgtgccctcgccgggttgcgccgacgcagcggcaccgagccaggccatggcgaacaacaacaaggcggcacgcagcatgcggcggtggggcaggcacatcgggggccagtgtatagacatcgccccggtcggggcacccgccaatctcctacaaaccctggtgcgggctaccgatgctgcgaggatgcaatcgcacccatcatggccggcatgaagaagaaaacccacctcctgcccggccccgacgtgcacggcctgcgcgagctcccgggcctcagggtggagggctacagcctgcagctgcgcgacaaggacggcttcgtcggcgaccaggccagccagaccgccttcagggcgttgctcgaacgctggcgcaagcgccgccgcaagacgggcatcgatcccctggggcgggagcactcgcgcgacctcagcaaggagcagcttgaccgcatcctgcagaagccctcggatgccggcgacctgatgcacggcgccatcgaggaatttgccgaagaactggccttcgtgatccagcgcttcacgcgccagccctcatggaagaaggtggagcgcatcgtggtgggcggcggcttcaccgaaagcgacgtgggcgagcgcgccatcctgcagaccgcggccatcctggaagacatgggtgtgcacgtacagctcgggcggctgtcgcacgaggtcgacgacggcggcctgatcggctgggtgcacctcacgccgccggccatgctgaagaagcacgacgccatcctggccgtggacatcggcggtaccaacgtgcgctgcggcatcgtgaaggcgcgccggcacaaggcgcgcgacctgtcgctggccaaggtcgtgcggcgggagaagtggcgccatgcggacgacagccccaaccgcaccgacatggtcgagcgcatcgcgctcatgctcgaggacatggcccgctactgcgagcgcaagcacatccgcctcgcgcccttcatcggcatcgcatgccccgggctgattcgcaaggacggctcgatcgagcgcggctcgcagaacctgcctggcgattgggaaagccgcgcgtttcacctgcccagcgcgctgtggcgccgcataccgatgatcggctccggccccacgctgatcctgatgcacaacgacgcggtggtgcaggggctgagcgagcttccgttcatgcgcgatgtttcccattggggcgtgctgaccatcggcaccggccttggcaacgcgagcttcaccaataccttctagtccggtgcggctgccgctccggcagcggacggtatggtgccgccgagtgccttgtagacggccaccatgccaaccgccatgcggttcgcgctctgcacgcggtcgcgccgggcctgcagcagcgtgcggcgggcgtcgagctcgacaccgaagtccgtgagcccgttggcatagcgcgcatgcgcgagtgtgagcgcgtcgcggctgttgcgctcgcgctcgatcagttccgcatggcgctggcgctcggcggcataggcgttcagcgccgaatcgatctcgtgccaggccttgagcaccgtctgctggaaggccaccgcggcttcctgctgctgcagctcgcgcagggtcaccgtgctccggcgccggccgttgtcgaagatcggcaggctgatggaagggccgatgtgccattgccggctgccccattcgccaaagcgctcgctgccagccgattcatagccgaagcccgcaccgagcgtgacgcgggggtagaggtccgccaccgcaatgccgatgcgtgcggcggcggcgtgcagctgcgcctccgccgccgcgatgtcgggccgccgtcgcgccacgtcggaaggcaggccgagggcaagttcaggcagcggcggtgcttgcaatgcttcgagcgggtcgcccgtgccgccgtcggaaggcgacgcgagttcggcgttctgcgtgccgggcggcgcgccggtcagcagcgtgatctggttcatggcttgggcttcctgctgcagcagcatcggaatgcgtgcacgcagctcggccagttgcgtgcgctggcgggtcgggtccaggtcggtgaccaggccgccgtccgcgcgcgcctgcaccagctcgagcgactcggccgccgccgaaatgtcggcgcgcgccagccgcagttcgcgctgcgcaccgcgcagttcgaagtagttgcgcgctacctcggcctgcacgctgagctgtgcctgccgcagcagggcggccgatgcgccggcatccgcatcggcggcctcgatgctgcgccgaacgcggccccacaggtcgatttcccacgacgcatcgaagccggcctggtagaggttgtagggctcgctcagcgtgcggatcaactggtcgcggttggacaccgacgaacccagcgcatcgatcatccgcgtggccgcgccggtctcgctctggcgttgccggttgacgccgccactggcattgagctgcggtgcctgctgcgccgccgccgcggtgcgctggacgcggctttgcgcaaagcgaagggcggcgctctgcaggtcgtgattggcctccagcgcgcgtgcctgcaggcgatcgagcagcggatcgttgaaggccttccagtcgccggatgcagcgcccgtgggcaccgctgtccgctcggtgccgagcagtgcttgcgagccgccgtgccatgcggaccagtcggcgggcgcctgcggttccgcgggccggtggtcgggacccacagcgcatccggcaagaagaagaagcgcgagcgcggaacaggagaagtatgcggagggggtgcgcgatgcaggcatgcggtgctcccggtttcaggccaggcgatggcgaaacagccaagccgccagcggcagcgtgacgagggcgatgatcgatagcggaatgaggttgtgccacactgtcgccaggcccacgccctcgaggtacacgcgctgcaccaggtcgatcgcaaagcgcagcggattggccatggtgatcagctgcagcacgtgcggcatgttgcgcaccggcgtggtcaggcccgacagcagcatcatcggcatcagcagcacgaaggtgtagagcatggcctgctgcatgttggccgacaccgccgagatcgagaggccgatgcccacgctggccatggtgaagaaaaccagcccggtgtagagcgtggcgagcgagcccgccatcgggatgccgaaccagaacagggccaccagcaggatcagcgtcgactgcgcaaggccgaccagcacgggcggcagcgctttgccgatcatgatttcgagcggcgacatcggcgtgaccagcaattggtcgaaggtgccttgctcgcgctcccttgcgaccgagagcgccgtgagcatcagcgtctgcagcatgctgagcgcggcgatcaggcccggcagcaggttccagcgtgtctggaggttcgggttgaaccaggcccgcgtttcgatggtgagcggtgtgggcggcgcgccggcccgcgtgcgcagctcggcgttgtagcgctcgaccaccgcgctcacgtagccggccgcggagcccgccgtgttggagttgcgcgcatccagtatcagctggatggccgcaggctggcccgcgccgagttgctgctcgaagttggatgcgatctggaccaccagcagcgccttctccgtgtcgatcacctcccggatgtccgcctgcgtgcgcagcgtggccacgcggtggaagacgccggtgctgtcgagatgcgcaatcagctcggtcgatgcaccggtgcggctctggtcgagcagcgcatagggcacgttcgtgaggtcgtaggtggcggcgtagccgaagatgaggctctgcatgatcgcgggaacgaacaggatcacgcggctcgccgggtccttgaagatggcgagcagctctttcctgcagaggttggcgatgcgcagcagaaaatcggtcatggggtgccgtccttcagtcgaggctcttgcgtgtgacggcgcgggcaagcagcagcaggcccaccgcatacgccagcaacactgcgcagttgcgccagatcagcggccagacgtcgcccgcgagaaacagcgtcttgatcaggtccatgaagtaggtggccggcagcacatggccgatcacgcgcacggcaaggggcacgttgcgcaggtcgaacaaaaatcccgagagcatcatcgaaggcatgaaggtggcgatgagcgccacctggctcgcgagaaactggttgcgcgtgaccgacgagatcacgaggcccaggctcaccgcgacgacgaggtagagcatggagctgagcaccaccgcgaacagcgagccgtacatgggcaccgcgaacaggaagcgcgcggccaggagacacagcgccaggcccagcatgccgaccgcaaagtacggaatgatcttggccagcagtatttccaccggccgcaccggcgtgacgaacagcgcctcgagcgtgccgcgctcccattcgcgggccatcaccagggcggtgagaaacgcgccgaccagggtcatgatcagcacgatgaggcccggcaccaggtaccaggtgctggtgttcgcggcgttgaaccacatgcgctgctccacggtcacgcggcccgttgggggtgcgtccgcaccggttctgccgccgccgcggtccgcctgccgcacggccgtttgcgcaagagcgccgctcacgtacgcctggatgatggtcgcgcgccccgcgtcggccccatgcacgatgagctgcacgcgcgcattgcccgcggccagcgcgcgcgaaaaatcggagggcacgcgcacgacgccgtcgatcttgcgttcgcgcatcaagacctcggcgtcgtgcatggagcccagcagcacgggcgcgatggtgggcgaaagctgcaggccggcaatggcttcgtgcgccgtgggcgaggggtcttcgagcaccacgcccaccggcgcgttcttcacgtcgagcgacatgccgtagccgaagatcaggatcagcaccatcggcagcaggatgccgatggccaggttgctgcggtcgcgcagcagctggcgaaactccttgcgcgtgagggagatcagccgggtccagaacttggtgttcattgggcgacctctgcgctcggatggccgattgcggctcggctgttgctccctctcccccggggagagggcaggggtgagggcgtcggccttcgcaaaagctcagaccacgccaccgtcgccggccctcacccccgccctctccccgaggggagagggggcaagagatggcattcataaggtgacccccgcggcggaatttcttccgttcgtgcgtgccttctcgacgatgccgatgaaggcctgctccatgtcgatgcgcttttcatgaccctcgccatcgagcgcctgcgcgcgcacctcccgcggcgtgccgatggccagcaccttgccggcgtcctggatcacgatgcggtcgcagtactcggcctcttccatgaagtgggtcgtgatgacgacggtggtgccgccttcggccagtgccgtgatgcggcgccagaactcgcgccgcgccagcggatcggcgccgctggtgggctcgtcgagaaacaggatctcgggctcgtgcagcaggccggtggccatcgccaatcgctgccggtagccgccgggcagctgcccgctgggcgcatcgagttcgcgctccaggtcgaactgccgcaacaccgtgtccatgcgcgcctgcagcttttctccgcgcaggccgtaggcgccgccaaagaaggagaggttctcgcgcaccgtgaggttgccgtagagcgcgaacttctgcgacacgtagccgatgcgctggcgggcctgcgcgcgtgcatggcgcaggtcgacgccggccacgcgcagctgcccgccgctcgcgggcagcaggccgcagagcatgcggaaggtggtggtcttgcccgcgccgttgggtccgagcaggccgaagatctcgccgcgccgcaccgagaagctggtgcttgccacggccacgaaatcgccgaagcggcgcaccaggtctttcacctcgatgaccacttcgccgggctcgccttcggccggtgcaagtccttcggccgcggcgagtggtgcgacgtgcggcgcagtggcctggtgggtacgcagcagcgtcatgaagccgtcttcgagccgcggcggcacgggctcggcgcgcgcgccgtccagcagcttctcgagcgccgcgtcgtccgcgccctggcggcggatgaagtgaacttcgccgccctgcggcacggcgtcgacgatgtcctgccgcgcatcgagcaggcgggcctgcatcaggcgcggcggctcgccctcgggcggcgcggcgacgaagcacatgccttgcgcatggccgcgaatctcggcgggcgtaccctctgcaatcagccggccctcgcgcagcacgaacacatggctgcagcgctcggcctcgtcgaggtaggcggtgctgacgatgaccgaaagcttttcgtcgtcgaccaactgctgcacgatctgccagagctcgcgccgagagagcggatcgacaccgacggtgggctcgtcgagcagcagcagctcgggcgagcgcaccagcgtgcaggccaggccgagcttctgcttcatgccgcccgagagcttgcccgcgggccggctggtgaagcgaccgaggtcggtcatttccatcagccgcgcatagcgctcgcggcgttggccggcggagacgccgtgcaggtcggcgtagagatcgaggttctcctgcacgctcaggtcgtcgtagaggccgaagcgctggggcatgtagctgatgcggtcctgcaccgcctgcgggttggccgatacatcgatgcccagcacgcgcagttcgccttcgtcggcacgcatcaggcccgccatcaaccgcaggagcgtggtcttgccggcgccgtccggcccgacgagcgcggtgagcgtgccggcgggcacctcgagcgagacgccggccagcgcatgcacgggctgcttcgacgccttgagggtgaagcgcttgtgcagggagcgtccggccacggccggctcagtgcgctgcattcaatgcccctccatgctggtggtcttgctccttccccctctgggggaaggttgggatgggggcaggcagggcgctcgatggacaggccgcttgcccccaccccagccctcccccggaaggggagggagcaatgcgcaacggcggtcgatgaggtccatcatcacggcttgccgttcggaggcagctgcagccgcacggtcgccggcatgccgagtcgcagccggtcttccttgtcgtcgaccatcacgcggatttcgtagaccaggctgctgcgcagctcttcggtctgtactgtcttgggcgtgaactcggccaccgacgagatatagccgaccttgcccgtgatctgctggccgggctggctgtcggtggtcacgctggcctcctggccgggccgcacgcggccgaggtcgggttcggccacgtaggcgcgcacccacttgggatcggtgatcgccagcgtgaaggccgggcgctgcggcgaggccatgtcgccgggctcgagcaggcgcgcgcgcaccacggcgtcgatgggcgacttgagctccgcctcctggagctggtggttcatgagcgccagatcggcgcgtgcggattcgagctgggccagtgcctgcgcgatgtcttccttgcgcggcccggcgacggcgagctgctgcgccttgcgcacgttgtccagttgcgccagcgccaccttgcggcgggcctgtgcgctgtcgaggtcctgctggctcacggcccggccggccgtggtctggccgatggcctgcaggcgcacgagttgctgctgcgcaaggtcggcatcggcctgcgccgcggccacctgggcgccggcctgcgcgagttcttcgggccggctgccagtcttcaggcgcagcagcgcctgctcctgcacgccgatgcgcgcctgcgactgcgccacgcgcagcacgagcgagcgggtgtcgagcctgcccagcaactgccccgcgcgcacgtggtcgccttcgcgcgccgtgagttcggccacgcgctcattggcattgaaggccagcgagacctggcgcacgtcgatgttgccgtacagcacgagctggtcggacggcgtggccgaacgatggaggtaccaccagccacccgccgcagcggccagcaccacgacggcagcggcaatgaggggtttcttgttcatgagaacgggctcctgccggttttcagaccggaacacggccggatgttatcaaatcgaaatttgaatttgaagtattttttcaattcgattaacctcggggccatggcttcccgctcttccagcacccgttctttcggcgccagtgcccctgctccgcgccaggctgcggcacgcatcccgcgcacctctcgcaccgacggcagcaccacgcgcctgcacatcctcgaaaccgcgggccagctgtttgccgaacgcggcttcgccgagagcaccagcaaggaaatctgcacgcgcgccggcaccaacatggccgcggtcaactaccacttcggcagcagggacgggctctacgaggccgtgctgatcgaggcgcatcgccagcttgtgagcatcgacgaactggtcagcctggccagcgcggcggccgatccgcggctcaagctgcgggcctttctcacgcacctgatcgagatgggcagccagcccaaggcaccctggggctttcgcgtggtgctgcgcgaggcgctctcgccgtcgccggccatgccggtgctgatccggcgggcggtgctgcccaaggccaagctgatccgcggcctggtcggcggcatcatggggttgcccgacgatcatccgtcggtgcagcgtgcgctgctgttcactgtgttgccctgcatcgtgatgacggtggcgcccaagaatctgcgcaacgaggtgctgccggccctgaagaacgccgagggcctggcggacgacctgatgcgttacgtcttcgcagggctcgatgcccttgcggtggaggccagggccttggcgcccggcaccacggcagccaaaactacagctggaaagcgacggtgagcagcagcccctcggccacgtcgcgcaacaggcccggccgccgcgcgcggtagggctcgccggcggaagccgtggtggcgacccattcggccagccagtcgatctcgcccgggccgtagaacaccacggccgcctcgtggttgagcagcaggctgcggaggtcgaggttgatcgagccgcacatggccagctcgttgtcgaccaccacggccttggcgtgcgccatgaagggcagcatgcgaaagctcacgcccgcgcgggccaggtcgcgcatggcccgcgcgcgcacgaagtcggccaggcggtggtttgaccgcgcggggatcgcgatggtcacttccacgccgcgccgcgcggccagccgcagcgcatcgcgcaggccgtcgccgggcacgaagtaaggcgtgatcgccagcacgcggtgctcggcccgaaagcaggcgtcgatgagcagcgcatgggccgtgtcctcggtctggtcggggccgctcggcaggaattgcgccatggcgccgcccgcgctttccacgtcgtcggccgtgatggcgcgcgccttgcggccgcgcaccgagctccagtcgtggtcgaactgacgcgccgccgcggcggccacgctgccgtgcaggtcgaacgaaagatcgcgccagccttcgggatgcttgtcgttgccggtgaagtattcgcccgccagattgcgcccgccggaccacagccagccgtcgtctgcaatggtgaacttgcggtggttgcgcaggttgcgcggcccgatgcggcgcaggctgaagaacgggcggaacacggcgacctcgccgcccgccgcgcgcagcagttcgaagtggcggcgcggcaatgtcagtgcaccgaagccgtcgagcagcacgcgcaccttgacgccttcgcgcgcacgctgcgccagccgctcgatgacggcgcggcccagcgtgtcgtcgccgatgatgaaggtgcacacgtcgatgcgctcgcgcgcgccgtccatcacttgccacagtgcctcgcgcgcggcctcgccgtcagcatgcaggcggatcgcgcagcggcccggcggcgcgaggccgaagctttcgatcaggtctgccgcccagtgccccggcggcaccgagcgcggcggccgcggcgagcccgccgggcgcagcttgcgctggccgaacaagaggtagatcggcaggatgaagtagggcatgagcaccagccccatgacccaggcaatggccgtggtgggcgcgcgctgctcgcggcgcgcgcgcgtggtcagcacatagaccagcagcgcgaaggtgatgacaaggaaatgctgtgacggtgaaggaagccagtcgaaactcgagttcggcatgcggcaatgatgcctgaggacccgggggagcggcgtgcgatcagcgtggcatcaggaacgaggccacgtcgcgcccttcggaagccaggaagcgcatcatcggctcgaccaccgttcgcaccgcgggccgctcgcccatgcggctgcgccaggccaggagccgcggcgtcgcctgcgtcatgcgggcacctttgcggtcggcaaagatgcaggccatgtagaaggcgatgtcggcgaaggagtagggccccgcaaggtactcgcgcgtggccagcaggccttccatctcgtcgtagtagcgggcgcacgcggcgcaggcggccacggcgggcgcgctctgcatgtcgcgctgcaggccgaagagcctgatcacgttgggaaaaaagacctcgtccgacttctgctcaagctgccgcgcgcgtgcccgttcggcaacatcctggggccacagcgccggcgtggggtaccggtcttcgaggtactcgaagatctgcgtcgagtcgaaaagcccgacctcgtcgtcgacgagtacgggcacctgctgcttcaccgggttgacgcgcagcacctcggggtgcttgggctcgtaggcgtcgtctttggtgaacggcaccatcaccagttcgaagtcgatgcctttttcgagcgcggcgatctgcaccttcgcgccgaacatgctgagggggcccgagtagatttttgtggtcgtcgtcgtcatgccccgactacatcagaaatgccggttcaggtcgagccccagacttcttgtgcggtctccaccaccagccgcagcttgttgcgctgcgcctccaccgcgatgttgttgccgtgcaccgtgctcgagaagccgcattgcggcgacagcgcgagctgctcgagcggggcgtacttggcggcatcctcgatgcggcgcttgagctcgtccttgtcttccatctcgccgaacttggtggtcacgaggccgagcaccacggtcttgcccttgggcaggtagcgcagcggcttgaagtcgccggagcgggcatcgtcgtattccatgaagtaggcgtccaggtccatctccttcaagagcgcttcggccaccggctcgtagttgccggccgccgcgtgggtgctcttgaagttgccgcggcacaggtgcatggccagcagcatgcccggcggcttttgcgcgaccaccttgttgatgaacgcggcatagcggtgcggcagttcgttcgggtcgtcgccgcgcttgcgggcggcttcgcgcatgtgctcgtcgcacaggtaggccaggttggtgtcgtccatctgaacgtaggtgcagcccgctgcggccagcgagcgcagctcgtcgccataggccttggccacgtcgtcgtagaacaccggatcgagctcgggatacgcgtccttgctgatgccggcgcggccgccacggaagtgcagcatggtgggcgaaggaatcgtcaccttcggtgtccggccggccgagacttggctcttcaggtattggaagtcagccagctggatgtccttcacgtggcgcaccttgtcgatcacgcgcatggccggcggcgcgagttcctcggtgccgtcgggcctgcggatggtgaccggaatgtcggtcttcacgccgccgagctggtcgagaaagtcgatgtggaaatacgtgcggcggaactcgccgtcggtgatgctcttcaggccgatgtcttcctggaagcggacgatctcggtgatggccttgtcttcgaccttgcggagctgctcgggcgtgatctcgcccttggccttctgctcgcgcgcctcgagcaggtatttggggcgcaggaagctgccgacgtggtcgtaccgggcgggcagggcggcgtgctgggacatggggaatctccgtcgtggctgtaaacgaatcgaagatcgtatcgccttggaaacacgcgtacctgtatacattaatctcggtgtttaccctgaattcggcgagtttcagtggaaattttctgatttatgtatacattgggtattcatgaaaacgcccacgaccgcctttccattgaacgcctggtatgccgccgcctatgacgtcgaagtgcgtcatgcgctgctgccgcgcaccatctgcaacgaaaaactggtgctgttccgccgtaccgacgggcaggttgccgcgctcgaagacgcctgctggcaccgcctgatgccgctctcgctgggcaagctcgaaggcgacgaagtggtgtgcggctaccacggcctggtctacaacagccagggccgctgcacccacatgccgagccaggaaacgctgaacccttcggcctgcgtgcgcagcttcccggtggtcgagaagcaccgcttcgtctggatctggcccggcgacccggccaaggccgacccggcgctggtgcccgacatgcactggaacgacgacccggcctgggccggcgacggcaagatgattcgcgtgaactgcgactaccgcctggtggtcgacaacctcatggacctgacgcacgagaccttcgtgcacggttcgtccatcggcaaccgcgaagtggccgaggcgcccttcgttgccacgcacggcgaccgctcggccaccgtcacgcgctggatggagaacatcgacccgccgccgttctggggtggccagatccgccatgcgcgcggctacgccggcaaagtcgatcgctggcagatcatccgattcgaagggccgtgcaccgtgaacatcgacgtcggcgtggccgaggcgggcagcggcgcggtgccgaaggacggcaaccccggcgaccgcagcaagggcgtgaacggctacgtgctcaacaccatcacgcccgagaccgacaagacctgcctctacttctgggcctttgcgcgcaactactgcctgggcgagcagcgcctgacgcacgaactgcgcgaaggcgtggccggcatctttcgcgaggacgagctcgtgctcgaggcgcagcaaaaggccatggacgagcggcccgaccaccagttctacaacctcaacatcgacgccggctcgatgtgggctcggcggctgatcgaccgcatggtcgagaaggaaaaacccgcgcgcgccgcgatcccgatccgccctgtcgaaaagagcgccgcatgaaggtcgcagccgtatcccccgtcgaacccggcgatggcggcagctcgcaggccgtgaaggcgcagctgcgattgcgcgaaatgatcctggccggcgaactgccgggcggtgcgcgcattgccgaggtggccatctccgaacagctcggcgtttcacgcacgccagtgcgcagcgcgctcatgcggctggaacaagaaggcctgctcgaggcgctgcccaacggtggttacgcagtgcgtactttttcggagcgcgacgtggccgatgccatcgagcttcgcggcacgctcgaaggcctggtggcgcggctcgcggccgagcgcggcgcggcgccggtggtgctgcgcgaagcgcgcgcctgcctggcacgcatcgacgaactgctgcgcgagcccgcgctggacgatgcggcgttttcgcgctacgtcacgcacaacgagaagttccattcgctgctgtgcgaaatggcggcaagcccggtcatcgcgcagcagctcgagcgcgtgatcaacctgccgttcgcgtcgccgtcgggcttcgtcatcgtgcaggccaactcgcccgccgcgcgcgacatgctcgtgatcgcgcaagaccagcacctgcaggtgctcgacgccatcgaggccggcgaaggctcgcgtgccgaagcgttgatgcgcgagcacagccgcatcgcgcggcgcaacctgcgcgaggcgctgcacggcacgcccaccgccgagcagcgccccctgcccggcgtgcagctgatccgtcgccgcggctgagcggccgatttactttttccgctgtttctccccgatgaaaaacgaccttcaatggatgcaggcgcaaatcgttgcgctgcgcgacgtcacgcccaccgtgcgcgaattcgaactgcggcccgagccgggctttgccgccacctacgagcccggatcgcatctgcaggtgcaggtgatggcggcccatggcaagctgcagacacgctcgtattcgctggtgggcgagggcgacggccagtgctggcgcattgccgtcaagcggctcgacgacggccgcggcggctcgctcgccatgtggcgactggccgtcggcgaccggctgcaggtgagcgcgccgcagaaccactttgcgctcgacctctcggcgcccggctatctgctggtggccggcggcatcggcatcacgccgctggtgatgatggcagagcgcctgggagaccatgcgcggcgcagcggcgtgccggtgaagatgctctacggcgcgcgccatgcgggcgagttcgcctacctcgaccggctccgcgaagcactgggcggcgatgtcgtcgcgcatgagggcgcggcgcccatcgatttcgcggcggccatcgcggccctgcccgcgggcggccagctttacacctgcggaccggtgcccatgctcgaagccgtcaagcgcgcctggcaggcggcgggccgcgccccggcagacctgcgcttcgaaaccttcggcagcagcggccggcttccgacgcaggccttcacggtgcgaattccccggcacgacctggcgatcaccgtgccggccgattgcaccttgctcgaagcgctcgacgccgccggggtggaaacgctctgggactgcaagcgcggcgagtgcggcctctgcgctatggacgtgctcgcggtcgatggcgaaatcgaccaccgcgacgtgttcctgagcgagcacgagaagcaggcgaccacccgcatctgcgcctgcgtgtcgcgggccgtgggcaccctcacgctcgactcggcgtatcggcctgacagctgaaaacgcgttgcgcgatcatcgcgcagttcatttgttcatcgcgcaacaatggttcgcctcgggggcggagtaggtgattgcctgctccgccgcatgttgcaaagtgttgaaaaatagcccggtatccgctttcgtcgttcaaggaaaacctcatgcaaagacgccaactcatccagaccgcaggcctcacggcgcttgcgctttccatgtcgcttgccagtgcgcaggacagcaacaagttcaagatcggcctgatcctgcccatgaccggccagcaggcgtccaccggccggcagatcgaagcggcggcgcggctgtacatggcgcagaacggcgacaccgtggcgggcaagaagatcgagctcatcatcaaggacgacgtggccacgcccgacgtgaccaagcgcctggcgcaggaactcatcgtcaacgacaaggtgaacgtgatcgcgggcttcggcgtcacgccggccgcgctggctgccgcaccgctggccacgcagtcgaagacgccgcaggtggtgatggccgccgccacgtcgagcatcaccgaagcctcgccctacatcgtgcgctcgagcttcacgctgccgcaggtgtcggtggccatgggcgactgggcgccgaagaacggcgtgaagacggtcgtcacgctggtggccgactacggccccggcaacgacgccgagaaattcttcagcgagcgcttccagctcaacggcggcaaggtgatcgagaagctgcgcgtgccgctgcgcaaccccgatttcgcgccgttcctgcagaaggtgcgcgacgccaagcccgacgcgctgttcgtctttgtgccctcgggcgccggcgcggccgtgatgaagcagtttctcgagcgcggcatggacaaggccggcatccgcatgattgccacgggcgacgtgaccgatgacgaccagctcaacgacatgggcgatggcgcgctgggcgtggtcacttcgcaccactactcggccgcgcatccgtcgcccgcgaacaagaagttcgtcgaagccttccagaaggccaacccgaagatgcgccccaacttcatggccgtgggcggctatgacggcatgcgcgtgatctatgaagccctgaaggccaccaaggggcagggcgggggcgatgcgctgctggccgccatgaagggccagatcttcgagagcccgcgcgggccggtgtacatcgatgcgcagacgcgcgacatcgtgcaggacgtgtatctgcgcaaggtcgagaagaaggacggccagttgtacaacgtcgagttcgacgtgatcaagggtgtgaaggatccgggcaaggcgaagtaatcgggtgcccgggtgttttgttcgggcgctgctgctgttcagggtggcgctcccgccgacggggtgccttgctccgcgaatgtcccccggcctgcggcctcctcctttatttcgctgcgcaaggcaccccatcgacggaatcgtccgtcagagcggtcgttgatcggcggtacacccagagcatgccctggtgcgcagggcgccgggtgctccccgcagcgaaataaaggaggaggcgaagccgggggacattcgcggaggggagtacccggtggcctgtgcacgcgccctgaacagcagcgcccaatacaagaaccaaagaagccaacgcgagccatgcaaacgccgtagcggaacactgacatgttgaccattcttttcgacggcattgcctacggcatgctgctcttcgtgctcgcagtaggactggccgtgacgctcgggctgatgaacttcatcaacctcgcgcacggtgcctttgccatggcgggtgggtacctcacggtatttgcgatgcagaagctgggcgtgccgttcctggcctgcctgccgctcgcgttcatcgtggtggcactggccggcgcgctgctcgagcgcacgctctaccggccgatgtacggcaagccccatctcgaccaggtgctgttctccatcggcctcgccttcatggcggtggcggccgtcgactattttgtcggttcgtcgcagcagaacatccagttgcccgaatggctgcgcggccgcaccgagatcggcgatggcgcgctgctgcttggcatgggccactaccggctcttcatcatcgcggtgtgtgccgtgctcacggtggtgctccagctcattctctcgaagacgcgcttcggcagccgcctgcgcgccgcggtcgatgacccgcgcgtggcggcggggctgggcatcaacgtcaacatcgtcttcttgctgacctttgcggtgggctccgggctcgcggggctgggcggcgcgctgggcgccgagattcttgggctcgatccgacctttccgctcaagtacatgatctatttcctgatcgtggtgtcggtcggcggcacctcgtcgatcaccgggccgctcgcggccgcgctgctgctcggcattgccgacgtggcgggcaagtacttcattcccaagatgggtgcgttcaccgtctacctgctcatgatcctgatattgatgtggcggccccaaggcctgttcacgcgcaagggaggccgctgaatgagcgcaccttcgtcgtacgaatcggccttgctgcacaaggcgcgctggcgcccgctcgagttcgtggtgtgggccgcggccttcgcgctgcctttcgtcatgccttcgcactcgctgctggtcaacgagatcgccatcgtcgcgctgttcgcgatgtcgctcgacctgattcttggctacaccggcatcgtgtcgctcggccatgccgcgttcttcggtttcggcgcctataccgcggcgctgttcgccaagctcgtgatgccggacccgaccgtggggctggtgctggccaccgcactgtcggcgctgctgggcctcgtggccagcgtgacgatcctgcgcggcagcgacctgacgcggctgatggttacgctcggcatcgcgctgctgttgctcgaactcgccaacaagctcgactggctcaccggcggtgccgacggcctgcagggcgtggtaatgggaccggtgctcggcctgttcgagttcgacctcttcggccgcacggccgcctggtattcattgagcgtgatgctcgtgctgttcctcgtgatgcgacggctcgtgcattcgcccttcggcgccacgctgaaggcgatccgcgacaaccggctgcgggccatggcgatcggcattccggtggtgtcgcggctggtcgtcatctacaccgtggccgccggcattgccggtgccgcgggtgcgctgctggcgcagactaccggcttcgcctcgctcgacgtgctggccttcgaccgctcggccgatgtgctgctgatgctggtgatcggcggcgtgggttggctctatggcggcgtggcgggcgccatcgtcttcaagctgctgcagaactggctctcggccgtgacgccgcaatactggatgttctggatcggcctcttgctggtgctgctggtgctcgtcgggcgcgatcgcgtgctcaagccatggacgtggctgggcaagaagaaggggagcggggcatgaccgaaaccgtgctctcgacgcaggggttggtgatgcgcttcggcggcatcacggccaccaacaacgtcacgatggaactcaagcgcggcgcgcgccatgcgctgatcggccccaacggcgccggcaagaccacgctcatcaacctcttgaccggcgtgctcacgccgaccgaaggccgcatctcgctgctgggcgaagacatcaccacgctggcgccgcacaagcgcgtggcgcgcgggctggtgcgcaccttccagatcaaccagttgttcgactcgatgacgccgctcgaaacgctggcgctcgtcgtgtcgcagcaccagggcatcgcgtcgcaatggtggcgtccgctgggggccacccgggccgtgacggcgcgcgcggcgcaactgctggagcagtttcatctgggcgacgtggcgcagcagcagaccaagttcatggcctatggcaagcgccgcctgctggagattgccatcgcactggcctgcgagccgcgcgtgctgctgctcgacgagcccgtggcgggcgttcccgcaggggagcgcgaggagctgctgcagaccgtggccgcattgccggccgatgtgtcggtgctgctgatcgagcacgacatggacctggtattcagctttgccgaccgcatgaccgtgctggtcaacggcacgctgctgaccgaaggcgaccccgaaaccattgccaacgatccgaaggtcaaagaggtctatctgggccacggggagcatgcccatgtctgaactgctgcgcatcgagaacctgagcgccggctacggcgaggcggtggtgctgcacgacgtggcgttcgcgctcggcgtgggccagacgctggcactgctgggccgcaacggcacgggcaagaccacgctgatcaacacgctggcgggggccactcggcagcacggcggcagcatctcgctcagtgggcaagccctgcacaagctggcgccgcaccagcgcgccgcggccggtatcggctgggtgccgcaggagcgcaacatcttcaagtcgctcacggtgcatgagaaccttaccgcggtggagcggcccggcaggcccggagggacttccaatccctggaatccgcagcgcgtctacgagatgttcccgcgcctggccgagcgcaagaccaacctgggcacgcagctttcgggaggcgagcagcagatgctcgccgtgggccgcgcactggtgctgaacccgaagctgctgctgctcgacgagccgctcgaagggctggcgccgatcatcgtggaggagttgctgcgcgccattcgccgcatcacgcaggacgaggggctggccgcgatcatcgtggagcagcacccgcaggcgatcctcgcgatttccgaccacgcggtggtgctcgatcacggcaccatcgtccacaccgacagcgcagcggcattgcgcagccagccgcaggtgctcgaacggttgctgggcgtggcccggtagcgattccgacgaacaagaaggagacagacacatggcgatcccgaagacactgttttgcgggggcgccatgtgggcctccgcgatgctgcttgcggcctgcagcaccaccggcccgcagagcctcacgctcggtggcaatccggccgcggcctgcgcggcgctcgttgcgccggtcgctcccgcggccatcggcctgccgagcggtgtggcgaccatcgattccgcaacactggtgcccgcctccgcacttgctgtcgcggagcgcggccccagtcccgctgcgcgcatcacgccgccgacgcccgcgcactgcaaggtgctgggccgcatcgcgccgctcgatgcgagcgcgccacccatcctgtttcaggtgaacttgccgctcgcgtggaacggccgcagcgtgcagtacggcggcggcgggttcaacggcgtgctgatcaccggcctttcgctggtgccggccggccgcttcgaccagcccacgccattggcacagggctacgtgacctacggcaccgactccggccaccagaacgtggcaggccagccgccgcaggcctttgcgctcaacgacgaggcgctggtcaattttgcccatgcctcgtacaagaaggtgcgcgacgtggcggtggcgctgatgcagcgcgcctacgggcaggcaccgcagaagctgtacttcgtgggcagctccgaaggcgggcgcgaggcgctcaccatggcgcagcgctatccgcaggacttcgacggcatcttcagccgcgtgccggtcatcaactggacggggctgcagcatgccggcacgcgcaacggcattgccaccttcggcgaagggtggctgcggccggcgcaggtgcagctggtgcataacgccgtgctcgcagcgtgcgatgccgcggacggcgcggcggaccgcatcgtgtcgaaccccgtggcctgcctgcagcgcttcgatcccgcgagcctgcgctgcgccgccggcaccagcggcgacaactgcctcaacgatgcgcaggtgcaggcggtgcgcacgctgcgctcgccctggcgctctcccgtgccgctggccaacggcgtcgcggtgtatccgggctggggcatcggcggcgagggcacaccggcctttgcatcgatgggaggctggaacgcctggtggacaggcaccgcagcgccgaccgtgccgccgcagccgagcaacggcattgcatagttctacggcagcggcgcactgcagtatttctatgcacgcaatccgtcgctcgacgtgcgcaactaccgcgcggaagactttgccgcgcgcatcgccaccgtgtcgcagctgatggattcgaccaaccccgacctcggcgccttccaggcgcgcggcggcaagctgctgatgttggagcacatggccgactattcgcagagcccgttcgccggcatcctctattacgaatcggtggtggcgcgcatggggcgcgacaacacggaccgcttcatgcgcctttacaccgcgcccggcgtggaccacgtgggcagcggcgccccggccaacgtcgacatgctcggcgcgctggccgactgggtcgagcgcggccgcgcgccggccggcctgcagctggccgagcaggaattgcagccgccgttcagggtcgttcgcgcccgtccgctgtgcgagtggccgctgtggccgcgctacgtgggcggcgatgtgtcgcaggccgcgagcttccagtgcagcaggtagcgcgacgcgcctgaagggcctagatcgcgcagctttccggaccgcaggatgccggaccggtaccggcatccgttgccgcgggcgagggcggcacgagcttggccagctgcgccttccattcctcgggtcgcccgagccaggggccgatgtcgatgcggctcgcggtgccgtcggcctgtgccagcacgaaagtcggaaagccctgaccgcccgcgcgttgcagccactggcggctttcggccatgtgcttcgaggttgcttcgcccgacaggcgcgcgaaggccgaggcaaaagcgtccgcatcgaagccgagctctttggctatcgcggcgagcacctgcgcatcggcgatgcgccggccttcgacgtaatgcgcgcgctgcagccgatggatcatgtccagcccgccgcccgtgcgcagcgcttcggccgcaagaatggccgtggtcggcggttcggaatccatcaccgcgccgatgtcgcgcagcaggccctcgaagtacgcctcgccaaaaggctggcccgtgagctcggcaatgcggcggtcgtgcggcaacacgtagtcgcgccactgcggcgtgatggcgcgccggttggcgccggtcatcatgccgccgccgtgaaacgcgacatcaaggcccggcacgctgcgcgcggcgtcgaccagtggtgcggccgcatagcaccagccgcacatcggatcgaagatgtagtgcagggtggcgctggacgttgaagtggtgttgtcgttcattgcgttcgtttcctttgttcgaatgttaggttccagaaaaggaaacaaaaaccccgctttcgccaatgaacagtttccgattccgttcgagtcagggtgcctagcgatctgtcccgcaccgttccagatgcgccaccagcagctgcgccgacagcgacagcgtcgcttcgtcgcgaaagcagatcgcgaagcgccggcgcgcccaggcatcggtgagcggcatcagccgcaggcggtaggtgtcggcaaagggctgcgccacttccgccggcaccacgctgatcgccagcccggcgcgcaccacgcgcaaggcggcatcgaagttggtcaccagcacgcggtacaccagcggcttgcccgccaccgcggcctcgcgggccagcatcagctgcacggcgctcagggcgggcatgccgacgaactcgtggtcgagcacgtcctcgaaccgcaccttgccgcggcgcgccgccgggtgcgacgggtgcgccacgatggccaggtggtcgctgcggtagctgcgccgctgcaggccttcgaggtccgcggcgtcccagcacaggccgatcgacgcgctgccctcgcggatgccgcgcacgatttccgggctcacgcgttcttccatatcgacccggatgtcgcggtgtttggggttctgcagaaagttggccacgtcctcggccagcgattcggccagcaccgaggccgaggcaaggattcgcacatgcccccgcgcaccgccggcgtaggccgccatgtcgcgctcgatgcgctgggcgctgccgagcatcgcgcgcgcatgttccagcagcgtttcgccggcgggggtcggcaccacgccgcgccgcttgcgtagcagcagcggcgtgcccaccgtgtcctccagctgcgccaggcgcttgctgatggccgagccgacgatgctggcctgctcgcccgcgcgcgcgatgctgcgcgtttcgcagacggagacgaagaggcggagggtggtcaggtcgaggtcgcgcatgggggttccgattgagcgatgtgatattccattttggaacgaatctgcttccaaaatctattttctgaatcgaataggaacttctaacatcgatgccagaccttcaaaggagacaccttgaacgaagccacggttgcgcccgcagcgcacgcctttctgccgccccgcgcggtcgtccgcgaagtggggttgcgcgacggcctgcagagcatcgcgagaacattgcccaccgcgcaaaaactcgaatggattcgcgatgcgcatgccgccggccagcgcgagatcgaagtcggctccttcgtgcccgcgcgcctgctgccgcaactggccgacacggccgagctgctggcgtacgccaagacgctgccggggctttttgcctcggtgctggtgcccaacctgcggggcgcggaactcgccattgcgggcgaggccgatctcatgatggtcccgctctcggccagccatgcgcacagccttgccaacctgcgcaagacgcccgacgaagtggtggccgaggtcgcgcgcatccgcgccgcgcgcgatgccgcgggctccaagacgctgatcgaaggcggtgtgggcaccgcgttcggttgcaccatccagggccacgtggagatcagcgaggtactgcggctgatgcaggcgctgctcgacgccggcgccgaccgcgtgggcctggccgacaccgtcggctatgccgatcccgcgatggtccgcagcctgttcgagcgtgcaaaacgcatcgccggcgaccgcgtgtggtgcggccatttccacgacacccggggccttgggctcgcgaacacctacgcggcgctcgaagtcggcatcgcgcgcttcgatgcctgcctggccggcatcggcggctgcccgcatgcgcccggcgccagcggcaatgtcgacaccgaagacctcgtgttcatgctcgagagcatgggcgttggcacgggtgtcgacctgccgaaactgctcgacctgcgcaagcgcgtggccggctggctggagggcgagacactgcagggcaccgtgtggcgcgcgggttttccgaagaccttcgtggcgacggcgggtgcagcggcatgagcgcgaacaccgaagaaaaacgcctgccgctcaccggcatccgcgtggtcgagttcacgcacatggtcatgggcccgacctgtggcatggtgctggccgacctgggcgcagaggtcatcaaggtcgagccgatcgacggcgaccgcacgcggcacctgctgggcgcgggtgccggtttcttccccatgttcaaccgcaacaagaagagcatcgcgctcgacctgcgccacccgcaggggctcgaagcggcgatgcgcctgtgcgccacggccgacgtggtggcacagaatttcaggcccggcaccatggagaagtacgggctcagccatgccgcgctcagcaagctcaatccgcgcctggtgtacgtgaaccacaccggcttcctgcccggcccctacgagcatcgcaccgcgctcgacgaggtggtgcagatgatgggcggcctggcctacatgaccggccgtcccggcgatccgctgcgcgcgggcactagcgtgaatgacatcatgggcggcatgttcggcgccattggcgccatggccgcgctgatgcagcgcgcgcagaccggcaagggacaggaagtgcagtcctcgctgttcgagaacaacgtgttcctggtcggccagcacatgctgcagtacgccatcaccggccaagccgcggcgccgatgcccgagcgcatctcggcctgggcgctgtacgacgtgttcacggtaaaggatggcgagcagatattcctggccgcggtgagcgatgcgcaatggacggtgttctgcgatgagctcggcttcgacgacctgaaggccgaccccaccttgcgcaccaacaacgacagggtccgcgtgcggcccacgctgctggcggacttgcgcaagcggctggccgaccggtcggctgccgagctgtcggcgatcttcgaggcgcgtggactgccattcgcgcccatcgtgcggcccgaagacctctacgaggatccgcacctgaaagcgaccgggggtctcgccgacatccgcctgcccgatggcgaacgcgccgggcagacggcgcagaccacgctgttcccgatcacgttgggcggccagcggctgggcgtgcgcctggacccgccgacactgggcgagcacacgcgcgaactgctcgccgagctcggctatgcggagtcgcagatggtggcgatgcaggccgaatctgccgttgcctgaacgcatttttcgaagacatacaaagagagacaagaccatgcacaagattcttcccccgatgacccgccgcgccgtactgggcttcggcgcctccgccgcggcgcttgccgcatgcccggtgctcgcgcagggctccgacaagcccattcgcttcatcctgccgatcagcgccggctcgggcgtggacgccatcgtgcgcgcggcctcggttgcgctcggcaaggccttcggccagccggtggtgatcgagaacctcccgggcgcgggcggcatcaccggcacgtcggcgctcgtcaaggcggcgcccgacgggctcacgctgggcgtggtgtcgaacaaccacgtcatcaacccggcggtgtacaagaagatgcccttcgacgccatcgccgacgtgacgccgatcagcgtggtgggcgcgacgccgctggtgctggtggtcaatccgaagctgcccgccaagaacgtgaaggaactggtggcgctgctgcgcgccaagcccgagggctacaactacgcctcgtcgggcaacggcaccatcattcacctggcgggcgaaatgttcatggacgaggccggcgtgaaggcgcggcacatcccttacaagggcacgggcccgatggtcaccgacatgatcgcaggccaggtcgagatgggggtggtggcgttgcccgcggtgcagccgcacctcaagagcggcgcgctgcgcgccatcggcctgtgcggccccacacgctcgccggccgcgcccgacattccgaccatcgccgagcaagggctgcccaactacgcggtcgaaggctggttcgcggtgatcgggccgccgaagatgcaggccgccgacatccagcgcgtgcacgacgcggtggccgctgccttcacgagcgccgaggtgcgcgaggccatggacaagcagggcaacatcatcaagcccacgtcacccgagcaggcggcgagctatttccgcaccgaagccgcgcgctatgcggcgctggtgaagaaggcgaacgtcgtgctggagtgagtgccgggctcaggcctggctcgtgaacttgagcccgaggatgcccgcgatgatcaggcccacgcagatcagccgcgccgcattcgagggctcctggaacaacacgatgccgagcaccacggtgcctacggcgccgatgccggtccacaccgcgtaagccgtgcccaccggcagcgtgcgcatcgcccagccaagcagcacgacgctgagcaccatcgagatggccgtgccgaccgagggccagagcttggtaaatccttcggtgtacttgaggccgatggcccagcccatttcgagcaggcccgccaccaacaaaacgacccacgccatgcgcgctccttgaaaaggttttcagttctccggccgcacggcacggtaaagggcgcgcacgaaatccgactgcgtgatcatgcccgtgagccgcttttcatggtcgatgatggggatatggtggtggccgccttcggagaacagcggcaccaggtcgatcaccggccggtcggcgctggccacgcgcacctggcgcgtcatgatctggccgaccacctccggcttgttcgagacgacggtgcgcgtggcgcggatcaggtcgcgcagcttgcctgcaatgccttcgtggtgctccaggtcgagcaggcggaagaagtcggcctgcgtcacgatgccgaccacgcggcgcgtgcggtcggtgaccggcagcgccttgatgcggcgctgggtcatcagcatccaggcctcttgcagcggcgtgccgaactccaccgacaccgggtcgcgcgacatgatgtcgccgcaatgcagcgtgccgagccgccgcttgtacgactcgagttcggtctgctggatcagcgactcgaggtcgtcgcggctgatgtccagcacctggttgtagcgcgccagcaccgcgtcgatgtcggcctggctgaaacgggcgtcggccgatggcggccgcgccacctgcacgtgcggatagcgcctgcccgtgaaggtgttgtaggccacgcccgccagcaccagcaagagcgaattcgccaaggtggggaacagcgccgccgagaagtggtcggtgtgcgtgagcacggcgagcagcgccgcggccccgcccggtggatgcaggctgcgcgtggcgaacatcagtccgatggccgcgcccacggcgattgccgcggcccaggccggatcgggtatccagcggacgcaggcgatgcccaccacggtcgacagggtgttgccgacgatgaccgaccagggctgcgccagcgggctcgcgggcacggcaaacaccagcaccgcgctggcgcccatcggtgcgatgagccagatgctgacgtccaccgcttcggccatccagcggcacagcagcgcggtgatcagaagcccgatggccgcgccggccacggcacgcaggcgctcgcgcgcatcgacggtgttgcggcccggcagccaggcgcgcgcatgcgtcaacaaagcggaaagctgcggcacggcttcaggcctccgcggccacccggcggccgatctcgggccattgcccgtgcagccagacccaggcgacaaggccgatgcccagcatcagcgtggaggtgagcgccagtgccagtgtggagtgcatgaccagcggcgccaccacgcccgccacgatgccgttggcggtggagccgatcacggcctgcagcgacgaggccatgccgcgtcgctcgggatggaggtcgagcaccagcagggtcaccacgggcaccatcagtgcccagccgaacgcgaacaccgccagcggccacagcgcccaggcgacgtgcgcggtgaagagcgaattggccaccacgttcaccagcgaggtcaccagcatgatcaggaagccgtcgcggatctgccgtttgggcgccaccttgcccgccatgcggccgctggcccatgcgcccaacatgatgccgccgatggtcagcaggaagaaccagaagaactgagtcggggccaacgccaggtggtcgccgaggaaggcgggcgcggccagcacgtagaggaacatgccgttgaacgggacgccgctcgcgaacgcgagcagcagaaagcgcgggtcggagcagaggtcccagtagccgcgcatcaggtgccgcacctggaaaggctggcgctggctctggtgcagcgtttcgggcagcagcttgtagttggccacgaacaggatcacgccgaccgcgaccaggaaccagaagatcgcgtgccatccggcatgcacgaaaagaaagccgccaacgatgggcgcgatggccggcgcaacgccgaagtagatggtcacctggctcatcacgcgctgcgcatcggcgggcgggaacatgtcgcggatcacggcgcgtgaaaccacgatgcccgcaccggtcgacaggccctgcagcccgcggaacagcaccagctgcgcaatgttctgcgacagcgcgcagcccagcgaggccagcgtgaacaccgcgagtccccacagcaccacgggccggcggccgaagctgtccgacagcgcgccgtggaacaggttcatgaacgcaaagccgaacaggtaggccgaaagtgtctgctgcatttcggccggcgtggcgccgatggagcgcgcaatgcccgagaaggccggaatgtaggtgtcgatggaaaagggaccgagcatgcccagcacggcgagcagcacggcaagcgcccatcgcggggcttgccagagcttgtctgcatcgggattcatgggatttgctccatttttcttgtcggtagaggccaaaaaagaaagcgcccttgcgggcgcctcctcgtcagagagaaataccggagaccggtcagagcgtatcaataaagctgcgcagtttgtcggaacggctcgggtgcttgagcttgcgcagtgcctttgcctcgatctggcggatgcgctcgcgggtcacgtcgaactgcttgccgacttcttccagcgtgtggtccgtgctcatctcgatgccgaagcgcatgcgcagcaccttggcttcgcgcggcgtgaggctgtcgagaatgtccttgaccacgtcgcgcaggcccgcctgcattgcggcttcgatgggcgccgtgttgctgctgtcctcgatgaagtcgcccaggtgcgaatcgtcgtcgtcgccgatgggggtttccatcgagatcggctctttcgcgatcttcatgatcttgcggatcttgtcttccgggatctccatcttggcggccaggatgccggcgtcgggctcgaagccgaactcctgcagatgctggcgcgagatgcggttcatcttgttgatcgtctcgatcatgtgcaccgggatgcggatggtgcgcgcctggtcggcgatcgaccgggtgatggcctggcggatccaccacgtggcgtaggtcgagaacttgtagccgcggcggtattcgaacttgtcgaccgccttcatgaggccgatgttgccttcctggatcaggtccaggaactgcaggccgcggttggtgtacttcttggcgatggagatcacgaggcgcaggttggcctcgatcatttccttcttggcatcgcgcgaggacgattcgccctcgttcatgcgcttgttgatttccttcagctgcgtgagcggcaccaccacgcgcgactggatgtcggtgagcttctgctgcagttcctgcaccggcggaatgttgcgcgcgagcacggcgctccagggcttgccggcggcggcctgcttctcgacccatttcaggttcagcaggttcgacgcgacgcggttgccgctcttgtcgtagccagagaagtcgcgaatgaactcgtcctgcgggaagccgcacttgtccacgatgatgcggcgcagctcgcgttccttcttgcgcacgtcgtcgacctgcgtgcgaaccaggtcgcacagcttctcgatggtcttggccgtgaagcggatggtcatgagctcgtccgacagggcctgctgggccttctggtaggccggcgtgccgtagccttccttgtcgtagatcttgtggaccttctcgaacatcccggcgatgcggtcgaaacgctcgagcgcgtcgcgcttgagttcctcgagcttcttggtgagggccttggagccgcccttgccgtcgtcgtcgtcttcttcgtcgaactcgtcgaagtcttcctcggccacgtagtcgtcggcctcgttggggttcgagaagccgtccaccacggtggagatgacgaccttgccttcacggatgtcggcggccaggcgcaggatttcggcgatggtggcgggggaggccgagatggcttccatcatggccatcaggccgccttcgatgcgcttggcgatttcgatttcgccttcgcgcgtcaggagctcgaccgtacccatttcgcgcatgtacatgcgcaccgggtcggtcgtgcggccgaattcgctgtccacggtggacagagccgcttcagcttcttcctcggcttcttcgaccgtggtggcggtgggcgcggtgttgttcagcagcagggtttcggcgtcgggcgtctgctcgtacaccgccacacccatgtcgttgagcatggtgaccacgacttccatggtctcggcgtcgaccagcttgtcgggcaggtggtcggagatttcgccgtgcgtgaggtagccgcgggtcttgcccagcgtgatcagggtcttcaggcgcgagcggcgcttggccaggtcttcctcggagagcacggtctcgtcgaggccgaattccttcatcaaggcgcgttccttcgccttgctgatcttcatgcgcagcggcttgaccttttcttcggtggtcgaggcaactgccggttcgtcgccggccaggtcgtcctcgatgtccgacaggtcgacgtcgctttcaggcgcttcgttgccggccttgggcttgcggccgcgcttggcgccagtggcgggcgcagcggcgccggcggccttgggcgggcggcctactttcttggcggcaggggcagccgtcttggcggcggcttttttcggatcgtcgatggaggtcgatttcgtgggcacggttttcactttcgttgcggctgccgatttggacgcggcggcacccgacttagttgccggcatagcgccggctttcaacggtttttctgcgacaggctttggggtggcgcctttggcgagtgaaggagcaggcttctttgaactgggcatacgacctcgttacagcaagatggaccaagcgaaatcacaggcgcaccgccacataggcagcgccaccacagcccgtgcacaggcacgggccaagactcaaagcccgcgcacaggcacggacaaaacaattgggaaagaggaagaaattcctcgtcaggcaagatgtcgggcgaacatttggtgtgcagtccttgcggtaagtgaccctttccgtcggattttttccgttggagtgcgttgcgctaggggtcggcccggaggtgctgctgtcgctcttgcctaatttcgccagttgcgaagccttacattatagcctactgcgcaaatttcaagcagttttatgcccctgacggcttgaggcgggcgcgcaattcgagtcttctcgcctccagcgccttgtagcgttccagggccttggggtccgagcccacggcggctatggcctcgctctgctgggctttcaggcggtcgtcgagcatgaagtcgagcacgctcgaaagctccttggcggcgtcggccaggtgctgctcttcctcgccttcagcgggcggggcgttctccgaaacggccatgagccgctccgcgagcgcttcgaagtcgagcccgcgcatgccttcgcgcaacgccgcccagggctgcacgccatgctcgtgcaactggctgtcgagccaggtgaaaagcgcaccgtgcgggccgggcaggtcgcacagcatcacgtgcaattcgtgcgacagcgcgtcccactgcgccatgttcgacagcaggagccgcaccgccacgtcgggccggctcggcggcttgccgcgcccgcgcagcggctcgatcggcgcctcgaacttgccgccccaccgcttgcccttggtaaatttgccccgcggcttgctatcgttttcgtagcgaggcggttcgtattccgagggcggcggcatgtcggagtagtcgaatgggtcgcccggctcattgccatggcgcggcactggcgccgccgccgccttgcgcgggccgggcgtggcggcccagagctccgacaaggcggccgcatcgagctgcaccagcgtggcgatctcgctcagcaactgccgcttgagcgcgccatcgggcatggcgctccagagcggccgggcgttgctgctcatgtgggcgcggccttcggcggcggtgaggtcgcagccttcgcgcgcggcctcgatcatgaagcgcgagagcggcgtggcttcctgcacgaagcgggcgaaggcgtcggcgccgaattcgcggatgaagctgtcggggtcgtgctcggccggcaggaacaaaaacttgatgctgcgcacgtcggtggcgtagggcagggcgccatcgagcgccttgcgcgcggcgcggcggccggccgcatcgccgtcgaagctgaaaaccaccgactcggtgaagcggaagagcttttgcacatgctcggtggtgcaggccgtgcccagggtggccaccgcgttcggaaacccgagctgcgccagcgccaccacgtccatgtagccctcggtcaccagcgcgtagccgcgctcgcggaaggcggcgcgcgcctcgtacaggccgtagagctcccggcccttgctgaacaccggcgtttcgggcgagttcaggtacttgggcttttcgtcgccgagcacccggccgccgaagccgatgcattcgcccttcacgttgcggatggggaacatcacgcggtcgcggaagcggtcgtagcgcttggcgtcttcggtgccgtcctcggtgttgacgatcaccagcccgctttcggcgagcagggggtcgtcgtaatcgggaaacacgctggccagggtgcgccagcccgcgggcgcatagccgatgccgaactgcttggccacctcgccggagacaccccggcccttcaggtattcgatggcgcccggcgcctgccgcaaggccttgcggtaagcgtctccggctttttcgagcacgtcggtcagcgtggcctgcttctggcgctggttcgcggcgcgtgcgcgttcggcgggggaggcgtcgtcttcgggcacctgcaggccgtattggccggccaggtcgtgcacagcctcgacaaaacccatgccggcgtgctccatgagaaagccgatggcgttgccgtgcaccccgcagccgaagcagtgatagaactgcttggtcgggctgaccgagaaagagggcgatttttcgccatggaacgggcacagccccatgaagttggcgccagccttcttgagctgcacgtagcgcccgacgatctccaccacatcggcgcgtgcgatgagttcctggatgaaagaggcggggatggtcatgtaggcgaagagcggcaaatcatacgcaagcggccgaacgcccgcgcgcgggcgccatactcggaatgatccggagtccacggatgacgacgcccaaaccattgcaccacgccgcaccgctgttgctgcgccatcccttgaattttgtctgggatgcgctcaaggccttccgcgccaaccagggcctgctgctcgcgggggcggtggcctactacgccttgctctccatcgtgccgctcctgatcgtgagcgtcattgcgatgtctcacctgatcgaacaggccgaactgctgcgcaccatcggccggtacctcgaatggctgctgccggggcagtcgagggcgattgtgaaggagctgtcgaactttctcgaccatcgcgacgtgatgggcccggtgctggtggtgacgatgattttcttcagctcgctggccttcagcgtgctcgaaagcgccatggcggtgatctttcaccaccgcaaggcggaccacaagcgccatttcctggtttcggccgtcatgccgtacctgtacatcctcttcctgtgcgtgggcctggtgctgatgacgctggtatcgggcgcgctgcagctggtcgggcaggaaagcgtcgacctgttcgggcgcgactggtcgctctcgggtgtgtcggggatgctgctctacctgctggggctgggcggcgagatcttcatgctgacctcgctctacctcgtgatgccggccggccgcatgtcgctgcgccacgcgctgctcggcggcgtgacggccgcgttgctgtgggagggcacgcggcatgtgctgatctggtatttctcgacgctttcgcaggtcaacgtggtctacggctcgctcaccacggccatcgtggtgctgctgagcctggagattgccgcgacgctcgtgctgctgggcgctcaggtcatcgcccagtacgagcgactggaccgcaccggcagcacggcggtcccgccgatcaccggggcggaagtcgaatcgctccgtcgagacgaatcacctccccgttgagcatgtcgttctcgatgatgtgcttcgcgagcctggcgtagtcctcgggtgtgcccaggcgggaggggaagggcacgctggcggccagcgcgtcctgcacttcctgcggcatgccgaagagcatgggggtgccgaagatgccgggcgcgatggtcatgttgcggatgccgttgcgtgccaggtcgcgcgcgatgggcagcgtcatgccgaccacgccgcccttcgaggcgctgtaggccgcctggccgatctggccatcgtaggctgcgaccgaggcggtcgagatcagcacgccgcgctcgcccgtggcttcgggctcgttgccgctcatggcctcggccgcgaggcggatcatgttgaagctgccgatcaggttgaccgtgacggtcttgctgaacaccgccagcgcgtgcgcgccgttcttgcccacggtcttctcggccggcgcgatgcctgcgcagttgaccaggcccaccagcttgccgagcttctgtgccgcggcaaccacggcctggccgtcggcctcctggctcacgtcgcacttgacgaacacgccgccgatgtcgctcgcgacggcttcgcccttgtcagcctgcatgtcggcgatgaccaccttgccgccgttcgcagccagcatgcgcgccgtgccttcgccgaggcccgaagcgccaccggtcacgataaaaaccttgccgtcgatctgcatagaaagtctcctgaaataagacccgcattatcgaaggcaggtgcgcgcagcctgggggtgagcaaaagtgctcgaaaaaaaaggcctcatccgaagatgaggccctgaattggatccgtgaggacccaaggagacaactggtgtagccggcggcttagcgcttgcgcgaagcggttgcggtcttggcggcggcaacggcttgcgtcgacacggcgttgaagttggcttcggcgacgtcggaagcctgcttgacagccttctggaccgattcgaaagcgttgttggcggcagccacggcgctcttcagcacggcaacggcggtttccgagccggcgggtgcattcttggaagcgctgtcgaccaggccgacgaaggtttgctgggcttcagcagccttggtttcgaaagccttggtgaattcggcgccggtgccttgggcgatgtcatacaggtgacggctgtaggcggcggtcttttcggccaggggctggaacaggctggcttgcagcgtcagcagttcttgtgcgtccttgacgttcagggcggcttgggcggtaccggcggcttcgaccagggcagccttggaagcggtgacgttcagctcgacgagcttctccacgccttcgaaagccttggtggtcaggccgaacagggtttcgaggtttgctttttgggcggcgaggatttggtcagcggtcagggccatttgagaatctccagaaagggatgggtggtcggttcacgattgcgctgcccctcgtcgtctatgttgcggtgcagcatggcctcaagtataggcagcacagctttgcgatcaagggggttttgctgctttgcagcaatttagaacacactttctaaattcgccccgggctccagaatgcaggcatgcgcgccttctattccggccagttcgtgttgcccttgcccccgggccaccgctttcccatgtcccgctacgcgctgctgcgcgaccgcctgctggagcacctgccgttggtggagatggaccaggcgccccgcgccactgatggcgagctggcgctggcgcacaccccgcagtggatcgccgccatcagcgacggcagcgtgaccacacacgccatgcgggagatcggctttccctggagcgaggcgatggtcgagcgatcgcgccgttccactggcgcgaccattgccgcctgccgcgccgcgtttgccggcggggtggcggccaacatggcgggcggcacccaccatgcccatgccgacaagggcgggggattctgtgtcttcaacgacgctgcggtggccgcgcggctgatgcaggcggagcatggccgcagcgggcggcaactgcgggtggccgtggtcgacctcgatgtgcaccaaggcaacggcacggccagcatcttccgcaacgaccccagcgttttcacgctctcgttgcatgggcagaagaactttcctttccgcaaggaggcgagcgacctcgacgtcgagctgcccgacggctgcggcgatgccgagtacctcaccgcgctcgaacacgcgctcgacgaactcgatcggcgcttctcgcccgggctggtgatctacctggcaggcgccgaccccttcgagcgcgaccggctcggccggctcaagctgagcttcgacggcctggaggcgcgcgaccggcgggtgttcgactgggcctggcagcgccgcattccgctggccttcgccatggccggaggctacgccagcgacattgcggagacggtgcaggtgcaagtcggcaccttcagggtggccttcgactactggcgccgctggcaaaatgccgcgcgatgagctccgccaacaaacccacgccgcacacccgagccggctaccgcgcgtttcgcagcatccccacgcgctgggccgacaacgacatgtacggccacgtcaacaacgtcgtctactacagctggttcgatacggccgtgaacgcgctgctgatcgagcgcggcgcgctcgacatccaccaggggcagacgatcggcttcgtggtcgagacgcagtgcaactatttcgccccgatcgcctttccagagacagtggaagcgggcatccgggtggcccaggccgggcgctcgagcgtgcgctacgagatcgcgctctttgcggagggcgcggaaaccgcggccgcacaaggccacttcgtgcacgtgtacgtggacagggccacgcagcggccggtgccattgcccgaggcgctgcaacgcgtggtcgacgcgctgaaagcctgatcccaaagcaaacggcgcccggggagggcgccgtttcttgagtcacgcggcccgctctcgggccgcggcggcttacatggtcttcttcttggccttgatatcggccttggcctgggcttcgtcggccttggcctgcttcacgcaggcggccttggcatcgccggcctggtcgtcgcacttttccttggcaacctcataggtggccttcgccttctcttcagccaccttgcgcgcatgcgcgtcgctcggcttgtactgctgttcgagttcggccttcgccacgtcttccttgcccttggcttccttctggcagacgtcctttgcgttgtccttcatcgcgtcgcactgggccttgtcggccttgtagtcggcttcgatcttttccttggcgaccttgtactcgtccttggtcatcgcgccggcctgggtggccatgaagcaggtagaggccagagcgagcatgagcagatgttttttcattggagttctttcttagaggttgagaagagttgaatgaggaggattgggagggcaggggccgcccttcggccgccccgcgtgctcagtacttttcgtaccagagggtttccggcgtgcggccgtcgcggttctcccagtccttgacctgtttttcggcctcgtcgcggctgatgccgtgacgctcctggatgcggccgagcagctggtcgcgcttgcccgcgatcacgtcgaagtcatcgtcggtcaatttgccccattgctccttgaccttgcccttgagctgtttccagttgccttcgatggtgtccttgttcatgcgaatctccttgaaaggttgattcggcgagcccatggccgccgtgaaaacactgtcgcggggcctattcaccctgacggtaggacgcccagtgttggcgccgtaggcacaagccgacgctgcccgtgataatcggtcgcacgccgaaaaagcccgggacaaacgcgcgccgtaccagcaccatgatcattcacagcctgctcgacacagacctctacaagttcaccatgatgcaggtcgtactgcatcacttcccgggagcccaggtcgagtaccggttcaagtgccgcaacccgggcatcgacctcgcgcagttcgcgggacagatccgcgaagaggtgcgaagcctctgttcgctccagttccgggacgccgagctgacttacctgcgttcgatgcgcttcatcaagagcgacttcgtcgacttcctgggcctgttccggctcaacgagaagtacatcagcatcacgccccagccctcgggcgaactcgagatccgcatcaagggcccgtggctgcacaccatcctgttcgagatcccggtgctggcgatcgtgaacgaggtctactttcgcaacacgcagaaaaagcccgatatcgaagaaggccggcggcgcctggaaaccaagatcgggcagctgcaggacgccggcctggccgatctcaagatcgccgactacggcacccgccgccgcttctccaaggactggcacgaagagattcttcgtacattgaacgcaaggctcggcgccgtcacctcgccgccggtgcaggcccctcccggcgcgcggctgccccagctcgcgggcaccagcaacgtgctctatgccatgaagctcggcctcattccgctcggcaccatggcgcacgaatatttgcaggcctgccaggggctcggcccgcggctgcgcgacagccagatcttcggcttcgagagctgggcccgcgaataccgcggcgacctcggcattgcgctgtccgacgtctatggcatgagcgccttcctgcgcgacttcgacctttacttctgcaagctgttcgacggcgcgcggcatgacagcggcgatccgttccagtggggcgagcgcatgctggcccactacattgccaaccgggtcgatccgcgcaccaagacgctgatcttcagcgacagcctcacggtgccgcgcaccgtcgagctctaccagcagttccgcggccgctgccagctggcgttcggcatcggcaccaacctcaccaacgacctcggctacgagccgctgcagatcgtcatcaagatgatcacctgcaacggccagccggtggccaagctgtcggacaccccgtccaagaacatgtgcgaggacgaaaaatacctggcgtatctgcgccaggtgttcgagatcgagcagccgcccgcctgatgcccgtctggtacggtacgggcccaatgaaaaaagcagttcgcctggcggcagccgcggtgctgccaatgctgtttcccgcgctggccatggccgccgacctcgacggcagccagctgtcggcgctctggggcgttccgttcgcaggcatcctgctgtcgatcgcgctcatgccgctgctcgccccttcggtctggcatcaccactacggcaagatttcggctgcctgggcgttggcgttcctgcttccctttgccgcgatccatggggcgcccctggccggatcccggctggtgcatgcgctggtcgaggaatacatccccttcatcatcctgctcaccgcgctgttcacggtggccgggggcatccacattcgcggcaacctgcatggcgcgcccggcctcaacacggccatcctggccatcggagcggtgcttgccagcctcatgggaaccacgggcgcctcgatgctgctgatccggccgctgatccgcgccaacgacaaccgcttgagcaaggcgcacgtggtggtgttcttcatcttcatcgtgtcgaatgcgggcggctcgctcacgccgctgggcgatccgccgctgttcctcggctttctgaagggcgtcgactttttctggacggcgcaaaacatcctgcctgaaacgctgtttctcgtcggcctgctgctcgcgctgttctacgtgatcgaccgccactactaccgcaaggagggcgtgctgccggtcgacccgacgccggacacccgccgcatcggcttcgacggcgccgccaatttctggctgctgggcggcgtggtcttcctggtgcttctctccggcatctggaaaacgcccgtgggcttcgacgtgttcggcacgcacgtcggcctgccggggctggtgcgcgacgtcggcctcatcgccatcacgctgctctcgttcaagaccacttcggccaaggtgcatgccgacaaccagttcgagtggggtccgatggccgaggtggccaagctgttcgcgggcatcttcctgaccatcatcccggtgatcgccatgctcaaggccggcgcgaacgggccgtttgcggcggtgattgcggcggtgacaaagcccgacggccagcctgatccggccatgtatttctgggcttcaggcatcctgagctcgtttctcgacaacgcgcccacctacctggtgttcttcaacaccgcgggcggcgatgcggccacgctcatgaccacctacgccaccacgctggccgccatttctgccggctcggtattcatgggcgccaacagctacatcggcaacgcgcccaacctcatggtcaaggccatcgccgagagccgaggcgtgcgcatgccgagcttcttcggctacatgggctggtccgtggccgtcctgattccgctgttcgttctttccaccttcatcttcttccgttgagtgcaaacatcatgagcaagccaaagatcctgatcgcgcgtgcgatctttcccgaaaccatcgagcgcctctcgcagcacttcgaggtcgagtcgaaccagtccgacgagagctggagcaaggagcaattgatcgccaggctcaagggcaagcagggcgccttcaccaccggcagcgagcgcatcgacgccgcggtgctcgacgcctgccccgacctgaagatctgcgccaacatggcggtgggctacaacaacttcgacgtcgatgcgatggctgcgcacggcgtgctcggcaccaacgcgcccgacgtgctcaccgaaaccacggccgacttcggctttgcattgttgatggccacggcccggcgcatcaccgaaagcgaacatttcctgcgcgcgggcaagtggcaaaaatggagcttcgacatgttcgcgggctccgacatccacggctcgacgctcggcatcatcggcatgggccgtatcgggcagggcattgccaagcgcggcgcgtacggcttcggcatgaaggtggtctatcacaaccgctcgcgcctcgacgccgcgctcgaggccgaaagcaaggccagctacgtcggcaaggaagagctcctcaagaccgccgaccacgtggtgctggtggtgccgtattcgccggcctcgcatcacaccatcggcgcggccgagatcgcgctgatgaagccgaccgccacgctcgtgaacatcgcgcgcggcggcatcgtcgacgacgcggcgctggccgtggccctgcgcgaaaagcgcattgcggcggcgggactcgacgtgttcgagggcgagcccaaggtccaccccgacctgctgaccgtgccgaacgtggtgctcacgccgcacatcgccagcgccaccgtgcccacgcgccgcgccatggccgagctcgcagccgacaacctcattgcctggttcggcggcaagggagcgctgacgcccgtcacgcccgttccgccagccggcaagtaacgaaccggcgagcagcgacgcggcgatccgaccttggaacttcccgacttgattcttcttttgctggctgcgctcgccgtcgtccagcttgccctgctgatctggctgctcgcgcgccggcaaccccggcccgaccatggcgaggtgctgtcggtgctggccgccatgggcgccgccaacgaacgcaccgagcgcgaactgcgccatgaaattggcgaaagctcgcgtggcgcgcggcaggaaaccgggcaggccttcgccactttccagcaggcgctggtgcagcagggcgcggaggccacgcgcacgcagaatgcccagctcgacgctttctcgctgcagctcgcctccctgcagaagaccctcgccgacacgctcaacacccagctgcagggcctgagcgagtcgaacgcgcgccgcctggccgaagtgcgcacgaccatggaaacgcagctcgcgcagctgcagcagagcaacaccgccaagctcgacgagatgcgcaagaccgtcgacgagaagctgcagagcacgctcgaagcccgcttgggcgagagcttcaagcaggtggccgaccggctcgagcaggtgcacaagggcctgggcgaaatgcagaccctggcggtgggggtcggcagcctgcagcgcgtgctgaccaacgtgaagacgcgcggcgtgttcggcgaagtgcagctcgaggcgctgctcgagcaggtgctcacgcccgaccagtacgccaagcaggtcgagaccaagccgcgcagcggccagcgcgtcgactttgccatccgcttcccgggacggggcggtgacggtgccccggtgtggctgcccatcgatgccaagtttccgcgcgacgactatgaacgcctgatcgatgcgcacgagcgcgccgacgccgtcggggccgagcttgcggccaaggcgctcgaagcgcgcgtgcgcagcgaggccaggtcgattgccgagaactacctggccgcgccgcacaccacggatttcgccatcctgttcctgcccgttgaaagcctctacgccgaagtgctgcggcggccaggcctgatggacgccatccagcgccagcaccgcgtcacgctggccggaccgaccaccttgcttgccatgctcaacagcctgcacatgggctttcgcacgctcgcgctggagcatcaggcgtccgaggtctggaaggtgctgggcgcggtcaagaccgagttcgagcgctatggcgaatgggtttcgcgcatcaaggagcaggtggccaaggcctccgacacgctcgacaaggccgacacgcgcgccaagcagatgcgcctggcgctgcgcaaggtcgaggcgctgcccgaggcgcagtcgcaggcgctgttgccttccacggccgacaccgcggacagcgagggcgacgacaccccgtgaaaggctccgaactgctgcgcgtcatcggcgcccaggtctgcttgcacgccaccatggccggcatgcggctcgcaacaccgctgctggcactgcaacagggatacagcgcggcggccgtgggcgtgttgattgcgctctttgcgctcacgcaggtgttcctggccctgccggcaggtcgctttaccgaccgctacggcttcaagcggccgctgtggctttcggtcatcgcggcttcggccggtgcgggtctcgcgctcgtcttcccgacattcccagtcatgtgcattgcggcgctgctcaccggtggtgccaccggcgcgaccgtgatcgcgctgcagcgccacgtgggccgctccgccaccaacgccgtgcagctcaagcgcgtgttcagctggctggccattgcgcccgccgtcgccaactttgtcgggccgttcctcgccggcctcttgatcgaccatgccgggcgcgcgccggccgacatgctggccttccgggtctgctttgcggtgatggcggtcttgcccttcatctgctggctgcttgcgcgcggcgcgcacgagccgccgcccaccctgcctgtcgcaggcgctgcgcctacccgggcctgggacctgctgcgcgagccgatgttccgccgcctgctgttcgtgaactggctgcagtcgtcgagctgggacgtgcatgccttcgtgctgccggtgctggggcacgaccgtggcatcagcgcctcggtcatcggctccattcttggcgctttcgccatcgccgcagcggccatccgggtggtgctgcccctgatcgcgtcgcgcgcctcggagcgcagcgtgatcctgatctccaccatcgtcacggccgcggtgtttgcggtctacccgctgctggactcggcctggaccatgggcctgtgctccgtggtgctgggattcgcgctcggggcggttcagccgatggtgatgagcatgctgcaccagatcacgccgcatgcacgccacggcgaggcactgggcctgcggctcatgaccatcaatgcctccagcgtggcgatgccgatgctgttcggatcgatcggtgcgctgatcggcatcgcgggcgttttctgggtggtgggcggtgtcatcgcgctgggcgcgcgggccacctggggtttgaaggcgcccttatagcttgtagaagcgcttgatcgcgtcccaggcgtcgtccgccgcatcgacgtattcgaagagcttcacgtcggccggcgagatcacgccttcttcgaccaggaagtcgaagtcgatcagcttcttccagtaggccgagccgaacagcacgatcggcaccggcttggacttcctggtctgcaccagcgtgatcacctcgaacagctcgtcgagcgtgccaaagccgcccggaaacgccaccagcgccttcgcacgcatcatgaaatgcatcttgcggatggcgaagtagtggaacttgaagctcagcgccggcgtgacgtaggggttggcttcttcctccatgggcagcgcgatggccaggccgaccgagattccgccgccttcgtgcgcgccgcggttggccgcctgcatgatgccggggccgccgccggtgcagacgaaaagcttgtcctcgggttccttgtcgctgctgtactgcgcaaccagcttgccgaaggcgcgcgctttctcgtagtaatgcgagctgcgcgccaggcgccgccagcgctcggccgccacggcgtctccggcggcatcagcctgtgcgaccagcgcggctgcatcttcctcgctgcgaaagcgcgcgctgccgaagaccaccacagtgttctcgatgccgtgggcgcgctgctccaggtcgggcttcatgagctccagctgcatgcggatgccgcgggtttcccggcgcagcaggaattccgggtcggcaaaggcgaggcgcgaaggatcgaggtcgagcgggaggcctttttcggagtgcgccttgagggtggcccaggcgtcggccaggcgtttgtcgtgaaggttgtgcgtgttgttcatggggaatcagacagaaagactcgctgcattgtgcagcgttgcggccgacatgcccggcggctcaaaaagcgccgtgccggccggcgccgcgaacgaagcgctcggcgcccgccgcgccttcggcggcaaccatggggacgccgagccggccttcctgccgcagcgcatcggccagcggcaggttccattgggcgtagacggaatggcggtccgccagcatgcactgctgggggaacgacgcgatctcgcgcgcgagcgcttcggccgcatggcgggattggccgcggggcaccacgcggttgaccaggcccatcgcgctcgcctcccgggcgtccaccggtcggccggtcaggatgaggtcgagcgcgcggcccatgccgacgatgcgcggcagccgcaccgtgccgccgtcgatcagcggcacgccccagcgccggcagaacacgcccagcacggcgtcttcctcggccacgcgcaggtcggccagcagcgcgagttccagcccgccggccacggcgtggccgctgatggcggcgatcagcggcttcgcaagcgccatgcgggtcggccccatcggccccgagccgccgccttccgcatcgagttcgttgcgccgctccgggtcgctgacggcgcccaggtccgcgcccgcgcagaaagtgccgtgctcgccccacagcaccgcgacgcgctggctttcgtcggcctcgaagcgctcgaaggcatcgcgcagcgcatcggccatggggcgatcgaccgcgttgcgctgcctggggcggttcatgacgatggtgctgaccggcccatcgatctcggtgcggacgctggcggttttgttcatggacggaagggtaagcccatcaacgaaaaaaggctccttgcggagcctttttgccatgcgccggccagtcggccggaagcgctcagacgcgcttgcggtattcgcccgtgcgggtgtcgatttcgatcttgtcgccttgtgcaacgaagagcggcacgccgatttcgaaaccggtggcgatcttggcgggcttcatgaccttgcccgacgtgtcgcccttgacggccggctcggtccaggtgatttcgcgttcgacgctggtgggcagttcgaccgagatggccttgccgtcgtagaacaccacttcgacagccatgccgtcttcgaggtagttgagggcgtcgcccatgttctcggcttcgacttcgtactggttgtactcggtgtccatgcagacgtacatcgggtctgcgaagtaggagtaggtgcactccttcttgtcgagcacgatctggtcgatcttgtcgtcggccttgaagaccacttcggtgttgaagttggcgatcaggctcttgagcttcatgcgcacggtggcggaattgcggccgccacggctgtattcggtcttcaggacgaccatcgggtccttgccgtgcatgatgacgttgccggcgcggatttcttgagcgattttcatatcaggttctctggatgttggccgctcggtgcacggggccatcggcgacgtttgcaatgttgcggtgcaacggcttgccggcgttattggccccgcggtacatgtcccgcggcaggtttggcggacagcatctcggatctgtgtaaatccgggccgaaatccgcaaagcccactattttagctttttccggcgaccagatgccgcagttgcgtgaccaagtcctcttggaggcacagcttttcgcgggcagcccgcacggtttcacgccacgggcccccggtttcgagagcgggcaggggggcgtcgccaaagccgttccaggcgtggtggaactgccggagggacggcggggcgccgagccagtccagccaggcgccgagcttgacgtggtgcgcatcgtcgtcctgcgggtagatctgccagaccagcggggcgccggcccagagggcgcgcaccagcgaatcttctccgcgcacgaaattgaggtcgcaggtccacagaagatggtcgaagtccggctgcgtcaggtagggaaggtacgaaatcgacagcgcaccgaacccttgcggcgagcggcctgcaggctgcttcggactggcaaaaaaggcccccaccgcgtgcgccgcgcggccggacgtgaccaggagccgtgtaggttcggcgccggctgccaactgttcgagcaattgggctagctcggggggctcgtaacagaagagggaaacgaggcgctcgccgtcctgccacggaatttcgtgcgccgccagccattgcgcgcggtcgaaatgcgcttgccgttccaagaggccgggctcccgcagcagcccccccgtggcgggcgtgaagcccggatagaaaaagcgtttcgccagccccgcacccggtcccttgaagatcggcgaaggcaggccgtgcagccgctcgacatagggttccgccgacaggtattcgaggttgatccaggcccgggcgggcgcgccggcggtcggcggctcggcaaatcgcgcaatcagttcgggcgccggatcgcagccgaaggcttcgatcagcacgtcgggcggcggggccaccacggctttgcgaatggctgcagggtcgagccagtcgatcacgctcacgccgtcgcagcccgcgggcgccatccagtgcagcgccgtggcgtcgtcgatccacaggcgcacgcgctcgccgagggccgccagctggctggccagccgccagcacacgcccaggtcgccatggttgtcgatgaccctgcagaaaatgtcccattgcatggggcaagtgtgcccgccttcggcgggtcggggcagtgcggctgcttggtatgctggccggcaccacaacatcccggagcgagaaaccatgcgtatgaagagccgtcgccattcgccgttgtcccttggttcccttgttggctttgggcgggccagaaccgtgctcgcgctgtccctggccctgtgtggcctggccgcatcggcgcagacgacgccgtcgctgaccccccagcagcagcgcttccacggcatctacaaggagttgatcgagatcaacaccagccattcggtgggggacaacacgctggcggcgcgcgccatggaaaagcgcctggtcgaatcgggctttgcgcccggcgacatccaggtcttcgagccgttcccgaagaagggcaacctggtgctgcgcttcaagggcaacggcagcaagaaaccgctcttgttgctggcccacatcgacgtggtcgaggccaggcgcgaagactggaagtccgatccgttcaagctgcaggaaaccggcggctacttcacggctcgcggcgccatcgacgacaaggccatggcctcggccctggtctcggtgctggggcagctcaagcaggaaggcttcaagccgagccgcgacatcatcctggccctgacggccgacgaggagcgcggcgacgcgctcagcaacggcgccttctggctcatcaacaacaagcccgaattgctgcaggcggagttcggcatcaacgaaggcggcggcggcgaactgcgcggcggcaagcccaacctgcaccgcatgcaggtggccgagaagatgtacaccacctacatgctcgaggcgcgcgacgcgggcggccacagctcggtgccgaccaagagcaacccgatctatgcgctgtccgcggggctggagcggctgggcaactacgcgttcccggtcaagctggcggacgtcaccaagacctatttcgcgcgcagcgcaccgtttgccacgggccagctggccgacgacatgcgcgccatcggcgccggcaaccccgacgccgcggtgatcgagcggctgtcggccaaccccgcctacaacgcgcagctgcgcaccacctgcgtgacgacgatggtgcaggccggccatgcagagaatgcgctgccgcaatcggccaaggccacggtcaactgccgcatcctgccgcacgacgacccggaagaagtcgagcgcctgctgacccaggccgtcggcaacgacaagatcgtggtgcgcaacctcggcaagcccatgcgcagccccgcctcgccgctgaacggcgacctggtgaagaccgtggagtcggtgacccaggccatgtggccgggcgtgccggtggtgcccgcgatgagcaccggcgccaccgacagccgcttcttgcgcaacgccggcatcccgatgtatggcgtgacgggcatgtttctcgatccggcggacgcgcgcgcccacgggctggacgagcgcatcgagatccagcggctctacgacggccgcgagttcctgtaccgcctggtgagcgaactcgcgaaataacttcgagtcctagtggaatgggggacggtggccgtgccggccgccgcctcgcccgcgcgccacaatagccgccatgtcagacgtgcattccgatcaattgctcagcgaagtcgcggccctgccgcagctgccgggcgtctaccgctatttcgacgcggccggcgcggtgctctatgtgggcaaggcgcgcaacctcaagaagcgggttgccaactattttcagaagagccacggcggcacgcgcatcggccacatgatctcgaagatcgtgcgcatggagaccacggtggtgcgctccgaggccgaggcgctgctgctcgagaacaatctcatcaagacgctcaagccgcgctacaacatcctgttccgcgacgacaagagctacccgtacctgaagatcgcctcgcacgagtttccgcggctggcctactaccgcggcgcggtcgacaagaagcaccgctacttcgggccttaccccagcgcctgggcggtgaaggaatcgatccagctgctgcagaaggtgttcaagctgcgcacctgtgaagacacggtgtatgccaaccgcacgcggccctgcctgctgtaccagatcaaacgctgcaccgggccctgcgtgggctacatcacacccgaggcctacgcgcaggacgtggccagcgccgaagccttcttgatgggggacacccagctggtgctgtcgaagctggagtcgcgcatgaccgggcacgccgagaagctcgaattcgaacaggcggccgagctgcgcaaccagatgtcggcgatctcgcgcgtgctgcaccagcagtcgatcgaaatcgcttcggacaaggacgtggacatcctcgccgtcaaggtgcagggcggcaaggcctgcgtcaacctggcgatggtgcgcggcggccggcacctgggcgaccgggcctattttcccgtgcacgtggaagacgccgcgcagatccaccatggcgaactcgatgcagaagaaggcgtggtgccggcgccggccgattcgatcgaggtgcaggtgctcgaagccttcattgcccagcactacatcgacgtgccggtgcctgccacgctggtgctgagccatctcgtgaatcgcgagctgatcgaggcgatttcgcagcaggccggcgcgcgcgtgacggccgtgttccagccgcgcgaacagcgccgacactggctcgagatggccgagaccaacgccggcctgcaattggcgcggcttctggccgaagagggttcgcagcaggcgcgcacccgcgcgctggccgattcgctggagctcgcgcccgacgacctcgacaacttccgcatcgaatgcttcgacatctcgcacaccgcgggcgaggccacccaggcttcctgcgtggtgttcgagcgccacacgatgcagaaccgcgaataccgccgctacaacatcgagggcatcacgcccggcgacgactacgccgcgatgcgccaggtgctgcaccgccgctacggcaagctggccgaggccatggccgccgagaccgatgcgccgcccatgggcgatgccggcggcgcgggcagcgacgcgccccccaagacgagggctgcgcgcatgcctgacctggtgctggtggacggcggcaagggccaggtgtcgatggcgcgcgaggtgttcagcgaactgggcctggcgctgtcgctcatcgtgggtgtcgagaagggcgagggccgcaaggtcgggctcgaggaactggtgttcgcggacggccgcgagaaggtctacctgggcaaggattccgcggcgctgatgctggtggcgcagattcgcgacgaggcgcaccgcttcgccatcaccggcatgcgcgccaagcgcgcgaaggtgcgcgtgggcggcagccagctcgaagacattccgggcatcgggccgaaacgccgcgcgcgcctgctgcagcgttttggcggaatccgcggcgtggcggcggccagcgtcgaggacatcgcatcggtcgaaggcattgccaccgacctggccgaggaaatttatcgcgcactgcattgaggccgattgcccctggctttcggcccgtcacgcgtgcatgacacaatcgcccgcatgttctggaccctcccgaccatcatgacctggacgcgcatcgtcgcgattccattgatcgttggtgtgttctatctgccgatggccgagccgatgcgcaatctgattgccacggtgatgttcatcgtctttgccgcgaccgactggctcgacggctacctggcgcgcaagctcaaccagacctcggccttcggcgccttcctggatccggtggccgacaagttcctggtgtgcgccgcgctgctggtgctggtgcacctgcagcgcgccgacgtgttcgtggcgctgatcatcatcggccgtgagatcgccatatcggcgctgcgcgaatggatggcacgaatcggcgccggcaagagcgtggcggtccacatgatcggcaaggtcaagacgaccgtgcagatgatcgcgattccgttcttgctctatgacggacagcttttcaagatcatcgacaccgggctgtggggccagtggctgatctggatctcggcggtgctcaccgtgtggtcgatggtctattacctgcaaaaggccattcccgagatccgggcccacagcaaatgacgacggcggccgtggcacgcggctcgggctggctgcgtgcaatgccggcgatcttcgtactgatatggagcacgggcttcatcgttgcgcgctatggcatgccctacgcgccgccgctcaagttcctggccgtgcgctatgcgctctgtctcgtgtgctttggcatctgggtcgcgctcgcgcgggtcgcctggccgaaggagcgcgcgcaatgggggcatcttgcggtcacgggcgtgctgatgcaggcgggctacctgggtggcgtctgggctgccgtgcatgcgggcatgggcgcggggctggtggcgctgctggtcggcatccagccggtgctgaccgccatctggctgtcgttcaatggcggacgcattacccagcgccaatgggcggggctggttctcggctttgcgggcctggtgctcgtggtgtcacgcaagttcgggcagggcaccgaggtcagcgcgctgaccatggggcttgcagtcatggccctcctttcgatcaccgcgggcacgctgtaccagaagcgcttcgtcgcgccctgcgacgttcgcagcgcgagcgccgtccagatggcggcggcgctgcttgtgtccctgccctttgcggcgatggaatcgcagggcatcgagtggaacgcgcactcgaccggcgccatggcgtggtcggtgctggtgctgtcgctcggtggcagttcgctgctctacatgctgattcagcgtggcacggccacggccgtcacgagcctgctctacctggtgccgccgtgcacggcggtgatggcctggctgcttttcggcgaaccgatcacattggtcacgttgctgggcatcgggctcaccgcagtcggcgtcagcctggtggtgcgcagcgggcgctgagccagtgttttctcagcgtggagaaccggccttgcccggcttccacggctcgccgcgaaactgttccgccaggtggtcgagcagcagccgcacgcggcgcggcgtcttgggccgccagggcgcaatccagtggatgtcggcatcgggcatggcgtagtggggcagcacgcgcaccagttcgccggaagccagttgcggcgcaatatcccagaggctgcgtagcatgatgccgtggccggccaggcaccagtcgcgcaccatttcgcccgaattgctcgtcaacgggccctgcacgcgaacgcgggccgtgctcccgtcgcgcgcatggcgcagtgtccagagcgaggactggcgctggttggcctcgccgttttcgcgcgccaccaggcagtcgtgcgctgccagcgcctcaaccgtggcgggcgtgccgcgccgctctatatatgcaggcgaagcggcaagcacgcgctggttgcgcgcaatgcggcgcgtgacccagtctgccgcgcggcgctgctgcacggcccagagccacagcgcgccgtcgtagccttcggcaccgagatcgggtagccgctcggtcaggagcaattcgatctgcagcgcggggtggcgggcctggaacgtggccagggcagggccgagccagcgccgcccgaagccgaaggtggccgccagccttatcgtgccgaccaggtcgttctgccgctcgcccagttcgctttcaagcgctgcaaaaccttcgagcagcgtcttggcgtgcaggcagacggcctcgccctcggccgtcacgctgagccggcgcgtggtgcgttcgaacaaccgctggcccagcctggcctcgagcgcgccaagccgcttggtgatcaccgagggcacgacgtcgagcgtggcggatgcgcccgcgaggcttccctggtcgcgtatggcgaccacgagctccagatcgctgcggtccatcgacaatggattcatgccagattggaaagtatgaattggctgattgttgcttgatggtcgacggagcgcaacgcacaattgcccgcgtgactgcttcatttttcgactttcctgaattcggcatcgagcgcaacggcgtgcgcgtgcatggccgcaccggcgggcgcggcgctcctttgctgctcttgcacggccatccgcagacgcacctgatctggcatcgcgtggcaccggcgctggccgagcgattcacggtggtggcgctcgaccttcgcggctacggcgactccggccgccccgcggacgatgacgatcacgtggcctacagcaagcgcgagatggcgctcgatgcgctcgccgccatgcaccaccacggcttcgagcgcttcggcgtgctggcccacgaccgcggggcacgggttgcgcaccggctggccgccgaccatgcggcggccgtcgaccggatgatgcttctcgacatcgcacccacgctctcgatgtacgagaacaccaccgaggcgtttgcccgcgcctactggcactggttttttctgatccagccgccgccgctgccagagtcgctgatcgcctccgatccggtgcgctacgtgcgcagcgtgatgggtggacgccacgcaggcctcgcgcccttcgcgcccgaggtgctggccgagtacgagcgctgcgccggcattccgggcacggccgaatccatctgcggcgactaccgcgcctccgccaccatcgacctggcgcacgaccgcgccgacatggccgccggccagcggctcgcgcagccgctgcgcgtgctgtggggcgagcacggcgcggtgggccgctgcttcgacgtgctggcgctctggcgcgagcgcgcacttcaggtctcgggccgcgcattgccgtgcggccattacgttccggaagaagcccctggcgagctgctcgccgaggcactccagtttttcacccctctccagcaagaaggaagcagatcatgaccacccacagaatcgcagtcatcgccggcgacggcatcggcaaggaaaccatgcccgaagggctgcgcgtgatggatgccgcggcacgcaagttcggcatcgacctgaagttcgaccacttcgacttttcgagctgggactactgcgagaagcacggcaagatgctgcccgacaactggaaggaccagatcggcgggcacgacgcaatctactttggcgcggtcggctggcccgagaaaattgccgaccacgtgtcgctctggggctcgctgctcttgttccgccgcgagttcgaccagtacatcaacctgcgtcccgcacggctgatgcccggcatcacggcccccgtggtgcggcgcgacggcacgccgcgccagcccggcgagatcgacatgtacatcgtgcgcgaaaacaccgaaggcgaatattcgagcattggcgggcgcatgtacgaaggcacgccgcgcgagatcgtggtgcaagagacggtgatgtcgcgcgtgggcgtcgaccgcgtgctcaagttcgctttcgagctggcgcagtcgcgccccaagaagcacctgaccagtgccaccaagtcgaacggcatctcgatcaccatgccgtattgggacgagcgcgtggccgagatggcgaagaactacgcgggcgtgaagctggacaagttccacatcgacatcctcaccgcgcacttcgtgcagcggcccgacttcttcgacgtggtggtggcgagcaacctgttcggcgacatcctgtccgacctgggcccggcgtgcaccggcaccatcggcattgcgcccagcgccaatctcaaccccgagcgcaccacgccgtcgctgttcgagccggtgcacggctcggcgcccgacatcgcaggcaagggcatcgccaacccgatcggacagatctggtgtggcgccatgatgctcgagttcctgggccacaaggatgcgcatgacgcggtcctgtccaccatcgaaaaggtgctggcgccccaaagcggagcaccgcgcacccccgacatcgggggtaacgcgagcaccagcgacctcggcaaggccattgccgaagccatttgaaattcggcttcatgaaacgcccctaaaatcgcgcgctccgctgttctgcatggcctcgtgtcgtattgacaccctgcagaccagtggttgtaatcctcgctggcagcgcgctgccgaggcgtcagtcctgccaggcttcgcgcgtcgcgacgtttcgcggccagctcgcagctgacgaaagccgacaaactttatttcttcgacaaggggcccttgtgaacaagaccgaactgattgagcacatcgcaaaaaacgccgatatttccaaggcagccgctacccgcgcgcttgaatccaccatcggcgcgattcgcaccacgctcaaaaaaggcggctcagtgtcgctcgtcggtttcggcactttcgcagtcggtaaacgcgccgcccgcaccggccgcaatccacgcaccggcgacgcgattaaaatcaaggccgccaagattccgaagttccgtccgggcaaggcgttgaaagacgcgctgaactaagacgtagactcggagagtattcccggtggggtgcttagctcagctggtagagcggcgcccttacaaggcgtaggtcgggggttcgagcccctcagcacccaccacccacccgatgcaaaggcgaacactggttcgccttttttattgccgtcccgacatccgtcgcaaaagagtgttcaagcatgtttgattttttccgcaagtacaacaagatcgtcctgattatcttgttcttgctgatcattccatcgttcgtcctttttggcgtggagcgctaccagggctccggcgacgagaaggttgcgcgcgtcgacggcaacaacatcacccggcccgagtgggatgcgcagcatcgcatcgaaagcgaccgcatccggcagcaatcgccgaatgtcgatgcggcgctgctcgaatccgacgtgatgcgctacggcacgctggagcgcatggtgcgcgatcgcgtgctggccgcggcggcggccaagtcgaacgtgacggtttccgaagagcgcctgacgcgactctttgcacaggatgcagggcttgccgcattccgtacgccggacggcaagttcgaccgcgagaccttccagcgcgtgacgggccgcacccccgagcagtacgaagccgcgatgcgcgccgacctggccacgcagcaggtgctgctgggtatctcgggcacggcgttcacgccgcccgcactggccgcggccacgatcaatgccttctatgacaggcgcgagatccaggtcgcacgtttcacccccgaaagctttgcgccgaaggtgacggtcagcgatgccgacgtcgaaacctactacaaggcccacacggcgcagttccaatcgcccgagcaggccaacatcgagtacctcgtgctcgatttggaggcggccaagaagaacatctcggtcaacgaggccgatctcaagacctactacgaacagaacacggcgcgcttcggcaccaaggaagagcgccgcgccagccacatcctgatcaccgcaccagcgagtgcgccggcggccgatcgcgccaaggcgaaagccaaggcggagcaactgctggccgaagtgaagaaggcgcccgccacctttgccgacgtcgcgcgcaagaattcgcaagaccccgggtcggcggagaagggcggcgacctcgacttcgtgacgcgcggtgcaatggtcaagcctttcgaagacgcgatgttcgcgctcaagaagggtgacatcagcgacgtgatcgaaaccgagttcggctatcacatcatccgcctggccgacatcaagccggccgtggtgccgccgttcgaacaggtgcgcgccaccatcgagaacgaggttcgtgcgcagcaggccacacaggagtttgccaaggccgcggaagccttcaccgatgcggtctaccaacagccggacagtctcaagcccgcggccgacaagctgaagctcacgatccagaccgcaagcaacgttgcgcgcacgcccgcacccggcgttaccggcgtgctggcaaaccgcaatttcctgaacgcactgttcgcggccgactcgttggagcgcaagcagaacaccgaggcgaccgaggtcggctccaaccagctcgcagctggccgcgtgacgaaatacacgcctgcgcatccgatgcccttggccgaagtcaaggacaagatccgtgcgcaactcgtcaccgagcgcgccgcggtcatggccaagaccgagggagaagccaagctcgctgcctggaccgcgaaggccgacggtgcaaccttcggcgcgccggtcacggtgtcgcgccgcgaagcacagaatcaacccatttcgatcatcgacgccgcgctgcgcgccgacgcagccaagctgcccgcactggtgggcgtggacctgggcacccagggttatgcggtggtgcgggtgaccaaggtcgttccgcgtacgccgtcggcgccggagcaggcccagcaggaaaacgcgcaggtcggccaatcggtcacagcggcggaagagctcgcctactacaacctgctcaaggaacgtttcaaggccgagatcctggtgccgaagccggcggatacgctgcccgcggcggcccggtgatgcacgacgcggtgtcgcgttcgggtcgctgacccggcgcgtcgtcgcacgtgggacaagcgcgccatgcgcttgttgccagaatccgttgcatgggaaccctctatctcgtgcgccacggccaggccagcttcggcgccgccgactatgacaacctgagcgagctcgggcacaagcagtcggtgcgcctcggcgaatactggcgcgagcgcggcatgcatttcgatgccgtgatcaccggcaccctgaagcgccatcgccagacctgggagggcattgccgaagggcttggcctccagcgcgacgacgtgctcccgtggccggggctcaacgagtacgacagcgaagcgctcattgccaccattcacgaaggcaagctcgagaagcccgattcgcccgagatgtaccggcaccactttcgccttttgcgcgatggcctgggcgcctggatgcaaggcaagacccagcctgtcggcatgccgagctacgtcgactttctggccggcgtgacgacggcgctcgaccatgtgcgcgatcggtaccatggcgccaaggtgctggtggtgtccagcggcgggccgatcagcacggccgtcggccatgtgcttggaacgagccctgaaaccacgatcgaactcaatctccgcatccgcaatacctcggtgaccgagttcgctttcacgcccaagcgccacatgctggtgacgtacaacaccctgccgcacctggacggcccggcctacgaaggctgggtgacctacgcgtgatgaagcaccagcctcaggcctgccagacgccgtagccgttcttgcgcagcgcgatgccaagctcgacctccatcgatcgcgcgtcctcgtagctcagggggttgtagcgttcgtacagggccggcagcagccgcaggccgaaggcctggacgaagctgttggcctggatgccggccttgtgcttgtcgaagcggatgtccgggtcgagcccggtcattcccacgtacacaaaaggcttgccgagctggtagtcgggattggcgcgcctgaagcggccgtgattccatacgcggtcgtcgagctcgatcacatagacgtgatgcttggctcttggcttgcgcggcacgtccgcaccacctgccgtactgtcgtactactagctcttgcgcttgatcaggccgtaaagaaccagcagcacgattgcaccgagcacggacgcgatgaagcccgcaccttgtccggccgtataccagcccatggcctggccgacataggtcacgatcaacgatcccgcaacgccgatcagcgtggtcacgatgaagcccgcggagtcgtcgcccggcttgacggcgcgtgccacgagacccacgatgaacccgatcagaatagtccagacgatgctcatgaaaaatcctttggcggtgaaatggaagcgcgtggaaaacctgcgccgtcggtgcaggcggcattcatgatagcggagcagttcaggcaccaagcttggtgaattccgttgaaccgtcgttcgggagttttggcggagacggccatgccgcgcatgctgtagcgtcctacaggccgccgcgccgcgcagcgctataccggcgccatgctcgagaaattgcctgaagtcatcggccacgcgctgcacggcatgcgcgcgggcctggacaagatcgttttcaacgcgctgggcatgcgccagggcatggcatcgatcgcactgaccagcgtggccttcgcggaccatgcacccctgccaccgcgctacacggccgatggggaaggcctctcgccgccgctgcaatgggccgatctgccgactgaaaccacctcgttggtgctggtggtcgaggatgccgattcgcccaccccgaatccgctggtgcacgcgatcgtggtggggctgcggccgagcgaaggcaagctcgacgaggcagccattccaggccggggcaacgagggcgccgccggcctgcacgtcggacgcaactccgggctgcaggcggcctggctgccacccgatccgccgccggggcatggcgcgcaccgctacgccttccagatatttgcgctgggcggcgcgccgttgttttctgccacacccgggcgcgacgaggtgttcaatgcgctgcgcgagcatgcgcttgccagcggcctcttgatcgggacctgcgaacggccggacggctcgatcaagatcgaggaggctgcgccagccggccccttggcagcgggataagaagattttcaggggtccgcaactgcgggggtggcgaaaacagccatttttaccgctacaattgcgggctctgcggtggctgtagctcagctggtagagtcccagattgtgattctggtcgtcgtgggttcgagtcccatcagccaccccaaaataccttcctgactgctattgcgcaatagcgtccatggaaaccactacgccgggcccgccccggcgttgtcatttccagctaccgcttccgccggtgcctggagtctctcccgtccttttttgttccataaaacgtccgcgcgggcgagttttcgttgtgcgctgccgcaatccgtgcgtgccggcgctttttctcgtcacggcctgcttgttttaaattggaattgaattaaaatccgccccgtttccaattttcaggagtccaaaatggcttcgacccttgccgatatcaattctcagatcaagaagtacgacgagcagattgcgcaattgcgcaagcaggccgaagaccttcgcaacgaagagcgcgctggcatcattgaagatgtgcgcagaaagatcgccgaatacggtttgacggcttctgacctgaaactgagcgcacgtggcgcctcggtcaagcgcagcgccggcgttcccgccgccaaggcagcggccaaataccgcggcccgaccggcgaaacctggtccggcggccgtggccgcaagccgcgttgggtcaccgaagcattggccgccggcaagtcgctgaccgaattcgagatcaagtaagcgtctcgcgaggcctctggcccgaaaaaaagcccgcatgcgcgggcttttttattggctgaacaaccgatggggcggcgcgttcagttcaccatcacgagttttcctttgacgccgcgcgagcccatgtgggcataggcggctttcaattgcgccatcggcatggtgctgtcgatgacgggcttgatctttccctggccgtaccagtgggccaattcggccatcatttgcgcattggccttgggctcgcgcttggcgaaatcgccccagaacacaccgaccagcgacgcgcctttcaacagcgtcagattcaatggcagcgatggaatcgggcccgaggcaaagccgacgaccaaatagcgcccgcgccaggcaatcgaacgaaatgccggctctgcgaaatcgccgcccactgggtcgtaaatgacatcgggccccttgccgtcggtcgcggccttgatcgcgtcgcgaaacccgcctggaagcgcgtgcgtcgtgtagttgattgtggcgtcggcgccaatggagcggcagagttcgcatttctcgtcggtcgaagccgctgctattactttggcgcctgccgcctttgcgatctggatggccgcggtgcccacgccgccggcggcgccgagcacgagcacggtttctccggccttcaattgcgcgcggtccatcaatgcatgccatgaggtggcatagatcatgatgaacgccgccgcatcgacgtggccgaagccttccggcagcggcatgcaaagtgcggccggggccaatgtgtgggttgcaaacccgcccgtgcccgagaggcacgccacgttctgcccaaccttcagatgcgtgacgccttcaccgactgcctggacgacgcccgcatattcggagcccggtacgaaaggcagcggcggcttcatctggtatttgttctgaacgatcagcagatcgggaaaattgaggctggcggctcttatttcgatcagcacctggcccggacccggcgttggtgtgggcagttctttccaggtcagcgcatcgacgccagtggggttttcgcaaagccatgcgtgcatgctcgggtctcctttgaatcagtcgtgtgtgggcaatgaatgcgaggcgatgatagggggcgcggcggggcgcccttgtccctgctgcgacgcacccggcgcctacaatccggggcaccgaaaagcaccatgaagatacttatttccaatgacgatggctttcaggctccaggcatcgtcgcattgcacgacgctctgaaagacatcgccgatgtcgaggtggttgcacccgagcacaacaacagcgccaagtcgaatgcactcaccctggcggcacctctctacgtgcacaaggcacacaacggttttcgctatgtgacaggcacgccggccgactgcgtgcacatcgcgctcaaggggctgctcgactaccggcccgatctggtggtgtccggcatcaacaacggcgccaacatgggcgacgacaccatttattcaggcaccgtgggcgcggcaatggaggcgtatctgttcggcattccggccgtcgcgttctcgcagatcgaaaaaggctgggcgcacgtcgatgcagctgcgcaggtggcgcggcggctggtgcagcagatcgagcgcgagcgcatgctcgatggcggcgcgttcctgctcaacgtgaatgtgccgaaccggcccttcgacgaactcaagccgatgaaggtgtgccggctgggccgccgccatgcggcggaaaaagtcatcacgcaggagagcccgcgcggcgagaccatgtactggatcgcaggcgccggcggtgccaaggacagcggcgaaggcaccgactttcatgccaccgcggccggccacatcgcattgacgccgttgcagatcgacctgacagaccatgccaacctggggcaatggcgcgagacggttgcccgtctcggcaattgacatggccacgcaacggcctggattcccggttcgcctgacacccactgcttcagccgccacgcgcgggcggctgccggccgtgccggcgaagccgatggtgccgaccaccccctcgatggcttccgacgccgtgcgcgcgcgcatggtgcagaaacttgccgcccagggcatcaccgatccgcgcgtgctgcgcgcattgggcgcggtagagcggcatcgcttcgtcgacagcgcactggtcaaccaggcctacgaagacacgagcctgcccatcgggctgggccagaccatctccaaacccagcgtggtggctcggatgatcgagctcctgctgggtgcgccggcgctcgccggaaagccgcaggagcgcctgggacgcgtgctggaaatcggcaccggctgcggttaccaggcggcagtgctgaaccatgtggccgccgaggtctacagcatcgagcgcctgcgcggcctgcacgagcgcgcgcgcaccaatctgcggcacttccggttggcgacggtgcacctgatgctgggtgacggcatggtcggctacgccaagggcgctccgtacgcgggcatcatcgccgcggcgggcggcgaagcggttccagaagcctggaccgaacaactcgccgtgggcggacgcatcgtcgcgcccacgcaatcgacggggggcggacaggccctcgtcgtcatcgataaaaccgcccgcggactcgagcgccgtattcttgaggcggttcattttgtccccctaaaatcgggcatcgcttgaaggaacaacacatgcagggttttggcaatcggagttggtgcgctggtatcacgttggccgttgtgctcgtgatcgcaggctgcgccgcaccgcgagggccggcaccggtcgaagaccgcggcaccatgacgcgtgcgcccggtgcggcacccggtggcccgctcatcaccaccgatgcctcgggcaagccgcttccgggcatcgaaaactatggcaagccgggctactacaccgtgcggcccggcgacacgattcgccgcatcggaaacgaaaccggccaaagctggcagaacatcgttcgctggaacaatctcgagaatcccgacctgatcgaagtcggccaggtgttgcgcgtgattccgccggtcggactggcgagcggcgccacctctctcgcgaccgcgcccgcacccgcagatggggtggtcaccaagcccgtggcgccgccgtctgttgtggtgcccacggcgcccgcgagcgcagcgaccggcaagccgccggtcaccgcgtcgccatcggcacctgcctcgaactcggctgacgaagacctcggctggatctggccggcgcatggcacgctcattgcgggcttcgacgatgccaagaacaagggattcgacatcggcggcaaggcgggcgatgcggtgctggctgcggccgacggacgcgtggtctatgcgggcgccggcctgcgcggctatggcaacctgatcatcctgaagcacaacaacacctatctcacggcgtatgcgcacaaccagacgctgctcgtgaaggaagatcagtcggttcaaaagggccagaagatcgccgaaatgggcaacagcgacgcggaccgcgtgaagctgcacttcgaaatccgccgccagggcaagccggtcgatccggcgcgctacctgccgagccggtgatgccatggccgcctctcgcctccgtcgcacgcttgctgtgcgtcggctggcgggccggggcggggcggtagaaaacaacagcgaagacgcggcaccggcaaagcccgctttcgccccggacttcgaagcggcagcagagccgtcgattggcggcgagggcgcggatgccctgacgatctacctgcgacaggtacggcgaaccgagctcttcacgccggaagaggaatacaaggccgcatgcgctgcgcgcgccggcagtttcgaagcgcggcaatcgatgatcgaacacaacctgaggctggttgtgaacatcgccaaggcctatctcggccgtggcgttccgctctccgatctcatcgaggaaggcaatctcggcctgatgcacgccatcaccaagttcgagcccgagcgcggtttccgcttttccacttacgccacgtggtggattcgccagtcggtggagcgcgcagtgatgacccaggcccgtgccatccgcctgccggtgcatgtggtgcgcgaactgcagcaggtgctgcgggcccgccgaacgctggaaggcgacgcggaattcctggtgcaccggcccgacggcgtgcgcgtggaagacatcgcggcactcctgggccgcgacgtgcaggcgatcacggaactgctggccctttcggaaccgccgcgctcactcgatgcgggcgacgcgcgcggcgaagagggcggctttacgctggccgacaccgtggcttccgacgatgagcggggcgatccgaccgacgtcacacaaacccacgaagtcgctcgcctgctcgatcagtgggtgcatgccctggatgcgcgcgagcgcgaggtgctggaaggccgctacggcctgcgcgaccgcgagcccgaaacgctcgaggtgctgagcgttcgtctcggcctgacgcgcgagcgcgtcaggcagatccagaacgaggcgctggccaagatgcggcgccagttggtccgctctggcgtggggcgagacgccctgttgtagccgtggctgccaccgccgtggaaggccgggccggcgctgagacaatcgggggatgacggaatccatcgaagaaaagaaagtccccgcgaaaaccccggcgaccgcgcgtgacgaatggctcaaggtcgagtcgctcgacctcgacgcgcaaggcgtggcgcacaacgccgaaggcatggtcgtgttcatcgaaggcgccctgcctttcgaagaagtgcagctcaacgttcaccgccgcaagaacaactgggagcagggcacggtcacggccatccggcgtgaatcgtcgcagcgggtgcgcccgggctgcccgcatttcggcttgcacaccggcgcatgcggcggctgcaagatgcagcatctggatgcggccgcgcaggtggcggtgaagcagcgcgcccttgaagacaacctgtggcacctcggcaaggtccggcccgagaacgtgctgcggccgctggaagggccggcctggcactaccgctatcgcgcgcggctctcggtgcgccacgtggtcaagaaaggcacggtgctgatcggtttccacgagcgcaagagccgctatctcgccgacatgcaggtctgcccggtgctgccgaaacagatgagcgacatgctgatgccgctgcgtgcgctgatcggctctatggatgcacgcgagacctgcccgcagatcgagctcgcctgcggcgatgcgcccggcacgaccgcgctcggcaccattgcgctggtactccggcacctgcagccactctccaacgccgacattggccggctgaaggcctttgcggcgcagaacacgggcgtccagtggtggctgcaggccaagggccccgaaaccgtgaagctgctggaagagggtggcacgccgctgtcgtacgagttgcccgagttcggcgtgaccatgccgttcaagccgaccgatttcacgcaggtcaatccgcacatcaaccgtgcgctggtgggcaaggcgctgcgcctgctcgacgtggcgccggaagagcgcgtgatcgactggttctgcggtctgggcaatttcaccttgccgctggccagccgggcgcgcgaggtgctgggcatcgagggcagcgacaccctggtggcgcgcgcgagcgacaacttcaggaaaaaccagcccgccacgtccgccaggcgggcgctttcgccgacccggttcgtggcccggaacctcttcgagatgacccccgccatgctggtggccgacggcagcgccgacaagtggctggtcgacccgccgcgcgagggagccttcgcgttggccaaggccatggccgatctgcacctgcagcccgagctgcgaaccgatggctggacgccgccgaagcgcatcgtgtacgtgagctgcaatccgtccaccctggcgcgcgatgccgggctgctggttcaccaggccggctaccgctgcacattcgcaggggtgatcaacatgttcccgcacacggcgcacgtcgagtcgatggcggtgttcgacctggcatgaaaaaagggcccgtcgggcccttttttcattggcgcacgcggcgccttctcgttcgttcagtcgcgctcgccgccggcaatgcccagcagggccagcaggctctggaacacgttgaacaggtccaggtagagcgcgagcgtggcgctgatgtagttggtctcgccgccgtccatgatctgcttcaggtcgtagagcatgaaggccgagaagatgccgatggccgccaccgagatggccatcatgcccgcgctggagcccacgaagacgttgatgatggcgcccaccatcagcaccatggcgccgacgaagagccacttgcccatgccggacaggtcgcgcttgatgacggtggccagcgaagccatcacgaagaacacgccagcggtgccgccgaaggcggtcatgacgagctcggggccgttcttgaagcccagcaccatcgcgatcaggcgcgacagcatgaggcccatgaagaaggtgaaggccagcagcaccggcacgccagcggcggagttcttggtcttctcgatggcgaacatgaagccgaaggcgccgccgaggaaaacgatgagacccagtccgcccgagagcgagcgggtgatgccggtgctgacgccgatccaggcgcccagcacggtgggcagcaggctcagtgccagcagccagtaggtgttgcgcagcacgcgctggcgttcagcctgcggcagcacctggccgtagccggtggaagtgtcgagggtggtaacgcggtcgttcatggccgtagctcctttgattgctgcagtgatgcagttgggcgcattctaggggtctgcaagagggggtaacgaaaagaccgtatgggcgatggtcctaagccccgccggggtttcggtcgcattgcccgttatgctgtcgggttttacgaacctgctccccaacatgaagaccaagtccttcctcgaactcgccgacgtcaaggccattgccgccgcagccgaagccgaagccctcaagaacaactgggccgtgactattgccatttccgacgatgccggcaacctgctctggctccagcgcctggacggcgccgcggcgctttcgtcgcacattgcccctgccaaggcgcacaccgcagccatgggacgccgcgagagcaaggtctacgaagacatcatcaacggcggccgcacggcgtttctcacggcgcctgcggtgcagggcctgctcgagggcggcgtgcccatcgtcaaggacggccaggtgatcggcgctgtcggcgtgagcggtgtcaagtcgaacgaagacgcccagattgccaaggccggcatcgcagcgctcggcctctgagaacctgaagccccaaagcaagacgccgaccaagggtcggcgtttttgttgaagtgctcagcgtggaaaaagagcttggctagtcggcgaaccgttggctagcaaaaaacgaccctcggagatgaaatctcctcaagtcgccccacgatgaaacttgcgcgaagggcgggctgattttttacttggtaagaatcagcttgccgagtttggtggcctggagcctatagagggaaccgttgtgcatgatgcccacggtcttgcttcccttcaaaagctccgtgctttcgaccatgggcgccggacgggcggcctggatggatgcatgaccgccacccgattgatcgagcgaaggatggctcagaacagaaaaggcgttgggcttggcttgcatttgaaattcccttatcgaagcgatgagtgaatgataatgattcgcaataaaaagtcaatcgcggcgatcaactttttttcgtgtgcgcaggggcctatttcgcgtcaggctctgtaatgaagccgatcttgcgcacgccggcttcccgcgcctgcgacatggccttggccacgcgctcgtagcgaacggccttgtcgccgcggatgtgcagctcgggctgcgggtccttggcggcctcggcggccaggcgggcgggcaactccccgtcttcgaccttctgctcgttccagtagtagctgccgtcggccgtgatgctgaacaggatgttctgcggcttgggctgctcgggttcgctggtggcgcggggcaggtcgatgttgactgcgtgcttcatcaccggcacggtgatgatgaagatgatcaggagcaccagcatgacgtcgaccagcggcgtcatgttgatctcgttcatcacctcatcgggttcgtcctgggtaccaaaagccatgatgctcagcccttcttgagcggaaccacaatggcgtcgccggcgccgctttgcacgcgtgcgccggtcacgaagtaggcgtgcaggtcatgcgcaaagctgttgagcttggtcagcacgaacttgttgccgcgcaccagcgcgttgtagcccagcaccgccggaatggccaccgcgaggcccagcgccgtcatgatcagggcttcgccgatcgggcccgccaccttgtcgatggtggcctggccggccgtgctgatgctcatgagcgcgtgatagatgccccagacggtgccgaacaggccgatgaaaggggccgttgaacccaccgacgccaggatggccaggccgctctggaggcgggcggtgaatgcgtcgatgccgttgcgcagtgcgcgcgtgatccagtcgctcacatccaatgcgtcatgcaaatgagccttggtgttgcggtggtgcgcagccgcttcgcggccttcgagcgcgagcgcgcgaaacgggttgccgtcgtccttgccgagcttgttcagcgcggttgcgaagtcttcgctgtgccagaaatcctgcgagtgcttggcaaggcgcttgtatttgatgacgtcgagggccttgatgatgatcacgatccacgacacaagcgacatgccgatcaacagcaccgcgacggccttggtgacgaaatcgccctggttccagacgttcatcaagccgaattgggaatccatacgaagttgctccagagaaaaattagttcagtttgaatgagaagggcgcccgcagaaggtaggtggtctgcgcattgcctcccgtttgcctgaaaggggtgacctgggcggtccgggcggcgctcagcgccgcttcgtcgagccgttcgaacccgctggacttgaagagttcgacgcgcttggcaaagccttcgctgtcgaaatagatcgagacgacggtggttccggcctcgcccagccgcttgctcatgctgggaaagacgagcttgggctcccttatatagcgcgtctggccttccgagatctcgatcgtccgcggtgcgggtggtgccggaggggctggcggcggcgccggtggagcgggtggcgccggggcttccgcgacaggcgccggtgcgggcggaggaggttcgggcacgcccaccggagcggcgggcgcgggtgtcggcttgggttcgcgcacggccaccgggcgcggcgggggcttaacggcctcgggcttgcgctgcggaggcggtgggggagggggcggcggctcggccggcttgggcggctcgacgaactggctcagtatctcgacggggatcaccacttcggcggcgcggcgcagcaagccgctttgcagcgcccacagcgcggccgcatgaaacaggatcacgcccccggcaatgagtgcattgcgcgagaggcccaggacggaagggggaggggcaaagcggtcagacacgatcaaccaattcgaatgcgggcgcgccgaagcgtgccccgattgcagcaaaaccgctacgactactgtttacttacgaaagatccaccagaccgagcctgcaacgaagatcaggctgccgccgagagccgagaagagttccatgccttgctttccgagatggaggtggcaagctggatcgcactcgttcccgattcgcggttcagcgcggcgaccggatgcgaggcgctgcactgcgcgacgatatcgcgcgcacaaccttcacattggccacattgggtggccacgccaagctcgaactggacttcgtcgaaagtcatgcccgctcgcacgtgacgtgcgatttcacggtcggagactcggcggcagacgcaaacgatcatggcggtgaaagcggcagttggctggctggtttgttcgaggcctgattataaatacgaatctctcgcattttcaataactatcccgacagaggtctttcgtgtgcattcgaggggtgttgcatctgaacaacatgcgaatctcaatgcgaatgattaagaactacgttcgcactacacttcagcccgatttcggcaagccactgccggtgtaagccaccgggaccagccagcccatccattcaaaccagccgtttgggctttctgggaggttatcttggccaatgtcgtccgccggcgcgctcgtgcgccgcgctccgtgtcttcttctgctcctgccgtgagggccgcaacggccggaatgccgcgggaagcggcaatgctcccattcggggccctgatgcttgcggcctcggtcagcagctgggcgcagacgccgccggccacggtgcaaggcggaacactgggcaccgtcacggtgacggagcaggccgagacgcaaggcaaggaccaggtccagaccaagaagaccaacatcggcaagggcacgcaggagattcgcgacattccccagtcgatcaacgtcatcaccgaaaaactgatcgacgacgtcaagctcgacacgcttcgcgacgccttgcactattcggccggcatcaccttcgccgcgaccgagaacggcaccgaccaggacatccggctgcgcggttttcccgtggcaaccgtcggcgacttgctcatcgacggcatgcgcgatccctcgcaatacgaccgcgataccttcaacctcgagcgcgtcgaggtgctgcgcggttcggcatcgatgatcttcggacgcggctccactggtggcgtgatcaaccaggtgaccaagaagcctatgctggctgaccagaccgacgtggaagccaccgtcggctcccgcggctactaccgcacgaccgccgacttcaatgtgcgcaccggcgaaacttcggcgctgcgcatcaacggcatgtggaacaaggccgacaacggcggtgccaaggtcgacaagtacggcattgcgccttcgtacagctggggtgtgggcacggccaacgaattcaccgtcgggctgttccacctgaacgtggacaacgtcccgctgtcggcggttcgctgggtggcgaccggccgccaaggcattaccggctacaacgcgagcggcgtgccgaccatcggcagcctgggaacgatcgcaccgatcaagcccggcagcttctatggcaccacggccgacaagcttcttggccaagccacctacggcacggcttcctggctccatcgcttcgatgacggcggcgaactgcgcacgcaggtgcgctccggcaccttcgaccgcaaccagtggtccacggccgccggtgccagcaccacgttcggtgcggccaccacgctcgcgaactttggcgactacacggtgctcacgcgcagcggcctcacgccgcgcaaggacgagtacaagggcacgtacctgcagagcgactacagcaaggagctgaactggggcggcatgaagcaccagttgctggccggtatcgatgcctccaaggaggaagcgagccgctaccagaacgatgctttcttcaacaacagcttccgcggccgcgcgctgggttcgcgggccaacaccttcgtcggcacgccgaacgatggtgccggcctgagcggcacgttcgtggagccggtgtaccgcgactcgagttcgtattccgccaagtcgatcggcctctacctgcaggacctggtccaggttgcgcccgactggaagattctgggcggcgttcgctacgaccggctcagcggcgacttcaaccagtacaactacacgaaccccgcgtgcgtgaggcccactccggccccgcgcggctatacgcaaacggcaaactgcaccgatccacgtgagcgctactccgctggcagcccgctgccgacggtcgcgaccacccatttgtcgcagggcgcctggagctaccgggccggcgtgctctatcagccttcgaccacgcagtcgtatcacctgtcgtacagcacgtcgttcaattcgtcggcggacacctatcagtatgtgtcgccccagactgccgggacgccgcctgagaagagccgcaacatcgaactcggcaccaagctcgactggctcgatggcaagctgtcgacgcgcgcggccctcttccgtaccgagaagaccaacgagcgcaccaccgattcggactttgcaagcacgtcctacctgctgtcgggcaagcgccattcccagggtctcgagctcgacgtggtcggccgcctgacctcgcagtgggaagtctatttctcgtactcctacattccgaaggcaacgatcgaccaggtcggcagcaccgcggcgcccggcaccgtcggctcgcgcgtcggcctgacgcccaagcacagcggcgctgcatggatcagctaccaggccacgcccaagttccgcattgcgggcggcgtgcgcggcgcgtccgagaaccggccgctgcaaggcgccagcggcgctgccagcctggccaacagcaccccgggctacgtggtgggcgacatgatgctcgagtacaagttcaccccggacctctatgcgcagctcaacgtcaacaacgtgacgaacaagctctacggcgatcagctctatccgggcttcgtgatcgccggtgccaagcgcacggtgctcttcacggtcggggcacgtttctagaatagtcagccacaaccgatcttccgctcttcatgctcttgcacattcgcgaagtgctctcgcctgacgaagttcgccaggccagggaaatcctgggccatgcgccctgggaggacggccgcctgaccgcaggcgagcagtcggccaaggcgaagaacaacgagcagctgagggaagactgcgaagaaacccgcgcggtccagcaattgctgctgcgcgggctggagcggcaccaggttttcttctcggccgcgcttccaaagcagatttcgccgccgcttttcaaccgctacggcggtgcgtcgaacagcttcggcaatcacgtggacagcgcggtccgttttctgcgcgacggcacgggcagggtgcgcaccgacatctcgtgcaccctgttcctggccgagcccgacgaatacgacggcggcgaactcgtgatcgaggacaccttcggcacgcagcgcgtcaagctcgcagcgggcgacatggtgctctatccaggcaccagcgttcaccgcgtgcttcccgtcactcgcggatatcgcctggcgagctatttctggatccagagcatggtgcgcagcgacgagcagcgccggctgctgttcgaaatggacaaccacctgcgccatctccgcagccaatatggggagaccgatccgggcgtgatcggactcaccagtacttatcacaacctgctgcgcatgtggctcgacatctgagccccggcgtggcgccctgcaatgccgggaggccattcatgaacaagtcacttctttatgtggcggctgcaaccgccgccctctggtccgcgtccgcatccgctcagttcgtcgagcatgacgcgatcaagtgcgcgccggttcccaaggaagaaatgcgtccgcagatggaactgcagcgcaaactgaccggcgaaggctggaaggtgcgccagataaagaacttcaatggctgctacgaggtctacggcttcgacgagaaaggccagcgcgccgaggcgttcttcgatcccaagaccttcgagaaggtcggacaagtcaagcagccttcctgaggcgccgcgcggtgcgtgcggtttccgggcgtccgtcgacgcgggtctgggcactttggctgcgcgcaacacactgggcgctggtggccgccattgcggtggcgtggttcagcggcgaggcgctgctgcggcagcatgaatgggcgggctacgcggcactcgccctggtcgcgggccgctgcatcggcggctggctcggtgggcgctacgcgaggttccgccagttcgttcgatcgccctccgaagtgcggtgctatgcgggcgaggtgctcgcccggcgagaaaagcgctacctgggccacaacccgctgggtggctggatggtcgttgccttgctggccgcggtggctgccgtcggcgtcacgggctggatgtattcgctcgacatgttctggggattggcgtgggtggaatggctccaccgcacattggcctggacgctggtggcgctgattgccctgcatctggccggcgtcgttttcacgagctggcggcacagggagaacctggtggctgccatgctcagcgggcgcaagcgaccgcaggcgccgggcgacgtcgattgacgaatgcgcccggcctcgccgatcagctgagttcgcccatctgcgattgcaggtagttctgcaggccgaccttgtcgatcagctcgatctgggtttcgaggaagtctatgtgctcttcggtgtcgtccaggatttcttgcagcaggtcgcgtgaaacgtagtcgcgcaccgtttcgcaataggcaatgccgtctttgatggtggcttgcgcgccggtttcggcgcccaggtcgcagcccagcagctcgggcacgtcttcgccgatgttcagcttgcccaggtcctgcaggttgggcaggccgtcgagcatgaagatgcggtccatcagcttgtcggcgtgcttcatttcgccgatcgattcctcgtattccttcttcgccagcttgtccaggccccaatgcttgagcatgcggtagtggaggaagtactggttgattgcggtgagctcgttcttgagctgcgcctgcagatgttcgatgaccttggggtcgcccttcatggtttttccttattctgaaagcaccgattgtgagaggggcgggcgggcacttgcaagcaatcccatgctgcgtcggtctgcatgcgtttgatggtgatacacgttcgtattcgttggtggcggctccatcgcaaacatagcaagccgcaatagttttgatagctcataactattaaaaatgaaatattggtagttatactgatggctcgttcttttcatcagccaccaccaaggaaacagtaaatgtccctgatcaacaccgaaatcattcccttcaaggccaccgcgtatcacaacggcaagttcgtgcccgtcagcaacgaaaacttcaagggcaaatggtcggtcgtggtgttctacccggctgacttcacgttcgtgtgccccaccgaactcggcgacctcgccgaccactacgcagaattccagaagctcggcgtcgaggtgtatggcgtgtcgaccgacacccacttcacccacaaggcatggcacgacacctcggacaccatcggcaaggtcaagtacccgctgatcggcgacccgagccagcaactggcccgcgccttccaggtgctgatcgaagaaggcgaagacgccggcctcgcataccgcggcaccttcgtgatcgaccccgaaggcaagatcaagaccatcgaagtgcacgacaacggcatcggccgcgacgccgccgaactgctgcgccgcgtgaaggctgcccagtacgtggccgcccaccccggtgaagtctgccccgccaagtggaccgaaggcgccgaaacgctgaagccctcgttcgacctcgtcggcaagatctaagcgttccgcgcgaaagcccgggcgctcacgaggccccgggcttttttgttccccgttgatagttttcagatatcgaaagtgattccgccatgctcgacgccagcaccaaagcccaattgaagagttatctcgaacgcgccacgcagccgatcgagatcgtcgcctcgctcgacgacagcaaggcctcgggcgaaatgctgtcgctgctgaaggacgtcgcagaagcgtcgccgctggtcaagctgaccgaaagccgcggcgacaaccatcgcaagccttctttctcggtcaatcgcccgagcgagaaccacggcccgcgctttgccggcctgccgatgggccatgaattcacgtcgctgatccttgcgttgctgcagatcggcggctacccacccaaggtcgagcaagccgtgctcgaccagatccgcgcactcgacggcgacttcgagttcgagatatacgtttcgctcacctgccacaactgtcccgacgtggtccaggcgctgaacctgatggcggtgcagaacccgcggatccgcacgacgatgatcgagggcggcaccttccaggacgaggtcaaggaacgccaagtgatggccgtgccgaccgtgttcctgaacggcaccgagttcggccagggccgcatgagcctggaagaaatccttgcgaagatcgacaccagcggcgtcgagcgcgaggcaaagaagatcgccgccaaggacccgttcgacgtgttgatcgtcggcggcggcccggctggtgccgcggctgccgtgtatgcggcccgcaagggcattcgcaccggcgtggcatccgagcgcttcggcggccaggtgctcgacacgctgggcatcgagaacttcatctcgatcaaggaaaccgaaggaccgaagttcgcccatgcgctcgaagagcatgtgcgcgactacgaggtcgacatcatgaacctgcagcgtgccaaggcgctggttccgggcaaggacctgatcgaagtgcagctcgaaagcggcgcctccttgaagagcaagtcgatcatcatctcgaccggcgcacgctggcgcaacatcaacgtgcccggcgagcacgagttcaagaacaagggcgtggcctactgcccgcactgcgacggtccgctgttcaagggcaagcgcgtggccgtgatcggcggcggcaactcgggtgtcgaagcggccatcgacctggccggcatcgtgggccacgtcacgctgatcgagttcgacaccgcgctgcgcgccgacgccgtgctgcagcgcaagctcaagagcctgaaaaacgtcgacgtgttcaccaacgcgcagaccaccgagatcaccggcgaccagaaggtcaacggcctggtctacaaggaccgcgcaacgggtgagctgaagaaggtcgagctcgaaggcgtgttcatccagatcggcctggtgcccaacaccgactggctcaagggcgtggtcgaactgacgaagcacggcgagatcgtggtcgatgccagggggcagacctcggtgcccggcgtgttcgcggcgggcgacgtgaccaccgtgccgttcaagcagatcatcatcgcggccggcgacggcgcgaaggcggcgctgggcgccttcgatcacctgattcgcacctcggcaccggccgagcaggttgccgcctgaaacgcggcagcggcgggctgaccgggcggcaggttcagtaaaccagccgctccggcttcagctcctgcaggatggtggtggcaatttcctcgatcgacttggtcgtggtggaaagccaccggatgcctgcccgtcgcatcatggcctcggcctcggccacctcgtgacggcagttttcgaggctggcgtagcgcgaatcgggccgccgctcgttgcggatctggctcagccgctcgggctggatcgtgagcccgaagatcttcttgcgatagggcatcaaggccggcggcagctggcggcgctcgaaatcttccggaatcagcgggtagttggccgctttgaggccgtgctgcatcgccagatagagagacgtgggcgtcttgccgctgcggctcacacccaccaggatcacgtccgcgccctcgaggtcgcggttgctctggccgtcgtcgtgcgccaggctgaagtcgatggctgcaatgcgggcgtcgtattccttgctcttgctggcgtcgctgaagcggccgatgcggtggttcgacttgaccgccaactcgatctccagcggccgcacgaaggtgccgaacatgtcgagcagcatgcctttgcagccggtttcgatgacttcgagcacctccatgttcgccagggtcgtgaagacgatggggcgcacgccttccagttcggccgtgtggttgatctgccgcaccgcctgatgtgccttgtcgaccgtatcggtgaaaggcagccggacgtggcgcggtttcatctcgaactgggccagcacggcgttaccgaaagtttcggcggtgatgccggtaccgtcggagatgaagaaaacagtgcgtgtgtgcatggtgttgctcttgcggccttgtcctgcggcgcatgcaatcttgccgcgcctacaatccgggccattatcgggaatccgctttcccttgccccaattctttccatgcacaccgcgcccgcacccaaagcaacgagaacgatcgtgccgcgccgcctgcatgcagcaccggtttcaacttctggagctttcccatgtctgcacttttcgacgcgaccgccctggtcgtaccgtttgaaaacctgaggatgaccgacgtcgagtcggtcggcggcaagaacgccagcctcggcgaaatgatttcccagctgccgcagggcgtgcgggtgcccacgggtttcgcgaccacggcgcatgcgttccgccagttcctggcccacgacgggctggccgacaagatcagcaagcggcttgccgcgctggacacggaagacgtgcgggcgctggccgcggccggcgccgaaatccgcgccatggtcgaggcccagccttttccggccgacttgcagaaagccattgccgaggcttttgcgaagctgagcgccggcaacccggccgcctcgttcgccgtgcgttcctcggccacggctgaagacctgccggacgcttcttttgccggccagcaggaaaccttcctcaacgtggtcggtatcgacgacgtgctgcacaagatgaaggaggtcttcgcctccctctacaacgaccgcgccatcagctaccgcgtgcacaagggctttgcgcacgacgtggtcgcgctctcggccggcgtgcagcgcatggtccgttccgacctcggcgcggccggcgtgatgttcaccatcgacaccgaatcgggctttgaagacgtggtgttcatcacctccagctacgggctgggcgagacggtggtgcagggcgccgtgaaccccgacgagttctacgtgcacaagcccacgctgcgcgccggcaagcgggcggtgatccgccgcaacctcggctccaagctgatccagatggaattcgcgacgcccgaagagaaaaaggcgaccggcaaattggtgaagaccaccgacgtcaaggccgagcagcgcaaccgctattcgctcagcgacgccgatgtcgaactgcttgccaaatacgcgctggtcatcgaagagcactatggccgcccgatggacatcgagtggggcaaagacggcaccgacggccagctctacatcctgcaggcgcggcccgaaaccgtgaagagccagcagcagggcaaggccgagcaacgctacaagctgctgggcaaggggacagtgctcgccgaaggccgtgccatcggccagaagatcggcaccggcccggttcggctcgtgcacaacatcagcgagatggacaaggtgcaggccggcgacgtgctcgtcaccgacatgaccgaccccaactgggagccggtgatgaagcgcgccgccgccatcgtcaccaaccgcggcgggcgaacctgccatgcggccatcattgcgcgcgaactcggcatccccgccgtggtgggctgcggcgacgccaccgacctgctgaaggaaggcaccctggtgaccgtgagctgcgccgagggcgacaccggcttcatctacgacggcctgctcgagaccgaggtgaccgaggtgcagcgcggcgtgatgcccgagatcgacatccagttgatgatgaacgtgggcaacccgcagctggccttcgacttcgcgcagctgccgaaccacggcgtcggcctggcgcggctcgagttcatcatcaacaacaacatcggcgtgcacccgaaggcgatcctcgactatccgaacgtcgacaacgacctgaagaaagccgtcgagtcggtggcccgcggccacgcttcgccgcgcgccttctatgtcgacaaggtggccgaaggcatcgcgaccattgcggcggccttctggcccaagaaggtcatcgtgcgcctgtccgacttcaagtcgaacgaataccgcaagctgatcggcggcagccgctatgagccggaagaagaaaacccgatgctcggcttccgcggcgccgcccgctacctgagcaaggatttcggcgaggcctttgccatggaatgcgaggcgctgaagcgtgtgcgcaacgacatgggcctcgtcaacgtgcagatcatggtgcctttcgtgcgcacgctgggccaggccgaacgcgtgaccacgctgcttggcgagcacggcctgaagcgcggcgagaacgaactcaagctgatcatgatgtgcgaggtgccgagcaatgccatcctgcccgaggagttcctgaagttcttcgacggtttctcgatcggctcgaacgacctgacccagctcacgctcggcctggaccgcgactcggggctcgagcttctggccgccgacttcgacgagcgcgacccggccatcaaggccctgctgagccgcgtcatcaaggcctgcaaggctgaaggcaagtacgtgggcatctgcggccagggccccagcgaccatccggacttcgcgctctggctggcggaacagggaatcgagtcgatttccctcaatccggacagcgtgatcgacacctggcagcaactcgccaagcgttgacggaacaggggccatcgcgcccctgtcgcgcggcagccactacggacgcccccaccgggaattcccgcgccggtgcttgcaagaattgaatcagaatgtgttactaatgtcaggcccgtgaattcatgggcttggccggtcgcttgcggactgcgcatggcgaagccgctcgtcgccgcacccgccggcattttgcggaagaaaccatcatgattcttgtcaagacagaagccggacagcaggttctcaaagatcgctcggtacccctttcgccgcgccagcgtaccgccttcatcctgttcgacggtaagcgctcggtcgacgaggtgcttgccggaacaggcattgcgcgggaagaaatcgatcagctcgtcacgctggggctgctcggtccggcggcgggcagcagcagcaaggcagccgttccggccaaggcgcctgaagcgccggccgcaagcccggcgcccgtcgtcgcgccaacgccgaaaccaaagccagccgaagccgccgcgccgtcttccgggcgcagcaggcagcagcgctacaaggacgcctatccgatcgccacccaattgacgggtgctctcgggctgaaggggttccggctcaacctgcaagtcgagggcaccaccagctacgaagatctggcggcgctggcgcccaagatacgtgccgccgtgggtcccgagaaggccgccgcgctcgacaaggccttgaacgactgaagctggacaggcgctgcgccagcagtgctacaatagccggctttgccttgccacactgcgcccgacgctgcaggtggcttttcctcttctacggaagaatccacaaggagtgccatgcgtcactacgaaatcattttgctgatccacccggatcagagcgaacaagttccggccatgctggagcgttacaagggcctcatcacggccggcggtggcaagatccaccgcgttgaagactggggccgccgccagctggcttaccagatcaacaagctcaacaaggcgcactacctgtgcgtcaacattgaagccgagcaaaccgtgatgggcgaactcgaacacgcgttcaagttcaacgatgccgtgctgcgccacctgaccgttcagaagaagaaggccgaaaccggtccttcgtcgatgatgaagacggtcgagcgcgaagaagcccgcaaggcccagcaggccgaatacgccgccaacaacagctgatggcgtgaccgctgccgctgctgcggcaaccggggtcaaccagcttctgctgactgcctctgttgccgaactcggagccttgcgatacacgccggccggccttcccgccatcgacctgaagcttgaacatgagtcgacgcttcaggaggcaggaaaagccaggcaggtgaaaacggccctcaaggctgttgccttcggcgccatcgccgaacggctcgcaacgcagtcgatgggaagcctctggcgttttcagggttttctcgcgacaccgggcaacggcaagcatccggtcctgcacatccaggattttcagcaagattaattttcgacaagaggtccccaaatggccacgttcaagaaattcaacaaagacaagcgcccgaagcgcaacacccagtcgctgctcttcaagcgcaagcgcttctgccgttttaccgtcgctggcgtcgaggaaatcgactacaaggatgtcgacacgctgcgtgacttcatcagcgaaaacggcaagatcatccccgcacgcctgaccggcacgcgcgcgatctaccagcgccagctcaacaccgcgatcaagcgcgcgcgcttcctcgcgatggtgccgtacagcgaccagcaccgcgtctaaggagccgtaccatgcaaatcattcttctggacaaggttctgaacgtcggtgccctgggcgatatcgtcaaggtcaaggacggctacgcccgcaacttcctgatccccaccggccgggcccgccgcgccaccgctgccaacaaggccgaattcgaagccaagcgcgtcgaactcgaaaaggctgcggccgccaagctggctgaaatgcaagcccagggcgagaagctcggcggcacgaccatcaagctgacccaaaaggccggcgtcgatggccgcctgttcggctcggtcaccaacggcgacatcgccgaagagctcggcaagcaaggctacaaggttgccaagtcgcaagtgcgcctgcccaacggcccgatcaaggtcgtcggcgacagcaccgtgagcgttgcgctgcacaccgacgtggtggtcgacatcaccgtcacggtctacggcgaaaccgcctgatcgtccacagcgccttgcgcgctgtcgcaaaagccgccctcgggcggcttttgtctttttgcacaccggttttccagctcggtgcactgaaagatcaccgtttattcacaaccttgtccacacacgccagcgcgtgtgcggcttagcatgcagggttgcaagggaagtccatgtccgccgttttctcctatgccgacaatgacccgtcggccgatcgccaagtcgccaagctccgtattccgcctcactcgatcgaggccgagtcgagtgtgctcggcgggctgctgctcgacaacggcgcgtgggaccgcatgggcgacctgctggtcgacggcgacttctaccgccacgagcacaagctgatctacgccgccatcggcgggctaatcaatgccagcaagccggccgacgtcatcaccgtctacgagcagttgcagggcctcggcaaggccgaggaaatcggcgggctggtgtatttgaattcgctcgcgcaatacgtgccgagcgcgagcaacatccgccgctatgcggagatcgtgcgcgagcgctccatcctgcgcaagctcgtctccgcgagcgacgagatcgcgaccaacgccttcaacacgcaaggcaagtcggtcgacaagatcctggacgaggccgagcagaagatcttcaacatcggcgaagaaggcacgcggatgaagcagggcttccagagcatggatgccctggtggtcgaactgctcgaccgcgtgaccgagatggcggagaacccgaacgacatcaccggcgtgcgcaccggcttctacgagttcgacaagatgacctcgggcctgcagccgggcgacatgatcgtgctggccgcgcggccttccatgggcaagacctcgctggccatcaacatcgccgagcacgtggccctgaacgaagggctgccggtggcggtcttctcgatggaaatgggtgcttcgcagctggcggtgcgtatcgtcggctcgatcgggcgcatcgatcaggggcacctgcggaccggcaagctcagcgacgaagagtggccgcgcctcacggaagccatcgaaaagctgcgtaacgtgtcgctgcacatcgacgagaccccgggcctcaccaccagcgagctgcgtgccaacgcgcgccgcctggcccgccagtacgggcggctcggcctgatcgtggtcgactacctgcagctcatgagcgtgtcgaccagcatgaacgacgaaaaccgcgccacggcggtgggcgaaatttcgcgcggcctgaagatgctcgccaaggagctcaagtgccccgtgatcgcgctgtcgcagttgagccgtggcgtcgaaagccgtaccgacaagcgccccatgatgagcgacctgcgcgaatccggcgccatcgagcaggacgcggacatcatcatgttcatctaccgcgacgactactacgacaagaacagcaaggagccgggcgtggccgaggtgatcatcagcaagcaccggaacgggccgacgggcaccgtcaagctgaccttcctcaagccgctcaccaagttcgagaatatggccagctacggcagcagcgacgactactgacgttgcggattcattggggccgttgctgtttctgcagttttgcattcggccgcagcccgcgccttcagctggcgcatcatgtcggccagcgtcttgcccgcttcgtcgcgaaaacgctccggcagcacctcgaccgcgtccatgcggtcgatgcgaaagccgcgaaagtcgtcgcgcagttcgcaccaggtcgaaagcgtccagaccttgccccagtagaagcagccgagcggacgcacggtgcgttcgctcgcatcgcccgacacgtcgcggtagttcaggcgcagcttgtggcgcgcctccactgcctcgcgcaaggtctgcagccggttgcgcatggcgtcgtccaggcccagtgcgggcgcgtagagcgccaacgcttccgccgagacgcgcgcggccggcggcagcaccgagaggatcttgcccagcccggtttcaatgttgcgcgccagcgccggatcgacccagctctgcgcgagccgcgccgcagccaccagcgctgaagcctcctcctgggtgaacatcagcggcggcagttcgaagcccgcgccgagccgatagcccacgccggcttcgccttcgatcggcacgccctggtgctgcaggtcggccacgtcgcggtacaccgtgcgctccgacacctccagccgctgcgcgaggaaggcggccgtggtgagccggcgcccacggatgagctgcacgagctggaagaggcggtcggcgcggcgcatcagcgcgctccttgcaattttggggcggcctcgccgggccggccctggggtgtactcatgaaactccgatgtggatcgccaccttgtccggcccttcgtaggcttcgaaatcgctgcagtagcggcgcgtgatttccgggtgcgcctcgaaatactgccagatgcgctcccaggtggcgatcaccatctgcggcatttcaccctggcccgaaaagacgaggtagttgccgggctcgatggccacgctgcccgttgcatccgagacggccacgcctaccgtcacgtcgaaggcgccatgagcgtcggattcatagctggaatagacgccgaagatccgggcgtcgcttgtgcgtccgggcgtcgaacggtaggtctcttcgccgaagaagcggttccacagtgcaccgatgcgggcggtcgcaggatcgttctcctcgcggttggtcgttcgagccgcgaggcccgcgacgtggaaagcgccatgatgctggcggacgggttccatcgggtgtgtcttctgcatgggtgatgtcgggattgtggtgctcaaagcgcgagcgccttcaggtcggctttcatggttcgggcgatcagcatcatgtcggcatcgctgatgtcgaacatgccgaagcggaacttgtagccccactgacgcgggttctcgacgaaggcaaggcgctcgatcaacggagcgatgggcgcctcatgcgaagcagcataagccacgtcgcggcgccaggggacgaagccgccgcccatgtcgaattcgtagggttcgccaggtcgcacgatgccgatcgacacgaagctctgcagcttgtccgtgccgccgaacaccgtggccggcgcgtagtaggccacgcgatcgccggctgaaacccgcttgagcggccccagcttgccgtggccgacctgtatgaagccgaccggctcgtggtcgcgcccgcgccgggcgtgctcggcgctggcaacggcgatccagttgcgctgtgccattgcgggtcagtccagggcgtgaaggccgacttcgttgccttcggtgtcgcgcagatgggcgatgaaacccatgccttcgggcagcgcggacttcggcgcgacgatctgaccgcctgccgcctcgacgcgggcaagcaccgcatcgatgctcggcatgcagtccagatagatgcggataccgctgcccgcgcgtgcgctggcattcacgccggcctgcagggcgccgcccgtggcgggattgtcgtagggaaaaacggccagcgtttcgcccccgaagtcctggcggcgcagcttgcggccgagcacggtttcgtagaaggcctgggcacggtcgatgtcggcgacggggatctcgaaccagctgatggcgttttgcatgaaggactctctttcgttgcgttggaaggagcctcgatggtgcggaccgcctcctgacaacgtcttgtcaggagcctgtcacggcggccaaagaaaaagcccgcgatgctccggggagcatcgcgggcctgatcggatccgacgaagcctagagcacgtcgctcgcgaagtccgccagccgcgagcgttcgccgcgcgccagcgtgatgtgtccgccgtgcggccagcccttgaacttgtcgaccgcgaaggtgaggcccgaggagccttcggtcaggtagggcgtgtcgatctgcgcgaggttgcccatgcagatgatcttggtccccgggccggcccgggtgatcagcgtcttcatctgcttgggcgtcaggttctgggcctcgtcgatgatcacgtacttgttcaggaaggtgcggccgcgcatgaagttcatgctcttgaccttgatgcggctgcggatcagctcgttggtggccgcgcggccccattcgccggcgccgccgccgtcgcccttggccaggaactcgaggttgtcgtcgagagcgcccatccaggggcccatcttttcttcctcggtgcctggcaggaaaccgatgtcctcgcccacgctcaccgtggcacgggtcatgatgatctcggtgtagcggcggtcgtcgagcacctgcgtcaggcccgaggccagcgccatcagcgtcttgccggtgccggcggtgcccgtcagcgtgacgaagtcgacttcggggtccatgagcaggttcatcgcgaagttctgctcgcggttgcgcgtgttcacgccccacaccgcgttcttgcccgagctgtagtccttcagggtcttgaagaccgcggtcttgtcgcggatctcggtgacgcgcgcgtacatgctcggctcgcccggggcctcgaaatagacgaactggttgatgtacaggttgggcaccagcggcccgctgacgcgatagaaggtgttgctgccgctttgccagctctcgaccgtcttgctctggcgcgtccagaaatcgggcggcagcgcgagcgaccctgcgtagagcaggtcgccgtcttccagcgtcttgtcgttctggtagtcgtctgcggccaggccgagggcacgcgccttgacgcgcatgttgatgtctttcgacaccagcaccacttcctgcttcggacggccgggctggtccttggcatacaggtcgcgcagggcctgcaccacgcccaggatctggttgtcggccttgccctggggcaggctgatcggcagcgagtagtcgagcggcgcggtctggaagaacagcttgccgccggcaccgcgatggcccgtggtgtcgagcttcaggcccttggcgatgtcggcgtcctgcgccgcggccagggcgtcgagcgtgcggctggtctggcggccgttgcgcgcgacttcggtggtgcccttcttgtggccgtctagttcctccagcacgatcatcggcaggaagatgtcgtgttcctcgaagcggaacaggcacatcgggtcgtgcaacagcacgttggtgtcgagcacgaacagcttggccgggccgttcgatttggcgcgcttggcacgggccggtgcctgcggcgccgctgcttgcgacggggccggcacatagacggggactgcgggcggcgcctcgggttcgccgcgggcggccggcctgtgttcctggctgcggtcctggctgcgttcggagttacgggagggggagggcgcggttttcgacctgccgcgggtcgaaggcgcggcctcggtgccgccgccgactgcctcggcggtattgcggtcgaacagttccaacggctgggagccgctcgacgaggtcgaatcggcacgcgaatcgcccgagcggcgcgagcccctgtgggaggagcgggcgggtgcatcgtgcgcatccggcgagagcaatgcggcgcgtttcgtgggggcaggaggcaatggcatgtgtcaggtcgctcgcaggaagtggaaaccagaaaacgaaaaagccgcctgtagaccaaggcggctttgttcgggggatgcggtcgtggagctcaacggcatgaggccattatgcacacccgcggtgacgcgtctcacgctctttgcaaagtccgttgggcatttcccacgggttgaagcaaaagcgcacagtccgcgctggttgtaacggtcaggcagccttcttgagcgccttgacggccttgagcacgtcgtcgacatggccggggaccttgaggccgcgccattcggccttcaggatgccgtcggcgccgatgaggaaggtgctgcgctcgatgcccttgaccttcttgccgtacatgatcttgttcttgaccacgccgaacatatggcacatcttttcttcggtatcggcgatgagttcgaacgggagttcgagcttggccttgaattcgtcgtgcgacttcatgttgtcgcgggacacgccgaacacggtggcgccggctttttcgaagtctttgtaacgatcgcgaaactgcatggcttcggtcgtgcaacccggagtgttatctttcgggtaaaaatacatgaccagcacgtggccgagatgcgaggtattcgagactttcaggccacccgtggcgttggcgtcgaattcaggaatgggtttgttgacaacgatcgccatgaaacttgttttctccgttggtttccattggatcgagcgctttgaggcacactcgacgaaatggaggattggtcgttgctaactgagggcagctggcctgttcgcaacccggtattttaccccgaaaacctccccctcagccatcgtggggcggttcgaccagcagggcggcaatcacatggcggccttcgccggccaggatgttgtaggtgcggcaggcagccggggtgtccatggtctccacgccggtgcgcttggccatgaggggctgcagccaggccggctgcggaaaccggatgcgggatccgctcccgaagatgaccaattcggcgccaagggatgcgagctgggcgaaatgctcgggccccaattggtcgaaacgggtgcaattccactcgaaacgctcgccgcgcgagccgaccaccacgctgccctcgaccttttcgttgttgatcgcgacccacccggggccgtgggcggtgagggactgggcgtcggatttgtcgggctggagcttcatcggggcactgggaactgtggtcaaattataggttttccccagtgacacgaggccttccagggcctttcgacatcgagtaacccgcgcccgggagggccctttgaagcagttcaagaaatcggccaagctggctaacgtgctctacgacattcgcggccccatcatggaggcagcccagcggatggaggaagagggccagaagatcatcaagctcaacatcggcaacctcgccgtgttcggtttcgatgcgcccgaagaggtgcagcaggacatgattcgcaacctgccgggctcggcgggttattcggacagcaagggcatcttcgcggcgcgcaaggccgtgatgcatgaaacgcagaagcaaggcattgccggcgtcgcgctcgacgacatctacctgggcaacggcgccagcgaactgatcgccatggccaccaacgcgctcctgaacgacggcgacgaaatgctgcttcccgcgcccgactacccgctgtggaccgcggtgaccagcctgtcgggcggcaagccggtgcactacctctgcgacgaggacaacggctggatgccccacctggacgacatccgcgccaagatcacgccgcgcaccaagggcatcgtggtcatcaaccccaacaacccgaccggggcgctctattccgacgagttgctcaagagcatcgtggccatcgcacgggagcaccagctggtgatctttgcggatgaggtctacgacaaggtgctgtacgaccacgcgaagcacaccgccatcgcgagcctttcgaccgatgtgctcacgctcaccttcaattcgctttccaagagctaccgttcgtgcggctatcgcgcgggctggctcgtggtgtcgggtgacaagaagcgcgcggaagactacatcgagggcctgaacatgctctcgaacatgcgcctgtgcgccaacgtgccggggcagtgggccatccagaccgcccttggcggctaccagagcatcaacgacctggtgggcgacggcggccgcctgcggcgccagcgcgacctcgcctacgagttgatcacggccattccgggcgtgagctgcgtcaagccgagtgccgcgctctacatgttccccaagctcgatccgaaggtctatccgatcgcggacgaccggcagttctttctcgatctgctgaaagaaaccaaggtgatgctggtgcagggcaccggcttcaactgggccacgcccgaccatttccgcatcgtgttcctgccgcacgaggaagacctgcgcgaggcgatccaccgcattgccaagttcctggagatgtaccgcttgcgcagccaggcagagccatgaaatccgcatgtgccgcggctttgccggcggcgcctggaacctgccgcgccgcgtgagccgcgtcgtgagcgtgccgcctgccaccccatccaaaccatgaacgcgaatctcccaatgaaacccatccaagtaggcctgctcggcgcaggcacggtcggcagcggcaccttcaaggtgctgctgcgcaatcaggaagaaatcaagcgccgtgccggccgcggcatcgagatcacgatggtggccgacctcgacacggcgcgcgcacgcgaagtggcaggtgagggcgtgaaggtggtcagcgatgcgcgcgccatcattgccaacccggacatcgacatcgtcatcgaactcatcggcggctacggcattgcgcggcagctggtgctcgaggcaattgcggccggcaagcacgtggtcacggccaacaaggcgctgcttgccgtgcatggcaccgaaatcttcgccgccgcccatgccaagggcgtgatggtggccttcgaagccgcggtggccggcggcatcccgatcatcaaggcgctgcgcgagggcctcacggccaacagcatccagtggctggccggcatcatcaacggcaccaccaatttcatcctctccgagatgcgcgacaagggcctggacttcgcgactgtgctcaaggaggcgcagcgcctgggctacgccgaagccgacccgaccttcgacatcgaaggggtcgacgcgggccacaaggtcacgctgatgagcgccattgccttcggcatcccggtgcagttcgacaaggcgcacatcgaaggcatcaccaagctcgccgcgcaagacatcaagtacgccgaacagctcggctaccgcatcaagctgctcggcatcaccaagcgcacagcgcagggcatcgagctgcgcgtgcatccctcgctcgtgccgtcgaagcggctgcttgcgaacgtcgaaggcgccatgaacgccgtcgtcgtgcatggcgatgccgtgggcaccacgctttactacggcaagggcgcgggcagcgagcccaccgccagcgcggtgatcgccgacctcgtcgacatcacgcgcctgcacacggccgacgccgcgcaccgcgtgccgcacctggccttccaccccgatgccatgagcgacctgaaggtgctgccgatggccgaggtcgtcaccagctactacctgcgcctgcgcgtggccgaccaggccggcgtgctggccaaggtgacgggcctgctcgccaccgccggtatcagcatcgacgcggtactgcagcgcgaagccgacgaagtcggcggcgaaggctccacccagaccgacctgatcatcctcacgcacgacgcgcgcgaaggcaccgtgaacgacgtgctcgccgaactgcaggcactgcccaccgtgctgcagccgatcgtgcgcatccgcaaggaagagctgtcctgagggcggcgcaagagaaccaccgtgaactacctgagcacccgcggccaccccgaccgcaagcgtttttgcgaaatcctgcttgaaggcctcgcgcccgacggcgggctctacctgcccgatcactatccgcaggtcgatgccgccacgctcgcgaaatggcgcaacctgccgtatgccgaactggcgttcgagattctgtcgctctacatcgacgacattccgccggccgacctgaaggcgatctgcgccaagacctacacgcccgaggtgttcggcaccgaagagatcgtgccgctgcgcgagctcgaagacggcgtgtacctcgaagccctgtccaacggccccacgctggccttcaaggacatggccatgcagctgctgggcaacctgttcgagtacgaactggcccgccgcggcgccgagctcaacatcctgggcgccaccagcggcgacaccggcagcgcagccgaatacgcgatgcgcggcaagaagggcgtgcgcgtcttcatgacctcgcccgacggccgcatgagcccgttccagcaggcgcagatgttcagcctgcaggacgagaacatccacaacattgccatcaccggcgtgttcgacgactgtcaggacatcgtcaaggcggtgtcgaacgacctgggcttcaagcgcaagtaccgcatcggcacggtcaactcgatcaactgggcgcggctgctcgcgcaagtcgtctactacttcgccggttatttccaggccacggcgagcaacgacaagccggtgagcttcaccgtgccgtcgggcaatttcggcaacgtctgtgcgggccacgtggcccgcatgatgggccttcccatccagacgctggtggtcgccaccaacgagaacgacgtgctcgacgagttcttccgcaccggcatctaccgcgttcgcgcggcggccgacacgcatgaaacctcgagcccgtcgatggacatcagcaaggccagcaacttcgagcgcttcgtgttcgacctggtgggccgcgacgccgccaggctgcgttcgctgttcgtggacgagctgggcggccagggccgtttcgacctgagcggcgatcccgccttcaggcaggctgcggagcgcttcggcttcaagagcagccgcagcacgcatgccgaccggctggccaccatccgcgacaccgacaagcggtttgccacattggtcgatccgcacacggccgacggtctcaaggccgcgcgggaacacctcgcgcccggcgtgccgatggtggtgctcgaaaccgcgctgccgatcaagtttgccgccacgctcgtggaggcgctcggccatgagcccgcgcggccggcgaggttcgaaggcatcgaggcgctgcccaagcgggtcgtcaagcttccgtccgatgtggaagccgtgaaggcctatatcgcccagaactgtgattgacctttgccgcacgccgcgcatggcggcggctgcctcgcaactgcatctgcattcggctgccgcgtagacggcagtcacaggaactcgacatgaaggtgatcggcttttccgggtattcgggttcaggcaagaccacgctggtcgagcgcctgatcccggtgctcaagctccatggccagcgtgtgtcggtggtcaagcatgcgcaccacaagttcgatatcgaccatccgggcaaggacacctatcgccaccgcgaggccggggccttcgaggtggtggtggcatcggacaagcggctcgcgctgatccgcgaattcgagcagcccgcgcagctgacggtgcacgacctgatcgcagagcttcatgacggcgtcgactgggtgctggtcgaaggcttcaagcacagcgacctgctcaagatcgaagtctggcgcgcccccgatgcgggccagccgccccggccttcgaagtacatcgaagacgccttcgtgaccgccattgccaccaacgcgcccgcgagcctgccggcgcccaccaacctgcccttgttcgacctcgacgacatcgagggcatcgcgcagtggttgatcgacagcggcagccgcttcgaatacaaccccgaacaccatggctgattctgctgtcacttcgcgccccccgctgatggcgctcgacgaagcgctggcaagcctgctcgagaaggcgcagcccaggctgcccgccgaaagcgtcgccacgttcgacgcagacggccgcgtgcttgcgcaagacctggtgtccgcgctcaccgtgccgccccgcgacaacagctcgatggacggctatgcggtgcgcgtcgccgactgcgccgcccccggtgcggtgctccaggtggcgcagcgcattcccgccggttccgtgggcacgccgctcgcggccggcaccgcggcacgcatcttcaccggcgcgcagattcccgaaggcgcggatgccatcatcatgcaggaagacacgcaggcgttgccacaggaaggcaccctgggcgcggtgcgcatccagaccgttcccgccgccggccagtggattcgccgtgcgggcgaagacgtcgcgtccggcgacgtggtgctgtgcaagggcgagcggctgacgcccgcggcgctgggcctcgcggccagcgtgggtttcgactggctccaggtggcacggcggccgcgcgtggcgctgctctccaccggcgacgaactggtcatgcccggcgaagtcacgcccgaggccatgaagcccggcgcgatctacaactccaaccgcttcttcatgcgcgccttgctgcaccggctcggctgcgaggtgaacgacctcggtatcgtgcccgacaagcgcgaagccaccatcgaggcgctgcgcggtgcggcgaagaacagcgatctgatcatcaccaccggcggcgtgtcggtaggggaagaagaccacatcaaggcggccgtgcagacgctcggcgaactgcagttgtggtcgctctcaatgaagccgggcaagcctttcgcctatggctctattccgagggccgggggcgaatcgcaaggccgctgccacgtcaccgggctgcccggaaacccggtgtcgagcttcctgacctttctgctgctcgttcgccccttcctgctgacgctgcagggcgccacgcgtgtggcacccgagcccgtacagatgcgtgcggatttcgactggccgcgtgccgacaagcgccgcgagttcctgcgcgcgcggcgcaacgctgcaggtgggctcgacttgttcaccaaccagagctcgggcgtgctgacgtcgatggtctggggcgatggcgtcatcgacaacccgccaggccagaccatcaaggcaggcgacacggtgaagttcattcccttggcctcgctgctggcctgaggcgcatccatgaaagtccaggtccgttactttgcctcagtgcgcgaggcgctcgacaccagcggtgaaaccgtggacaccgccgccgccacgttggccgcattgcgcgacgaactcatcgcccgcggcggcgcttacgccacggcgctcgcacgcggcaaggccgtgcgcatggcactcgaccaggccatgagcgacgaggcggccgcgctgcgcgagggctgcgaggtcgccttcttcccacccgttacgggcggctgagccgggcgttcaacgccaccaggcgttcgcgcaacgcgccggatgcgcgggtcatcggcgagcgcagttcgtcgctcatcgatccgccgtgtgccagcagtgccttgagcggcccggggttcggttcggcaaacagcatctcgatcagcggctgcagcggctgccattcggcgcgcgcttccgcgagccggttttcggccagcaggcgcagcaccttcacgaagcggcgcgtctgcacatgcccgctcgccgcgatggcacccacgccgccctcggccaccgtgccgaagatctggtggtcttcaccggagagcacctgaagcctgccgtcggcgatcacggcgcgcgtcttggccatgtcgccgccgcagtccttgatgccgcggatgcgcgggtgctcggccagggccagcagcgtttcgcgtgcgagggtcgcgccggtgcggtagggaatgtcgtagatgagcaccggcgcagcgctggcatcggcgatggcgcggaaccattcgagcagtccggcctgcgagggccggatgtaatgcggcgcgggcaccagcagccccgccagcggacgttcggccagccggcgcacccgggccgtcgtcttgcccaggtggtagcccgacaggcccatgacgatcggcagcccctcggcggcagcttgcaccgtctcgagtgcggcgagctgttccgtttcgtcgagcgcggcggcttcgccggtcgaaccgcagaccacgaagccggccacgccgtcgcccgcgagccgatgggtcagcgccgagagtgcggcatggtcgatggcgccgccgcgaaacggcgtgacaagaggaatccagaggcccgagaaatcagggcgggaggaggggtgagatggttgcggcacgcgaggcttccttacgggaatcgaccgatggaaaagaaccgtcgttcgatgcgcgcgcaacccaatcgggggccaaggcctttgcaggttccgtcgctcatccgacgacggaaccgcagctccggtcagacgagcttgggtttttgggctttgctgccctggcgcgcagcgctgctttcaaggtgcgaaagcaccgtggagagcgtggcgaggcaaggcattgccgaagtctagcgcggtgccacaatcccggcatgagtggtgcacgcgtttcgatccagacagccgatttcgacctgggacaggaggtcgccgcgttgcgtgccggcgacaaacgcgtgggcgcggtctgcagcttcatcggcaccgtcagagatcgcaatgacggcagcaccatcgcctctatggagttggagcactacccgggcatgaccgagaaggccatcgaggccatgatcgacgaggcgcacaagcgcttcgacattttgggcgcacgggtgatccaccgcgtgggcctgctgcagccgctcgaccagatcatgatggtggccgtcgtctcggcccatcgcggccagagcttcgaggcctgcgagttcctgatggactatctgaagacccaggccccgttctggaaaaaagaacagacgcccgaaggcgcacgatgggtggatgcgcgcgtcagcgatgacgcggccctggcgcgctggggcatcacggccaacaacgcttgattctcttttccctctccctctgggagagggcagggtgagggagcagcggccttcgttgagcgccgcgcctagtcggcggcacagtgccctcaccccaaccctctcccagagggagagggggcaagagaactcagaggggcttgaaaccgctcgactggatgatccgctcccaggtctgcgtgtaagtgcgcacgcggcctgcgaactggccttgcggctcgtacgccacggtgaggcccatcgtggtcagcttctgcttcacgtcgggcatcgccagcaccttctgcagcgcatcgccgtacttgtcgatgatcggctgcggcgtgcccacgggggcgaagatgccgtagtagggcaggtcttcaagattggagaagcccagttcggtgaaggtcggcacattcggcagcacggcctggcgcttggcgccgatcgaggccacgatgcgcaccttgccggccttgtggttctctatgaagtcgggcaccgaggcgattccggcagtgatctggttgcccagcatgtccgccgtcatcggcgcgctgccgcggtagggcgcgggctgcacgtcgatcttgtatttttccgagatcatcttcaccaggaactcgggaatcgaagccggagccgggatgccgatggtttccttgccgccgcgctgggtgcgaacccacttcacgtactcatccatgctcttggccggcgtgccgcccgagacggccagcacattggcaaaggtggcgaatccggccacgggcacgaagtcggtcgcggggttgaagcccgggttcttcaccacctgcggcaggatggaaatcgagtggtcgtgggagaggaacagcgtgtgcccgtcggccggcgccgccttgagcgcctgcgccgcgatctgcccgccagcgccggcgcggttctcgaccaccaccggcacgcccagcacgtccttgagtttttcgccgagtgtgcgtgcaatggcgtccgagccggcaccggccggaaatccgaccagcaggcggatgggcgtgccttgcgcctgcgcaagacccgcgaggcccatggccgctacaaagaggccgacgccgagcgcccggcgaaccggatgggcgcgctgcattgaaaaaaccatgatcgactccattcgaaagatgagcaggcacagtgcaatagacgtgcccgaagccccgggcaccttgaatcgcgcccgaacagtcctattttgagtgcaggaacaccaccatgcgacaagacaaactcaccaccaaattccaggaagcgctgggcgatgcgcagacgctcgcgctcggcaacgacaacgcctacatcgaaccggcccacctgctggtcgcgatgctgcgccaggaagacggaccgcgcgccttgctggaacgcgccggcgtcaacgtccacggtcttgcgaacgcggccgaagccgccatcaagaaactgccgcaggtgcagggccacgacatcgtgcaggtcgggcccgaactcggcaagctgctgcaggccaccgagaaagaggccatcaagcgcaacgaccagttcattgcgggcgagctctttctcctggccgtggccgacagcaagtcggacatcggccgcatcgcgaaggaaaacggcctgacccgcaagtcgctcgagtccgccatcgatgccgtgcgcggcggccagggcgtgaacagcgccgacgccgaaggccagcgcgaagccctcaagaagtactgcctcgacctgaccgagcgcgcccggctgggcaagctcgacccggtcatcggccgcgacgaggaaatccgccgtgccatccaggtgctgcagcgccgcaccaagaacaacccggtgctcatcggtgagccgggcgtcggcaagaccgccatcgtcgaaggcctggcgcagcgtatcgtggctggcgaggtgcccgagtcgctcaagggcaaaagggtgctgtcgctcgacatggctgcgctgctggccggcgccaaattccgcggtgagttcgaagaacgcctgaagaccgtcttgaacgaactggccaaggacgaaggccagaccatcgtcttcatcgacgaactgcacaccatggtgggcgccggcaaggccgagggcgcgatggacgcgggcaacatgctcaagcccgcccttgcgcgcggcgagctgcattgcgtgggcgccaccacgctcgacgaataccgcaagtacatcgagaaggacgccgcgctggagcgccgcttccagaagatcatcgtgggcgagccgagcgtggaggcgaccatcgccatcctgcgcggcctgcaggaaaagtacgaagtgcaccatggcgtgcagatcaccgacccggccatcgtggccgcggccgagctgagcgaccgctacatcaccgaccgcttcctgcccgacaaggccatcgacctgatcgacgaggccgcggccaagatcaagatcgagatggactccaagcccgaagtcatggaccggctcgaccgccgcctcattcagctgcagatcgagcgcgaagccgtgcgccgcgaaaaggacgaggcctcgcagaagcgcttcaatctcatcgaagaggaaattgcgcgcctgcagaaggagatcgccgactacgacgagatctggcaggccgagaaggcgcaggcgcagggcagcgcgaagatccgcgaggacatcgacaagatcaagttcgagatcgaggaatggaagcgcaagggcgacttcaacaagctcgccgaactgcaatacggccagctgccggcgctggaaaagcgcctgcgcgaggccgaggagagcgaggcgagcaagggcaagtcgagcgcgcccacgctgctgcgcacgcaagtcggctcggaagaaatcgccgaggtcgtggcgcgtgccaccggcattccggtcgccaagctgatgcagggcgagcgcgacaagctgctcgtcatggaagacaagctgcacgaacgcgtggtggggcaggacgaggccatcggtgcggtcgccaacgcgatccgccgctcgcgctcgggcctttccgatccgaaccgcccgaccggctccttcctgttcctcggccccaccggcgtgggcaagaccgagctgtgcaaggcgcttgcgggcttcatgttcgacagcgaagaccacctcatccgcatcgacatgagcgagttcatggagaagcattcggtcgcccgcctgatcggcgcgccgccgggctacgtgggctacgaggagggcggctacctcacggaagccgtgcgccgcaagccctacagcgtggtgctgctcgacgaggtcgagaaggctcaccacgacgtgttcaacgtgctgctgcaagtgctcgacgacggccgcctgaccgacggccagggccgcaccgtcgacttcaagaacaccgtgatcgtgatgaccagcaacatcggttcgcccatcatccaggccatggtgggccagccggccgaggagatcaaggaagcggtgtgggacgagctgaagaactacttccgccccgagttcctgaaccgcatcgacgagacggtggtgttccatgcgctcgacgcgaagaacatcgaatcgattgccgcgatccagctcaaggtgctgcaggcgcggctcgcgaagatggacctgggactcgaggtgtcgcccgcggcgctggccgagattgccaaggtcggcttcgacccggtgttcggcgcacggccgctgaagcgcgccattcagcagcgtatcgagaacccgctctcgaggctgctgctcgacggcagcttcgggccgaaggacacgatcgaggtgaataccgacccgatccggaccccgggccagttttcgttcaccaaggccggggaaccatcggaggccattgcggcctaaagtcggatgatgaacttcatttttcgcgtcattcttctgctccttggcctggttttcgcggccagcctcgcggtggcggtcatgctgcttgcggctgtgtggggcgtgcgctacgcctgggggcgcatcacaggtaagcccgtgacgccctgggtggcttcgatgggcgggcgtttcaacccgcgctcgggcttcgagcgttttcgcaatgcggcacaaccggccgagcccactgccgccgacatggccaatgcgcgtgcgcgcggcgaatccgtcgtgcgcccggagcgcattcgcggcagcgccagcgacgtgaccgacgtgtctccgaaatcagtctcgcgcggctgacccgccgcgcctgggcggggatatgccgcccgcgacagccgggttgcgccgttcgccgtcaaaatcgtcctcctgcgaccgctgccataggcggatcccgctttcatccaggagagacattcccatgacccaacgcgacatcttcgtggtcggcaccgcccgcaccgccatcggcaccttcggcggcgcgctgaaagacgtgcccaacacgcaactggccaccaccgccgtcaaggccgccatcgaacgcagcggcgtggcggccgatgccatcgggcacgtggtgatgggcaacgtgattcccaccgacgtgaaggacgcgtacctgagccgcgtggccgccatcgatgccggctgccccatcgagacgccggccttcaacgtcaaccgcctctgcggctcgggcttgcaggccatcgtgtcggcggcgcaggccattgcgctcggcgactgcgacatcgccatcggcggtggctccgaatcgatgagccgcggcccgtacttcgacacctcggcgcgctacggcgcgcgcatgggcgacgcggtgctggtcgactacatgctgggcatcctgcacgacccatgggagaagatccacatgggcatcacggccgagaacgtggcggcgcgctacggcatcacgcgcgagcagatggacgaactggccgtggtcagccagcagcgcgcggcagccgccattgctgtggggcgcttcaaggagcagatcgttccggtcgaagtgaagacgcgcaagggcatcgtgctgttcgacaccgacgagcacgtgcgcgccgacaccacggtcgacacgctcgcgaagatgaagcctgcgttcaagaaggacggcctcgtcaccgccggcaatgcctcgggcatcaacgacggcgccgccgccgtggtgctggccgaaggcggtcgcgtgaaggcgctggggctcaagccgctggcgcgcctggtcggctatgcgcacgcgggtgtcgagcccgcgtacatgggcatcggcccggtgccggccacgcgcaaggtgctggagcgcacgggcctgaaggtcggcgatttcgacgtgatcgaatcgaacgaagccttcgcggcgcaggcctgcgcggtcatcaaggagctgggcttcgatccggccaaggtgaatccgaacggctcgggcatttcactcggccacccggtgggcgcgaccggcgcaatcatcacgaccaaggcgattgccgagctgcaccgcactggcggccgctacgcgctggtcacgatgtgcatcggcggcggccagggcatcgccgccgtcttcgagcgcgtttgaaggcacacttgcggacatgctccgcccacccctcctgatcgaccccgacgaggtcgagatcagcgccatccgggcgcagggcgcgggcgggcagaacgtcaacaaggtgtcgagcgcggtgcatctgcgctacgacattcacgccagctcattgcccaccgacgtgaaggagcggctgctcgcactgcgcgacagccgcatcacgcaggaaggcgtcttcgtgctgaaggcacagcagcaccgcacgcaggagatgaaccgggccgacgcgttcgcgcgcctgcaggcggtggtcgacagcgtggccgcgccgccgcgcgtgcggcgtgccaccaagcccacctatggttcgaagcagcgccggctcgaaggcaagagccagcgttcgcagatcaagaacctgcgcggaccggtgcgggactgaccggctttccgccgcgcagccgcctgatctgcagcgtcacgccgaccagatacagcacgcccagcaccgcggtgatcgccttgagttcgggcgcgtcggcgttcggcagcaggggcgcgcccagcggcaggcgagtcagggtttcggtgaaggccggaatccagtggaacaggaagctggccgagaaagccacggcttcgacgtagcgcgaggcctggccgaagaaggcgccgcggccggctgccgcacccacggccagcgccgcgagcgtcaggatgcccagcgcatgcggcttgccgaaaccgccgtgctggaagatgccgaagccggtcaggcaggtcagcacggtggtccacacgaagacctggcccaggccggtgcgcagcgtgatttccttgtggcggaacagggccatcagccccgcaatgacggcgatcaggctgatcgcggtgtgaacaatgccgagggacgtgagtcccagccatccggtcgctgccatgcggaactcctcagaatcgtggtggcgcgattctggccgcgcgcgggcaatttgtctccatcattaaggctccactaagctgggggacatgggccgcaagcacaataggagccatgagagccttcttccgccgcgctttgccggcttttctgctggcgctgggtgcggctgccctggcgggctgcggcccggccgccgacaccagcgcggctgccatgggcgcggtgcaggaactcaagtgggaagagctcgttcccaagaactgggacccgaccaagcgctaccgcaacctcagcctggaggcgctgcgcgacaacgacccgcgcgccatccagatgctcgacgagatgcgtgccgtctgggacaacgcgccggtcaacgtggcgctcgacggcacggcggcgcgcctctcgggtttcgtcgttccgctcgacaacacgcagggcggcattcgcgaatttttgctggtgccgtatttcggcgcctgcatccacaccccgccgccgcccgccaaccagatcgtgcacgtgattgcagccgacaccgtgaagggcctgcatgcgatggacacggtgcgcgtcagcgggctgctgaaggcggcgcgctattcctcggtggacatgggcgtgagcggctatgagatcaagtcggcttctgtggaatcttttgtcgcggcgcgctgatccgcttcccgctgtgccagcgccgccagcgcctcggcatcggtgcggtagctgaaaagcatcggtcccggcccgagcagcccggcacgctccagcacctgcatggccggcagcttcaggccgctcaggtgcaggcgcacgcccttggattccatcatccggcggatcgagccgaatacttcggcgcccgtgatgtcgatgcggttgatgggctgcgcaaagaggcacacgtccgtcagatcggggcgctcggccagcgcaaccgtgagcgcgcgctcgagcgtggaagccgatgcgaagtcgagctcggcgtccatgcgcagcgcgtagagatgcggcgccagcggcggcaacttccagaggtggcgatcgcgcaggctgccgtcgggatgcaggcccacctcgatgatgcgcggatgcaggtggcggtacatgtagtgcgccatgctcgcgagcagtccgcccagcacgccccagtagatgctcggcgcggtggcaatggtcagcgcgaaggtaccgaacgcgatgcccgcctcgatgcgcgacacgcgccacaacgcgacgaagctcgcgggcttgaccagccccagaatggcagtgaccaccacgcccgccagcaccgcctgcggcacgtggtagagcagtggcatcagccacagcagcgcaccggccaccaccatcacgctgaacagggtggcccacccggtctgcgcgcccgcatacagcgtgatggccgagcgcgagaacgacgagctggtgggaaaggcgcccgagaaacccgaggccagcttggcgaggccctggccgatcaggtcctggttctcgttccagagcgtgccggcccgcgcgttgtcgatcttggcgctcgacgcggtctccagaaagctcaccaaggtgatcatcagtgcgggcagcaccagtgcgctgaacgtgttcaagggcagcatgcccggccagtagaaagagggcaggccagaaggcaggctgcccaccacggccccgccgcgcaacgcgtagttgaccgtccagctgatggccgcggcgcccgccaccagcgccatcgtgattggaaaacgcggcgccagccgcttgcccagccacagcacggcgatgctgcccagcccgaaggcaatggcgacaaggtctggcagcgggccgccccgcagcacttgcggaatggtgcggcccgtgaagccgagcaacgccggcaactgcgaaatggcgatcagcaccgccgcgccctgcgtgaagccgatcagcaccggcgagttcaccagccgcagcagccagccgaaacgccccgcgcccagcaccatctggatggcacccgacatcagcgtgagccacaccgccatggccacccaatcggtgctgccgggcaccgccagcggcgcgagcgaggcgcccaccagcaggctcgtgagcgcggtgggcccgaccgacagccgctgcgacgaactgaagatcaccgcaatcagtgccgggaacagcgccgcgtacacgccggtgaccagcggcatgcccgccagcgccgcgtaggccacgccctgcggaatgaccatcagcgccaccgtgatgcccgccatcgcctcgttgcgcagcagcgcggcggaagggcggggccatgcgaggcagggaatccagcgcgcgaggcggcggcgcaaagaagaagaggaggaagtgggggctgccggattcatgaagcgttacgagcgcacgaaagagaacggaagagcacatgcgcggtgcgccgcgcgcgtggcacgcaggcgcgttgtcagatcagcgaggtggcgtttttcagcacatagtcgcaggccttcaccttcagcttcgacgagagcatcttgaggttgagcgtcttgccgtcgccgcccttgagcaggcccttggcgccgctctcgaagttcttttcctgctgcttctggccggtgatcttggccaggagcttgtccttcaccgaggccgcatcgccgcccaggtagttgttcttgacgcagtactgcagcaccccggccgcgctgccgatggtgctggagccgatggcgggcatcttgaagccgaggttgccgagcgccgagccggcctggtctttcagctggccgaggaggtccgactgggccaagaccgtgccgctggccgcgaccagcgcgagagaaaccagtgcggagcgaaagcgcatgacgaactcccgtctgtggatgtgaatgaagattccatcgtcagcatacccccgacggaatccggcctcacgcgcggcgaaagagcagtacggaattcgtgccgccgaaagcgaaggagttgctcatggccgcttcgagcgcaggcgcgcccgtgtcgttctgcctcaccaggttcaggctgcaggccggatcgatatcgctgcagttggcattgggcggcaactgccggcggtgcagcgcaagcaccgtgatgagcgcctcgatggcgcccgccgcgccgagcaggtggccgtgcagcgccttggtggagctgacgcgcaactgatcgaggtcgtcgccccacacgtccgccagcgcattgcgctcgaccacgtcgccgatgcgcgtggccgtgccgtgcgcgttgcagtagcccacgtcgcgcggctgcagcccggcctggcgcagggcggcgcgcaatgcgcgggcctggccgggagcgtcgggcttggtgaggtgcgtggcgtcgctgctgaggccccagccggccaaggtggcatagctgcgggcgccgcggctgcgcgcgcgttcggcggactcgagcaccaggaaggccgcgccttcgcccagcgcaaagccgctgcggtcgctggcaaagggccgcaccgcgccggctgcttcgccgggctggaaggtggccagtgtctgcatcgcctgccaggccagcaccacgccgggcacgataagcgcctcgctgccgccggcaatggccaggtcgacttcgccgcgctggatggccttggcggcttcggcaatggccaccgacgacgaggcgcaggccaccgaataggtgagcaccggcccctgcacgccgtggcgcatggccacgtgggcggcgggcgcattgggcatgaaggcgggaatggtgagcggcgacacgcgcccattgccgcggtaggccgcctcgagtgccgcggcaccgcccatgccgcagccggcatagacgcccacgcgctcgggatcggcgtcgctcgtggcaaggcccgcgtcgcgcatcgcgaggtcggccgccgccacggcaagctggctcacgcggtcgacgccggcgagctgcagcttggtgaaccagcgtgtttcgtcgaaagcgaccgtggccgcggcggccggcttgggcaggtcgggaaagatgggctggatggccgattggccgtccagcagggcctggaacagcgtgccgggctcgccgccatgcggcgccatgacgcccagtccggtgacgcagacctcgtggttcacgctgtcttcgcggacctgaccctgtcgaccagcagggccagttcgcccagggtgtcgatgttcgcgtcgtcgtcgggcatggtgatgccgaagtgatcttcgatggcaaacaggaactcggccaatgccagcgagtcgagcccgccggtttcacgcatcgatgcgttggggtcgagcttcgacggttcgataccgtacttctcgtggatcaggtcctgcaattccttcagcgaactcatcgtgcgatgcctgtcgtcttgtactagccgctgatcgatcgccgcccgggggcgctcctttggatcgaccccttcctcgctcggcttgtgggtcagtgatgaccaatgatatccgctccaaccaatgtattgccccggctcctgccttccggacgccagcgcagcgacgggagtgcaaaggccattcccagcagggcgccggccagcgcgtcgagcaccacgtgctgcttgacggccagcgtcgaccaggcaatggcggcgaaccaggcccagttggcaagccgcaggaacgacggcgtgcgcgcctcgcgcagcacgtggtccagacggatggccgtgaagatggccacggccacgtgcatcgaggggcaggcgttgcccgcggcatccacgccctgcagcatggcaaagccggggtagcccgacacgtcgatggcaagcggcggtatctgcgtgggccagaagtagaagaggcccaggccggtgaggcacagcgcgccgatccacagcccatagaccaccagttcgcgaaagctcagctgcagcccgggcgcgatgcccacatagaaccagagcgaaaggtaggcgcccagtgcatacggctggaacggaatcaggcggtcgagggccgtgagcggcatcaccgtgaccggataggccggattgcgcaacagatgaaagtagccgatgaagaaaagccaggtgaagaccgtggtgccgatcgccttgagccagaagaggcggcggatccgctcgccgacgtcggtggtccaggcctgggggcgatgcgatcgggggaggggcgccatgggcaggtcggtcgggtggtccgtgtttcttcggcccttcgatcttgccagagcgccgtgacggcctggcgccattcaggagagggcggcggatcgcttccggtgctggaacgaagtgggcgagcgccccgtggccgccttgaacatggcgcagaacgcgctgtcagtggcatagccgctggccgccgccacctggctgacggccatgccgcgcgccagcagcggcagcgcgtgcgccatcacggcctgttgccgccattgctgccagctcatgccgagctggtcgcggaacagccgcgccaccgtgcgctcgctggcgccgatggtggcggcgcgctcggccagcgtggcccggtcggccggattgcgcagcagcgtttcgcacagctgccgcagccgcttatcggtgggcagtggcacgtcgatgcggatttgcgtggcgcgctccagctcgtccaccagcagcggggcgatcatgcgttcgcgctgcggcgcatgcgggtcggccggcggcagcccgtcaggggtggtgtcgagcgcgagcatcagcgcgcgcagcagggggctgatttcgagcacctcgcacttttcccacggcggtccgagccaggcatgcaggtacacggtgcgcagctccgcgtcttctatcagcatgatgctgtgcggcatgttggccggcacccagaccgcgcgcgacggcggcacgatgtagctgccatcctgcgtgctgagccggatcacgccgcgggtcgagaaggtgagctgcggccacggatgctggtgcagctcgacgaaagtgtcggcgctcaggaagtgttctttcgcgcgcagcggccgcacggcgtcgggtgcgtagaggtgcggcgtgagcgaggccacgctggtgaccggggaaggggtggaaacggcgcttggcatagtttcgacaaatgttgtcgctgtatcgccattctgccgcggcctgcgcgcatagcatcggtgcctgccccggttttttgtagcaatccatgtcttcaacttctactccgacagccgcttcttccaccaacttgcgcggtgacgcgcagctgatcggactggtcggcctggcccatgccatcagccacttcagccagctgatcctcgcgccgctgtttccctggctgaaggacgcgttcaacgtcagctacaccgagcttggggcggtgctgacggtgttcttcgtggtctcttgcatcgtgcaggcggcctcgggcttcatcgtcgacaagctggggccgcggccggtgctcttcgtggggcttggcgcgctggcgctggcggctttcggctatgccctggcccagagctactggatgctgctgctgtgcgccatcgtgggcggcatcggcaacggcgtgttccacccggtcgactacacgctcttcaaccgcaaggtcgcaccgacgcggctcggccacgcatacagcgtgcacggcatcaccggcagcctcggttgggcgctggcgccggccttcgtggtgccgattgccatcgccttctcgtggcgcgtggcgctggcatcggcgggggtgctggccatcgtggtgctgctggtgctctgggcgtatcgcagcgtgctctctcttgacgtgaagacggtgcagaaggccaccggacacggcgaaccggcgcccatcggcggcgagttcgacttcctgcgcattcccgccgtgtggatgtgcttcggcttctttttcttctatgccgtcgtgatcagcgtggtgcagaccttcgccccgggggcggcaggccacctgcacgcggtgccggtggcgctggtggcggtctgcctcacggtgtacatggtggccagcgcggctggtatggtggtgggcggctttctcgcctccgacccgtcgcgctgcgaacgcatcgtgggaaccggcttcggcattgcggccgcgttggcgctggtgctcgcctttgcgcagtttccgccggtgatggtgccggtgctgttcggcgccatgggcttcgtctccggcgtggccgggccttcgcgcgacttgctggtcaagcgttcgacgccgcccaacgccaccggccgcgtctatggcgtggtgtatgcgggcctcgacatcggacaggccgtggccccgctggtgttcggccgcctcatggaccacgcgcaatatacgagcgtgatcgtcggccttgcactggtgcaggccgtgctgatcgccagcgccttcaacgtgacgcgggtgcgccgcacggcgctggtgccggcctcggcctgagcggttcgcgcttgcccgggatgcggtcgatatcatcggccgcatgcaggccttgtatgtgtatgtgatcgccggtgccgtgctggcgggttttgtgcagggcctgtcgggctttgccttcggaatggtcgccatgtcggtctgggcctggaccctcgaaccgcaactggcggcggtcctcgccctgttcggcgcgctcaccggccaggtgattgccgccgtcacggtgcgccgaaccttcgacaggcacgtgctgtggcccttcgtgctcggcgggctggtcggcgtccctttcggcgtgtggctgttgccgcacctcgacctcgtggtcttcaaggtctgcctcggtgtgctgctggtgctgtggtgtcctgccatgctgctgtcgcagcacctgccgaaggtcaccttcggcggacgaatcgccgacggcatcgcagggagcatcggcggtgccatggcgggcatcgggggcttctcgggcaccattcccacgctgtggtgcacgctccgcggctttcagcgcgacacgcagcgcgcggtgatccagaacttcaatctctcgatgctgatggtggcgttcgcgatccatctcgcgagcggcagcatcggccgctcgatggtgccgctgctggggttggtggcgctggccgtcgccgtgccggtgctgttgggcgcgcggctctatatcggcatcagcgagacggcgttccgcaaggtggtgctgggcctgctgacagcatcgggcgtggcgatgctggcttcgggcgtgcctgcgctgctgcagcgcgcctgagcgccggctcggctacgccgcgggcaagatctcgcgcacgcgtgcccagggccggcacatcagcgtgccgcgcggagagacgacgatgggccgctgcagcaggatcgggttcgcgacgatgaagtcgaacagctggtcgtcggtccatttcggatcggccagccccagctcctcgtagggcgcttccttcgtgcgcagcaggtcgcgcgggcccatgcccatggcctttgccaactcacgcagcttcttcttcgtgggcggcgtctccaggtaaagaacgatctcgggctctacgccgctctcccggatcaagcccagcacattgcgcgaggtgctgcagttgggcttgtggaagatggtcatcgggtaggcggtggtcggcgtgcgtgcggtcatgtctccgggtccatcgagaagggatagcgcaccgcccagaactcggccaggcgcggatcggcatcgacgcgccgcaccacgccggccatgcgcggcgcttcgcggtagaagcgggtgcggtgcggcgtccagcgcgacagcaccgtgacgtacaggtcgagcatgctcagcttctcgccgagcaggtagggcgcgggttcgtcgatctgcgtgtccatcaggtgccagcagtgggctatgcgctcggccgtgcgttcgagcatcacggcctgcgctgccggatcgggcgtgaggcgcgtgggttcgtcgcgcacccagtacatcgaatagatcgccgccggcaggtagaccatccagcgcaggtagcgcgcacgcagcggatcgtccggcgcggggcaaagccccgcttccggatagcgatcgccgagccagatcaggatggccgcgctctcggtcatcacctcgcccgaagggagcaccagcgcgggcacctggcgcatcgggttgatgctcgacacgcgctcgcgctcggactccccctcccagggagagacgtcgacgacgtcgacctgcgcgccgatcagcgtcagcgccgcatggacgggcgttgcgcccgagccgggtgcgccgtaaagggtgtagcggtcattcgaagcggatgaagaagccatccgcgcagattactgcagccttgtatcggttgtcacgcggccagcagcgtgtcgaccttcttcaagccttcgagcgtcttcacgcaggcttcggccacttcggtgcccttgacggcaaagtgccggtggaagtatttgcggtgctccacgtgctcgtggaaatggtgcggcgtgagcacggccgagaaaatcggcacgtcggtttcgagctgcagcgacatcagcgtgctgaccacggtgctggccacgaactcgtggcggtagatgccgccatccaccaccagtgcacagcccacgatggccgcgtacttgcccgagttggcgagccgcttggcatgcagcgggatctcgaaggcgccaggcacgtcgaacacgtcgatgaggtcgcgcgccacgccgagccgttccatttcggcaaggaaggcgtcgcgcgcctggtggacgatgtcggaatgccactgcgcttcgacaaaagcgatgcgctcgccgcgcgggttgcccgacgcgttgatggcggaaaggggaaggtcgttgatctgactcatggtgtgcctcttgcttgaaagcaggtttcctgaatcagggcgcacgaaaccgcaagccagaccgcgcgctccaatggaaagcgcgcgggccggcccgcatttcgcgctctctttcatccggactgtgaccgtcggcttcggaattgcaccgaaatctgctgaccccgcagcccattgcaggccgcgggcgctcgcgggctcgtgcggcccctctctcgaagaagccgccattaccgccggtggggaatttcgccccgccctgagaacgcttgccatccggcatgccggacgacgggccgattctagaagccagcggcggcgcgggttgtcgcccgtgcgccagaccttcagcggcgcggggattctgccggggcggctcagcggccggccaggaactgcgtcatgcggtgcaattcctcatcgagcgcttcgcgaaacgccgcgtcgtgcggcttcttgtcgacgtagccaaaggccggctgcagccggccctccggcgcgctcacgttggcccagccgatcacgcggtcgtgccagagcatcggcagcgcgtagtagccgaactgccgcttcggcgccggcgtgtaggcctcgaacttgtacgtccagccccacagcagctcgaagcggcggcggtcccacaccacgggatcgaagggggcgagcaggcgcaccgcgtcgtcgggcgcgtggcgcttcgaggccgggttctcgccggcgggccagtaccaggtggtgccgtcgattttgcaactggcgagttgttcttcgcgcgccaggcgaagggccgcctgcgtctgcgccgcgaggtgcggggcgccgtagccgagcagccgcacgaggtaggtcaggcttgcagcgggcagcggtgcgtacttgcgcaccaccaggtcgatgagcgcggcggcacgttgcgcgcggccggcggggctttcgtcggcgggcagatgggtcacggcctcatagacacgcgtgccgctgtcgcgccgcaccacgcgcagcatgccgcggtagtgcaagccgtcgagcaggcgcgtggtggcgttgctcgaaccgccccagtagttcttcacgcggccatgcgcgaagtactgttcaacttcgcgcggatgcaccggtccgcgttcgcgcacgaaggccaacacatcggcggccttgcggcgggtgtcctcgtcccagggctgcctggcttcgcgcggatgcatcagggccaggtgttcgcgcggcaaaaagccgtagttgacgaggcagtcttcctcgatggcaagccgcgtgtagcggctttcgagatcgcccgcgcggtagtccttcacgcggtggcgcagcgtcaggtcttgggcacgtgcgggcgcgcggatcgggtcggcctgaacgaagccgagttggcggatcgctgacggcagcgtggtcggcttgaagagggtgcgcgctattgcgtagcggcgcaggtcgtcgagggtcggggtggccatgggtgaattgcagcacaagctttgcggcgctgctgttcggggcacgctgctgttcagggcggcgctcccgccgacggggtaccttgctccgcgaatgtcccccggcctgcggcctcctcctttatttcgctgcgcaaggcaccccgccagcgggagcgttattcagtgcagtggttgatcagccagcacgacagccgcgtccggtgtgcgcagggcgccgggtgctccccgcagcgaaataaaggaggaggcgaagccgggggacattcgcggaggggagtacccggtggcctgtgcacgcgccccgaacaagagcggacaaaaggcaatctagacggcttgcttgtgccgctcgatacacacgtcgagcgtttcggcgcccgtccgctgccaccaatccaggttggaaaaaatctcgacctcgctgaaccccgcgaaccccgcgtcttcgacccaaccgcggatcttcttcaactcgaccacgccgtcgcccatcatcccgcggtcggacagcaaatcacgcgtgggcgtgagccagtcgcagacgtggtacgccaagaggcgttcgcggccggcgcgggcgatctgctgctgcagcttcgggtcccaccagacgtgatagatgtccagtgccacgccgagcatgccgctcttgcccgcgtccagctcgtcgcagatgtcgagcgcatgttcgagcgtgttgatgcaggcgcggtcggcggcttgcatcggatgcagcggctcgatggccagcggcatgccgactttgcgggcgtattcgagcgacgcggcgatgccgtcgcgcacctcgccacgcgcgcgggcaatgtctttgtacgcggccttgccttcgagcgcgccgggcagggcgccgaccaccagcacgaggcaaggtgcgtccagcgtcttggcttcgtcgatggcgcggcggttgtcgtccagcgcggctttcaggcccgctgcatcggccgccggaaagaagccgccgcggcagtagcccgagaggccaatgccatgcgccttcagctgctttgcaaccttgtcgagcccgacggcggccacctggtcgcgccaggggctgatcgcgcgaatgccgcgctcggcgcactggtcgatgatgcggtccagcggcacctcggcgcccagttgcttgcgaacggtcgcggtgttgatcgacagccagtcgtggttctgcgagaaatcgcgcatgggttcgctcagccttcaacgccgtgcagggccagcagcgtcttcatgcgttgcaccgccagttccgggtgttccagcagatttgccgcatcggccaggcggaacaactcggcaaagtgctgcagcgaacgcgtgctctgctggccgccgaccatcgtgaaatgcttctggtggccgttgagccaggccatgaacaccacgccggtcttgtagaagcgcgtcggcgctgcaaagatgtggcgcgacagcggcaccgtcgggccgaggattgcgtggaatttttcggcgttgccctgcgccagcgcgcccagcgcagcgctcgctgccggggcaatggcgtcgaagatgccaagcagcgcatcgctctggccatgcgtgggttcgctgccgaagccgtcgccggcaatcagctcggcgtagttgaagtcatcgcccgtgtacatgcgaacgcctgccggcaggcggcgccgcatcgcaatttccttgtccttgtcgagcagcgaaatcttgatgccgtccaccttgtgcggatgcgcggcaatcacggccagggccgtgtccatcgcggtatcagcatccttgctgccccagtagcccgcgagcgccggatcgaacatgtcgcccagccaatgcagcaccaccggctgcttcgactgactgaggatgcggtcgtacacgcgctcgtagtcggcggggctctttgccacgcgggccaatgcacggctcgccatcacgatcagcttcccgcccagcgcctcgatggcggccatctgctcttcgtagccgcggatcacgtcgtcgacgctcttcacgtcgtcgatgttcaggtggtcggtgccgcagcccgaggccaccagcgcgcccggcacgtccctggccgcatcgagcgaacggcggatcagttcgagcgaggtcggccagtccaggcccatgccgcgctgcgccgtgtccatcgcctcggccacgcccaggcccagcgagaacaagtgacggcggtaggcgatggtggtgtcccagtcgactgcagcttgcagccacgggtcgacggccgcgagcggatcggccaccacatgcgcggccgaataggcgatacggttgaacttggcgcccgcatcgggcttgaccggcgcggtgccgcgcagggcgtacggcgcgagcgagccgctcgcggtgggaaggatcagcgaaagtgccatgctgcctgcctcagaccttcagcgcgggcacgtcgatccagcggcgttccttccacgactcgagtgcggcctcgaccagctgcacgcccttggcgccttcgggcagcgtccacttgtagggctcgttctcgaccacgtggcgaatgaagtgctcccactggatcttgaagccgttgtcgtacgcctgcgaatccggaatctcctgccactggtcgaagaaattcatcatctgcttctcgtcggggttccacaccggacgcggcgtggccacgcgcgactgggcgcggcagctcgacaggccggccacggccgaaccgtcggtgccgtcgacgtggaaagtcacgaggtcgtcgcggcgcacccgcgtgacccagctcatgttgatctgcgcgatgaccggctcgccgttgtggccggtgagctcgcaggtggcgtaggccgcgtcgtcggccgtggcttcatacggcttgccggcttcgtcccagcgcttggggatgtgggtggcgccgaggcacgacaccgacttcacctcgccgaacaagttgtccagcacatagcgccagtggcacatcatgtccaggatcatgccgccgccgtcttccttgcggtagttccagctcggacgttgaatcggctgcaggtcgccctcgaacacccagtagccgaactccaggcgcacgctgagcatgcggccgaagaagccggcgcggcgcagcatgtcgagcttgcgcaggccgggcaaaaagagcttgtcctgcacggcgccatgcttcaggcccgagccttcagcgaggcgcgcgatctcgaccgcttcattgaggttggtggcgatcggcttctcgcaatacacgtgcttgccggcgcggatggccttggccagcagcgtggggcgcatctgcgtggtgccggcgtcgaagaagatcgtgtcgtccttgttctccagcgccttgtcgaggtccgtgccccagcgcgcgatgttgtgtgtcttggcgagcgcttccatcttctcggcgttgcggccgatgaggatcgggtcgggcatgaccctgtcgccgttcgacagcgtgacgccgccttgcgcgcggatcgcgcagatcgagcggatcaggtgctggttcatgcccatgcggccggtgacgccgtgcatgatgattccgagtcgttgtgtagccatgtcttcagccgaaaaggagttggagaaagtcaaagagaaaggaagggggcggattactgcgtcggcgtgaggccggcggccttgaccaacgtcgcgttggtcttgatctcgtccttgatgtaggcgtcgaactgctcgggcttgagcgtccaggcgtcggcgccgagcttcaggaagcgctccttgacctcgggcgaagccaaggccttggccacttcgtcgtgcagccggttgacgatgtcgcgcggcgtcttggccggcgccatcatgccgatccagaagttgaactcggagccgggcacgccggcctcggtggtggtgggcacatcgggcagggcggcggcgcgcttgggcgaacccactgccagtgcgatcaactggccgtccttgatttggccgatgaccggcgcgatgggcgagaagtagtagtcgacccggcccgacagcacttccgtcactgcctcggccgagcccttgaacggaatgttggtggcgtcgatcttcgcggccagcttgaacttctcggcgttgaggtgggtggcgctgccctggccggccgatgcgaagttgatggtgccgggcttggccttggccgccgcaaccagctcctgcagcgtcttgatgttcttcgcaggcgagatcaccagcgcattgggcagcgacgagatcggcgtgacaccggcgaagtcgttcaccgtgtcgaacggcagcttcgcgaaggtggaagggctcaccgtgtgcgacgacgagtgaatcatgaccgtgtagccgtccggcgcggccgtggccacggcctgctggccgatggtgccgctggcgccgccgcggttgtccaccaccagcgtctggcccatgctctggcccatcttgtcggcaatggcgcgggcaatgatgtcggtggtgctgccggccgcaaacggcacgatgacgcggatgggcttgttgggatacccgctctgtgccgacgccaggcccggcatcaaggcggcgaggcaggtgagcgtggcgagtgcagtggtgcgtacaagttgcttcatgggttgtctccgtgcggtcgggccgctttgtcttgccgattaattcaccagtgagtgaattgtagattttagaaaggctgccgccgcagcgcaaccgctgctgatcggtaaatacccggagatgcaggaaggcgcccgaagggctcagtgcagcacgtagcccagcacgaggtcggtcatgtgcgagaggcgctgcgccattgccttgggtgcgcgcaggtcacggccgaagacggccgagagcgtgtggttgttcgagaggtagaagtagcagagcgaggcgatcgagatgtaaagctgcaccgggtcgacgccggcgcgaaacagcttgtcgcgcttgccgcgctcgagcaccgtgtcgagcagttgcaccagcggcgagttcatttcctggatgcgctcggagcgcttgaggtgctctgcgcaatgcaggttctcgctgttcagcagcgtgatgaactcggggtgctcgaggtagtagtgccaggtgaacgagaccagctggcgaatggcctcgaccgggtcgatttcgtccaggtgcaacttttgctcggcctcgcggatgtcggcgtaggtgcgttcgagcaccgccaggaacaggtcgtccttgctgccgaagtagtagtagatgaggcgcttgttcaggcctgcgcgcgcggcgatgctgtccatgcgcgcgccggccaggccccgttcggcaaactcgtcgcgcgccgacgcaagaatcgcgagttgcgagcggtcggcgtcgcgcgagcgcggctcgaccgtttcgggcgggagatccttgggggctttcatggcgcgaatttaaccagttggtgaattaacgcaaggcgttgagagcagacgcacataattgccggagacatttgcagctgaggttcgacttctcatgagtacatcacaacccgccggccacctgatcgtcgaatgcctgatcgagcagggcatggagatcgcgttcggtgttccgggtgaaagctttctggcggtgctcgacggctttcatgcctaccgcgaccgcgcccgcttcatcgtcaaccggcaggagggcggcgcggccttcatggcggacgctcacggcaagctcaccgggcgaccgggcgtgtgcttcgtcacccgcgggccgggcgccaccaacgcatcgatcggcgtgcacaacgccttccaggattcgacgcccatggtgctgttcgtcggcgacgtgggaagcgacttccgcgatcgcgaagccttccaggaggtcgactacggcagtttcttcgggccgagcaccaagggctttgccaagcgcgtggagcgcatcgacgacgcgaaccgcatccccgaatacgtggcgcgcgcttttgccactgcaatgaacgggcggccggggcccgtggtgctggtgctgcccgaagacatgctgcgtgcgcagaccgcagcgcggcccctgccgcgcgtcgaagccgtgcagccctggagcgaccccggcgcgctgcgcaccctgcgcgagctgctgctcaagtccgagcggccgctggtgatcgcgggcggcggcggatggacggcgcaggccgcgcaggcgctgcagcgctttgccgagaactggcggctgccggtgaccaacgcctttcgcttccaggacaccttcgacaaccaccatccgctgtacgcgggcgacgtcggcattgccatcaaccccaagctggcgcagcgcgtgaaagacagcgacctgatcatcgccatcggcccgcggctgggcgagatgaccaccggcggctacacgctgctggaggcgcccaaggcacggcagaagctggtgcacatccacgccagtgccgaagagctcaaccgcgtctaccaggccgaccttgccatcaacgccggcatgagcgcggccgcgcgcagcctcgaggtgctgagcgcgcccaccaccctgccgtgggaagagtgggccgtgcaggcccatgccgactacgaggccaacctggagccgcaggcgctggccggcatgccggccgaaacgccgagaggcctcgtcgacatggcggctgtggtcgcgctgctgcaaaagcacctgccgccggatgcggccatcaccaacggcgcgggcaattttgcgagctgggtgcatcgctacttccgctatcacgggctcgcgaaaggccacaagacgcagctcgcgcccaccagcggcgccatgggctatggggtgcctgcgggcatcgccgccaacctggccaccggccgcgtggccttcaccattgcgggcgacggcgattttctgatgaccgggcaggagctcgccacggcttcgcagcacggcggcaagagcatcatcgtgctgctgaacaacggcatgttcggcaccatccgcatgcaccaggagcgtgaatatccggaccgcacgagcggcaccgcgctgcaaaaccccgacttctgcggccttgcgcgggcctacggctacgttgccgagcgggtcacggaaacctcgcagttcgaagccgcgctgctgcgtgcgctggctgccgacacgggcacgctgatcgagattccgctcgaccccgaggtgatcaccacccgcggcacgctcgcgtcgatcacgcgtgcggcccaggcgcgggcgtgagaagagcggcgcagcgagccggtgtgcgcgccggccgcggacaaaaaaaagccggcatgtgccggctttttgattcgggagcgcgatgaacgcgcagtgcccgagcgcttacttgacgtgcttgccgatcagagcggccagttcgaacatcgacacttgcggcttgccgaagatttccttcagcttggcgtcggcgttgatgttgcgcttgttggccttgtcttgaaggttgttcttcttgatgtagtcccacagcttgctcacgactgcggtgcgcggcagaggcgtcgaaccgaccacagcggcgagtgccgggctgggggtcagggccttcatgaacgcggcgttgggcgtgcgcttcttggcgggagcggccttctttgcaggagccttcttcgcaggagcagcagccttcttcgcaggagcggcagccttctttgcgggagcagcagccttcttggccggtgcggccttcttcgcaggagccgcagccttctttgcgggagcggccttctttgccggagctttcttggccggagccttctttgcagttgccatggttgatttccttttttggttgaacgttcaccaatgaaaaacttgcgtctccagtggcattgcggatgctaaaggagaaaaaactcgtttccaagggaaaaagagcttttttcattgggagttgttgttttttcagaggggagaacccgaggttttcagcttcggcgttcgggccacgtcgccagcaccacgccaatgagcgcaagcgcgaacgcaatgagctgtgccgaagagaggctctcgccgagcaccagcacgcccacgagggccgcgctcacgggcagcatcaccgcgaaaacacccgcttgcgcagcgggcacgtggcgcaggcccgtcatccacagccacaccgtccagatgcttgcggcaagcgcatagaccacgagcagggcccaggtgccgatgcgcacggccgagaaatcgaactgcagcgcgaaccagatgccgaagggcatcgacagcacgaagccccacaggttgatgagcgacgagatccgcttggggccgaggcggccggtgagcgacttgccgatcaccgcgtaggccgtttcgcaaagcaccgcgcagaacacgagcaggttgcccagccacggcatcgacgagcgcgaagggccttctgcagtggctggagcgtgcgccggcgtgagcgcgagcaggccgatgccgatcgccgcgcagccgattgccaggccgatgcgcaccgtgatgcgctcgcgcaggaagagccagctcgcaaccgccacggccgccggcatggacgccatgatcacaccggccgacaccgcgctcgtgaggctcacgccgaacagcatgcagacggagaacaggaagttgccgagaaacgattcgagaaagaccaggccgcgggtgcggccgctcatcggcggttcccccggcgggcgctgcagccagtgcggcatggcgagcgcggcgatgccaaagcgaagccatgcgagcagcagcaccgggaagacggcgaccaatggtttggagagggcgacataaccgccgacgagcgacatgctcagggccaggcagccataggcgacgaggcggctggaggcggggacagcagcggtgttcaatagactcgatggcttgttgctggaacgatggattcaatgatgccgcaatcgacgaaatccgatggcctgccaggcgcacgcacctcgcgccacgtgttcgtctacggcacgctgcgccgcggcgggcgcaatgacatcgcgcgctttcggcctgaacccttccacgtggccgacgccgccattgcgggcacgctgtacgacctgggcgcctatcctggcgtagtgctgggcggaaaagggcgcgtcgtgggcgagatctacagcgtcgagcctgaagtggaagcggcgctcgacgcgctcgaagaagttgccgacgatgacgcgggcgaatacatcaggcgccatgtgatggtggaagcgggcgtgcagcagttcgaatgcctggtctacgaaattcatccgtcgcgcatcgcaggccgtgcggtgatccggagcggcgactggatcgcgcacgcggcggccaggtaagaccagtttcgcgagcctcgttttcacgcctgaaaggcgcattgcgcatcgtgaaatgagcaactgctgcgccgcaatattttttctcaatatgagaaaaataattttgcattgagaaatctatccgtaagccattgattttgctgagataaaaatatgtcttctataagacataagagtccagagatcggtttacagtgactccacggccgcagcgcccatccttcaatcaacctcacggagtgaccatgccccagaccctcaccgaacaactgagccgcgaacagcaaattgccgccctcgagaaagaatgggccaccaatccccgctggaagggcatcaagcgcggctacagcgccgccgacgtcgtgcgccttcgcgggtcgttccccatcgagcacacgctggcacgccgcggtgcagagaagctctgggagctggtgaacaacgagccctacgtcaattgcctcggcgcgctcacgggcggccaggccatgcagcaggtgaaggccggcgtgaaggccatctacctgtcgggctggcaggttgccgcggacgccaacacctactcggccatgtaccccgaccagtcgctgtacccggtggactcggtgccgaccgtggtcgagcgcatcaacaacaccttccgccgcgcggacgaaatccagtggtccaagaatgtgaaccccggcgacaagggctacgtcgactacttcgcgcccatcgttgcagacgctgaagccggctttggcggcgtgctgaacggcttcgagctgatgaaggccatgatcaaggccggcgccggcggcgtgcacttcgaagaccagcttgcctcggtcaagaagtgcggccacatgggcggcaaggtgctcgtgccgacgaccgaagctgtgcagaagctcgtcgccgcgcgcatggcggctgacgtctgcggtacgcccacgctcgtgattgcccgcaccgacgccgaggcagccgacctcatcaccagcgactacgacgagaacgacaagccgttcctgaccggtgagcgcaccgccgaaggcttctacaagacgaagaagggcatggaccaggccatcagccgcgccgtcgcctatgcgtactacgccgacctggtgtggtgcgaaaccggcacgcccgacctcgagttcgcccgcaagttcgctgaagccgtgcacaaggtgcaccccggcaagatgctggcctacaactgctcgccttcgttcaactggaagaagaacctcgacgacgccaccattgccaagttccagaaggaactgggcgccatgggctacaagtaccagttcatcacgctggccggcatccattcgatgtggttcaacatgttcgacctggcccaggactacgtgcaacgcggcatgtcggcctacgtcgaaaaggtgcaggagcccgagttcgcggcgcgcgaccgcggctacaccttcgtctcgcaccagcaggaagtgggcaccggttacttcgacgaggtgaccacggtcatccagggcggcaagtccagcgtcacggcgctgaccggctcgaccgaggaagaacagttccactgacccgctgatcgccgataaagacgattcgctgtcaccttcgagcccggccgagcgccgggcttttttttgggccggcaccggccaagacctcgcgccgatggccccggcgggcaacggatagaatcacggctctctgcacccaacaagagcgagaaaggcaccttggttatgacaccgcgaactactccgcaaggattcagcggctttttcttcgtctccgaaggaaagggccggtagcccgcgctcgctggtttctgccagctcccaaaccaagcaaagcgcggccagtcaccgcgctttttgttttttcgccccgaggtttttcatgatccagatcacgcttcccgacaactcgcgccgcgagttcccaggcccggtttcggtggcccaagttgcccagtccatcggacccgggctcgccaagatgacggtggccggcaaggtcgacggcaagctcgtcgatgccagcgacgtcatcgaccgcgacgccaagctccagatcatcacgcccaaggacgacgagggcttggagatcatccgccactcgacggcccacctggtcggccatgccgtgaagcagctctacccaacggccaagatggtcatcgggccggtgatcgaagagggcttttattacgacatctcgtacgagcgccccttcacgcccgaagacatggccgccatcgaggcgcgcatgaaggagctgattgcgcaagactacgacgtggtcaagaagatgacgccgcgtgccgaggtcatcgaggtcttcaagtcgcgcggcgaagactacaagctgcgcctcgtcgaagacatgcccgacgagcaggccatgggcctctactaccaccaggaatacgtcgacatgtgccgcggcccgcacgtgcccaacacgcgcttcctgaaggtcttcaagctcaccaagctggccggcgcctactggcgcggcgacgccaagaacgagcagctgcagcgcgtctacggcacggcctgggccgacaagaagcagctcgaccagtacatccagcgcatcgaagaagccgagaagcgcgaccaccgcaagctcggcaaggaactcgacctgttccacatcgatgaagtggcgccaggcgtcgtgttctggcaccccaagggctgggccgtgtggcaggcggtggagcagtacatgcgcggcatctaccgcgacacgggctactgggaagtgaagggcccgcagattctcgacaagagcctgtgggagaaaacgggccactggcagaactaccgcgacaacatgttcacgacggagtcggaaaagcgcgaatacgcgctcaagccgatgaactgccccggccacgtgctcatcttcaagagcgacctgcgcagctaccgcgacctgccgctgcgctacggcgagttcggccagtgccaccgcaacgaacccagcggcgcgctgcacggcatcatgcgcgtgcgcggcttcacgcaggacgacggccacatcttctgcaccgaagaccagattcttgatgaatgcatcgcctacacggagcagctgcagaaggtctacgccgacttcggcttcacggacatcctctacaaggtggccacgcggcccgacaaccgcgtgggctccgacgagctctgggacaaggccgagcacgccgtcatggaggccctgcgccgttcgggcgtcgacttcatcatctcgcccggcgacggcgccttctacggccccaagatcgaatacacgctgaaggacgcgctgggccgccagtggcagtgcggcacgatgcaggtcgacttcaacacggccgagcggctgggcggcgaatacgttaccgaatcgagcggccgcgcgcatcccgtcatgctgcaccgcgccatcgtgggcagcctcgagcgtttcatcggcatgctgatcgaacaccacgctggcgcgctgcccgcatggctcgccccggtgcaggtggcggtgctcaatatcagcgaagggcaggccgattacgctgcttcagtggcgaaaacgttgcagaatcaagggcttagggttcagctcgatctgcacaacgagaagattacgtataaaatccgcaagcattcgttgcaaaagcttccctacatcctcgtcgtaggcgacaaagagaaggaagctggtgccgtcgcagtgcgcgcccggggcaaccaagacctcggtgcaatgtccctcgaatcgttcaagcagcggctcgaccaggatgttgctgacaagcgttgatttgtccctgaagcaccccaacttgtgtttctcgatcaaatcatgccgcttgtccgcgaggactgccccggcttccgctacagattttgtagcaacttttgaaggattctgaccatcgctactgcatttcgcgaccgccgccaccgcgaggaacgccaacaccgcctgaaccgggaaatcatggccccggaagtccgccttgtaggcccggaaaacgagccattgggtgttatgagtctctccgaggccttgcgccttgccggtgaggctgacgtggatctggtagaggtcgtcgccgcggccaatccgccagtgtgccgcctgatcgagtacggcaagttcaagtaccacgagcagaagaaggcggccgaggcgaagtcgaagcagaaggtcatcgaggtcaaggaaatcaagttccggcccggtaccgacgatggcgactacaacatcaagatgcgcaacatcaagcgctttcttgaagagggcgacaaatgcaagatcacgctgcgcttccgtggccgcgagatcacgcaccaggagctcggtctggctttgctgcagcgtattcgcgatgaactggctgacctgatcgtcgtggagcagtttcccaagctcgaaggccggcagatgatcatgatgatcgctccgggccgcaagaagccgggtggcggtggtgccgccaagcccgcgtcgacggaaacgtcgtcggcgcccgcggcagcctgaaaaggctggtcgggcgagagagatagtcagcagggttttaaagaatttcgccgttgccggcgcttcgcaagaagggcaggcaggggcgagataaagaagtgtctcggggccaacaagtccgtggagtatccgcggcgcctcacgagcacaaactaaaggagcatttacatgcccaaaatgaagaccaagagcagcgcgaaaaaacgtttccgcgttcgtcccggtggcaccgtcaagcgcggtcaagccttcaagcgtcacatcttgacgaagaagaccaccaagaacaagcgtcacctccgtggtgcagtcgcagtgcatgaaaccaacatggtttctgtcgccgccatgctgcccggccgtggcatttaactcagacgaacaaggagtacacacatgcctcgcgtcaaacgtggtgtaacggctcgcgcccgccacaagaaagttctcgcactcgccaagggtttccgtggtcgccgcggtaatgtcttccgcatcgccaaacaggcggtaatgaaggctgggcaatatgcctaccgtgaccgccgcaacaagaagcgcgtgttccgtcaactgtggatcgcgcgtatcaacgccgcctcgcgtgaactgggcctgacctacagccagtttgcaaacggcatccgcaaggccggaatcgagatcgaccgcaagatgcttgcggacatcgcagtgcacgacaaggccgcttttgccggcatcgtggagcaggtcaaggccaagctggctgcttgatcctgtaaagcaagggcggctgtcttcgtggcagtctcctgcgcccacgacacaagggctggcgcttgaaaaggctccagctctttttttatttccccgcctattttctgttgctatgaacgagttggactccctggtagccaccgcacgcgccgccttcgccgaagcgaaaacgcccgccgagctcgagaacgccaaggcgcagttcctcggcaagtcgggccgcatcaccgagctgatgaagggcatggccgcgctcagcgtcgacgagaagaagtcgcgcggcgccgcaatcaacgtggccaagcaggccatcgagtcctcgctgaccgaacgccgccagcagctggccgacgaagagctttcgctgcaattgcgcgctgaggccctcgacgtgagcctgcccggcagccgtcgcattccgggtggcctgcaccccgtgagccgcaccctggagcgcatcgaagagatcttctccagcatgggcttcgacgtggccgacggccccgagatcgagagcgactggcacagcttcacctcgctcaacaacccgccgaaccatcctgcgcgttcgatgcaggacaccttttatgtcgatctgaacggcgacgacggcattccgtacaacctgcgtccgcacaccagcccgatgcaggtgcgctatgcgcatcagcacatcaagaaatacgcggccgagtttgccgccgcggcagccgacaccaccggtgccgtcaaggcgcccgagatccgcgtgattgcgcccggccgcacctaccgcgttgacagcgacgccacccactcgcccatgttccaccagtgcgaaggcctgtggctcggcgagaacgtgagcttcaaggacctgaaggtcgtcttcaccgacttctgccgcaccttcttcgagagcgacgacctcgtgctgcgctttcgcccgagcttttttccttttaccgagcccagcgccgaaatcgacatccagtttgcgagcggcccgctggccggccgctggctcgaggttgcgggttcgggccaggtgcacccgaacgtggtgcgcaacatgggcctcgaccccgagcgctacatcggctttgcctttggcatggggcccgaccggctcacgatgctgcgctacggcgtgaacgacttgcggctgttcttcgacggcgacttgcgctttctctcgcagttccagtaagcacccacccatagaaaaccgaatacgagatcgaagagatgcaattcccggaatcctggctgcgcgagttctgcaacccgcccctcggcagcgccgagctggccgaaacgctcaccatgggcggcttcgaggtcgaagagcgccgccccgtggcgccgcccttcagccgcatcgtggttggcgagatcaaggaagccgtgcagcaccccaacgccgatcgcctgcgcgtgtgccaggtagacgcggggcagggcgccttgctcaacatcgtgtgcggcgcgcccaatgcgcgcgttggcatcaaagtgccctgcgcgctggttggcgccgaactcccgccgggtgaagacggcaagccctttctcatcaagctcggcaagctgcgcggcgtcgagagccagggcatgctgtgctcggcccgcgagctgcagctgagcgaagaccacggcggcctgctcgagctcgacgccgacgcgcccattggcgccgacgtgcgcgacgtgctcaagctcgacgacgcgctgctcacgctcaagctcacgcccaacctcgcgcacggcctgagcgtgtacggcattgcacgcgaactcgcggcgctcaccggcgcaccgctcaagacgcccgccattgcgccggttgcaacatcgtttgccgacgtgctgccggtgaaggtggaggcgcctgaactctgcggccgtttttcgggccgcattgtgcgcggcgtgaacaccaaggtgagcacgccggcctggatggtcgagcgcctcgcgcgctgcggccagcgcagcgtgacgccgctggtcgacatttcgaactacgtcatgttcgagtacggccagcccagccacatcttcgacctcgacaagatccacggcggcctgaccgtgcgctggggcaaggcgggcgagcagctcaagctgctgaacggcaacaccatcagcgtcgacgacaaggtcggcgtgattgccgacgatcaggccgtcgagtcgctcgccggcatcatgggcggcgacgccacctcggtgtccgacgacacgcgcaacatctacgtcgaggccgcgttctggtggcccgaagccgttcagggccgctcgcgccgcttcaacttcacgaccgatgccgggcatcgctacgagcgcggcgtcgatccgagccgctcggtggaaatcatcgagcgcatcacgcaactcatcatcgagatctgcggcggccaggccggcgccatggacgacaagatcttgaacgtgcccgaggccatgcccgtcacgctgcgcgtggcgcgtgccgcgcgcgtcatcggcatgccgctctcgcaggcgcaatgcgccgacgcactgcgccgcctgggttttgcgcttggcgaaggcgagggcacattgaccgtcacgcccccgccgcaccgcttcgacctgctcatcgaagaagacctcatcgaagaagtggcgcgcctgatcggcttcaacaacctgccgaccaccgcgccgctggcgcccattaccgcccgcgtgcggcccgaggcccagcgcagtcgcttcgcggtgcgccgcagcctggcggcgctcggctaccaggaaaccatcaacttcagttttgtggaagcgcactgggagcaagacctggccggcaacgccaaccccgtcaagctgctgaaccccatcgccagccagatgagcgtgatgcgctcgtcgctgatcggctcgctgctgcaggtgctcaagttcaacctcgaccgcaaggccccgcgcgtgcgcgtgttcgaagtgggccgcgtattcttgcgcgacgacagcgtggccaccaccgacagcaccgtgcgcggcgttcaccagcccatgcgcgtggccggccttgccttgggcgatgccgaagaagcgcgctgggacggcaagccgcaccgcgtcgacttttacgacgccaagggcgacgtcgaagcgctgctcgcacccctggtgcccagcttcgaggcggccgagcatccggccctgcaccccggccgctccgcccgcgtgctgatcgacggcaaggccatcggctttgtcggcgagctgcatccgcgctggcgccagaagtgggactttgccctggcccccgtggtttttgaactcgacctcgacgccgtgaccgcgcgccccgtgcccgtggcccagccggtgcccaagcaccaggccgtcgagcgagacattgccgtggtcgtggccgaatccgtcacgcacaatgcgttgatgcaggccattcaatcggcggccgcggcgcaagggctgctgcgcgacgccacgctgttcgacatctatcgcccgcaacctgcgcgcgacggcacggcgcccgcatcgggcggcctggcgcaaggggagaagagcatggcggttcgcctgagcttccaggacgacaacgccacgctgaccgacgagcaggtggaacctgccgtgcgcgccatcgtcgaacaactgagcgccagactcggcgcgcgcttgagagggtgatgagaatgaacgccgcggaattcacgctcgaagccctcgaaacgcccgcactcaccaaggcgcacctggccgacctgctttttgagcagatcggcctcaacaagcgcgaatccaaggacatggtcgaggctttcttcgacctcattgccaacagcctgatcgaaggcaccgacgtcaagatttctggctttggcaacttccagatccgcgtgaaggcaccccggccgggccgcaatccgcgcaccggcgaagccattcccatcggcgagcggcgcgtggccacctttcacgccagcgccaagctgaaggaacaaattcacggaagcatcgagcccagcggcacttccgaggtcgagtggagcctgggcgccgaataagtgcttggtgctgcgcgggtgcgtagagtaatctctaaggtttcctgcgcacggtcttgatttcaatggaaataatggagaaagcgctcccgcccattcccgtcaaacgctacttcaccatcggtgaggttggcgagctgtgtggcgtcaagccgcacgtgctgcgctattgggagcaggagttcacgcaactgcgccccatgaagcggcgcggcaaccggcgctactaccagcaccacgaggtgctcatgattcgccgcatccgcgatctgctctacgaccagggctttaccatcagcggcgcgcgcaacaagctgcaagaactcgtgcaaggcgagcgcgagcgccgcaaggccggcatcgttccgctggagggcatggaagccgtcgaaatcgaccaggaagagttcgatgcggccatgcaccaggacgaagacacccaccacagccccgagccccagcaagccacggcccgcaccgtcgatccgtcgcagctggtgcacctgcggcgcgagctttttgaaattcgtgagctgcttaccgtcggacggtgatttcagccggctataattgagagcttcggtgtgtggcgcagcctggtagcgcacttgcatggggtgcaaggggtcgaaggttcgaatcctttcacaccgaccaatatcgtcagatagaaaaacgggtcagagccacaagctctgacccgtttttttttgctgcgcgacagcttcagtcgtcagaccgcgcgacgaagagcaggcacatgctcagaacgccgagcaacgtgccggccacaaatattccgatgtcgagtgcgagggtgtacataggttttcaacaacaggtgctctcccgatactttctaagtattgaagcttgttcacctgacccactcctgattagcggattagaggcatcagcccaaagataagttgtccggaaaacgatagatattgggacacggtttcgcccagcggcccagcccgcaacaaggcataaccgaaagcatgcatggaggcccgtctggcaggcaccaaatgcggccgaccccacgcaccaaaacgtgacgtccatcacacttacgccaactcatgggtagcaaactgtaattttcgctatttatgtctaaaaaggtgatttccgtctctttttacgaatcgctacgtctggggtcaaaagttaaactatgtgaacaagaggaggcatcgagcgacaggtagtcctctgtcgcctctgtcgggctttcacccggagtgaaacaacacagaggtttgctttgagacgtcaagtcaacacggcggcgtgctccgctgccctatttgtgggtaccctaggtaccctgttgctccaaggctgcaccatcgtgcccggcatgggcaccgtggagccgtatcagagcgccgaggatctgccgcccaagttccagtacctgcccgacgcagcgcctgaggaccggatcacccccatcacgccggcccttgtacgcacgttcgccaagatgacgcccaagagcgtgccgtcggaagtgcaggcgctcttcggcaagtcgcagcgctacaccatcggccccggagacgtggtgggcgtcatcgtgtatgaccaccccgaactgctgcccaatgctggtgcagtcatctcgcagcagtccgaccccacgggcgtgagcgtggcaccgggcttcatcgtcgactcgtcgggcgaaatcgcctttccgtatgtgggccgcgtcagggttgcggggctcaccgaggccgaagccggcgagctcatctccaagctgatcgtcacccaggtgcgcgagccccaagtgacggtgcgcattcagtcgttcagaagccgccgcgcctatgtagaaggcgaagtgcgcgcaccgggctcgcaggtcttcaccgacttgcccatgacgctgaacgaggccatcaaccgggccggcggcatcaccgcaaacggaaactttgcggccgtgaccctggttcgtgatggcaagtccgtcgacatcaacctgacgcgcctgcgcgaagccggccgcgacggcaacgacattcccttgaggagcggcgacaccattcgcgtaggccaccgcgaagacgccaaggtgtatgtgatgggcgaaatcttgcgcccatcggcgctcacggtgcgcagcaacggccgcctcaacctgaacgaagcgctgggcgaagccggcgggccgattctcaccacgtccaaccccggccagatctacgtgattcgccagggggccaccggcttaccagccatctttcatctggacgccaagaaccccgccgcaatggtgctggccaggcagttcggcctggaggcgcaagacgtggtctacatcgacccggttccgcttgtgaagtggaaccgcgtgatcagtttgattctgccggctgcacagattgtgaatctgggtagtgaatcggcggatcggtttcgctgatagcgccgattggaggtgatcgtgtctcctctgcacattggacgtttgttaggccttcaattttttatctgggcgcttgtgtgtgccgatctgtgttcagaaacttgtcggcccttcctggtaattcaaaaatgaatataaaaattgcggttgcgggaaccggatacgtcggaatatccaatgccattttgctggctcagcacaatgaagtcgtggcacttgatattgtgcggtcgaaagtcgagatgcttaatgacaagtgctcacctattgatgatgcggatgtcaagacttatcttgcaaccaaacgactgaatctacgcgctaccacagataaggaacaggcgtatgtcggcgcagagttcgttttagtcgcaacaccaacgaactacgatcccgctacgaatttttttaataccgaatcggttgagacggttattcgagatgtgattgcaataaatccgaacgcgactgtggtgattaagtcgactgtcccggtcggatacacagcaagtttgcgggaaaaactcggatttaacaatttgatattttcccccgagtttctacgagagggaaaatctttgcatgacaacctgtttcccagccgaatcgtggtcggtgggaaatctgaagcggcaaaacggtttgccgagcttttactgcaaggtgcgattaagggtgatgtaccggtgctttttactgagagctcagaggcggaggcgatcaaactattcgcgaatacgtacttggccatgagggtcgcatactttaatgagctcgacacgtatgccgtcacccaccagctcgactctcgagaaattattagcggagtgtgtctggatccgcgaatcgggcttcactataacaaccctagcttcgggtacgggggatactgtttgccaaaagacaccaagcaacttttggccaactaccaagatatccctcaaacgctaataagcgccatcgtcacggccaatactgtgcggcaagaattcattgccgaagatattcttcgcttgcgcccgagatcagttggagttcatcgactcattatgaagtccggcagcgacaactttagagaaagcagcgtacaaggaataattagccgacttcaggcgaaaggtatacccatttcgatttacgagccggtgctgcagcagagcgaatatttaggcattcctgtaatccgtgatttaggggattttaaggaacgctcagatctgatcttggccaaccgccgcgttccagaactcgctgacgtttccgatcgactttacactcgagatgtattcgggaatgactaaataccaatacgcgcaggtcgatcgcaatataaaaataaggttgcgcccacaggaaaactgctccctttgtcgtggctcgccggtgtaatcaggtgaaatccgcttctttacaaataatagtagggcaagctttttgggcgttagcccaagcgctcattgttctgctacttgcgcgacaagctggtggcgtggaacttatcggcacatttacgctggctttggcaattttcacccctttgtgcttagtggggggcttaaatctgaggaatgtgatagcgattgacgaagacaaaaacattaacatagtcgcagcgttggttctccgcactatcgtagtcattttggcactcgccataaccatcctcgttttgcagttcacgggacacttggacctccactggccgatagtagtcgttctcatggggacgcgtgctttagatcatgtaagcgatgtagccgctggtttttatcaaaacaacaatcggcttgggaaaataggcgtctcctttttcgccagaggcaccgcaaattttttcccgatgattattatttggaatctcggaggagggttgggtctagcagtaggagccgcttttgtggtaacactaatggctgtggtaatttttgatttgttgtcgattaaaaagatagcggaagcctccaaaaagaagaatgatttcacactgcgccttctttttagaacgctggttccctcatggtctgcgtcactatttccattttttgacagtttgcatgcgaacagcttgcgctacgcaatagtttttttgttctcaagttctgtgctgggattagtcgggattgctcaaactctctttgcaccaatccagttattgattagcgcattgggatacgcatatctgccaaaaatgcgagccttggttaaggctggagagcgcgataaaataatttcgtttgtcaggatagggagcttgcgggggttgcttcctacgattgcgtttctattgttttctttgattgttccggattccctactccgcattttatttggagatattgatctcaaggggcttcgagatgctttatatatggtttcggtggccatgctgttctttggggtaactggttatttggcgcagtctgtgctggcaattaagcaggagcgatactacttgttgtcgccgctgattggctcaatgtcatttcttgctctaattgttctgttccatggttttgaatccaagtttgaattgatttacattggaatcattttttccgcgagctttttttcaagaatagtctgcaacttgattgggctaaattctaagctcgggagtccggcatgagttacacgggtggaaaggtattgtttccttttagagtgaccagaaaaatcgctgcatacttttctggaatggtgaattcattcttatatcggatggcttgtaaatcagtcggaagaggaagtcggtttcgaggtggcgcatttatagctgaaccaaaggcggttgagatcggggaaggctgttttatcggtcgtggtttaacggcatcctccgagatcgcaggaaaacatttgaaaatcggcgatggcgtacaaataaactcagacgtaaagttggatcacacgggtggattgtctataggaaataagacgcttatttctgagcaggtaataatatatagccatgaccacggcctagatccgcgctcatcgcctattccaatgcaaaaagtaatagggcgtggagtttggattggcgctcgcgcagtagttatgcccggctgcagagtaattggagaccacgcaataatcggggctggtgcaatagtgacgcgcgatgtacccgagaacgccattgttgcgggcaatccggcaaagattataagaatcaaaatagactagtatgctggcccttttgattcttttgctaatctttattcatcttttgccttggttgaattcaaggcgagatggcgttggcaaaaatcctgcaaaactgatatctattatcagcggcattatgtcaattccatatctctgcatcattgcatgggatggggaaaaatcggctgttaagtcaatcttgaaaagcggtgactttgagcatctcttgaccgtatttattgtctattactgcgctggaatgctctgtctgtttgcgggcatttctctcggtgcaagaattaaattgcccatcctcaatgtcttttccctccacaagcccgtgggaacgaggttttatcgaaggttctcgcatttcttcttggtggtggttcttctgctttccgccttgaagatgcaacaggttggcggtctactgggattttgggccgatattggcatgcgagcccagaatttatcggggacgggaattctggatgtctttattttgccttcgagttatttggcaattttcttcgcactctatgcacgatcaatcgatggtcgtccaagtcgatattggatagtttttctggtggtggcgatgttcgtggctttatcgctgtttggcgggcgcaaaaattccataatgcttgtaattttctcgttgcttgcggccagtgtattcaatttgcgcttcaagttgatttccctgaaggctttgattgcgtatgcttttcttggaatattttttgtcgcaatattgatatttcggctaggcagccaaatcgactccgccagcggttcatttgatttgttggacgcaattcaaaatacaagttatgtcgatacctacctattcatcattgattatttttctgaccggccgttttggtacggggccggcttcggagatctagcgatcaggctattgagctcgggagatcctagcctccttccgcccattgatgatggcgtctatatcagatcgcttgtggaagggtggagcgttaagccgcctatgccttttaatgagttatatcccagttcttggccgccggagactttcggttctgggtatgtcaatttcggatttatcggcgtcgtttttttctttttcctcaaggggctcatttccgggatgctttttcgatgggctcgagcgcgagccttcgctcctatccccctatttttgatgatttacttttccgcgaacttccatctttcgaacctaagaatagtgcaaaccggatttttgttcgccgttactttcatcgtcgtgatgttcttaagaatttcgaccagtacacgcaaagttaggatggctagctagtatgcgaccagtcgttttgatttttattgcccactatcttcccggctttaaaatgggcgggcctctccgaagcatttcaaatttaatcgatcacctgtccacagaatttgatttttatgttttcacgagtgatcgcgatttaggtgatctccgtccttattccgacgtggttgtggatcgctggacgcgagttggcagtgcgatggtgtactacgcatcacccaagatgaaaacgctgtctgggattgcgaaggtcttaaagcgaactccgcatgatttgctatatctaaatagctttttctcgtttaagcattcaatgctgccggtactgactttgcggcacgtccgacgatcatcagtgccggtggtccttgctccgcgtggggagttttcgcgtggagcactggcgctcaaagcgtggaaaaagaggccgtacaccgccgctgcaaagatgagcggcctattgcgaggactgacttggcaagcctcgaccgagtacgaagctgaggacattcgagccgtcgttggacctgcaacacaaatcacaatcgcgcgaaacttggctacccgattgtctccggttcctcctgaccattccgtccgtccccacggatttcctcttcgcataattttcctatctcggatatcaccaaagaaaaatctagacttcgctctaaaagttctagctcgagtcagggctcctgtgaaatttcggatttatgggccacccgaagatcttgcgtatctgaatgaatgcaaggttttggaagaagcgttacccgctcatatttccgttgaatggcacgatgccgtcgcgcctgaaagtgtgtctacgatcatagccgagcatgatcttttcttttttccgactaaaggtgaaaacttcggccacgtaatcgcggaggcactcggtgccggaacgccggtcctgatctcggatacaacgccttggcggaatttaggggtggaaggcgttgggaacgattttcccctcacgaacaccgaagcctttgtgtcgcggatcgaagaaattgccgaactaatgccgcaggagatgctaagtcttcgcgctcgcgccgccaaatacgcgcgggagttgcaggccaacgatgagagtgttgactcccatcggaacctctttttcgggtcattggctggtcaaaaagtttattgatttattggtcgtttaaggcgaggctggcatctccgccgattcataacgtgaagttgatttgcttgagtttgcgcttgaggattgaacatgtttaaagaaaagattcttttaattactggcggaacagggtcgtttggaggcgcagttcttcatcgtttcctggagagcgatattgcagaaattcgggtattcagtcgtgacgaaaagaagcaggacgacatgcggaagaggttcaatagtcccaaactgaaattttatctcggtgacgtacgcgacattcgcagcgtcaatcacgcaatgcgaggagttgattttgtttttcacgccgccgcgctaaaacaggttccctcttgcgaattccacccaatgcaagcagttcgcaccaacgtcctcggcaccgagaatgtcttggaagcagcaactgccgccgatgtcaaacgcgtcgtgtgcctgagcacggacaaggccgtctatcccatcaacgcgatgggcatcagtaaagccatgatggaaaaagtcatggtcgccgctagccgaaatctggagagcacaaacaccgttatttgtggcacccgctacggcaatgtcatggcctcccgcggctccgtcattccgctgttcgtggagcaggttctggcgggcaagcccatcactgtgacggacccgactatgactcgtttcatgatgaccctggaggacgcggtcgaactggttctgcatgccttcaagcatggcgacaacggcgacatctttgtgcagaaggctccggcggctacggtgcgggtgttaacgcaggccatcttagaggtaatgcgcaagccggatcatgaagtgcgtgagatcggcacccgccatggcgaaaagctctatgaagcgctgttgagccgcgaagaaatggcgtgcgccgaagaccaaggcgattactaccgtgtgccgcctgatgggcgcgacctgaattacgccaagtacgtggaaaagggcgagcagcgcattacccggagcacgcacggcgaagactacaactcgcacaacaccacccaactggatgtggacggcatgaagactctgctgctcaagctcgacttcatgcgacgcattgcgcgcggtgagcccgccctggcgcaggaataagggcatgaaggtattgattaccggcgcccgcggcttcgtgggcaagaacctgcagttgcacctggccgagcgcaaagacgtgcaagtggtctacttcacccgcgccgacagcgtggagcaactgcccacgctgctgcagggggtggacttcgtgttccacctggcgggcgtcaatcgccctcaagacccggaagagtttgctagaggcaatgcagaactcacacggagcttgtgccatgccgtctgcgccgtggccgaatccaccggcaagaaggtgcccgtcgtctacacctcgtccacccaggcaggcttcgacagcccttacggccgcagcaagcgcggagcggaagagacgctgcaggccgccgcccgcagtcacggcattccggtgcatatctttcggctgcccaacgtgtttggcaaatggtgccgtcccaactacaactcggctgtggcaacgttctgccacaacattgcgcgcgacttgcccattcagatcaatgacccggctgcgcccgtcacgctggtgtacgtcgatgatgtcgtcgaacgttttgtacaactgatggatggagccaatgcggcggtagacgcggatggcttcgcgactgtcgccccgcagtacaccaccacggtcggcgaactggctcggcagatcaagtcgttcagagacagccgcagcacgctcatgaccgatcgcgtgggaactggactggtgcgggcgctttattccacctatgtgagctacctgccggtcgagtcgtttgcctattccgttccgcaatacggggacgcgcgcggcgtgttcgtcgaaatgctcaagacgcctgatgccgggcagttctcgtacttcacggcgcaccccggaatcacgcgaggcggccactaccaccacagcaagaccgaaaagtttctggtcatcaaagggcacgcgcgcttcaagttccggcacatgcaaaccggcgaagcatatgaactgaccactgcgggccaaaagcctgaaattgtcgaaaccgtgccaggctggacacacgacatcaccaacatcggcaccgacgaaatggtcgtcatgctctgggcgaacgaggtgttcgaccgcgcacggccagacacttttgcatgcccgttagaccccttcgacttctgatcttttccatgaaaaaactcaaagtcatgaccgtggtcggcacccggcccgaaatcatccgcctctcgcgcgtgctcgctcggctggacgagcattgcgaccacgtgctggtgcataccggccagaactacgactacgaactcaaccaggttttcttcgacgacctgggcgtgcgtaagcccgaccatttcttgaacagtgcggccaacgccaccagcgcggcgcacaccattggcaacctcatcattgctgtggaccaggtgttgggcgaagtgcaaccagaggccatgctggtgctgggcgacaccaatagctgcctttcggtgattccggccaagcgccgcaagattccaatctttcacatggaggcgggcaaccgatgcttcgatcagcgggtgcctgaagaaaccaatcgccgtatcgtggaccacacggctgatgtcaacctgacctacagcaccattgcgcgcgactatctcttgcgcgaggggctgccacctgatctggtcatcaaaaccggcagtccgatgtttgaggtgctcacgcactaccgtcctcgcattgaggcgtccgatgtgctgcagcgcctgggcctgcaagctgcgcagtacttcgtggtcagcgcccatcgtgaagaaaacatcgagtcgccgcagtccttcggcaagctggtggcggtgctgaatgccgtggccgaagaccacggcctacccgtcatcgtttcaacgcacccgcgcacgcaaaagcgcattgatgcgacaggcgcgcgctttcatccggaggtgcgtctgttaaagccactgggttttcacgactacgtgaaactgcaggtctcggcgcgcgccacgctgtccgacagcggcaccatcaatgaagagtcgtcgatcctcaactttccggcactcaacctgcgcgaggcgcatgagcggcccgagggaatggaagaagccgccgtgatgatggtcggcctggaggtggaacgtgtgcgccaggggctggccattctggacacacagccgcgtggagaagcgcgtggcctgcgccaggtggcggactacagcatgcccaacgtgtccgacaaggtgctgcgcatcgttcacagctacaccgactacgtgaatcgcgtggtgtggaagaagtactgaagtcactatgcgcttgctcgtcgtctctcagtacttttggccggaaaacttcaggatcaatgatcttgtcgccgagttcgtgcggcgtggtcaccaagtcacggtgctgactggcgtgcccaactaccccgatggcaaagtcttccctgcgtaccgcaatgatcccgagatgtttgcgcgctacgaaggagcggaggttgtccgggtgcccatgtctgcacgtggaaagggcggggttcggttgatgctgaactttgcgaccttcgcaatcagtgcctccgtgcttgggctgtggaagctgcgaggacgcgactttgacgcgattcttgcctatgagccatcgcccatcacggtcggcgtgcccgcggttgcattgcgagcggttaaacgagcaccgctggctttctgggttcttgacctttggcccgaaacgttggaagccatcggcgtggttcgttcgcgtctcatcctccgtgcagtggggcggcttgtgtcgttcatctacaagcgttgcgacctgatcctggcgcagtcgaaaagctttgtgccccaaatcaagaaatacgcgggcaacagcggccgaatcgagtacttccccagttgggcggagatgctgttcgatgtggatcaagcggttgctgcgcctgaggtggaggtccaaccggagagcttcaatgtgatgttcgcaggaaacatcggtgatgctcaagatttcccggcgatcctcgcggcggcagaaattctcaaggcacaccggaacatccgttggttgatcgtcggtgatggccgaatggcgcaatgggtgaccgatgaaatccagcgtcgcggtttacaagagtgcgtccacatcctcggacggcatccagtggaacgaatgtcctcgttcttcaagcatgcagacgcattgctggtcagcttgaagaacgagccgattttttctatgaccataccgggcaagctgcagtcctacttggccgccggcattcccgttctcgccatgctgaatggcgaaggtgccgacgtggtgagaaatgccgcggctggtttgacttgcaacgcgggggatcacaaggagcttgccaaggctgttctggacctctcaaaaaaatcagctgaagaacgcaaggcaatgggcgcgaatggccttgcgttgagcgccagcgaattcgagcgtggctcgctgatcaatcgcttggaaggatggcttcagtcgctgtcctttcccgcctcggccacaaagaagcaaagcgaggcaacatgatcttggtaacaggagcgactggctttgtaggcactgcgctgattgagcggctgctcgctgatggcctgtctgtccgcgcggctattcgccgtgaatccgcgctcgaggattccaatgtcgaagccacgttggttggcgacctcagtgcggaaactgactggcgaaaggctgtcgcaaacgttgacgctgtgatccacactgccgcccgcgtccatgtgatgtcggatcgtgctagtgatccactgacggaatatcggcgcaccaatcttcacggaacgttgcgactggcgcggcaagcggcagaggctggggtgcgacgctttgtcttcgtaagctccattaaagccaatggagaggccacgcggattggaagtgcgttttcagcggacggggccacagctccgatggatccgtacggcatctctaaactggaagcggagcaggccttgcgagagctggcaaagcagaccggaatggaagtggcgatagttcgcccgcctcttgtgtacggccccggcgtcaaggcgaacttccgcacaatgatgagcatcgtcgcgcgacgaattccgttgccgctcgggggcgtcaccggcaatcgcagaagcatggtgtcgctcgacaatttggtggacctgttgtttgcttgcgtgcatcaccctgcagcgggcaatcagacttttatggtctcggacggcgaagacctttccaccgcacagctgctgaaacgtctagggcaagccatgggaaagcctacgcacctgctccctgttccggcgagctggctggagcgaggtgcttcgatgctgggtcgagcccatgtcgcacaacgactctgtggctcgttgcaagtcgacatttcaaagacgaaagacttgctgggatggaccccccccattaccgttgacgagggtttgaaaagggctgcagaagggtatttgcgtgaagcgtctgtttgatttgttcttggccttgtgcgccggggcggtgttgctgctcctggtcgcggtggtcgcgctggcggtacgtttgacttcgcgcggcccggctctctattggtctgaccgcgtcggcagcaacaaccgaatcttcaggatgcccaaatttcgcagcatgcgggtcggcacgcccgcggtcgccactcacttgctgtctgaccctgcggtgtacctgacgccgatcggttccttcttgcgcaggagcagtctcgatgaattgccacaactgtggagcatcttggtcggcgacatgagttttgttggacctcgccccgcgctttttaatcagcaggatctgatcgatctgcgaacgcggcatggtgttcatgtattggtgccgggactgacgggctgggcgcaggtcaacgggcgcgatgagttgcccatccctgccaaggtccagctcgatattcaatatcttcagcgtcgctcgttctggttcgatatccgcatcctgtggctcaccttcgtcaaggtgctgaggcgcgaaggtgtgacgcactgaatatgggacagcaatgataaaaaaacgcttgctgatcattggtgccggtggtcatggccgttccgtagctgaggccgcattgctacgacaggactatgaattgacggcgttcctggacgatgcggccaagccccagcaacatctgtgggactgtccggtctggggcacaacggagatgctggcagactgccgcggccgaatcgatgtggtgatagcggcaatcggcaataacgcattgcgtgaggcgttgcaccagcaggtgcaggcgcagggtatggcgcttgcgacggtcatacatccggcggcgatggtgtcgcccacggcgaccataggcgagggaagtgcaatcatggccggcgctatcttgggaaccggggctcaacttggtgagggcgtgatcgtcaactgtggcgccgtggttgatcatgactgcgtggtggaggcttttgcccacctgggcggcaacgccagtatggccggtgggtcggtcctcggtcgaggcgcgtggatgcaaacgggtacttcgttgggccatggcgccggcttgccagcggaagcggtcctgcgcgtgggcgagacgttcatcgatcagaaaactagacatggcatcttggccttctcccacggagcgacagaatgagcaagcttcctattgttcgcaagaacttttggcgctattgcttctggatctgcgccagcgcgattctggtgatgtcacttgcgccaccctcgattcctatgccgacgaccggctgggacaaagccaaccatgctttgggttttgccgtgctgggcctgctgggccaatgggcttggccggggcgcacggccatcgtgttgactgcgttgctggcctacggcgggctcatcgaactgctgcaatcgttcacgcccgatcgcgttgccgaggctatcgatttgatggccgattgggtggggctgctgttgggcgctggcttggcgtttttgctggagcgtctgcgccccacagggcagggggcgcaatgacggattcacagcattgctggcttgaaaagaatttctcaggagacttctcatgatcgatcgtctggctcagcctgtgttggcgctgccgcgccccgtaaagcgggtgttggccttgtcggtggacgccggcctgtgtgtgctgtgcgtgtggctggcgctcagcctgcgttacgagcggtggattgaactgacgggtgtgcattggctggcggtagccggtgcggtcatgttggcgctgccgctgttcgtggtctcgggcctgtaccgtgcaatctttcgctatgccggcagcgcggcgttgatggctgtcgtgcgcgcctgctccctgttcagcgtgggctatgtcctgatattcaccgcgttcggcgtggaaggcgttccgcgcacagtgggcctgctggtgcctgcgctgctgctgttcacggtgggcgcttcgcgcctgtttgcgcgctattggttaggcggcctttactctcaggtgttgcgcggcaaggcgctgccgcaggtggtgatctacggcgccggcaaggccggccgtcagttggccgcagcgctcgcccacagcccggagatggtggtgcggggcttcgtcgacgatggcgtgcagctgcagggcagcacgctcaatgggttgcccattcacccgccgtcctggctcaaggcccaggctgccgccgagggcataaccgacgtgctgctggcgctgccgtcggtctcgcaaggccgcagggcgcaaattttgaacgaactcttgtcgctgcgcctgcacgtgcgcacgctccctggcatggccgatctggcgcagggccgggtgcaggtcaaggatctgatggaagtcgacatcgaagacctgctgggccgcgacccggtggcaccggtcgagcatctgctgcatcgccacgtgcgtggcaaggtggtgctggtcaccggtgcgggtggttccattggcagcgagttgtgccgccagattgcgcagttgaggccctcggcgctgctgctggtcgaatggagcgaatatgcgctctatgccattcaccgcgagctggagcaacaagcacctgcgctcagcgtggtgccgctgctggcatcggtgagcgatgccgtgcgcatgcgccagatcatgagcgtgtggcggcccaatacggtctaccacgccgcggcctataagcatgtgccgcttgtggagcacaaccccgtagaaggcctcatcaacaacacgttgggcacgctcacaacggcattggcggcgcgggacaacggcgtcagccagtttgtgctggtcagcaccgacaaggcggtgcggccgaccaacatcatgggcgcaagcaagcgtctggccgagatgacgctgcagggcctggcccagcaaaagccacgcacctgcttttcaatggtgcgcttcggcaatgtgctgggctccagcggctcggtggtgccgctgtttcgccagcagatcgaagcgggcggaccgatcacgctcacgcacgaagacatcacgcgctatttcatgaccattccagaggcggcccaactggtgatccaggccggcgccatggccgagggcggtgatgtgtttgtgctggagatgggcgcgccggtgcgcatcatcgacctggcgcgccgcttggtggaactgtcggggcgcacggtgtgcgacgcacggaacccggaaggtgatatcgagctgctgatcaccggcctgcgtcccggcgaaaagctgtatgaagaactgctgattggcgacaacgccatgcccaccgcgcatccgcgcgtgatgaaggcgcatgaagcatgcccgccgtgggcagagctggcgacacagatcgatgagcttcgcacgctgctcgcgctcaacgatgtgcctgcaatcaagcgaaaactgcagctgcttctgggcggctacctgccgcatgcggaagtggtcgactgggtgcacctggagcgtgaacgccagagtgcggcgctgccggcgccggtaacaaatgcacccaatacctcggcgccagttgctgctgtctcgccttcggcgctcgctgcaatctgaactgatctgttagtggaaagccggggaattccccggcaccatcctgactggctcctgccgcccgctctactcgttgtacttgtacttcgtgtaccggtagccgccgtatcggtagccttggctgccatagtggcgccgcgtcaggtcaataccgttgaagatcacgccggtgactgccttgccaccatgtgcgaggcgcttggcgctttcattgagttcgccaagctgggtctgatccgcgcgtgccaccagcagcaccgcacccatgtacggcgccacggcagccgtgtcggcggccaccagcaccggcggcgtgtcgataacgaccagttcgtattgcgcggacaccatgtcgagaaggcgcacaaagctttccgacatcagcatgtcggccggattggacggcagctttccggtcgtcaatatgtcgaggttgggcagcacctgtgagcggattgcctgctgcgccgaaagctcgccagccagcagttccgagaggccgttttcgcgcggcaggccaaactgcttgttcaagtggcccttgcgcatgtccgcgtcaatcagcagcactcgcttgccggcgtgggccatgatggcggcaaagttgcctgaaacaaagctcttgccaatgcccggtgtcgcaccggtaatgagtacccggttatttccagcttccagtgtggcaaattgcagcgcaatgcgcaggctgcgcaatgcctcaatggatgggctgtccgaatgggtcaccgccagcagttggattcccttggcacctgtggcaatgctttggtcaagcgctatctgctcaggcgtgaaaggcaccaccgaatagaccgacaggccggtgtgggactcgatctcctgcggatcctgaatgcccctgaagaaccaactgcgcatgagggccaacgccgcgccgctcagcaggcctagcaccagcgctaacgccacgatcagtagcttctgcggtttgattggtttcttgggcttcactgccttgtcgagcaggcgcacgttgccggtcttgccttccttcaccaggcgcagttgcagcgcgttgttctgcagcgactggtaaaggccactgttcacccgcacgtcgcgttcgaggcgcagcgcatcttgctgcagcgtgggcatgcggctcacgcgtgcgttgaggccgccaatctctttctcgatggcggaaatttgcccatcgattgtctttacgcgtaagttggcatccgcaaagtgcgcgaccagttcacgccgcttttgctgggcttcgagcagcttggtctgcagctcgatggtctgggccagcacgcccttggcttcttcgtcgaaagccacggtgccgttcttgtttcgaaagagcgtgtaggcatcttcggaggcttcgagctggcgtttgaattcaggcaattgctcgtccaagaagaccagcgttttctgcgcctcggcagccttgcgttcgacgttctgctgcacgtactgctcgccaatggcattgaggattcgggaaagtctgtcgcgatcgctgtcttccagcgctacgttgatcacgttcgattgcttaccttgttcggcgagctgcaggcgtttctgcagatcctcaatggtgcgcaattgcgaagcgcgcgacacgacgaattgcgcaccaggcttgccttcgagtgtgtcgatcagtaggtcaatggcgccatcttctagcacctgatgcagcggcaggccgacggtgccggtcagtggccgattcagtgcctcgtgcgtcagcgtgtatttgccttcgccttgcgcggtgatcatgaaaggctcatcatcttcaaactcgggcggcacgtcgaagcgggcgacgtcgatactttcgttgccattgacataaccaccgatcccgaggaaaccaggatccgacagcccgtccgcccgccgtgccaaccaggtgccgagcaccggcagatagcgcgggctagcgtcgatatagaagcgtgtcttctctaccgcggcaccgagcaccatacgggagcggatgacttgtatctcgccgctggcgggcgtctttacgtcgaagaggctagaagcctcgccaagaaagcccttggcgtcgggtgcggcgtcctcgacctggaccagcaagttggactgataaatgggggtggagattagcgcgtaggccacgccgagtactagcgcaaacgcagtgacggctgcaaccagccactttcgatcgatcaggatgtcgatccattccgacagattgatatcgtcgtcgtccgttgctgcagtcgaaatagcagcaggctgaccgacgcgcacggcatttgaattagtgacagcaggagtgttcatttgaattgccgaatgcgttcggcccaggtcttgacgccagcgtcgatgagttggagcgcgtgctcgaaggcttcctgtccctggcggtaggggtcgggaatattcagcttggcggtttcggcaagccgaaagaccctgccgcgcgcgagcgggtagttgttttcaatgtggcggcgctggccatcgtccatggtcaggatcaggtcggcgccaacgcacatggcttgggtgacctggcgcgcacggtggtagccaaggtcgagcccccgctcggccatcagcgcctgggcaatagggtccgctgggtggcctatcaacgcaccagtgccggccgaagttacggtgtgctgcggcagggccttggcgagcagtatttgcgccatcgggctgcggcagatattgccaatgcaaacgacaagaacggagttcatgggcttcgatcgaaattcaagatgttgtctccggcatggggcttgttgtcttgcggggccgcaaagttgaaggcacccttgtcccgcacagaggtcagttcataaagtgtgttgctgcggcccaggcgggcgccgccgtcgcgcgtgagcggtgaccatccaaagctcagcgaaaacttggtcgaccggggcagcagtgcgtccagcggaatcgaaagataaatgcccttgtcaaaatcgccttcgccaaagcgcgcggcagacacgttggtcttggtggcataggcgccaagcacaaagccgttgtcaaagcggcgaatcacttcaagggtcacgccgcggtcgcccgccaggtactggcccgcgctgatcttggccatgacgccgttccagccggtgtcccaatacagggtggcgtggccggtggtcaccttgtagtcgcgcaggccaaagtcctggttgaagtcgcgctgccgcacgcggttgatgtccacgccaaaggccacgggtgagcgtgcgggccggtacagccactcggcgcccacgccggcaaacatggattcgagcaggccgccatacatgctgtagtagtggttgctcgacatctgccccacgtgcgtgagctgcagcgacggaatggtaaagcgcttggaggtgacgtactcgcgctggaaggtgcgcacgcgcggcaggtcgctgggcgcggtgtaggtgaacttgtcgtagttgtcggccagccgcaggttgaccgcgccgctgagccaggtgcgcggagtaaagcggtattcggccgtggcctggatgccaagctggtacagaagaaacgcgtcgggcccgccaacaatctggccatagctcggcgcaattccaaaggtgaacttgtcgcgggggcgcacccaaggggcctgtgtctgggtggcggcggcttcggtggcaacgctgccttgcgcggtgctgctcttgtcgttgggccggggcagttcgggttcgtagtcgcgcttggacacggcgcgcgccgcatgcggcggcagggcctgtatgcgcacggccacccactcggcgcgatcgatggcctgtgcatgcaccgcgagcccgcgttccgagtaatgaaagacaaagctcttgatggtgtccggcgcatcgtggtggagcactgcaatggctttttccacgcgcgcggtgcggtagacggtgttgctgtcgctcacccacacatgcagcacgtcgtccttgggcgcaatgcgctcgacggtccactcggtcagtgcctcgatctctgccgcggttgccgcccagccgggcgagcgctcggccgcctggggcctgaattccggcagcggccggtcggccggcttgggcgactgcgacgccgccaggttgcttgccagcgtaaggccaatcatgaacttgtcgccacgctcgaagccggcagacagcgtgaccttgggcgacacgcggtaagaaaggccgatgttgaagggcgagcgctggcgctggttgttgctctgcggctcgctttgatagtcgttgccgtcgtactcgagcttgagtgtgagcggctcccacggcgtgcgccactgcacgccgccaaagagggcggccgggccacggaagtaggagccgaatctggcttcattggtgctcgaccgggcgcgagtgtcgaagcggctgcccagcagcttgaaggggttgctgatgttgccgctcgcgcccaggtaaccccacccaatgccaaggctgaaatcgaagtcgtgccagcgcttgctggccaccaggtactcaccggagaaaaggccggtaccgccaaggtcgcgaaaacccagcgcaagctcgggcacgcgggcggtttccttgagcagccgcaccttgatgtcgatgctcttgtccttgttcgactggccggtcgtgctggcttcatacgcgcgattagagatcgacgtgtagcgaaagccggcttccagccagtccagcggctggaacatgaagttcagccgcgtgtagggccagatcgaagtgaacgacgagcgcacgtcgccggccagtcccatgcgggccgatggcgtttggagcaggccgatttcgccccagtcgttgccgctgatgtcgagcgggcgcggctgcgaggccacggcctcggggagggtgccggtgacggtggcggtcgcagtgggtgctgcgaacaccggcgcgttggcagccgggggcgccttgaattcctgcggcgacgggccttgcactgccaggaacttgatcatgccttccgacaggcccgccaggtcggccatgcggctcggcggggcccagatccatgcgccgggcgagggttcatcggcgggctcggcgttccagcctgcaacgccggcgcgcgcggtgcggccgtcgggctgcgcaatccaggcccagtcggcctggccgccgagtccgcaggcgctgagatagtcgagcaccgagcgtccgctttcgtgtggcacctggcaaaagctgccgtcgggctgcaccacggtcaaagaccgcagcggagccggcggcacggcaagccgctggccttcgctgagcaccgggtcttctctcgggttcgcctgcagccagcgcgcatcgacgatgcccagcgccacgcggccggtggccggcaggctgttcagcatggcaaggagccgctcgcgcgtggcacgttccttgggcgagggggccgatcgaacagacgcttcaacgcgcaccagcagcgtgtccttcaggtattgctgggccagcacttcttgtggcacctgccatgcgaggcccgggccggctgcttgctcgggctggcgcagcagccagtcgctgagccgctcgcccgggcgcacttgcgcggcgtccgcaggggcgctggtggtggcatgggcgggggacatcatcagcacgctcgctgcggccagcagggtgaggtgaagtgggtgggtgaccgggccgggcgggggcaaggtcatgaaccggcgcttgacgaagcaactttggccggcgcagacggattccaccgttcaaagctcaagcacagatcacgggaaaggcactgctcggaatagaccacctcgagcttgtcgccaacaggggccaagccaaagcgggctggcggcagcgaggccgaagccgggcgcgtgctgctgcgttcctcgatccagcgcagcgaactggcgggcctgccggccagcgcggtgtcggtggggggctcgatgggccgctgctcgacgtcgtcgcgtatggccgagcggtagccgggcatcaggtcgcgctcgcgctgaaagcgtgctgtcgcgcgattagaagcagtggcagagggccaagcaggcgcattgaaaagacgcacggcgcgccagtcggttgcgaggccggccgttcccaccaggcgcccatggcgcaagcgcaccgcttcacccgaggcgctgtaccagacctctgtaggaccttcgggatgaggatcgacgtttccgagcacgagaaagacggtgcggccctcgaaagtggcgcgcaaatagctgaattccggtcgaaatgtgtgggagtccgaggccgaggcgttgtcgttataaaggtgccgggccgtggctagcattgccgaggagcccgacgagcatccggccaaaaaaaaggatgatgcgagtacgcagcatcctagtttttgcactgcgccagcggtgcatccgactctcgctaggaacccccccttgcggagggctccagtcattacctggtgccggtggttccagtgccagtaccggtgccagtgccgccgccaggaaggaggaagccgccgccaccattgccaccgccgccaccagcggcagccgccagcagcacgccgctaccggcgatgatgccgacctgttgggtcgtcaggccgccgccgccggctgcgcgcacggcagcagcagcgtccactggtggcgtgggcagcgtttgggccagtgcgggcgcggttgccacggctgcaagggccaaagctgcgatcaggtgacggtgtttcatggatcttccttcgaacagaacttggaagtgaacggggttctacaaatcgtagtaacgcagtgcgcgttgttacccgtgaacgggttgcatgttaccactgcacagagggcggcggtaggcgcaagtaggtaacagcgaaggtggcgttgcgtcgaagcggcagtgctttcgctcgtagaaaactaaaatctgaacgcgccgggccgaattgaaggtggtaaaacttcagcactacttgttgggtaactctgttacacgtgcaccaaagctcaattgaggggttttctgctccgcaactgcgtcggcgccatgcaccagccgctcgaacgcgtcctccgatcccatctgaccccccccttgagcatgatctccgtcgagcgccgggttgtcgctgtgaacccggcatagcgacgcgcccgcgcccatgtcggccacgtaagaaagcccccaggcatcgagcgcccgcacggcgtggctcgaggtgtcgccaccggcaatgccgacgcgttgcagtggcaccttggccagcaccttggccagcaggtcgccgccggcgcgcgcgagcgcctgggcatcgagcatgaattcagtgacgtcccggccggcggggcgggtacaggccagcacgttgcagccgcgtatcagcgcgtgggcgatttcttgcgcgtgacgctccagcgtggcggcgttccgttgcgcgagctttggcgcgtcgagccacacgaggtcgaaggactgtgccgccgccacctgacgcgccgtcacgggcgacaagctccccgcgagcaccagcacggggccgcgcgcaggagcgacggggcgttgttcggcctccgcgttgctgcgggcgccgagtgcggtggccagcgcatcgaccacgctgctaggcccgacggccagcagcgtggcgcggcgggcctgcgcccacagcacctggccgatggctgcgagctgcggtgcgtcggccacgtcgaacagcacggcggcggtttcatcgctgtcggcaaaaggtgcatgccatgtgcgccgcagcgcctcgccgagcacttccggtcacttggaatcgggcaagaacgtttggtggcaatctggacgtgtggacggcgcgtcatgggctggcaggcctgtggaaaacctggattgacaagaccacgggcgagatccgcaagagctacacactgctgacgctcaacgctgacgggcaccctctgatgagccgcaggcaaaaagcccgatccgaagcggccaccctacaagaagctgttgaagctgctgcccgtcgaagtgctcgaagctgcgccagttgcggcttagtgcatgtgccatgcaatcttccaccttactccttgccgggcggcgtctggtgattcagaaggaagtctacaggcacaccctaacggtctgtaacgtcgccctttgggtagctctcaccgggacaaaatggcttcctttgctctgtgcagggtcaatcatgttgaattgggttcagcgattcaaaaaagtatcttctcgcgacgccccggcgcgccgcgggttgatggtttcggccctgttgcttcctttcgctgcaagggccgccggcgagcagactccagctgtgagtgaaggcaacgcatcgccaggtatcgcgaagcgggtgggcgaagaggtcgggagtcaattgcggggattggccgcgaccgatggcgcatctcggatcggtttttctcgcggtgaggagggcgcggtggcgcgctcggtagagaagaagctgcgctccctccccgtgacgcccgatgactttgataccgggggggcggacaaggccgccgccattcagaagggcttcaacactgtccgatctcgattgaacattgcgctttctcagtcggtgatgcgttacggcagcagagttattgaactcgagccgggcgtttacgactatggcacgacactcgaattcgacggcgacgtgaagattgcagccaaaggccccaagggctccgtgatcttgcgctacaccggctcagacatcgctgtggtggtgaactcaaagcaaatgacattgcagggggcgcctggaaacacccgagttttcgagtggcataacgtcgcactgcgcggggaccgagcgaaagaaggcattcgcatcggggccaacaccaacttgtcgatcctatttcaaggcagcgaagtgtctggaattcaggggccaccgatcaattgcggcgtgtccgtttactttctcgcgttgagaaaccacacttctcgattcaaccaggcgcccatgtacgttggtgagtactgcgacatgttcaccatcgacgacaggtctctattttcagccaacaacaacgggtcgttgttgctcgaatgcccgacggcgctgatcagcaacagcgattttgagctgggcagcggtcttgctgagatcgaggtgcgcagtcgggccgcgccgatttccaacgcgcgccacatcaacattttcaagaatcgttttggccccgaggtgtactcgggacgatccccagtgcagtttgatattgcgatcactgaggagtcggggctcccggcggggaatgccatcgcagggctacagtgctgggcaaacgaccactttagcggtgggaggtttgcgaagaagaaagctccgattctgatggcagcacgcacgcgaagatttgatttccgcggcgagaagttcgctcccccctccttcgagcttccgtacctgatcgtgcctggcacagacgattctgggccaacaggcactggcgcagaatttaactctcgcaccgatgatttatcgctcgttcacccctctcttcgaggcctctttgccggcgagatggtcagtcaaacgagggtgcgcgcggtcaaggcttgcccggcgttcacagtcgtctatgccctcgggcatggcgccgtggccggcgttcccgggggcatgttgaacgtctcggcactggttccatctgtcagcggcgcgaactacgacagggccgtgggcgtcacatcgtcggatgcaccggcggcacagccgtgctgggtcgcagtcgatggagcgcaaatcacaacctctgtgaatggctcccgcggttcgttctggcaaccggtctatcttggcgcctctggccagctgacacttgccgcaccggccgagcccagggctgcgttgcgtgtcggacgcctcctgacccttgttgaaaacgcgcaggttttgatcgatattcaaaagcccagttaagcgacatgcgtgagcatcctcgccaacgccggcgaaggcgcggcaacctgcgcttgccaagaccctcaagaagcccactgccatcgaccgtgtacggtgcccacttcgacagcgcttctcatgaaagagcaatcgatccagccttcggaaagagccctccttgatctgcgaggtccagcgtcttgcgcaagatttcgtcgactagctcagtcatcgggtgaaggtagccaccgatctcttggtgctccagaaaaattccctcaccgaatccaatgtaggtcttcattgagacctccggttgggctccaagtcttgggtcaaacaacagaaacaacagctcttgggattcctcggaccagcgagggggaagaatcaagacgggctcgaacatgcagtcgttgagcccttccgggtacttcaaaagtatctggccgtcgatacgggatctgacattcagcaggctagccccgtgactacatggaaccaagtagcgatgttcgttgatatttctcagggtcgccagcgcatagagcaagcggttgccgtcaagttcgtcatgtgccttgcaatccagcatgtaggtcagaacgggttctggaatgtctttgctgttgcctgtgcgaagcttgtcgaactcagctttcgttttggcgaaagggaagtatgtcttcttgggcactgcaatccccgaggcctgggcacaggcataaccagcatgatcgagcgccgatctcaagtcatgcgcggcgcttctcacggccagcgggatcgacgtgggtataggtatcttgacgcgcattgagatcgcgctgtatggtgtgtctttgactggtgcgaccactgactcgaatggctcacttgcgtaccaggcatggatcaactgccttagcccgtcaagagttgctctcgtctgttcaagaaggtgaaagctgctgtccaacgggtgtgccatccgtgtctcctcgttcgggcctgctcagcgaaatgcctggtcgagccgggcaagcgtagcactccagtcgagcggaccaaccggtctaagcgcggagttcccgctggatttgccgaagaccctcgcgcgacgctttcgccagacgcagttcttttccgtggcgcacggtacgcccaaggagttcctgctgatttagccactgatgcgcgcttgtgcccgttgtcgcctgcggtcgcccaatggctccagccagtgaggaattcgtgggagacgcattagcgataatggaagcttgcaaggcgaattacccagacggatcggttgacgcggcgcagagggtgttttgggcggcggcttgctaaactgttgatttcattggattagttccgattgcaaatccgtctagcccggttcgactccgggtcgcgcctccactaaattccctgctaaatcaacagcttagatgcctcggacctcccgaggcatttttgtttctgatgtcgcccgcctcgatgcagccgcccgaagtggtgggctgcccagcgcctccgcctatccccgcgagcttgcggcaagccggcgagcgactgaaaacgcaagaggactattccttgcgtgcgcagcggaatatcagagcgccttcagtaagccgcgcgcgaggcaggctccgcggcaggcggcgcaccggtgaaatcggcggccagcttgcgggcggcgcccgcgtacagcagcacgtcgacacccaccgcgacaaaggtgcagcccagttccaggtagcgccgcgccagcttcgggtccgaggtcagcgtgcccgcggccttgccggaggccacgatggttcgaattgcggcttcgatggcggcctgcacatcggggtggccgggccggccccgatgccccatcgacgcggccaggtcggccgggccgatgaaaacgccgtccacgccatccacatcgcatatctgcgccaggttggcgagggccgccacggtttccgcctgcaccagcaggcagacttcctcgtcggcgatgtcgaggtagtcggtgcgcgcgctccactgcgacgcgcggcccacggcgctgccgacgccgcgaatgcccagcggcggatagcgcgtggccgacaccaatgcccgtgcctgttcggccgtatcgaccatcggcaccagcaggttcttggcgccgatgtcgagcagttgcttgatgagggccgtgtcgccctgcaccgcgcgcaccaccggttgcgcggcatggggcgccacggcctgcagcgcggccagggttgagcgcaggtcgttgggtgcgtgttcgccgtcgatcagcagccactcgaagcccgcggtggcgctcacctccgccatgtacgggtcggccatcgagagccagaggccgatctgcgggcggtgcgcggccagggccgtcttgaaagggttgttggcgggcatgggagaggtctcttcagtaggtgatgttgcgtgcgtgcggtgtcagctcacgatccccaggtgccatgggacgaattcatgatcgccaaggcccagcgtttcgctgcgcgtccgctcgccggaggcatggcgcaatatctgctcgaagatctgctgccccagctcgggcaccgagagttcgccgtcgatcaccacgccgcagttgatgtccatgtcctcttcgaggcgcttgaacatcggcgtgttgctggccagcttgatggtcggcgccggcttgctgccaaacatcgagccgcggccggtggtgaagcagatcagctgcgcgccgctggcaatctgcccggtgacggccacggggtcgtagcccggcgaatccatgaagacgaagccggcctggtcgataggctccgcgtactcgtacacggcctgcagcggcgtggttccgcccttcatggccgagccgagcgatttttcgaagatgttggccagcccgcccgcctggttgccgtgcccgaccacgccgttgaactgcgcgttctggccggccgcatagcgctcccaccaggccagccggtcgagcagtttctggccgacctcgggcgtgacggcgcgccgcgtgagcatgaattccacgccgtggatttcgggggtttccgaaagaatggccgtgccgccgtggcgcaccagcacgtccatggccgcgcccagtgcggggttggccgtgatgcccgagaagccgtccgagccaccgcactccaggccgatcttcaggtggttggcgccgacgcgggtgcgctgcgcggcgttggcgtcgggcagcatttcctcgatggcgcgaatgccggcctcgatggtctggcgggtgccgcccacgtcctgcatcaccatcgtgcgcatgaggcggccttgctggaggccttgcgagtcgaccagcgcatcgacctggttgcgctcgcagcccaggcccacgatgagcacgccggccaggttggggtggcgcgcatagcccgccagcgtgcggcgcagcacgtcgaaatgctcgctcggcgaagacatgccgcagccgctggtctgcgcaaaggcggccacgccgtccacgttgggaaaggccaccagccgctcgggcgtgaagtgcgccgcaatgcgcttgatgacggtggccgagcagttgaccgacgacaggatgccgatgaagttgcgcgtgcccacgcggccgtcggcacgcacaaagcccatgaaggtggcgcgctccgcatcgggcacgtaggccaccggccgcacgtcctggcaaaaggccggatcgcggtaggagtcgaccagcgtgaggttgtggctgtgcacgtagtcgcccgcctccaggtcgcgcgaggccacgccaatgacggtgtcgtacttcttcacctgctcgccggccgcaatggcgcgcgacgcgatcttgtgccccgcgggtatctgcgcacgcgcgcgcacgccgaactcggcaatcgtttcgcccagggcgatcgggctcttggcaaccagcacgttgtcgtgcgggtgcaggcgaagcagggggctgtcgttcatcaacccttctccatcagttccttgaggttgagcttgcggatcagctcggtctcctgcttgtagacggcttcgacatacttctggtagtcggggccgtcctggtacatgaccggcgcatcgatgctgtcggcaaccttcttgaattcttcgctgttcaccgccacgcggaacgcatcgcgcagtttcttttccaccgcgggcggcagcccgcgcggcgcgccgatgccgttgggtgcttccaccaccacgtcgtagcccagctccttgagcgtgggcgtgtccttgaagcgcggcgtgcgtgcttcgccccaggtggcgagcaggcgcagcttgccgctttccacgtgcggtgcccaggagctgctgtcggccagcatgtcgacctgttcgcccagcacgtcctgcagcgccgcggcgccgcccttgtaggcaatggcgttgaacttgacgccggcagcctgcgcgaactgctccatgcccacgtgcgtggcaccgcccacgccggcgtgggcatagctgatcgcgcccggcttggccttggcctgcgccaccagctctttcagcgacttgtacggcgagctggcgggcaccgcaatgccgaaggtctggcccgaggtgcgggcgaggtaggccaggtccttgagcggattgatctgcacggtgccgatctgtgcaaagcgcgtcaccgagatgggaatctgtccgatcgtgtagccgtcggggcgggccgaagccagcgccttggtgccaatcattccggaagcgccggcgcggttttccagcgcgatgggctggccgagttcacgcgcggcgatctggcagatggcgcgcatcgagcggtccgcggtgccgccggcgggccacgggcagatgaaggtgatggggcggtcgggatagtcggcggccaatgcgcggccgtgtacggtggccagcgcggcggcgccgaggccgcccagcatcagttgacgccgctgcagggagcgatggatggtcatgtgtcttgtctccgacgatttgtagttcgatgaaagccgagaccggattcttcagtagacaatcattgcaatccaatgaaatagcggactcgcttcatagcctggaggttatgtagtcgaagaacgggccgcaacaaccacgatgagccagatcgaccgcgtcctgcgttccaacctcaagctgcgccacctgcaaatgctggtggcgctcgaccagttccgccacctggggcgcgcggccgagttcctgtcggtgacgcagccggcggtttccaagtcgctggcagaaatcgagcgcatgttcggcctcgcgttgttcgagcgctccacgcgcggcaccgagcccacaccgtacggcgacagcgtggtgcgctttgcgcgctcggtgctcgccgactacgaccgcacgcgcgacgagatcgccgcggtggccagcggtgccgcgggccgcaccagcgtgggcgcaatggtggtggccatgccggtgctgatggctcgcgcggtcgagatgctcaagacgcactcgtcgcaaaccacggtgctggtggaggagggcgacctcacgcgcctcctgcccaagctgcgcctgggcgagctcgacttgttcgtcgggcgcctggaacccggctacgccgcgccggacctggaaaccgagccgctgctcgcagagcccatgaccgcggtggtgcggcccgggcacgcgctcgtcgccaagcgccggctgggctgggccgaccttgccaaagagcgctgcgtgatgccgcccccttgggcgtcgctgcgcgtcaagctcgaccagatgtttttcaaggacggcgtgcatccgccggccgacatcatcgaatcggcgtcctttctggcgcagatcagctttctgcagcagcgcgatgccgtagctttcatggcgcgctccgtcgcgcggcatttccagcagcaggggctgctgaaggtgctgtcgctcaaggtgccgatcgacctgccgccggtcggcctcatcaccatgcgcggccgcaggcgcacgcccagcacgcagcaactcatcgagtgcctgcggcgcgctgccaggatgaagtgatgcggcgagcgaagccgtgcgccggcattgctcagcctgcaccgttgcgcttgcccgcgtttgctgtgagaatcgcgaccattaacaattgttaacactttggtggtatttcctcgatgaaccgcggcgtctctttaccgggtgtgcattccacgctgcagaacggcattgcccacagccgtttcagcgtggccgcggagccgccgcagcggcggctgacggcgtggagggagcgcgtcgggcacgtgatcgacgtgctgccttcgcggtccgacctcgagaagccgttcaacgcgtcgatcgaccgctatgagctggacggcctggccttcaccgattgccgctcggacgccatgtcgctggaccgctcgctggcccgcatctcgcgcgacagcgtgcgcagttttgccttgcacgtgttcgtcgagggggaggtccgagacgtctcggttcgatcgctctcgcgtgccgccgcgccctttgccgccaaggtgctcgcgctcgacatgggacagccggtgcgcatgcggcgcaccgattgccgggtgctcaccctgtttgtgccggccgccgtggtggaagaggtgtttcccgatccggaagccatccacggacttgccatcgagcaggccgagacgccggtcgccaggctggcggtcgaacacgtggccgcgctggccagccgcgtggggcgcatgaacgccgccgccgtgcaagccgatgcgcgtgcgggcgcgcagcttctggtcgcggccctgggcaggcaggcgcgcctgggcgacagtggccgcgcgggcgcccgggccgccgtgttcggccaggcccggcgttacatccaggcccatctgcaccgtgcggacctttcgcccgacgacgtgatcgcggcgttgcagctctcacgcccgactgtgtaccggctgttccagcatgaaggcggcctgggttcctacattcggcacctgaggctgcgccatgcggccgacgaactggcaaggcacccgagcgcgatggtggcggacgttggctatggcgccggcttcaagagcgcatcggacttctcgcgggccttccgccgtgcctatgacatgtcgcctcaggatttccgggccctgtcgagaaaggccgcttaggttgcctgccgcggggtcattcggtgacccctccgggttcagcggaacgaatcatggaaaatcgtgaaataagtcctgttctcaccgatttttttcgaggattgagacgcacggtcaagcccgtgagccaacaacgcgcaatctcgtgcctgtgcgagaggccccgaggccgccgccaagcctgaagacaaacgtcgttcccatgtacctgcatcctcttttcgccaacgtgccgccggctgagcgcgcggcgttgatcaagtgcagcgagcttcgctcctatcggcgcagcgagacggtgatggcggcgcaagagtggacggaccgcatcttttgtgtgacgagcggcttgttgcgcgtggtcgagcatggcagcgaccccaccggggacgtaacgaccgacttcattcgccgaaacgattttttcctgggacccactctccgcgaagaccgctacatggcccggcagacgctggtcgccgcgctgccgtcgtcagcctacctggtcccgattccggcggctcgcaagctctgcgaagcctatccggaggttgcaatgggaatgttcgaatacgcggcaacgcgcatccggtcgcttcgcagccagcttcgcaagatctcggcgctgtcgtccgaagacctggtgagccgggtgctccaccagctgacccagctcgcgccggcaagtaccggcggcttcgacaagcgcattacccaggcggtgatcgcgtcttacacggggctctcgcgcgaagtggtcaacaagatcatgcgcgacatggagagccgcggcctcgtctggcgcgacgaacacgcggttcatgtgccggccgatttcgcgtcgacggacatcggtggcttgcacgaaagcgggccggagaccgacgagttccaggggggagcggggacggaggcgaattcgtaaccacccgccgggtgggctccagagttgcattcgcgctgcctccccaattcatgggtatgcgtcaggcggtgccgtcccccatcatctcgatatgtatctgaataccttggtctcggtgttgccgcccgcagaccgtgtggcattggtcaaggccagcgaactgcgttcctaccgccgcaatgaaaccgttcttgccgtcgacgaatggacggatcgcttctactgcgtggggagcgggcttttgcgcgtggtcgaacacggacgcggcagcggcggcgacgtcaccaccgaattcatccgccgggacgatttttttctcggttcctctttcaccgaagaccgccaccaggccacccagacgctgattgccgcgctgccttcgtcggtgtacctcatccccattgccgcaatgcgcaagctgtgcgagcgccatccgcagctgtccttggctctgctcgagatcgccatgaagcgggtgggcgtgatgcgggggcagcttcgcagggtttccgcgctgtcgtccgaagatctcgtgggccgcgtgcttcatcaactgacccagctggcgcccgcaaaaacgggtgggtacgacaagcgcatcacccagtcggtcatcgcgtcctattcgggcctctcgcgcgaggtggtcaacaaaaccatgcgcggcatggaaaaccgtgggctggtgcaccgcgacgatcacggcgtgcatgtgcgcgcggatttcgtgacaaccgatttcgatctgccgctggccgaaccgggtttgggcggggctgcagcggcttcgttgcagccgtgcgcctgagacggcgaaaaccttagttctcgttccttttcggcgccagttcacatttgtgacatgcgccacatccggtgttcgaaagcagagctacaaggcgtttcgttcgtagcatggtgtctgtttcatccatgttctccgaggcttgcagcgggaatttcttcagttgccaagtcttgtggaacgccagagacagggagcttttcaaatgcacagcgcaaacacagtaacaagaacaacgtggcacccatcctggcagcaggcgggccagttcacgatcggcaggttcccagccgcgaacgaagatcggcgcgtaaattgcgccgcggctgcgggggctttgcgcgatctcttcgcgaaggcgaatgcaaccgatctcgcttccctgatgcgctctgtcgaattgggcgactctcccgcggcatcgcaaattgcgcggcgtatcctccgttcgctttccgcgtccgccgagcagaaggctcccgcggaaccgagggggctgctgtcgccccgtgaactgaaagtgcttcggctcatctcgcagggccggagcaaccggcagatcgccgaagaagcccatcgttcgatcaacacgatcgaagcccagctcaagagcatctaccgcaagctgaacgtcaagtcgcgcacccaggcggtttgcgcggccacgcagtggggcctcatgaactgggacgaaacctcctgagttgcaggaggctcttcgtgcggggctacttgccctgcgtagttgcaggcggggcctggggcgcggtgatcgaaggtgcggtattcgagggagcgacctgcggtgcgctctgggtcgtcggcgcgaccggcacttcttcccgcgtctggggcatgaagttataggcaagcgcgagcaggaagatgaagattgccgcgccgatgccccaccggaacacgcgctggttgtcgcgctcgtcgcttctggcttgttgaggagtcatctcggtcacccttcagtgcagttcttcgacgctgcaccggcgcccgagaacgagatgtcggacagcggctcggctcgctgtcgcgaaaaagcagaacaatgcggcgcctgatcaggccgtggccttggcgtgctcgatgatttcatgcaccgtgtgcgaaagattcgagagatagagggcatccgccgaaaacgaacggctcatggcactgatgagctggctgaaatcctcgtccgcggggccattgcgggcatcgccgctcccacgatgcagcagcaattcatcgatccggttctgcacccgcatgtagtcggcacgcagcagcacgctgcgcgcaagcagtacatccagggtcagaaggtccagtgcggtcatgggatgttcgcctgtccgaaggttcggatggcgggcgactgcaatgcgtaggaacctttctcgtgtgagccggctcggcagactacacgcggaggaaagcgccctcggcaaaatcgaggggaaaaacagccgcaaaaccgaaatccggcaccgacaaggggcagaatttgagaatcgaacgagcgcgcggcaagccccagggcgttggctgcgcaaccgacattccatgcccaccacatcgaatccgcctccgccttctgccgccaccaatgaacgcaagctcacgcccagcacgctgagcttcccggtcatcggtatcggtgcctccgcgggcgggctggaagcattgatccgtttcttcgagcaaatgccggccgacccgggcatggcctttgtcgtcatcctgcatctctcgccccagcacgagagcaacgcggcggagatcttgcagcgttcgacgcaaatgtccgtgaggcaggtcacgcagcccgagcctgtggaagcgaaccatgtctacgtgattccgccgggcgtcgagctgaccatggacgatggctacgtgcgggtgactcccaacgagcacgtcaagcgcccccaggtggcggtggacgtgttctttcgcaccatggccgaggtgcacaaggagagggctgtctgcatcgtgatgtcgggcaccggcagcgacggcgctgtggggctcacgcgcgtgaaggagagcggcggcctcaccatggcgcagtcgcccgaggacgcggcgcacgacggcatgccgcgcgcggccatcggcaccggcgtggtggacatcgtgctgcccgcggccgagatgggcccgcgcctggtcgagcattggcgcaatgcccagcgcattcgcatgcccggcgacgagcaggcggaactcgccccggaggcccccagcggcgacgccaccaagcaggccgagaaggcactgcaggagatcatgacgctcttgcgcacctacacgcggcacgacttcgtccactacaagcgcgccacggtgctgcgccgcatcgaacgccggctccaggtgaatcgcctggtcgacctgccggcgtaccgcgacttcctgcacgaacatccggaagaggcgagtccgctgctgcaggacatgctcatcagcgtgaccaacttctttcgcgacccggaggccttcggggcgttcgagcgcgacgcgcttgtcccgctggtcgcgagcaagcagccccgcgagcaggtgcgcgcctgggtggcgggctgcgccacgggcgaggaggcctattcgctgagcatgctgctgcgcgagcaggtgcacctgcagtccaagccgctcgacatccagatctttgccaccgacatcgacgagcgcgccattgccacggcacgcaagggcctctatccgcagggcattgccgaggacatctcgccttcgcggctgcagcaattcttcatggccgagcaggaccggtaccgcgtcgcgacatcggtgcgcgagccggtgctcttcgcgctgcacaacctgctgcgcgacccgccgttttcgcggctggacatcatctgctgccgcaacctgctgatctatctcgaccgtgcggcgcagacccatgtgctggagatgttccgcgtcgcgctgcggccgggcggctatctgtttctgggcacttcggaatcgatcgatgcggtgggcagcctgtttacttcggtcgacaagaagaaccgcatctaccgcgtgaacccggagctgccgcccgggcgccacttgccgctcatcagcgatacgccgctcaagcccggctgggccggaccgatggaagcgctgcgctcgcccaagcgctccgaacggccgagctttgcggagctgcaccagcgcgcgctggaacagttctccccgcccagcgtgctgatcaacagcgagcacgaggtgctgcacctgtccaacggcgtggggcggtttctcgagcgggcgagcggcgagccgtcgaaccacctgctgaacaacgtacggcccgatttgcgcctggagctgcgaaccgcgctcttcaaggctgcgcagacggcccgcagcgtggagacccgcctggtgcacaggcgggacgacgggcggcaggtgttcctcaacatcacggtgcgtccgctgcagccgcagaaggacgacgacgacaacaaggaagccgctccacaactcacgctcgtggtgttcgacgaggtggaagacagcatgcgcacggaaggcggcgagccggccgacgcggcgcgcgagctgctcatcggccagatggaaggcgagatgcgccagctcaagctgcatctgcaggacaccattgaaggcgccgaaacatcgacccaggagctgaaggcctccaacgaggaactgcaggcgatcaatgaagagctgcgctccgccaccgaagaactcgagaccagcaaggaagagctgcagtcgatgaacgaggagctcgtgacggtgaacttcgagctcaagatgaaggtggaagagcgcggccgcatcaacgacgacctgcagaacctgatcacctcgtcagagattgcgaccgtgttcgtggaccgcggcatgcatgtgaagcgcttcacgccgcatgcgagcaacctgttcaacctgattgcatcggacctcgggcgttcgctgttcgacatcaccagccggctcgactatccggagctggcggacgacacggccgcggccttcaaggagctgcgaagcaccgaacgccacgtaaccagcgcggacgggcggcactacctggcgcggatactcccgtaccgcacggcggaagacaagatcgaaggcgcgatcctcaacttcttcgacatcaccgacctgaccgccgccgaggagcaggtgcgcgcaggcgaagaaaggctgcggctggtggcagccaccacgcgcgacttcgccatcatcacgaccgacgaccagggcttgatcgcgacctggaatgcgggtgcccggcgcatcttcggctactcggaagaagaaatgctgcgcaagccgcttgcgacgatctacacgtccgaggaccaggcgagtggcgtgcccgaaaaggaaatgcagcgcgcactggcgtcgggccgctccgaggacgagcgctggcacctgcgcaaggacggcagccgctttttctgcagtggcgtcacgaccccgctggagctcgccgcgggcggcggcttcgccaagatcgcgcgcgacatgacgggcaccaagcagcatgagcttgcgcaggagcaccggctttccaaggaaaagaaggccagcctcagcgcgcagatggccaacgagctcaaggacaagttcctggccgtgatgtcgcacgaactgaagcagccgctcaacctgatccagatgaacgccgagctgctgatgcacatgccggccaccgccgagagcccgtccgtgcggcgcgttggcgaaaccatcaagcgcgccgtggccagccagacgcgcatcatcaacgacctgctcgatctgtcgcgcatccgcaccggcaagctgcggctgagccacgtgcccgtcgacctgggcgagctggtgcaagccacggcgcacgccgcggtgagtggcgcgactggcaagaagctcgcgctggaggcggactgcgaagccggcgtgatctgcgatggcgaccgcgtgcggatcgagcagatcgtgtggaacctgttgagcaacgcagtgaagttcacgcccgatggcgggcgcatttcagtgcgcgtggcgggcgacgagaattttggctggctcaaggtgagcgacacgggttgcggcattgcaccggaatttcttccgtacgtgttcggcatgttcaatcaggcgagcagcgaagtcactcccatcaacggtggccttggcatcggcttggcactggtcaacgaactgacgcgggcccacggtggccgggtggaggtgcattcggcgggactggggaagggcgcggagttcgacgtctggctgccgcgggtgggagcacatgtggagcccccggcgcacaggacgccggccgaagtcgacctgagcggatggcgcgtgctcgcggtggacgactacgccgatgcgctggccccgttcgccgaggtgctgcggctcgagggcgcgattgtcgacgtggcgccaagcgcaaagaagggcctggagctgctcgagacgaacagctacgacctgttggtgtcggacctgggcatgcccgagatggacggctaccagttcattgcggaggtgcggcggcggccggccacgcgcgagctgcgctccattgccatgtcgggcttcggccggcgcgccgatgcgcgccgcgcgctcgaagcaggcttcaacgcgcatttgcccaaacctgcttcgctcgaggacctcaaggcgaccatcggcaggctgtgaatccgcaggcctggccggcgtcggcgggcggtcagccgatccaccggaagatgaagccgcttgccggcgcgatccactcgactttgtcatccgcgtgcaccgcgggcatggcggccgtgccggtgaagagggtgcgttcctcggccagcagaaactgccgcgcggccgcgccatcggccgccggccccggctgcaggacgcgcaacgtggcgccgctcagttccagggtgtcgcccggttccggccacagcaccgtggcgtccggccatgatgaagatcggagttctccgagcgctgcggccgattcctgcgtgcgtgccgctgtcgagagcagccagcgcacggacccgggagccgcctggccctccgccgaaccgcgccccgctgggtcgatcaatgcccactggccgtcttcgccgccgacgaaatagctgtgcggcgaaccgtcctcgccggccacgcggtggatgcgcgccgagagctgcgtgaccaggccggcctccagcgcatagcgtgcatcgccttggccgtcggggtcgaggcggccgatctcctcgtaggcggcttcttcgatgttcacggcgcggcggcctgcgggcccatcggccaggcgcggcatgttgagcggaatctcggtgagggcgtgcgcatgggccatgcaatggtcggcgctgtcgaagcgtgccagttgctcgagcgtgcgccgtgtcacgttcatcagcttgagcccgcggcgagggtccaccgcgtcggccggcttcagccacatgtgctcgacgatctcgcggccatcgggcttcacgccttgtgcgggcggcatcgctgcgatgaagaagcgggtgtcgaaccggcgcggcatgccgggcggcgtcagccagtggctgaaataggccagccggtccatcgcgagacgccagccctgtgcgtcgcacatggcaagcagcgcatcggtgccttgctcggccgcatggcgcatggcctcgagccggccggtgggcagccggtcgagttcgaccaggcggtcttcgctgtcgctcgcgaacaggatgccggcctcctcgaagcattcgcgcaccgcggcggcgtagtagtcgaggccgccttcgggcatgcccaggtgcgtgctggcctcgctgtcgtccagtcccttgcacatcaggtgcaggctgcggtcgtgcgtgtcgaccacgccgcccggaaacacgctggcgccgctgttctggtcgttggctttttcggcgcggcgcagcagcagcacttccatgccctgggcgctgtcgcgcaagaggatcagactggctgcagtgcgaatggggcgcggcacggacgatggcggggccggcgcggccgcctgaggcttggcgttcatgggcgccgattgtcgggccaaagcctcagatggcgcgctgcttcacccgcttcgaaagctgctcggcgctttccttgcgctcgctgtagcggtcgacgaggtagtcggccgcatcgcgcgtgagcagggtgaacttcatgagttcttccatcacgtcgaccacgcgctcgtagtaggaagacggcttcatccggccggcttcgtcgaactccagaaacgccttggcgacggacgactggttgggaatggtcagcatgcgcatccagcgcccgagcacgcgcagctggttcaccgcattgaacgattgcgacccgccggacacctgcatgactgccagcgtcttgccctgcgtcggccgcacggcgcccacgctgagcggaatccaatcgatctgcgtcttcatgatgccggtcatggcgccgtggcgctcgggcgagcaccacaccatgccctcggcccattgagcgagcgtgcgcagttcctgcaccttgggatggtcgtccggtgcgctgtccggcaagggcaggccggcgggatcgaagatccgcgtttcgccgcccatggcctgcagcagccgcgcggcctcttcggtcaagaggcggctgtaggaccgctcgcgcagcgagccgtacagcagcagaaagcgtggcgcgtggcgcgaaggcgccgcgctggcaaggcgctcgggcgagggccggtcgaacagctcggcatcgatgttggggagatcaagcagggcgatcgacacggcggccctccgcatcgatgacgacttcgccgtcttccttggtgaacgcgcctttttgcggcgccggcaggatgtcgagcacctcttcggaggggcggcacagccgcgtgccgatgggcgtcaccacgatcgggcggttgatgaggatcgggtgcgcgagcatgaagtcgatcagctgctcgtccgtccatttcggatcgtccaggccgagctcttcgtacggcgtgcccttcttgcgcagtagtgcgcgcggcgccatggccatcgcggcgagcagttcgcgcagcgtttccttgctgggcggcgtcttcagatattcgatgacctgcggctcttcgccgctgttgcggatcatcgccagcgtgttgcgcgaagtgccgcatgccgggttgtgaaagatggtgatggaggaggtcggtgattgcattcatgcgattatgcaactattattgaaatatggaagaacaagacatcgtcaagtcgctcgcagcgctggctcaacccatgcgccttcaggtgtttcgcgccttggtggttgcgggccccgcggggctcacgcccggcgcgctggtcgatgcgcttggtgtgcaggccaccagcctgtcgtttcacctcaaggagctgacccattcggggttggtgacgcaggagcgcagcggccgcaacctgatctaccgcgcggcgttcgggcagatgaacgcgctcatcggctacctgaccgaaaactgctgccagggcgaggcgtgcctgccccaggcagcgcaggcctgtgcttgctgaacaaggagcaaccatgaagcgattccatgtgcatctgaacgtccaggatctgccggcgagcatcgccttttattccaggctttttgcctcggagccggcgcgcgtcgagagcgactacgccaagtggatgctcaccgatccgccggtgaactttgcggtgtcgacccgcgccaactccctgggcatcgaccatctcggcctgcaggcggagaacgaggaagaactcgcggagttgaaggctcgcgttgctgacgcagacatccaggtgttcgacgagggtgccgccacctgttgctacgcccgcagcgaaaagcactggatcaccgatccgcagggcattgcctgggagcacttccatacgctgggcgacgtgccggtgtatggcgagaagcgggcggatgccagcgaggaggccgcctgctgcgcaccgaagacgcctcgcggccgggccgtcggaataccgctcgttgcaaagccggccgcgccggttcaaacccccttctaggcaaactccccatggctcaaaaaatctacaacgtgctcttcgtgtgcacgggcaactccgcgcggtcgatcatggccgaaggcctgctcaactacatgggcgcgggccggttcaaggcgtattcggcgggcagtcatccgtcgggcaaggtcagtccgcatgcgctgcgcacgctcgaaagactgcggctttccgcagagggctatcgcagcaagaactgggacgagttcgccaggcccggtgctctcgccatggactttgtgctgacagtgtgcgacaaggccgccggcgaggtgtgtccggtatggcccggccagcccatgaccgcccattggggtgtggccgatcctgcggctttcgagggctcggaagaagccgtcgagcggcagttcatggatacggcgctgaccttgaagcgccgcatcgagctgatgctggcgttgccgatggagcggctcgacgccatggccatccagcacgagatgcgcgacatcggcaaggtccaggagaccgcgcaatgaccgtcaacgtgttgatcctgtgcacgcacaactcggcccgcagcgtgctggccgaaggcatgctcaatcacctggcgcaaaaggcggggaaggacgtgcgggcctacagcgccggcagcgcgccgagcgggcggctgaatcctttcgcgctcgaggcgcttgccggcgccggcgtggacgtgtcgccgtaccgcagcaagagctgggacgaattcgcgggcgacacaagcccggtgatgcgtatcgtcatcacggtctgcgacagtgcggcgcaagagacctgcccctattggcccggcagcccggtgaaggtgcattggggctaccccgatccttcgaacgcacccggtggcgacgagggcaagcgagtggctttcgagctgacgcgccaggccattgcctaccgcctcgtgcagctgctggcgctgccgctcgaatcgatgcccgacaccgaactccaggcggcgctgaccgcgatttccgaaagctgaaccatccatgagctcccataccgccactgccgcatcgatcgcgccgccccccgccatcggcttcttcgaacgctacctcacgatctgggtcgcgctgtgcatcgtggccggcattgcgctcggccagtggctgccgggcttgttccgcggcatcgcgtcgctggaggtggccaaggtcaacgtgccggtgggcgtgctcatctgggtgatgatcatcccgatgctgctgaagatcgacttcgcggcgctcggccaggtcaaggcgcattggcgcggcatcggtgtcacgcttttcatcaactgggcggtgaagcctttctcgatggcgctgctgggctggattttcattcgccacgtgttcgctccgatgctgccgccggcgcagctcgatagctacatcgcgggcctcatcctgctggccgccgcgccttgcacggcgatggtgttcgtctggagccagctgtgcaagggcgatccgtacttcacgctgtcgcaggtggcgctcaacgacgcgatcatggtggtggccttcgcgcccgtggtcgcgctgctgctcggactctcgtcgatcacggtgccgtgggacacgctgctgacgtcagtgggcctgtacatcgtggtgccggtgatcattgcgcagttgctgcgcaagcatctgctgaagaagggcgtggcgcacttccaggcggttgcggcgcggctggggccgtggtcgatctctgcgctgctgctcacgctggtgctgctcttcgccttccagggcgaggccatcctgcggcagccgctggtgattgcgctgctcgcggtgcccatcctgatccaggtgttcctgaactcgggcctggcctatgtgctcaaccgcaagctgggcgtggcgcattgcgtggccggcccgtcggcactcatcggcgccagcaacttcttcgagcttgcggtggccacggccatcagcctgttcggcttccagtcgggcgccgcgctggccacggtggtgggagtgctgatcgaagtgcctgtgatgctgctggtggtcgcggtggtcaaccggtcgcagggctggtacgaaaagggcgcgaagacggcctgacgacgggggcaggtgatcggcagggggcgccgccgggctccccgcagtgcatgttctccgacatggccggggcggcttcagggccatgatccggaatccggttcttcttcggtgcagggttcatgaagatcgcgaccttcaacgtcaacggcgtcaacggccggttgccgcgcctcctggagtggctggccgagtcccgccccgacgtcgcgtgcctgcaggaactcaaggcgcccgacatgggctttcccgcggccgcgatccgcgacgcgggctacggcgtggtgttccatgggcagcgctcctggaacggcgtggccatcctggcgcgcggaagcgagccgatcgaaaccggccgcggcctcgacggcaattctgaagacagccagagccggtatatcgaagccgtggtcaacggcgtgatcgtcggttgcctgtacctgcccaacggcaacccgcagcccggccccaagttcgactacaagctggagtggttcgagcggctgaacgcccatgcagggcgcctcttcaattgcggcatgccggccgtgctggccggcgacttcaacgtggtgcccaccgacgccgatatttacaacccggcctcatggcgcgacgatgcgttgctgcagcccgaaagccgtgccgccttcgcgcggctgctcgagcaggggtggaccgacgccatccgcgcccggcatccgggcgaggcggtctacacctattgggattactggcgaaaccggtggccgcgcaacgcagggttgcgcatcgaccatctgctgctgaacgacgaactcgcgcccctgctggtcgatgcgaacgtggaccgcgaggtgcgcggccgccccggggcaagcgatcacgcgccggcgtgggtcgaactggcgctgcccgcgggctgggcttgagcgcggaaaattggaaactgcggcggaaaaaccacggttaaccggagtggtgacagacaggttacatttgaagactgtgcactattcaattacttggcctattcctgaggatccattccagtgattaccggagcaacggccgatgccagcttttcccgaggtttcgacgccgggtttgtcatggcttttcagcccatcgtggacttcgagcggcgggaagtctttgcgcacgaggcgctggtgcggggcgctgcgggagagggcgcccaggaagtcttctcgcgcgtgaacccgcagcaccggttcgcgtttcatgaggcttgccgcgtcaaggccattgaaacggcgtccgagctgggcatgcaatcgaagctcagcctcaacatcatgcccaacgacgtggccgggccgacagagtgctttcatacggccatggcggccgccgagcgctgcaactttccggtccaccgcctgatgttcgagatcaccgaaggcgaacgcgtggccgacctgccggcattggcggccgcctttcgcacctacaagggctacggcttcacgtcggccatcgacgacttcggcgccgcctatgcgggcttcgaactgcttgcgggattccagcccgacgtggtgaagatcgacatgggcctggtgcgcaacattcacaacgacccggtccggctcagcatcgtgcggggttttgtcggcacctgtctggagctgggcatccgcgccgtggcggaaggcgtcgagtcttccgacgaagtgcacgcgctccagtcgctgggcgtggaactgttccagggattcctgttcgctcggcccgccatcgccacgctgccgccggttgcgtgggacgccgcctgaggcggaggcacccgcgccctcgggcgccgactcacatgttgctggtcgcgcggacctcttcgatgctggtcttgcccgcaagaaccttgtcgatgccgtcctggcgcagggtgcgcatgccctcctgcatggcggcgtcttgcagttcctcggcgcgggcgccgttctggaccaggcggcgcagcgtcctggagatcaccatcagttcgtgaatgccgacgcgcccgttgaaaccggtgctgtcgcagtgcgggcatccggtgctcgtgaaggcttgcagctgcccgtcgcggccatactggccgagccagtgcttgtgtaccgtctcgcgctcggcctgcatggcatcgtgcgcggcgaatgaatgcatgtagtcggccagcagttcctcgacttcgtcggggcgcatggggcggctctggatgcaatgggtgcagaggcggcgcaccagccgctgcgccaataccgccagcagcgaatccgcaaaattgaacgggtccatgcccatgtccagcagccgcgtcacggtttcgggcgcgctgttggtgtgcagcgtcgacagcacgaggtggccggtgagcgaggcctcgatggccgtcttggcggtttcctcgtcgcggatttcgccgaccatgatcacgtcgggatcggcgcgcacgaaagcccgcagcgccttggcaaaggtccagtcgatgcgtggattgacctggacctggcgcaggccgggctgggtgatttcgaccgggtcctcggccgtccagatctttcgctcgggcgtgttgatgtgcatcagcgccgagtgcagggtggtggtcttgcccgagcccgtggggcccacgcaaagcaccatgccgtaggggcgttcgaccgccttcgtgaactgcgcgaggttgtgctgcgagagcccgagcttgtccagcgcaatgggttgcgccgaggccaggatccgcatcaccacgtcttcgaggccgttggccgtgggaatggtggccacgcgcagctcgatgcggtgctgcggcgaatacttggcgaaattgatcttgccgtcctgcggcttgcgcctttcgctgatgtccaggtcgcacatgatcttgatgcgcgccaccaccacgttgcggtaggtggccggcagctccaggtgggtgtgcagccgcccgtcgcggcggaaccggatgcgggtcttctcctggcccggatagctttcgatgtggatgtccgacgcgccttcgcggtgcgcgtcgatgatcatgctgttgatcatccgcaccagcgagttgtccgactgttcgatgggcgcctcttcgaccatgggaacgcgctcttccttctcgagggtcaccagcagttcgctgctggtacctgccgtgtcgaattcgagcggccgcgaggggtcgtggacgatggtggggtcggtgctctcgctgccgagctttccgtaggccttgtagagcacggtgtccagcaccaggcattccccgatcaccggcaccaccttcaactgcgtgatgaactccacctcgtcgatggccgcatgccggctggccggatcgtcgagcgcaagaatgaggcgcccctcgtggatcatgagcggcatgacctgcaggcgccgcgccgcgccgtgggtgatggttcgcaaggcgttcaccgccaccgggaacacatgcaggttcacgagcggatagcccatcttgcgcaccagcgccgactgcagctgggcgcgggtgaccacgcccatgcgcaccagcgtttcgccgagcggcacgctgcggtcgagcttctgctgctccaggcccgcgcgcaactgttcttcggtgaggacgccgagcgccatcagtgcctggccgatgcgcaggatcggcatgtggctttgaacctccagcgcatgcagcaattgctcgggcgtgacgacttcggtgggggacatgaatggatctccagtggagtgattctgctggggccggcggggcttgtcagcaaaggaacggcgccggctccgcgcgggcgcaattcggcactacgaaagttctcaaatgaagatggcccggtcgatgcgggcgcatcaatccgaaaacccgaaggtgttgcggcccgccgacttggcgcggtagagcgctgcgtcggcgcgcgccagcaggtcggcgtcggtgatggcggcgtcggtgacggcggcttcggtgggctggtggaacgcaatgccgatgctggtcgtgaccctgaggctctggccgtcgagctcgaaggccgaggtgccgatctgctggacgattttccgcgccacggccacggcggcttcgcgcgtgtgcacgttttccagcaccaccacgaactcgtcgccggccaggcgcgcgaccatgtcggtgcttcgcacgctggccagcaggcgctttgcgtattccaccaacacgccgtcgccggtcgcatggccgaaggtgtcgttgatggtcttgaaatggtcgacgtccagaaacagcaccgccagcgcgttgcccgagcgctgggcgcgggccagggcgctgggcaggtactcgttgaaggcgagccggttcgacaagcccgtgagcgggtcgagccgggccaggtcgatcaactggcgctccaccgccttcaaggcgctgatgtccaggctgagcgagaagattccgcgcgtgacgccgtcggggccgatgtcgggcacgtagctcacgcgggtcgtgcggtcgaagtccttcgtccgggtcttggcctcgaactcaacacgctcgccggccagcgcacgcgcgatcatgggcttgcgcgaaagatacagttcttcgcccgccacctcgctcacatggcggcccagcagccgggcggggtccacgcccatccactcccggtacgtggcgttggcaaaggtgatcttttcgtcgcggtcgatgtaggtgatgagtgccggcaggttgtcggtgatggtgcgcaggcgcatctcgctttcggcctggcgcagctccgcctgcttcagcgcggtgatgttgaaggtcatgagatagaagccgacgaagtttccctcggcgtccatgtctggaatcaggttgacctggaaatagccggtctttccgtagagcggcgcctggaccggaaagcgcaccgacttgccctcgcgcaccagcggaaggtagggccgctgctgccggtacaccgccttgcccaccgccttgcgcagggtcacgccgtcgagcgggccgtcgcccaggcccgccatgcgccgcgcgcggctgttggcgaacaggcagttctcgttgctgtcgaagtagcccaccagcgccggaatgctgtcggtcacgtcgcgcagccgcttttcctgcgcggtgagggccttgcgtatgttcacctcgtcggtgacgtcgaaggtcatggcgaacacgccctgcaccacgccgttcgcgtcctggtcgggaatgtagtgggccttgaaggtccgctcgccgatgcccagcgccgcatcgccggctttctcgatgaccaccgtttcgccggccagcgcgcgctcgtaggccggagccacgatcgcgaaatcggccgggccacgcacctcgggcatcgaccggccgaccatcgcgcgctctctgtgcagcgccatgacctgtgcattgacgaaggtgtatttgagcgacgcatcgacgtgcgacaccagcgcaggaatgttgtccgcgatgatgcgcacctgcgcttcgctgtgcgccaggctgaattcgatgcgcttgcgctccgtcacgtcggaggtcatggcgtagtagccgcgaacctgtccggccttgtcgagatcgggaatgagttcggtctggaagtagcggtcttgctcgccacgtctcgcatcgcctcgcctctcgaaactgacggcctcgccggccagcacgcgctcgacggcggccttcatggccgcgtcgtcttcgccgaagctttgagcctcccgcccgatcagctgggccgccccgcggtcgagctttttgcagagcggcgcgttcacgaaggtgtagcggccttgcgcatcgacgtgcgacaccatcgcgggcaggttgtcggtgatgtcgcgcaggaacttctcgctcgacttgcgctgccacatcagcgtgtcgaaggtgcgcgcaatgtcgccgatctcgtcgcgcggataggtgcgcggccccgccgtttcgagggccgggttgtccacgtcgagcatgtgccggtgcaggtgcgtgagcggcctgagctgccggcgcacgaggcccagtgcggcggcgcccgcgaccattgcgagcaccaccgccccgatccatgccgaacgctcgatggcgtcgacccgggcgaaggcttccctgctgggatacatggaccccatgacccagttggtctcgcgcagccgcttgaaggcatacagcccgtgcacgcccgcatggttgacgccctcggccgcgccttcgtagccttccatcggacgttcgatctcggggttgccgacacccttcaggcccgtctggttgatgacgcgttccgtgcgcgggtggtcgatcacgccaccttcggtgctggtgatgaacaggtagccgctctggccgaatttcacttcggcaagctcgcccaggatgttccgttccttcaggttgatggcacccgagatcacgtacttcacatcgcccgcggggtcgagcaccggcgcggtcagggcgatctgcgccaggccggtgagccggttcagatacggttcggagatgacgctggccttggcggcgagcgtctgctggaagtagggccggtccttgatgttcaccctgccgggctgctgcgcaccgctgaggctcgcgatcagatcgccgtcggccgtaaagaatgcgacgttgctgaaggccttccgaagcgacgggtgcttttcgacaaaagcctgcagcgttgccgcatccgggaagtcgttggtcttcacgctgtcggcaaaggtttcgagcaggatgcgccggctgacgaacttttgatctaccgtatttgcaatggccgacagccgcgcgaaggcttcgttttcgatcgaggccttcatgctcttcttcaccagctgcaatgccacggtggcaatggcgaaggtggccgccaggaccacagcggccacaccgagactgaggcgtgtgttcaagctgatgtggatattcctgagacctgatgagttcattggggtggaaaaagcatcgcgatgcggcctgctgcataccgagtgtgtcagaagcgaggagcagggtacctcgcgcaatcccccatgactcgtgggttggcccacggcgtcgcgatcgcccggctttccgctttctttttttcaggctgccgctacttgccggacggataggtttccggaacctcggcatccgatgccgccgcgtcgcgctccagcggctcgaccgcccgggtccggtcgaaatgcagcaacgcatcgaactgcaccggcaggcgggcgaagaaatagtggctctgccgttcggtctcggggcggtagatgacgccgatggcgcgctccagccgccgttcccgcagcgcgaagaagtggcttccttcgccgcgcaggggcagtatgaagcgttcgagtccggtctcgtgcatgaggccttcgtagctgtcgggccgcgaaggaagaacctgcttgcgctcggcggccgcaccccagtcggaagccgccatcacggtgccggtgtgggtggtgaagcccacgagcaccgcgtcgcggccctggcgctcgcgcaccagctggcccacgttgagctcgccgcgctgctcgcccatgtcggtggcgcgcgcatcgcccaggtgcgagttgtgcgcccacaccacgatcttcgggcgctcgctgccacgccacaggtggcgctcgagctcgcccagcgtctcggccatgtgccggtcgcgcaggttccacgacgacacgtcgtcgaggtacatcgagcggtagtacgcctcggcgttcttcaccaggcgcgcgttctgctcggcgtcgaaggcggcttcctcgtcggccgcaatgccgccgcgccatgcggtggccgaagcgcggcgcatctcgaccagcatatcgatcacttcctgccggcaggaggccgtgttgccgagcccggccatgagcccgtagacctgcccgccatcgccgaagcggtcgaagcaggcgtagcgttcgcgcgcgctctgcgcggtgtccggatcggtccgctcgaagtaggcgagcaccgcctcgatcgaggcatgcaggctgtacaggtccagcccgtagaagccggtctttccctgcgccgggccggcctcgttgaaggcgcgctgccactcgatgaagcccgctacgtcttcgttgcgccacatccaggtcggaaagcgccggaagcccgccagcgcatcgcgcgcgctggcgtcttcgctgtcgccgcggacgtagcggttgacgcgataggtatcgggccagtcgccctcgatcgccacggcgttgaatcccttttcggccagcaggcggcgcgtgatgtctgcgcgcgccgcatagaactcgtgcgtgccgtgcgaggcttcgccgagcagcacgtagtgcgcatcgccgatcaggtcgagcagggcgtcgtggtcgcccgaggagccgtccatcgggtgggccgcgaggcgcaatgcctcggtttccttcgaaatgcgtgatggctgcatcgttcgttgtcctcaagagagcgggctgtggcggcgcgcgttgtgaagcaggcggcacacttcctcgtcgctggtctgcgagaaatccaggtaccagcggcccactcccagaaaggggtccggcatctcggcgcagacgacctcgtcggcttcgctgcgcaggagctcgcaggcttcgggcgccgccacgggtgcggccaccacgacgcgggcgggcgcctgccggcgcaccgcgcgcacggcgacgcgcatggtcgaaccggtggcgagtccgtcgtccaccaggatcacggtgcggccgcgcagatcgggcgcgggccgcccgccgcggtacacgtgttcgcgccgttcgagctcgtacgcttcgttgcttgcgacttcctcgacgtccctggtggagatgccgagctcgcgcaccagcatgtcgtcgatgagccgctcgccgccgctggcaatggcgcccatggcaaattcaggattccacggcacgccgagcttgcgcaccaccagcacgtcgagcggggcgtggagcgccttggccacctcgtacgccaccggcatgccgccgcgcggcaaggcaagcaccgtcacgtctgggcggccggccaggctggccaaccgcctggccagcgcgcgacccgcgtacttgcgatcgcgaaaagattcgaaagccatttcgatgtccttgcgcccaccttatttttgcgggcgcacggacgttgtggggccgatgcgcagatcggcgtaggcatgcgctgccacggggagcagcacgccgcgcgcgccggatcgtcaggcgccggattgcctgggttccgacgacgcgtgccgcccggcccgccatgcgtcgacgatcagcgcgcgcgccttcgggtgctccgggtcggtcaccacccattcgggatacgcatgcggaaggctggcggcggtgacgcgtatcgcatcgaactcaaccggcgacagcggtgccgccgcgctggcgcggtgcgtcagcgtcttgcgcaggcccgccttccacgcatccggcaggtgttcgacggcgggcaggagcgcgagcgcaatgtgcgcggcgcgcgggctcagggctgcggcgtcggcgcgcaagcgcgccaggcgttcggtaccgctcatctttcacctccggagcgcatgtgcatttcaatcaggacgcctggatctcgatgcgccgcggctgggcgtgctgggccttgggaatgcgcagcttcagcacgccctgcttgagctccgccgagatggcgcccgtgtccagctccttgctcagcgtgaacacgcggcggaagcggcccaggcccacttcagtgtggctcgattcgagaccctcgggcaccgacaggtcggactccgcctcgatggtgagcgtgtccgaagccacgtgcaggccgagcttgtcgcgcgagacgcccggcaggtcggcatagagcgtgatgccgccgctgtcctcgatcacgtccaccgggggcgtgagcgctgcgtcgctgtagcgcgtggcgtcctccttgcgggcgagctgcgcccgttcggcaacgcgaggcgatgtgttggtggtcatggttgtctctcctttcaaatttgcctcggctcttttcgtttcactgaacggcaatgcggcgcggctgcgacgaagcgcggcgctgcaccgagatgtgcagcacgccgtcgcggcacttggccgtcaccgcctcggggtcggcgtcgtcgggcagggtcagcaccctgcggaactggccctcgaagcgctcgttgatgtggaccgccgccttctcgtcctcttgcgggagcgcgttttcgcgctttccggcgatggtgagaagaccgcgctccaggttgacttcgaggctcgacgggtcgacaccgggcgcgaacgcgtagatctccaccgattgcggcgtgccgccgatgttcaaggcgggaaagccgctctggccgaagccacggatggtgggtgacagatcgaaggcctgctgcatctcgcgttgcaggcgatccatttcggcgagcatgtcgcgcgggaacagggatcggtacatggcgaaaacctccattcaagacaaaagttgaacggagcgccggaggcgtctccagcgcttccgatgagcgaaataggcgctgccggcgctttttcaagaggtttttttggagcccgatgccacaggcgcgcatgccggacatggattgcagcaatttttacgtgcgcgcggccacgattcccgcccctctcgaggcgcgcaaggcgcatcctcttgaatacgcgcggaaatccatgccgccgggtggatgggtccgcgctgaattcgagctgcaatgcaagcgctcaagagatcaggagacgatcaggagacgatcaggagacgatcaggagacgatcaggagacagccatggacttcgaagggatttactgctttgacacggcgaccgtccgctttgcaatctaccccgatggccgcgatggcgcgcggatcatcgcgcagatttcagaggaaaccctgcacgatgtgttcggcaccagggatctgggcgaccgcctgctggatacatgcaagacgcacttcatggctctcagcgtcgccgcgctccggcgccaccgggccgacccgaaagcgcccatctgcctgacgatcgacgacttctcgccgcgcgccttgccaaagtccgccaacgatcatgacgccacgtcgggggcgccggttgccgcgtaagtagaaatgctgcgcctcgcgcgtgggtcttccagatccaggttgcgggatgggcaactctccgacaccgcaaggcggcttcagccgtaaccgccgggcccggattttttgcaaattgggcggtcaggtcttgtgaaagccgaaagcgtgccccgttgggcacccggttcgctggccttcatgcaagcaaggaacaccggtgccagtgaaccagccgccaagaacgccagaagcacaagacgcctacctgttccgggagggaacccattcccgcttgtacgacctgctcggctgtcacccggggaaggaagggggcgcgcatttcgcggtctgggcaccgaatgcggagtcggtggcggtggtgggtgactggaactactggtcgggcgaagccgacccgctttcgccgtcgccggacggcacgggcatctggcaaggccatgttccccaagcggcgctgggccaagcctacaaataccgcattcgatcccgcctgggcggctacgtggtcgacaaggccgaccccttcgcgttctgcagcgagctgccgcccgccacgggctcgcgcatctgcgaactttcctacgaatggcaggaccacgaatggatggccacgcgcggcgcgcgcaatgcgctggacgcgcccacgtcggtctacgaggtgcacctgggctcatggcgccgccgcgatggccagttcatgggctaccgcgagatcgctcacgaactcgcggcctacgtgaagcagatgggcttcacgcatgtcgaactcatgcccgtgaccgagcatccgttctacggttcctggggctaccagaccaccggctactttgcgcccaccgcgcgcttcggttcgccgcaggacttcatgtacctggtcgaccacctgcaccagaacgacatcggagtgctgctggactgggtgccttcgcactttccgaccgacgagcacggcctggcgtatttcgatggcacgcatctctacgagcacgccgatccgcgccagggctttcacccggagtggaactcgagcatcttcaactatggccgttcggaggtgcgcagcttcctcgtgtcgtcgggcctgttctggctcgaccggtaccacctggacggcctgcgcgtcgatgccgtggcgtcgatgctgtacctggactatgcccgcaaccacggcgaatggattcccaaccgccacggcggccgcgagaacctggaggcgatcgatttcctgcagacgctgaaccgcgccgtgtaccgcgagcatcccgacaccatcaccgtggccgaggagtcgaccgcgtggccgcgcgtctcgcggccgaccgacatggacggcctgggcttcggcgagaaatggaacatgggctggatgcacgacgtgctcgcctacatggaggaagagcccatccatcgcaagtaccaccaccacaagatgacgttctcgctggtctatgcgttccacgagaacttcgtgctgccgctctcgcacgacgaggtggtccacggcaagggctcgctgctgggcaagatgcccggcgacccctggcagcagttcgcgaacctgcgcgcgctgttcggtttcatgtgggcgcacccgggcaagaagctgctcttcatgggcggcgagttcgggcagcggcgcgagtggacgcacgacggcgaactcgaatggtgggtgtgcgacctggaagggcactcgggcctgcagcggctggtggcgcagctcaaccgcgtgtaccgcggcgcgcccgcgctctaccagcaggacttcaccgcctcgggcttcgagtggatcacggcggacgatgccgaacgcagcgtgttcgccttcgtgcgcaaggggcgcgacggccatccgccgctgctggtggtcagcaacatgacgccggtgccgcgcaccaactacctcttgggcgtgccgcagggcggcttctggcacgaactcatcaacaccgatgccgtggagtttggcggttcgggctggggcaacctgggcggcgtcgagtccgcgcccgtgcgttcgcatggccgcatgcagtcggtgtccatgaccctgccgcctctttccacgctgatcctggaacaccggccatcatgaaaaaactgttcgcaaattcagagacgcccacggcttcgagaatgcccgacgtgcgcgacggcaaccggcgcgcggtcatcgacgccatcctgccttcggtggacaacggccgctttccggtcaagtgcgtggtgggagagcaggtgcgtgtgaaggcgcattgcttcaccgacggccacgatgtgctgcgcgtgcagctgtgctggcgtccgcacgacaaggccgagttccgcgaggtgccgatgaagctgctcgtcaacgacgtgtgggagggcgccttctcgccgcccgcgctcgggcgctactactacaccgcggtggcgtgggtcgatcccttcgaatcgtggcgctccgagatggcacgccgcgtcgaggccgacgacgtgcgcattgcatcacaggtgggcgcattggaagtggccgcggccgccgagcgggcagagggcgccgaccggcaggcgctggcccgctgggccaccgagctcgatgccgtggcggcccacccgtcatcggaggtgtcgaccctcaaggcgctggcgctcgacgaagagctggccacgctggcgcgccgccatcccgaccggcggcacgaggtgcgcttttcggtcgagctgccgctggaggccgagcgcgagcgcgcgcgcttcagcacctggtacgagctgtttcctcgctcggcaggcaccacgcccggcgtacacggcaccttcaaggacgtggagacgcggctgcccgccatcgcggccatgggcttcgacgtgctctactttccgccgatccaccccgttggccgcgtgcagcgcaaggggcccaacaacgcactggccagcggacccgacgacgtggggagcccctgggccatcggcgcggccgaaggagggcacaaggcgatccttccggcacttggcacggcagaagattttcgccgtctctacgcgcaggccgcggcgcacgggctcgagatcgcgctggacatcgcgttccagtgcgcgcccgatcatccctacgtgaaggcgcatcccgactggttccgctggcggcccgacggcagcgttcagtacgccgagaacccgcccaagaagtaccaggacatctatcccttcaatttcgagagcgaagactggcgcggcctgtgggccgagctgcgcagcgtcatcgagcactggataggcgagggcgtgcgcatcttccgggtcgacaacccgcacaccaaggcctttccgttctgggaatgggccatcggcgaaatccggcgcgagcacccggaggcgatctttcttgccgaggccttcacgcggcccaaggtgatgcaccggctggccaagctgggcttctcgcagtcctacacctacttcacctggcgcaacaccaagcaggagctcatcgaatatttcaccgagctttccacctcgcccggcgtcgactatttcaggcccaacgtgtggccgaacacgcccgacatcctgcacgagcagctgcagggcggggagccctctgtgttcatgtcgcggctggtgcttgccgccacgctgtccgccaactacggcatctacggcccggcctacgagttgcgcgagcacctgccacgctcgcccggcagcgaggaatacctggactctgaaaaataccagttgcgccactggaaccacgacgacccggccagcctggcgccgttcatcgcccgcgtgaaccgcatccgccgcgagaacccggcactgcaatgggaccgcagcctgcgctttttgcccatcgacaacgagcagctgctggcctacgccaagacttcggagggcggcgacaacgtgatcgtcacggtggtcaacctcgacccctacaacgtgcagtcgggctgggtggagctcgatcccaagagcgtgggcgtggaccccctgcgtgcattccagatgcacgacctgctgagcgggcagcgcttcacctgggaaggcgggcggcactacatccggctcgacccacacagcgtgcccgcgcacatcttcgtcgtcaggcgccgccacggcgacgaacgcgacttcgactacttcctgtgaggccgcgcccatgaacgcccccgtatcccacattgcgcttgaaacggtcgagatcgacatcagcgacgatccgctgtggtaccgcgacgcggtcatctaccagctcaacgtcaaggcgttcttcgactcgaacaacgacggcatgggcgacttcaagggcgtgacggccaagctcgactacgtgaaggaactgggcgtcaacaccatctggctgatgccgttctatccctcgccgctgcgcgacgacggctacgacattgcggcctatgaagacgtgaacccgcagtacggcacgctcgacgactttcgcgagatgctcgacgccgcgcacgagcgcgggctgcgcgtgatcaccgagctggtcatcaaccacacctcgagcgaccacccctggttccaggctgcgcgccgcgcgccggcgggctcgcccgagcgcgacttctacgtgtggagcgacaccgaccagatctaccagggcacgcgcatcatcttcaccgacacggagacctcgaactgggcctgggacccggtggccaaggcctactactggcaccgcttcttcagccaccagccggacctgaacttcgacaacccggccgtgctggaggccatcttcaaggtgatgcgcttctggctcgacatgggcgtggacggcttccgcctggacgccattccctacctggtggagcgcgacggcaccagcaacgagaacctgcccgagacccacgcggtgatcaagaaggtgcgtgccgccatcgatgcgcagtacaagaaccgctttctgctggccgaagccaacatgtggccggaggacgtgcgcgaatacttcggcgatggcgacgagtgccacatggcgtaccactttccgctgatgccgcgcatgtacatggccattgcgcaggaagaccggcaccccatcgtcgagatcatgcagcagacgccggacattcccgagggctgccagtgggcgatttttctgcgcaaccacgacgagctcacgctcgagatggtgaccagcaaggagcgcgactacatgtacaccatgtatgccgccgacatgcgcgcgcgcatcaacctgggcatccgccggcgcctggcgccgctgatggaaaacgacatcgaccgcgtgaagctcatgaacggcatgctgctgtcgatgccgggctcgcccatcatctactacggcgacgagatcggcatgggcgacaacgtgttcgtgggcgaccgcaacggcgtgcgcacgcccatgcagtggagccccgaccgcaacgccggcttctcgcgcgccgacccgcagcgcctgtacctgcagcccatcatggacccgatgttcggctacgaggcgctcaacgtggaggcgcaggcgcgcgacagcagctcgctgctcaactggaccaagcgcatgctggcggttcgcaagaccagccatgccttcggccgcggcaagcgccgcttcctgaagccgggcaaccgcaagatcctggcctacctgagcgaatacggcgacgacatcatcctgacggtgttcaacctctcgcgcgccgcgcagccggtggagctcgacctctcggccttcaagggccgcgtgcccatcgagatgctgggccgcgcgccgtttccgcccatcggcgaactgccgtacctgctcacgctggcctcgtacggcttctactggttccggctcacgtccgacgccgagatgcccagctggcaccaggagggcgtggcgctccaggagtggcccacgctggtgctgttcgacggctggaccagcttcttccgcgaccgcgtgatgccgtggcgcatcggcatgtcggagcgcatgcgcaaccagttcgaactggagacgctgccgcgccacatcgagatccagcgctggtatgcatcgaagggcaccaccatcgaacgcgctcggctggccgaccacgtgatctgggaagcgggcccgctgagctggatgctgcccctgctcgaactcgacggtccgcccggcggcgccacctatttcatgccgctggcgctggcctgggaagagcgcgacgaagagcgcatggccggtgtcgcgcaggcggcgctcgccaaggtgcggcagcaggcgcaggtcggcctgatgggcgatgcgttctacgacgaggctttttgccgcgcgctgttgcaggcgatccgcagcggcatggaactggaaaccgcgaacgggcggatgcggttccgcgcgacggccgcctttgccgcgatcgaccccgacatcgcgagcctgccggtcgggcggccgagcggcgtgagcagcaacaccgtggtcacgctcgacgaaaccctgttcctcaagggctaccggcacctgcgcgaaggcctcaaccccgagctcgaaatgggccgcttcctgaccgaggtggcaaggtacccgcactgcgtgccggtgctgggcgcgctcgaatacaccggcaacgacggccgcaccatgacgctggcgatggtgcagtcgtatgtgtccaaccagggcgacggctgggaccacacgctgggctacctggagcgcttcctgcgcgactttgccaccaccagcggcgcgctgccggaccccatcgcggcccacggcggcttcctcgcgctcatggccacgctgggccggcgcaccgccgagctgcaccaggcgctggcaatacgcaccggcgcggcggcgttcgaccccgagccgctgctggccgacgacatcgcgcgctacacggcgcaggcccgcgccgatgccaccgccacgctggcgctgctgcgcgaaaggctgggccagctgcccgcggcggcgcaacccgatgccgaggccctgcttgccatggaagacgcgctgcaggcgtcggtcgatgcgcgcaagccgcaagcacagggcggcatcaagagccgctaccacggcgatttccatctgggccaggtgctgctgcgcgacaacgatttcgtcatcatcgatttcgagggcgagccggcccgcggcttcgacgaacgccgggccaagggctcgccgctgcgcgacgtggccggcatgctgcgctcgttcaactacgcgcgctggtcggccctcaggcgcgtggcgcaaagcgcggaagaggccgcctatctggcgccccccgccgccggctgggagcaggccgcgcgccaggccttcatggacggctacacggaagcgtttggcacggagggcggcgcggcgcgcatcgactccgaactgctcgcgctgttcgagctcgagaaggcgctgtacgagcttcgctacgagctcaacaaccgcgccgactgggcgcaggtgcccttgaacggcgtgctcgcgatcctgcaggccgagcggcccggttgatgcttgcatcgcatctgccgctttcgtccgccaccgcaaccgcactcgcaaccgcaatcacgcaccggagagaaacatggacagatttggcattcacctggagccgctgaacgcaatgctctaccaggttggagccttcgtgccccgcctggccattgcgctggtcgtggtgctggccggctggctcatcgccaagacggtgcgttttgcggtgaccaaggcgctgcgcgccatcaatttcaacgtgctgaccgagcgcgccgggctggacaacttcctgcgccagggcggatggcccggcgacaccagcagcctgttcggcgtgctggcctactggctggtcattcttgcggcgctgctgatagcgttcaacggcctgggcctgagctacattgccgacctgctcgggcgcgtggtgtggttcgtgccgaatctcttcgtggccttgctggtgctggccttcggctcgtacttcgcccgcttcgtgggcgaggcggtgtcgagctactttcgcggcgcccagctgcgcgatgccgtgctgctggggcaggtcgcgcgttatgcggtcatggccttcgtgatcctgattgcgctcgaccaggtcaaggtgggtggcgacatcgtgcgcgaaagcttcctggtggtgctggccggcgtggtgtttgcgttggcgctggccttcggcctggcgggcaaggactgggcggcggagcagatcgaacgctggtggccgcgtcagccgaaggacagcagcctgcccagggatcacagtccgccgaggagcagcccgcacgacgatcgcccgccgcgctgatattcatgacacgcagcccacgcaactcgatcacggccgtctggccggggcggccgtatccgcgcggcgccaactgggacggggaaggcgtgaatttcgcgcttttttcccagcacgcacacggcgtggagctgtgtcttttcgacgagaagggccgccatgagatccagcgcatcccgatccgggagcgcaccgacggcgtgtggcactgctacctgcccgaggcacgaccggggcaggcctacggctaccgcgtgcacggcccctacaagccggaggagggtcaccgcttcaatgcgcacaagctgctggtcgacccctacgccaaagaccttgtcggcgagctgcgctggggcgatgcgctctacggctacacggtgggcagcaagcgcgaagacctgtcgttcgaccgccgcgacagcgcgccgctggtgcccaagggccgcgtgctggagcccgccttcacctggggcgacgaccaccggccgtcggtgccctggcaggacatggtgatctacgagctgcacgtgcgcggcttcaccatgcgccaccccgaggttccgcccgagctgcgcggcacctacggcggcctgtgctgcgcgcctgtggtcgactacctgaagcgcctgggcgtgaccaccatcgagctgctgccggtgcacagcttcttgaacgaccggcacctggccgagaagggcctgcagaactactggggctacaactcgctggcctactttgcccccgagacacgctacagcgcctcgggcaaggtgaaggaattcaagaccatggtgaagaccctgcactcggcaggcatcgaggtgatcctcgacgtggtctacaaccacacctgcgaaggcaaccagctcgggcccacgctctcgatgcgcggcgtggacaacgcctcctactacatcgtcaacgccgagcgccgtcgctactacgacgacttcacgggctgcggcaacaccgtgaatctcgagcatccgcatgccctgcagctggtgatggattcgctgcgctactgggccgaggagatgcacgtcgacggtttccgcttcgacctggcctcggcactcgcacgcgaatcgggcaaggtcgagaacctgggcggtttcttcgacgccattcgtcaggacccgacgctcaaccgcgtcaagctcatcgccgagccctgggacctggggcacggcggctatcaggtaggcaactttccgcttggctgggccgagtggaacgaccgctaccgcgacggcatgcgcggtttctggaagggcgatgcgggcgtgatcggcgaggtcggcaagcggatctccggctcggaagacctgtacggctggtcgggcaagcggcccaacgcgagcatcaacttcatcaccgcgcacgacggcttcacgctcaacgacctggtctcctacaacgagaagcacaacgaggccaacggcgaagacaaccgcgacggaaacagccacaacatctcctggaactgcggcgccgaagggccgaccacggacccggagatagaaggcctgcgcgagcgccagaagcgcaacctgctggccacgctgctgctgtcgcaaggcgtgccgatgctgctggccggcgacgagcgcggccatacgcaaaacggcaacaacaacgcctattgccaggacaacgacatcagctggatcgactggacgccgaccccggagcgccaggcgctgatcaccttcgtggagcgcaccatcgcgctgcgccgtgcccacccctcgttccggcggcgcagcttctttgccggcaagccctccgaggccgagagcgtgaccgacgtggtctggctcaagcccgacggtgccgagatgcgccccgaagactggagcgacaccaacgcccggtgcattgcgatgtatatgtccggcggcggcattgccgaccgcgggccgcggggcgagtcgcagcacgacgacgattttctggtgctgttcaacgcgcaccacgacgagatttcattcacgctgccggccgcacgatatggtgcgtggcggttgctgctcgacaccgccagcggcacgccgccacctgccatcgaggacgtggccgcgctcgcacccgcctggtcggagcccgcctatccgctgcaatgccgctcgctcgtggtgctgagccggccggacgtgcggccatgagccgggttcatgagatgcccttcggtgtcgcggtgcacggcggcggggtcgactttgcgctctgggcgccctcggccgacagcatcgtgctgctgcacacgccggccggcgcggcgaccgcatcgcacgccatgcagcgcagtgccgatggctggcaccgcctcacgctcgccgatgcgcgccacggcgacagctatgcctaccgcctgcccgacggcaccaccatgcccgacccggcttcgcgcttcaatccgcaagacgtgcacaagccgagccaggtcgtcgatccgggccgcttcgaatggaccgacgcggcctggcgcggccgcccctggcatgaggccgtggtgtatgagctgcacgtgggcaccttcaccgaggaaggcactttcaaggccgcgcgcgagcggcttggcgaactggcggagcttggcatcaccgccgtcgagctcatgcccctcgcggattttccgggtgcgcgcaactggggctacgacggtgtgctgcagtttgcgcccgatgccagctatgggacgccggacgatctcaaggcgctggtcgccgccgcgcatgcgctggggctcatggtgctgctcgacgtggtctacaaccacttcgggccggagggcaactacctgcatgcgtgctgccctgagttcttcaacgcggcggagcgcacgccctggggctcggccatcaacttcgacggccccggttcgcgcacggtgcgcgacttcttcattcacaacgcgctctactgggtggaagaatttcacctcgacggcctgcgcatggatgccatccacgccattcgcgatacgtctcccaagcacatcgtgcaggagatccgcgaggcgctgaacgccgggccggcgcgcgataggcatgtgcacctggtgctggagaacgatgccaaccaggcctcgttgctcgcgcgcgatggcagcggcctgcccattgcgggcaccgcgcagtggaacgacgaccttcaccatgccgtgcacacgctggccaccggcgagcacgacggctactacgcggactatgccgacgacccgccggccggctttgcgcgcgcgctggccgagggcttcatctaccaggggcagccgtcggcatttcgcggcggagaaccgcggggcgaacccagcacgcagctgccgcctgcggccttcgtgtcttacctgcagacccacgaccaggtcggcaaccgcgccttcggcgagcgcattcatgcgctgggcgaccctgtgctggtgcgcgccgcgttcgcctgcctgctcttgtcgccgcacgtgcccatgttcttcatgggggacgagttcgcggcctcctcgccgtttctttatttttgcgatttcggtcccgagcttgcgtcggccgtggccgaggggcgccgcgcggagttcggtggctttgcggcctttgccgatgaggcggctcgcgcgcgcattcccgatcccaatgccaacgagacctttcttgcctcgaagctccggtggcgcgagcgcggcacgcagccgcacttcgcgcgcttgtgcgaggtgcagaaattgctcgacgtgcgccggcgccttttggtgccgcacttcgcgggcgctcgccgcgcgggaagccatcgctgcgaggagggcgtcattcgagtcgaatgggagctggcgggcaggcgccttcatctgatcgccaactttggcgcgcagcaagctctgcaagccgcggtgccgcccggcgcggtgatctacagcgcgggtgccgcagccgacggggagcgcctgcggctcgagcgcggcgcggtgcgtgcgacgctggaggagatggaggagatcgaggagatggagggcagcaccggtggctgatccgggtcattggtctcacgacgtgctggagcgcctgtgtcggcaccacggcatttcgccaacctacgtcgacgcgtttggaacgcagcgccacgccacgcccgagagcctggccgcgctgctggccgagttcggcgtggaggcgggtgctgttgaaacggatgcagccggctcgtcgcccgtgcccgccatgccgccggtgctggtggtggaggcgcacacgccgcactggtcgctgcagctgccgcatctctccggcaggctccactggcggttgagcgacgaggacgggcgctcgcgccagggcgacgccgacgcagagccgtggccgcatggcagctgcacgctgcagttggcggagccgctcgcgcctggctatcactggctgcacatcgacggactggtgggccgaaccctggtcgtcgcttcgcccggccgctgctaccggccgcccgcggtgcgcgatggcggccgcgtctgggggccggcggtgcagctgtacgcgctgcgttcgcagcgcaactggggcatgggcgattttggcgatctggaggcgttgatcgacgacatggccgggcagggcgccgatgtggtcgggctgaatccgctgcatgcgctgtttccgaccgacccgctgcgtgccagcccctacagcccgtcgtcgcggcagtggctcaacgtgctgtacatcgacgtcgaggcggccgacgattttgcgcactgcgaggccgcgcgccggcgtgtggagtcgcccgagttccagggccggctcgcggcgctgcgggctgcgccgctggtcgaccatgccggcgtggcagccgcaaagttcgaagtgctggagctgctgttcgagcactttcgctcgcgccatctgccgcaggccggtgcgcccgacgaaagaggcaaggccttcctcgccttcgtctcggcgcaaggcgagccgcttcgtcagcacgcgcttttcgaagcgctgcaggcccactttgccgcggccgatccacagtgctggggctggctcgcatggcccgaagcctaccgcgaggccgatgcgcccgaggtgcgggccttcgaggcgcagcacgcggatcgcctgcaatatcaccagtacctgcagtgggtggccgattgccagctggcgcgcgctggcgaacgctgcgcggcacttggcatgggcatcgggctctacctggacctggccgtctcggcggaccgcggcgggtcggacgcgtggactgcgcagcattgcttcgcggtcggcgccagcatcggcgcgccgcccgacgagttcaaccccgccgggcagaactggggactgccgccgctgcgcccggaccggcttcgctcccatcactacgagcccttcgtgcagatgctgcgcgccaacatgcggcatgcgggcgcgctgcgcatcgaccacgtgatggggttgatgcgcctgttctggattccgccggggcgcaccgcgcacgacggtgcctacgtgcgctactccgtggaagaaatgctggccatcgtggcggtcgagagccaccgccatcgctgcatggtggtgggcgaagacctgggcacggtggaagacgcgatgcgcgaagcgctcgcgcgcgccgatgtgctgtcctatcgcctgttgtacttcgagaagcagcacgacggcgggttcacgccgcccgagacctacccggcggccgcgctggtcgccatcagcacgcacgatctcgccacgctggcgggctggtggtcgggccatgaccttcggctgcgcctggcgctcgggctctttcccgacccgcggctgttcgacgcgcaactgctgggccgcgcccaggagcggatccgcttgctgctggccgtgcgcgaggcgggcctgctgtcgcaggacgaagccgcgcaggccctcgcgcatgccacgccttcgccgcggaccatgcaggccgcgcatgcctaccttgccgcggcgccgtcggcgctgatggtgttccagctcgaagacgtggccggcgaggtggagcaggccaacatgcccggcaccaccgacacgcatcccaactggcggcgcaagctggtgccgaccgtgcacgaacttgcggccggcgacaccatgcggggcctgaccgaacgcctgcgcgccgcacggccgcgccgcagcgcggctgcggaaccggcgccgctgcggcttcaggcgcgcgtgccgcgggccacctaccgacttcagtttcacaagggctttggcttcgacgacgccattcgcgtgctgccttacctggcgcaactcggcgtgagccacgtgtattgctcgccgatccagcgggcccgcgcgggcagcacgcacggctacgacgtggtggcccatgccgagatcaaccccgagctcggcggcgccgaaggctttgcgcgcttcgtcgaggcgctgcaagcgaacgggctggggcagctgctcgacatggtgcccaaccacatgggcgtgctcggcgccgacaacgcgtggtggatggacgtgctggagaacggcccggcctcgctgttcgcgcatcacttcgacatcgactggcagccgctcaacaaggagctggccggcaaggtgctgctgccggtgcttggcggccactacggtgaggtgctttccagcggagagctggtgctgcacttcgaaacggcagagggcagcttcgcgctgcgctacttcgaccaccggtttccgctggcgcccgaaacctatcccgtggtgctggcgcgcgcgctgccgcacctgaaggacccggcgctcaccgcgcaactggcgagcctctcgaccgccttcgggcacctgcccggccgccacgcacaaacgccttccgaatgcacggagcgcgtgcgcgacaaggaactgttcaaggcccgcctcgcgcacctggccgaggcgcatccgtcgctggcgcgcgccgtgctggctgcggtggccgagctcaaccttgcgtcgcaggaggcacgcgacgagctgcacaagctcatcgacgtgcaggcctaccggctcgcctactggcgcgtggcggccgacgaaatcaactaccggcgcttcttcgacatcaacgacctggcggcagtgcgcatggagcgcgaggaggtgttcgaggccacgcaatccttcgcgctcgacctggcggcggctggcgcggtggacggcttgcgcatcgaccatcccgatggcctgtacgaccccgcgcgctacttcaggcaactgcaggaagggtatgcgcgccgcgcgggcatcgtgctgccggtcaccatgggcccggacggccggccgccgcgcccgctgtacgtcgtcgccgagaagatcgccgcctcggaagaagaagtgccggtcgaatggcacgtgcacggcaccaccggctaccgctttgccaacgtggccaacggcgtgctggtcgacaccgccgcggccacagccttgcggaagacgtggcatgagttcacgggcgagacgcaggacttcgaatccgtggcccggtcgagcaagcgcgaggtcatgcgcaatgcgctgtcgtcggaactgaacgtgctctccaccgagctgctcaggattgcgagggccgaccgcagcacgcgcgactacacgctcaatgcgttgcgccgcgcgctcacgggcgtggcggcatgcatgcccgtgtaccgcacttacatcgtcgaggcgccgtccgcccaagacgcgcatttcatcgacgccgccaccgagtcggccgagcaccagagccgcgatgccgaccgctccgtcttcgcctttgtgcgacgcgcgttgcgcggcgaggcggccgagcatgcgacacccgcgctggccgaacgcgtgcggcgcttcgccatgcgctttcagcagttcagcgcgccggtcgcggccaagggtgtggaggacacctcgttctatcgctactttccactcagttcgctcaacgaagtgggcggcgagcccgaccatttcggcttcgacgttgccgagtttcacctgctcagcgccgaccgcgctttgcactggccgcacaccatgctcgcgacctcgacgcacgacaacaagcgttcggaagacgtgcgcaaccgcatcggcgtgctctccgaaatacccggcgagtggcgcgatgcgctggcgcgctggcacgcgctctgccatggcgggcacgaggctgctgcgccttcccgcgctgacgaatacctgctgtaccagaccctgctcggcaccttgcccttcggcggcctcgatgcggccgcagtgccggcgtatgccgcgcgcatctggcagtacatgcagaaggccgcgcgcgaagccaagctccatacgcgctggacccagcccgacccgaactacgaagccgcgctcgaagacctggtgaaaaggattctctcgggccgttcagcggatgcgtgtcttgcgaacatccagcgcatggccgatcgcctgtcgtggttcggcgcatggaacggcttgaccctcacgctgctgaagtacgcctcgcccggcgtgcccgatctctaccaaggcagcgagcttatcgacctgagcctggtcgaccccgacaaccggcggccggtggactatgaactgcgcagccggcggctggaccaacttcaagcgatggcaggcgagacctaccttcccgcgcgcgtgcaggcgctcgccgcggcgccgcacgacgggggcgcgaagctgtggttcatctggcggatgctgtcgatgcggcacgagaacgcggagctttttcgtgaaggcggatatgaaggactggcggtcgaagggccgctggcgcggcatgtggtggcctttgcgcggaggcacgaagggcggtcgctggtggtgatggcggggcggttgtttgccggcattgcgccgactggggcggatggtgtggtaccgatgcttcccgatgcgagcgcttggcgggggacgaaggttgtgctgcctgaggggttcggaagtgcggaattggagaacgtgcttagcggggagtcgctaacggtcaacggcaatgtcgtttcgctcgacgaggcgttttgtcgcatgccttgggctgcattcaaaagctgagttcctggttcatcggccggcttgacagtcgtgccgcgacaacagtgctcgcgaacttattgccattggctctttggcggctccagtgttgaaggcggcggctgcggattcgtctcaatgtcaatccgctggaggcgcgctttcttgtcgcaaggcaaatattgagtttgtggcgcagaggggcgcagtagagcgccagagattctcaacaggcgacgcagcctgtgcggcaattgttgccggccgtagaaccccttatcctcaggttttcacccaacccgaggagagagcatggcggtttctggttttttcaaggtccagttcagcgctctggcgcctggagctggtggcgtagtttcggttgaggatggcaaagtccgaggtggcgacaaccaatacctctactctggaacattcgcggccactgatgccggtgccacggcaacactgcgagtgaaggcgcacactccgaacgcaaaggatgtctttggtggcacaggcgcttcgttcaacctcagcctgacagggcagatcgacgacacgaaattctcgttcaccggtccgtcgcccaggccgggaagcccgcccatcacgattcaagggacgagggtcgctcaattagatctgctctaaaccgttccccgccacgcgaacccgcccagtctttggactcggcgggtttctttatttttgaggtgttccatgggcagactgatcgcttgagcttttcgcgttttgacaggcaagcccaatgagcaactgtccgaacaccggcattggaatttctttgtgactcgttcccgaatcaaggcgtgctggcgcacgttgtgcgcctggctgcgtgtagtgcaggccccagcagacggtgggcaaaccgttggccaccaggaagtccgtcgggaccggcgggcggaatggacaggcttagaaagcacgtctgtgtgaggctacccgaagagtggcggggcgccgcgccaggtcaaagactctagcgtcaaggcaatcaaacctgttgttatttgataggaatggttgcgcgttccagtccggtggaaatagattcccgcccagtagacctcttcccggctattgaggaaaagcctgggagagagtatttgtccctcgacaccatatttttgatggtgacttcgtctgctgggggcaagaactgaactgcgggcacatgcattttgttcataaaaggccctcgaagtgagacgttcgcgcgatagtattcgccgctggcgctgtcatctttcttccaagtaccttttgcgttgacaattccataattgccttcggcgagcttttttgccttggtgaatcgattgacggtaaccttggtgagggttactccggatacacaccaatagcgggttgttggtccaaatgacgcgggtgtattttgttggcaccattccagattcaccgcgtcatcagtgatcgaaacgatttcctcaacaataatttcatccatagtggatttgcttctgccggccttcaggaatccagctatggagccttccaactcaaactcaccttcgatcttgtttttaaaaacgaaggagctttttaggtctaccttttttgcagttgtgggcaatcccgttggtcgaccggcggtatcgagtacgctcccattctggtagacgtatgtgccaattaccgagtctattgaacttctccatacgctggtttctgagtcaggcaagaaggtgcggctgttgtagctttgaagcgcagcgtctgttgtgaagttcgtgttcgcttggctattagtgaccacgaaaagagccagacccaggataaaggctatgcgtgtctgatggtggatggttttcatgtgtttgcgccagtggtgaagggtgcatacaacctatcactgtttgtacgttttgtaatcacctgaagcggtgggcaacttgcgccgacgctttgacgttgtttgggctcgggtagtccatgagcttcccaccctcaagcccaggctcggcatgaccgctaggtacgacaacaccgacagccgcatgcgtggccggaagccgcaggagcgtcgcctgagggtgtggagcaaagatcttcgatgcgcgatgtgccgcacgttgaccgacttccccgcaggcttccagcttgatcacaaggtgcctctctttaagggaggcaaggagagagtcgctgaagctggcctccgacctgagcggcgtgtcgctcgacaaggtggccaccgcgtcggtcaagctcacatcggaacttcgaagacccctcggcgattggtcaaagcagtagctcgagcgctgatcgaagaggcgcggacggccggacagtcgtgccgcgacaacagcacccgcgaactttcatattcatttcgaccgagaagtgcgaacgacttttgaactgtcgttggttggctgcagcctttcggctaatctgaaacaacttgtacggaatgcgctgcgtggcagcgcatgtcacctgaggggtgatcgaccggacgccaaaacattgaccatcacgtacgcataaagagtccaccgtcaatgttctgacatgtaggcaaaaaaatgagggagcgggcgatgagggtttcaaatgcggtactgggcggcattgctcatgttcttcgcgtgatcgctgcgtggatgctgtgtgtggtttctgcgtcctcttgggcgttgatcccggcgtctgatgtctggttctataacggcggggcctatggcagtcctgattcagtcgggaacaattttgcgtcggctagcgctgcctgtgatgcctatgtgactgcgcaacaagctcggctccccagttgggtgtttggcacggggtccataggtgccgccgcgctacctccgaattactatggtgatttcaaatgcactgtctacgcagacacacaatacgtgagccatgtaggcccgatggaggtagggctttataaggtcggtggtggcgcatgccctgcaaatagcaccgctgtaactggtggctgcaagtgcaaaaatggcactcaagaggacggctctcaaacgtcctgccttccggctgctcctcagccagccatgtgcatggctggcggattggaaggcaaccccattttgccgtccacggccgagaagtaccgcttcgaaaccgactggtccgactccagctccggggccttgtccttcacgcgcacctaccgcagcaactgggccagtgattcgagccggaccagcaatccactcggtcaagtctggtcgcataacttcagcaccaagctggttgctacgcccagcactgctcccttgggcgtcgccatcaccaccggcgaagggtatgtgcgcaccttcggcaaagcatcaggtgccactacctggatcgccagcaacagcgccgacaccctgacgcaactctcctcgggcacctggagctaccaccgcgccgacgacgacaccacgctcagcttcgacggttccggcaagctgcagaccgtagcggatcgcaacggctgggtcactgtctacacctacaacggtgccggccaactggcctctgtcacaaacggattcgggcgcaccctcgcgcttgcgtacaacagcgcgggccagttgaccaccgtcacgaccccggatgcgcgcgtcatcgcctacgcctacgacagcaccggtcgcctggtctcggtcgtgtaccccgacggcaagggccgcaatttcgtctacgagaacgcttcattcccccaagcgctgaccggcatctttgatgaagccggtgtccgctggggcacgttcgcgtatgacagcacgggccgtgcgatcagtacccagctcgcaggctcggttgacagttatcaagtcagctatccgtcctcaagttccgccacagtggtcgatccgctcggcacgagccgcaactacagctatggcaccacgctgggcaagctcgccgtcactggaggctcgctgccctcgggcgaaggcaagagcgatgccgccagccgcgtgcaggacatcaacggcctcataacctcccagaccgacttcaagggggtagtcacgaccaccacctgggacgtcacgcgccgcctgccgaccaccgtggtctacgcctccggcacccccgacgcgcagaccgtcacaacccaatggcatgcgaccttcgttttgccggtgttggtcaccgagtccggccgtaccaccgcctacacctacgacgctttgggcaacatgctcacgcgaacggtcaccgacaccgccaccagcaaagcccagctctggcagtggacctacaacgcccagcaactggtggccacggcgacggagcccaacggcgccgtcaccagctacacctacgaccctcggggcaacgtcctcacatcgaccaacgccctgggccacgtcaccagctacacctacgacagcgccaaccgcgtcgtgagttcgacggcccccaatggcctggccaccacctacacctacgatgcccgcgaccgcctgttgacccagaccaccggcggccagaccacggtcctgacctacaagccctacggcagcgtcgaatcgatcacgctgcccaccggcctggcgctcacctacacctacgacgccgcccaccgcctcaccggctggagcaacaaccgtggcgagtctgggctctacaccctggacggcatgggcaaccgcaccaccgagcagatcaaggacagcgccggcaatgtcgcgtggaacgccgcgcgcaccatcaacaccatcaaccggctgtccgcgaagaccgaaggccccaaccaggcgagttccttcggctacgacgccaacggcgaactcacacgcaccaccaacgccctgaaccagagcacccagtacggcctggacggcctgcgccgcgtcaaggctgtgaccgatgtgatcaatagtgcgaccgcatcggtgaagtacaacgccctggacgccgtcaccgaagccaaggacttcaagggcgtggccaccacctacgcacgcgatgcccagggcaatgccaccgcagaggccagcgccgacatcggcagtaccagtacccagtacgacaacctcggcctgcccagccagaccaccgattctttgggtcaggcgaccaccatcacccgcgatgcactgggccgtcccaccggcctcgtcttcgccgacggcaagaccaccaccctgcgctacgacctcacggccaacagcaagggctacctctcggagatcgtcgaccgcagcggcaccaccgagtacacccgcgacaccttcggccgggtcaccctgaagaagcagactctcgcgaacggcagcgtgcagcaggtcagttacagctaccaccctaacggcaccctggcgagcatcggctacccgaacggcggtgggctgctcgcgcacagctacgacagcaccggccgcctcacgggcctgagcctgaacggcaatccgctggtcaccggcattgcctggaacccgctgggccagcccaccgcctggagctgggcctttgcttcccccggcctcgcggccagccgcagctacgacaccgcgggccgcatgaccgccaccgagttcagcagctacgtctacgatgctgcagggcgaatcagtagcctgacccaaaacctttatcggcctggtgatggtgacccgacgcacagcaccattgcgaacagcaacatcagttggagcacgttcttcagtgcgaccggtcgcttacgccaattcgatacctccggcgatacagcggcgttcacctacgacttcaatggcaaccgcgctaccagcattcgggtgctcaacggccagaccaccagccgcacctacaccgtgggcgccaccagcaaccagctcaccggcttcacccagaacatcaacggcgccagcagcaccagcgtcacctacggctacaacgccaacggcgacctcgtgagcgacggcctgcgcagctacacctacgacgccgagggccgcctggccgcggccaccaccggcgccaccgacgtgagcccgaccacgcgctacgcgcacaacgcgctgggccagcgggtgttcaagaccgagccgctgtacccgcccagccagggcgacgaggccgacccgggcttcatgcagagcctgatcgcgttcttcacgaagctgtggagcccgagcacaacccaggccgagcagctgggctatgcctatgtctacgacgagcagggcacgctgatctcggaggctggcagcggaggcgccaacagcgcggggcaggccagctacatctacctgccgacggcgaacgggccgatgccgattgcggccgtgatcaatggcgccacctatgcggtgcacagcgaccacctgaacacgccgcgcaagctcagcaatgccgacggacaacccgtctggcagtggagctacagcgcgttcggggaggacaagccgacgattgcgaagaatcggttcgccaacctcgagatcacgccgaaccccggcaccaccagcctgtcggaggtgaagttcaaccttcggtatccggggcagtatgcggatgaggagagtgggctgttctacaactacttccgcagctacgacgcgaggaccgggcggtacagccagccggatccgatcgggcttaaaggaggatggaaccggtttggatatgtgaacgaaaacccgctgggtgatactgatccactagggctatgcggtaaagatacaagctcatgcatgagcgggcctaacaacccatggaagacaaatcctagataccacgaatatgaaactgacatggtcgtgtgcaggctctcggcaacctgcacaagagactcggtgttcaaggctgtgaaagagtttccgacgcctgccggtcctgttcctggcggagtgaacagttgcggcatctctgacatcggaggcaataaggtcgagcacttcgtggacgaggaaaactatggcgtgttcaacatcgcaatgccggggcatatgtttgaacctgggtacgtccttcggaatgtgttcgtcgatgcgaatggcaacgtcatcttgcgcacgtacggagaaggaacgggggggtggcgaggttttaataattggtttggaaaacatggttggcctttggtcgatcagcgaattccgaaggccgtaaggcgataaggagcagatatacatgggtggcgaaaacctattcatcatcgcggcactgctaggtggagcaatgcttctgtacttggcgtaccgaagtctgcgaacttccacgcgcgcatatgcactgccaacactggtgttctcaatcggggtcgggatttggtcggcgcacgacatgccattgcacagttatcacatctatttttttgtgggcttcttgttgggggcggtggtattcaatttgcatgcgagagcgatcaaggcgcttctcaatcacaaggaaaaggaccatttgaccggttgaaccggaatgctatggcgccaaacggcaatcgtctcagcagcaatgagagaaatcggcggccagatgcccaggatggatcagtagccggggcgaaacgaaagtacatccgttgacccaagggttgatggatgccgtgattggcatctttaagaaatgaggaattggatgaagatggccatcgttgaacctttgtggcttcgtcttcacgcggcgctgttagcgttctcggagaaacttgagaagatcgactcgtcgttgatctgcgatcttgggcgtatccagaacgatgcgtttctacttagagcttacttggccttccgacgaggtgccggtaacgaagaagtcgctatcacagtggatgtccagagcgatggcaagcagatgaagattgagtcagatgcctgcaaagacgacggtacggtcttggcggtcgggccctttgccgagattcaactgtctgaggacgatctgggtgttcagcatgcccttgacggttgggtgcgtgagtttgagcagttcctgtcggatagcgagacagagatcgtcgcggccgcttctcgtttggacaattgaattcccggataggcatgtcgcaagtgcaaccctaaaaagggggcgatggtggagtgcacgatcaggctgcttcagcgtatagagaagacggccgcagtcctcccaaccctgcggcccgcttcctcctacagcccgtaatacttgtcgatggtcccgctgtacctgtcgtcgtagtcaggcacacggtcgctcgcatagcgcggcgcgccgtcgatctgctccttggtcaacggcactacgtagccgtcctgcgaagtgtcgtacttcagcatggaccaggggaggggatagcggtcggtgccaatgccgaggaagccgccgaactccaagacggcgtagcggacctggcccgagatcttgtcgatcatgagatcgtcgatgctgccgagcttgtctcccgccgcgttgtagacggatgttccctcgacacgttctgaagaaataactggattggcgcttgccatggaagtaagtctccggccgccatctctggggaatgacggcgttggttgcaatgcccagacatgccactttgggtccggaaaattcccgccgcatcggccaaaagatcgtcgtgttgtaggaggctgtctggcaccgggggcagaactcggaccgggctttttcggcccgctgttgctgctgctgcgtgtgtgccttgccgacaggttggcgtcaaagcaagacgagcaacaccaggcatgcagtggtcaagcccacttccaacatttccttgcccgacatgctgcgcagccgccgtgcggtcagggtcaccagcggcagcagaagggcgaggccgatccagcggtccagcggtacgaggcaggtgcgtgcgagtgcccacagccaggcgcagtgggcgagaaagacccagaactctgcgcggctggtcgtggaggtcaggtccagcgcattgcgccagcctttggccacggcgtcccaccagtcgatctgctctatgtccagcagcttttgcagaccgtgcagcgccagcacgcacagcagaatgggcccgaagtagacaccccacaaggcgatgccggtgtacagcggatggccgtagccggtgccaccaccgcccaggctcgcggtggccagcaccgtaaggcccgtgccggccagcagcgtgcccgccgccacggcgaacttcggcatgcccacgcgcagcaggccgcgcccgccggcaaacaaggcaagcgcgagcacggtggcggccaggaagtacttcagcgccgcagcagacgacttccagccctggtggggccgcgcggcccaacggctcgacacgggcggctccagcgggagggcgccgggcgcccattgccgcgcaggctcttggcgtgccgtcaacagccgccggccccagtcttcggcttgcggcgcgagttccgtcagcgccagttccaggtgatacaggcgccgtgcgttgtccagatcgtgcggcaccagaaacggctttgttgcggtggcgccggccgccatgagcgctggcaattgctcgcgccaatacgcgggggcgggctgcgcctcgcacgccaatggcccggatgcctcgccgggctgcaccatggtcaccgcattggcctgcatgacgctcaggttgtgttccggtcgatcccacgcgcaggcaaaggccaggccgccgagcccggtgccgggcgcaccgcccagaatgatgtcgggccgaaaaacgggaagcggctgcgtggaggtgttggccaggcgcagcgccagcatcaggcgaaccctgccgtcggcggccggcgcagcccacaggccgggcgcgatgggctgcatgtcgcgcctctcaatcgcgaagaagggcgtgcgcgcggccccggtctcccaccgtggggccagcccctggttgagcgcgccttgccaggcggcgcgaaagggtgcgtcgagcacgtcgcttcgcgtgtggccacgggcaatcgcggcggccacggtgtctttcggggcgggtgccatgccgggcagttggcgcttcaatgactcccagacgccgggccggggcgcgggtgcagcggccgggccagtgatctgggccacatacgcatgcaggaggtcgcggcgcaagtcctccacctcggcagcgggcgcgtcggcgctgcgcaacatgcgaatgagaaagaaggcctgggctgcattgccgcccactgtcgtttcgcgcagggcggcggtgaattcggtgggccccgacgcaaaggccaatgccggcaggcagagcaagacacagaggatgcggcgcaggtagtgcgtcatgggcaatgcaggggccgatggcggagttcagggcggggggatcatagtgttgaatcaggtacgtggctcctgtgtcgtcgctccgcgttcaagaaggaacgcccggttgcttgcctttctttccttgcgccttgatggctccagacgcagccgcccgcaggatgcggcggaacgtcgggcattccatgtggctgggagcagggcaggcggccgcatgccgcaggccgtcgcgcatggcgcccagtttgcggatcgtccggtccagttcgtccgccttggacgcgagcatctgccggtcgatgcgcggcttgccttccggcgcgaacatgagtgcaatctcatcgagcgagaagcccgcggcgcgcccgacggcgatcagcgccagccgttccagcacgccagaatcgaacaggcggcgcaggccgcgccggccggtggaggcgatgagccccttctcctcatagaaccgcaacgtcgatgcgggaacgccggatcgctgcgccacttgggcaatgtccagatgtgtcgttgttgttgttgtcacctcttgacctcaagtcgacttgaagttgcacagtctagcttccgcctctcgaggccagccaaaggagaaacgatcatggacatcacgcaacagcaacagcaacagcaacagcaaaaggaaaccgaacagaccgcgctctggaatggccgcgccggtcatgcctgggtcgacgcgcaagagttgctcgacgcgatactgcagccgttcgaagaccggctcgtcgacgcggtgcgcgccgggtcggcgcagcgggtgctcgacgtgggttgcggcacgggcgcgaccacgctggcggttgcgcggctgctggccggcgcgcaaggcagctgcatcggcgtcgacatctcgcagccgatgatcgccgccgcccgggcacgcgcgcagcaagagggcgtgccggcaagcttcatctgcgccgatgcgcagcgccacgccttcgagcctgcgagcttcgacatgatcatttcgcgcttcggcgtcatgtttttcgacagcccggtgcaggcctttgcaaacctgcggcacgccgcgcggggcggcgcggcgcttcgggccctcgcctggcgcagccccgcggaaaatccgttcatgacgacggccgagcgggccgccgcaccgctgctgcccaacatgccggcccgccagccggatgcgccgggacagttcgccttcgccgacccgcatcgggtgcgttccattctggaggagagcggctggagcggcatcgacatccagcccgtggatgtagcctgcacgatgcccgagaaggatctgcgcggctatttcacccggctcggcccgctgggcctgatgcttcaggagcaggcggcggacgagcgcacgcgcgcgcaggtcatcgacacggtgcgcgccgcgttcgacccgtacatgcacggcagcgaggttcgctttacggcggcctgctggatgatcggcgcccaggcagcttccgcgtagcggcgcctaacccagcagccgcggcaccagttgcaccgtgagcgccgccaagatcccttgcgcggtcacgcagtgccacatcggcccggtgttgtcgattgttgcgcgtgctgcgggctgcagccggccggaccacgagcgcaccagcacgtagccgcccatcagcagcagcacggcgatgtggaacgcctggtagcccagcagcatgccgaccgatgcgctccagccttgcgcgcgcggctcgagcccggccagcagatggccgccgatgtcgagcgcggccgaggcggctgcagaggccatggccagcgccatgaagaggcgcaacaagcgctgcccgcgcgcatcggccgtgcgcagtgcgcgcgtggccagtgccatggcggcggagccggccgcgagcagcagcgccgcgcccagcggccagcgcgcagccggcagcgcggcaccgggtggcgggcacacgtcgctcgccatggcgaggtgcacgtgggtgtacagcagcgacacgaagatcgtcatgtccaccgcaatcaacacgatcatggcccaccacgaatgcgatgcccggccctgcgcgccgaccggcaggcgcaggccatggcccacgtcgaccacggcggtcggtggcggacggtcggaatcccagagccagcgcatgatgcacgccaccgcgatcaccccgcatgcaaaggccggcagggtttgagacaccgtgagaagaagaaagaacccggccgtgctcgccgccgcagccaacggccaccaactgtccgtcggcaggcgcagcaggtgcatcgggcgggcatcgcgccagctggtcaccagcgtttcgcggccgccgaagacggtgcccggcagcaagtgccggccggcatcgacctcttgcggcagcgtggggcgcttccacagcgggtagcgcgaatccacctgcgggatgctgcgcgcgccgtattcgcgcgacggcagccattcgagcgtgcccgcgcgccacgggtcgccgtggtcgcgcgagggccggcgcagcgtgcgaaacgcatcgaccatgaagagcagcacgccggccgccagcgtgtaggcgccgacggtcgacagcatgttgagcgtgttccagcccaggtcgccgccataggtgtacacgcgcctcggcatgccgagcatgccggcaaggtgcatgggaaagaacgcaaggttgaagccgccgaacatgagcccgaacacccagcggccccagcgctccgaaaggcagtggccgttgtagagcggcgcccagtagtagaaccccgcgaacaccggaaacaccatgccgccgatcagcacgtagtgcaggtgcgcaaccacgaagtagctgtcgtgcgcctgccagtcgaagggcagcaccgccaccatcacgcccgtgaggccgcccagcacgaagatgaaatgaaagccgagcaggaacagcgttggcgcattgagcatcacgcggccgcgccagaaggtcgcgatccacgcgaacacctgcacgccgctcggtagggcgacgatgaagctcgcggcggacaccaccaacaaagacaggttgccgaggccggcggtgaacatgtggtgcgcccacagcgcaaagctcaccgcgcccacgccgacgagcgccagcaccaccgcgcggtggcccaccagcggcgtgcccgcgagtgtggccaccatcatcgagaccatgcccgccgcgggcaggaagatgatgtagacctccgggtggccgaagaaccagaacaggtgctgccacagcagcggatcgccgccgcgtgcgggaatgaaaaatggccagtcgaatgcgcgctccagctccagcagcatggtggcggcaatcacggccgggaacgcgatggcgatcatcagcgcggtgaccagcatggcccaggcgaagatgggcatgcgcgcgagcgtcatgccgggcgcgcgcgtgaagagaatgcccacgatcagctcgatggcgccggcaatggccgagatctcgatgaacccgatgcccagcagccaccagtcggcaccgcgtccgggcgaaaactccttgccggtgagcggcgggtacatgaaccagccgccgtcgggcgattggccgaagaagatggtgcagaaaaaagcgaatccgccgatggcataggcccagaacgcgtaggccgaaagcagcggaaacggcaggtcgcgtgcgccgatcatgcccggcagcaaatagatggccaccgcttcgacaatgggaaccgcaaacaagaacatcatcacggtgccgtgcatcgtgaagagctggttgtaggtgcgggcgtcgatcaggccgttgtcgggcacggcgagttgcgtgcgcatcatcagcgccaggatgccggccagcacgaagaagagcatcgccgtcacgatgtagaaaacgccaatgcgcgtgttgttcaccgccgagagctgccgccacccgctgggcgggcgccatgcacgctcgagcgcctcgcgttctccggcggggcgcggctgcgggttcgaagtgtggtcgagggcttgcgtcatctacttcagctgcgtgagccaggcggcgatcgattgcaggtctgcgtccgcgatgcgttcgcccgacgacggcatgcgcgcgccgggcttcagctgctgcgtgtgggccacccatgccgcgagttgcgccggctcgttgggcacggtgccggcgcccaggtgcagccggctgcccacgtgggtgaggtcgggcccgaggcggctttcttcgctcacgccgcgcacggtgtggcaggcgttgcagcggtgcgccagaaaggcttggcggccgcgctcgatctcgggcgatgccaccgatgcaacggcgggcctcgcctgtgctgctagccaggcatcgaatgcggccggcgcttcggccaccacgtgcagcgccatgcgcgcatgctgctcgccgcaatactcggcgcactgtccacgccatgtgccgggccggtcggcctgcagttgcaggtgctgcacgtggccgggcagcatgtccatcttgccgccgagcgacggcacccagaaactgtggatcacatccgcgctgccaaggccgaagtacacgggccggccgaccgggatgcggatctcattggccgtgaccacctcggccccggtggccgggtcgcgatagcgaatctcccaccaccacatgtggcccgtgatcccgacgatcagcgcgttcggcggcggaacgggcttccacggcggccggtgccattcgctgtaggcgaagagcgccgcaagcaccacggccggaaacacgaggccgccgccgatgatccaccagcgggtgtcgaccgtaccgccgctgcggcggcgaaccgcaagggcgagcagccccatcaccgcggcaaagatcagcgtcccgcccacggccagcacgccgcttacttccagcagcgcttccgcgacggggcccgcggcccgcagggcggattggggcagccccgcggcagtcatcgccgtcattcgagcgcaagcaggtaggccgccatgtcgcgcgcatcctccggcgacacgcccatggccggcatgatggtgccgggcaccagcgtggcgggcgccacgatccagcgcaccagatgctcgggcccgttgggcacttgcccggcaatgtagctgcggcgcccgaaggccgcgagcgtggggcccgtgcgtccgcgcgcggcctgcacgtcaggaatggtgtggcagcttccgcactggtactgggccagcagcagccgcccgcgttcgcgctgggaggagggggcgcgaagctgttgctcctcgggcgtgcacccggccgcaagcactgccagcaccagcacggcgagcgggcagacagcgcggtacgacggggcggccaccatgccgcgattctccggactggaacgcggcttgcgccgacacggcggcgccggtgcgcgtcggacaatgccgccaattgattgctgccgatgggtgcgccgaagaccgttcttctcaccgttgccgtgctgggcctaggaggcgcggcggtggctgcgctggtggtgtacggcggcttgtacaacgtggccgcgacggtgcagcacacgcagccggtccattcgctgctcgaaacggccatgcaccaatcggtgaagctgcgcgcccgcaacatcaaaacgccgcggctcgacgacgagcagctcgtgatgcgcggcgcggcctgctttcgcgacaagtgcgtgcaatgccatggcgcaccgggcgttgcgcagggcgacatcggcaagagcatgcagcccctgccaggcccgctggtggatgcgcggctccactggaaaccgcgcgagctctactggatcacccggcacggcatcaagatgagcggcatgccggcgtgggagttcaggatgtccgacgaagagctctggtcggtggtggcgttcctggcgcgcctgcccgatctcacgccgcagcagtatgcgcaagccacgcacgtggaagcgacgggcgcagagggcgcgccgaccccatcggcatgcggggccgtggccggcccggcgccggtccatgcgggcgatgtgcggcgtggcgcgcgggcgctctttcaatacgcctgcaacgcctgccacacgattccgggcatcacgagttcgtctcccaacgtggggccgccactcgccggtatcggcggccgttcgctcatcgcgggaaaactcgccaacacgccggacaacatggtccgctggctgcgccagacgcatggggtcgaccccctcacggccatgccggaaatgggcgtgacggagcaggacgcgcgcgacattgccgcgtacctggcaacgctgcggtgatgctggctagggcctgttcacactactaacggagatcgcgttgttcggcaaaggggctggctgcaaggcgcccgtgcgcagcaaggcttgtgccttgcaagcgcgggcaacgccgcagacggcccctttgccgaacaacccgaagggaaggcatgccaaagcggccaactccgcgttgcactccttgcgtgtgccgacgcacacgcatcgtcgtgcgccttgatttgtccgctttggcatgccttcgcgactccgttagtagtgtgaacaggccctagtacttggcggtgatgcgctcgtcgtcgaccgtggcaatccgcagccgggcccgctcgtgcttgatgacgagctcggcgcatcgccgctgcacggatgcgtccgccgaaggccgatcgctgcagtccacgagaagctgcgactcttcaaagtccaggccgtgaagaacctcctggccgtgcgaattgagggccaggaggttttccgccgacaactgggcgcgcagggcttccgaaatggcaagcgtctgcaatggcttcaccgtttcgtctttggagcgctggttctttccgccattcattatttcttcattgccttgatgtcggccttgccctttgcctcttcggccttggcttccttcacgcaggcgttcttggcatcacccttcaggtcgtcgcacttttccttggcgaccttgtaggtggcctccaccttggcttcggcgaccttgcgtgtgttgccgtcgctgggcttctgcttctggtcgagttcagccttggcaatcttttccttgcccttggcttcttcgatgcagacgtccttggcgttgtccttcattgcatcgcaggcagccttggcggccttgtagtcggcctcgatcttgtcgcgggcagccttgaattcggcaattgccggatcggccggaggcgcggggttcacttgcgcatgcacctgaacgacggtcaggcaggaagctgcggcacacatcaataacagtctcttcatggtgtgatctcctggacgcgcgggggtttttattgcaacggaggctccggcgtcgaaatcaatatagaagccggcggccctgcgccggtaggacgcttcgcggagcggccgtaagcacatgccgacgcttgggcatggcgtcgtctggcgggcaggtcgtcggcacccgccgccgcaggcgatgcgccccgtcctaccgggcgggctggtgcggggcgcacactgcctgaacgcgaatccacaggagatcgccatgcaaaagcttcacgcgttgttcgttgccatctgggtcatgtgcgcggccgtggttcaagtggctgcgcagaccccgccgccgcatccggccgagatcgaccccaccctcgtcgaatacagcgccgcccgggaacggatcggcgccacttccaaggtggctttgggccagtgcgaggcattggccgggccgggccgcatcgtctgcatcaaggaagcccagggccgtgaaaaaatcgccctggctgaactcgatcagcagcgcaatccgagcgacgccaatgcccgccggctcgcggaaatgagagtggcggtgaactacgagattgccgtcgagaagtgcaacgaccgccagggcagggacaaggccgaatgcctttcacgcgccagcgccgaagaatcgaaggcccgcgccggtatcaaggcatcgggaagctagtcgttgcgaatgacgctgacctttccgtcgccctcaagccgcgcgatcttgatcacgctcaggtcgtcgatgccttcttcgcgcagctttgccagcacctcttcgacggtgatgcgctccttgcgcagcgtgcgcgccacgaacttgccgtgcctcaccagcggttcggccggcggctccagaaaggccgcgacctttgcaaagcggtaggcaagcacgtccagcaggtagttccatccgatcagcgtgcccaatagggcgatgccgttggtgacggacctgtattcgccctgcatggcattgctcgacgcatcggccaccagcacgatgaacagcaggtcggccatgctcatcgagcccacgtcgcgccgcagcacgaaccggaagacgatcagcaggaaccagtagatgacgctgccgcggaccaccatctcgagcagcggctggtcgggggagaacagatcggacaggttcatatacgcccttcggcggcggcgagggcggccacctgcactcgaaatgttccgcgcatgcgagggtgccgggtgtcgtgcaatcggcttcaggggccgtcggcgcaatcccacatcgggccggcgggccgcatggcatttgcgtgcccgccagactgctccgacgtacaggtcctgcatcttccgaccctcgtcgcgagtgggcggcgcacgatgcaatcccatcacacttcaggagagcaaacatgccaagaggtgacaagtcgtcctatacggacaagcagaaacgcaaggccgagcacatcgaggaaggctacgagcaccgcggcgtgggcaaggccgaagccgagaagcgcgcatgggccacggtcaatgccgaaaccggcggtggcaagaagagcggcagcgggcgcggcaaggccgagaaccacgcgccttcgcgcaagggcgggcacaagggcggcgctgcggcggcatcgcgcaccgccgccgagcgctcggcctctgccaagaaagcggccgccacccgcaagcgcaacgccgagcatcgcagcggctgagccgatgaacccaggagattccccatgactcgcgtatctgaactgatgacccgtggcgttcgaaccctgtcgccctcggactcggtggcactggccgcccaggccatggacgagctggacatcggcgccgttcccgtgtgcgacggccagcggctgatgggcatggtgaccgaccgcgacatcgttcttcgcgtggtggcgcaaaagcttccgccggagaccgcgttgtccgacgtgatgtcgaaggacgtcaagtggtgcagagacagcgacaacgtcgaaacggtgatggacgagatggccggctaccaggttcgccggatgccggtggtcgatggcgaccgcaggctggtgggcattctctcgctcggcgacgtggcggcgaagggcgacgccggcaaagcgggcgatacgctcaacatcatttctcagccggccgaaccggaccgctcgaagcaatccgcggcaagcgggcctgcgggtggaggctcgtcctgagcgaggcctttgccggttttttcagcgcttcgcgggcagccggatgcgcgagccgggcgtggtggagacccgcagcgcttcctccgcctggcgcagaaagcgctggttgcgcgcgggcgtctgcgaggccacgcagtcgcgcggaaccacggcttgcagatcgcgcatgcccgcatcggccacggtggccaggatgcactggtcgctcgccacgccggtcacgatcagccggttggccttcaggtaggcgagcagcaattcgagcggcgtggcaaagaaggccgactgcttgggtttgaggacgaaatagtccgtctcctcgggcaggagcgccgaagtgatctcggcgccggcacctcccgcggccagcgacagttccaccagccttggaaagtccgagcgccagcgcccccggttgtcgttaacgtaaatggtgggcacgccggcgcgcgtgcagcgtgccttcagcgccgcaatccgcccggcgatggcgtgcgcaccgggcaggagcttctcggcgtcgggaaaatcccagcagccgatcatgtcgatgatcagcagggccgtatggccggccgcgggaacgggtgcaagtacgggaggcccgctcaccggtcgtcgggcacgccgaacgcagcgcgcatctcgtcgagccgcgcctgcgcgacgtgaaagcactcggaaatctgctcggccgttgccgcgggatagccgggtggcggctgcagcgcattgcccagccgttcccaagcggcctcccacgccagcttggcgagcgcgcgggactccgaggtggttggagcgaccatgttcgtccttggtttgcaaacgcaatgaagtatgcgcccggatatcactaaagtggtgggggctggcggcgcgtaggaggccgctttcacgacgacgcgcgttatcccgccctgccgggacgaaagctgttcaaccatggcggcgaggaggatgacggtttctgcatgctgcagtaaattcaaaactagacccgcgcacgaagagttcttgtaggagccggacccatcgacatgcacggatcaccgccgcgcgccccagccaccgttcacaaggagctgccccgatgaaaacgaccgatctcagccggccctctgccatcgtcgccggcgcgttgtccggcatcggcccggaatggggacgccgctggttggccgggcccggcacggcgcagcaccgctgaacccgggccgatcccatggacacccttttcgggtccggagtcgccgtcgtggacacggttcgcaagagcaccggcggcagcgtcgtggtctggagcgcggatccacaggcctatgccagcgaccatgaacgcgccacgcgcagcaattttgcgcagcggctggcggcgctgaagcagtaccgctttgccggcgaatacgacgcctcgcgcgcccacgagaacacgccgctgtacttcgtgccgagcgacaccgtctccagcacgcaactggcgcgctcgctcggcatctcgacgctgcacgacctgttcgggggcgtggttccgtaccccttcgtggccaccaaggccatcacgcacccgcttgccggccgcgcggccgcctgtcccgaggggtggacgccggcctttccctccggcgtatcggatgcggtgctcgacggcttctccgtgttttcgctcgaggacgcgcgatgggccgggcgccagctgctggaaaacggcacggtgcgcgtcaagcccgtgtgcgccaccggtggccggggccagaccatggtcaccgacgccgaggcgctggaccgctgccttgccgccatggaagagagcgagattgcgctccatggcgtggtgctcgaagagaacctcgagaaccccgagacctacagcgtggggcaggtgctggtcgatcacctgatcatgagctactacggccgccagcgcatgacccgcggcaacgatgggcagagcgtctatggcggctccgacctgacgctcgtgcggggcaacttcgatgcgctgctcgcgatgaccagcccgccaccggcgctgtgcctggccatcgagcaggcgcggcactataaccaggccgtgatcgactgcttcccgggtttctttgcctcgcgcgtgaactacgacgtggcgcagggcgtgggcgcgggcggcacctggcgctcgggcgtgctggagcagtcgtggcgcgtcggcggcgcgaccggcgccgaaatggtcgcgctcgaactcttctggggcgacccgacgctcgaccgggtgcgtgtttcctgtttcgaggcgtatggtgcggaagcgccgatcccggccgatgcaaaggtgcactaccgcggtatcgacaaacaggcaggacacctcaccaaatacgcattgcaaaagccgtatgacagcgacccgacataacttcatagacatatccgtagacggtcagcacattgccggaacgctggttgccgcctccaccatggtgcccggcgttctcctggtccacggctgggatggcagccaggagcagtacatcgcgcgcgcgcacgagattgccgcgctcggctgcgtgtgcctgaccttcgacctccgcggccatgcgcgccacgcctcgctgcgccaggaggtcacccgcgaggacaacctgcgcgacgtgctcgcggcctacgacacgctcatcagccacccgaccgtcgaccccggcgccattgccatcgtcggcagcagctacggcggctacctggcggcactggtcagcgccatgcggccggtgcgctggctcgcgctgcgcgcgccggcgctctacagggaccgcgaatggctggccccgaaggggcaattgagcaggcccgacctcgtggcctaccggcgcacgctggtcggcccgcgcgacaaccgcgcgctggcggcatgcgaggcgttcgtgggcgacgtgctcattgtcgagtcggagcacgaccagatcgtgccgcacccggtgatcgagaactacctgggtgcgttcaagcgcgtgcgctcggcgacgtaccgggttctctcgggcgccgaccatgcgctttccaaacaggcgcaccgccaggcctacgggcaactgctcgtgtcctggatgaccgagatgaccatcggcgccagggcgaccggcgccatgacgcggcccgtggccgcgagtcctgcgtaggaggccctatgaaccccatgaagtctgcaagcccgcggcagctgcaggtgttgcgaaccggcctggtggccggcaccttggcaagccttgcctccaccggggcgctgatgctgtgcggccgccgcgaggccggcagcatggtggcgcccaccaatgccaccagccactggctgtggggcgaccaggcctttgcggtgcgacaacctacgctgaagcacacggccattggatacgccacgcatcacgcgagcgccatcttctgggcgctgctctatgcctggctgcacgcgagtcggcaccctgcgcagtcggtgcccgcggcgctcgccagtgccggtgccgccacggcggtggcctgcgcggtcgactacacgatcaccccgcgccggctcacgccgggtttcgagcatcacctttcgaaacgttcgatgggcatcgtttacggcctcttcgccgtggggctggcggccggctgcctgctggcgcagcgcgggcgcgaccaggcttgatgggggcgggagcgcacgggtagtgcgccgtgctacgtgcactcaaggagctttcctacgtggcggggtttgctgtcctttcatcgttcagcttccatcaacccaaccggagcccacgatgcccacctccaccaagcgtgcagcacccgatgcctgcagccttctcgacaccgaccaccgcaacgtcaagaagatgttcaaggagtacgaggaactgacccattcgcgagctgccgatgcgcagcagaagaagcgcgagcttgccaaccagatctgcaccgagctgaccgttcacgcgcagatcgaggaagaaattttctacccggcgttgcgcaaggcgatcagcgaaaccgatctgctggacgaggccgaagtcgagcacggcactgccaaggaactgatcgcgcagatcgaatcggccaccgacgtggacgacaagttcgacgccaaggtcatcgtgctgggcgagtacatcgaccaccacgtgaaggaagagcgcaacgagatcttcgtcaaggcacgcgccgccaagggcctggacctgatggccatgcgcgagcagcttgcaacgcgcaaggaagaattgatggaagagctcacgggcgtggccgcctgagcgggcggtccgacccggcctttggccattgatcccgacgatcccgacgcccggccggcatcggccgggcgcccccgctttttccctctcgccttggagctcaccatgacaagcatcgtctcccggctgtttcccacggcgaccaacatgattcgcctggaccacacgcatgtgctttccacctttcaccagtacaaggcaagtgcgccgtcccgcgtgaaaaagggcctggtcaacaccatctgcactgcactcgaaattcatgcgcagctcgaagaagaaatcttctatcccgagatgcgcaaggtctgcgaggacgagcgcatcacgaaggcgctcgacgagcattcggagatgcgccgcctcatcagcctgctgcgcaccatggagcccgaagcgcacgactacgacgagactctgtcgtcgctgatgcgcgacgtgatgcatcacgtcgcggacgaagaaacgattctgctgcccgcggccgagaaactgctggccgacaagctcggcgaaatgggcgcgcagatgaccaagcgccggctgcagcttgccgggccgcgctccggcgagatcgccctggacatgggccgcgcggcttcgggcaacaccgcggccatcgcgatggtcgggctggccgctgccgggctcttgctggcacggcgctccggccaccggcgctggcatgcgcgcgcctgagcacgccggagcacgcactctgttgctgcgacagcgacgcaagtcattgaatggagttttcatgccaacttccaagacgcctcccggttccgaccgcgccaccaccagcgctgcggcagccgcccgcaacaccgacagcggcgcggcgaacctgccgggcggaataccgcccgacccaccatcgcagaaggccgcgcacacgcaggcgcttgcggcttcgataccgttcaacgcgaacaagccgctcgagcatggacacgacaacgcgcttcacccccaagccggccagacagccgagccgttgtcgtccgcggcaacggccagcacgctttcggaagagatcggctcggagaaggctggcggcatggccatgccgggcctgaacgccaccatcgaatccctcgaccgggtgcgcgtggactcgggtggccagcggctcaccaccaatcagggtgtgcccatcgcggacaaccagaactcgctgaaggccggcctgcgcggccccgcgctgctggaagacttcattcttcgcgagaagatcacccacttcgaccacgagcgcattccagagcgcatcgtgcacgcgcgcggctcgggcgcccacggctttttcgaatgctacgaaggcattccgcagttcaccaaggcggcccccttgcgcgaagcgggaaaaatcacaccggtcttcgtgcgtttttccaccgtggcgggcgagcgcggctccaaggacaccgcgcgcgacgtgcgcggcttcgccgtcaagttctacacggacgaaggcaactgggacctggtgggcaacaacatgcccgtgttcttcatccaggacgcgatgaaattcccggatctcattcacgccgtgaagcccgagccgcatcaccagatgccacaggccgcgagcgcgcacgataccttctgggattttgtcgggctcatgcccgagtccacccacatgctgatgtgggcgatgtcggaccgcgccattccgcgcagctttcgcatgatgcagggctttggcgtgcacaccttcaggcttgtgaacgaagccggcgattcggtgttctgcaagttccactggacacctgttctcggaacccattcgctggtgtgggacgaggcggtgaagatctcgggcgccgaccctgactttcatcgccgcgacctgtgggaggccatcgaggccggggagtttccggaatgggaactcggcctgcagatcttcaccgaggaagaggccgatgccttcagtttcgacgtgctcgacgccacgaagatcgtgccggaagaactggtgccgctcacgccggttggccgcctggtgctcaaccgcaatcccgacaatttctttgccgagacggagcaggtggcgttctgtgccgcgcacgtggtgccgggcatcgacttcaccaacgaccccctgctggccgggcgcatccactcgtatgtcgacacgcagatcacgcggctgggcggaccgaactttcatgagctgccgatcaacgcgccgatggcgcaggtgcacaacaaccagcgcgacggaatgcaccgccaggccgtccaccgcgggcgcgcggcctacgagcccaactcgctgggcggcggctgtccgttccaggccggcgcttcggcgggcttcatgacctttccgcagcgcgtggagcaggacaaggtgcgcggcaagcccgagaaatttgccgatcactacacgcaggccaggcttttcttcgacagccagacgcccaccgagcaggctcacatcgcggcggcgtttcgcttcgagctctcgaagtgctccgtgcctgccgtgcgcgaacgcatggtggcgagcctcgtcaacgcatcgccgctgctggcgcagcaggtggccgatgggctgggcatgccgctgccgcccgcgctgcccaaggcactcgagcagcccgtgaagccggaagtgacgcgctcgccctcgctctcgctgatggcgcggcccggcgacggatcggtgcgaacgcgcaaggtggcattgctggtggcggacggcatacagggcgagcagatcgcgaccatccaggcggcgctgttggccgaaggcgccgtgggccgattggtgggcccgcgcatcggcccgttccgcaccgccgagggcgagacgatggaagccgatgcatcgatggagaacgagcccggcttcctgttcgacgcgctcgtgctgcccgatggagcaggcggcgtggagcttctctccgccaatccccacaccgagccgttcatcaaggatcagttccagcacggcaagacgattcttgcgctcggcgcgtccgccgtcctattggccgaagcgaagattcccgagaccctgccttcgggcgatccggatccgggcgtgctgcgcgccggggcggagaatttcgagtccgcggtcgaggccttcgtcgcggcgctcgcgaagcatcggcatccggcacgcgaactcggcgtgctggtggcgggcgacgactaaggggagaaagaggcgcgctacagaagatcccgcaggcggtaatacatcatccccagcacgagcgcgggggtgcgcagcatggtgccgccgggaaaggcgtggtgcccgatgcgggcgaagagatcgaagcgttccgcctgtcccgcaatggcttcggccgccagcttgcccgccatgccggtgagcgccaggccatggccggagaagccctgcaggtagtagatgttgcttccgatgcgcccgaaatccggcgcctggttcatggtgatgtcgacgaagccgccccatgcgtggtcgatgcccaggtccgacagttggggaaacaccgcgagcatgctcctgcggattttttcgatgaggttgcgcggcgtcctcgcgctgtagctgtcgcccgagccgaacagcaggcgatggtcagcgctcaggcggaaatagtcgaggacgaagttcgtgtccgatgccgccggcctgcctcgcatgagcgaatccgcgcgcgccttgtccatcggttcggtggcgatcatgtaggtgcccacgggcatgatgcgcgacgacacctcgggcgccacgtcgtccccgtattcggcgaggtagacattgcccgccagcacgacgtagctgcaccgcacctcgccctgagcggtcttgacgacggggtggggcccgcgctcgatcatttgcgccgccgagttctcgtgcaactgagcacccgcggcgcgcgcggcgctcgcaaggcccagcgaatatttcaacggatgcagatggcccgaacgcgcatcgaaggtgccggcgtcgaagcgctcgctggccacgcactccgcaacgtctttggggcccagccattggagcggatagccgtgcacgcggtgcacgtggtccatccattcgcgaagcgcacgcgacttggagggcttgaccgaaaggttgagatagccgggctgccagtcgcagtcgatcgcgtagctcgcaatccggtcctgcatgagatccagcccttcgaccgagatgttccaggcgcggcgcacgtcctcgggcggaaactggttttcaatcgcttcttcgccgtccgagccgaagccgacgatcacctgtccgccgttgcggcccgaagcgccccagcccacgcgctgggcttcgagcagcaccacggcaaagccgcgcgaggcaagttcgagcgctgccgagagccctgcgagcccgccgcccaccacgcagacgtcggcggtggcaatgccttcgagcgggcgcgtggcctcgaaccgcgccgcccgctgcacgctggcttcgtagtatgaattctcgacgacgccgagttccttgcgcagcagcaatcacgtcacccggaagttgaggaactgccacggatcttccctgtccatttcctccttgaagagcggacagcggtccttcagcggcgtccagtcgccatacacgcccaccacttcgccgagatagggcatggcggcctccagcaccacgcggtggtcgaggtcgtccggctccaccaggcccgcatcagggttctgcagcgcccacagcattccgcccaaaatgccggccaccacctgcaggctggtggcgctgttggcgggcgcgagttcgcgcgcctgttcgatggtgagccgggagccataccagtagacgcccttggggttgcccatcagcagcacgccgagttcgtccatgccttgggcgatttcgtcgcggacgattctctggcggtgctgcagctgccagttctttcccgccaattcgtgcagcgagagcacggcgtcgtcgcaggggtgataggcgtagtgcaccgtgggccggtaaaccacctcgccgtccttgcgcagcgtcaggtggtcggcaatggagatcgactcggcatgcgtgaccaggaagccgtggtacgggccttcgagcggcgtccagctgcgaacccgcgtgccgatgcccgggcgctcgaggtagatggccgcatcgctgccgaagccgtgccgcgccgcgtcggccggccagtgccgctcgtgcgtgccccatcccagttcggcgggttgaagcccttcgtcaacgaagccacgtatcgaccaggtgttgacgaattcgtttctctgcttgcgctggctggcaacctgcgagtcgcgttcggcaatgtgaatcaccttgatctcgagccgctgcgcgagcgcggcccagccttcgtagctggtgggcatcgattcgatttcggcgtgcgtgtcggccgcgatgttcagcagcgcctgcttgacaagggccgaaaccacgccgggattggcgccttgcgtgatgaccgccgtgggcccgctgcgcttgtcgaggcgccaggccagcagctcctcgcgcaggctgtagttcgaacggcgcgaagggggaaggccggggttgtcgtagcggccatcccagggttcgttgcaggtgtcgaggtagaagacaccgcgttcgcggcagagcttgatgagcgcgaggctggagacatcgaccgacaggttgacaaggaagtcgcccttgtcgagcaacggctcgagcacggcggccaaattgccttcttcgagccgggtgggaatgacttcgacccccagcttttttgccagcccgctgcggtcttcgccggccttcacgatcttgatgtccgaggccttgagatcgaaatgacgcagcagcacgggcagcagcgcctggccgatggagccgaagccgatcatcgtcagcttgccgccaaggcgcgccagcaattcgttgttgttcttcttcttcgtcgtcatccgcatacctcgctgagtggcaccggccgggcatccgaaatgccggtgcctgcttcggttcagccccaatgtggcgccgccgcaatggcgggtgcgtcagcttggctttgccaatggtgtaggaagactccatgcgcgcagcttgccgcggcttcatggtagaaaccggccaccctgcgcgcgtcgcgcaccgcatcgacccgatgtcagaacacctcaacccgcgaatttcagagacggccggcagcgccggtttgcgccgctcctgggcgcagtggccgctgtggctgctgcttggccttgccttgctggtcatgggcggctgcgcaggcctgccgtcgggggtggaacgcaaaccgtcggtggccatcacggacggcgccgacacggagcttggccgaatggtcgccgcggcatcgccgccggggcaggggctgagcggcttccggctgctgccgatgccgcagtattcgctgcatgcgcgcatcgagctcgcgcgccgggcccagcgctccatcgacgtgcagtactacctggtgcagaacgacgaaaccggtcgctacctgctgcgtgcgctgcgcgatgcggcggagcgcggcgtgcgcgtgcggctcctggtggacgacctctacaccgccggcgccgacccgttgttcgcgggattcgcggcgcacccgaacgtcgaggtgcgaatgttcaatccgttcccggccgggcgcgaccggctgggaacgcgatgggcgtcgtcgctgctcgacttcgaccgcgtgcaccgccgcatgcacaacaagctgttcgtggtggacaacaccatggcggtgatgggcgggcgcaacatcgccaacgaatactttctgcgcgatggcggctccaacttcatcgacatcgacacgctggtggccggcaccgtcgtgccgcggctctcgtcgctgttcgacatgtactggaacagcccctatgtgtatcccgtcgagtcgctggtctcgaccggcggcgccacgccgcagcagctgcgcgagcgcttcgagcagctgaccggaacgccggacacgctgcaccccgagcccattgtttccaccgacctgctgggaaacaatgcgctcgccaaggacctggacgagggcgtgctgtccctcgtctgggcgcgcgccgaagcgtatgccgacgcgcccgccaaggcactggggcccacggacgaggcccgcgggctgccggccgacgaatcgaccgacagcgtgctctacaacgtgcggcgctacctgcgcggcgcgcagcagaacatcctgcagaccacgccctatctgattccgggccgcggcggcatggagacgatgcgcctcgtgcggcagcggggcgtgagctacaccatcgtcaccaattcgctggcggccacggacgaatcgctggtgcacatcggctaccgccgctaccggcccgagatgctgggcctgggcgtggaactctacgagctgagccccaagcgcgtcgaagaaaccaggcgcttcggcatctacggctcggccagcggccggctgcacggaaagtcggccgtggtcgacagcaacatcgtcttcatcggctcgatgaacttcgacccgcgctcgatgctgcacaacaccgagatcgccatcttcatcttcagcccgcagattgcgcagcagctcaccagcctgatcggtttcatccgcctggacggcgcctaccaactgcagctggggccgcgcggcggcatcgaatgggtgagccccgcgtcgggcgacgcggccgacaccatcctgcacgtggagccggaaacggatttctggtcgcgctggaaactggagctgctcgccccgctggtgccggagagcctgctttgaggcgcgttctctgctactgctgcaggcgcccgctcagatagggctcgggatcgacggcggtgccgttcttgcggatctcgaagtgcaccttcacgcggtcggcgtcgctcttgcccatttcggcgatcttctggccctgccggaccaccgcgttctccttcacgaggatggtttgcgcgtgggcgtaggcggtgaggaaggtctcgttgtgcttgatgatgaccatgttgccgtagctgcgcagctcgccgcccacgtacaccactcggccgtcggccgaggccacgatgggatcgccggcattgccggcaatgtcgagccccttgttgcgcacgccgtcgaaccgggcaatggtggtgccgctggcgggccggatgaacatggcctgcggctgctggaccggcggcggtatgtgcaggcccggccgcccgggcggctgcggcgtggtgcaggctgcgaggccggccgccacgagaaccgcggcgccggtacgaaaagctagatctagaaggtgcatggctctgttggaacgatttcgttgcggagggttccttcgggtcggcgcgccgggcgagccaccgcggggcatgctagcaaactctcgaaagctgcccgagggggccggaccgccgggcccggacgtgaaactacttgagcgggatcggggtgccgcggtcgatgggtaccgccgtgacgctgttcttgggcgagccgtcgatcagcaggtcggaataggtgaggtagaccagcgtgttgcgcttggggtcgaccatgcgcaccacccgcagccgcttgaagagaatcgacagccgctcggtgtagacctcctcgcgcttgggcaggggctgcgtgacgctgaccgggccgacctggcggcaggcaatggaggcctccgatttgtcttcggccacgccgaaggcgccggccagtccgcccgtcttggcacgcgagacgtagcaggtcacgccgttgaccttggggtcgtcataggcctcgaccacgatcttgtggtcggggccgatgagcttgaacgcggtgtcgacgtcgcccacgacttcagcgtgcgccactgcagccaggcccgcgccgagggcaaggctgcaggcgagggcgccgcgacgcagcaagatggtcgaggtggcggtggtgaggggtgcctgggtcatgcgtttcaaacgatgctgagttcatgcacgcggtcgaagctgccgcgccgccggtcttcgaagaagtgctccaacgcctcgcgcacggtgcgaaaggcaatttcttcccacggaatttcttcctccgtgaaaagccgggcctcgatggtctcgtggccggggtcgaagcggtcgtccagcaggcgggcgcgatagaacagatgcacctggcctacgcgcaccacgctgatcaccgcgaacaggccctgcatctcgtagtgggcaccggcctcttcgtcggtctcgcgggccgcgccctgggccgcggtttcgccgagctccatgaaccccgcgggcagtgtccacttgccccagcgcggctcgatgttgcgcttgcacagcagcaccttgtcgccgagaacggggatggtgcccaccacgttcagcgggttttcgtagtggatggtgctgcaggccgggcagaccgcgcgctccttggtgtcgccgtcgtcgggaacgcggtagaccactgcggtgccgcagttcttgcagtgcttgatgggtacgcggaggatcatgaagagagggggctcagacgaccttgacggtcagcttgggcagtccggccacttcgcccaccagcgtatcgcccgccaccaccgcggccacgccttcgggcgtgccggtgaagatcaggtcgccgggctgcagctcccaggcggccgacagatgctcgatggtctcggccacgttccagatcagcttggcgaccgtgctgcgctggcggtcggtgccgttcacctgcagcgagatctcggctttttcggcgtcgccggccgcggccacgggcacgatcggaccgatgggcgcgctctgctcgaagctcttgccgatgtcccaggggcggccctgcttcttcatgtcgttctgcaggtcgcggcgcgtcatgtccaggcccacggcgtagccgaagatgtgcttgtgcgcatcggcggccaggatgttccggccgccggtgccgatggccaccacgagctcgatctcgtggtgcaggttcttggtcagggtggggtaggcaatggtgccggtctgtcccgcatcgaccaccaccgcggcgtccgccggcttcatgaagaagaagggcggttcacggccggtgaagcccatttccttggcgtgatcttcgtagttgcggcccacgcagtagatgcggtgcaccggaaagcgggccggctggccgaccaccggaaccgaaacggtggcgggcggggcaaaaacaaactcggaagccattgcgacggtccctttcagcgaaactggaaaaaacggcagtgtgccagaggcaggcgggggctgccggtgagcgctatgctctccggatcatgaagctgcacaactacttccgctcctcttcatcgttccgggtgcgcattgcgctgaacctcaagggcctggagttcgactacgtgccggtgcacattgcccgtggcgaccatcgcaccgggccttactcggccatttcgcccgacatgctggtgccgctgctcgaagacgagggcgagcgcttttcgcaatcgatggccatcatcgaatacctcgacgagaccaaccccgagccgccgctgctgccgagcgacccggtcggccgtgcgcatgtgcgcgcgctggcccagtcgatcgcctgcgagatccatccgctgaacaacctgcgggtgctcaagtacctggtgaaagaactcaagctcgacgacgccgccaagaatgcctggtatcgccactgggtgcgcgacggcatgctggccttcgagcgccagctggcgctgcatcccggcggcatcttctgctacggcaatacgcccacgctggctgactgctgcctggtaccgcagatcttcaacggcaagcgcttcgactgcgacttcagcggcctgccgcgcaccatggcggcctacgaggcctgcatggaactggacgccttccagcgcgcccagccctcgcaggcgcccgacgcggaagcctgaacgagtgacggggcccgccatgatggacgcgcactggctcgtgcccgactggccggcgccaccgaacgtgcgggccgtgtgcaccacgcggcagggcggtgtttcgcagggccgctatgaaagcctcaacctgggcgaccacgtgggcgacctggccgaccatgtcgccgagaaccgccgccttctcgaacaagccatcggcgcgcacccggtcttcctgcagcaggtgcacggcatcggtgtcgcggcgctcgatgaggccgaatcggcgggcgtcgtgcgcgacggcacggcggccgatgcctgcaccgccaccgccgtcgggtcggcctgcacgatcatggtcgccgactgcctgcccgtgctcttcaccgatggatcgggcgaacgggtggcagccgcacacgccggctggcgcggccttgccggcggtgtgctcgaagccactgcccggtgcttcacgcccgagcctgaaaccggtccaccgcacggcgctagcaaagtcatagcttggctcggcccctgcatcgggcccaaggctttcgaagtcgggccagaggtcaaggcggcgttcgaggctcatgggcccgaggccgcaagctgctttcaacctgccacggccgccggcaaatggctcgccgacctgccagcgctcgcgcgtcagcgcttgcgcgcggccggcgtggaggacgtgtacggcaatgacggcagcgacggctggtgcaccgtcgccaacccgtcacggttcttttcgcaccggcgggacggcgtcagcgggcgcttcgctgccctggtctggaaggtttgaatcatttttggctgccgctgcatccgcggccgcggccgcggcggcggcctggcgtgccgcttcctgcgcctcggcctcgcgctgcctcatggcgcggcgccggcccggcgttcccatcaggtaaaccaccaacgccaccggcgccaatccgtacaaaagaaatgtgaagatggcgcccagcacggtgcccgtggtgttggtggcttcggccacggccatcatcacggcgacgtagagccagccgatcacgatcaggtggatgaacacaacaagtttcagtcggtaagtgagtgggcggcgttgtgagcgcctcgtgaaatgcagcatactcaaaacacgagcagccatccgtacagactcaggcgaggaccaggagacatgatgaagcaacaagcgacgggggccgatgcgttcgcgcccttccagcaggcactttcagagggatggaacaaggcgctggaatcgttccagcaatccgccgcacagggggcttcggccttcaatgtcaccggcggcacgcccctgtggcagattccgtcgtcggccaggatgcccgagctgcccaagatctccatcgaccccgaaaagctccaatccatccagcagcagtacgtggccgaggccgccgaactctggcgccagggccccgccgccaagcccgaaggcgacaggcgctttgcgtccgaagcctggggcagcaatccgctcgcggctttttcggcggccgtttacctgctcaacggccgcacgctgctgaacatggccgaggccatcgacggcgacgaaaagaccaaggcgcgcctgcgctttgcgatcgaacaatggatggccgcctcgtcgccgagcaactcgctcgccttcaatgccgaggcgcagaaaaaagccatcgagacgcagggcgagagcatcgccaagggcatccagaacctgctgcacgacgtgaagcaaggccacctcagcatgaccgacgagagcgccttcgaagtagggcgcaacgtggcgaccaccgaaggcgcggtggtgttcgagaacgagctgttccagctgctcgaatacaagccgctcacggccaaggtgtacgagcggcccttcctgctggtgccgccctgcatcaacaagttctacatcctcgacctgcagcccgagaattcgctgatccgctatgccaacgagcaaggccaccgcgtgttcgtggtgagctggcgcaaccctgacgaatcgctggccaacgccacctgggacgactacatcgagaacgccgtcatcaaggcgatccacacggtgcaggagatcagcgcaagcaagcaggtcaatgcgctcgggttctgcgtgggcggcaccatcctcagcaccgcgctggccgtgctcgcggcgcgcggcgaaaagccggcggcgtcggtcacgctgctcaccacgttcctcgacttcagcgacaccggcattctcgacatcttcgtggacgaggccatggtggcgtaccgcgaaatgcaactgggcaagggcggcctgctgccgggcatggacctggcctcgaccttcagcttcttgcgcccgaacgatctggtgtggaactacgtggtgggcaactacctgaagggcgagacgccgcctcccttcgacctgctctactggaacagcgacgccaccaacctgccgggcccgttctacacctggtacctgcgcaacacgtaccacgagaacaagctggcgaagccgaacgcgctcaccgtctgcggcgagaagatcgacctcggcaagatcgacatcccggcctacatctacggctcgcgcgaagaccacatcgtgcccatcggcggcgcctatgcctccacgcaactgctgccgggcaagaagcgcttcgtcatgggcgcctcgggccacatcgccggggtgatcaatccgcccgccaagaaaaagcgcagccactggatccgcgacgacggcaagtttccgaagacgcaggccgaatggttgaccggcgcagaggagcatcccggcagctggtggaccgactgggcacaatggctcaagggccatgcgggcaagcagatccccgcgcccaaggcatacggcgacggaaaaaaatacaaggccatcgagccggccccgggccgctacgtcaaggccagggcctgactggccggcacacgcactcgttcactcacttcaaatcacttcaacggagaacctcatggaagacatcgtcatcgtttcggctgcacgcacggcggtcggcaagttcggcggctcgctcgccggcattgcggccacggagctgggcgccctcgtgatcaaggaagtgattgcgcgtgccaatctcacggccgaccaggtcggcgaagcgatcatggggcaggtgctggccgccggcgcgggccagaaccccgcgcgccaggcatggctcaagggcggtggcgccaaggaaaccccggcgctcaccatcaacgccgtctgcggctcgggtttgaaggccgtgatgctcgcggcgcagtccgtggccacgggcgacagcgaaatcgtgattgccggcggacaagagaacatgagcatggcgccgcacgtgctgcccaactcgcgcaacggccagcgtatgggcgactggaagctggtcgacaccatgatcgtggacggcctgtgggacgtctacaaccagtaccacatgggcatcacggccgagaacgtggccaagaagttcggcatcgaccgcagcgcgcaggacgagctcgcgctcggcagccagaccaaggccgcggccgcgcaggatgccggcaagttcaaggacgagatcgtcggtgtgagcattccgcagaagaagggcgatcccatcgtcttcgacaaggacgagttcatcaaccgcaagaccaacgccgaaggcctggccggcctgcgtcccgccttcgacaaggccggtggcgtgaccgcgggcaatgcctcgggcctgaacgacggcgctgccgccgtgatggtgatgaccgccaagaaggccgcctcgctcggcctcaagccgctgggccgtatcgcgagctatgccaccgccggcctcgacccggccatcatgggcatgggcccggtgcccgcgtcgaccaaggcgctgcagcgcgccggctggaaggccgccgacctcgacctgctcgagatcaacgaagcctttgccgcgcaggcctgcgccgtgaacaaggaaatgggctgggacgtgaacaaggtgaacgtgaacggcggcgccatcgccatcggccaccccatcggcgcgtcgggctgccgcatcctggtgacgctgctgcatgaaatgcagcgccagaacgccaagaagggcattgcctcgctgtgcatcggcggcggcatgggcgtggcgctgacgatcgagcgataggtcgttcatcgggcggcgcactttgtgcaccgcccaaattttgagcaaactgattatttcttatataaaacaacgacttaaatcgcgtttacaaggaagcacatcagttatccccaaagttgtccacggaaattggggacggcaagcgcttcttcacgattcggttgcaagcccttgttttcagtagaacggagcggccatcaggcgatggccgcctgctcgccggcatagtgccggcatagcgtctcgaccagcgcctgcgcatagatgggcagcgccgcccggtcccgcaccagcagataccgctcccgtacgcaccacgcatcgctgagatcgatcagcgcgagctgcatgctctcctggttgcgccgtgccgccgactccggcaccacgccaatgcccacgccgctaccgatcatccggcacatggcgtcgaagctgccgagctggatgcgcagcttctgccgcttgcccaggttgtcggtgatctgcgcgagaaaggcctgcaaggtgctgccctgctgcatgccgatcgcgtcttcgtcgagcgtctcggcgaatgaaatcttgcggcgcttcgcgaagcggtgcttgcgcgaggtgacaagcaccagccggtcggtgctgaagtggatggcttccaggcccagcgtgtcgacgcggcccgccacgatgccgatgtcggcgcggccgtcgagcacgccgcgcgggatctgagcattcggtttttcctgaaggtcgacgttgatgcgcggattgcgcgcaaggaagccgggcaggatttcaggcaagaaatcggtcaccgccgtggtgttggcaaatacgcgcagatggccgcggaggcctccgccgtattcgagcaggtcggcgcgcagctgttcggtctggtgcagcaccagccgcgcatgatgcaagaaggcttctcccggcggcagcaggcgaacgccccgggcttcccgctgcagcagctgcaacccggcttgggtctcgagcgccttgatgcgcgcactggccgccgcgagcgacagatgctgccgctcggccgcccgcgtgaggttgccgagttcggccgtggcaacgaaaaggcgcaggtcggtcaggtcgaaaagcatggcgccatcgtacccaagccttcgggatttcagaaggctgggttccgaaatcgcagattgcgcgaaggcggggggccaacgaccatgcgggcatggagacaacacacatgaacctcaaattccgcgtcggcgcgctgctttcgctggcggccgcgcttgtgcttgcgatgagcccggcgggcgcagagccttatccctcccggcccatcacgctggtcgtgccgcaggccgcgggcggcaccaacgacatcgtcgggcgtctcgtggggcagaagctcggcgaggtgatgaacaacgccagcgtggtggtcgacaaccggcccggcgcgggcggcaacatcggcacgcaactggtcgccaggggcccgaaggacggctacacgctgctcatgaccatcagcagcagccaggcgatcaatccggcgctctacaagaacccgggcttcgacccggtgaaagacttcaagcccgtgggcctgatcggcgcggtgcccaacgtgctgctggtcaacccctcgtttccggccaaggacttcaacgagttcctgaagctcgcgcggcagaagggcgccaactaccagtacgcctccgccggcaacggcacgctcaaccacctgctcggtgaaatgctcaacagcatggccggcatctctttgcagcacgtgccgtacaagggcgtggcgcctgcgatcaacgacgtgctcggcgggcagttgccgatcgtgttcgcgagcctgccgtcggcgctctcgcacatcaaggcgggcaagctgcgggcgctggccgtgagcggcgacaagcgctcgcccgtgctgcccgacgtgcccgccatcggcgaggcggtgccgggctacaacggcacgctgtggatcggcctgttcgcgcccgcgggcgtgccggccgatgtgctggccacgctgcaggatgcaacgcgcaaggcgctggccgccaaggacctgcgcgacaagctcgaccagcagggcgtcgaaatcgcggcgcccaccacgcccgatcaattctcgaaattgctgcaggacgaccttgccaagtgggcacgcatcgtcaaggcatccggcgctgcggtggattgaaagaaccatgaacgattcgatgcatgaaacttcttccgcgctgatcgacggcgatgcgctggccaggctccaggcgtggcagggccgcagcgaaacgctggccgacgaggtcactgccgcgcccgtgcgtgctctctccgccacgctggatcgcgacgatgcgctgcctgtggccggcacgcgcctgccggagctttggcactggctctacttcctgccgcaccatcgccagtccgaaatcggtgacgacgggcatgcgaagcgcggcggcttcctgccgcccgtgccgctgccgcgccgcatgtgggccggcgggcggctggcatgggagcaaggcaatccgctgcaagtgggcgacaaggtggagcgcacctcgaccatcgcctcggtcacccacaaggcgggccgcagcggcgagctggtgttcgtgctggtgcgccatgaagtgcgcaatgaacgcggccttgctctcaccgaagagcacgacatcgtctaccgcgccgcggccgcacccggcgagaagaccccgccgcccacgccggcaccgaaggacgccgccttcagccgcgagatcgtgcccgacgacgtgctgctgtttcgctactcggcgctcaccttcaatggccaccgcatccactacgaccgccgctacgtgacgcaggtcgagggctatccaggcctgatcgtgcacgggccgctcatcgccacgctgctggtcgacctgctgcgccggaacgcgccgggcgcgcagctcgcgcgctttgaattccgcgccgtgcggccgaccttcgacatcgcgccgttccgcgtgcatggcaagccggccgaaggcagcacggacggcaagactttcagcctctggggcgaagacgccgatggctggctcacgatgcaggccacggccgtgctcgcatgaacaacaggaagaacaagcccatgaccagacctctagacggcatcacggtggtttcgctcgaacatgcgattgcggcaccgttctgtacccgccagctggccgatcttggcgcccgcgtcatcaaggtggagcgacccggcgtcggcgactttgcacgcgcctacgacgcacgcgtgggcggcgaggcctcgcacttcgtgtgggtcaaccgctcgaaggaaagcctcacgctcgacctcaagcagcccgccgcgctcgcggtgctgcaagaactggtggccgaggccgacgtgctggtgcagaacctcgcacccggcgcggccgcccgcatgggcctgggcgccgaagcgctgcaggcgaagcatcccaggctcatcgtctgcgacatctccggctacggcgaagacggtccgtaccgcgacaagaaagcctacgacctgctgatccagagcgaggcgggtttcctgtcggtcacgggcacgccggacgatccgtgcaagtcgggcaattccatcgccgacattgcggcgggcatgtacgcctacaccggcatcctcgcggcgctgctccagcgcggcaagaccggcaagggctcgcacatcgacgtgtcgatgctcgagtcgctcgccgaatggatgggctacccgatgtactacgcctacgggggcgcgccgccgccgccgcgcagcgccgcctcgcacgccaccatctacccgtacgggccgtttcctgcgggcgatggcggcacggtgatgctgggcctgcagaacgagcgcgaatggcgcgtgttctgcgagaaggtgctgctgcagccggggctcgcgaccgacgcgcgcttcgacagcaacgcgcggcgcaacgaaaaccgcgatgcgctgcgcgcgatcatcgtggaaactttcagcgcgctcggcactgtgcaggtggtggagcgcctcgatgccgcgcagattgccaatgcgcgcatgaacgacatggcgggcctctgggcgcatccgcaattgcaggcgcgcgagcgctggcggcaggtgggttcgccggcaggcgacattccggccctgttgccggcggggcgccagagcgccttcgactaccgcatggacgcgataccggctgttggggagcacaccgaatccatcctgcgcagcctggggcgcggcgatgccgagattgccgcgctgcgcgaggcgggggcggtgtgagcacggctgtgaatccgccgctggccctggcacgcacttttctcttcgtgcccgccgaccggcccgagcgccacgcgcgcgcgctggccaccggtgcgggaggcgtcatcgtcgatctcgaagatgccgtggcgcccgatcgcaaggtggcggcgcgcgagcagctgaaatcttctttcgctgcattgtcggccgcggaaagagggcgcctgctggtgcgcatcaatgcccatggcacaccgtggcacgacggcgaccgcgcgctggtgggtgagcttgccgccgaaggcctgattgccggcgtggtgctgcccaaggccgaacgcgctgcggacttgcatcggctcgccgcggacatcggccccaagggcctgctcgtgcccttgatcgaatccgccgcgggcctcgaagccgccgccgaactcgcggccgcgccgcaggtgctgcggctcgcgttcggcaacctcgacttccaggccgacctgggccttgcctgcgatgcggacgaggccgaactggtgccggtgcgcctggcgttggtgctggcctcgcgccgtgccggcctggccgcacccatcgatggcgtcacgcccgattggcgcgatgcgccgcggctcgcggccgacgccgcgcgtgcacgccgcggcggcttcggcgccaagctctgcattcaccccgaccaggtggcgccggtgcacgccgccctcggcccgagcgccgatgagttggcatgggcgcgccgcgtgatggatgcgacccgcaccgccggcggcggcgtggcgagcctcgacgggcgcatggtcgacgcacccgtggtgcgcctggccgagcggctgctcgcgctcgatacgtaaacggtgccctgacgagcgccgcagatttacatcaagacaaaggagacaacgaagtgaacgcaacaagcaactggaaatcacgggcaatgcatgcggctgcgctgggcgcctgcctgctggcggtccaatcgcccgcggcggcgcaggccccgtggcccgagaagcccatcaccatggtcgtgccgtattcggccgggggccccaccgacgtggtcgcgcgcatgctcgcgattcccatgggcaagtcgctcgggcagaccgtgatcgtcgagaacaccgtgggcgcgggcggcaccatcgcacccggccgcgtggccaaggcggcgcccaacggctacaccatcctcatccatcacatgggcatggccaccgcgcccgcgctctacaagaagctcaactacgacccgctgaaagacttcgaatacgtcggccaggtgatggacgtgcccatgaccttgctctcgcgcaaggactttccggccaacaacttccaggagctgctggcctacgtgaagacccacaaggacaaggtgacactcgccaacgccggcatcggtgccgtgtcgcaactgtgcggcatgctcttcgcgcaccagatcggcgtgcagctcaccaccgtgccctacaagggcgccggtcccgcgctcaacgacctgatgggcgggcaggtcgatctgctgtgcgaccagaccacacagaccgcgccggtcatcaaggacggcaaccgggtcaaggtgttcggcgtgaccacgcccaagcgcctgtccagcatgcccaacgttcccacgctcgacgagcagggcctgaagggtttcgacgtgaaggtgtggcacggcatctacgcacccaagggcacgccgccagccgtgatggaaaagctcaacacggccctgcgcgccgcgctgcaggacgacatggtgaagcaacgctttgccgagctgagcaccgaggccgtgccgatggacaaggtgacgcccgaggcgctgcgcaagcacctggcggccgagaccgagaagtggggcaaggtgatccgggcggcgggcgtgcaggcggattagcctgccgaggattgcgcccgcagcgtctcgtcgaacagcaagagcaattgccgcgcgaacacgtccatgttcgacacgcggtccgcgtcgccggtctcgatggtcctgcttgcggtggccgcacccgcgatggccacgcacacatggcccggcgcgtcgccgtaagggctgccggacgggccggccgcgccgctctcggcgattccccacgtggcgcggtggccgtcgcggatcctgcccgcgatgaacctggcatagggttcggtctcggcgcgcatgccgtcggtcatgtcttcgggggtcagccccagcagcgctttggcggcgcgccgcgagtagacgaccgcgccgcccaaaaagaaagccgatgcgccgggaatggctagcagggcggccgacacgaggccgccggccgaagattcggccacggccaccgtctggcgccgctcgcgcagcgtggcgccgacgcgggcggcgagcacggagagcggctcgaggccggaaatgtcaggcattgaaccgccgcatgtacgccggcgcccgctcgcggctcgccgtgctggcgtagaccgtgccggcgacctcggggaagatgatgatcccgaaattcatgctttcgaactccttggtagaggaagagcgccttcgcaacaacagtggcagtgccgcggagattgcgcgcgcccggaacgggagtcaccgccgcgtcatcgtcggtttctagcatgcgcccacatagcgcaggtctgccatgcaggggcgcctgactgcattcactcaccaacgaggagactcccttgaacagcttgagaaaagtctgcaattcccttttcggcctggccatgttgcttgccgcggcaacaccggtcgcggcgcatgaggagaacgcgcggcgtcgtgccgacaatgcaccgctggtgatcggacaccggggcggcgccaacggttacctgcccgagcacacgctggaggcttatgcgctgggcatctcgctgggcgccgactacatcgagccggacctggtcgccacgaaggacggctatctgatcgcacggcacgaacccaacctgatcgacaccaccaacgtcaaggacctgccgcagttcgccaatcggcggcgcacggtcatgctcgacggtgttgcgaccgacggcttcttcgccagcgacttcacattggccgagatcaagcaattgcgcgccgtgcagtcttttccggagcgcgaccagggcttcaacggcaggttccagattccgacgctggtcgaagtgatcgaactcgccaagcgcaaatcccgggaggaggggcggcgcatcgggatctatccggagaccaagcatccgacctaccaccagggcatcggcctgccgctggaagaccggctgctgggcgtactgagtgcggcgggttggaaccagcgcaacgccccggtcttcatccagtccttcgaaaccgccaatcttcgctacctgcgcagcaagacgagcgtgcggttgattcagctggtcgatgcgaacgacgtcaagcccgatggttcgctggacttcagcaagccctacgacaagccatacgactgggtggtgtcgaaccgcgacggccaattcaaggatctgctgacgccgcgcggcctgcaggaagtaaggggctatgccgacggcatcgggccatggaagccatatctgatctccagcgcctgcaagtcgatccagggtggcgcatgcgccgacgtcacgggcgatggcgtggtggacgagcgcgaccgcgtgctgctgccgccgagcgacgtgatcgcgaacgcgcacaagctggggttgctggtgcacccctacaccttcaggagcgaacagaagcgcttgactggaagcttcggaggcaatccgatcaacgagtacctggcgttctacgaggccggcgtggacggcctgttcagcgacttcgcggacaccgccgttgccgcgcgcgccatgttcctgctgaagcatgaccccgactatgccggctgtctcgtcaacgcgcgcaaatgcgaacgcaataacgattgacggagcggcgttcgcacattcgcaattagcccgtgaaaattaatccttaagcaaataccgactcgaaattacgccatatgtcttatggaaaaaattcgcgaacaaaggctaaaagatcatttgccctgattcaagtcacaaacaagtaactgttcctaactagagttaactttgaatccaaggattccgagaggcattgcagcaaagccagttgcatgcctgtcgaatcgcactgcccaccttgggcaatctcgttttcaaggactccaggaggaattcatcatggcagtagacatgttcatgcgcgtcgagggcgcaaacggcgaatccaaggactcgaaccataaggactggacggatatcaagtcgtttgcatggggagcgacgcagcctggaaacatggtcagcggcggtggcggcggtgtgggcaaggcgagcttcaacgacctgcaggttcttgcgcgcatcgacaaggcggccccgtccgtcatgaagaactgcgccagcggcaagcacctgagcaaggtcgaggtgtcggtgtgcaaggccgggggctcgcagatcgaatacacgcgcgtcacgctggaagaagtgctggtgacctcggtgcagtacacggccgagcagggcagcgatgcggtgctggtgcagttcgcgttccaggccgccaaggtcaagcagcagtactgggagcagacggacaagggcggcaagggcgccgagaccgtgctgggctggaacatcaaggaaaacaaggaggcctgagcctctcgtcgttcgatgcctccagggcctcatcgcgcatgaggtcccgggcatcccggccacgcctctttccgtagggccaactcagggagatctcatgccaacaggctcggcgcagcttgcgcgtgttctcagcatttcgtcgtccgccatgccgacgctgggcggcgagccggcgttggagcccattgccatcgacggcaatgaagggctgagccgcctgtttcgctacaccctgaccctggccacgccggagcagcccggctacaacgagcgccaggccgccaacgtggccatcaagcaactggtgggcgagggcctcaccgcccacatcgtgctcgatgggcgtccgggtgcggggccgcagcggcgccacatctcgggcctggtgacgcgcgtgcgcttcctgcggctggagaaccggcgcgcactgtacgaagccgtgatcgaaccctggctcaccctggccatgcgcaccagcgactaccgcatcttccagaaccagaacgtgctggacatcgcccgggaggtgctcggcaagtacggctttccgttcgacgtgcgggccacccgcagctatccgccgcgcgagttccaggtgcagtacggcgagagcgaccatgacttcgtcgcgcggctgctgcacgagtggggcctgtatttctacttcgagcacgaagagggcaatcacaagctggtcatcgtcgacgacatggcgtcgcaccagcccttcgcccatgcgggctaccagcgcattcccttccatgcggccgacgccaccgtgcgcgaggaacgttgcgaccgcttcaatgcctgcgaggagctgcaaagcggccgctgggtcacggacgacttcgacttcaagcgccccaaggccgagttgcagcaggtcagcgccatgccgcgcaagaccgcgcagaacacctgggaacgctatggctggccgggcgactacgtggtggaggccgaaggcgagcaactcgtgcgcacgcgcatggaagagaccggtggccagggagagcgcgccagcggctcgggcaatctccgtgcggtggtgccggggtatctgctcacgctggagcgccatccccagaacgagtcgaaccgccagtacctggtgaccggcgcccacttgcggctgcaggatgtgggcgatgccagcgaccagcaggagttcgagtgccgcgtggatttcgaggtgattccaagcagcaaggtgttccgggcgccggcaccgctggtgcccaggccgcgcaccacgggcccgcagacagcgatcgtcaccggccccgcgggccgtgagatctggaccgacgaatacggccgcgtgaagctgagctttcactggaaccgctactgcaccaaggacgagaacagctcgtgctgggtgcgcgtgtcctcgccctgggccggcacccacttcggcgggatccagattccgcgcatcggccaggaggtgatcgtcgatttcgagaacggcgatcccgaccgtcccatcgtgaccgggcgcgtctacaacgccgacaacatgccgccgtggaagctgccggacaacgccacgcaaagcggcctgctcacgcgcagctccgaaggcgcgacggatgccaacgccaacgcgctgcgcttcgaggacaagaaggggcaggagcaggtgtggctacatgcggagcgcaaccaggacatcgaagtcgagaaggacgaaacgcactgggtgggccatgaccgcagcaagaccatcgaccatgacgagacggttcacgtcaaacatgaccgcaccgagaccgtggaccacgacgagaccatcacgatcggcaacaaccgcatggagacgatcaaggccaacgagctgttgaccgtgctgcagaacatgaatcgcttcgtggcgctcacctcgtcggaggaggtcggcatcgcgaagacctcgctggtcggactcacccagacggtggccgtgggcaagagcaagaacgaaaccatcggcgaggacttttcgctcgacgtgggcgagaagcttgtcatcaccgtcggcaagagccggctcgagatgacgaaggatggacaggtgacgctgaccggcgccaagttcgacttccgtgccaccggcgcggtgcggatcaacggcaaggtcatcgacctctgctgaggcccgggcctcaagaacaagacaccgttcatggcgctggaccccaaggccactgcatcggcggcttcttcgctcgcaacgccgggcggcacgctctcgggtggcttgggcgcgggccggattgcgcgcctcgcggtgatcgtgggcaagcccgcaccgaagacgcccgcgagcgaagcgccgcccgagggcgggcgagatgtgggccaggcgatcgtggtgtgcaccgcgcccgatgtctgcaagacgcccatcggctcctcgacgccgcccattccctaccagatcaccggcaagctcggcgacgatgccaacacctcgcagaacgtgtttctcacgggcctcaaggccttcaagttcgacagtgtcgtcacgaacgtcaagggcgacgagccgggcgcggccaaggggatcaagtcgggcacggtcggcgacatcgcggagccgaagacggcctccaccgtcgtccgcgtcaacggccagtggttggtgcgcgacggcgacacgttctggatgaacaagcgcaacaccgtcggcgaactgaactacaagaaggaccgcagcacctactggccggccgccgacgccagcgcgatcgacgacagcgaggccgaggcgctgctggcgcgggcgcaggccgatggcgccgccatcgactactacgagacggaccaggaaaagaccggcaaggcgcgcctcattcccgcgtcgagcatggccgactatgcgagcctggtgcgcacgacgatgggcgaaaagccgatcctgctggcacaggcccagttgcagcagatgcccaacgcgacggtcagcgacgcgcgcgccggcgcgatcccgcagacgcggccggcgccgacgccgaccttccagcctggcccagcggccaacgacaacaacttccgtccgcccgcgggcatgccccgccccggtggcagtacggggatggccggcaaggcggccggcgcggcgggcaagatgctgttcctgctctggatcgtccagggtgcgccgatgccgggcgacaacctcatcctcggcaaggccgcggcgaagcgcgtcctggagggcatcaacccgcagacgccgcaggagcaggcaatctacgaccaggcggtggaccatctcgccgaatacaaggcgagcgtgtacgactcgtggtggcccacgggctccgacaagttcgacgcggaggtgcgcaaggccgtcgaggaccagatcgccgaagagcgcacgcgcgcgcagcagcaacagcagcagccctcgcagtcctcgcagccccaggcgaatccggctcctgaggccggcgtacgcgtcgaaggccagcccgacccctgcaaccccggggcgcacggcaagaacaactgcccgcccggccaggattcacatcacatcattgcggactacatcatgcggctcggaacccgcagggagccgggtgcgcggctgccgggtgctccctcgctcgacgacggccccgcgatctgcctgaccgagaaggagcatgcgcgcgtgcaccaactgatggatggtgcaatcaaggccgccggcggggatgccggaacggtgtccttcgaaaaagccaagcagatcgcctacgaagcgctgggagcagcgaaaaaggactgcaagggaaaattcgaagcggcgaccgatgaatacttcaagaaggtccccgaagatgcgttggctcgcgctttcaagacggccccgaaagcgatcaaggacaaggcactccagacattggaatcggcgtgggaaaaactccgccccctcaatccgcccaaataggcacaccacccaggcatcacccatggagcaattcgattccccccccgagaaacccgaactcagggtcgaaaccggcgtcgcggcgacgaaagacttcctgatcatttcctgttcgaagaaggaggatcgcttcgaggggttcgcccgcgtctgcgtgttcaatgccggtgcgcaggtgccatggcattacttcgatctccccttgaccatcagcgccagcgcggcgttccacccttccgcggcaacggccgcgtcgctggccctggtcgcggaggacggcgatgtctttcgcctgccgctcgatgcaagtccggtcatggagcgcgtggtgggttccggcctgtggaacgacgattccgaaggttggggctatctgacgggtgcgcgccagatcggcgagcacctgcatgtctacgggggtgggggtcagatctaccggcgtgcggaggacggcacctggcagcacatcgacgatggccttctgcagaaaccggacggcgtgcacaacgtcttcatgaacgccgtcgacggcgcaggggagggcgaaatctatgccgcgggctgggactcgaagaccgacgcgggcctgctgttctttcgcgagggcgacgcctggaaaaagatccaggtggaaacggccgagctcaacggcctgtgcgtcgaagaccgcgagaccgtctgggtctgcggtaaggacggaaccttgctgcgcggaaaccagaagacagggttcctcgacgtctccggaaccgaaaacgtcagtgactacagcgacgtgaagatctacgcgggcaaggtctacctggcggcccccgaaggattgttcgtccgcgagaacgaagtcatcgagcccgtcgtgacgggcttggtgcccgagtaccgcgacggccacgtgctgcaggtggtcgacggcgtgctgtggtccattggctatgcggacatcgcacgcttcgacggccaggcgtgggagcgcattccgttcccgggcaacccgccgatcgcgtaggcccgatggccttgtggaaacgcgacgtggactgggtgggcgaggcggcccagcgcatcggctgctgcggcctggccgcatggctgccggagttcgcgacctgggccgaactgacgcccgccgagtgcccaccgtcgaagcccaatcgcaaggccgactacgccagcctgtcgcgcggcgtgaagatgacgcttcactaccccttcgccgctcgcgccccgggcgccgatgcgcaggcgtgggtgctctacgaactcgagatcgatgcggccaggcttccgctgcccttcggtctcgatgccggccgcgagactccccagggcgcgaggcgcaagctctcgaacgacacggccctcggccgcccgggcgatccgcgcgacggtcatcggcgcatcgttcactacctgcccgacggccgcgtggtcggcgtcggcttcaaggcctcgctggcgggcatcgagcacctgcatctgcagcgcatcgttgcgatgcccgatttccgcacactgggcgcgggcgtcgcgtgacgaacacgccagcggatccaccgggcacgcccttcctgccggcccggccggtgccggaggcgcccgatgccggcgacgtcgttcatgtcgatgcctgcggcacgcgctgcccggtgcccatcctgcggctgcgcaaggccgtggtccgcagcatgccggggcaggtcgtggtcctcgtgacggacgaccccgcggcgatcgtcaatgtgcaggaggcggtggcctcgctcccggcccagctcttcgacatccggcgcgaagacgatcgcgtcatcttcaccctgctgcgccaatgacggcattgccttgcagccttccactgcccaggacccggcatggcccccacgcttgagaaccgcacgcccttttctgctcttgccttctcgcagttccaccgcgacggcaccgacatggccgtgctctcggtgcgcggcaccttccatgtcgtgcccgacgcgccgctggtgctcgcgccgcggcaggacgaggtcgagctcgccgatcgctacgagggcgatcccgccggcgggctgctggtgcgcacctgcgacctcgtccccttcaagcccgccgccgacctgacgatcctgggctcgagctgggcaccgcgtggcgcacaggcgcagtcatggatcacgggcgtgcggttgggcaggctcgagaaggtcgtgcgcgtccatggcccgagggcgtggcaacccgtcgcggtcgaaggcgaaaagagcggatcgaccggcaaggactggacgctttcgccagcccaccccgccagggccgtctcgctcggctggtgccaggccttcggcggcccgatccctggaacgggcgacgaagaaacgcccatcgacgtccaccgcttcaaccccatcggtcgcggtatcgtcgatgccgaccacagccccgcggacgccgacatcgccgcgccttccatcgaggaccccgccgaccctgtgctcgactggcgtcgccatgaccatgtgccgcagggcttcgctccgcttccgccggtctggcgttcccggcagcagtacgcaggcacctacgacgatgcctggctcgcagagaagcatccgctgctgcccgacgatttcgactaccgcttctaccagtacgcagcgccggatctcatccaccgggagcgcctggctggcgacgaggaactgcagctcctccacatgcacccggaccatacccacatccaggtctggctgcctggcgtgcaactgtcgaccactgcgcattggcatgacggaaccaccgcctcattggcgttgatgctcgacggcatccatgtggacctgacctcggatgtggcgacgatctaccttacctggcggtgctgggcacccaagcgttcaggtcttcattcgatggagctgcaggtcgaaaacccttcgagtctcctggaaatcgggagccggtacgtcaagcatgaccgggtgaccggcgcgccatatcgagagcccgcaaactcatactttcgaactccttgaaggcgcccttgatgcgcaagaaggtacagactcatgcatatggttgcacatcggccctgcattgacagctgcttgccagcttggctcagtgttttcctcagcgatgggtggcttgaaattcgctagagtgaaggtggccgttcaggcttttgcttcgtacacatcaaggaaaatttcatgagcaagaaagttgcatatgtcaccggaggcatgggtggcatcggaactgccatctgccagcgtctgcacaaggacggcttcaccgtcatcgcaggctgcggccccacgcgcgaccatgccaaatggctggccgagcagaaggccctgggcttcgagttccatgcgtcggtcggcaatgtcggcgactggcaatccaccgtcgaggcgttttcggccgccaaggctgcgcacggtcccatcgacgtgctggtcaacaacgccggcatcacgcgggaccgcatgttcctgaagatgacgcccgaagactggagcgcggtcatcgagaccaacctcaacagcatgttcaacgtcaccaagcaggtggtgagcgacatggtcgaaaaaggctggggccgcatcatcaacatcagctcggtcaacggtgccaagggccaggctgggcagaccaactactcggcggccaaggccggcatgcacggcttcacgatggcgctggcgcaggagctggcgaacaagggcgtgacggtcaacaccgtgagcccgggctacatcggcaccgacatggtcaaggccatccgccaggaagtgctcgacaagatcgtggccaccatcccggtcaagcgcctgggcgaaccgagcgaaattgcctccatcatctcgtggcttgccacggacgagggcggctacagcaccggggccgatttctcggtcaacggcggcctgcacatgcactgacgctgccgaccggaacccgatcgacaagacccgcttcggcgggttttttcatttgaaggctgtgccttcaacgaatggaacgtggctgaaacggtcctgaagtttttgtcggcgcagggcaagggaaatacatcgctcctgcaaaatggaacgatgccgcacagcgtttccctgatcaacaccattgccgccggcctgggcctggcgctcgtgttcggtttcctggccgtgcggctgcggctgccggcgttggtgggctacctgctggcgggcgtgatcatcgggcccttcacgccgggcttcgtggccgatgcgggcattgcggcgcaactggccgaaatcggcgtgatgctgctgatgttcggcgtgggcctgcatttttcgctcgacgacctgctggcggtgcgcaagatcgctctgccgggcgcgttggcgcagatcgcggtggccaccctgctcggcggcgcgctggcgctctggtggggctggtcctggggcgaggcgctggtcttcggcctggcgttgtcggtggcgagcacggtcgtgctgctgcgggcgctcgagagcctgggcattctcgactcgttcacgggccgcattgccgtggggtggctggtggtcgaagacctggccatggtgctggtcctggtgctgatgccgccgcttgcgggcgccctgggcgggactgtcggcgatccggcgcgcggcgcgccggaccctctgtggcagacgctcgggctcacgctgctgcaggtgggaggcttcgtggcgctgatgctggtggtcggaaggcgggccttcccctggattctctggcaagtcacgcgcaccggctcgcgcgaactgttcacgctgtgcgtgatagcggcggccgtgagcatcgccttcgcatcggcagcactgttcggcgtgtcgtttgcgcttggcgcgttcttcgcgggcatggtgatgcgcgaatcggagttcagccaccgcgccgcgcaggaatcgctgccgctgcgcgacgccttcgcggtgctgttcttcgtgtccgtgggcatgctcttcgatccttcggtgctcatcgaacgcccgctgcaggtgctggcggtggtggccgtgatcgtgctgggcaagtcgcttgccgcctgcgcgctggtgctggcgtttcgctatccgctgcgcaccgcgctcaccgtgagcgcgagcctcgcgcagatcggggagttctcgttcattcttgcggggctcggtgtatcgcttggcgtgctgccggtcgaaggccagagcctcattctggccggcgcgctcatttccattgccaccaatccgctgtggttcagcctgatcgtgccattgcaaaaatggctgcatgcccgtcttccgtttgcggcgaaactcgaatcgcgcgaccatccgctggccgaattgcccacaaccaccgaagccaggtacctctccaggcaggtggtgctggtgggctacggccgggtcgggcgccgcatcgcgtccgagctggaggcgaacgacgttccttatgtggtggcggagcagaaccgcgaactggtggagaagctccgcgaagccggggtggcggccgtgtggggcgatgcggctgatccttcggtgttgatccaggcacatattgcgcgcgcccgggtgctggtggtggcaacgccggacgccatcaacgcgcgccagatgatggaaatcgcgcgcacgctcaatccggcaatcgagaccgtgatccgcagccacaacgaagatgaagcccggctgctcacgcaggagacgaccgcaaccgtctttctgggcgaacatgaactggcgcaggccatggcccgcgacgtggtgcggcgcgccgtggctgctgcggcctccgctgccgccggatcggggagtcaaaggtcttcgatgaccagcgtgcgatagcgctgcgcgatcgaatagggcacggtgcgcaccacctccatcaggtgattggcggcttcttcgttttttgttctgaccaggaggccggtgtggccctcgcgcgccagctgggtgtaggcgcgcacggtggccgcatcggtgccggcggagggcagcggatcgtcggcttccctcacggtgggggtgatctcttccaggatcgtggcagcgggaagcaggtagatctcgtcgccgctcacgccgttttcgatcagtttgtggccgatgcggttggcgtcttccgcgctcggaaacatcaccatcgaatagccagtggggtagaaagcgccgccgaagctcgcccgcatgcggggctctaggaagaatctcttcatgatgctgcctcctggatgatgcagttcttttctcacgacattaggctcgctgcgggcagagatgtgtaggcctgctccccgtatttccgcgggtcttgcgcgggaagtcccctgcgccagatgggtcttgtgtacactccctgcttcatgccgtgccatttcttccccaccaccgtctgcgcagcctcgctggcccgcctgacgtcgcctgccttcgcgcgggcgaacggggcgttggttgcacgaatgattaccaccattaccaccgcggccccctgagcacgcgcaggtggccgtttcggcagccacctggtgtatcgctctttctccgaatgaatgaacccagctctggcagctgggttttttgttttttcatccggagatttccatgtaccgcgatccagtccagtcactcgaacccctgcccagccgtcctgcggcccttcgcgcactgcgcgtgggcatgatcggcatcggcaccgtcggcgcgggcacgttccgggtgctgtcgcgcaaccaggccgacatcgcgggacgcgcgggccggccgatccaactggtaatggtggcggcacgcaacctggcacgcgccgccagcatcgtgggcggcactgttccggtgacggacgacccgctgcgcctggccacgcaccccgacgtcgacgtggtggtggaagcggctggcggcaccggcccggcgcgcgactgggtgctggccgccattgcgcacggcaagcacgtggtcacggccaacaaggccctgctggcggtgcacggcgccgagatctttgccgcagcccggcagcatggcgtggccgtggcctacgagggcgccgtggcggtgagcatccccatcgtcaaggcgctgcgcgaaggcctcacggccaaccgcatcgagtgggtggcgggcatcatcaacggcaccaccaatttcatcctgagcaagatggaggacgaaggcctggactttgccgccgcgctcgcagaggcccaggcactgggctatgccgaggccgatccggccttcgacatcgagggcatcgatgccgcgcacaagctcaccctgctggccgccaatgcgttcggcacctccgtgcggcttgccgacgtgcaggtggaaggcatcacgtcgcttcagcggatggacgtggcctgcgccgctcagctgggctttcgcatcaagctgctgggcgtggcgtaccggagggaagagggcatggagctgcgcgtgcagcccgcgctggtgcccgcgtcgcacctcatggcgcatgtgaacgggtcgatgaacggcgtcatggtcaagggcgatgcggccggcgtcaccatgtactacggtgcgggtgccgggtccgagcagaccgcttcggcggtgatcgccgatctggtggacgtggcgcggctcgacggcacccatgcggcgcagcgcgtgccgcacctcgggtttcatgcgcacgcgatgcgcgccttgccggtgctgcctcgtgccgcgacatgctcatcgcactacctgcgggtgcccgtgcatgccgccggcgacatcgaggcggtttcgggctggctcgtgcagcagcaggtgccggtacgccaggtgacgctggctgctgctgcgcagcccggctcgggcccgcaggtgctggtgctgacgcagccggtgcagcagggcacgatggacctggcgctgcacgcgctgcaggcacatccctcggtcgcggggaaagtcaccgcgctgcgggtggaggaactggcgtgaggggccttcttacgtcctgacctgggacagaatcaggcaaagcggaccctggcaccgccaacaaacgggagtcgcaatgaaattcgatcggcacggtggccctcaggaccgcaacgggagccgtgcgtgaaacgctgcctccccgtcattgcgctggccctggcaatgcccgccttcgcccaatccacgccgcctgcgcaacctgcggaaccggcggggggcacttcttgccatgcggaagaagctgcgctggagcgcgacatggacctggcgcgctccagggggcagatgctgtgtcggcggcaactcgccgagacactggccgcgcttcgcacgcgctgccagggggcggaaccgcctcagagccgtgcggcgcgcatcgacaagctggagcacgacatccggctgctcagggcagaactcgagcatgccgaggagcaactgcgcgagttgaaaaaccaacggccctgaggcccggcctcacagccgcggcaactgcatgcgcaggcgccgcgccgcttcctcttcgcgcgcatcgtccacctcgcgcagcacgttgcccaggtcgaccggcccggtgtcgcgcacgtgcgtgccggtcagaatcgattcgacgcgcagcaggccgcgctcgtacaggtgccagatctcgtcgccgtagtgcgtgccaaggagccccggcgcaaactggccaaagaagttgcgcaggttttcaacatcgcgcagcagcatgcgcctggcgtggttgttgcccgccgcatccacggcctgcggcaggtcgatgaccaccgggccgtcggccgccagcagcacgttgaactccgacaggtcaccgtgcacgacacccgcgcacagcatgcgcaccacctccttcagcaggctggcgtggtgctgcatggcttcttcgggtgtgaacgccacgtcgttcaggcgcggggccgcatcgccgttggcgtcggtcaccagctccatcagcagcacgccttccaggaagttgtagggaaccggcacgcgcaccccggccgccgcgaggcggtagagcgcatcgacctcggcgctctgccagatggcctcggtcacctggcggccgaagcgcgtgcccttggccatggcgcgcgtctcgcgcgaattgcgcacgcggcggttttccgtgtagtcgacggcctgccgaaaactgcgcttgtcggcttccttgtagaccttggcgcagcgcgtctcgtcgccgcaacgcaccacgtagaccatggcttccttgccgctcatcagctggcgtaccaccgtgtcgatcaggccttcgttgaccagcgcctgcaggcgtggtggtgctttcatgggtaccgctccgtcggttccagcggccgggtcgagaggaaggtcctcaggctctccgggccgatctggtagaccgcatcatgcctgtgcgtggccgctatcgctggttgcgccgcatcccgaacactgcgcgaagcgggcgggtgacgcgccacgagttcgagtcgtagacggcctgcatggacgttgccagctgttccgcatgaaccctcagcgtgttcagttcctcttgcagcgcgtgtgcagcctgtgctgcctgttccacctgtgcggcctgcgcggcctgcgcagcatgggacggctgcaccgcggcgtccagcgcgcggttcaatgcaagcatctccccacgcatttgcgccaccgcgttcgcgagccggcggttctcttcgcgtgcgtcttccaggtcgaggctgcgctgctgcaaggttgcggcttgcgcttcgaggctttgtgcgtacttcgtggcctcggcaatcgacatttggagctgggtgttctggtcgcgcaggctcaatgcgtattcctcggcctgggtggccttgtcggtctgcgcggcatgctcctgctgcagctggcgcacaaacggatcaggcttggaggactgctcgccgaacacgaccggaaaatgatcgcctgtcaggatgccgcgcgtgcgggcatccatgcagcacatggtgaaggcgcgccgtggcgtggatgaagggttgatgccggagcgatggatgagccagttgtgcagaagcactgcgtgtcccgcaggcacctcgagcggcacgctcagctcttcatggcagtactggcgcacatgctcttcggtcaaggtactgccgtgcatgctcagcaagcccaggcgatgcgagccccggatggcatccatgcagccgttgtcccgggtggcggggtcgagcgcaacccagatggtcgtcagcgggtcgcgatcgagttgccacaccgtgccgccgtcctggtgccatgggaggtaggtgccttggcctgcgggcttgttcatgaccatggcgcggaagatcgacaccgccgcatgggcgccgtacacgtgcgcgcaaatctcgcgaaagagcggcctgtcgatcagcgctgcgaacaggtcgtcggtttccagcccttgaatcttccggtacaggcgagtgccttcttcgaactggctcacggcctcgggcaacgcctcgtagtcgccgcccgtgtcgtactgcatctggatcgctggattcgagatctggcccagggccagagcgtcggcacgcagctgcagcgcctgtacctgttgtgcatcgagcacctgcccaaggtgcaggaacccgtcgcgcgaaaaactctgccagtctgcgtcggtcagcatctttggatcctttttgagatggagtgacgcgggctgcgcgcggcccgcagtcgcgtggcgcggcagcgcctcggtcatcggcgccgccctggtcggttcccccgaaccgaagggcgccgtcaaggcatccggttcgcgcacggcggtggccagaatgccggccagccgatcgggttgcggcgtgtccaccggcgctcgctgcatgaccagccggacgagctgacgccgacggcgctgctcgtccgcatcgttgtgcaggcccagcgcatgaattttctcgcgcgctgccgcgcggttgttccacagctcggccagcttccgcgccagctgttgcccacggatgccttcgaggctgcacgaatcgtcggcacggtcgaagtgctgcagggcaccgcacaacttggtgcgggtgtacaggtcggcccagatgccgaggcacggcacgccctgcgccagcccgaagacgatcgggtggtagcgcgaactcacgatcatttgtgcctgcccggtcagccgggccacctggcgcgccgagagaaccggcatcaggtgaagcaccgtcgaccgcatgcgccgtgccagcgcccgacccacatcctcgtcggaccagggagcgcccatggtcgcggcggccctggcatgcggaatgaacaccagccggcaacccgttcgcgcggaggtctgttccagttgatcggccaactggtcgagcaatggatcgtcgctcgtcggatcgacgaatggatggaacgtgatcccgatccacggcgtctccgcggagaagggcaggcatgcggcgggctcggtgtcggcggcttctttccagagttctgccgcatcgtcgatctggtaggacaagcgctcgggccgcgcaccgagctccagcgcgaacgtgaagctctgcgcttccctgacgccgaaccaccacgctgcgcggacgatctccgacaccagttcgcgatgccgcgcgttcagctccggtccgagggtctggcccaggacgacgatcggcgctccgttcgccaaggctcttctgcacagggccacccgctcatagatgcagttcggccaggtgcttcgcagattgccgccgccggagatcagcaggccgtccgattcgtcagccatgcgcgcgaaggcgccgggcgtttcgctggtccagtgaacgtgcgaaagctttgccagcagcgcttcgcgcgcttcgtccgatgcgcagttgtcgaagcccaggcgcggcagaccctcgacttcatacgttgccgcggtgaaggcagggtcggcggagaccacgtgcagtgtggcctccgggtcgatggtgcgcagcagccgcacgttgctttcgagcatggcctcgtcgcccacgtgatagctgtgtgcgccgccgacatcgccgatcaaggtccagcgcctcgggcgcctgcccaccacggattgcgcttcgcgcggcgctttatccggcacggtcttcctccggcgcgcgggccattgccgacgcctgcaatggcgggccggccgattccagctcttgaaggcgcagtcgcatgcgtgtgccgcagttctcggcactgaactgctgtttcagcatggcgcgcgcggtatcggcacgacgctgtgcctcgcgccggttgtggaacacctggcgcatttgccaggctgcatggttctcgtcaggttcggcccagacctggccttggtggaacggatactggttttcgggtaccggcacgagcttgaagtcgacgggccagccggtgtccgaggagaccagctcggcgcttgccgagtagtcggtcgcgatcaccggcttgccgagcgccatggcttcggcaatcagcaggcccagtccttcgctgcggtgcagggatacgaccgcgtcgcatgcagtgatcagctgcagcgtctcggtgcgggtcagcgtctgttcgatcagggtcaggtcgaggtcggtacgcaggatgtcgcgcagggcctggctgtgtgccggcgcgatgtcggcgttgagtgtcttgagcacgaggcgcacgttgggatgggcgccgccatcgcgaaatgccttcttgaatgcacgcaccagggccatggggttcttgcgttcggcataggaaagaaaatcgaagctgaagaagaacaggaatgcgtgctccggaagtccgaagcgtgcacggtccaaggccggtggggcctcgaagtccagcggcagcggcatatgcaccacgggcttgccgatcctgcgggcgagcatggtctgaatgaaacgggtcggcgcccagatttcgtccaccagatcgaaggctgccagccatggcgccgggaagtgctccagctcccagaaaggcatcgccacgcggtaggcgtccggccgcagggctgtccccaggtgcgcgatgacggccggcaactggtcggcgttgacgttgaagacctgcaccctggcggtggccgtgtcgtcgaacagcggctccagcgacttgtccacggcggcggacatggagttgaattggatcggcaggccgcgggcctcgagtccggcgtgccgcagcgtgcggagcacctggcggcccgcctcgccaacgccgagtgccaggcgcaggtagccgatgaccgccgcgtccggctccgcaccgcgccttgcgggcgggcgccggccgcggccgggcgccgcctgagcgccggcgcgcaaggcgacgggtgcgacgagccggctgtccttcaatatggttcgcgcattctggacgtaccagtcgatgtagcggcctgcgccttcactcgttgcgagatcgtagatgcctcgcagccagggctcgcgctcgtgcaggtacgacatcaggttcgtgaccccgcgggatgcggcgccggcggttcgtgcgcacggcaggtgcagatactcctcgtaggagtggaacggatcgcccccggaccagtggacatggcggtcgcggaacatccggcgcaccacctcgggcagcagcgtgcctgatgcaaagcgcccgtaggcgtaaatggcgttcgggacccggccgtggccgttcgcgagcacctgggcggcataacggcgcaagagctcgccaagcagcggcgactgctggtcatcacggaatgactcggtgtgcttggacagggtcctcgggttggacgggtcgataccgctgaaatggaaaaagcgaagcggcgcgccgtcgatcttccagtcgcccggtgccccgccgagggtgcgctgctgcaggttccagtacgccacgttgtaggcggtgtcgcgcaggatgcgggcgccttccgcgaagcccggcaccaggtccatgaatttctgatccacgaagatgccgcgatccggctcgttgacgcattcatactgcaggcgccgcgaccaccagcgaaggatccggtcggcttcctcaccagcgcccaccccgagaaagcccaggttgtagacgcccgcgcgcatgatcccgagatcgttcggaaagttgggctgctccagcggttgagtgaggtgcggcgtgagcacgaaggaggcgccttcgtcgagcagcgagaacacccgttcgagcggggcgaagacctcgatgtcagggtccaggtacaccacggactcgtgtccgcgcgcgagcagatgccgcatcatgaacggcttgatggccgtgttgaactccatgatgtcgtagcggaacgcgaactctcggaagttcgtaatgccgagcgtcttggccacaatgagctcgcattgccccggatagaaaccggcctctggcagcgcctcgtcggcaaggcacaggtaaacctcggcttccggatggtggcgttttgcgctttccagcaacaccctcgccatcggcacgtagttgttggagcagatggtgaatatcgcgcggggacggattgccatggcgtgaggtgttttcagcggccgtttggagcgacgaccattccctgatcatccatgcgggtcacgtgcgccccacaggagtggcgctgaaatctcgaaagagtttcatcaatgttacgcaaaacagacataaaccccgatatgccgtttggctacatcattcccgatgccctccggcccggcgctggtgcagcagggtggacaacatgtctcggggtcaagcaagaactgaaatgaacaagagcaagctcgccatcttcctcctcgcatgcgcgatggccgcgggcgcctcggcacaggaatggccgacgaagccggtgcgcgtgatcgttcccgcgccggcgggcagttcgctcgacctcatcgcgcgcacgctggccgaccggttgcgcaccatgtggaagcagcccatcgtcatcgagaccaagcccggcgcgggcggcctgatcggcatggacgccgtcgccaaggcgccgaacgacggctacaccctgggcatcggcttcaacgggccgatcgccttcggcccctacatgtacagccgcatgccgtatgcacccgcgcgcgacctggtgccgatcgtgctcaccacctcgcagcccaacgtgctggcggtgcaggccggcaatccggcaaacaacttgacggagttcgtggcctgggcgaagaagcagggccaccagttcagctatgcgtcggtgggggcggggagttcttcgcatctcacgatggagctatttcgcagcgtcgccggcatcgacgcggtgcacgtgccatatgcggggtcgccgcccgcggggctgtcggtggcatcgggcgacacgcaggcgctgttcaccgtggcgcccgcgctgctgcctctcgtgcagggcaagcgcatcaagctgctcgcggtcacgagcgcggggcgatccgagctcatgaaagacctgcccacggtggccgaggccggctatccgggtttcgaggcactggcgtggaacggcctgttcactgcgagcggcacgccgcccgaggtggttcgccgcatcaatgccgatgtgaacacggtgctgcaggagccggccgtgcgcgaactgctggccaaccagggcctcgtggcgggcggcgggtcggcggacgaattcaagtcgttcatcgacagcgagggccgcaagtggggcgcgatcatcgccaggcgcggcatccggttggagcagtgagcgacgagcgtctgcgcgtcatctgaaattcggatcaattgatccgaattttcgattttacggatgatggtgggctgcctaaagtcggcccccatgaatgccattgcaccgcctccattgctgatcggctgcgcggccggcttttccggcgaccgcaccgatgccgccgggccggtggtcgacacgctgatcgagcggctggccagcgggccggccgggcagcgcgctttcctgattttcgaaaccctggccgaacgcacgctcgcgctcgcccagctgcgccgccgcgacaaccccgacgccggctacgagcccttgctcgacgcgatgctgcgccccgtgctggcgcgctgcctggcgcacggcatccgcatcgtcagcaactttggcgcggccaacccgcgcgccgcagcccgccacatcgcgcgcatggcgcgcgagcttggcgcctccgcgccacgcattgcggtggtggagggcgacgatctctccggccccgagcaccgcgcgctgttgcatgaaacgctcggcgcgcagatggaggggctgcgcatcgtcagcgccaacgcctacatcggcgccgagccgattgccgccgcgctcgacgccggcgcgcagatcgtggtgtgcggccgcgtggccgatccgtcgctcaccgtcggccccgccatgtcgcacttcggctggcgagcggacgactggcaccggctgggccgcgccaccatggcgggccacttgctcgagtgcggcgcgcaggtgtgcggcggttactttgccgacccgggctacaaggaggtgccgggcctcgaagcggtgggcttccccatcgccgagatcgatgccgacgggaactgcaccatcggcaaggccgacggaaccggcggcctcgtgagcgaagccacggtcaaggagcagctgctgtacgaggtgcacgacccgagcgcctatctcacgcccgacgtggtggccgacattgccgaggccgaggtgaagcagcaaccgggcgtggcggatcgcgtggcgctctccggcgtgcgcggccacgcgcggccgagccactacaaggtcaatgtctgccatgaaggcggctggctcgccgaaggcgaaatctcctacgcggggccgcgtgccgaggcgcgtgcgcggctcgcggccgaggtgcttcgcaagcggctcgatgggctcgcgctgcgcgtggacctgatcggcgcgctgagcattttgggcgacgacgccggccgcatgctcgcggacacgcccgacacaggcctttgcgacgtgcgcctgcgcgtggcggccacgcatgcggagcgcgggcaggccgagcgcctcgcgcgcgaagtcatggcgctctacacctgcgggccggcgggcggcggcggggtgcgcaccgcactcacgccacggctcaacaccttgtcctgcctgctgccgcgagaagcggtgccggtgcgcttcgaactgctcggcgcggaggccctcgcatgaacacgaacaccacggcagacatgatcgaagtaccgctgtaccgtgccgcccatggccgcacgggcgacaagggcgaccgctccaacatcagcgtgatcgcctggcatccggatctctacccgttgctcgctgaacagctcacgccagaaagcgtgtcgatgcagttccgccaccgcgcgcccgcaagggtgcagcgcttcctgctgccccggctgcacgcgatgaacttcgtgctcgacgcggtgctcgacggcggcgtcaacgatgcgctgaacctcgatgcgcatggcaaggcgctgtcgttcctgctgctcgacatgcccatccgcgtgccgcgctcgctggcgcccctcctggccgggccgtagcggctgcctcttttttccctatccatccacccggagacaaaacaatgaaacgacgttccctgaccctctcggccgccgcgctggccctggcgccgctgctgggctacgcgcagcaggcctttccagaaaagcccattaccttcgtcgtgcccttcgcggccggcacggccaccgaccagatcgcgcgcgcgctgggcaacagcatcacggccgaaacgaagcagccggtcgtgatcgacaacaaggccggggccagcggcttcatcgcctcgcagcaggcggccaaggccgcggccgacggctacacggtgctgatcaccaccaacaccacgcatgctgccaacgagcacctgttcaagaagctgccctacgacccggtgaaagactttgcgcccatcacggcgctgggaaagggcggccagatcatggtggtgaacccgtcgttcccggccaagagcgtggccgagttcgtggcgctggccaagcaagagccgggcaagtacagcttcggcagcggcagttcgtcgagccgcatggcgggcgagctgctgcagcagatggccgacatcaagctgctgcacgtgccctacaagagcaatacgctggccgtcaccgacctcttgggcgggcagatccacatgatgatcaccgacgcggccaccggcctgccgcaggtgaagggcggcaagctgcgcgcactgggtgtttcgagcgccgcgcgttcgccgttggctcctgatgtgcccaccatttcggaagccggcgtgaagggctacgagatgggctactggttcgcggcctatgcacccgcgaagacgccgccggccgtggtcaagcggctcaacgaactgcttgtcaaggctgcgaagagcgaatccgccaagaccgctttctatgaacccaccggcaccgaggtgttcaccacctcgcctgaagaactcgccaaattccagacggccgagtcgcagaagtggggtcgcatcgtgaaggccgccggcatcgaagccgaataagcgcgctggccgtagcggagaccggcaccgcacaaatacctcaacgacggagacaaaccatgaaacgctggagcctgttggctgccacggtggcttcggccgccctttttctgagcgcttgcggtggaagcggcggcggaggcggtggcttcgtgctgccgccgccggccgcgacgacgccaccccccgccgcctccgaagcgccgaagttcaagctcgccatctccaggaccgaggacgttgccggcaccttcggcagcgtgggagcctacgagaagatcaccggcaccttcacgggcgaggtcgaccccaaagatgcgcacaacgccgtcatccaggacttgtcgctcgcgccgcgcaacgccaacggcaaggtggaatacagcgccgacttcgtgctcttcaagcccaaggacatgggcaaggccaacggcgtgctgcgctacgacgcacccaaccgcggcaacatcgtcaatctcgatccgtactttgcgtcgcgcggctacgtctttctcacggctgcgtggcagggcgacgtgccggccgcggccggcaagctcacgctccaggtgcccgtggccaggaacgcggacggcagcaccatcaccggcacctaccgcgccgagctgctgcccacggcggccaccaacgattcgctgccgctgccgggcgggccgtacaactctgcgatgcaggcctatgcaaccgcgagcctggacaacacgcagcccggctacgtgctcacgcggcgcatcaacgaaaccgatgcgcgccagctcattcccgcgagcgactggaagtttgccaagtgcagcgccgccgcgccgttccccggcacacccgacgagacgagcgtgtgcctcagggacaaatgggacccggcctacatgtacgagctggtctatgtcgcgaaggacccgaaggtcatgggcctggggctcgcggccgtgcgcgacatgatcgcctttttccatcatgacgcgagcgacgccgcaggcaccgccaacccggtggccgccgccatcaagaacaccattgcttccggcgtgtcgcagtgcggcaacttcatgaagaccttcgtccatctcggcttcaacgaggaccgcgcgggccgcaaggtgttcgacggcgtgttcgcgcagattgcggcgcggcagaccaacatcaacatgcgctttgcgattcccggcggtggcgggggcgtacgcaccgaccacacggccttcggccaggccggtacgcgcgggctgtcgaaggactacgtggacgacgtggcccagcgccgcggcggcatcctgtcgcgctgcgaggcgagcggcacctgccccaagctcttcatcggcttcagcggcacggagttcttcgtgctgcagggttcgccgctcttgacggacgcctggggcacggccgacctcgtgcagcccggcaacgcgcgcatctactactacgcgagcacgcaccatctgctgggccttccttcgctgccgggcgcgagcgccggggcgctctacgccactaacgcgaacgcgggcgtggtgccggtggtgcgcgcgctctaccagaacctcgaggagtgggtcgtcaagggcaccacgccgcccgacaaccaggtgcccaagctggccgatgccacgctggtgcggccgcagcagctcaagtttccggccattccgggcgccgcctatacgggcctggtcaacacctattcattgctcggctggggtccgaactaccggccgcaggacgagaccggcattgccacgcaagtgccaccggcctaccttggccgcgactacgccgttctcgtgccgcaggtggacgccgacggcaacgacgtcgcgggcatccgcagcctggacgtggcggtgcccgtaggcaccaacaccggttggaactacaccagcaagccgggcaccatcgacctggcgggcctcttcggctcgtactttccttttgcgaagacggcggccgatcgttcgggcagcggcgatccacggctctcgctcgaggagcgctacaccaaccaggctggctacgtcgcggccgtgaccgccgccgccaacgacctggtctccaggcgctttctgctgcaggtggatgccgatgcggccatcgcgaaagcagtggcgaatccggtgctgccttagcgcgtgttcttgtccgatgcggtggtgtgcaccgcaaagccttcctcacccggtgcaatgtcgtcgcgcaaggtgagggcgggaatctcgtagtcgccgaagttctgcggccggaacgggatcgggtcggtggtccacagcgtgtcgagccggcggcccaggtcgtcggtgatgcgcccgtaagcggcggcatcgaccttgtcggtgcggtacacgacgaaaggcggcagcacctcgaagcccgggtagtagaggatgccgtggtgaatgggaaacagcaggtcgtccatcggcccgttgatgccgcgggccccgtagtgcgaggcccagccgccggtcgtgaccaccagcatggcgcgcttgccggccatcacgccctggccgaagcggtcgccccagtgcctgtcggaatgctcgcccacgccgtagccaaagccataggcgtagacacggtcgacccagcccttgaggatggccggcatcgtgtaccaccagagcggaaactggaagatcacagtgtcggcccacagcagcttggcctgctcggcggcgacttcttcgcgctgggtgccggactcgaaggcgcgcagcgaatccgcgacgggatcgaagtgagcaccgggctcgaggtgcgcaaagtcgtcggcggccagtgtcgccttccattgcatggcgtagaggtcggacacgcgcacttcgtgccccgactgcacgaggcgttcgaccatgaactgcttcaacgatccgttgagcgagcgggcttcggggtgggcatgaacaagaaggattttcatggcggcatggttcgtcggatgaagaagcacgcaggttaggcgccgtgaggctatattggaaatgaatattcagaattccaggaatagccatggacaatttcatgcggctcgatctcaacctgctgctcacgctcgacgtgctcctggccgagcgcagcgtgacgcgcgcggcgcagcgcctgaatctgtcgcagccttcggtcagcgtgcagctcgccaagctgcgcgaggtgttcaacgatccgctgctggtgcctgcgcagcgcggcatgctccccaccgcgcgcgccgaagagctgcgcgagccgctgcgcgaagcgctggagtcattgggccgcgcggtggcgcccacgagatctttcgacccggcagaggcgaccaccacctggcgcgtggcggcggccgactatgccgagtcggcgatcctgctgcccgcgctcgccgggctgcgcgcggccgcgccgaacacccggctcgccgtggtggaggcggtgccctcgcgcatggcgcggcagctagagcagggcgagatcgatcttttctttcataccagcgtgggcgcgccgcccgggctgcaccggcgcgtgctgttccatgagcgctacgtgctggccgggcgggccggccatccacgccttaagcgccggcccacgctcgcgcagttctgcgcgctggagcatgtggtggtgtcgcccggcggtggcgggttcgtcgggccgaccgacgacgcgttggccgagaagggcctggcgcggcgcgtggcgctgtcggtgccgcattttcttttcatgatgtcggtgctggccggcaccgacatggtcgcgatgctgcccgagcggctggcgcgcggcgcgcccgggctgcgcgtggtggaggcgccgctcgaagtgccgggctatgaaatggcgatgctgtggcacgagcggcggcaccgcgactcggcgcaccgttggctgcgggagcggattgccgcaagcgtgtagtcgtcgcctacggaaccgtcggcgatccggacggctacttgccccgagcgtcgaagacgctcttcaacagcggcaccgtcgagaagacattgggccacgcggcgtggcaggcaaggcgcgagacgatctccggcactgttgcttgcggcgggccgttgtcgtccgccgccccgccaaggtgataggaaatccggggaaaccggccgccgatcaccttcttgaagtagcccgcatcgcgcgggacatcggactcggccaccagctcgagtttctcaaccgggcgcggcgagaaggccggctcaagatgcgggacgagtctttcgggaagcggtcctgagaaccccggtcgggcgagatgccagcgccggctgtgctgcccctgcttggcgaacacatgcgcgaggtgcttcttgaccgtgttgacgctgatgccgagctgctcggcaatctgcttgttcgacatatcccggttcatcagcgacagcacctcgtcctcccgcgcagtgaggccgactgcaggcagtgccgcaccggaccccggacgcccgccggccaccgccagccgcagcaaggacagatacagcgcctgcaataccgggcccggaaaagccagggtgcctgccagcacggcatccagcgatcgtgcgaattgctctgcgctcgctccccactccacacagccgtgcgcctggatccggatggccgcctccagcccctgtgtcgagggctgctcccagccgaggagccagtcgatggtgggaaagtggcggcgcagatcgtccagtttgccgacgccttcctgcgaaagcagcgcgatgtccaccaccatcaaacgaggcacctgctgccggcagcggacttccaggtcggaggtgctgctcatttccgtgtgctcgacccggtacgtccgctcggcccggtgcctcgaggccaacaggctcagtccgcacagcgtcgatgagcggcttggacaggttgcgatcaggaccgaaacaccggtttcgaatgccgggtggcgctcaggaggcgggatctcgagcaagtcgggttgaaaacagctcgacgcgcgcaacgccgggagcgcgaatggcgacggcgggtgagagccttgcattgacggctgccgatctgcgttccacgcagattccagccccgcaaacgagcgtgggacctgtttcatgtttccccccgggcgcttgttgagtgcaccgagaaagtaatgataaaggttacacaatcgttcgtatcgattcgtggcccctgcaaggtatcgagatgtgttgcgactcaaaggcgtgaatcagcgggcgcggcgcgtcatcctttgggtgacaactttcgacctatggacagtgcgcggggccgcggttcagcatcgtctcccctttgctgataagtgaacctggtcaattgccagcgaacgcagctcgttcggagttgcgctgttctccgtcggcgtttttttaaccaactcgaggagcgtttatgcctgcgttcacttttacacctggctcgaccgtcactctggacgaatccgacggtttgcagaacgctgtcgctacccccgcacctgcggaagacggtaacgacaatgacatcctcgtaacttcgctgccggccaccttcaccacccgcctgactgccgcgggtgcgccagccccaaccaaagccgccttgagtggctatacggggagtggcaccggcgccaacgcattcacgttcagcgggaccggcgctttcaccggtatgtcattcacggacgcggccggcgctccgctcaatggcttggacagcggcctcaataccgcggatggcgacgacatcttcctttacaccgacacgaccaacaacaacgtcgtcttggggaagaccggcgccggtgtcgtcgtgttcgcggcctatctggaggagacaggaaccccggtgacgggcgcaaagatctggatggtccagtatgaagcgatatcgaaccccgatgcgaccaaccccgacgatgcagtcgacctgactgagaaggtctacgtcagtgtcagccaggatgcggagttcaatctcgcagacgcgccatctggccagaacctgttcctgatgttcacgaagaccaatccgacgatcgacgctgacggccggattaccgacgtgtcgatcatcgcgacgggaaaggacccggcaaatcagtccggggccaatcccgacatcaccgacgatgacatcaacattggcaccggcgacacgatcaactccagcaaggccggcgggccgaccacgttcggtaccaacaaccagatgatcacagagcaggagggcatccgcttcacgttcgtgaccggcgccagggcggacgtcaccattccggaactggaaccgggcgaggcccatctggagtcgaacatcgacttcaccggcatgttcggggcgaggactgccgatttcgacgttgtgcagttgcaaagcggaaagagtgcccaggtcagggtcaccgcatacagcacggcggttgagtctggcaacagcttcgtcgacggctatgcgggcgacgcgacggttccgatcacgagcgtgcgcgtgctcgactccgtcaccaacgcggttctcgaaaccttctcgaacggcagcgagggcggagtgagtccgaccatcgccatcagcatcaccggtggcgtcgcgctgatcaccggcgtcaaggccgactactcgatcgaatacacgacgtcagcggaccacaaccgcgtactcgttgaaaacggggcggccctcaatgcctcgggcaacacccacgccgacttcgacgtcgggggcttccggctgctgcaggtttccgccgcaacgtcagaggtcggctcgatgatgaacttcgaggacgacggcccgtccgtcgtgctggcgacgcccaccgacaccgcggtggtcaacacgcaggacgccgacaccatcggcgaagccaccgactccgccaccacgaacttcgcgaccgccttcaccacgagttcgagcagctacggcgccgatggggcgggctccaccggctcggtcttcgctctcggtgtgaaaacgcagggtggcgactcaggcctcaagagcgataccgcgaccatctacctgtatttggtgagcggcaaggtcatcggttcgacgtccaacacggaagccggcattcttgcgggcaacaccattttcgacctggccgtgagcgcaagcggctccgtgacgctgcagcagtttgccgaaatcgaccacgcgctgccgggggcttcgtcgaactacgcggcccaggaggcctcgatggccgacgacctggtcacgctgtccgatacggtgacgctcaccgaccaggatggcgataccgcgagcgactccgaggtgctcaacatcggcgccaacatcaggttcgacgacgacggcccgtccatcgtgctggcaacacctaccgactcggcgctgctcactacgcaggatgccgactccgccggagtcgattccgccacgcaggacttctcgaccgccttcggcgcgacctccagcagccacggcgccgatggagcgggctccaccgcttcgaccttcgcactcggcctgtccacgccgggcgaagcttcagggctcacgagcgatggcgcggtcatcaggttgtacctggtgggcgggaatgtcatcggatcgacggcggccaccgtgggcgccatcacggcgggcaacaccatcttcgacctggccgtgagcgcaagcggctcagtgacgctgcagcagtttgccgaaatcgatcacgcgctgccgggcgtggggtccaactacgcggcccagcaggccacgatgctcgacaccttgatcaccctcaccaatacagtgacgctcaccgatggggatggcgacaccgcgaccgataccgaggtgctcaacatcggcgccaacatcaagttcgacgatcacggcccgacggtgactgccatctcggacctcaccggcgcgaatgacgcccagtccattgcgggaacttataacttcgccgtcggcgccgatgacgtgggcaacgcgtcgaccgacggcatcgtgctgaacagcctgaccggaacgaccggcggcggccggcccatcaccgatgcggccgtcgcgcactttgcggaagatgccaccacggtcacctacaacttcagcttcaactacttccccgggccaacctcgaccacgacgcaggcggcaacaggcacggtcatcttcaacaagacggacggtaccttcacctttgatctggaccaggtcttcagtggacaatcgacgttctccacgagttcgccgctggcctccttcaactacgacacggaaggcaacaactcgccggagatcgtggtccagcagtacagcagcgacttcttcggcgtgctgtccgccagggccgccacgcctccaagcgattccagcgacctggtgtcgggcagcgatcatgcgttcacggcgggggaaaccttcaacagcgtgagtgccggttttgtcaatgtcgcgaccaacacccttggcgtgaactccgacaccgtccagaacggcgagttgctgaacttcgacttcttcaggtcgaatccggtgaacaaccccagtgtgacaagcccgccgccgcggcccgacgcaacggtcgtcggtacggacagggcctacgccgacgcgatcaacatcacgatcgatcagatcacggacggcgaagacgtggctgtcctgctgaagttggtcaatacgtcgaccaatgccaccacgacccggctgttgatcgccaactccgcgacggactatcaatcggccggaggcggcatgaagatcgtcagcatcggagaggacgactacgacagcgccaacttccagatctcgggcgtacaggtcctgagcagcaccgaagacctcaccggcacgggcatcagcctgagcacccacaacgcggtgaacctgacggcgactggaaataactatgccgatacggaggacaacgatgtattcaagatcatcaagatcgacgtgatcacatcggcgaccatcaactcggacgtggacctgaactttgcaggccagctgatcgacggcgatgccgactttgcgaacttcgacttcgatgtccacctggagatcgatggcgtggccaacctgatcggcacaaccaaccagacggagcctatcgcgtaacgagctcttgacaagggggcggcaggaatgctgccccttgccgctttggcctgtgccaaggcgtactgaattccaaatctgcgaggtggcatgaaacctcaggaaaagtcaggcgaattgcggcaggcggtgacagccctcaacgcctacttcgtgcgggcggcgtggttcagtgtgtgctcgggtcttctgctgctggctccgagcgcgtacatgctggaggtgtatgggcgggtcgtgaacagccgcagcacgctcacgctggccatgctgacactgctggtgctggccgctttctgcctgatggaagtgctcgactgggcccgcaccgaggtgatgtaccgggccgggcagaagctcgaccagaagctgcggaaccgcgtcttcgtcgccatcttcgaagccggcctcaagcgcttgccgggcgggaccgtgcaaccgctcaacgaccttcgcaccttgcgcgagttcctgtattcaccaccgttgctggcgctgatggaagcgccggttgcgctggtcttcatggggctcatgttcgccatcagccccgtgctgggctggtcggccgtggtgggctcgctgctgcaggtgttcgtcggctggctcaacgaccggaacacgcggccgccgctggtgtcggccaatcgatgcgcgatcgaggcgcagcagtatgcggacgccgcgctccgaaactcgcaggtcatcgagtcgatgggcatgctgcgggacgtgcatcgccgctggatgggcaagcggcgcgattttctgcagcgcgaggccgtggcctcggaccacgccgggacctaccaggcgctcggcaagttcttgcaggtcaccatgggttccctgttgctgggcctgggtgcctggctgctgctgaagaaccagctcaacggcgacgccggaatgatggtggtcggctccatcctcggcggccgggccttggtgccgctggtgcagatcgtgacgcagtggcgcacggtggtgaatgcgtgcgatgcatggcagcgcctgggcggcctgctgagcgccattgcgccgccgccggacacgatggctctgccgccgcccaagggcgcgctgcaggtcgaaaaccttgtggcagccgctccgggcagtggttcggccatcctgaagaacgtggccttcagcctgtcgcccggcgaggtgcttgccgtggtggggccctctgccgcgggcaagacgaccctggcgcgcctgatcgtcggactttggccggcggcaagcggcaaggtgcggctggacggcgcggacgtgttcgggtgggacaaggccgagctcggcccgcacatcggttatctgccgcaggaagtggaattgctcgaaggcaccatcgccgaaaacattgcacgcttcgctgaggtgcggccttcgaaggtcaaggaggccgcgctggccgtcgacctgcatgcctacatcaccagccttccgctgggctacgacaccccgatcgggaccgaaggcacggtgctgtcgggcgggcagcggcagcgggtcgcattggcgcgcgcgatctatggcgagcccgcgctggtggtgctcgatgaaccgaattcgagcctggacgaggccggtgatgccgcattgacggccgccattttgaaactcaaggcgcgcggcaccacgttcgtcgtcatgacacaccgcaccagcgtgctggccgtggccgacaagatgctggtgctgtgcgatggcgcgatgcaggggttcggcccacgcgacgaagttctggccgcgctgcggcaagccggcgagcaggcggtggaccggatacgcaaggccgccaaccagcctgtgtcgatacggcgcaatgccgagaacgccgcgagcgtcacgccagaggcgagcccacagccatgaacaaaccctcgttcttcaaccgcagcgaactggcgcgcgccctttgggggttccgaagggagttcctgctggtcggctcgctgagcttcctggccaatgtgctcatgctcgcgccgacgctgtacatgctgcagatattcgaccgcgtgctgtccagccaaagcgaactgacgctgctcgcggtgtccctgatcacgctgctcctgttcgtggcgctggccttgtcggaatggctgcgctcgcgcctcttggtgcgggccagcctgcgcttcgaccggcaactgagcacccgggtgttcaacgggagcttccaggcctatctcggccagccgtcgtccaacaagtccaggccgttcgcagacctcaatcacatccgccagttcctcaccggtccaggcgtctttgcgctcttcgatgcgccttggacgccgatctacatcgcggtgatcttctttcttcacccctggctcggaatcgtggcgctggggttcgcgctggtccaggccgcactggcgtggttcggccagcggcagaccgccgcgccggcggaagaggccctgaaagccacgggcgagacgatcggcgacctccagggcaagcttcggaacgtggaggtgctcgaatcgatgggcatgatcgccaacctgcaaaagcgctggaatcgccagcatgcggcctccatggagaagggcgccttggcgcagggcttcatcaatcgcgtggccggctggagcaagttcatacgctacagccaacagtcgctcgcattgggggcaggtgcgctgctggtgatcgatggccagttgtcgccaggcgccatgattgcggcgaacgtgctcatggtccgtgccctggcgcccatcgaccagctggtcggcacgtggcgcggctttgtctcctgccgcagtgcattccagcgtcttgaaagactgttggacgaatttccggagcaggaccatgtcccttcccgggacgggcccaccggcaccatcggcttgcaaggcgtctttgcaggggccgcggggcgcccggcgcccatcctgaagaatatttcgtttgcggttcccgcaggaaccgtggtcgcggtgctgggcccctcgggctcgggcaagtcgacgctggcgaaggtcatggtgggcatctggagcccgtcttctggcgcggtgctgctcgacggggtgccgatcggaggctggaatcgtccggagctggggccgcatatcggctatctgccgcaggacgtggagttgttcggcggctccatagccgagaacattgcgcggctcggcgagatcgactcgcgcaaggtcatcgaggccgccagcagtgccggcatgcacgagacgatcctgcgttttccgaaaggctacgacaccctcatcggggacgcaggcaacctgctttccggcgggcaaaggcagcgcatcggactggcgcgtgcgatctatggcgacccttcgctcattgtcctggatgagccgaatgccaacctggacgatgccggcgaggccgcgctggtgcgcgccatacgggaactgaaggccaagggaaaaacggtgttcctcataacgcaccgccaaggcgtggttgccgtggccgaccgcctcatggtcttgagcgatggcgaattgaccgcggacggtccacgcgatgccgtgctcgcgtctttccgtcgcccgcagcctgctgccgtgcgaacggcggccctggtgcagtcggcttgacccgacgcccgtcctgtcatcgatccatctccgggagcttcaaatggccaaaccgaatcttctcagggacgtcactacttcaaacccctcgccggtcgtcgacgacgacacgtcgcaggatgatgcaaatggcctcagaagcgagttcggccgcgcaggccgcatcggcgcgtgggcgctggctgccggattcggcgggtttctgctgtgggctgcgttcgctccgctggacgagggcgtgccgagccaggggcaggtggccatcgacaccaagcgcaaggcggtccagcatcagattggcggcatcctcaaggaggtgcgggtcggcgagggcgatcaggtccaggaggggcagttgctgttcaagctcgacgacgccgcggccagggcgagcttcgaaaccgtgcggcagcgctatctgggctttcgcgccatacaggggcgcttgctggcggaacaggggggacagaacgccatcgagttccatcccgacttgcaggcggccgccgcggacccgctgatccggcaacagatgttcaaccaggaacaactgctcaggtcgcgccgcgccgcgttgcgggccgacctgcaatcaatcgaagagaacatccagggtcagcaagagttgtctcaagcgtacgcaagcatgttgggcagccgccgaacccagctttctcttctcaacgaagaactggcgcagacgcgcaagatggtcgccgaagggtatgccccgcgcaatcgccagctggagatggaacgccaggttgcggaatcgaataccttcattgccgagctcatcggcaacatgggccgggcccggcgaacggtctcggagcttcgccagcgtgccattgccaggcagcaggagtaccacaaggaggtggaaacccagcaggccgaagtcagccgcgaagtgcttggcgactacgagaagttcgtcgccttgcgcgatgaactgggccgaaccgagatccgctcgcccgcttcgggccaggtggtggcgctggtggcgcaaaccgttggcggcgtgattgcgccggggcaaaaactgatggacgtggttcctgtcaacgagcccttgctgctcgagacccgagtgccgcctcatctgatcgaccgcatccgcgccggcataccggtggacgtgcgcttctcgagctttgcccactctccgcagctcgtggtgcagggcaagctggtttcggtctccggcgacttgctgaccgacccgcagaccaacaccagctactaccttgcgcgggtcgccgtgacgcaggagggccttcagaagctcggcaagcgttcgctgcagccgggcatgccggtcgaagtggtcttcaagacaggggagcgctcgctgctcgtctacctcttgcatccgctcaccaagcgcatcgcagcctcgatgacggaagaatgagcgtgaagaagaaaaccctgttggcattcgctgctgccggccttctctcggggcaggcctggtcgctcgatctgtcgcaggcctatgcggaagcgctggagcaagactcgaccatccgcgcggtgcgggcggccaccgatgcccggcgcgaacgcctgccgcaggcccgcgcgcaactgcttcccaacctgtcggcgagcgtctcgcgctatcgaaactggctggagagaacttcgccggatgcctccgggcagctcgtcacggccaacctgcgctacaccagcagcaccgaggcgctgaccttgcggcaacccatcttccgcatgtaccagatggccgactaccgccaggcgaaggcgcaggtcgaagatgccgaagcgaatctcgaacgcgaattgcagagtcttggagttcgggtgagcggcgcgtacttcgaggcactgctggccgaggaacacctcacgctggtgctcgcccagaagacggcctatacgacccagttcgatgccgcgcagaagcgactcggcgccggttttggcacccgcaccgacatcgacgaagcgcgtgcggccctggacctcaacgtagcgcaggaactcgaggcgcgccagaaccaggacttcacacgcaggcaactccaaggcctggtcaatcgcccgatcgaccgattggcgccgctcgactcgtccaggatgcagctcgtgcggccggcgcccgatcggctggaagactgggtcgaacgggccgagacgaacagccccgagcttcagtcgctggtcgcgcaggtggaagcagccaagcatgagctggagaaggcgcaagccggccactacccgaccttggacgcggtcgcccagtggtcgcgcaacgacagcgacacgatcaacaacatcaagacccgctacaacaacaagtccatcggcttgcagctcaacattcctctctattcgggcggccatgtgagttcgaccgtgaggcaggcaatcgcgggccagcatcgggcggaagaggccctcgaggccatgcgccgcgacctgggtgtgcggctgcatcgtgagttccgcggcgtgacggaaggcgtcttgcgggttcgggccctcgaacaggcggtgcgttccgcggagcaggtggtcatctcgaacagccgctcgttcgaggctggcagccgcaccttgcccgacgtgctgaacgcggagcagcagaaggtgtcggcccagcgtgacctggcccaggcccgcttcgtctacctgatgtcgcgggtacgcttgcaggcgctctcgggcggcgccaaggtcgaagtcatcgacgagatcaacggctggctcgtgcgctgacggatgcggcggcatggccccgtcaaatgacgggcgcgctggtctccttcagcacgcgcagcacgaagtgcgacttgctgtggcggatgcccggaatcttgtagagcttttcgcgcagcagccgctcgtagtcgcgcgtgtcgcgcaccgcgatgcggatgtagtagtcgtagtcgcccgacacgagatacgcctcctggatctccggaatggtcgcaagcacgcggccgaagtcgtacagcgtttcgtcggtgtggctttcgagcgtgacctgcacgatgaccgaatcgtgatagccgagcttggccggatcgacgtcgatggtgtagcgcttgatcacgccctgggcttcgagcttcttgatgcgcgtccagcaactggtgggcgacaggccgacctcgttgccgatctcctgcagggtcttgcgcgagtcgagcagcagcacccgcaggatcgccatgtcgatcttgtcgaaagatccttcttcatttgctggaatttttcgaagagttttcatgaaataggccgagagagccaaaagaaagaagcaaattctgcatcaaaaccggaagaatcgacggcatgcgactgctcgaccttcctcccctccttcccgcttcttccccatccccccagccgggagtcgccgcggctgcggcccgtccccgcaacggggccgaggccctgctcgacacgctggtcgaatgcggcgtcgacactctttttggctacccgggcggtgccgcgctgccgctttatgacgcgctccacggcgagccgcggctgcgccatgtgctggtccggcacgagcaggccgcggtgcatgccgccgaaggctatgcgcgcaccacggggcgcgtgggcgtggtgctcgtcacgtcggggccgggcgtgggcaacaccatcagcgggctgctcgacgcgatcagcgattcggtgccgctcttgtgcatcagcgggcaggtcgcgaccggggtgatcggcacacaggccttccaggagagcgacgcgctcggcatgtctcgcccggtgaccaagtggaaccagcaggtgcgcgcggccgacgacatgccgcagctggtgcgccgcgcgctggagattgccgcctcggggcggccggggccggtgctgctcgacgtgcccaaggatgtccagctcatgcgcctgggccatggtgccgcggccaagccgctgcgcgcgctgcgcacgggcagggccgcgctgccgccgcgggccatgctgcagcgcgcggccgatctgatatcgacggcgcgccggccggtgctctacggtggcggcgggctgatcaactcggggccggccgcgtgcgaggccttcgcgcagctggtgcaccgcctgcatgcgccgtgcacgctcacgctgatggggctcggcgcctttcctgcgtcggacccgaagttcatcggcatgctgggcatgcacggcatgctcgaagccaacctggccatgcacgaggccgacctggtggtgtgcgtcggcgcgcgcttcgacgaccgcgtgaccggcaagctcgacgagttctgcccgcatgcgcgcaagatccacatcgacatcgatccgggcagcatcaacaaggtggtgaaggtcgacgtgccgatggtcggcgactgcggcgccatcgtccaaggcttgctcgcgctgctgcccgcggatgcgttggcgcccgaacggcttgcgccctggtggcagcgcatcgaacgctggcgcgcggaagattgcctcggcttcacgccgcgcgctgatgccatcctgccgcagcagctgatgtcgtcgctgcagcgcgccattgccgggcgcgacgccatcgtgtcgaccgacgtgggccagcaccagatgtgggccgcgcaatacctgcgcttcgatcggccgcggcgctggctcacttcgggcggtgccggcaccatgggctacggattgccggccgccattggcgcgcaggttgcgcaccccggcgcgctcacggtgtgcgtgagcggcgacgcctcggtgctcatgaacatccaggagctctcgacggccgtgcagcaccgcacgccggtgaagctggtgctgtgcaacaacggctacatgggcatggtgcgccagtggcaggagctcaaccacggcaaccggctgagccacagctggaacgaggcgctgcccgatttcgtggcgctggccaaggccttcggctggggtgcgcggcgcgtttgtgatccggctgagctggaggcggcgcttgccgaatgccttgccagcgaggggccgttcttcctcgacgtgcaggttgcagcgcaggagaactgctttccgatgatgccggcagggtgtgggcaccaccgggtgatgctttcgaaggaccggtggtacgaagaagagccttgagggtttgactttctcccggtttgactccctctccctctgggagagggcaggggtgagggcatgtgcctgtgagaaggcgcggccgtttcattgaggccgatgccctcatcccaacccctctcccagagggagagggggcaagagcggaacgctcaggacttgatgaacgccagcaggtcggcgttgaacttgtccttgtgcgtgtcggtcaggccgtgcggggcgcccggatagacgatgagcttgttgttcttcaccagcttggccgaggccaggcccgaggcgccgatcggcacgatctggtcgtcgtcgccgtggacgatgagcgtcggcacgtcgaacttcttcaggtcttcggtgaagtcggtttccgagaacgccttgatcgagtcataggtgttcttgtggccggccatcatgccctgcgcccaccacgcgtcgatcagcccttgcgagaccttggcgcccgggcggttgaagccgaagaacggacccgtgggcaagtccttgtagaactgcgaacggttggccagctgcgccgcgcgcaggccgtcgaacacctccattggcaggccaccggggttggcggcggtcttcagcatttgcggcggcacggccgagatcagcgcggccttggccacgcgcttggtgccgtggcggccgatgtagcgcgccacctcgccgccgccggtcgagaagcccaccaggatggcgttcttcaggtccagcgtttcgatcaccgtggccaggtcgtcggcgtaggtgttcatgtcgttgccgttccagggctggctggagcggccgtggccgcggcggtcgtgcgccacggcgcgatagccctgcgaggcaaggaacagcatctgcgattcccagctgtcggaattgagcggccagccgtggctgaacacgacgggttggccggtgctggggccccagtccttgaagtagagctgggtgccgtctttggtgacgatggtgttgctcatgacttgctttccttttgaagatgcaggaaccgcaccggctttcggcgcggcggttgaagcggcggatgccgctttggagaagccggtcgccacgagggccccggctgcaacggaaacgccgccggccagcaggctgcggcgggtcggggtggcggtgaaattcttgctgttcgtggacatggtgcgttccttttttgacgtcgtggttaatgcaggttaaaactatcgttcgtattaatatcgcgtgcgatataaatgagaaagaaaagcaggaaggcggatgcggcgtgccatcacgcgttcctgtcgaggttggaacgcagcgttttcaactgcgtacgcagcttgacgatgtccttgggcggcagctccatggccgcggcgaggcatgacggaagcgccttggccttgccgcgaagtgcacggccttcggcggtgagcgacacgatcacctgccgttcgtccgttgccgaccgcacgcgctggatgaggccgcgcgcttcgagtcgcttgaggaggggcgtgagggtggtcgtttcgagcgcgagccgtgcgcagatctcggatacgttgacgccgtcctgctcccacagcacgagcatgacaaggtattgcaggtacgtcaggtccaggtcgcgcagcaggccgcggtacaccttgttgaggctcagcatcgtcgaatagagcgcgaagcagagctgctcgtccagcgccagcgagtcgcctgggggggcgtcggcggcttgggtggaggggtgcttggcaggcatgggccgaatgatatatcgcatgcgatctaattgcaagcgataggccggcggatgccttcaatgagtagctcctgcatttgtgcgcctgaggcccaggccaaaaaaaagggcagcattgctgctgccccccttgccgaagagctcgctacgcgatggcctccgtttgctgggtggtgccgatcaggttggccacgccatcgatctccaggtggacatcgaagtcgaagttcgcaaagtcggcatcgccgtcgatcaactggcctgcaaagttcaggtccacgtccgagttgatggtcgtttctgtgaccacatcgatctttatgatcttgaacacatcgttgtccgacgtatcggcatagttatttccagccgcggtcaggttcaccgcgttgtgggtactcaggctcacgcccgtgccggtgaggtcttcggtgctgctcaggatctgcacgcccgcgatctggaagttggcgctgtcgtagtcgtcctctccgatgctgacgatcttcgtgcctcctgcggccgattgatagtccgtcgcggagttggcgatcaacagccgggtcgtggtggtgttggtcgatgcattgaacaacttcagaaggatcgccacgtcttcgccgtccgtgatctgatcgatcgtgatgttaatcgcgtcggcgtaggccttgtccgtaccgacaatggcagcgctgggccgttggggcggactcgtgaggttggggttgctcactggattcgacctgtagaagtcgaagttcagcagctcgccagcctgcacggtgtcggagttcacgccgagggtgtcggttgcgacgttgacaaagcccgcacttgcgctgttgaaggtttcgccggcaacaaacgcgtgattcccgcccgccaccaggtcgctggagtcactcggcggcgtggcagccctggcggacagcacgccgaagaagtcgctgctgtactgctggaccacgatctccggcgagttgttgccttccgtgtcgtagttgaaggaagccagcggcgaactcgtggagaacgtcgtttgtccaccgatgagctgattcagatcgaaggtgaaagtaccgtccgtcttgttgaagacgaccgtgcctgttgccgcctgcgtcgtcgtcgaggttggccccgggtagtagttgaagctgaagttgtaggtgaccgtggtggcatcttcggcaaagtgagtgacggcagcatcggtgatgggccggccgccgccggtcgttccggtcaggctgttcagcacgatgccgtcggtcgacgcgttgtccacatcgtcggcgcccacgaagaagttgtaggttcccgcaatgggcaggccgtcgttcgctccggtgagatcggagatggcggtcaccgtcgggccgtcgtcgtcgaaccggatgttggcgccgatgttgagcaccttcgaatcgctggcggtgtcgccatccccatcggtgaccgttacggaattggtcaaggtgatcagcgtgtcggccagagtggcttcctggtccgcgtagttcgaccccacacctggcagcgcgtgatcaatctcggcgaactgctgcagcgtgaccgagccagccgcgctgactgcgacgtcgaagatggtgttgcccgccgtgatgccagcctcagtggccgaagtcgacccgatgaccttgccggccaccaggtacagccggatggtggcgccatcgctcttgagcccggaatcgccaccctgcgtggccacgccgagcgcgaagctcgagacggtggtgcccggcccgtcggcgccgtagctgctcgacgccacgctgaaggcggtcgagaagtcctcggtgtccgagtcggtggccgcgccgatggtgtcggcgtcctgcgtgttgagcaccgccgtgtcgatgggcgctgccagcacgacggacggaccgtcgtcatcgaaccggatgttggcaccgatgttgagcacctcggaatcggtggccgtatcgccgtccccatcagtaaccgtcaccgtgttggtcagggtgatcaaggtgtcggccagcgaggcctcctgggccgcgtagttggacgagtcacccggcagtgcgtgatcgatctcggcgaactgctgcagcgtcaccgagccggtggcactgaccgcgacgtcgaagatggtgttgcctgccgtgatgccggcttcggtggccgaagtcgacccgatgaccgttccagccaccacgtacaggtaaatggtggcgccgtcgctcttgagcccggagtcaccgccctgcgtggccacgccgagcgcgaagctcgatgtggtggtgcccggcccgtcggcgccgtagctggtcgacgccacgctgaaggcggtcgcgaagttcgtggtggcggagtcggtattggcgccgatggtgtcggcgtcctgcgtgttgagcaccgccgtgtcgatgggcgcagccagcacgacggacggaccgtcgtcgtcgaacttgatgttggcaccgatgttgagcacctcggaatcagtggccgtatcgccgtccccgtcggtgaccgtcacggtattggtcagggtgatcaaggtgtcggccagcgaggcctcctgggccgcgtagttggacgagtcacccggcagtgcgtgatcgatctcggcgaactgctgcagcgtcaccgaaccggtggcgctgaccgcgacgtcgaagatggtgttgcctgccgtgatgccggcttcggtggccgaagtcgacccgatgaccgttccggccaccaggtaaaggtagatggtcgcgccatcgctcttgagccccgagtcgccgccttgcgtggccacgccgagtgcgaagctcgacgtggtggtgcccggcccgtcggcgccgtagctgctcgacgccacgctgaaggcggtcgagaagtcctgcgtgtcggagtcggtggctgcgccgatggtgtcagcgtcctgcgtgttgagcaccgccgtgtcgatgggcgctgccagcacgacggacggaccgtcgtcgtcgaacttgatgttggcaccgatgttgagcacctcggagtcggtcgccgtgtcgccatcgccatcggtgaccgtcaccgtgttggtgagcgtgatcagcgtgtcggccagcgaggcctcctgggccgcgtagttggacgaatcacctggcagcgcgtgatcgatctcggcgaactgctgcagcgtcaccgtaccggtggcactgaccgcgacgtcgaagatggtgttgcccgctgtgatggcacccacggtggcggccgtcgatccaacgaccttgccgctcacgaggtacaggtagatggtggcgccatcgctcttgagccccgagtcgccaccctgcgtggccacgccgagcgcgaagctcgagacggtggtgcccggcccgtcggcgccgtagctgctcgacgccacgctgaaggcggtcgagaagtcctgcgtgtcggagtcggtggccgcgccaatggtgtcggcatcctgcgtgttgagcagcaccgtgtcggtaggcgctgccagcacgacggacggaccgtcgtcatcgaagcggatgttggcgccgatgttgagcacctcggaatcggtggccgtatcgccgtccccatcagtaaccgtcacggtattggtcagggtgatcaaggtgtcggccagcgtggcctcctggtccgcatagttggacgaatcacccggcagcgcgtgatcgatctcggcgaactgctgcagcgtcaccgaaccggtggcactgaccgtcacgtcgaagatggtgttgcccgccgtgatgccggcctcggtggccgaagtcgacccgatgaccgttccagccaccacgtacaggtagatggtcgcgccgtcgctcttgagcccggaatccccgccctgcgtggccacgccgagcgcgaagctcgatgtggtggtgcccggcccgtcggcgccgtagctggtcgacgccacgccaaaggccgtcgcaaagctctgcgtgtcggagtcggtggccgcgccgatggtgtcggcatcctgcgtgttgagcagcaccgtgtcggtaggcgctgccagcacgacggacggaccgtcgtcgtcgaaccggatgttggcaccgatgttgagcacctcggaatcagtggccgtatcgccgtccccgtcggtgaccgtcacggtattggtcagggtgatcaaggtgtcggccagcgaggcttcctgggccgcgtagttggacgaatcacccggcagtgcgtgatcgatctcggcgaactgctgcagcgtcaccgaaccggtggcgctgaccgagacgtcgaagatggtgttgcccgccgtgatgccggcctcggtggccgacgtcgacccgatgaccgttccagccaccacgtacaggtagatggtcgcgccgtcgctcttgagcccggaatccccgccctgcgtggccacgccgagcgcgaagctcgatgtggtggtgcccggcccgtcggcgccgtagctggtcgacgccacgccaaaggccgtcgcaaagctctgcgtgtcggagtcggtggccgcgccaatggtgtcagcatcctgcgtgttgagcagcaccgtgtcggtgggcgccgcaagcgaggcggacgggccgtcgtcctcgaagatcatcattgagccgatttctcccgtcgactgcacggtccggggcagactgaatccaccgatgtcgaaactggcgttgaaatcgttgtcggtcgagccgacgttttcaatcaatacgcggttgtggtcgccactcgtctggtattcgatcacatagccggccttgactccgctgatcacggcggtgtcgccgctgagatcaatggacaggcccgttaccaggtttccggccgaatcacgaacgacgaccgagctgatattgacggccgtattattttgaaggttgtccacataattgtcgccagtcgccagcaccgtcgtataggcactgatcttgagcgtggccgctttattgggctgcaattgcgcgaccgtgaaagctgccgaagtggtgccgataagcccggtgaaatcgatgttcgattcttcgtcggcctcgttctgatcgagattgggaaccgtgttgtcggtgttggcgccactcacgaaagtgaaatacatcccttcggcaccgttcttgccgtcggggggatcaatcatctggttgttggtgcccaggctcgtgaacccgccgccctgactggaattgaccgtgtctccgtcgttgaatttggcgcccgtcgattcatttgccggattcttgccagtcgcaacgatggcggcgcttgcatcaccgaacatcgcgaacagattctggcctgagggaacattggcaaaagaaaacgcgttatccgaagtgaccgagacaaatatcttgtccgcgagattgaccgcgtcgtccgggttcgaagcatccggatgcgatatcgcttcatattgaaccgtccagagcttggcgcccgacaccggggttcccgtttcctccaggtaggccgcaaacacgacgacattgagggccgtctttccgtagacgatgttgttgttggttgtgtcggtataaagaaagatatcttcgccgtcggtggtattgaggccgctgtcgacaccattgagcaaagcgccgttgctgtccgtgaatgcaagatcggcgaccgtgccggatacgctgaatgtgaatgcgttggtgccggtgttggtaccgtcatagccgctcaacgcggcattgatggcggttcccacgctctgggccgccaggcggccgctgaaggccgtcggtagcgagcttgcggaaatatcgttgtcgttactgtcgccggcaacggcgggagtagcggcaaggttctgcaaattggcggattcgtccagagtgacgactgagccggccgttatatttagcgcggtcataaaaacactcctttactgaaaaaaatactccaatggaaatagcaatttcgaggatggcgctggcgatcattcaggttcgtgtatccagcgggatatcgatgctgaaccgccggcctgcaccttgtccataggccgaaagttgtcacccaaagggtgacgcgcagtgccggtggcgcgtgagtcaggagtgcccgtccacccgcatctggaagagaaagtagggcggtatgcaggccccgcggccttcgggttggccttcggcctgggcacagatgaagtcgtcgcggcaaggctgctgtgccgagcagctgcgcaggttgccgggccgcgtgtgcttgcccaggcattcgccaaagggcttgttcgccgccaggcattggttgaagtcgctgaggattgcgatgccgccgcaggtgccgttcttgtcgagcggatcgcaagggcccgagcacatgccgccgggaaagccgaccgaggttttctcgcacacggagagcgcaccttcgcaggcaacgcgcggaaatttctcggcgcggtcgagccaggggttggcggattgcgtgatgcgggtgggctcgcagctcgcgccaaccgtggctttctcgggcgcggtgttcgcgtcgtccgcttcggcgagcggccggaacggatcgggccgcggcgtcgagagcgcggcatgcacatagcggccgcgccgcgccagctcgtccttaaggtgcggtgagtgcggcagcgccagcgcattgcccgccgtaaaggtgcgcgatgcgccgcgccggtcgacacccagcaggtgaaagcccgcgaccgcgcggctctgatggcagcctgcgcagctcagatcgtcgaggcggcgcagcatcgcttgcggcgactgcagcgtgcggctgccgggcacggcctgccattcgccggccgaaaaaatctgggcgaacggacggttggccagccgttcgaggccccgcggcgccaccgagatggcttcggtcgcaaggaacttctcggggagctgcagcgtggcttcgtccagcgcgcgcaggttggcaggctgccgcaaccactgctgcagttccttgcgcagcggggcattggccttgagcttcgcgacgtcgggcgtgttctcgagcggtgccacgtcgaagcgttgcatgccggcattccagcgaaaggcgcgcagcatgtactctgcatggccgccgaggtcgggacgcacggccgagggccagcgcacgctttgcaggttggtggtgatctgcgcgatgcgtgcgggcgcaagacgctgcggcgccagcgggccgtcgggcgacaccagccagcggccgagcgcctcgtccgccatcgaaggccgtggcggctgccagcgccgcgcggtgctcgcgcaactgccgtcggcgtccggcgcatcgccgcgcagttcgacattgaccgtcatcggcaggcgcgactgcatcgcgggcgtgcgataggcgagccggtaaaccaaccgggtctcgccgcaggcgccgctctggaacggccggcggtccatgcggttggtaacgcccaccagctcgaagaaggcatccgggctcgcaagccagcgcgcatcgaacagccggtgcggatagcgcgagatgccgacaccggcctgccggtcgccgcgctggatgcgcgcgatactttcggcgagcggacgtgcgatggattgccacgccggcgagcgcatcagcgcctggttggccgtggtgccatcgggcgaagcgggtgcttcgccgaaccagtgggtaaagctggcgccggatttttcggcagcctgcaaggcggctggcgaggtgacgagaagcagcggctcggttgcgtgcgccatgggcgcggcgaaggcgagggccgacgcgagaaatgcaggcaggctgtgcttcaggagcggcatgcgcgcgattgtgcccgcgccgcccgggcccggacgtacggcgtgacacagtgtcccgctcctgggacatcgcccgccttctccacgcgcgaagccgcggtgcgcccctgtggaggcccgcacggaacggcccttgctatgacaagcgggtccatgacttcgccgcgccgtccaccaacgcccatgaactccgccgatctcgccttcgccccccggcacgacctgggtatccgcacggtgagcgtgagtgcccccgggcgcctgcacctgggttttctcgatccctccggctcgctcgggcgcgccttcggcagcctgggggtggtgatcgacggtttcacgaccgagctcgagctttcggcttcatcgtcggaccacctggcggccgacacgccagccgccgaagcggagctggcacgcgccgccgcgcatctctcgctgctccggcagcgcagcggctgccatgcgccgctgtcgttgcggctgtgccaggtgctgccaccgcatgcgggcttcggttcgggcacgcagctcgcctcggccatcgggcgcgcctttgccgaatggcacggcctggacgtgggcaccgcgacgctggcgcactggctcggccgcggcctgcgctcgggcatcggcattgcgggcttcgacaccggcggcctgctgctcgatggcggccccggcgccgatggcctgccggcgccgctgctctcgcgcattccgtttccggatgaatggcgcatcgtcgtggttcaggatccggtgcaccggggcctgtcgggcggggccgaaaaaaatgccattgcggccttgccgccgctgccgcagccggtggccgccgacatctgccaccaggtcctgatgcgcgtgctgcccggtgcggccagcgaggagttcgcgccgtttgccgccggcatcaaccgcatgcagcaattgctcggcgagcacttcgcgccggcgcagggcggtgtcttcaccagcctggccgtcgcgcggctgatgcaatggtttgccgatgcgagccgcgccaacggggcggccatcgggcaaagctcctggggccccaccggcttcgcgatcgtgtcttcggaaacccgggctcagttgctcgtcgacgccgcgcgggccggcgggcacgtcgacccgcagctcgagatccgcatcgtcaccggccgcaaccgcggtgccgtggtgcgcgaccgcagcgcggcggcacgcatgcgctgaagttgcccatcaacttttttccatctattcccaacgcaggctctctctcatggaacgtccccgcatcctccacatgttcacccccggcccgcagatgagtccattcgacatcaacatggcggcggacgcgggctaccagatcatcgtgccgtactgcggcgtggcactcgaccgcatcaccgggctcacgcaggacaccatcttctcgcgcgggcccaagggcgttgcgcgcaccggcatcttcatcggcgggcgcgatgcacagctggccgccgacatgctcgagcgcgcaagaacctcgatggtcaagcccttcgtcgtctcgctgatggccgacccgagcggtgcctacaccacggccgcggccatggtcgcatgcgtggaggcggcgttgaagcgcaaccatggccacggcctggagggccagcgtgtggtgatcctcggcggcacgggtccggtgggccgcgtggccggcgtgatcgcggcagaggccggggcggacgtttatttgtcgagccgcaacggcatcgacgcggcgcaggaagccgccgacgaaaccgggcagcgcttcggcgtgagcctgcacggcctctcgggcggcgaccccgatgcggtgcgccgctccatcgccgatgccgacgtgttgctggcctgcgcggccgcgggcgtgcaggtggtgtccgcagaagcgctcggcgccgcgacgcgcctcaaggtggcggccgacgtgaacgccgtgccgcccgaaggcattgccggcgtgggcgtgatggacgacgccaagccgctggccggcacgcaggccgtgggcatcggtgcgctggccgtgggcaacgtcaagtaccagacgcagcatcgcctgctggtgcagatgtgcgaggccgagaaggcacaggtgctgagctttgccgaagcctttgccgtggcacgcgccttcctggtcgagcaggccgcgaagacggcttgaagcgcctccgccccatgccgacgattgccgttgccgccatctccgcgcgcgccatggcccaggcggcggccagcgatggcttcaaggtggtcgcgctcgacctcttcggcgacatcgacacgtgccgcgccgcgtcgcgctggctgcccatcggcacgccgggcagcttgcagatcgatgccgccagcgtgatggcggcattgcgcacgctggcagaagagggcgtggacggcgagccggtgctgggctggatcgcgggcagcggcttcgaaggcgagcccgacttgctcgaagagggcgcggccgtgctgccgctgatcggaatcgcgcccgccgccgtgcgccgcttgcgcgacccggcggcattcttcggctttctttcggcgcgtgtcctgccgtttccgcaggttttgctgcagccgcccgaggacccctcgggatggttgatgaaagacgcgcatggctgcggcggctggcacgtgcgccatgcgccctggtcgatggatgagccgccttcgtcgcaccactacttccagcgcgagatgccggggctgccgatgtcggccaccttcatcgccaatggccgggacgtgcatgtgctcggcttcaacgagcagagcgtgcgcagcttcggcacgcggccctacgtgttctgcggcgccatcgggccggtgcctttggcggacgacctcgcgagccgagtgaccgacattgcgcgcgcattgaccgtcgagttcgagctgcgcggcctgtgcagcctcgacttcatgcgcgacggcgacgccatcggcgtgctcgagatcaacccccgtccgccggccagcatgagcctctaccgttggcccgacggctcgccgggcgtgatgcaggcgcatgtgcgtgcctgcctgcagggcgagcttccgccgtcaacggtttcttcgcctgcgcaagacatcgaaggcatcgagatcgtgttcgcacggcaacccgtcgaactcgatgcggccgcggcagagcggctcgccgcatggcccggcctctgcgacgtgccggccccgggccagcgtttcgacatcgacgaccccgtgtgcaccctgaccgcgagcggcaccagcgcacagcaggtgcgcgcccgcttgaacgaaggccgcgaacggctgctgcaatcattggagacccacgcatgagcaacacatcctcgcccacggccgccgcgggcctgagcgtcaacctgctggcccgtccgctggtcgagcgcctgctggccgacgccgatgtgctcgggctgcgcgtgcgccgtgacgacaccggcgtgcatatcgtcgatgccggcatcgaggcagcgggcagcgtggcggcggggctgcgcgtgggcgagatctgcatgggcgggctcggacacgtgaacctgcgcagcggcgccggcacggaggtttggcccacgtggctcgacgtgcgcagctcgcagccggtgctggcgtgcctgggcagccagtacgcgggctggagcctcgcggcatccaaggaagagacgggcggcaagaaattcttttcgctcggctccggtccggcacgcgcactggcggtgaaggaaaaactctttgccgaactggactaccgcgaccacgcgccatgcggcgtgctggtgctcgaggtcgaccgggccccgcccaaggtcgtgatcgacaagctgctgcgcgactgcggcctggcccccgaggcgctgacgctgatcctcacgcccaccaccagcctggcgggcaccacccaggtggtggcgcgcgtgctcgaagtggcactgcacaaggcgcacgaactgggctttgcgctggccaacatcgtcgatggcgcgggcaccgcgccgctgccgtcgccaagtgccgatggcgtcgaggccatgggccgcaccaacgacgccatcttgtacggcggccgcgtgcacctgacggttcggggcgacgacgatgcggcgcgcgagctggcccgtgcattgccgtcgcgcaattcacgcgatcacggccgctccttcgcccacatcttcaaggaggtcgaatacgacttctacaagatcgacggcgcgctgttcgcaccggccgaggtgtgggtcagcaacatcgacagcggcaacacctggcacggcggtgcgcccgacatggggctgctgcagcggctctggctgcaggaagcatgaaggcaatcccatgaccatgcgtatcgtcatcatgacggacgagatcggctggcacacccgccagctgcaggctgcgctgcgcgcacgcggcgcggtggggcgctgcgtcgatctggccgactgcaacatcgacaccaccgcggcctggcatggcctggtcattcccggctatggccgcgaactgcccgacgcggtgctggtgcgcggcattgcgggcggcagcttcgagcaggtcaccaagcgcctcggcgtgctgcatgcgctgcgcgaactgggggtgccggtctacaacgatgcgcgcgccatcgagcgcacggtcgacaagtcgatgaccagcctgctgctgcatgccgcgcgcattccggcaccggccacctgggccaccgaatcggcggcccaggcgcggcgcatcgccatgcgcgaggtggccgcggggcatgcgctggtgctcaagcctttgttcggctcccagggcaagaacctccggctcgtgggcgaggtcgacggtgtgcaccatcccatgcccgacatcgatgccggctatgcgggcctcgcctacctgcagcgcttcgttccaccgatggcctcgcccggcttcgactggcgcgtgatggtggtgggcgggcgtgccatcaccgccatgcggcgcgtcagcacgcactgggtccacaacgtggcgcagggcgcgcgctgtgagccggccgagctggagccggcgctcgcgcacatggccgaaggcgcggcgcgcgcgctggacatggactacgcgggcgtggacctcatcgccgcggccagcggaccgaagatccaggtgctggaggtcaacggcgtggccgcgtggcaagggctgcagcgcgtcacgggtttcaacatcgcgcgcgcgctcgtcgatgacctgctcgaccgcaagatggcgcaggtccagcgccgcgtgcaggagagcgtggctccggagcgccgcgcctgatggccatgcgccaagcggccaccgagcgtgcccgggcctgtttccttcgggcctgctggctcgacgtggccgtgcgcaagccgggcaacgtgagcctggcctcgcccggccatggcatgcaggcttcgatgttcatcgccagcgcgcgcgccgcggccggtgcgctgttcgagcccggcttgcgcgtgggggagcgcatcgaggccgcggtggaggccacctgggcggtggccgggtgcaacaccaacctcggcatcctgctgctgtgcgcgccgattgcgctggccgtggaacggcagcccggcgccgcgacgcccgcggccttgcgcgccgccatcgaaggggtgctggccacgctcgacatcgacgacgccagcgcggcctaccgcgccattgcacgcgcgcatccgggaggccttggaagcgcggcggagcaggacgtgcacgacgctcccaccatcgacctgcgcgccgccatggcgctggccgcggaccgcgatctcatcgcacgccagtaccgcgacggcttcgcggatctgttcgcgctggcgttccaggcgccggcctgccagcccggttgcggggcggtcctggccgatgccgacatgccgccggatgcggccactgtggcttctgtccaacggctttacctggcttacctcggcgcctttcccgattcacacattgttcgaaaacacggcgagcgcgtggcacagactgtcatgacggcggcgcaggcctggcgtgagcgcgccggcgcgggcgctgtgctcgatgctgatcctgcctttgccgagtgggacctttcgctaaaggctgagggcgtcaaccccgggacgagcgccgatttcaccgtggcggcgctgctgctttcgggctggatccagtcgtgcgcggcacccgcgcgcgatgccgcgaacgcatggcacggatcgtgatacccatggcattgcgctggtcttcctgaccggtgtcgtaatgaccctaatcaccttggacctctgagaggagactcgaaaccatggcaaaaatcgatcgactgatggtgggcgaatcgctcgttggcgacggcaatgaagtagcccatatcgacctgatcatcgggccgcgcggcagcgctgccgagaccgccttcgccaacgcgttgacgaacaacaaggacggcttcacttcgctgctcgcagtcgtggcgcccaacctgctgaccaaaccggccaccgtgatgttcaacaaggtgaccatcaagggcgccaagcaggcggtgcagatgttcggcccggcgcagcgcggcgtggcgctggcggtggccgacagcgtggaggatggcaccatccccatggcggaggcggacaacctgttcatctgcgtcggcgtgttcatccactggcttgccgacgacgacaagaagatccaggactacaactaccaggccacccgcgagtccatccagcgtgcagtggccggtttgccgaccgccgccgaggtggtcgacaagaagggcacgacggcgcatccgttcgctgcccacctctgaagcgcacaaacaaaaaccgacgcgtgaaccgcgtcggtttttttccatgtgccgccgcaagaagcggcggagggcgctattcagtgcttggcgggcaccatgccgctcgcgagaaagttcagcaccgtggcaccgggcgccgacttggaagcgcggtgcgtgggcgcatggcgttcgatctgcacgcccacggcctgcacgtcgtcgaacttgcgtggcttcaccaccttcacgcggacccagctggcaccgaactcgtcgatgaggatgtcggcgatggcttcggcaaaggcctcgagcagttgcagccggtgctcggccatgagccgcaccagccgctcgcgcaccacgccgtagtcgatcgtgtcgccgatgcgatcggtgtcgcaggcgcgcgcacgcggcacgccggcatgcacgtcgatcatcagtggttgcggatgatgcagttccgaatcgtggatgccgatcaccgtctggccgctgaagccttcgatgaagatcaggtccatgggcgcgggcgcctcggccgcgcccaccgcgccggaggcatgcgagacattcgaagcaaagggaccggtggaaggacgcgggctggtgttcaagtggtgtctccagtgattcgaatgtgtttgaaagtgtgtcttgcggccgatagtcagccaacgacaggattcatcaacgcaaaatgcaggccagagatcggacccgccgcggggctgcgagtgcttggtgtttcaccgggtgcgcagtaactcagcaggcacaacaatgggccgaccaaggagacatatggaacgcgccggagaactccaatgacattgacgctgcgacaaggcgacaggcacgctgaccgtgtgctcgacgtggtgaggcgagggtttcacgaagaaggcaacgacctggtcacgcgctcgtggagccgttgcctcaatcaataccagctcgacccgggccgcccgcgcgaacccgtgatcatcgcgtcgtctgccttgcagagccggcgcaaccagcatgccgacgtgatcgagtgcgcgcgctacgagatgaccacgctctaccagcagctcgcggatgcggaatccgccgtggtgctgaccgataccgatggcgtcatcgtgcacatggtgtcctcgcccgagttcgcggccgaggcggagcccatgggcctgcgcgccggcggcatgtggggcgaggccgaggccggcaccaacggcatgggcacctgccttgctgccgcacacccgatctccgtgcggcgcgaagagcatttcttcagccacttcacgcagctcacctgttcggcggtgccggtgttcgatccgtccggcgagatcattgccgtgctcgacgtgaccagccgctccagcctgatgcagcagcacgtgctggtgctgctcggcatgacggcgcgcatgatcgaaaaccggctcatcgacaagcgcttttcgaatgcgcatccgctgcacttccacagccggccggagttcgtctacacgctgcacgaaggcaagctcgcggtcggcgacgacgggcgcattctcgcggccaaccgcagcgcgctgttccagctcggcctgcaatcgatggacgagatccgcacgcaacgcatcgacgatctgttccagacctcgctcgaagacatcgtgcagcgcagcctttcttcttcattccatccggtggtggcctaccgggccaacgcggcgctgcgcttcttcgcggtggccaggcggccggcatccgatgcggccacgccttcgcgtgtgcgcggcgcgggcgcagggacggcacccgtcatcgcagagacgggcgccgaggctttccgcgcgccgctgcggccatcggccacgcgtgcgcctggcattcgcaccttcaaggatgcgcgcctggttgcgcacctggacaccgcgcgccgcgtggttgcgcgccgcacgcccgtgctgctgtgcggcgaaacgggctcgggcaaggaagtgttcgcgcgcgccatccacgagaccagcccgcatgccgaaggcgccttcgtcgccgtcaattgcgcgagcctgcccgagacgctgatcgaatccgaactcttcggctacaaggccggtgccttcacgggcgcgcagcgcagcggccggcgcggcaagatcctgcaagccgatggcggtacgctgtttctcgatgaaattgccgacatgccgctggagctgcaggcccgcctgctgcgcgtgctcgacgagcgccaggtcacgccgctcggcaccgaggaaacccacccggtggatttccagctcgtgagcgcaagccatcaacacctgccgagcctggtgcgcgaaggccgcttccgcgaggacctctattaccggctcgccggcatcgagctcgacctgccgccgctgcgcgaccgcacagacaagcgcgaactgatccacgacgtgctgaaggacgagggcggcagcgacagccgactcggcgaagatgccgagcgcgtgctcatggcctatccgtggcccggcaacctgcggcagctgcgtcacgtgctgcgcagcgccgccgcgctggccgacggcaagaccatcacgcgcgagcacctgccgtcgctggccgcaagggtggtgccttcgcccgtatcggcctattccgcgctgcctgccgcatccgaacccacggaagtttcagcggacgccgcgccctccgatgcggcacccgccgtcaaactcaacccgatccaggccaacgagcggcaagtgctgttgcagatgctcgagcagcatcgttggaacgtgagcaacgtcgccaaggcgctcgatgtcagccgcaacaccttgtaccgaaaactccacaagcttcacatcgaaatctctccacccgattgagccggcaggctcgctggacatgacgacgaatggggagccaccggccacgggcaacaagatcgatccacgcggcgcggcgctggtggccgaagacggagagccgccgctgccggcctcgccgccgcgctcgcgcatcgcctggtgcatcacgggttccggccactttctcgaggagtcgctggcgctcgcctcgcggctgccctcggtagacctgtttctctcggccgccgccgaggaagtgctgcccatctacaagctgcacatcgaagcattgaaggcgcgctttcgcgtctttcgcgacaagaccgcgagcggcgtgccggtgggcatgctctacgacgacatctatcacacggtggtggtggcgccggccaccagcaacacggtggccaagtgcgctttcggcatcagcgacagcctgccgaccaacatgttcgcccaggccggcaagctcggaattcctggcatcgtgtttgcatgcgatacggaaccggtggtggtgaccaagtcgccgcatgactgggtaacgctgcgtccgcggcgcatcgaactggacaacgtggagcggctgcgcggcatcgacttctgccaggtggtcgcgtcgccggccgaactcgaagccgtgctcgatgcacgcatgaaggaactctctctcgcatggaacacatcgtcttcctgaccgggcgcctcgcccaagccagcctcacgcgggtgctggcgggcatcgaggcggcaccgttcacgtgggaagtgcgggagatcggtttgcaggtggccgcgttgatgacggccgacatgatccgccgccgcgtcgcggctccggtgtgcaccgagggtgaaggcgagggcgccgcgccgcgccgcgccgaccgcatcatggtgccgggccgctgccgcggcgacgtcgaggccttgagccttcacttcggcgttccggtggagcgcggcccgcaagagctgaaagacctgccgcgccacttcaaccgcaccgcgcgcgcagtcgacctgaacgagtacgaggtcgcgatctttgccgagatcgtcgatgcgccgcggctctcggtgccgcagatcgtcgagcgtgcgcggcagctggcggccgacggtgccaacgtcatcgacctgggctgcctgcccgagacgcgcttcgaccacctggccgacagcgtgcgggcgctgaaagccgaaggctttcaggtgagcgtcgattcgagcgaggcgcaagagcttttgaccggcggcaaggccggtgccgactacctgctgagcctcacgctcgacaccctgtggatcgccgacgaagtcgaggccacgccggtgctgattccgcgcgttccggccgacgaagaatcgctgtaccaggcggtggcgcagatgcagcagcgtggccgcgccttcctggccgattcgatcctcgacccgatcccgttcggcctgacggcgtcgatcgtgcgctatcaccggctgcgcgagcgcttccccgatgcgccgatcatgctcggcgtgggcaacctcacggagctgacggaggccgacaccagcggcatcaacgcggtgctgttcggcattgccgccgagctgaacgtggcggccgtgctgaccacgcaggtgagccagcatgcgcgccgcgcggtgagcgaggccgactgggcgcgccgcatcatgcatgccgcggtccggcacggcaccttgcccaagggcatgagcgacgcgctgatgacggtgcatgccaagcatccgttccccgacacgcccgaagagatcggcgagatcgcctcgcaggtgcgcgacccgaacttccgcgtgcagatatcgccgctgggtctgcacgtgtacaaccgcgacggcctgcggctggggcagggcgccttcgagctctggccgcagctcaagctgcaggacgatgccgaccatgcgttctacatgggcgtggaactcgcgcgcgccgagatcgcctggcagctcggcaagcgctatgtgcaggaccagccgctcgactggggctgcgccgcgccgcggcccaccgaagaccttgcgcgctggtgcgcaccgggaaccaccatgaagacatcgaagaagaacaacgccgcagccgaacccggggccgtgggcaccaccaccgcgccaacaccctcatgaacgaccagatcttcgaagccgtggtcaccaccgtggcccccggcggccaaccgcacgtggcgccgatgggcatccgctaccaggagggtggcatcctgctgatgccgttcaagccctcgaccacgcacgacaacatcgtggccaccggccatgcggtgctcaacatcgtctgcgacacccgcgtgttcgccggctgcgtgaccggccgcaaggcctggcctacgctcccggccgaacgcatcgaaggcgtgcgcctggccgccgcgctgcgccacgtcgaattgaagctggccgagcagcgagacgacgcgcagcgcccggtgctgcgcatgctggccgtgcacgaggccacgcatgcgcccttcatcggcttcaaccgcgcgcaggccgcggtgatcgaaggcgcggtgctggtcagccgccttcacatgctgcccccagagaaagtggaaaccgaaatgacctacctgcagattgcgatcgacaagaccgccggacccgaagagcgcgaggcctgggagtggctctgcgccgcggtcgcgcagcaccgcacgggcatgccggagcgcgcatcatgacgcgcatgctggtgagcgttcgcagcgtggaagaagccttgctcgcggcccgcggcggggccgacttcatcgacctgaaggagcccagcgacggcgcgctgggcggcttgcctgtggcgaccatcggcgccatcgtgggtgcactgcgcgcgcatggcatcggcctgcccgtgagcgcaaccatcggcgatctgcccatgcatgcgctggaccgcatccgcgcgcaagtggacgcggtgggcgcttgcggtgtcgactacgtgaaggtcggcatagagcgtggccttgaggccttcgcggtgctcgatgcattggcagcctgcgagtggccggtggtgccggtcttcattgccgacaaagggctcgacgccgcgctcatcgcgcacgcttgtgcgctcgattttccggggatcatggtcgacaccgccgacaagctggccggcagcctgttcgatgcggtgcccatggcggacctgcgcgccttcgtggcaaaggtgcgcgcatcgggccgcatggccggtgcggcgggtgcgctgcgtgtggcgcacattcccttgctgcaggcgctggcgcccgacttcgcgggattccgcagcgcggtttgcgtggccgaccgcaaaacggcgctctgccccgagcggctcgcggcgctggccgcgttgctgcatggcgaagcggtcgtggaagcggcggcggcttgagcttttcggcgccgggcgatctcgcccgcgtgctcggtcgctcggcgttcgtcagcgtggcgtgaaggtggcctcgcccagcagcagcgcacgcatggtcgacagctggttcttgtgaagcagcgtgatcggaaaggccgcgtcatcggactgcttcgcaaactgctggtcgagcaccccggtatcgccaagctccgccagcgtcatccgcggatcgatggcgcaggacttgaccagcaccagctgctcggcgttgagatgtttcgcgagatcgagcgcaatggtgtccgatgtggcgtcccagccggtgcgctcgtcggggtggtcgcggcgcaattcgagcggcagccacaaggccgtctttccctggcgcagcaagtcggggatgtcggtcttgcgcgtggccagctgcagccccggattcagcgcatgcagctggtaggccgtctgcgccatggccagcacggccatgttgtgggcggccaggtcgttgaactgccagtgcgattgcacgcgccgcacttcatccgcaaaggtgccgccgccgcagaccacggtgacgcgcccgccgccgatctgcgtcaggaggtcgagccacagcggcagcaccgggtccgaacaaaggctgccgccgatcttgacgacccacatcagtcgtgctccctttcgaacagcgccgccaccgcgacgctcggtgcgcacacctgtgcccaggtggtggtgcccgcggccgcatggcgggccacgctcgcgacgtcgccgccataggcggcaaaacggcgcggcacggagccgggggtttcgcccgcggccgcggcggccaggtcgggcaccaggaaggcaccgcagcccgcgctcacgatcacggcctcgcgcgagagcgcatgcgcggccagcacgcggcgcagctgtgcggcaatggcttcgacctgtgcggcgcgccaggcctgcgcaagatccagccattcgcccgcggaggcatcgcgctcgtccagccccaccatgcgcgcgaggcgctggcgcgtggcgggcaggcccttgtccgcgttgtcggcgctcgggtacaggtcgtgcgccggatcgagctcaccgcacagccggtagacgtcggccgtggtggcgaaaaactcgttcatcacgtgtcgtgcctggccgcgccattcgatgcgctgcgtcagcgcgcacaccggggtccgcaccacgccgtggtaggcgagctcgccgctcaccaggcgttcggcgtcggtgcggctggtggtcagcacgccctcgttgccgaaggcgatcaggtcggtggtcgtgctgccgatgtcgaccagcacgccttctgaaaacaccagcgcggcatgccgtgcggtggcgagccagttggccgaggcaatgtgctcccagtgccgcgccacgtccgcggcggtggcgcaccagccggcatcgccggcaaagaagtgcagggcgcctggcggcacggggagcgatgccgacagcgcggtggcaatgccgcgcacgccggcttcgcggtcagtgaagaggtcgaccatttcgcccgtcatggtcgccgcatgctgggctgcgccgagatcgggccagcgcgcctgtgcagcctggagcgctcgcgtcagatggtcgagcccctgccagagcggacagccccattgggccacgtcgaccacctcgccgccttgcagcaggcaggccttgacgtgcgcgccgccgatgtcccacccgatggtgatgcgttcaggcgactgcacgcgcaagttcccgttcttgggcgccgccgccgtgcaggcggtctgccagcagctccgcggccaggttgcggcccagcgccgccgagagcccgacataggcgcaggtgacacgcggattgacctcgatcaccaccggcccgcgctctgggtgccagaccaggtcgatgcccgcgaagcctcgcaggccggggatggcgcgcgccacctgccgggccagtgccgccaggggagcccggcgcggatcgctgcggcccaccgcatcgacgctcacgccatcgaaagacagccttccgtgcgtgtcgatcgagatgcgttggcggttgatgctcagcatttcggcattctgcgccgtgcacagcagtgagaggctgagggcttcgccttcgatccagggctcgagcgtcaaggtggcgccggcctcggtgcgccgtgccatgtcgcccagtgcatccgcatggcgggtgtgcacgtgggtggccacgccgcccgcgccatcgtcgggcttgaccacccagcgcgtgatatcgggcgcatcggcaaaagccagggtcgtctgcacgccgtgggcggccaggtgcgcgagcgtggccttcttgcctgccgtgagttcgatggcttcgacgctgcagccgagccagcgcgcgttgcccaccgtgcgctggaagcgcgccagcaggccgtccgtttcgggcgccaccagccacaccaggtcatgcagcgcgctttgccgcgccacgaagtcgagggccgattcgttggcacgtggccgcagcggcgccgtgccggcgggcagggtgttccccggttcgcagactgccgccgagaccgaacaatcggcagcgcgccgcaggtccgccaccatggcatcgcgcatcgacaggcccagcggcaacagctcgtgggcggccgcatcgtcgccgtagtcgctccagccgccgccgctgagatactcgtaaacaaaaacgcgtgtcgtcatttcatcatccactttccgggctcttccccatgacttccgaactgaacctgatccccgtcgtcgacctgctgcagggccaggtggtgagggccgtgcgcggcgaccgcaaggcgtaccggccgatcgtgtcggcgctgtgcgccagcagcgacccggtgacggtggcgcgcatcctgtgcgaccactgcgcagcgcggcagctgtacgtggccgacctcgatgccctgcaaggcgggccggtgcagatcgcggtgctggccgatctgctgcaggcgctgcccgaggtcgagctgtggctcgatgcgggcctggccgacgctgatgacggccaagcgttgcgcggccagctggcgccattcgcctcgcgcatcgtgctggtgttcggcagcgaatcgctgcgttcgcgcgaggcgctggagcgctgttttgcgatggacgaagacggcgcggttgaaggcccgctgggcgccgcgctgtcgctggaccggcgcgacggccagcgcctggaccacgccggctgctgggaggcggtcgacctgtggccggagcgcctgatcgtcatgacgctcgagcgcgtgggctccggcgcagggcccgacctggaaaccctgcaggaggtaagacgcctggctccgggcgccaccgtgatcggtgccggcgggatccgcagcgaggacgacctggcgcgtgccagcgcggccggcgccaatgcctggctggtggccagcgcgctgcacgacctgcaactgccgcgcgtgcgccgctgatctaccgggggtggcgcaacggggggggttgaggcatgccatcaacccgctgcactcacgaaccgtgccatccccgatggcgctcgcaggcgccgccggaagccgctgccgtcacgcattgaccgccaaaagcgcaacactatgtctcacaaactgtgtgtcatagggcgctacccctaggcgcgcgggccttgcggctgaatggcacatcgcttgcgtggttgcctgcccatgaatgatttcgacactgtcacgcagccccgcaatgccccgtggacctgtccgttctgtcccttgttgtgcgacaccttcggcgtcgacatcgggccgcccggcgcgccgctgaaactcacgggcagcgattgcccgcgtgcgcgcaatggcctggccaatttcgatgccaacgccagcgcgggccagccccgggtcgatggccgcgactgcgatctcaacaccgcgttggccgccgccgcctcgctgctggccgccagccgccagcccctgttcggcggcctcggcaccgacgttgccggcgcacgagccctctatgcgctggcttgcgaaacaggtgccatctgcgaccccgcgcagggaaaggcgctgatgcatggcctgcgcgcattgcaggatcgcggcggcttcagcaccacgctggcggaggtgcgcacgcgggccgacctgatcgtctgcatgaccgaggagcccacggcgcattaccctgaatttttccaccgctgcggagcgggggaacgcgaagacctggccatcgagacattgcccttgcacggcgacctgttcgacaccgtgtccctgctggccgcgctcgtggcgggccgtgtccgggcggacgacgatcgcgtgcccgccgatctggcggcgttgtcggcgcgtttgaaggcggcccgctatgcggtgctggtgtacgaatcggcccgcctgcctgcccagggtgcgctgatcatcgaggccatccagcgcatcgtcggaacgctcaaccgcacaacgcgcgcggcctcgctgccgctgggcggcggcgacggcgcgtccaccgtgaaccaggtgttcgcctggctgtcgggcctgccgctgcgctcgcgcgccgggccgcgaggcctcgagcacgagccgctgtgcttcgacgcagaacgcctgttggcagatcgcgcggccgacacgctgctgtgggtgtcgagctacggccccgagcccgcgccgccagccaccgacgtgccgctcatcgtgctcggccatccggccatgcgcttgccgcaaggtggggccgaaggcgtattcattcccgtgtcgacgccgggcatcggttccggcggccatctgttccgcaccgatggctcggtgatgatgccgctgcggccgctgtacgacgacggactgcccagcgttggcgacgtggtccggcgcctggtgcatgcggtcaaggcacagaagaaagggcgcgtgcaatgacggccacgcttcgcctgcgcggcggccgcgtgatcgaccctgcgaacggtcgtgacaaggtgcgcgacctgtatgtgcgcgacggccgcatgatcgagctggcgccgcacgaggccgccaccgaggagatcgacatcggcggctgcatcgtgatggcgggcggcatcgacatgcacacccacatcggcggcggcaaggtcaacctcgcgcgcatgctgttgcccgaagaccaccgcgccaacgcaaaccccgtggcgctgcccgacaacgtgctggagctggcgtcctgcggcacctgcacgcccggcacgctggccaccggctaccgctacgtcgagatgggctacaccgcggccttcgagccggccatgatggcgtgcaacgcgcgccacacgcacatggagatgggcgacacgcccatcctcgaccatggcgcctacgtgatgctcggcaacgacgagctgtttctgcgcatgctggccgagcgctgggatttcgagcgcattcgcgactacgcgggttggaccatcaacgccagcaaggcgatgggcgtgaaggtggtgaaccccggcgggatctcggccttcaagttcaaccagcgcaagctcgacgtcgacgagaaccacgtgcactggcaggtcacgccgcggcaggtggtgcacacgctggcccgtgcgctgcgggagctcggcgtgccgcatccgctgcacatccacggcagcaacctgggcgtggccggcaacatccagtccacgctcgacaccatcgccgcgctggacggcctgcccgggcacctcacgcacatccagttccatgcctacggcaccgaggggccgaagaagttttcttcggccgcgctgcagctggccgaagtggtgaacgcgaacaagaacgtcagcatcgacgtgggccagatcatgttcggccagaccgtcacggcatcgggcgacacgatgcgccagcacgcgcagtcgggcctggccgatccgcgcaagtggatcggcgccgacatcgaatgcgaagccggctgcggcgtggtgccgttccgctaccgcgagcagagctatgtgaatgcgctgcagtgggtcatcgggctggagatcttcttgctggtcgacgatccgtggcgcgtggtgctgaccaccgaccatcccaatggcggcccgttcacgagctacccgcatctgatccgccttttgatggaccgcagctttcgggaggaacaactggccaggctgcatcccgaggtggcggcgcaggccgcgctgcgctccatcacgcgcgagctttcgctgtacgagattgccatcatgacccgcgccggccctgcgcgcctgctgggcctgcccgaccgcggccacctgggcacgggcgccgcggccgacattgcggtgtaccgcgagaacgccgaccgcgaggccatgttcgcgacccccgaatacgtgttcaaggatggtgtgctggtgtcgcgcgcggggcgggtcactgcggcgccggtgggcggcacgcacttcctcgcgccggactacgaccgcggcatcgagcagcgcctgcgccggcatcttgcggcgcagggctcggtcaacttcgaccacattgccatcggccacgacgagctgtgccagtgctgcaacggcgggcgcctgctgccggcggcatgtttccaggcggtgtcgtcatgaaggcgggtgcggcatgacggcgccatcatccgtgctgcgcaacggcgtcgtcatcgacgagacctttgccgaagcctttccgatgaaggccacgcgcatcgtcatcacggcccacacgctcgagtgggcgcgccacgccgcggtgtcggccaccggcttcgcaacctcggtgatcgcctgcggctgcgaggccggcatcgaacgcgagctcggcctgcatgaaacgcccgatggccggccgggcgtgagcgtgctgatgttctccatgtcgggcaaggagctgggcaagcagctcgagcgccgcgtcggccagtgcgtgctgacctgtccgaccacggccgtgttcgcgggcctgccgaagggcgccggcagcgacgtggcagcgctcggcaagaacctgcgcttcttcggcgacggctggcagatttcgaaggtgatcgacggcgtgcgctactggcgcgtgccggtgatggacggcgagttcgtcgccgaggaagacacgccagtggtcaaggccgtgggcggcggcaacctgctgctgctggcgcgcgacaccgatggtgcgctggccgccgccgaggccgcggtggcggcgatgaagcggctgcccaatgtggtcatgccgtttcccggcggcgtggtgcgctcgggctccaaggtcggcagccgctatgcgaacctgagcgcctcgaccaacgatgcgttctgccccagcctcgtcggcctggtgcctcacagcgaattggcgcagggcggtgcgtcggcacaggagatcggctgcgtgatggagatcgtgatcgacggcctgaccgaggcggacgtggccgcggccatgcgggtcggcatggaggcggccatcggcatcggccccgccggcgggctgctgcgcatctcggccggcaactatggcggcaagctgggcccgttccacttccacttgcacaagctgctcggcgatgcgggagatgccttatgagcggatggcatttcaggctgcggcaggccccggcattgcgtgtcgacttgcgcggcgtcacgccggcggcgcttgcagaactctcggccgcccagatcgaacggctgccggtgggccatggcagcgagatgctggcgctggccgaactgttcgacgttgcgccgggcgaggagggcgtgcttcgcttcgagggcggcctcgaccgcttcgaccgcatcggctggcagatggatggcggcagcatccgtatcgagggccacgcaggccactacgcgggtggctgcatgcgcggtggcgagctgcgcatcgacggccatgcgggcctcttggccgcctgcgagatggccggcggcagcatcgacgtgaagggcgacgtgggcgatttcgccgcgagcaccttgcccggcagcatggacggcatgcgcggcggcaccttggtcgtgcatggcaatgcgggcgagcgcttcggcgatcgcatgcgccgcggcaccgcccttgtccatggcggcgcgggcgctttcctgggctcgcgcatggtggcgggtacgatcggcgtgggtggcagcgccggcgcgcatgcgggctttggcatgcgccgcggcagcatcgtcttcgcggaggccggcgcggccttgccagaaagcattggaacggcgctgacctttgtgcccaaccgggccgcgacgccggtgttctgggcgctgctggcgcgagacctcgcgcgccacggcggattgttcagcgacttgccagtacgccgcatcgagcgccatttgggcgatctttcggcggatggcaagggcgagctgatcgtgtgtctatgacttccttcccaagcttttaacctcgagcgtttatgacgaatccttatctttttcatgccggcgaagccaccgtgcttgccagggaaggccagttcaccgacgccatgccggagatcctgatcggcgcgaccgacggccccgtgggccaggcctttgccaacatgatggcgcagagcaagggccatactgcgatgttcgcgattcgcgcctgcaaccagctcgtgcggccggcgaccatcatggtgcccaaggtcacgctgaaggacgcggccaacatcgacctgttcggtggcgtggtgcagagcgccacggccgacgcggtggtcgattgcctgatcgaaggcatcattcccaaagaacatgccaatacgctgtgcatcatcagcctggtgtggatcgatccgcgctgcgccaaggaccaggacctcgacaagaaagacatgtaccgtaccaactacgaagccaccaagctcgcgatccgccgcgcgctccacaacgagccctccgtggacgagctgattgccaaccgccatcgcatcaagcacgatatggacgattggagttgaccgtgccttccttcgcgctcctcgacgattgcggctcgacgcccgagcagcccaccagccggctgcacaccggcttcgtgcgcgagcaccggtgcaccgacgcagccggccttgacggcgtgtgggcgcgggtcgatgccgatcttcggcagggcctgcacgcggtgctgctggccgactacgaatggggcgccaagctgctgcacgcggggcaggcgcggcttgcggccgacgatgcgtcggcactgcgcgtgctgatgttccgcgattgcgaaaggctctcggccgatgaggtcgcgggctggctcgaaaagttcgagcagtacggggccggcgaggtgctcgacggcggccacccgcagcccgccggtgcgatggacctgcagcccagcatcgacgaagccgccttcaccgatgccattgcgcgcattcacgacgccatcgcggcgggcgagacctaccaggtcaacttcacctaccggttgcagggccggagccatggttcgccggtggcgctgtaccggcgcctgcgcgagcggcagcccgtggcctatggcgcgctgatcgcgctgccggaaagcgacgaagacgacatcacccacgtgctcacccacgtgctctcgtgctcgcccgagctcttcctgcgccatgacggcggcgtgctcaccgcgcggcccatgaagggcaccgcggcgcgcgtcgatgcgcccgagggcgacagcgagatggcgcgcctgctgtcggtcgacaccaagaaccgggccgagaacgtgatgatcgtcgacctgctgcgcaacgacatcggccgcgtggcgtgcaccggctcggtcaaggtgcccacgctctttgccatcgagccgtacgccacggtgttccagatgacctcgaccgtgcaggcggcgctgcgtccgggtgtgggcatgcccgagctgctgcgcgcggtgttcccctgcggctcgatcaccggtgcgcccaagcatcgcaccatggaatggatcgcccagctggagagcacgccgcgcggcctttactgcggcgccatcggctggatcgatgcgcctgcagcgggcgcgtcgatcggcgacttctgtctctcggtggccattcgcacgctcacgctgggcgcggaatcggaaggcgcgaggccgctgcgcctgggcatcggcgccggcatcgtgcaagacagcgttgcggccgacgagttcgaagagtgcctgctcaaggcgcgcttcctgacggccctcgaccccggtttcgagctgttcgaaaccatgctggccacgccgtgcgacggcatccgctatctggaccggcacctggcgcggttggcgcgcagtgcgcgcgtgctgggcttcgaattcaatcgcgatgctgcgatggaggcgctgcgcaatgcgctgcccgcgttggcccccggccagccgtcgcgcctgcgcctggcgcttgcgcacgacgggcgaatcggcatcacgcattcggcgctgccgccgttgccgcccggtgcgttgaagctgctcattgcgagccagcgcttgcccaatgccaacccgctggccgcgcacaagaccacggtgcgccagcactacgatgccggcgtgcgaaccgccgagcgcgccggtgccttcgacagcctgttcttcacggaggacggccggctcgtcgaaggcgggcgcagcacggtgttcgcgcgcgtcgacgggcgctggtgcacgcctccggtgtccgacggcgcactgcccggcgtgatgcgcggcgtgctgatcgaagactcgatatgggaggccatggagcgcagcctgtcgctggaagacctgcagtcggcgcagaagctggtggtgtgcaatgcgctgcgcggcgtgctgccggcgcagctgcaacttcctcaggtgccatcgcggctgcggccgccgttgcagccgcatgcccatgcggcttcggccgcctgaggcgggtgcgcgcttcgacgccggttccgcgatgaagctcgcgctgttcgacctcgaccacacgctgatcccgttcgacagcggcatggcctggacacgcttcctggtggcgcgcggcgtgctggcggcggatgccgagacggtctacctgggctattgccagcagtacgtggacggcacgctggacatccgcgaactgcatcgcgccagcgtcacgccgttggcaagctttggcatggcccagctccggcagtggtcggcggagttcgaggccgagatggcgccgcgcgtgcccgagccgatgcgtgcgctggtgaaaaagcaccaggatgcgggccacctctgcgccatcgtgaccgccaccacccgcttcatcgccgagcccttcggccgcgtgttcggcgtggccgacgtgctggcaacgcgctcgctggtgacgggcgacacgctcgacggcggcatcgatggcgacccatgcttcggcgtgcacaagctgatgcacgtgagccaatggctggcgctccacggcacgcgcctcgatgcgctcgaacgctcgtggttctattccgattcgaccagcgatctgccgttgctggaggcggtgtccgacccggtggcggtggccccggacgggcgcctgcgcgcccacgcgctgaaggtcggctggccgattctcgagcgcagctgagccgcaaggccagtgcgtcgacgcgctcgctaaacctggatcaacccccagcgcagcgccacccaggtcagctcggcctggttggcggcgcccagcttctgcttcacgcggtacaggtgcgagcccaccgtgctgagcgagaggttcagcgtgctcgcgatctgcgccaccgtcatgccgcgtgcgagctggatgaagaccgagaactcgcgctcgctgagcaggtcggccgggttggcctcgccttcgatctgcgccgtggccagggcctgcgcggtggtcgcgtcgatgtagcgctcgcctcgcgccacggccttcacggcggcaatcagcgcctcgggcgcgctgcgcttggccaggtagcccagggcgcccgcgcgcagcacgcggcgcggatggatcgtgtcttcgtgcgcggacaaggccagcacgcgcgccttggggtcgtgggccagcaggcgccgcagcgcctccaggccgcccatgccgggcatcgagaggtccatcaccaccaggtcgggccgcacctgcggatagtcctggcaggcctgctcgccggtgtcggcttcggccgccacctcgatctgcgcatcggccagcagcatgcgaaagcccatgcgcaccagcgcatggtcgtcgaccagcatcactcgaatcgtctgatccgcttggttgttcatgagttctccgtggcggccgccggcaagggcaggcgcaccttcaatcgggcaccgctgggcacggcgggttcaaggcgcaattcgccgcccaggctgtcgatgcgttcggcgagccaacgcaggccatagtgtcctacgctggtttcccttgcggcttcagggccgggaaggccgcggccgtcgtcggtgagcgtgagattcacagcgtgttcgtcgcccgcgagcgccagcacgatccggtgcgcttcgccgtggcgcagcgcattggtgatgccttcctgcgcggcgcggtacaggaccagcgccgtgtcggtatcgagccgcaggcggtcgagctcgatgtccaggcgccactcgatctccaccccgccatggctgttgcgcgtgcgctcgaccaggtcttcgagcgcggccaccaggccgaacttgtcgagcaccagcggcgtcaggcgcgggatcatgccgtgcatggcggtgtaaaggcgcgccgattcctcggcgatgagccgcgccgcctgctccgcctgcggatcgagcgcctgcacgcgctgcgcgatcgacaaggccatgctgcgcattgcggtgaccgattggcccagctcgtcgtgcagttcgcgtgcgatgaggcggcgttcctgctcgatcttctggtcgacccagcggcccagctcgcggctttcggacaagcggctttcggcccgcaccgcgcgccgctcggtttcgatgtgctgctgcagcatgcccaccatgcggttgaatgcggcgccgatggccgcggcctcggtgccgggcagggcgcgcagcgcgacgtcgaagcgcccgctctcgagctggttcagcgcatcgacgatgtcggcgaacgggcgcgtcgcgcggcccacgagccagaacacgcccgcgttgacgaccgccaggaggccgagcgcgctcagcatcagcaatgcgaagtcgtcccaggcatcgagtacggcgcgcgaggcgttggaattcaccatcagcttgccgcccggaaaggcgatggacagcttcgagggcggcggcgagaccaggccggcgaaccagtcgggcgcgtcgcggccggccttgtagaccgaggtcggcgagctgtacaagaccttgtcgtcgttgtcgagcagcgtgatgtcgttggagcgcacacgccccacgccctgcaggaacgacagcatcgccggcgtgccctgggccgcatagagccatgcggtgcggttgagcaactgcgcggccacgcggttggccgccacgacttcttcgtgcaccgattcgcgcatggcgcgcagctgcagcgcgagcattgcagtcacgaacagcagggtcagcaggctgacgatgaggttgatcttcaggcgcagcgtcatgacgcgggtccgtcgccgaagcggccgtgccgcgcgtagccgtcgagcgcggcaaccatcgcggaggccatggctggatgcgaggggtcgtgccccgcgccatcgatccatcgcagctggctgtgcgcgatgcgatcgtgcacagcctgtgcgccttcggggcggcagatgcggtcgtcgcgcgaatgcagcagcagggtgggaacctgcggcagcgcgccgaggcggtcgagcagcggcggcgcatcgagccagcatcggtgctgcaggtagtggctctgcacgcggtagcggtcgaccagtgcgtcgagcgtggcgcggtcgggttcgatgggcgtgggctcttcgtttcgtgtggccgtgccgcgcgccagtgtctgttcccagcgccaccaggccaaggcgaggcgccgcggcagatcgccggacgatgcgttcagcagcccgagagccagaaagctcagcatgtcgtggcgctgatcggccggcgccacagaagcgaagcgcgcccatgcggccggctcgcggccagccgtgtcctggaaaaaatcctcgatgtcttcagcccggggcaggaacaccgcgcgcagcagcagggccgccaccgcttgcggctcgaacgccgcatgcgcgagcgccagcgtggcaccccacgagccgccggccacgagccagcgcggcacttcgagctgttcgcgcacgtgccgcagatcgcccagaagatcggccgtgctgttgtgcgccgtcgcgccgcgcgggcggctccggccggcgccgcgctggtcgatggtgatcacgcggtaccgcgcggggtcgaagaagcggcgcagcagcggcgaactgcccgatccgggtccgccatgcagcactacggcgcagatacccgccggatcaccactttcttctacgtgcaggacgtggccgtgcgagaccgccaatgcatgggttcgccagggcggagattcggggtacaggccggtaggaagcacgggggccatggtacgcggtgaccccacggccgctattcatgaaaatcatgaagtcccattcatgatttcacggctaggtcttcgtggtccatgggttcaatatgcgtgctggagcgtacgaagttcccgcagccgccacatggcgctgtgcaacctctgcaggagacactacatgaaatgggaaaccccgacggcaactgatcttcgcttcggtttcgagatcacgatgtacgtcagcgcacgctgaattgcgcgcctcgtcacaatccgccccggcacgcccggggcggattgtttcgaacctcttctttcttcttccttttctcgatgcgcatcaccgtactgggctcggccgccggcggcggctttccgcaatggaactgcaattgcctcaattgcgccggtgtgcgcgcgggcacggtgcgtgccaggccgcgcacccagtcctcgatcttcgtgcggcccgacgacagcaccgacggcgtgctgttcaatgcgtcacccgacatcctggagcagatccgcagcagcccggtgctgcagccggcccgcaagatgcgcgacaccgcgattgccggcgtggtgctgatcgacggacagatcgaccatgccaccggtctcttcatgctgcgcgagcgcggcacgccgctgccgctgtggtgcaccgacccggtcgccgaagacctgagtcagggtaatcccgtgctgcgcgtgctctcgcactattgcggcgtggctcgccacccgattgcgctcgacggcagcgccttcgaggtgcccggcgtgcccgacctgagctttcgcgcgatggcgctgaccggcaaggccgcgccgtattcgccgcaccgcgagcatcaggtagcgggcgacaacatcggcgtgacgctcctggaccgcaaaagcggcaagagcctgttctacgcgccgggcctgggcgccatcacgccgcccgtgttcgacgccatggccagcgccgatgcggtcatggtcgacggcaccttctggaccgacgacgagatggtgcgcctgggcgtcggcaccaagcgtgcgcgcgagatcggccacctgccgcagtcgggcgagggcggaatgatcgagtggttgtcccgcttgccgccgaccacccagcgccgcatgctgatccacatcaacaacaccaaccccatcctcgacgaagattccgaagagcatgcggcgctcaggcgtgcaggcatcgaaccgtgcgaagacggaatgaccattcaactctgattcaaagcgcctcagcgcgatacgcgacaccatgtacgccgacagaatccaggacccgtttcgcgccgccgcgggcagcgacaaatccgcgccggcatggagccgcgaagaattcgaagccaagctgcgcgagcgcggccgcagctatcacatccaccatccgttcaacgtcatgctcaacagcggccgggccacacccgagcagatccgcggctgggtggcgaatcgcttctactaccagatcgcgattccgatcaaggatggcgcggtgatctcgaactgccccgatcccgctgtgcggcgcggctgggtgcagcgcatcctcgaccacgacggcttcgagcttggcggcatcaaggacgaaggcggcatcgaagcctggctgcgcctggccgaggccgttggcctctcgcgcgaagaagtgctcgacctgcgccacgtggtgccggccatgcgcttcgcggttgatgcctacgtgaactttgcgcgccgtgcgccgtggcaggaggcggtgtgctcgtcgctcaccgaactcttcgcgcccgagatccacaagcagcgcctggccacctggcccgagcactacggctggatcgagccgggcggcctgacctactttcgcaatcgggtgagccaggcgcggcgcgacgtggagcagggcctggccatcacgctcgaccacttcgacacccgggcgctgcaggagcgcgcgctggaggtgctgcagttcaagctcgacatcctctgggccatgaacgacgcgatggccacgcgctacggcgtgagcggcacatgagcggacacaaagccatgctcaccgccgaaagcaagccccgcgtcggccccggttttcgcctgcaatgggagccggcgcaagagtgtcatgtgctgctctaccccgagggcatggtgcggctcaacggcagcgcgggcgagatcatgaagcgctgcgacggcgagcgcagcgttgcgcagatcgtggccgacctggagcaggccttcgacaccaccgggctcgaacccgaggtgcgcggcttcgtcgaaatggcggcgcagcagaactggctgcgctgggacgccgcatgaccaccgcgaccccgcgccccggaccgccgctctggctcttggccgagctgacctaccgttgcccgctgcactgcgtgttctgcttcaacccggtcgactttgcgacgcaagagaacgagcttggcaccgaagactggctgcgcgtgctgcgcgagggtcgcgagctcggcgcggtgcaatgcggcctctcgggcggcgagccgctcttgcgcgacgatctcgaagtcatcatcgccgaggctgcacgcctgggctactacaccaacctgctgacctccggcgtcggcctcacggcgcagcgcgccgcggcgctcaaggccgcgggcctggaccacgtgcagctgtcgttccaggactccacgcgcgagatgaacgactttctctcgcacaccaagaccttcgagctgaagaaccgggtggcgaagatcatcaaggaccagggctggccgatggtgctcaacgtggtgatccaccgcatgaacatcgaccacatcgaccgcatcatcgagatggcgcacgagatgggcgccgagtacctcgagctggccaacacgcagtactactcgtgggccttcgtcaaccgcgaccagctgctgcccacgcacgagcagcttcgccacgccgaggaggtgaccgacgcctggcgcaagcggctaggcgagcgcatgcgcatcttcttcgtggcgcccgactatcacgagggcaaggccaagaagtgcgtcaacggctggggcagcatgttccttaccgtggcacccgatggcaccgcgctgccttgccacaccgccaagatgctgccgggcctcgagtttccgaacgtgaaggcacacagcctgcgcgagatctggttcgactcggaaggcttcaaccgctaccgcggcaccggctggatgaaggagccctgcgcgagctgcgaccagcgcgagcaggacctgggcggctgccgctgccaggcctacctgctggcacaggatgccgccgccgccgacccggtgtgcgcgaagagcccggaccatcaccgcgtggtggaggcggtggagcgtgcggccgcgcgggacccggcggcgcctaccgaacatccgctggtgttccgcgatccggccaattcgcggcggctctccgcggcgctcgtcacgccggacgcgtgaggccgcgcggcggcacgcggtcaatcgtcttcttgtcccgcttcactgggcgccgctcgcgcagccagccccgatccggcgcgaatcgccacaccagcagcagcagcgccagcagcgcgggaatccaccgcaggtccgcatccgccggcatgtgccgcgcgtagcggcggtcgagcatggccatcatcagcgcatccggcttgttcaggcgccggtagttcacgccaaccagctcggccagcgagcgcaggtggtcttgccggagctccgaaagatgctcgtggttcagcgtgccgccgatcgccgagccttgcaccacctcgtcggcccgccagtagccggcgggttcgccgttgctgccggtcttggggatcggcaccggcacgtcgccacccacgccgatcagccaacccttcacgtcgccgggcttgatgtcggtcatcggcggtgtctcgttgatgcgcagcggcggcgattcctgcccatcgctgatgaagacgaagtgggtgtccggcccgatgctgcgggccccgcgcaccgcccaggtcacgcccttgctgacgttgctggcgttgacccagcgcatgcggccgtcgatgcgttccagcgaggccagcagctcttcatagtggctgcagacttcgaccggcgtgaggatcaccaccgagcggtagtccgcaaacacgctccaccccaccttggagccgcagggcagcgcgcccagcacgccgcgcatggccgcgcgcgcgaacgtgagccggctgacggccgcatgatcgagctcgacgtcttcgacgttcatgctttgcgtgatgtcgaagctcacctgccagttgaacaccgggcgctgcagctgcacgcgcggcggccagacggcgagcgccagcaggagcagggcgagcacgagcgggccgttgccgctgctgccgccgaagcgccgcaaggcggaaaaccattgccgaaatgagagtctcacggcagatccccggcaacgaagcccggaacgcggacccggcgctgctcgtgcgcaggctgctgctcggcggagaaggcctcgtggtcttcgggcgcgagccgcagcgcgcgctccaggttgtagcgcgcgtcccagtcctgcggcgcggcgcgcagcaggtcgcgcagccgctgcttgcccagttcgaacaggggcagcgcgccggcctcttgcgccatgccttggcgcaggtacatgttgcccaggttgaacaacgcctgctgcgcgacggggtcgcgttcaccgccctggatcaggggcgcaaagcccttgagcgcggcatcgtgcgcgccggccttggacagcgccagcgcctgggccaattgcagctggcgcggcgccgagacgggcgcgggcgccgcgtccttgccgaccggcgcggcagcgatgcgggcgatctcggcgttcaggcccattgcctggcgcaggcgcagcccgcgctccagcgccacgccggcgcagcacaggctcacaacgccaaagaccaggtgaaccgtacgtcgtttcatgtgtttttccgccagctctgcagctgtaccgcgcggcaggcgagcaggcccgcgcagcacagcatcgccgccagatagaacgcggcgccatggtcctgccgcggtacccgctcatgaatggtcagcggaaaattctgctgccggtcgatctcggccatggctgccgccatcgcattggaatcgtccacctgatagagccggtagggtgtgcggagcgtcttgaagaactggtgcagcgccagttcttcgccgaggccgtaggccgacaccgtctcggtgttgaggttgggcgagttcgggccgctgcgcacgtagatccagtacaggccgatcttctcgcgcgcaaggccggcatggacgcgctggcgcgtggcttcgtcgagctgggcgccgccatccgagacgatcaggatcacgcggcttcccgaatagctgcggccctcgaattcctcgatggcggccagcagcgcagtacccatgcgggtctcgggcaggccgcggccgatggcggtggcggcgagcgcggcctgcacggtgtcggccttctgcgtgaaaggcacggccacgatcggcaccgtgctgaaggtcatgaaggcaaaacggttgtcgggccgcttggcgacgaattcgcccagcaggtcgcgcacgaccttggccttgggttcctgcgacatccggcccgcggtctgcaggccgttggtgtgcacggtcgcgtccatgctgctgctgcggtccatgaggatgagcacctccgcgccgcggccggggcgctcgaccacggcgcccgattgccccggtcccgcgagcccgagcaccgtgaaagccatggcgcccgccgcaaaggtgcgccacatgaaacccaccaggcggccgacccgatcggccggcagccaggccaggtaggagaagcccagcgtgtcgctgcgcctgcgcagcagcggcagcagcgcgagtggcagcagcatgagcatccagggctgggcgaggtcgaagcgcatggttccggcggctgtcaatgcctgtggtgcttttccgcattgcgcaagtcacggcacagcggcctgagcgggtaggcggcttgcggccgggccggcgcggcaacgctctcggcaaagaagaagcgccgcgtcgactcgcgatagaaatcctctaggcgcggttgcagcgggcgcaggtagggtgcgtcggccagcagctgcggcaggctcgcgccatgcaccacgcggccggcgctcctgttcaacgcccgatgcaccacgcgccacgcctcggggctcgccgggtcgtcgatgcggttcagttcgcgccaggcattcgcgaatggaagctgctgcacttcgcgccggttgcgccacgcccaccagccgagccacgcagcgagcaccgccagcagcgcaagaagcgagaacttcagttgctgctcgacggcaaaggtgggaagcgccgcgacggggcggtccggccgcagcggctgcaggtcgccttcgcccagcagttcgagcggtgtcagcgggccgatgctgatcggccatgcaggcagcgccagcgccgggcccgatgcggtcgcgatgctgagcgccggcaacgagatggcggtcagcgcgcgcggggcgttgacgacctggtagtcgatggccagccagcgccgcccctcggcatcggtctcgatgcgcgacggcctgcgttccagccagagatcgatccgcgccgcgctgggcaatgcgcctggctgcagcggctggccggcctgctcgagcagcacgcgctgcgtgagcacgtcgccgatcacgtggccgaaggcgcgcggctgctcgacggtggccgcggttgctgcgcccgccgcgccggccgtcatgaccagcgccagcacggcggcgtggagccggttcatgccgtcgtctccatgaagtagcgcgtgagcgcctcggcatcgaaacggccatgcagatgaaagggcggcatgccatgcgcttcgaacaaggcggtgagctcggcgcgccgcgtggcgaccgcgtcgcgccaccgcgtgcgcagcgaatcgcgcatccacaagctgcgccgcacgccggtttcggcatcgctcagggcgaccagcgcgcgcgcatccggcggttcggtttcggccgggtcccagacgaccagcggaacgacgcaggccggcgcgaactgctcgagcagttctccaagtgcggcaatcggccagtgaaagtcggaagccagaaacaccagaccgccgcggccgaccaggcgttcggtggcgcggcgcaaacctgccagcgcgctgtcgtccatgaggggagcgccgggtgtggcgcggcagtcgcgcagcatccgcgccatcaggctgccgttgccgcggctgtgacgcgcgggcacgaacaaatcttcgcgctcgcggtggtcgaaggccagcaggccgacggtgtcgccggcacgaaacgcgctgtagcccagcgcctcgaccaggtcggccaccacgtcgagcttgcgccgctcggcgccgaaatgcatcgacgccgacacgtccaccaccacgtgtacgggaatggccacgcgcagccggtggatgcgcactagccagtcgccgcggccgtcgcgcacgctggcacgcaggtcgatgcgccgcgggtcgggatgatcgaacaggcgccggtgcgcagcaaattcctgcccgctgccctggctcagtccgcgctgcgcgcccggccgccagccgccgaagcggcgcggcagctggtagtggaattcgtcgaagcgctccatggccggctcggtatgtcagggggctgcgatcttgtccatgatctgcccgaccagtgcctcggataactccgcccggcgcaactcgtacaccggcgtgaagaacacgcgatgtccgagcaccgagggcagcaccgccgcaagatcggccggctccaggtgcgagcgcccctcgagccaggcgaccgtgcgtgccgcgcgcagcagcgcgctcatgccgcgcgggctggcgccggcaaggatcaggcggtccatgtcgacgttgtcgagccggatgccgaacttctgcggtgcctcggtggcttcccacacgtcgagcacatagcgttcgatggtctcgctggcgcgcacgctgcgctgcacttcggcgccgatggcgttgagccggtcccagagcaggatggccggggccaccttgtcgatcaggctttcggtgtcgtggtaggcggtgtcgaacaccagcgactggcgaatgccgcggtcgctgggcttgggcatgttcagctcgaacatgaagcggtcacgcgccgccgaggccagctcgaaggtctcctcgcgctcgaccttgttgcggtcggcaaacaccgtcatgtgtggaaagctgtactcgcggtcgaaggccgagaccgtgcgctcggccatggcgcgcagcagcagcgactgcacctgcggccgggcccggttgatctcgttgaagaagaaggtgaccaggcgctcgccgtggcggagcaagggccccgggtcgatgcgcggccggccttgcgcgtcgacgtaggtgtgatagaccagatcgcccggcatcaggtcgaccgtgccctccacgcgctcgaagtcgccgccgatggcgcgcgagaaggcgcgcagcaccgtcgtcttgccgacccccacgtcgccttcgagcagcacgtggccgcgcgcgaacagcgccacgttgatgaggcggatcgtctcggcctgcccgatgatcgccttcgcgacttcggtttcgacgcgcagcgcaaggcgccgccagtcttcgagttgttcttcgttgcccatggtgtgcctctgtcgtgcgatgccgcgggctatttcgattccatcatcttcttcagattgccaaggccgctgcggtagacgtcagtgacggccttgagcgcggcttcgtcgttctggtcaggcggggggttgttgttcggaaaggcgcgatagaaggcgccgcgccactcgacgacggacttgccgccgtccgccaccaccgagagggtggaggtgtagttggtgaccggcaatgcgccgccatccttggcgcggtagctgtacttcttttgcgcatcgtcgaagctctcgatcgtctcgaccagcgtgccgccgcccttgagcttgagggtccgcaccgagccttcggcgttgcccttgtcggacgggctttctgccaccgccgggtgccagtctttcagcgcattgaaattcttgatcttggcccacacggcgtcggccggcgcctcgatggtgaccttctcgctcaccttctggcgcgtgggaccgtgggccaggccgggagccgacgcggccaggagaacggatgcgagaagggcggagagggcccgtcggctggaaggatgtgtcggcatggaaacgtccgtgatgaagaatgagaaaggtcggtcgaaaaaattcagtggtccatcggcgcgccgatgaaggcgccgaacccgcggctgttctgtcccgtggcaatggtcttgagcttctgtccgctggcggaatcgagcacctgcacgttgtcgtccatccagttcacgacgtacacgcggtcggcgtgcgcggcaatgccttcggggtacgcgaagccggggagggtgcgcagcaccttcagcgaggcggcgtcgatcacgctgaccgtgtcttcgtgctggttggtcacgtagagcagcgcgccgccttgggcaagcgccgcgccgtagggcgccttgccgaccttcacggtgccaatgacggagggccggcgggtgtcgcgcatgtcgaccaccgagacgtcgttgctctgcacgttgagcgcatagaggcgcgagcgcggggcgtcgtagagcagcgcgaacggatggctgccgacgcgcacgcgcgccagcacgcgccgcgcacgagcgtcgaccacggccacgctgtcgtcgtcgcgctcggccacgaacaccgtggtgccgtcagggtgcgcggccacgccggcgggtgcgcggccgaccgcggtcgaagccaggggctttgcggcattggcagcctgcgcatcgaacgccagcagccggttgcggtaccaatccgccacgtacaagcgctttccgtcgcccgagatgtcgatgccgaccggaccgtcgcccgccggcagcgtgttcacgaccttctgccggcgcatgtcgatgaccgatatggtcttgctgtcggggttggacacgaacactcggcccgcgcggcttgacgccaccacgcccgctggcgagcgcccgacgggcacggtggccaccacgtgctgcgttgcaaggtcgatcaccgacacgtcgtggctgccctggttggtgatgtaggcgaagggcgcagccccggccgacgcgcagcagaacaagaccgcggcaaccccggtgcgcacaggtgttgcggagcccgtcatggcgatgtgcccgagccgtggctcagcgcgcggtgggagggccgatgaagcagcccttgttcaccttggcctgcagcgccttgtagcgcttgatgtcggcctgcagtttttccgagtcgcggatatagccgccgcgctcgccgccgatggtggtggccttggccgcggtgctcaggtccacgtattccgaatacttgatctccttggcgatggcgtcgaccgcgcaggagcacttgttcgtcatctcgaagcggcccgcgtccggatgcgcggcgatgcattcctgcacgtacagcacacggtcgacggtgggaaagtcgttcgcgcgctgcggggcgccatgcacggccatcggcaggccgagaaggcaaagaaggcggaagatttttttcattggcgttcgctggaatttcgagagagagagatgcggcactatcgcgccggcgccttggccccgtcgatgaggagttcctcgacgaccaggggctgggctgctgcgctctcgcccggtatggaggtgcgaatgccgtagacaccgcccggcaccgcgtcggacagcgtgaagcgataggtcttgcccgcgaacttttcgtacttcggccggttggggtcatcgaggaaagggctgaacgcgatctccttgcccttgaccgtgcggccctggtagcgcagcgacacgtcgcgcacctcggcgtcctggtagatcgccatgcggatgcgcttgcggaagtgatactcggagccgcgcgtgatgcgcttcatttcgcgcacgtcatgctccagaaaataaaggatgacggggttgccctcggcggccggcacgtcgggcaccgcgatcttgcgcgcgccgctcaggaacacgcccttggcgtcgcagcagctgccgtcggccttggcgatcagcgccacggtgacgttgtcggcaaaggcttcttcgaagctgccggtcttgccgaagttgtagcgcagcagcatgggcgcctgcagccccttcagctgcggcgtcatgaagaggaggcgctccgcggccgagaagtcgcgcttgtcggcctcggcatgcggggccaggggagcacagagcagggcgcagagcgaaaagcggagcggaagggcaatggcgaggcgcatgaaagacctggtcagttgttgggcactccgaacgatgcatcgaccagcggaacgccgaactccttcaggatggcctggatctcgggtgccttggattcgatcagcccctcgatctgctgcttccattcgcgttcgccgtagcgcacgcccatggccatctggtagtcgagccgcaagcctttttcggacttgagcggcaccacgacgagcgcggggttcttgacgcgccgggcaaagaaaccggcaatcggcccccagaccaggacggcatcgagcttgccttcggccaggtccttctcgacgatctcgccggggtactgtgcggggtcggcactcatgagcttgtacggcacgccctgttcgagcaggccgtgtttgttgagccattgcgaagccggcgaacggtcgtagatgccgatgcgcatcgacttgagcttggccggatcgagcttcaggaaatcttccgccgaagccaccttgtccatgcccttgccctttggaaagaccagtgcgtaggtcgagcggtagtagggcttggtgaccgagacttcgtcgagcccgacgggcacgcccatcacgatgtcgcacggatagtcctgccccggcagcttgtagcgcagcgtgttgcgaaagaatgccagccgctgcggaaacgagtagtagacgaccggcagacccagcgtcttgccgaacagctcggcgatgcggttctcgatgccttctcccttggtgttggagaagggcatgttgttggggtcctggcagacgcgaaactccttgcgtggagggctctcctgggccattgcgggaagcagcgcgcagcagcatgccgcgcccaggaggcccgcccgcaggcgagcgccgaagggggtgggcctgccagcacgcggccgggcggtcatttgttttcttccacgcgggcgcgcgtgatcgcgccgtcggaccggcccttcaggtaggcgtagagctggttgatgttttccatcaccgcagggttgttgccgaagctctgcatgcccttgtcgagccgcccgtcgcgcacgaccttgacgaagtcttctttcttcattgtcttcaggctgctgatcagcgaggggccgaccatgccttcctggttcgggccgtggcagcggtcgcaggccgcggagcgccaggtgcggaaacccttcatggtttcaggatctaccttgtagccatcggtgactttgtagggcgccgggtccggcgcggcggcgacggccagtgtgcaggcgacgccggcaagcagtacgagggaaggcagcaacgttgacttacgaaatttcatggctcctgggtctccggtatcttttgaaagtacgggggagagcgctccagcgagtgctctcccgatccgcatgctgcgtctatctattgatgatggacgcctcggtcataacgcttcacttgggcagcgcgaagacagtcagcgagccgccgagttcggtgtactggctcagctccttgtagccgccgacggcgccgaggccttcggtgctcttttcggggtcgatgcccgcggccatgccgatgccggcccagccgccgatgcccgagaacacaccgatgtattgcctgcccttgtgctcataggtgaacacgttgccgatgatccccgacggggtcttgaacttgaacagctccttgttgatgtccttggcatccacgcacttcaggtagccttcgagcgtgccgtagcaggagatcccgccggcggtgttgagcgaaccgctccacaccgagaacttctcggccttggtctgcacgatcttgccggtgcccgcgtcccaggtgatgaagttgcccatgccgccatggctgcccggcgtggggtacatcgagagcgtggcacccacgtacggctggcccgccgtgtactcgaccttgaacggctcgtagtccatgcagacgtggttggtcggcacgtagaagagcttggtgttggggtcgtaggaagcgggttgctggtccttgctgcccagcgcggcggggcagatgcccttggtgttgacgtcggcgccgttctgcgcggtcgagtacttggcaaccacctgcggccggcccgtcttcatgtcgacgtgcgtggcccagttcaccttggggtcgtacttctcggccaccagcagcgcgccggtcacgcggtccagcgtgtaggcgaagccgttgcggtcgaagtgcaccaacgccttggtcggcttgcccttgacgttgatgtcggccaggatcatttcgttgatgccgtcgaagtcccactcgtcaaagggcgtcatctggtagacccagttgaccttgccggtgtccacatcgcgcgagaagatgctcatcgaccacttgttgtcgccgggccgctgcgcagggttccaggtcgacgggttgccggtgccgtagtacacggcgttggttgccttgtcgtagctgtaccagccccaggtggtgccgccgccgatcttccactggtcgcccttccaggtcttcagcgatgagtccttgccgacaggcgcgagcttgccgtcggtccaggtcatggtcttggccgggtccatcagcatctcgtcgtcgggacccgtgctgaagcccttccaggccagcttgccatccttgacgttgtaggcggccaggaagccgcgcacgccgaactcgccgccgctgatgccggtgatgaccttgtccttgaagacgtggggcgcgttggtgttggtggccccgaccttcggatcgccgttcttcaccgtccacaccaccttgccggtcttgctgtcgagcgcaacgagcgtggtgtcggcctgttgcaggaagacctttccttccgcataggcaaggccccggttcaccgtgtcgcagcacatgaccgcgatcactgactgatcctgcttgggttcgtacttccacaggattttctgggtctcgacgtcgaccgcgaacaccttgttcgggaacggcgagtgcaggtacatcgtgccgtcgaccaccaggggcgagccctcgtgaccgcgcagcacgccggtggagaacgtccacgcgacctgcatcttgcccacgttgctcttggtgatctggttcaacttgctgtagcgctggttgaacatatcgcccgcttgcgtggcccagttcttggagttggcgatgtttttctccacgtcggcattggcaagcgccaaagccggaagagccaacatcgcgacgccgatgtgccgtacaagacggccggcgatctgcctggaaaacttcataaatgtctcctcacatttcagtgggtttcgaacacgatcatggcagcacccgcggatctttcgatcgctttggcgaatgctgcggtccgcaacatccatgcctgccagttccagcacggagcacgtcgaagacccatgtgcgctccaagcgaagacacacgattccattcggaagaggcgtgcgcgacacagcgttcgcgcagcatgcggcggcctgccgcaacgcgatcagaacctagggaaatcccgagcgttcgatgcgtggtcccgcgccggacgccatgcattgccgcggccttgcaacgggtgcgcatccaaatttgacgcaaagtgtctcgtgcgaagtacggctgcacggcgcagagaggcgcaaaggcacctgcgcggccgttgggaagcgacctggcacagtgaaaaccctcgtcgcgcagaggcacagaatttgcgaattgaatgcgaacggcaaataccatcggagcccgaactgctcgacacatcccaccggcctacatgctgcgaaccatcgacttaaccaagcgctatggcacgcgcacggcgctgcaatcgttgtcgctgcgtttgcccgcaggccagttcgtggcactgctcggacccaacggcgcgggcaagtccacgctgttccaggtgctgaccggcatgttcgcggccgacgagggcgaagtcgaagtggcgggccattctttgcgccgctccgccactgctgcgctgcggcacatcggcgtggtgttccagcagatgtcgctcgatctggacctgagcatccggcgcaacctgctgttccaggccgacctgcacggcctgccgcgtcggctggcgcaagagcgcattgcgtcggcgtgcgagcgcctgaacatcgacgccgacctggaccgcaaggtgcgcgaactgtcgggcggcaaccggcgcaaggtcgaactcgcgcgtgcgggcctgcaccggccggccgtgctgctgatggacgaagccacggtcgggctcgacccgaagtcgcgccaggatctgctggccgcattgcatgccgacgtgcgcgagcgcggcgtgtgcgtgctgtgggcaacgcaccgggtcgaagaagccgaggaggccgaccgcgtgctcgtgctgcacaagggctccctgctggcggacggcacgccggcggaggtgtgccagctgctcggcggcgccacgctcgaggcaggcttcatcgcgcgcaccgcctgaaacaagaagaaatccgagtcagaaaaatggagacatcgcatgccgcaaccttccttcctttcgcatcccggcgcgctcgttcgcgcggcctgtagccgcagcgcgctctcactggtgctggccgcggcgagcggtgccgcgctggcgcagggcaccgcctatgtgtcgagcgaaaaggacaacgcgctcacgatgatcgacctgggtaccctggcggtgaagggcacgatcccgacctgcaagcgcgcgcgccacatccagctcacgcccgagcgccagatcatggtggcctgcaccgactccaaccaggccgacctgatcgaccccgcgagcggcaagtcggtgcggcggattccgctcggcgacgaacccgaggccttcgacctctcgccggacggcaaggtgatctacgtttccaatgaagatgcgggcgaggccagcttcatcgatgtggccagcggcaagaagctgcgctcggtcaaggtgggcgcggagcctgagggcgtcaaggtcagcgcggacggcaagaccctgtacgtgacctcggaggtggcgagcctcgtgcacgtgatcgacaccgccagcggcaaggtcgtgaagaacatccgggccggcaaacgcccgcggcgcatggccatcacgcccgacggcaaggagctgtggatcaccaacgagctgggagccagcgtcagcatcgtctccaccgccacgcacgaggtgatccacacgctgaagttcgaagtgaagggcgcacgcgccgaagacatcacgccggtcggcatccagatgacgagcgacggcaagcgcgccttcgtgggcctcggccgcgccaaccacgtggccttcgtggacgtgccgggccgcaaggtgagctcgctggtgctggttggcaagcgggcctggaacgtcacgctcgacaaggcgcaggcgcggctctacgtggtcaacggattgagcgacgacgtcaccgtggtcgacgtggccggcgcgaaggccatcaagagcgttccggtgggacgcgtgccctatgggctcgtgatcgtcgaatgaggctgcgcgcaacggtttgccggttgtggggcgcgtggctggccgtggtgctcgccgggccctttgccgtggacgcggccagcgcggcggtgctcaaggcgacactgatcacacccgccgacgatccgcgcatggagcgtacgcgcaccgagcgggcctacctcggacaccccggcggcccgctggcggaaggggtcgaggtggggctcgacgaggccaggttcgagctcgacgcggccggtgccgaggtggcgctggcgacggcgccggcggcctcgctcgatgcggcgcgcgctgcggccgtggcggccgagaaggctggcgcggcggtgctgctgaccgatctccccgccgactggacgctggccgtggccgatgccgtgaagctgccggtgctgaacctcagcgacgcatccgaccgtctgcgccagaaggactgccgcgcccgcctgttccatctgattccgagcgaacgcatgcgcagcgatgcgttggtgcaggccctggtgtcacgcaaatggagcaaggtgctcctgctggtgggcggcagtccgcaagacgcgatgcgcgcggccaccgtgcaggcgtcgatcaagcgctacggcctgcaggtggtggccagcaagcccttcaagctctcggccgacccgcgcgagcgcgatctggccagcccgctgctgctcacggccggcaacagctatgacgccgtgtgggtggtcgacagcgacggcgaatttgcccgcacgctgccctaccgcaccgtgctgccgcggccggtggtgggcgacggcgggctggtggcgctggcctggcatgcgcagttcgaacgttacggcgcgccgcaggtgtcgcggcgttttaccaaggtcgcccggcgcccgatgaccgcgcaggactgggccgcgtggatggccggcaagaccctggcggcagccgccatcggcgcgcccaagggcccgaacgcggcgtgggcgcaggccatcgccaagggcaccctcgacggttccaagggcaccaacctgagcttccgcgcatgggacggccagttgcgccagcccatgctgctgagcgacgggcagggcgtggtctcgcaggccccggccgagggcatgctgcatccgcgcgacgtgctcgacacgctgggcgccgacgcaccggagaagctatgtccgatcgcacgctgaagacggcaaagacccccgcgggcgaaaacgccgagccgctggcaaggcggggcgtggctcatgcgctgcaggcgatgcgcgccatcatgctgcgcgagctctacaagttctcgcagcagaccgggcggctggtgtcggcgctggtgcggccgctgttgtggctggccgtgttcgcggcgggctttcgcaacgtgttcggcgtggcgatcgtcgagccctacgacacctacattccctacgacgtctacatcgtgccggggctggtcggcatggtgctgctgttcaacggcatgcagtcgtctctcgccatggtgtacgaccgcgagatggggttgatgcgcctcctgctcaccgcgccgctgccgcggccgtggctgctgttctccaagctctgcgccacggcgctgctgtcggtgctgcaggcgctggccttcgtgatcgtggcggcgctcatcggcaccgagctgccgctgctgtcactctccgggctgcatgcgctggtggcgctggctgccggcgcgctcatgctcggcgcgctcgggctgctgctgtcggtgcacatcaagcagctggaaaatttcgcgggcacgatgaacttcgtcatctttccgatgtacttcctgtcgaccgcgctgtatccgctgtggaagctgcaggagtccggggccgagtgggtgtaccagctggcgcgtttcaatccctttacctatgcggtggagtggatccgattcgcgctctacggtaaggacccgggccttgcgccctatgtggtgcttggctgcctcgcggttttcttcggcctcgcgtgctggggctacgacccgcagcgcggcttcggcggcctgaccaagcgcggcggcggaggcgggccatgaacgggcagggcgctgccacccggcgccgctggctgcgcgatgcgggcgcgctggcgctgggcgcattgccgctggcgcgcgcgttggcgtcgaccgagccttttccttcccgtccggtcacgctctgggtgccctggcccgcgggcggcgccaccgacatctcgctgcggatcctggccgagctggcctcggctgcgctgggacagccggtactgaccgagaaccgcggcggtgccggcggcacgctggccatgccggtgctgcagcaggcgcggcccgacggctacaccatcgcgcaaatgccgcagccggtgttccgcgcgccgcacacgcaaaaggtgctgtgggatccgatccgcgacgtgacgccgatcatccaggtctccagcgtgaccttcggcatgctggttgcggcgggcagcggcttccgttcgctggaagacatgttcgcgttcgcgcgtgcgcggcccggcgagctgaccattgccaccaacggcatcggcaccacgccgcacatggtgctggaggcgctgttcacggcgcgcggcctgcgctacatccacgtgccgtacaagggcacggccgagcagctgaacgcgattgcgggcggacaggtgatggccggcgtcaactccaccggcttcgggcccgcggtcgactcgggcacgctccggctgctggcgatcttttcgggcgagcgctcgaagcgctggccgcaggtgcccgtgctgcgcgagctcggcttcgacatcgtggccaagtcgccgtatgggctggccgggccgcgcggcatgtcgcgcgcggtggtcgcggcgctgcacgacgccttcaagaaagccatgttcgaccagcgcttcaaggacgaactggccaagtacgaccaggaggtcgactacctcgggccggaggcgtatgcgcagtcgtgccgcgagatcttcgcgcaggagcgcgccatcgtggagaaactgggccttgcgcgcatcggcacctgagggggaaagcaccgtgatccgaccgaccaagcaaacgagccgccggctgatcggccttgccgtggccgctgcggcctgcccgataccgggacaggcgcaggagaccgcgccgcaggcgggcagcctgccgaccgtggaggtggtcagcaccacgcccgtgccgggcatcgaggtgccgaaggatcagattccgtccaacgtgcagaccgcggacgatgcgcacctgcgccgcgcgcagagcctgaacctgcccgacttcctggccacgcagatgccgagcgtgaacgtgaacgagatccagggcaacccgtaccaggtcgacgtgaactaccgcggcttcagtgcgagcccggtgctcggaacaccgcagggcctgtcggtgtaccaggacggcgtgcgcatcaacgagccctttggcgacgtggtcaactgggacctgattccgaaggcggccatctcgagcatcacgctgctgcccggctccaacccgctgttcggcctgaacacgctgggcggcgcgctgtcgctgcagaccaagcggggcgacacccatcccggcaccgagctggagttgcaggccggctccttcggccgcgtgagcacggagctttcgcacggccgcaagctggccgagggcgggcacctgttcctcgcattcggcggactcaacgaagacggctggcgcaactactcgccctcgcgcgtgcgccagctgtttgccaaggtggggcaggacagcggcaaactctcgtgggacctgagctttacccatggcgacaaccggctggtgggcaacggcctgctgcccgagtccatgctgatgcagaaccgcaagcaggtctatacgcggcccgaccgtaccggcaaccgcatgtcgatgctcacgctcaatggcagctatcgattgagcgaccagcagacgatctcgatgaccgcgtacacgcggcgttcgcgctacagcacgctcaacggcgacctgaacgacgatttcgatccggccgagaacggaaattcaggcgtggagaaccgcacctacacgcgccagcacggcgaaggcgtcgcgctgcaatcgacctataccgctggcatgcatcagctcaccttcggcgcctcggtggaccgcgcgcgtacgcactttttgcagaccgaggccgaaggcctcctcgacgcgacacgggccgtggtgccacacgaagaagccgaggtgaatgcgctgcttgcaggcaagagccgcaccgcaagcgtctatttttccgacctggtaacgctgcggcccgacctgcagctcagcctctcgggccgctacaacaacacccgcgtgacgacccgcgacgacgggcgcgccttgctcggactcccgacccagctcgacggcgaaggccgctacaagaagttcaatcccgcgatcggcctcacatggcaggccacgccgcagctcacggcctatgcgggctggagccagggcaaccgcgcgccgagcccgatcgaactcggctgctccgatccggcaaacgcctgcgtgctgcccaatgcgctgcagtccgatccgccgctcaagcaggtggtgtcgcagaccttcgagaccggcctgcgcggaactttcgccaaggacttgcgatggaatgcatcggtgttccgcacggtcaacaaggacgatctgctgttcatcagcagcgggctctcgcgcggctacttcagcaacttcggccgcaccctgcgccagggcattgaactcggcctctcgcagcagaccgagcgcgtcgactggtcgctgtcgtacagctacctgcgcgcaagatacgactccccggcgtgcctggtggccgaagcgaacagcagcgcagagaccagcgccgcctgcaccggcgaaggcgaaatcgcggtgcggcgcggcgatcggttgccgggcctgccggcgcattcgctcaagttcaacgtcgattggcgcgtgacgcccggctggaccttgggcgcgcagtaccgcgcctattcgcggcagacggtgcgcggcaacgagaacggcctgcacacgcccgacggcgacgctttcagcggcagcggccgcatcggcggctatacgcttctcgacctcacgacgcgctggaagctgggccgcaacgtggagctctttgccaaggtggcgaatgtgttcaaccgccgctatgccaccgccggccaactggggcgcagtggcttcgatgcgaacggcgcggtgctggcgccagatgcatggcgcaatgcgcagttcgtggcaccgggtgcgccgcgcgcggtgtgggtcggcgtgcggatgcagctcggggtctgaggccgcgcgccgaaaggctcaggcggtgcgccgcgcgctgcgtttttttgcggcggggcgcgcagccggcagcgtgccgagctgccgcaggatctgcgcctggccgtgcgtgcgcaggtaatcctcgaacgccagcgccacctgcggcagttgccgcgacgccaggtgcatcacgtaccagtcgcgcaccacgggattgcccggcaccggcagcacgccgaggaggccggcgttcatctcgagcacgcaggtgtgcatagacagaaaggcgatgccgaagcccgcggcgcacatctgcttgatggcctcgttgctcgacagctcggagccgatgcgcagcggcaggccctggtccttgaaaaagcgttcgaccgtggtgcgcgtgcccgagccgcgctcgcgcaccagcatgcgcgtgtccgacagcatggcgagcgtgggcttgggcgccgacatcagcggatgagagggcgccgcgagaaaggccatcgggtgcttggcgaaggcgctggaatcggttttcagctcggcgggagggcggcccatgatggcgatgtcgatctcctggcccgcgagcatgcgcacgatttcgtcgcggttgccgacctgcagcttgaccttcaccttcggatgttccttggcgaagttcaccaggatgggcggcagcaggtattcggccgtggtgatggcacccacgcgcagcgtgcccgagaacacgccctgcagcatggccatttcgtcgccggcctcgcgccacaggtcgaggatgcggccggcataggcggccagcagttcgcccgcctcggtgaggcggatgccgcggcccgtgcgctgcaacagcggcgtgccggccgactcctcgagcgtaccgatctgaatcgacaccgcgggttgcgtcaggtgcatttcgtccgcagcaagtgaaacgctgccgagccgcgccacggcgtggaaggtggcgagctggcgaaagctcgcgtgcttggaaagaggcatgcagtgatattaggtttgataaatgtgaatgtcaaaagatctaatttttctttatctgtcatgcggcctacattcacttcaccgacagcaccaaaccccttcactcgagaggcactccatgggcaacatgaacgaagcaatccagatcaccgacgccaagaagcgctactcggccggtgtgctgaagtatgcgcaaatgggctattgggacggcgactaccagcccaaggacaccgacatcctcgcgctgttccgcatcacgccgcaggatggcgtggatgcggtcgaagccgctgcagcggtggccggcgaatcgtccaccgcgacctggaccgtggtgtggaccgaccgcctcaccgcctgtgacatgtaccgcgccaaggcctacaaggtggagccggtgcccaacaacccgggccagtatttctgctacgtggcttatgacctctcgctgttcgaagaaggctccatcaccaacgtcacggcctccatcatcggcaacgtcttcagcttcaagccgctgaaggccgcgcggctggaggacatgaagtttcccgtcgcctacgtcaagaccttccccggcccgccgaccggcatcgtggtggagcgcgagcggctcgacaagttcggccggccgttgctgggcgccaccaccaagccgaagctcggcctctcggcccgcaactacggccgggtggtgtacgagggccttcgcggcgggctcgacttcatgaaggacgacgagaacatcaactcgcaaccgttcatgcactggcgcgaccgcttcctgttcgtgatggacgcggtcaacaaggccagcgccgccaccggcgaggtcaagggcagctacctgaacgtcaccgccggcaccatggaagagatgtaccgccgcgcgcagttcgccaaggagctcggctcggtgatcgtgatgatcgacctcgtggtcggctacacggccatccagtcgatgagccactggtgccgccagaacgacatgatcctgcacctgcaccgcgcgggccacggcacctacacgcgccagaagaaccacggcgtgagcttccgcgtgattgccaagtggatgcgcctggccggcgtggaccacatccatgcgggcacggcggtcggcaagctcgagggcgacccgatgacggttcagggctactacaacgtctgccgtgacacgcacaccaaggtcgacctgccgcgcggcatctacttcgaccaggactggggcgcgctgcgcaaggtgatgccggtggcttcgggcggcatccatgcagggcagatgcaccaactgctcgacctgttcggcgacgacgtggtgctgcagttcggcggcggaaccatcggccatccgcaaggcatccaggccggcgccacggccaaccgcgtggcgctcgaagccatggtgctggcccgcaacgaaggccgcgacattgccaacgaggggccgcagatcctgcgcgacgcggccaagtggtgcacgccgctggccgccgcgctcgacacctggggcgagatctccttcaactacgcctctaccgacacctccgactacgtgccgacgccgtcgatggcttgaacacacgttccccgttccgcagttctccaggagcaacagacatgcgaatcacacaaggcactttttccttcctgcccgacctcagcgacgagcagatcagccgccaggtcgagtattgcctcgacaagggctgggccatcggcctcgagtacaccgacgacccgcatccgcgcaacaccttctgggagatgttcggcaacccgatgttcgacatcaaggatgcggccggcgtgatgctcgaactcgcgtcctgccgcaagacctttccgcagcaatacatccgcgtgaccgcgttcgactcgacgcacggcaccgagtcggtggtgatgtccttcatcgtcaaccggccttccaacgagccgggctttcgcctcatccgctcggaggagccgggccgcacgatccgctacagcatcgaaagctatgcggtgcaggcgcggcccgaaggcagccggtactgagctgagcgaaccccgccgcaaggacattgccagaggcacgcatggacgccaccgaaacccccaccgccccggccgttgccacggcgcccaggcagctcttcgagtcttcgggcgtgaaggcgctgctcgaccagctcgacgccgagctgatcggactggcgccggtcaagggccgcattcgcgacattgcggcgctgctcctgatcgacaagctgcgccaggagcaggggctgcagtcgcagccgccctcgctgcacatgtcgttcaccggcaacccgggcaccggcaagaccacggtggccatgcgcatggccgaggtgctcaagcagctgggctacgtgcgcaagggccatctggtggcggtgacgcgcgacgatctggtggggcagttcatcggccacacggcgcccaagaccaaggaagtgatcaagaaggccatgggcggcgtgctgttcatcgacgaggcctactacctctaccggccggagaacgagcgcgactacgggcaggagtcgatcgagattctgctgcaggtgatggaaaaccagcgcgacgacctggtggtgattcttgcgggctacaaggaccgaatggagaccttcttcagcagcaacccgggcatggcctcgcgcattgcgcaccacatcgattttccggactacagcgaagccgagctgatgcagattgcgcagctcatgctgaggcggctcaactacagcttcgacgacggcgcggcttccaccttttcgcgctacgtgagcctcaggcgcagccagccgcactttgccaatgcgcgatcgatccgcaacgcgctcgaccgcatccggctgcgccacgccacgcgcctcttcggcagcgaagaggccctgacgcgcgagcagctctgcacgctgcaagcgcaggacattctcgcgagccgcgtcttcaatccaccggcggccacctcgcagaacgaaggagcagcacgatgagcatcgaagccctcgtattcgacgtcgatggcaccttggccgacaccgaggaagtgcatcgcatggccttcaacctcgcgttcgagcagctcggcctcggctggcactgggcgcaggccgagtaccgctcgctgctgtcggtcacgggcggcaaggagcgcatgaagacctacatcgattcgctgcccctgggtgcatcggagaagaagcggctgcacgagcgggtgccggcgatccatgccgccaagacgcagcactacaccgacatcgcgcggcgcggcggcatcgagctgcgtcccggcgtgctgcgttttctcgaagaggcacaggacgccggcttgcggctggccattgccagcaccaccacggccgtcaacatcgatgcgctgctgcaggccacgctcggtgcgcgcggcctcgcgatgttcgacgtgatcgcctgcggcgaccaggtgcgcgccaagaagccggcgtccgacatctacctgctggcgctcgacacgctcggcgtgccgcccgagcgcgcgatcgcgatcgaagactcggtgaacgggttgcactcggcgctcggtgcaggcctctggacgctggtcacgcccaccttctggaccgacggcagcgatttcagcggcgccggcctggtgctgcccagcctcggcgaccctggccagccactgcccggcgagcccggaggacgccttgcgttttctgcgtggctcggcatcgaagaactcctgcggatggccagcgtggccccgccattgaatgccgtgcaggcgctttaccgtgagggcagctagatgcagaaaaaccaaaacgccatgcggatcgcgccaagcctgctgtcggccgacttcgcgcggctcggcgaagaggtcacggcggtcatccaggccggcgccgatctgatccatttcgatgtcatggacaaccactatgtaccgaatctgacaatcggtccgctggtgtgcgaagccatcaagccctacgcgacggtgccgatcgacgtgcacctgatggtcaagccggtcgatgcgctgatcccgatgttcgcgcaggcgggcgcctcgatcatctcgttccaccccgaggccagcgagcacatcgaccgcacgatccggctgatcacggccagcggctgcaaggccggcctggtgctcaaccccgccacgccgctgcagatgctcgaccacgtgctggaccagctcgacctggcgctgctgatgtcggtcaaccccggcttcggcgggcagagcttcatcgagagcgtgctgccgaagatcgaggcggtgcgccgccgcatcgatgccagcgggcgcgacatctggctcgaggtcgatggcggcgtgaagcccgacaacgccgcgcgcatcggcgccgcgggggccgacacgctggtggcgggctcggcggtgttcagtggcggccgctaccgcgaagccatcgacgcgatccgcacccaggcgctgcagggcaggcacgacatggaaaggtctcccgcatgacgaaagacctgcgcgatatcgatgcgatcgccttcgacctcgacggcacgctggtcgacagcgcgccggacatccgtatggccctgaatgtcgcgctcgaagaggcggggcttgaacgtttcgacctggagaccgtgcgcgcgtggatcggcgatggccccgatgcgctgattctccaggcgctgcggcggcaggacctcggcggcagcgaggcactgcgcattcggctgcgcaaggccttcgacgcggccacgctggcggccccgctgaagcacggcggcgtgttcgagggcattgccgaactcgtcgagggcctgcgccgtgcgctgccgatggtggtggtcaccaacaagccgacaccgctggcacgcgccgtgctggatgcagccggcctgctgcagccgatggcgggggttttcggtgccgacgcggcggcagagcgcaagcccgcgccctttctgctgcaggccgtggcgcggcagctgggtgtggaacccgcgcgcctgctgatggtgggcgacggcccggccgacctgctggctgcgcaagcggccggctcgccggcggcgctggtggcgtggggctatggcggccatgcggcttcggacgcggcggctgtggcgccggcctggcgagtcgcaacgccgcagcagctgctgttgacggtgcgcgagtcgcgcgccgtccgccgggatgaagaaacgacgacaacgacccgatattgaaatcaaccaggagacgatcatgcccattgcaggcaaggccacgctgacccaatacatcatcgaggagcgccgccgccaccccggggccacgggcgcgctcaacgcgctcatcaccgacgtctctcttgcctgcaaggcgatctcgcgcaaggtggcgctcggcgccctgggcgacgtgctgggcagcgccaacacgcagaacgtgcagggcgaggaacagaagacgctcgacgtggtgagcaacgacatgttcctgcgcgccaacgagtggggcggccatgtggcgggtatggtgtccgaagagatggaagagccctatctgccgccgcggcaatacccgcgcggcaagtacctgctgctgttcgatccgctcgatggatcttcgaacatcgacgtgaacgtggcggtgggcagcatcttctcgatcttgcgcgcacccacgccagaggccgatgcaaagcccgaagactttttgcagccgggcaccgaacaggtcggcgcgggctacgcgatctacggtccatcgaccatgctggttctgaccctaggcaacggcacgcatgcgttcacgctcgacccgcagctgggcgaatgggtgctgagccatccgaacctgcgcattccgaagcagaccaacgagtttgcgatcaacgcgtcgaacagccgcttctgggaaccggccgtgaagcgctacgtcgacgaatgcctggccggcaaggagggcacgcgcggcatcgacttcaacatgcggtggatcgcctcgctggtggccgagacgcaccgcatcctgatgcgcggcggcgtctttatgtacccgcgcgacagcaaggagtcgggccgggacgggcggctgcggctgctctatgaagccaacccgatctccttcctgatcgagcaggccggcggcatgtcgagcaccggccgcaggcggctgatgtcggtcgagccggagtcgatccaccagcgcatcggcctggtcttcggctcctccgaagaggtggcgcgcgtggaggcctatcacaacgaggcgccgcaagacacctaccaagcgccgctgttcggcaagcgcggcctctttgcgaccgccgcctgaaaagcaccagagcacccacacacacaccggggccgagcccgagcggccccgcaagaaattctttatctccccgaggccaccatgtcagccaaacatcccatcgttgccatcaccggctcgtccggcgcgggcaccacttctgtcacgcgaaccttcgagaacatcttcaggcgcgagagcgtcaaggccgccatcgtggagggcgacagctttcaccgctacgaccgcacgtccatgaaggtggccatggccgaggccgaggccgcgggcaaccgtaatttcagccactttggcgaggacgcgaacctgttcgcggaactggaggcgctgtttcgcgactacggcgaagcgggcgtgggccggagccgcaagtacctgcacgacgccacggaggcggcgccctacaagcaggagcccggcaccttcacgccatgggaaacgctgcccgacagcgaactgctgttctatgaaggcctgcatggcggcgtgacgacggagaaggtcgacatcgcgcgccacgtcgacctgctgatcggcgtggtgccggtgatcaacctcgagtggatccagaagctgcaccgcgacaagaacacgcgcggctattccaccgaggccgtgaccgacgtgatcctgcgccgcatgaacgagtacgtgcactacatctgcccgcagttcacgcgcacgcacatcaactttcagcgcgtgccggtggtcgacacctccgacccgttcattgcgcgcaccattccaagcccggacgagagcctggtggtgatccgtttctccaaccccacgggcttcgactttccctatctgctgagcatgctgcacgactcgttcatgtcgcgcgccaacacgctggtggtgccgggcggaaagatggagctcgccatgcagctgatcttcacgccgatgatcctgcggctcatggaacgccgcaagaagtcgtacgcgatctgacgcgccgcccacccccggtctaccgctgacataccgcacaactctcaccaggatttttcggcatgacgattgacaacctcgccttgcgcacgcagtgcgccaatgccatccgcgcgctggccatggacgccgtgcaagccgccaactccggccatccgggcatgccgatgggcatggccgacatcgccgaggcgctgtggcggcaccggctgcggcacgacccggccgacccacactggatgaaccgcgaccgcttcgtggtctcgaacggccacggctcgatgctgctgtatgcgctgttgcacctgagcggctatgcactgcccatcgacgagctgcggcgctttcggcagttgcattcgcgcacgccggggcatcctgaggtcggtgtcacgccgggcgtggaaacgaccaccgggccgctggggcagggcatcagcaacgcggtcggcatggccctggcggagaagctgctggccgaggaattcaaccacccgggccacgaggtgatcgaccaccgaacctatgtgttcctcggcgacggctgcctgatggaaggcatcagccacgaggcctgctcgctggcgggcacctggcgcctcaagaagctggtggcgttctacgacgacaacggcatctcgatcgacggcgaggtccgcggctggttcagcgacgacacgccggcccgcttcgaagcctacggctggaccgtgctgcgcaacgtcgacggccacgatgccgcggcgctcgacgcggccatttctcgggccatcaccgcggaccggccggtgctggtgtgctgcaagacccgcatcggccagggctccccgaaccgagcgggaaccgcgaaggcgcacggcgaggcactgggcgatgccgagatcgcgctgacgcggcaggcgctgggctggaacgccgcgccgttcgaagtgccgcccgtggttgcaaaggcgtggtcggcgcgcgaatcgggcgccgcgctgcacaaggcctggcaagaacgctttgccgcttatgcggaagaatttccggtgctggcgcgcgagctgctgcggcgccatcgcagcgatgcgccgctcaccgcgcaggtcgaagcggcgttggcttcggccgcgtcgggtgcggagcagcgcaaggcttctgtcgccacacgcaaggcttcgcaggtggtgctcgacgaggtcgggcccgcgatgccagagctgatcggcggctcggccgatctcacgggatcgaacctcacggactggaagggccaccgcgcgctcaagggcatcggcacgggcaaccacgtgcactacggcgtgcgcgagttcggcatggcggccatcatgaacgggctggcactgcacggcggcttccgtcccttcggcggcaccttcctgaccttctccgactacgcgcgcaacggcgttcgcatgtcggcgctgatgaagctgcccgtggtctacgtcttcactcacgactccatcgggctcggcgaagacggcccgacgcaccagcccgtggagcatgcctcgagcctgcggctgatccccgatgtcgacgtctggcgcccggccgatgccacggaaacggccgtggcctggcggcaggcgctgcgccgcgtggacggaccgagctgcctgctactgacgcgccaggcgctgccgcatgcgggcggtggcgaggagcgcatcgagtccattgcgcgcggtgcctatgtgctgcggcgcccggaggccgagtgcgtcgcgctgctggcgagcggctccgaagtcggcgtggcattggctgccgcggccttgctggcagaggagggcatcgccgcgcgcgtggtgtcggtgccgtgcatggacgtgttcgaacgccaggacaaggaatggcgccacgcggtgattccgcgccatctgccgcgggtggcggtggaggcgggcagcaccggcttgtggtggaagttcgtcggtgaatacggcgacgtggtcgggctcgaccgcttcggcgaatcggcgccggccggcgaactgttcaagctgttcggcctgaccgccgaggtggtggccgagcgcgcgcgccggctgctggccgctgcttcagaggctcaggtgaaagaggccgcatgagcttcaacacgctggaccggatcgacctgcgcggacagcgcgtgtgacgttccacacccatttccaacatccacaggagcttcccccatggccatgatttcgctgcgtcaactgctggaccacgccgccgagcatcagtacggcgtgccggcgttcaacgtcaacaacctggagcagatccaggccatcatgcaggccgcgaaaaaaaccgacagcccggtcatcctgcaggcctcggcgggtgcacgcaaatacgcgggcgaaccgttcctccgcaagatggtcgaggccgcggtcgagatgtaccccgggatcccgatcgtgatgcaccaggaccacggcgccagcccgtcgatgtgcatgcaggccatccgctcgggcttcaccagcgtgatgatggacggctcgctgatggaagacgcgaagaccccggccagctacgactacaacgtggacgtgacccgccgcgtggtcgaaatggcgcaggcggtcggcgtctcggtcgaaggcgaactgggctgcctcggatcgctcgagtcaggcatggctggcgaggaagacggcagtggcgccgagggcgtgctgtcgcacgaccagctcctgaccgatccgcagcaggcggccgattttgtgtcgcgcactggcgtggatgcactggccattgccatcggcacctcgcacggcgcctacaagttcagccgcaagccgaccggcgacatcctcgcgatcgaccgcatcaaggacattcacgcgcgcattccgaagacgcacctggtgatgcacggctcttcatccgtgccgcaggaatggctggcggtgattcgcgactacggcggcgacatcaaggaaacctacggcgtgccggtggaggagatccaggaaggcatccggcacggggtgcgcaaggtcaacatcgacaccgacatccgcctggccatgaccggcgccatgcgccgcgccatgggcagcgaccgcagcgagttcgacccgcgcaagtttctgaaggaagccacggcagccgcgcgcgatctctgcatcgatcggttccaggccttcggtagcgcgggcatggcggcgaggatcaggcccgtggcgctgtagcggcgccggcttcaaggccccgtgcacctggccgtccggcgcggggctggttgacgcttcagcaggacaaatgccccaggcttttctgggccgttccagtacttatagaaggagaaggaaaggacattccttccatgtgcccgcgtcggcggcgcgatccaattgccaacaaacggatcaacgtcgagacgaaacgcgccggcccgccggcgttcaccaaggaagcacatgaccacgattaccggctccaacggcagcgaccttctcaccggcacggccggaagcgacaccatcaacagcggcaacggggacgacaccgtcagcggcggagccgggagcgattcgctgaatggtggcgcgggaagcgacacgctcgatggcggcagcggcagtgaccagctcaacgggggatcggggagcgacaccctgatctacaacgtcagcgaaaacatcgcggcgggcaccaaggacgtctacacgggcggggcgggcgtcgatacgctccagctccagttcacgcgggcccagtggctggagtcttccacccagacgcagatcgccgcctatctggcccatcttgcggccgtgaccaacgcgaagaccggcgaggtttccaatgcttcggccagcgatttcgttttcaggttcgggtcgtccacgttgaccgtccagatgaccgaaaccctggcaatccttgtggacggggtcgagatgaatccggccaacgaggcggtgaacgcgctgggcgacgcggccacgacaaccgaagacggcccggggatccagatccatgtgctgcagaacgattcggttccggacctggtcaagagcttggcgatggcctcggcgccggcccacgggacggtgacgctcgttcagccggcgatgggcgatccgtcgacctggtacttccaataccagccccatgcaaccgattttcagtacctggccgcgggcgagagcgcaaccgacaccttcagctacgaggtgaccgacgccgatggcgggaccggacttgccacggtgaccgtcaccatcaccggcagcaacgatggtccggtcatcacggcccaggacctggtgggtgcggtgaccgagcaggtcgcgccggcaggcacgctcagcgacagcggcgtcatcggcttcagcgacctggacctgagcgatgtgcacctggtgagcgccaccggcacgccggtcggcagcgtgctgggcagcctgaccgcggtgaaggacggcgacaccacggggaccggcacgggcggccaactcacctggacctataccgtggacgccacggccgtcgagtacctggccgcgggcgagacccgggtcgagagcttcaccatcacggtcgacgaccagcacggcggcatcgtcacccggcagatcgacgtgaccatcaccggcaccaacgacgcaccgacgatcggcgcggccgatgcggctgcggcagtgaccgaggatgcggccgagccaaccctgagcgacagcggcacgatcaccttcgacgacgtggacctgagcgatgcgcacggcgtcagcgtggcggtcggtgcgggcaacacgctgggcggggtcttgacggccgacgtcagcgatgcggccacgggcgcgggcgacggcacggtgaactggacctacagcgtcgccaacgcggcgacgcaatatttggcccaggaccagacggcgacggagaccttcatcgtcagcatcgacgacggccacggcggcacggcccagcagcagatcaccgtgacggtgaccgggaccaacgacgtgccggtgatcggcggcgtggcctgcggggcggtgaccgaagatgactcggcgccgaacctgagcaccagtggtgcgctgacgatcactgatatcgaccagggccagtcgaacttcgcgccacaggcgagcgtcctcggcagcagcggatacggcagcttcgcattggcagccgacggcaactggacctacacggccaacaatggccaggtggcgatccaacagctgggcgctggccagtcgatcagcgacagctttactgcagtctcctccgatggcagcgccagccaggtggtgacggtgactatcaccgggaccaacgatgtgccggtgattggtggtgtggccagcggggcagtgagcgaagatgactcgacgccgaatctgagcaccagcggtgcgttgacgatcgccgatgtcgatgcaggacagtccagcttcacagcccagcccgacactgccggcagcaacggctacggcagcttcacgctggcggccgacggcaactggacctacaccgccaacaacagccaggcagcgatccagcagttgggcgccggcgagtcgatcagcgatagcttcaccgctgtgtcgtccgacgggaccgccagccaactcgtgaccgtgaccatcaccggaaccaatgacgtgccggtgattgctggtgtggccagcggcgcagtgcaagaagacgttgcggtgtctggtggcagcctcgcggccagcggcgcgctgacgatcgccgatgtggatgcggaccagtcgaacttcgcgcctcaagcgagcactggcggcagcagcggctatggcagcttcacgctggcggccgacggcacttggacttatgcggccgacaacaaccaaaatgcgatccaacagctgggcgcaggtcaatcgatcagcgacagcttcactgcggtgtcgtcggatggcgccgccagccagctcgtgaccgtgaccatcaccgggaccaacgatgtgccggtgatcggcggcgtcgccagcggtgcggtgaccgaggatgcctcgacgccgaacctgagcaccagcggtgcgctgacgatcgctgatgtggatgcgggccagtcgagcttcgtgcctcaagtgagcaccgcgggtagcaacggctacggcagcttcaacctgctggccgacggcaactggacctacaccgccaacaacagccaggcagcgatccagcagctggccgcaggccaatcgttcagcgacagcttcactgcggtctcgtccgacggcactgccagccaactggtgaccgtgaccatcgccggcaccaacgatgcacccgtcctgagcgccgccgcgacacccgctctggcatcggtcgaccagggtgccggcgcaccggccggggccgtcgggacgctcgtatcgagcctggtgaatctgaatccgccgagcggcggcttggacaacgtgagcgatgcggacaacggcgcgaccaccggtatcgcgttgacgggcgcgaatgccgtcaacggaagctggtggtattccaccgacggcggcaccaactgggtcgcggtgggggcggtgtcggacgcgtccgcactgctgttggccgcggacgcgaacacgcgtgtctacttccaggcgaattcgaacttcagcgggacggtcagcgatggcatcaccttccgcgcctgggaccagacgagcggcaccgcgggaaccacggtgagcaccgtgacgaacggaggcagctccgcgttctcgagcgcgaccgatacggcgagcatcaccgtcaacgtggtgaatgtgaatccggtcaccgccagcgatgtgctctatgtgtcgaacaacaccgccgtgacgctgtcgaccagcgtgctgctggccaatgacacggacatcgatggtgctgcgctcagcgtgacggcaatcagcgtcgtgacgggggcgctggccactccgatcgccatcaacgccgacggaaccttctcgttcaccaccggggcgaccggcggcacggtcggcagcccgaccgtcgtcacgctcagctacacgctcagcgacggcgccggggggagtgcgaccggctccgtcacgctgaacgtgctggacacgacttcgggcgcgaacaccgtcgacctcaccggcgtctctgcctatcaaggcgcctatatcgacggcaagacgggaggcgacaccctgcgcgatggcgctttccaggcggttctcgtcggcagcaacggcaacgatcagttattcggcaacgcgggttcggacctgctgatcggcggcgagaacgtcgacaccctcgacggcggagccgggaacgatgtgctgcgcggggggaacaacaacgacgaaatcgatggcggggccggtacggaggatctcatcgacttttccgacggtctcaacggcatcgccttcacgctgacgcagtccagcggcaataccgtcttcaacggtcctggttcgctcgggaacgatacctacagaaacatcgagggcgtcatcggcacagccgtcgccgacactctcaccggcagtgcctcgaacgacgtcctccgcggcggcggcggtaacgacacgctcgacggagcggggggcgccggtgacctgctcgacttctccgacggcacggccggcctcgtgttcacgctgacgcaaagcagcagcacgacaagcttcaatgccagcgccgtcgggctcggcaccgacggctacaagaacttcgagggcgtcatcggcacggccttcgccgacgcgatcaccggttcggcgttgaacgaccaattgcgcggcggcggcggcaacgatgtgatcaacggccttgcaggcgacgaccgcatcgctggcgggaccggtgccgacatactcaccggcggcgccgataacgacaccttcgtcttcgactcggcacccaatgcggtggattcggtcacagacttcaatgcctcgggatcggcggcgagcggcgacctggtcgagctgtcgctcggcaccttcacggccctttcgaccgcaagcggaagcacgctgtcggcggccgagttcgcgtcctcgaacggcggtggtgcgggagacgcggtgggcgcgggcgtgcatgtgatctacgacagcgccacgggcaacctgtactacgacgcagacggcctgagcgccgccaaccgcacgctggtggcgacgttgacgctgagcaacccggccgacaccttcgacagcaacgacatcaaggtcggccagtgaccttgcgccagccgcccgcggatgcgggcggcagcacgcgagggacatcgacatgaagcctcttctccagctgctcaagcgaccgcttctctttgtcggcggcttctcgttcttcgtgaacctgctgctgttggcgcccgcgctcttcatgctgcaggttttcgaccgggtgctgacgagtcaaagtcgggagacgctggtggtgctgttgctgggcgtcggcgtggcgctcggcctgatgctgctgctggactacctgcgcagccggctgcagggcgtcgcgggcaacctgattgccgagcagctgtctccggtggtggccaaggtcatgttggcccacacggcgcgccgtgccgagcgcgcgccctcggaaggcttgcgcgacgtcgcggcgctgcgcaacctgttttcctcccaggggctgctggccctgttcgatgtgccatgggcattcgtttatgtcgcggtcatctggctggcgcatccgatgctgggcatggctgccgccgccgcgtcggtgctgatgctcgtccttgccgtgctgaacgaccgcctcacgcgccgcgatatcgaagccctgcagaaagaagccgcccgggccacgcgctacctcgaatcgtcgatgcagaacgcggagctggcgcagtcgctcggaatgggggatgcggtgatcgggcgctggcggactctcaacgccggtgtcgccgcgctgcaaggcccgaccgcgcgcaagtcggtggcaatggctgcgctcacgcgcaccacgcgccaggcggtgcaggtgctgttgcaggcactgggcgcctacctcgtcatcacgggcgaaggcacgccgggcatcctggtggcctgcaccatcctgctcggccgggcgctggcgccggtcgaacaggtggtggggagctggcgcgtgctggccgaggggcgcctggccttcgcgcgcctgtccgaggtgctgggcgccgccgagcgccagccgcaacgcatggcgctgccggcaccgaagggccgcctgcacgcggaaggcctcgtgttccggcctgcgcagggcgagcggatgattctcgctggcgtgtcgctgagcctggagcctggcgagtcgctggccatcaccggcgccagcggtgcgggcaagtcgacgctggtgcgcctgctgaccggcctgtggcggccccacgcaggtgtcgtgcggctggacgacgtcgacatcgcgcaatggccgcgcgaggaactcggcccctggctgggctatgtgccgcaggatgtcgagctgttcgccggcaccgttgccgacaacatcgcgcggctgggcgaggtcgacccggacaaagtcgtgcaagcggcgcagcgtgccggcgtgcatgcgctgatcctgacgctgcccgagggctacgacaccgtcgtcgacaacatgggcgtgatgctgtcgccgggccagcgccagcgcattgcgctggcacgcgcgctctatggcaacccgaagctgctggtgctggacgagcccaactccaacctggacggggcgggcgaactggcgctgggcgaggccctgaaggcgctgcgcggccaggtgacggtgatcgtcgtcacgcaccgcagcgcgctggtgcagcacatggacaaactgatggtgctggaagccggccgcgtcaagcaatacgggccggtggcggacgtgatgcaggcgatccggcgtccgggccagaaccagggcggcgcccaggtggtcatgatgccggcgcgcgctgcggagaaggtgtcatgagcgccgcgccgggccgccccaagcaagctcgcaccgcagtgcgcagcacggaggttgtccgatgaatcattcggcgcttgcgatcgcggccaatgaccccctggcgctccatgtgcgcgaagcgcgtcgcctggcgcactggggcctggccgtgctggtttgcggcctgctgccggcggccgcctggctgagcttcgcgccgctgtcgtccgccgtggtggcgcaggcccatgtgaaggtggacctgaaccggcgcccggtgcagcatgccgaaggcggcatggtgcgcgaagtattggtgcgcgacggccagcatgtgcggcagggggagcccttgctggtgctgggcgacgtctcggtcgatgccgacaggaaccggctggaccaccgcgtcaagaccgagcgtgccagcctcgcgcggctcgacgcggagcagacgatggcgcgcgcgatcgtcttcccgcccgacgtggtcgagaccgcggcagccgatccgcgcctggccgcgcagctggacaaggagcacgcactgttcgaggcaaggcgtgatgcgctggtggggcaggtgcgcctcttgcgctcgcaacgcgagaaagtggccgaggaaatcgtcgcactgcgcgcccagatcatgcgggcgagcgagtcgatgacgttccagaaaaacgatctggaaaccaaccgcaagctgctcaaggacggcttcatctcggccgcgcgcattgcgcagctcgaaggcactgtggccgactacggcgtgaagatcgaggagcggcgcgcggagctcgcgcgcgccgagcagcgcacggtcgatgccgatctgcgcatccgctcgctggagagcgactaccgccagcaggcgagcgaccagctcaaggtcacggcggcccggctggcggaaatcgagcaggagcggcgcaagtcggccgacgcctcggcgcggcaggtgatcacggcgccggccagcggcgagatcatcgatctgaagtattcgacgcccggcgcagtgatccccccccgcgagaccattgccgacgtcgtgcccgacgacacccgcctggtgaccgatgcgcgcgtccgtcccgaagacatcggccggatccagcgcgggcagccggccgagatccgcttcacggcgttcaagtaccgcaccacgcagctggtgcatggcaaggtggtctatgtgtcgggcgaccgcctgatcgaccgggcgaccagcgctccctactactcggtgctggtcgaggccgatgcggcttcgctcgcgacggcgggagacctgaagctgctggccggaatgccggccgagatctacctgcagggggacgagcgcaccgcgctccagtacctgttggagccgatcaccgaggtgctgcgccgcgccgcgcgcgagcgttgacgcgtcgtgccgggtgtcgactgaccgacgcggcttgcaacgcgccggtatcgagcggatcattcatcagcttgccccgcctgccttgttgcgcccacggtctgtcagcgtggtaatgccctatggccgtcatagccaaagcttttgcatattcgtgcgtgcaacatccagaatcacagatctcattcaaagttggagacgccccatgagccagatacaaacggaagccaagtgccccgtccaccatgcggtcggccgcggccctgtcaatcgtgactggtggcctaaccagttgcgggtggacctgcttcaccaacactcctccaagtccgatccgatgggcaaggacttcaattacgcgaaggaattcaagagcctcgactacgaggcgctgaagaaggatttgcgtgcgctgatgacggactcgcaggactggtggccggcggacttcggccactatgggcccctgttcatccgcatggcctggcacagcgccggtacctaccgtaccggcgacgggcgtggcggcggcggccggggccagcaacgctttgcgccgctcaacagctggcccgacaacgtcaacctcgacaaggcccggcgcctgttgtggccgatcaaacagaagtacggccgcaagatctcgtgggccgacctgatgatcctgaccggcaacgtggccctggaatccatgggcttcaagaccttcggcttcggcggcggccgcccggacacgtgggaacccgaccaggacgtctactggggtaatgagacaacctggctcgaagacaagaggtacaccggcgaccgcgacctggagaacccccttgcggctgttcagatgggtctgatctacgtcaaccccgaaggtccgaacggcaacggcgacccggtctcggcggcgcgggacatccgcgagactttcgcccgcatggcgatgaacgacgaggaaaccgttgctttgattgccggcggccacacctttggcaagacccacggcgctggtccggcggacctcgtcggctcggtcccggaagcgaccgacctggaagaaatgggcatgggctggaagagcacccacgccagcggcatcgccggcgatgcgatcagcagcggcctcgaagtcacctggacgcagacgccgacgcagtggagcaaccacttcttcgagaacctgttcaagttcgagtgggagccggtcaagagcccggccggcgccggacagtggcaggccaagggcgctgcggcggacattccggatgcccacgacaagtcgaagacgcgcgtgcccaccatgctgaccaccgacctctcgctgcgcttggaccccgcctacgaaaagatctcgcggcgcttcctcgagcaccccgagcagttcgccgacgccttctcgcgtgcctggttcaagctgacgcatcgcgacatgggcccgcgctcgcgctacctgggtccggaagtgcccgccgaagagctgatctggcaagacccgatcccgaaggtcgaccatcccctgatcgacgacaaggacgttgcggcgctcaaggccaagatcctggccccgggcctgtcggtgtccgacctggtgctgacggcctgggcttcggccgcgaccttccgcggctccgacatgcggggcggcaccgatggcggccgcatccgcctggcgcctcagaaggactgggaagtcaacgagccgaccaggctggccaaggtgctcaagacgctggaaggaatccagggcgagttcaacaaggcgcaaacgggtggcaagaaggtctcgatggccgacctgatcgtgctggccggctgcgccgccgtcgagcagggcgccaagaacgcgggtcacaacctgacggtgcccttcaccccgggccgcatggatgcgtcgcaggagcagaccgacgtggaatccatgaaggtgctcgagcccgtggccgacggctttcgcaactacctgaagaaggactatgcggttcctgccgacgcgctgctgatcgacaaggcgcagctgctgacgctgacggcgcccgagatgacggtgctggtgggcggcatgcgcgcactgggcgccaacgtcggcgctaccaagcacggcatcttcagccagaaggagcacgcgctgaccaacgagttcttcgtgcgcctgctcgacctgaacacgacctggaaggctgtgcccggcgagaacaacctgtacgagggagttgaccgcaagacgagcgagcgcaagggcagcgcgacgcgcgtggatctggccatcggctccaattcagtgctgcgcgctctggccgaggtgtacggcagcgcggacgcagaagagaagttcgcgcgggacttcatcgcggcgtggaccaaggtaatgaaccttggccgcttcaacatgggctaaagacaatcctcgcggttaccgattcgatgcagtagctggaagcagtcgccgttgcgagggcggcgcaatttggcgccgctacgcctatgcagaaaagcgcaggagacaagcgcaggagacaacgatgacggccagctacgtagaaatacaaggcgcccaggcggatgttgacctctgggatggattgatctcagatcaaaacgccctcatcggcgtcatgatgcagaagatgtcccaagtgggatgcacggatgcagcatggctcgatgagcggatcacggaggcggaaagtatcgagaaccggctggtcgtcgggctcgaccgtgcccagcgccgattgcgggcattgatctaggggacgtctgggcggagttcgcagcgcccttcaaccggcgcagacagcgcccgcacattcggcttccaatggaaggcctccgttcttgacggacgggaagaaactgtcgtaaccagctacaacgcgtgcaattgacgccaggcgggtccaacatgcaccgcgttccgactcctggcgccaacaagtattgagttgcaatgcttctgttgaagccttagaggacggtacagccacgcggcccccgtctcgcaaagcaacgagattgcgcacgcgaggaaatgacgtcgaaaacctgttgcgtgctgctgcagggataagttccgctcgcgcctactccgttgggtaattgtcagacttaattattaagttcagtatccgcgcgttctccggacgccgcgacgttgacctcatcgccagcaccgagacgcacccaagaacagatgattattcaaactaacttggagagccaatatgaaaaagtcattactaatagcggcagcgttgacgtttggagcaggacaggcgctcgccgcggcacactttttcagtgccgatgcatccgtcaattcgaatggggcgctggtggtcagttttgatgaagccggagtggcgaacgcaacagtggttgaaagccttactgctcaaggttcggcggtgtacgcgtgcatcaaccgcgggggaaagaatccgagcgccagcaacaagacctccgtctcgggagccgtgcgtgctgacaatactttctcagccaccaagaacggccgagtgaggggaaccttggaagccggccctccggacgagggcaatttttcgtgcccaaatggtcaagatctcgtagtggcatgcgtcagatacacggacgtgctgctctctgatctgaccaacggtgtctcgattgtgccaactggcaccttctccagaaacttcttgagcatccctggctcttgtcccaattaagcaagagaccgcgtcgaaacggccctgggcaagcccggggccacaccaaggacacagtcgtggcgcatcgacaacgtaaaacgcgcctagcgcttgcaggtctttgcctggcagccctgtctgcaaccgcgggtgcaccggtgttcgcagccgaagctcagaagccgtcctccgtcgaagccgatcggatcgaacaatcagccggcgccgacgcgtctggcttggtcagccatggtggcgcgctctacaacccgttcagcaccgctgttgactcggccgcgtcaaaacctcacgccaacgccgcgccgacacgacaagacgcggacgaaagattgcccgacctcatggcgacggcagttaccgcgctcgttgctgctgggttcctcgtcattcttgttcgcgtcctgattgcgagttagggacgcctgggccttgaccgccaacggcagctcgttcttcagcccggatcggcagcttcagcttcaggttcagctgatgaaccgcacagcaagcagcgcgagcaaatacaagaacaccatgaagaaatttcccggtagcaggttgcgttccatgtgcgttctccagtgaggtggacaaccggcgccgcttgtttggctgtcttggaacaaagcgtttcgtcgtgaagtcactgtaggaattgcgccgcacgcgcgcatgagcggtacgcacctttttccggggagacaaatgccctcactgctgctgcccacgacaaagagccttccggaggccggaatgaatggagtcggaaggagcggcgagctttccttgcaccgaacgaaggcgccggccgacggtaaaagcgatgtgccggcccagcattgcttgcatgagccgctcccgctttcttgtactggaggttgagatgctccggtctggagcgttcgaatgggtgctgcgcgagtccttcaatgacgcacctgacttcgagctcttcacgcgctcggatctcagcttcatcacatccaaggacgcctgggaggccgggtgcctggcacttcaatcacgcatggaagatccaaaactggatctactcgacgaagaggactagcagtcggaccagctcagcaattttgagatgccgcaccggattgctgttctcggatcaggaattcggcgatccattcgcgcgccttggccgcgagcagtttcttcgccttttcctcttcgggcacaccgcagacgccgacccggaacatcaccttcccggcccgcttcacatcggcaaagaagtagatgccttcgcccacaggctcagcccccacctcgatggtccaatcgggtggagcagcaggcgggtcggcggggtcgcgcgccggagaaatgttcatggctggtcaaggtgagtgcttccgcagggcagtatgcgccactcggacgcgcacacaaggggagcaatgtcatgcttggcggcttactcgccagaaggcgaccacggccgggcacctactgatgaaggaaagccagagcatcggctgcactcgccttcgcgctgcctaccgtgtcttggccgccggccggtcactggcgcaacgtggctgtgccgatcggcctatcgccgtcgcccgttgcgtgaagagtttctactcaagaggcgggtcgtcgcccagggttttcagctcgctttcgagttccgcaatcttcgcctcgatgagtttcttgtctccgaccgtctttaagggcggatggccgctcttttcgggctccgaagatggggtcttgctcatcttttcgaggctcatcaattgctcgcgcatttcggcaagctctttctcaatcacaggcgctgaccgctttgttgccatcatgatcaccttgggacaatgggcttgcgcctttatacgccgggtgatctgcccgcgctagatcgtaagtccacatcgcaatgtctctgcgaaccgttcctgccgctcggaggcactttgtcatgggaagtcgtaaacctgatcggacgattgtctctgtggagaaagtgcgtctcgctcatgtgcacatgcggcgcaatttctacagtgacttcacggcgaagcgccttgttccaagacgggcaacaagcggcgccagttggccacctcactggagaacgtgtatggaatcgtacaacctgccgctggcaaatttcttcatgaatctgctgcgtgaagacgtggggatgtcgtctacgcagttcgctgtcgtcagtgcgctcgtggtgtttttgtacttgctcgtgctgcttgcagtgcggctcagcaactgagcgctgagctgccggagagcatgaagcggtgggctacagagttgctggttagcgtccgacatgccggccggggcagtggcatagcttcgagttctccaacgaaggagcgacgcgagcaagcgcccaatctcgacaacaaacgcatcgaagaggtaacggctatgcccctgttctatttgctaagcctgcagcacgtcgcactgcccaaggtggtgacgagatccgaagacgtccagcatgtgagcgtcctgaaagcgaccggtctcatcgaagcggagattgcgccagcactggacccggccggcaagtacaacgtcgcccgaacagccgtcgtgacgcgcatcaccgaagatggccacgcagaaatcaacaggatgctcaacgaaccccggcgaatgggcaggacgttgcaaatggtcaggaaccggatgcggagttcttcgccgagttgaacgctcgctcacgtagccactgccggcagggtggggcgcctctcgcgctggttctatggcttcggcaaaagtggggtcaggtgccctgagtttttccaatgccccaggcttggcgaggtcgatctcacggttcttcatccagagcttggcggccggctcacggtcgaaggtctccgtctccgtgtggatgacgacaccgtcctcccgaattcggattcgagccatgtgcgctacgcttccgtccgcgcgcttgcgtttggtaatgctgcccaaggggtccctctcgttggtacaagccaaatttgtggcaaaaatgtaccggcgaagcccagaaaatagcgacaaacgatatcgaatgacaccgaaagagaacagcggaaaccccgcgtcagaccttgattttcctcgggaggaccgtgcttccgaggctatgcgcgtctccgtggcgcccatgatggactggaccgatcgccattgccggtacttccaccgcctgctgtcgcgccacgcgctgctctataccgagatggtgaccaccggcgcgctgatccatggcgacgtgccgcggcacctgcgtttcaacgccgaagagcaccccgtggccctgcagctgggtggtagcgagcccgccgacctggcgcactgcgcgaagctcggtgaagagtggggctacgacgagatcaacctgaattgcggctgccccagcgagcgcgtgcagcgcggcgcttttggcgcctgcctgatggccgaaccggcgttggtggctgactgcgtgaaggcgatggtcgacgcggcgagcctgccggtcacggtcaagcaccgcatcggcatcgacaagatcgaaagctacgacttcgtgcgcgattttgtcggcgcggtgagcgaggccggttgcggcactttcatcgtccacgcgcgcaacgcctggctgcagggcctgagcccgaagcagaaccgcgagattccgcccctgcgctacgaactcgtgcaccggctgaagcacgactttccggccctgggcttttcgatcaacggcggcatttcggccactgcgcaggtgcatgagcacctgcggctgctggatggcgttatggtcgggcgggaggcctatcacaacccctggtggctggccgagtgggacgcggagttcttcggtgccgcaccgcagccgctgacccgggaagaggtggagtcgctgatgtgcgactacatggtgcgcgaggcggccgagcacggcacccagtggtcgtcgattgcgcggcatatgctgggcttgcgcaacgggctgccgggcgcgcgccgctggcgccaggtctggagcgaccatcggctcaagacgcgccccccgcacgaggtgatggcgctggcgcacgagcccgtggcgcaggctgcctagccggtagtaccgcccgccgtttgaccgggggcgcgcaactgcggtaaggctttgcacttcagcaacacgaagtgttccaaaatgataatgatttaccgggggctgcaacttttcaatttttctgctgaagaatcaagaaacactaataagtagaggtttcgattcatgactgaaacggttgggggcaaggaagaagtcactgcgctcggccgcgggctggccctgctcaaggtcatcggcatggcggcggctccggtgagcaaccgcgaactggcggacaccaccggcatccccaaggcgacggtatcgcgcctgaccgccacgctggtgagcgcggggtatctgcggcaggcgccggacagcgagcgcttcagcctgggcccggcgctgctcgacatgagcagccgttatcttcgccagttcgaccttcgggcggtggcgaggccccacctggcggagttgtcggaattcgcgggcgccagcgtccatgtcgcggtgcgcgacgagctcgacatgctggtcatcgattcgctgcgtccgcgctcggcgctgatcagctcgcgcctggagatcggcacgcgcttgaccgtcgtcacctcggccgccggccgggcttgtcttgcggccctgccggccgccgagcagaccgcgctgctggagcggatccgggaagaaagcggcgaaaactggccttccatcgagccgcgcctgatggccggaatcgacgaatacacccgcctgggctattgcagctcgttcggcgaatggcatccgcacatccacgcgctcggcttcgcgctgaaaggccctcatggcgagcactacggcgtgagctgcggcggccccgcgtacctgctgcccaaggaaatgatgctcacgcaggtcgcgccgcgcctgctcgaagtggcccggcgcatctcggccgaagccggaaccgcaaatcccgattagcgacccggcagcgtggcccttcgtggaacaccgaggaaccggctttgccgggcctctggtgttgcccccggtagggggttggcgtagcgacacgaagtgcgcgaagactgggggcgagcctagtgccaccgaggaaccggctttgccgggcctctggtgttgcccccggtagggggttggcgtagcgacacgaagtgcgcgaagactgggggcgagcctagtgccaccgaggaaccggctttgccgggcctctggtgttgcccccggtagggggttggcgtagcgacacgaagtgcgcgaagactgggggcgagcctataccgcggcttccaggccattcctgaaatgctcgcgcatgcgagccatggccgcggtggcgtcgcgtgcctcgatcgccgccatcatcgaccggtgctccgccagcgattcagcaatgcgcccctccttgagcagcgagttgtggcggttgagcttcatcaccttgcgcaggtccgccaccatctggtcgcgccacttgttgttggcaatggccagaaggcgcatgtggaagcgctcgttcagcgcaaagaagtgctcccggttttccttgcccggtgcgccggcggcctccagttcggcatgcagcgccttcagctcggcgcgctgggcgtcggtggcgcgctcggccaccacgccggccgcgtcgctctccagcagcgagagcaggtggtagacgtccgccaggtcctgttccgatacttcggtcacataggcgccgcgccgcaccttcatcgtcaccaggccttcggccgcgagcaccttcagggcttcgcgcagcggcgtgcggctgatgccgtattcctcggccagcttgagttcgtcgatccagctgcccggctcgagctcgcggcggaagatccgctggcgcagcagctcggccacctcttcatagagggcgcgcggggtgagggtgagggcggacatggggcggactgtaccgcaaaaattgcgtttgaattaataattatggatcggttagactcgctgcggcttgcaaatcccttgcaggcgaatttgcgactaccctgcaagacactgcaaaacggcccctcatgagcagcacacccgaacccaccttcaagcctgccaacctcgacgactgggccaaggccgccgccaagtcggcgccgggcggtgacctgagtgcgctcaactggctcacaccggacggcatcagcgtgaagccgctttataccgcggccgatctgcagggcctgaagtacaccgacacgctccccggtttcgagccctacctgcgcgggccgcaggccaccatgtacgcggtgcggccgtggaccatccggcagtacgccggcttttcgaccgccgaggaatcgaacgcgttctaccgcaaggcactggccgcgggcgggcagggtgtgagcgtggccttcgacctggccacccaccgcggctacgacagcgaccatccgcgcgtgaccggcgacgtcggcaaggccggcgtggccatcgattcggtcgaggacatgaagatcctgttcgaccagatcccgctcgacaaggtgagcgtgtccatgacgatgaacggcgccgtgctgccggtgctggcgggctacgtggtcgcggccgaagagcagggcgtggcgcaagaccagctgagcggaaccatccagaacgacatcctcaaggagttcatggtccgcaacacttacatctttccgcccgcgccgagcatgcggatcatcggcgacatcatcgagtacacggcgcagcacatgcccaagttcaactcgatctcgatcagcggctaccacatgcaggaagccggcgccaaccaagcgctggagctggccttcacgctggccgacggcaaggaatatgtgaagaccgcgctggccaagggcctggacgtggacggctttgccgggcgcctctccttcttctgggccatcggcatgaacttctatctcgaggtggccaagatgcgtgccgcgcgcctcctgtggtgccgcatcatgaaggagttcaaccccaagaaccccaagagcctgatgctgcgcacacactgccagacctcgggctggtcgctcaccgaacaagacccgtacaacaacatcgtgcgcaccaccatcgaggccatggccgcggtgttcggcggcacgcagagcctgcacaccaacgcgctcgacgaagccattgcgctgcccaccgagttcagctcgcgcatcgcgcgcaacacgcaactcatcatccaggaagagacgcacatcaccaatgtggtcgacccatgggccggcagctacatgatggagaagctcacgcaggacatggccgatgcggcctgggccatcatcgaagaggtcgaggcgatgggcggcatgaccaaggcggtcgacagcggctgggccaagctcaagatcgaagcggccgccgccgagaagcaggcgcgcatcgactcgggcaaggacgtgatcgtgggcgtcaacaagtacaagctcaagaacgaggacgcgatcgacagcctctccatcgacaacgtgatggtgcgcgaccagcaggtggcgcggctgcagaagatccgcgcctcgcgcgacacggccaaggtgcaggccgcgctcgacgcgctgaccgaagccgccgagaacggaaccggcaacctgctcgcgctcagcgtcgacgcggtgcgcctgcgcgccacggtgggcgagatttcggacgcgctcgaaaaatcattcggccgccatcgggccgacacgcaaaaggtgaccggtgtgtacgctgctgcctatgactcggccgaaggctgggaagccctcaagaccgaaatcaacgccttcgccgaagcgcagggccgccgtccgcgcgtgatgatctccaagctggggcaggacgggcacgaccgtggtgccaaggtggtggctaccgcgttcgccgatctgggcttcgacgtggacatggggccgttgtttcagacacccgaagaatgtgcgcggcaggccatcgagaacgacgtgcatgccgtgggcgtgagcaccctcgcggccggccacaagacgcttgtgccggccatcatcaacgagctcaagaagcagggcgcggacgacatcatcgtgttcgttggcggcgtgattccgcggcaggactacgactttctctacgaggccggcgtcaagggcatctatggcccgggcacgccgatccccgccagcgccaaggacgtgctggaacagattcgcgcggcggtctcggcctgatcgggacgctagacgtgggcgatctcttgtcgcggctgtctctgcagccggtggattccagcgatttcgaggccatgctcgccttgcgcgtcgatgcgatgcgcccgagcctggagcgtgtcgggcgcttcgaccccgcgcgttcgcgcgagcggctccaggccggttttgtcgtgcccttcatgcatcacatcgtgctcgacggcgccgggcgcatcgggttcgtcaccctcaagcccgagggcaccgaggcgctgcggctcgaccatctctacctgcgcaccggcttccagggcctgggcatcggcgaatgggtgctggagtgggccaagtcacaggcgcgcgaagagcggctggacatcaagctcaccgcgctcgtgcagagcgatgccaaccgcttctatctgcggcatggtttcgtgctcgaaggcgaggagggcgtcgacctgcactaccgctggcgcgtggcctcggagggcgcgtgctgaagtcggccgaagcactcgagcgcgccatcacccagccggacggtatggtgcagcgccgcgccatcgccaaggccatcacgctgctcgaatccacccgcgccgaccatcgcgttcaggccgacgaactgctcaccgcgctgctgccgcgcaccggcaactcgtttcgcctgggtatctcgggggtgccgggcgtcggcaaatcgaccttcatcgaaacgttgggcctgctgctgatcggcaagggccaccgcgtggcggtgctcaccatcgatccctcgtccaccgtctcgggcggctccatcctgggcgacaagacgcgcatggagcggctctcggtgcacgagcgcgcctacatccggcccagcccgtcgagcggcacgctcggcggcgtggctgaaaaaacgcgtgaagccatgctggtgtgcgaggccgccggctacgacatcgtgatcgtcgagaccgtgggcgtgggccagagcgaaaccgccgtggccggcatgaccgacatgttcgtgctgatgcagctgcccaatgcgggcgacgacctgcaggccatcaagaagggcgtgatggagctggccgacctcgtcgtcatcaacaaggccgacatcgacaaggatgccgccacgcgcgcgcaggcgcagatcacctctgccctgcgcctcttcggccaccagggcaacccggaccatgcgcatgcggtgcatgacgcacacagcggcgcggagatccgtttctggctgcccagggtgctccagctgagtgcgctggccggtacgggcgtcgatgccttctgggaagcggtgctgcagttcaaggccttgcagaccgccaatggcaagctcgccaagcggcgcgaaaagcaggccaccgcgtggatgtgggaacgcatcgacgccgggctcaagcaggccttcaggcagcatgcgcaggtgcgcgaactgctcccgcaactcacccagcaagtggcggagggcgcgctgcccgcatcgacggcggcacgccagctgctcgcggccgccgccatcaccgccaggccatgacggccaacaaaattcaggaccaccagcttcggaagcacaccatgcaagaactgatcgaacaactcgaaaagcgccgcgcccaggcgcgcctcggcggcggacagaagcgcatcgatgcgcagcacgccaaaggcaagctcacggcgcgcgagcgcatcgagctgctgctggacgacaacacctttgaagagtgggacatgttcgtcgagcaccgctcggtcgatttcggcatggccgagcagaagatcccgggcgacggcgtggtcaccggctacggcatgatcaatggccgcctggtgttcgtgttcagccaggacttcaccgtcttcggcggtgcgctcagcgaagcgcatgccgagaaaatctgcaaggtcatggaccaggccatgaaggtcggcgcaccggtcatcggcctcaacgattcgggcggcgcgcgcatccaggaaggcgtggcctcgctcggcggctatgccgacgtgttccagcgcaacgtgatggcttcgggcgtggtgccgcagatcagcatgatcatgggcccctgcgcgggcggcgcggtgtattcgcccgccatgaccgacttcatcttcatggtgaaggattcgagctacatgttcgtcaccggccccgaggttgtgaagaccgtgacgcacgagagcgtgacggccgaagaactcggaggtgccatcacccacaccacgcgcagcggcgtggccgacatggcgttcgagaacgacgtcgaggcgctgatgatgctgcgccgcctgtacaactacctgccgctcagcaaccgcgagaagccgccggtgcgcctgggcaacaacggccagggcgacccggccgaccggcccgactattcgctcgacaccctggtgcccgacaacccgaacaagccctacgacatcaaggagctgatcctcaaggtggcggacgacggcgacttcttcgagctgcagcccgactacgcgaagaacatcgtgatcggctttgcgcgcatggaaggccagaccatcggcatcgtggccaaccagccgctggtgctcgcaggctgcctggacatcaagagcagcatcaaggccgcgcgcttcgtgcgtttctgcgatgccttcaatattcccgtagtcaccttcgtcgacgtgcccggcttcatgcccggcaccggccaggagtacggcggcatcatcaagcacggcgccaagctgctctatgcgtatgcggaatgcacggtgccgaagatcaccgtcatcacgcgcaaggcctatggcggtgcgtacgacgtgatggcctccaagcatctgcgcggcgacgtcaacctggcctggccgcgcgccgagatcgcggtgatgggcgcgaagggcgcggtggaaatcatcttccgcgaggacaagaacgaccccgagaagctcgcagcccgcgaggccgagtacaaggcgcgctttgccaacccctacgtggcgggcgcgcgcggctacatcgacgacgtgatcctgccgcacgagacgcgcaagcgcatctgccgctcactggtgatgctgcgcgagaagaagctcgagaacccgtggcgcaagcacggcaacattccgctctgattcgtatgcgcagccactacccccagttccgtgagggagcggaacccggacttgttcccaagctcggcggcctgccctggggcctccctccgcgtctctggccggtttgcgctgaatgcaaccgggccatgagccatcttgcgcaattgccggccgacggcgacgcattgccgcttgcgagcgacgaggtgctgttcctgttcaagtgcgagtgggacagcatctgcagcttctgggagcatggcgccggtgcgaacgctgcattcgtcgtgcagcgcaccgctctgggcgccgggccgacgccgcggccttcggaccccgccgacggatcgcctgcacttctgcgcgagatcgccatcaccggatggcacgcagatgacgatggcgcccccgccgaattggaggacgcgttctatgactatcaggcccacttcgatctgccggacgaagtcaaacatccccacgattgggcgagcccgtggtgtaccaagagcggcggcgtgccgtactggacggccaacggcgcacagctgatgccggcgggacgcttgttcctgcagatcgacaactggctcgagctcccaggtggcgagtgtgtcgaggtggcgaacttctgttccgacggcatcgcatatgtgttcgtcgatcggtcgcaagcaaagccggcgtactcgatgttcatcaaccgctgaggcggtcagcaaaataaaacggattcagcatgttcaagaaaatactgatcgccaaccgcggtgaaatcgcctgccgcgtgatacagacggccaagaagatgggcatcctcaccgtcgccgtctattccgacgcggacaaggaagcccgccacgtcgagctggccgacgaggccgtgcacatcggcgctgcgcccagccgcgagagctacctgcaagccgaccgcatcattgcggcctgcaagcagacccgcgccgaggccgtgcatccgggctacggtttcctgtcggagaacgaagcctttgcgcgcaaggtcgaggaagaaggcattgccttcatcgggcccaagcactactcgatcgcggcgatgggcgacaagatcgcctcgaaaaagctcgcgaacgaagccaaggtcaacaccattcctggctggaacgacgccatcgaaacggccgagcgcgcggtcgagatcgccaaggacatcggctaccccgtgatgatcaaagcctcggccggcggtggcggcaagggcctgcgcgtggcgttcaacgacaaggaggccttcgagggcttcacctcgtgccgcaacgaggcgctgagcagcttcggcgacgaccgcgtgttcatcgagaagttcgtcgaggagccgcgccacatcgagatccaggtgctgggcgattcgcatggcaacgtcatctacctgaacgagcgcgaatgctcgatccagcgccgccaccagaaggtgatcgaggaggcgccgtcgcccttcatctctgacgcgacgcgcaaggcaatgggcgagcaggcggtgcagctggccaaggccgtgaagtaccagagcgccggcacggtggagttcgtggtcggcaaggaccagagcttttatttcctggagatgaacacgcggctgcaggtggagcatccggtcaccgaatgcatcacggggctcgacctggtcgagctgatgatccgcgtggcggccggcgaagagctgccgctcacgcaggccgaggtcaagcgcaacggttgggccatcgagtgccgcatcaatgccgaagatccattccgcaatttcctgccttcgacgggccggctggtgaagttccagccgccggccgaaaccatgtttgccagcgacaccgggcacttgaacggcgtgcgcgtggacaccggcgtttacgacggcggcgagatcccgatgtactacgactcgatgatcgccaagctcatcgtgcacggcaaggatcggcagcatgcgatcgcgcggatgcgcgaggcgctcaatggcttcgtgatccgcggcatcagcagcaacattccgttccaggcggcgctgctcgcgcacccgaagttcgtggcgggcgacttcaacaccggcttcatcgccgagcactacggcaagggctttcacgcagaagacgtgccgcacgccgatccgtcgttcctcgtcgcgctcgcggcctatgtgcaccgccgctaccgcgcgcgtgcctcgggcatcagcgggcagctcgaaggccatggcgtgaaggtgggcgagcggttcgtggtggtggagctgggcgcggaaggcaaacacgtgcaccacccggtgtcggtgagtgacttccacggcaagaccggcgccagcgccgtggccgtgggcggcaagagctacaagatcgacagcggctttgcgctcggcgccgttcgcgtgcaaggcatggtcaacgaccggccctttaccgcgcaggtggagcgcggcgcgggcaagaatccgctggcgctgcgcgtgtcgcacgacggcacccagatcgaggccatggtactgtcgccgctcggcgcgcggctgctcgagctgatgccctacaaggcgccgcccgacctcagcaagttcctgatgtcgccgatgccgggcttgcttgtcgaggtgtcggtgcagccgggccagcaggtgcgcgccggcgagaagctggccgtgatcgaggccatgaaaatggaaaacgtgctgttcgccacgcaagacggcgtggtgggcaaggtttcggccaacaagggcgagtcgctcgcggtcgatcaaatcattctggagttcaattgatgggtgccaacgacctgcaacagccgatcacgctgcacaagccttcgaaagtccctgcgccgcaaggcccctggtcgatcgaggcgatccaggcgctgctcgacaagccgctgatggaactgctgttcgaggcgcagacggtgcatcgccggcactttcccgaaggcgacatcgaactggcgaccttgctgtcggtcaagaccggcggctgtcccgagaattgcggctattgcccgcagtcggccgagttcgacaccggcgtgaaggcgcagaagctcatggaagtcgacgaggtggtgcgcgccgcgcaagccgccaaggacgcgggcgccacgcgcttctgcatgggcgccgcatggcgtgcgccgaaggaccgcgacgtggagaaggtcgcggtgctggtcgaggcggtgaagggcctcggcctgcagacctgtgccacgctcggcatgctggagccgcaccatgcgcaccagctcaaggccgcgggcctcgactattacaaccacaacctcgacaccgcccccgagtactacaccgacatcgtcgacacgcgcacctaccaggaccggctcgacacgctggcccatgtgcgcagcgccggcatcagcgtgtgctgcggcggcatcgtcggcatgggcgagcagccggtgcatcgcgccgggttgatcgcgcaactggccaacctcgatccctatccggagtcggtgccgatcaacagcctggtgcgcgtgcccggcacgccgctggccgattcggaaccggtcgatcctttcgacttcgtgcgcatgatcgccgttgctcgcatcacgatgccgacggcgcgcgtgcggttgtcggccgggcgccagcagatgggcgatgcggtgcaggcgctgtgcttcatggccggcgccaactcgatcttctacggcgacaagctgctggtcaccggcaaccccgatgtggaagccgacgtgcagttgctgcgcaagctcggcctgcaggcgcgccgcacgaccgaagccgaggagcatggcgcgtgaccggaacggcacgtcctttcaaggtgctgggcatccagcagatcgccatcggcggacccgacaagctgcggctgcagaagctctgggtcgacatgctggggctcgaggtcacgggcaccttcaagagcgaacgcgagaacgtcgacgaagacatctgtgcgataggcagcgggccattcaaggtcgaggtcgacctgatgcagccgctcgacccggaaaagaaacccgcagtccacaccacgccgctcaaccacgtgggcctgtggatcgacgacttgcccaaggccgtcgagtggctcacggcgcaaggcgtgcgctttgcgcccggaggcatccgcaagggcgcggccggcttcgacatctgctttctgcatccgaaggcgaatgacgaatttccgatcgcgggcgagggcgtgctgatcgagatggtccaggcgccgcccgaggtggtgaccgccttcaacgcgctcgccgctacgcgttgagcaccttcttgatgggcggcttcacgtcggaacgctgaggcggcagcatcggctggtgctcgcgcgccgggttcaggatgatcgaggtcgcggtctcggtgaggatgcagaacttggtgaccaccgcatcgagatggctcacgtcgatgacggcgatctccaggatccagctgtcgtcgccggtcacgttgtaggcattgacgcattcgggcgtctgctgaaccagctcgaccacgcgtgcatagtcggcgcggccgacacggatgatggcgcggatgccatagcccagcttgccgagattgaccgtggcgcggtagccgctgatcacgcctgcagcctccagtttttttacgcgctcggtcacggccggctggctcaggtgcacgcggcggccgagctcggccatggagagccgtgcatcgccctgcagttcggccaggatgcgggtgtcgtgggcatccagcgcggggttcaaggggaagtccatgcaactcctttaaatcgacggtgcaagacagttggaaccatgaattgtgcatggccgcggaggggtcgctttcataccatcgaaggcgttccaataccaacaagacgacttcgcatgcctactcttgcatcccccgcccaagccgcgcccggatcctcgcgcagcgcgctcccgccgattctctggctctgcctggccgccacctgggtggtctggggctcgacctatcttgcgatcaagtacgcgctgatcagtttcgcgccctttcttcaaatgggttcgcgcttcctgttcgcgggcgtgctgttggccgcctggatgcgctggcgcggcgcggcctggccctcgcgcttgcaatggcgcaatgcgctcgtggtcggcgcgttgatgctgggcggcggcatgggcggcacggcccatgccgaagtgtcgatcggttcggggctggtggtggcgttcatcgcggtggtgccgctgctgatcgcgttgctgaacctggtctggggcgtgaagccgacgcggctggaggcagctggcattgcgctcgggctcgtcggcgtgctgatgctgacgcagggcagcggcttccagtcctcgcccgcgggccttgtcgccatttcgatcgcctgcgtctgctggtcgatgggcagcgtgctgagccagcgcagcctcccgctcgcgcccggcgccatgggttttgcgagcgagatgatctgcggcggcgtggtgctgctggtgctctccgccatctccggtgaagagctggcgtggccgccgcagcccgaggcggtcgcggcctggctgtacctcgtggtgttcggctcgctgatcgcgttcaatgcctacatggtgctgctcgccaaggcgccggccgcgctggccgcaagctacaccttcgtcaatccggtgatcgcgatgctgctgggcgtgtggattgccaacgagaccgtgacgcgcttcgagtggtacgcggtggccgtcgtgctggccggtgtgctgctgttgctcttcaagcgcccgcagaagatgcagaagggctgagtgccgcgccgttcaggtgcccggtcggcgccagaaggcaagcgtggccgccagcagccacatgcccgccgcgcagctgcggttcagcaccttgaggccgcggcgcgacagcaagcgcacggcctgcgttccggcggccgcataggcgagcatcacgaaggtgtcgagcaccacgaagatcgcgcccagcaacaagtattgcgcaccctgcggcttggcaatgtcgatgaactgcggcaggaaagccgcaaagaacagcaccgtcttggggttggacagcgccacgagcaggctgcgcatgagcgcaacgcggccgtgcgggcgaacctcgatggccgacttggccagcgccgtgccgagatcggtcgcctcgctgcgccacagcttgatgccgagccagaccaagtaggcgacacccgccacgcggatcgcattgaagagaagctccgatgcggcgagcagcgagccaaggccgagcgcgaccaccgcgatcagcgtgacgctgccgagcgatgcgccggcaatgccccaactcgcacggcgcatgccgccgtcgatgccgttggatagcgccagcagcatcgtaggcccagggatcaccgccaacgcgagcgaggcgacggcgtagatcagcagcgtgtcgagtgtcatggcttggcggcgggtggacgttgttgggaggcggcgcgggcacgcgccaatgcagcttcgacgatggatcgcttgcgcgtgtcggcggcttgcggttcagcggccggagccgattcattgccttgcggcttgtcggcacggcgatgctcgccatgcaacttgtagcgctgcaacgcggcgtcggcctgggcttgcgaccacgcttgccaaccggtgcggcccggtgtctcgacctcgagcgagatgcagtcgacggggcagaccggaatgcaaagctcgcagcccgtgcagtgcgcttcgatcacggtgtgcatgcgcttgttgatgccgacgatggcatcggtcgggcaggcgtcgaggcagagcgtgcagccgatgcaccaggcttcgtcgatgaccgccatggcgcgtgggccttcggtgccgaactgcggatcgagcggcagtggctcgcggcccgtgagccgtgccagtttggcgatgccttccgcaccgccgggagggcattggttgagcttggcctcgccgtcagccaccgcctgggcgtagccggcgcagtcggggtagccgcagcgcgtgcactgcgtttgcggcagtgcatcgtggatgcgtgcggccagcccgatcacttccttcgtgccgcgggcttcttcacggcggcgaccgccaccgctttcttggctgcgacattcttcctggctgcaacggctggcgtgctccggcccggcttgatccgatcttcggccggcaggctatcgggcgtaccgctgcgccgctggggctggtcgtgagcggcgatgaacttctgcatcttggggtagaccaggtcgcgccagcggcggccgctgaagatgccgtagtggcccgcgcccttgacttcgaagtgttcgcgctgcgagtcttcgatgccggtgcacaggctgtgcgcggcctcggtctgacccgaacccgaaatgtcgtcgagctcgccctcgacggtgagcagggccgtggagtggatgtcttgcgggcgcacgcgctcgatctggcctttggggttcttgacgtcccaggtgccgttcacgagttcgaagtcctggaacaccacgcgaatcgtgtccaggtagtagtcggcgtccatgtcgagcacggcgttgtactcgtcgtagaacttgcgatgggcctcggcgctggcgtcgtcgcccttgatcaggtccttgaagtagtcgtagtggctgctggcgtggcggtcggggttcatggccacgaagcccgtgtgctgcaggaagcccggatacacgcggcggccttcacccgcaaagccttgcggcacgcggtagatcacgttgttctcgaaccactcgaaactcttgttcatcgcgaggttgttcaccgcggtgggcgacagccgcgcgtcgatggggccacccatcatcgtcatggtgagcggcagctgctcaccgcggcttgccatgagtgacacggccgccagcaccgggaccgtgggctggcacacgctcaccacgtggcagttgccgtactcggcctgcaggcggcggatgaactcctgcacgtagttgatgtagtcgtcgaggtggaactcgccttcggacatcggcacgaggcgcgcgttcttccagtcggtgatgtagaccttgtggtcctgcagcatggtgcgcaccgtgtcgcgcagcagcgtggcgtaatggcccgacagcggcgccacgaccagcaccacgggctggctcttgagcgtcttgaggatgtgcggctcgtcggtgaagcgcttgaagcggcgcagctcgcagaaaggcttgtcgagctcgacggcctcctggatgaccacatcttcgccctcgaccttcacggacttgatgttgaactcgggcttctcgtagtccttgcccagccgatagagcaggtcgtaacccgccgccatgcgctgggccatgggtgcttgtccccagacggcaccttggccgaacagcttggacgccgcttgcgcgaagtccgaaaacggttccatcagggaacgctgggcttcgtagagttgatagagcatcgctgatcttggagtggaatgttgcggtgcaatatatcagcgccaattgccttggcgcagggggccttcccctacgtagattccaccgcagggcttacgttttcaccaaatgtgaaggaattgtcgcgaaacgcattccctcacattttcctgacagtcagatgaccttggcaatcgaggcgcagacgtagtcgatgttcttgctgttgagcgcggccacgcacatgcggccggtgtcggtgccgtacacgccaaattcgttgcgcaggcgcaccatctggtccttgctgaggcccgagtagctgaacatgccgatttgcgtggtgatgaagctcatgtcttccttcacgccggcggccttgaggccgtcgaccagcttctggcgcatggccttgatgcgcacgcgcatttcgccgagttccttttcccagagggcgcgcagttcggggttgccgagcaccgcggcaaccacggcgccgccgtggatcggcgggttgctgtagttggtgcggatcgcgatcttgagctgcgagagcacgcggccggcttcttccttgctttcgcacagcaccgacagggcgcccacgcgctcgccgtagaggctgaagctcttcgagaacgaggtcgagacgaagaaggtcaggccggcgtcgacgaacttggcaaccgcggcgccgtcttccttgaggccgtaaccgaagccctggtaggccatgtcgaggaaggggacgagatttttggccttgacggtggcgacgacctggtcccactgctcggacgtgatgtcgtagccggtcgggttgtggcagcaggcatgcagcacgacgatggtgccggccggcgccgcgttcagggcggccagcatgccgtcgaagttgatgccgcggctggcggcgtcgtagtaggggtagctttcgacctcgaagcccgcgttggtgaacagggcgcggtggttttcccagctcgggtcgctgatcagcaccttggcgttggggttgagcttcttgagaaagtcggcgccgaccttgaggccgccggtgccgccgatggcctggatcgtggccacgcggcccgattgcacaggttcgctgtcgacgccgaagaccaggcccttgaccgcgttgtcgtacgccacgatgccgtcgatcggcaggtagccacgcgccgagggcgctttcatcatgttctgttcggcggcctgcacgcactggagcaggggcagcttgccgttgtcgtcgtaatagacgccgacgccgaggttgaccttgttggggttggtgtcggctgcaaactgctcgttgaggccgaggatcgggtcgcgcggtgccatttcgaccgcggtgaacatagacatggaaaggtcctttggatgaaagcttcgctggcaaccggaggaggctttatcctttccggttgccttgaattttaccggcgctaccgccacctgtcgggaacagccatgccagagaacaacgaagccatagcagacctgaagaaactggacccgatcggtccggcaaaacagggcgaattcatcaaatatccgggttcgcctttcgaacttttccagccctatccgcccgccggcgaccagccgaaggcgattgacgggctggtcgagggcgtgctggacggcgaggtgttccagacgctgctgggggtcaccggatccggcaagaccttcaccatggccaacgtgattgcccggctgggacgcccggccatcgtgtttgcccccaacaagacgctggcggcgcagctctacagcgagtttcgcgagtttttcccgaagaacgcggtcgagtatttcgtcagctactacgactactaccagcccgaggcctacgtgccccagcgggacctgttcatcgagaaagactcgtccatcaacgagcacatcgagcagatgcggctgtcggccaccaagagcgtgctggagcggcgcgacacggtcatcgtggccacggtgagcgccatctacggcatcggcacgcccgaggactacacgcagatgcgtttcatcatgcgggtgggcgacaagatcggccagcgcgacgtgatcgggcggctgattcgcatgcagtacacccgcaacgagcaggatttttcccgcggcaccttccgcgtgcgcggcgacaccatcgacgtgtttccggccgagcacagcgaactggcgatccggatcgagctgttcgacgacgagatcgagacgctgcagctgttcgacccgctcacgggccgcatccgccagaagattccgcgcttcacggtgtacccgtcgagccactacgtgacgccgcgcgacaaggtgctgggcgccgtggaaaccatcaagatcgagctggccgagcggctcaaggaattcgtcagccagggcaagctggtggaggcgcagcggctggagcagcgcacccgcttcgacctggaaatgctggccgagatcggccactgcaagggcatcgagaactactcgcgccacctctcgggcgccgcgccgggcgacccaccggccacgctgaccgactacctgccgaaggacgcgctgatgttcctcgacgagagccaccagatgatcggccagctcaacgccatgtacagcggtgaccgggcgcgcaagaccacgctggtcgagtacggctttcgcctgccgagcgcgatggacaaccggccgctcaagttcgaggagttcgagacgcgcatgcggcaggcgatcttcgtttcggccaccccggcgcagtacgaaaaggaccacgccggcaacgtggtcgagcagctggtgcggccaaccggcctgatcgaccccgaggtcgaggtgcgtcccgccacgcaccaggtggacgacgtgctgggcgagatccgcatccgcgtcgagaaaaacgagcgcgtgctcatcaccacgctgaccaagcgcatggccgagcagctgacagactacctgggcgacaacggcgtgaaggtgcgctacctgcacagtgacgtcgacacggtcgagcgggtggagattttgcgcgacctgcggctgggcaccttcgacgtgctggtaggcatcaacctgctgcgcgaaggcctggacattcccgaggtgtcgctggtggccatcctcgatgccgacaaggaaggctttctgcgcgccgagcgctcgctgatccagaccatcggccgggcggcgcggaacctgagcggcaaggccattctgtacgccgaccggatgaccgactcgatgaagaaggccatcgacgaaaccgagcgccgccgcgcccggcaaattgcccacaacgaggccaacggcatcaccccgcgcagcatcgtcaagcaggtccgcgacctgatcgacggcgtctacagcgaaaaaaccggcaaggaaatggccaagctcgacctggaacgcgccaaggtcgaggacatgagcgaaaaggacattgcccgggaaatcaagcggctcgaaaagctcatgctcgagcacgcccgcaatctcgagttcgagaaggcggcgcgggtgcgcgaccagttggcgctgctgcgtgagcaggcgtttggcgcctccggcggggacaatatcgctgtgttgccgtcgtaggacggggtttcggtttcttcaaggggttttcgctggggtttacccgagcaaactccagggccttctgctatacttgaccgaaacactcaacaacaagaaaaaagaacttcgcgatgaaggaccgatcccactgactggttcaccagcatcaggggtcgggcagggcggagacgaagtcaccgcggccccccgtgccacggtgtcatttcaacggtaagcacttgaaggagcttgcgatgcgtctcactaccaaaggccgttttgcggtcacggcaatgatcgatctggcgttgcgtcagaacaccggtccggtcacgctggctgcgatcagccagcggcagcaaatttcattgtcgtatctcgagcagctgttcggcaaattgcgccgtcacgagttggtcgaatcgacccgcggccccggcggcggctacagcctgggtcgcaaggcagccgatatcaccgtcgcagacatcattgtttccgtcgatgagcccatcgatgccacgcagtgcggtggcaaggaaaactgcctcggcgaagccggccgctgcatgacgcacgagctctgggcgtcgctgaaccagcgcatggtcgagtttctcgattccgtcacgctgcagaagctggtcgacgaccagatcgccaagggcgttcagatcgagaacaagccggtcgtcaagcgcgccatttccgcgcagcccgtggtcaagccgattcgcgtgaatgcgccgaattcggtgtttgccctgggcaacgcgttcgcgaagtcctgatgccctctgtcgcaggcggcgccttcgggcgctgctgcgaaaagccgcccagaccaaagaaacaacccccacgccagcccgagccagccatggacgtcactcctcatttcccgatctacctcgattacggcgccaccacgccggttgacccgcgtgtggtcgacgccatgattccctggttgcgcgagcatttcggcaacccggcatcgcgcagccatgcctggggctgggaggctgaagaggcggtcgagaaggcgcgcggccaggtggccgacctgatcagcgcagatccgcgcgaaatcgtctggacgtcgggtgccaccgagtcgatcaatctggcgctcaaaggcgcggcccatttctacaagggcaagggcaagcacctgatcaccctgaagaccgagcacaaggccgtgctcgacaccatgcgcgaactcgagcgccagggcttcgaagtgacctacctcgacgtcgaggaaaacggcctcgtcgacctggagaagttcaaggccgcgctccgtcccgacaccatcctggccagcgtgctgttcgtgaacaacgaaatcggcgtgattcaggacgtggtcgcgctgggcaacgtctgccgtgagaagggtgtgatttttcacgtcgactcggcccaggccaccggcaagatcgacatcgatatcacgaagctgcccatcgacctgatgagcctcgcttcgcacaagacctacggcccgaagggcatcggcgcgctgtatgtgcgccgcaagccgcggatccgcctcgaagcgcagatgcacggcggtggccacgagcgcggcatgcgttcgggcaccttgcccacgcaccagattgtcggcatgggcgaggcctatcgcatcgccaagctcgaaatgaaggacgacatcgcccatgctgcccgactgcagaagcgtctgctcgacggcctgaaggatgtcgagcaggtgttcatcaacggcgacctcgcgcagcgtgtgccgcacaacctgaacatgagcttcaactacgtcgaaggcgagtcgctgatcatgggcatcaagggcctggcggtgtcgtcgggttcggcctgcacgtcggccagcctggagcccagctacgtgctgcgcgccctgggccgcagcgacgaactggcccacagcagccttcgcatgaccatcggccgtttcacgaccgaggaagaaatcgactacgccatctcgaccatcaagcacaacgttgccaagctgcgcgagctgagccccttgtgggagatgttccaggacggcgtcgacatcagcacgatccagtggtcggcccactgacgcattgacgtactggcccaccagcgctccacgattgaacaaagtttgagaggtacaccatggcatattcttccaaggtcatcgaccactacgaaaatccacgcaacgtcggctccttcgaaaagggcgacgattccgtcggcaccggcatggtcggcgcgccggcctgcggcgacgtcatgaagctgcagatcaaggtcaaccccgaaaccggcgtgatcgaagacgcgcgcttcaagacctacggctgcggttccgccatcgcctcgtcctcgctcgtgaccgaatgggtcaagggcaagacgctcgacgaagcggctgcgctcaagaacgcgcaaatcgccgaagaactggcgctgccgccggtcaagatccactgctcgatcctcgcggaagacgccatcaaggcggccgtgagcgactacaaggccaagcacggcgccaagaccgccgaagctgttcactgagatggccgtcacgctgaccgaagccgctgcgcgccacgtcacccgctaccttggcaaacgaggcaagggcgtgggtgtgcggctgggcgtgaagaccaccggctgctccggccttgcctacaagctcgagtacgtggacgagttcacgcccgaagacgtggtgttcgaagaccatggcgtgaaagtcctggtcgatccgaagagcctggcttacatcgacggcacgcagctcgacttcgtgcgcgaaggcttgaacgaaggcttcaagttcatcaacccgaacgaacgcgaccgttgcggctgcggggaaagttttcgcatctgatgcactgtcgctgaccgcgacaacagccgccaccatgtcatgtgctggcggttttttcttgatccatatgagcccccacgttcggcactttgtgtcctcactgctccgcgagggggcgcaggcagtctgatgaacctgaacgacaccgactttcaactgttcgccgtcccggccactttcgcgcaggaccgcgccgctctcgacgcgcgctggaaagagctgcagcgggaggcccatccggaccgctttgccgcgcaaggcgccgcggcgcagcgcgtggccatgcagtggtcggtgcgcatcaacgaggcctatcagcggctcaaggacccgatccggcgtgccagctacatctgcgaactcaacggcgcgccgctgaatagcgagaacaacacggccatgccacccgacttcctgatgcagcagatggaatggcgcgaggagctcgacgacgccggcgacatcgcggcgatcgagaagctgcaggccgaggtcgaagccggccgcgcccgcgcgctgtcctcgctcgactggctgatcgacgagaagggcgactatcccgctgccgcgcagcaggtgagagccctcatgttcattgagcgtttcgggcaggacgtcgaagccaggttcgatcagttgggacaataggccttatatatggctcttctacagatttccgaacccggccaggcgcccgatccgcatcagcgccgcattgccgtgggcatcgacctcggcaccacgcattcgctggtggccgcggtgcgcaacggcgtggccgaatgcctgcccgacgaccagggccgcgtgctgctgccttcggccgtgcgctacctggagggcgaccgccggcagatcggcttcgacgccgtggcggcgcgcgggcaagaccccgccaacactatcacctcggtcaagcggctcatgggccgcgggctcgccgacatttcgaaccgtgaatcgatgtcgtatcacatcgatggcagcgagggcggcatggtgaaggtgcagaccctcgcgggcgagaagtcgccggtcgagatcagcgccgaaatcctggcgacgctgcgcttccgcgccgaagacaccttcgacgacgagctctacggcgccgtcatcaccgtgccggcctacttcgacgaaggccagcgccaagccaccaaggatgccgcgcagctcgcgggcctcaacgtgctgcggctcatcagcgaacccacggccgctgccatcgcctacggcctggacaacgcaagtgagggcgtctatgcggtctacgacctgggcggcggcactttcgacatctcgatcctgcggctgacgcagggtgtgttcgaagtgatcgccaccggtggcgactcggccctgggcggcgacgactacgaccacgcgctggccggcttcgtgctcgcgcagaccggcctcgaagtcggcagcgacaacgacaaggccgccatgctcgtggccgcacgtgccgcgaaagaggcgctgaccgagaccgagtcgaccaccttccgtgcggagcttgcaggcggggcgattcaattcgaactcacacgccatcagttcgacgccgccaccaaggcgctcaccgaccgcacgattgcatcggttcgcaaggcgctgcgcgacgccaggctcaagcccgacgatctgaagggcatagtgctggtgggcggttccacgcgcatgccccagatccgccgcgccgtggccgagttcttcgggcgcgagcccttggtcaacctgaaccccgacgaagtcgtggcgctcggcgccgccatccaggccaaccagctggccggcaacaacggcgcgggcgatctgctgctgctcgacgtgattccgctgtcgctgggcatcgagaccatgggcggcctggtcgagcgcatcgtgccgcgcaaccagaccatcccgaccgcgatggcgcaggacttcaccacctaccaggacggccagacggccctggcgctgcacgtggtgcagggcgagcgcgacctggtggccgactgccgcagcctcgcgcgcttcacgctgcgcggcattccgccgatggcggcgggtgcggcgcgcatccgcgtgaccttcactgtcgatgccgatggcttgctgagcgtcagcgccaaggagcagggcagcggcgtcgaggccagcgttaccgtcaagccttcgtacgggctctcggacgaccagatcgcgaccatgctgcaggagagcttttccaccgcgcagcaggacatgcaggcgcgtgcgctcgtcgaggcgcgcgtcgatgccgagcgcatgctgctcgccacgcagagcgcgctcaacgccgacggcgatctgctgggcgaacaggagcgtgcggtcatcgatgcatcgatggcgaggctgcgcgaggccgcgaagggcagcaacgacgcggcggccatcgaggcggccaccaaggccctggccaacgacaccgaagcttttgccgcccagcgcatgaacgcgggcattgcgcgcgcgttgtcgggccgcaaggtcgaatccctctaagaactacatgcccaccatcaagatatttccgcatccggaatactgcccgacgggtgcagaaatcacggcgccggccggcacctcgatctgcgaggcgctgctggagaaccacatcaacatcgagcatgcgtgcgagatgagctgcgcctgcaccacctgccacgtcatcgtgcgccaggggttcagttcgctgaacgaagccgaggagggcgaagaagacctgctcgaccgcgcctggggcctggagccacaatcgcgcctcagctgccaggccatcctggcgcagcaagacgtgacgattgagattcccaagtactcgatcaaccacgccaaggaaaatcactgatgtcgcgccagatcgtcctcgatactgaaaccaccggcctttccgccgagaacggcgaccgcgtcatcgagcttggctgcgtggagctgttcgcgcgcaagctcaccggcaacgacctgcacatctacttcaaccccgagcgcgagagccatgaagacgcgctcaaggtgcacggcctgacgaccgacttcctgcgcgacaagccgaagttcgccacgctggccaacgacatcgtcgaatacctgcgcggcgccgaactgatcattcacaacgcggccttcgacgtcggctttctcaacaaggagctcgagctcgcaggcctgcccccgctgcgcagcttcgtcggcgaagtgaccgacacgctggccatggccaagcaggtctacccgggcaagcgcaattcgctggacgcgctgtgcgaccgcttcggcgtcgatcgctcgaaccgcaccttccacggcgccaagctcgacgcgcagctgctggccgacgtctacatcaacctcacgcgcggccaggatgcgctcttgatcgacgtgtcgtccagcgagccggcgcagggcaccaccgtcgtcaccatcgacctgagccagttcgacctgccggtgatcctggcgggcgaacaggagcttgcggcacacgaagcgctgttgtcgcagctcgacaaatccagcaacggacgcacgctgtttcgccaaaacggctgaaatgctgtggcataatcgaaggcttcgcgcaacgcgattaattccaaggcactgcaactgcggcgccaaggggtttgcagggcggttagctcaggggtagagcacagcattcacactgctggggtcggaggttcgaaacctccaccgcccaccaatttcctcgaaatgaacagcgacttggattgcccaggtcgctttttgttttgtgcgctgccttttcgctccggcaaggcggcacatgcgcggctcccttcaactgtcggctcgtgctgacgccagctgccgtctcgcaccggctcaatttgctggcggagcgcgtatacccaccgggaaggagaccgatcatggccactcatcccgacatcccgcccgacctgcccgtggaacccgacgaagggccgagcacgccgccggacgacccgaccgatcccgagcctcctcccaccacgtcgtgaatccggcgcgcgagccgcgataagctcgcgccatggatgaacttgattgcgccgtcatcggcggcggagtggtgggcttggccgtggcgcgcgcgttggcgctcgcaggccgtgaagtggtggtgctggaggcggaaggtgccatcggcacgggcaccagttcgcgcaacagcgaggtgattcacgcgggcatctactatccgcaaggttcgctcaaggcccgcctttgcgtcgagggcaagcaggcgctctatgcctacgcggcggagcgaggcgtgccgcaccggcgctgcggcaagctcatcgtggcgacttcgcctgagcaggtgggcgagcttgaaaccatccgcgccaaggcggccgccaacggcgtcgacgacctcgtgctgctgacggcgcagcaggccatggcgatggagccgcagctgcattgcgaagcggcgctgcattcgccgagtaccggcatcgtcgacagccacgcactgatgctgagcctcttgggcgacgtggagaacgcgggcggcatgctggcgctcaagtcacccatcgcgcgggcggaatgcggcacggacgccatcgtcctggtcgcggaagacgggacggcattgcgctgcaacaccgtggtcaatgcggcgggccttggcgcccctgacctcgccaggcggttcgaaggcttgcccaccaccgccataccgaccgcctacttcgccaagggcagctatttcaccctgtcgggccgtgcgcctttcagccggctcgtctatccggtccccgaaccgggcggactgggcgtgcacctgaccatcgacctgggcgggcaggccaagttcgggcccgacgtgcaatgggtgcagtcggccgacgacctagtggtggacccggcacgcggcgacggcttctacgccgaggtgcgcaagtattggccggccttgcccgatggcgggctgattcccggctacgcgggcatgcggcccaagatctcgggtccgggcgaacccgcgcgcgacttcatgatcgaggggccaaaggcgcatggcgtgcgcggcctggtcaatctcttcggcatcgagtcgcccgggctcacgagcagccttgccatcgggcgctacgtcgcaagcttgctcgacggcagctgacggaagcaatgcgggccccgcgtgcagaagtctgcagaactgtcgcgcacgaggggcttttgtgcctgtaacatgacaccacgccattagctggcgtgaagccgccggcgcggtgccggtgtcatcacggaggaaagattccaatgagtgcatccaacaacatcgaagcggcagccgaagacatcgcgagcgacgtgcgcggcgtgctggccagcaaggacctggattcggttccccacatcaaggcgctgcgtcagcgcatcgacaccaagctcgccattgcgcgcgagcttgcggcagagaagagcaagcttgcagcccagaaggcccgtgaagcggccaacagtgccaacgcctacgcccacgacgaaccgtggcagattgccggcgcagcgctggccgtcggcgtgctggtgggtttgctgcttggccgccgctgacctgaacgcacactgccgcgtcgtccaccgccgagcgggagccggcgcatgaggttgctgtccctgttcgggctcgacgcccgtctgcgacggctgcggattgctgcggccgaaggcgcgctggccgccgaagaccgtgtgcagttgctgcgcatggcctgggaggacgagaagcagcgcctcaagctgatgctcgtcttggtggttgccgtgctcggcctgaccacggtggctgtggccttgctgtcgatggcggtggtggtgcatttctgggaaacgcctcaccgcatcgcggcggcgtgggccgttgctggcgtgtggatcgtgctttggctgggcgccgcatcgggcctgtacctgagccttcgcaatgcctcgaacagcttcatgccggcgcggcacgagtttgaacgcgactgggcctgggttcaggacagcttcggactcggcaaggatccagaccaggacgaggaagcgccgcgcccgccgcggccagccacgcgcgaagagctgctcgcgcgcatggatcgccagcgcgaacgcatcgccacgatgcagggcgcaggcgcggcgcagcagtctgcaggcgcagcagggggctcttcttccgaagcgcctccgaccgacgagtcggctgccgccgcggcattgcgcatcgcgcgggagcacccggttgccacaggcgtggtggccgcggtggccgtggtggtgatccgtcccaggcggctgctgcgctgggcggcgttcattgcgccagtgctctggcgcatgcgctgagagagaagagaaaaaagaagcgaacgaaggctcaggcggcgctgcggctttgctgcagcagcgcctgggccgcttcgcgcacaagggccgggccgcggtagatgaggccggtgtagatctgcaccacgtcggcgcccgcggcaatcttggccttggcatcggccgcgctcaggatgccgccaaccccgatgatcggaaaacccggccccagggcggcccgcagctgcgcaatcacgcggttgctggcttcgcgcaccggcgcgcccgagagtccgcccgcttcgccggcatgcggcaggcccgccaccgcgtcacgcgccagcgtggtgttggtggcaatcacgccgtccatgccgtggcgctgcagcgtggcggcaatcacggcgacctggttttcgtcgagatcgggagcgatcttcacgaacagcggcacgcgccggcggctgcgttcggccagcgcatggcggcgctcggcgatggcacccagcagggcatcgagcgcctcgtcgctttgcagcgtccgcaggttggccgtgttggggctcgagatattgatggtcacgtagtcggcatgcgcatacacgccgtccaggcaagccaggtagtcgtcgaccgcgcgctcgatgggcgtggtggcgttcttcccgatgttgagcccgagcagcatcggcttcttgccggcgctgccgccgccgttcttgcgaaagcgggccttctgcacgttggcgagaaaggcatcgagcccttcgttgttgaagccgagccggttgatgagcgcatcgcgctgcggcagacggaacatgcgcggcttggggttgcccggctgcgccttgggcgtcacggtgccgacttcgacgaagccgaagcccatggcggcaaaagcgtcgatgcagcgggcgttcttgtcgagcccggccgccagcccgacgcgattcggaaactccagcccggcgagcgtaaccgggtcatcgatgcgcggcgcggcgtaggcgcaggccagcggcgtgttctgcgtgcgggccaggccgtcgagcgtgagttcgtgggcgtgctccgggtcgaagccgaacagaaagggccgggccaggccgtagagcgaagaggggagcaggagcatcggataattctcgacttcaatgagccaaggattctccgcgatgaccgcacccgtttctccttcttccgctcccggcgccgccgccatctctcaggacgagctcaaggcccaggttggccgcgccgcgctggcctacgtggtgaagggtgaaatcgtcggcgtgggcaccggctcgaccgtgaacaagttcatcgacgcgctggccacgatcaaggaccagatcaagggcgcggtgtccagctcagtggcttcgaccgaacgcctgcgcgcgctcggcattccggtgttcgacagcaacgaggtcgaggagctcggcgtctacatcgacggcgccgacgaaatcgaccaccgcggcttcatggtgaagggcggcggcgcggcgctcacgcgcgaaaagatcgtcgcggcgcagtcgcggcgcttcgtctgcattgccgatgcgtccaagctggtcgatacgctcggcgcctttccgctccccgtggaggtgattccgatggcggcgcgccgcgtgatgcgccagttcgaggccatgggcggcattgcgcaagtgcgggaaaaagacggcctgccgctcgtgacggacaacggtcagcacatcgtcgacgtgacggggctgcggatcagcgatccgctggctttcgaatccgaggtgagccagtggcccggcgtggtcacggtcggcgtgttcgcgcgccagaaggccgacgtgtgcctgctcggcacgccttccggcgtgcaaaccatgcagttcgactgaaaaagcctttggcagcaaaggcccggcggccgctcagaacttgatgcccgctggattgctcgggctcgggccactgggagcgggcgcggcctgctgcggcgcaggcgccggaggtgctgcctcgggcgcagcgggtgccgcctgctgcgcaaccaacggacgggccggcggattgcggtagccggcaggcaggctgttgctcttcgggtagcccgcggcatcgaggtattgcgaccattcggcgtcggagaaacccttgagctgctgcgcaccgatcgtcagcagcggcagcgaagcctgggcggtcagccgctgcagggcctcgacgtcctggttgctcttgacggtgcgctcctcgaaggggacgccgcgcgtggtgagcatcgagcgggcggtgctgcaaggcgcgcattcctcgccgctgtacagggtgacgggatagcgctgcgccacctgccgcaactcatagggcaggccggcgttggcgggcggcgcgctggcggcctgcggcccggcggccggttcggtgctggcggtgggcgcgcggtcggagaaagtgactttgccgttcttgtcgacgttgcgatagatcggctgggctatggcacccgcggcaatcagcagcagggcggtggcggacaggcgatgcaagggaaatttcttgtggatcgaaggcatcgcccgagtatcgcaagcttcaggcccgcatcaagcgggctgggcctcggccatgccctggtgtcgcagcaatgcatcaagctgcggctcgcggccgcggaaggccttgaacgaatccatggcgctgcggctgccgcccgcttcgagaatggcctggcggtaacggcggccggtttcgatgttcggctggccgtcggcgcccacggtttcctcgaaggccgcataggcgtcggcgctcagcacctcggcccacttgtagctgtagtagccggccgcgtagccgcccgagaagatgtggctgaaggtgttgggcgtgcgactgaagggcggcgagggcatcacggccacctcggcgcgcaccttgccgagcagcgcgagcacaccgcccggctgcgcggtggctgcctggtattcggtgtgcagcagcatgtcgaacagcgagaactcgatctggcgcagcgtctgcaggccgctctggaagttcttggcggcggtcatcttgtcgaacagcgcgcgcggcagcggctcgccggtatcgacgtgggccgtcatgtgcgtaagcacgtcccactcccagcagaagttttccatgaactggctcggcagctcgacggcgtcccactcgacgccgctgatgcccgagacgtcgcgctcgttcacctgcgtgagcatgtggtgcaggccgtggccgaattcgtggaagagggtggtcacgtcgtcgtgcgtgagcagcggcggcttgccgtccacaccgctcgcgaagttgcacacgagctgcgccaccggcgtttgcagcgcgccatcgtccggccgcagccagcgcgcgcgcacgtcgtccatccaggcgccgccgcgcttggcggcacgggccgatgggtccaggtagaactgacccaccttctggccggcccgctcgatgcgatagaactcgacgctcggatgccacgtgggcgcgctgtcgcggcgaatggacacctcgaagagcgtctcgacgatcttgaacaggccggccatcaccttgggtgccgggaaatactgcttcacctcctgctcgctgaaggcatagcgcgcctccttcagcttctcgccgatgtagctccagtcccaggcttgcggatcggtgatgctcagttgttccgacgcgaacacgcgcagatcggccaggtcgcgttcgccatagggcttggccttggccgcgaggtcgcgcaggaacttgaccacctgctcgggcgattccgccatcttgggcacgaccgagagttcgccgaaattcttgtagccgagcagctttgcttcttcttcccgcagcgcaagaatctcgctgatcagcgccgtgttgtcgaaggccggatcgccgagttcgctggcgcgcgtgacgtacgcgcggtagagcgtttcgcgcagcgcgctgctcttggcaaactgcatcacgggcaaatagcagggcatcttgagcgtgagcttgtagccttgcttgccttcggcttcggcggccgcgcgcgccgcgccaatcacgtcttccggcacgccgtcgagctcgcccagcgctgcgtaataggagaaggcgtcggtggcgtcgagtgcgttctcgctgaatttctggctcagctcggcctgccgttcctggatgtcggcaaagcgcttcttcgcgtcgccctgcagttccgcgccgccgagcacgaagttgcgcaccgcattgcgatgcgcctggcgctgctcggtgttgagggtggctacgtcgatggccttgtactttgcatacaggcgctcgtccgagcccagacgggtccagaacgccgtaacgcgcggcatggcctcgttgtaggcggcgcgcagctccggcgtatcggctacggcgttgaggtggccaaccgcaccccaggcgcggctgaagcgttcggacgccacgtcgagcaccttggaaatcgcattccagtcggctggaaagtcagccgcggtgacggtctgcagcgccgcctccgcatcggccagcaagatgtcgaccgcaggcgcaacgtgctcgggcttgatgcggtcgaacagcgggagatcggcgaaatcgaggagggggttggtcatggagatcactttgcggcgcgttccgcagcttcaagggtgttggcgagcagcatcgcgcgggtcatggggccgacgccgccgggcacgggggtgatccagctggccacttccttcacgccgtcgaagtcgacgtcgcccgcgagcttgccgtcttccttgcggttcatgcccacgtcgatcacgaccgcaccgggcttcaccatgtcggccgtgagaatgttgcgcttgccgaccgcggcaaccaccacgtcggcctggcgcgtgatggcggccaagtcctgggtggcgctgtggcagatggtcacggtggcgttcttggccagcagcatcatggccatgggcttgccgacgatgttgctgcggccgatgaccaccgcatgcttgccgcgcaggtcgtagccgatggattcgagcatcttcatgcagccatacggcgtgcagggccagaagccgggcgcaccggtcatcagcgcgccggcgctggccacgtgaaaaccgtccacgtccttggccggcgagatcgtctcgatgactttctggctgtccatgtgcttgggcagcggcagttgcaccaggattccgtgcaccagcgggtcgtcgttgagggcgcgaatgcgggccagcagttcggcctcgctcatgtcggcgggatagcgttccagcgtggcttgcagcccggtttcggtgctgtcgttgaccttgtgcttcgtatagacctggctggccggatcctcaccgacgaggatgatggagagggccgggttcacgccgctggccttcagtgccgcggtacggccggcgacctcggcgcggatggtttttgcgagggcgttgccgtcgatcagttgggcggtcatcggtttcgattttccaagtaaaaacgcccgcttgcgcaggcgtggtggacatgtattgctatcgggacgatagcttctaggccttggagggcgccgcctgcccgagggcgatcttgagcagatcggccacggtgttggcgttgagcttttccatgatgttggcgcggtgcgcctcgaccgtcttgatgctgatgcccaggtcgtcggcaatctgcttgttcaggcggccggccacgatgcgctcgagcacctgggcttcgcggccggtgagcttggacagcagcgcgtcgcggctggccgattgctggtgctgggtgaaggcaccgcgcgcatgctcgagcatgcgctcgaccagcgtgacaagttcttcgtcgttgaacggcttctggatgaaatccatggcgcccttcttcatgctgtcgacagccatcggcacgtcgccgtggccggtgatcaccacgatgggcagcggggagcgccgctcgatcagccgatcctgcagttcgaggcccgtcatcccggccatgcggatgtcgacgatcagacaagcgacttcgcgcgggtcgtatcgggaaagaaaggactcggcggaatcgaaacagcggaccctgtagtccttgccttcgagcagccattgcagcgaatctcgtaccgcctcgtcgtcgtcgacgacatagacagtgcccttcttcggaatcaaactcatgcaggtacctttgcctcgtcgcttgctacggaactgggagcatccaacaccggaatccagaaggaaaaacggcatccgatcacatccgggccattgtagatgttctccgcctgcatgcgcccgcgatgcgactcgacgatggtgcggcaaaggttcaacccgatgcccatgccttccggcttggtagagaaaaatgcttcatacagccggtccatcacttcgggcgccaggcccttgccggtgtcctgcaccgagaattcgatggcgttgtggccctcgatcaccttcggcagcacgcgcagctcgacgctccggcgcgccagggggcgctcggcaatgtcgatcgcctcggctgcgttcttcagcaggttgaccatcacctgctcgatcaggatcgggtccacctgcaccaccggcagacgggccgccacgtagtggttgagccgcacgttgcgccggcgcagctcgatgcccgcgagctcgaccgcctcgctcaccatggtggcgacgtcggcggcggtgcggttgggctcgctgcgcttcacgaaggagcggatgcgctggatgatctggcccgcgcgctgcgcctgcttcgaggttttttccagcgccgcgagcagcgcgtcggagtcgatcgcctggcccttgatgcgcgacatcatcccgttgcagtagttggtgatggccgtcagcggctggttgagttcgtgcgccacgctggaggccatctcgcccatcgtgatcaggcggctcgcggcctgggcgcggtcggcctgcgcggccgcctgctcttcggcgtcgcgccgcggcgtgatgtcggtggcaatcaccagctgggcgagccggccgtcgacccatgtgaggtagcgcgaacgcacctcgagccatttgcccaggtgcggcacgaagatctcgttgttggcggtctgggcggcggtcagggtatcgatcggcaggccggcgtaggggtcgacgtcgtccaagccctcgtcgtgtgcattggaggcgggcacgccggcttgcgccaccatgcccaggtggcccacggtgtcggagccgaaccaaagccggtacagcttgttcgcgaacagcagttcctcgctgccgatgggcgccaccgacaccgcggcatcgagcgcctctagcactgtggtgaagcgctcgtaagacgccgacaactgctcgcggatgcgcgtgggctcggtgatgtcggtcatcgacgtcatccatccggtctggtggccgcgcgcgtcgatcagcggcgacacatagagccgggcgttgaacacgctcccgttcttgcgtttcacgcgcacctggaagccgccgggcagggcgcgcccgtgcagttcttcttcgaggcgctcgttcatgacctcgcggtccgattccagccagtaggggaagggcggcgattgccccaccagctcggcctcgctccagcccgtcatggcgcagaaagcggcgttcacgtaggtgatgcggccctgcaagtcgagcacgcgcatgccggtgagcatggagttttccatggcgcgccggaaattggtctcggccaccagccgctgctgggcctgctggcgccgccgggtgtggcgccaggtgccgatcagcatccagctcgtcagcacgctgagcgcgcagaccagccagaagaggccattgccgaccaccccctgcgaggtacggtaggcctgggcccgcagcaccagcgcgttgccgacgggcgacaccggcacttcgtattcgttggttctctcggaccagggcaagagccgcgtgccgctctccctggtgctggcggtggtgttgcccgcgatcacgttgcccttggcatcgagcagcgaaacggcatagcgcgcttgcacttccgagggcatgccgtagcgcagcaggccgtcgaccgagaactcgcccagcaccacgcccgcgaacaggccctggtcgaaaagcggaatgtgcagctgcaacatggccgtgggatcgccgccggcgatcggctgcgagaaaaccggctggcgcagctcgcgcgccagcgcgtagttgctctcgatgtcgcccgggcgaagcacgtcgccgatcaggtgctgctgggcgggatgcacgctcggcgcggagtagccggccttgaagcggcgccggtcgtcgatccaggcgacggtctgcaactcgggaaactggctcaccagcgattcggcccggctcgcgaactcgaccggatcgatctcccggttcgaggcgtcgcgcgcgatgcgcatcagctgctcctggcgttcaaggaggcgcaggcgcatgcgctgctgggcgtactcgacgtcgcgccgcaccgactcctgctcgcgctcgacctcttcggtgcgcagataccagaacgacgagacgatggcggcgagaaacagcagcaccgccgcgatcggcgcgagcatggcgacggcgtcctgcagcaccggtgtctgccggcgccaccagcggcgccaccacgagaggagcgacacattcacggcgctgcgggccgccgccagcggagagggaaaaggcatcttgcgagtttaggggatgccccttgcgcgataagtgaaatgctgcagtgacactggttgcggcacggttggccgccagataggtctgttttaaaatatcacattaagaaatcatcatgcgccatttgaaatatcggaatttctgtgcgaaactcgcccgcgtttattgcagagcgcactaaattacagccacagccctaaaaggagagacaagcatgtcggcaaatccagagaacctgttcggctcggccgcgaacgacgcggacgcccaggaaacccgtgaatggatggatgcactgtcctccgtgattcaaagcgaggggcctgagcgggctcactttcttctggagcaattgctcgagcatgcgcggcagcacagcatcgacaagccgttctccgccaataccgcctacgtcaacaccctggagcccgatcaggaagagcgttgccccggcaacctcgagatcgaggagcgcctgcgcgcctacatgcgctggaacgccatggccatggtggtcaaggccaaccgccatcatccgcccgaaggcggcgacctgggcggtcacatcggctcctttgcttcgctggccaacatgttcggcgccggcttcaaccacttctggcatgccgagagcgaaaaccacggtggcgactgcctgtacatccagggccacgtttcgcccggcatctatgcccgcgcctacctcgaagggcgcctgagcgaagagcaattgctcaacttccgccaggaagtggacggcaagggcctgtccagctacccgcatccgaagctgatgcccgagttctggcagttccccacggtgtcgatgggcctgggcccgctgatggccatctaccaggcccgcttcctcaagtacctgcatgcccgcggcatcgccaacaccgagaaccgcaaggtctgggtgttctgcggcgacggcgagatggacgaggtcgaatcgctgggcgccatcggcctggccgcgcgcgaaggcctggacaacctgatcttcgtcatcaactgcaacctgcagcgcctcgacggcccggtgcgcggcaacggcaagatcatccaggagctcgaaggcgagttccgcggttcgggctggaacgtcctcaagctgatctggggcagcggctgggacccgctgatcgcacgcgacaaggaaggtgcgctgcgcaagatcatgatggagaccaatgacggcgactaccagtcgttcaaggccaacgatggcgcctacgtgcgcaagcacttcttcggccgcgatccgcgcacgctcgaaatggtgtccaagatgagcgacgacgacatctggcagctgcgacgcggcggccacgattcgcagaaggtctacgcggccttcgacgcggccgtgaagcacaagggccagccgaccgtgctcctgatcaagacggtcaagggcttcggcatgggcaagatcggcgagggcaagaacacggtccaccagaccaagaagctcggcgacgaggacatcaaggccttccgcgaccgcttcaacatcccgatccccgacagccagattgccgacctgccgttctacaggccggccgacgacacgccagaaatgaagtacctgcacgagcgccgcaaggccctcggcggctacctgccgcaccgccgcaccaaggccgacgagagcttcacggtgccgtcgctcgatgtcttcaagtcggtgatggagcccacggccgatggccgcgaaatctcgaccacgcaggcctacgtgcgcttcctcacgcagcttttgcgcgacaaggcgctgggcccgcgcgtcgtccccatcctggtggacgaagcgcgcaccttcggcatggaagggttgttccgccagatcggcatctacaaccccgcaggccagcagtacaccccggtcgacaaggaccaggtcatgtactacaaggaagacaaggccggccagatcctgcaggaaggcatcaacgaagccggcggcatgtcgagctggatcgcggcggccacgtcgtacagcaccaacaaccgcatcatggtgccgttctacgtgtactactcgatgttcggcttccagcgcatcggcgacctggcctgggcggccggcgacatgcaggcgcgcggcttcctgctgggcggcacctccgggcgcaccacgctgaacggcgaaggcctgcagcatgaagacggccacagccacatcctggccaacacgatcccgaactgcgtgagctacgacccgaccttcgcgcatgaagtgggcgtgatcctgcaccacggcttgaagcgcatggtcgagaagcaggacaacgtctactactacctgacgctgctcaacgagaactacccgatgcccggcctccagcccggcaccgaagagcagatcatcaagggcatgtacctgtcgaagcagggccccgcgctcaaggccaaggcgcccacggtgcaactgctgggcagcggcaccatcctgcgcgagagctttgccgcgcaagagctgctcgagaaggactggggcgtgtcggcttccgtgtggagctgcccgagcttcaacgagctgacgcgcgacggccaggacgccgaccgctggaacctgctgcacccggaccaggagccgcgcgtgcccttcgtggccgagcaactcgcgcccacgaccggcccggtggtggcatcgaccgactacatgaaggcctacgcggaacagatccgccccttcattccgaagggccgcacctacaaggtgttgggcaccgatggcttcggtcgcagcgatttccgcagcaagctgcgtgagcacttcgaagtcaaccgccactacatcgtggtggccgcgctcaaggcgctctccgaagacggtgcggtgccggtggccaaggtggtcgaggcgatcaagaagtacggcatcaatgtcgacaaggtcaacccgctttacgcctgaacatcaacaatcaacgaacgaacggcgcctcacggcgggagacaaacgatatggcagcagtggaagtcaaggtgccggacatcggcgatttcgatgaagtcgcggtgatcgaggtgctggtgaaggtgggcgacacggtcaaggccgagcagtcgctcatcaccgtggaatcggacaaggcgtcgatggagattccgtcgtcgaccgccggtgtggtgaaagaaatcaaggtcgcagtcggcggcaaggtcaaggagggttccgtggtgctcgtgctcgaggccgagggtgcgggtgcgggtgctgctgcagcaccggcccccgcgcctgcagcggccccggctgccgcagcgcccgcacaggccgcagcggcgcctgccccggctgccgcaccggccgcctcgggtccggtcgaagtcaaggtgcccgacatcggcgacttcaaggatgtcgcggtcatcgagctgctggtcaagcccggcgaccagatcgcggccgaccagtcgctgatcacggtggagtcggacaaggcctcgatggaaattccgtcgtcggctgccggcgtgctcaaggaactcaaggtcaaggtgggggatacggtcaacatcggggacctgatcgcaatactcgaaggttcggcggccgccagcccctcaccccaaccctctccccagaggggcgagggagccaattccccggccgcagccgctgctcccgtttcctctccctctcccgcctctgcgggagagggccggggtgagggtgcacccgcaccggcagcgcacgaacccaccgtggcgcccacgggcaagctgccgcatgcgtcgccctcggtgcgcaagttcgcacgcgaactcggtgtgccgctcgaagaagtcaagggttccggtcccaagggccgcatcacgcaggaagacgtccagagcttcaccaaggccgtgatgagcggccaggccagcaccaaggcctcggcggccaaggcgccggcaggcgacggcgcggcactgggcctcattccgtggcccaaggtcgacttcacgaagttcggcacggtcgagcgcaaggacctgtcgcgcatcaagaagctcagcggcgccaacctgcaccgcaactgggtgatgattccgcacgtcaccaacaacgacgaagccgacatcaccgagctcgaagccttccgcgtctccaccaacaaggagaacgagaagtcgggcgtcaaggtcacgatgctggccttcgtgatcaaggcggtggttgcggcgctgaagaagttccctgatttcaatgccagcctcgacggcgaccaactggtctacaagcagtacttccacgtcggctttgcggccgacacgcccaacgggctggtggtgccggtgctgaaggatgccgacaagaagggcatcctgcagatcagccaggaaatgggcgagctcgccaagaaggcgcgcgacggcaagctcggctccgccgacatgcagggcggctgcttctcgatcagctcgctcggcggcatcggcggcacgcatttcacgcccatcatcaacgcccccgaagtggccatcctcggcctctccaagggccagatgaagccggtgtgggacggcaagcagttcgtgccgcgcctgacgctgccgctgtcgctgtcgtacgaccaccgggtgatcgacggggccctggctgcgcgtttcaacgcgtacctaggccaggtgcttgcggactatcgccgaatcctgctatgaccaccgtagtggccgtccgcaaaggcggccaggtcacgatggcggcggattcgttggtgaccttcggcgacacgcggctttcgcacagcgccgaggccaaccagaagatcttcaccgtcgaggatgcggcggggcaaagcctgtttgccgtggccggcgccgccgcgcacttcctggtgctgcaacacgcgctggccgcgcagccgcgcgaggcgctgctgttcggcagcaagcacgagatcttccgcaccttcacgctgctgcacccggtgctgaaagattcgttcttcatgcagaccaaggaagacgagcacgagccctacgagtcgagccagttcacgatgctgatggcgaatgccagcggcatctacggcatctacagctaccgcgaggtgttcgagttcaagcagttctgggccatcggctcgggacgcagctttgcgctgggcgccatgcacacggcctatgacatcaagtcgcgcacctcgcgcgacgtggcggaggcgggaatcgccgccgcctgcgaattcgatcgcaattcggccccgccggtcgacgttctcacactcaaactgaaagtgtccaaatgagcgaacaacaaatcaaggtgcccgacatcggtgacttcgacgaagtcgcggtgatcgaggtgctggtcaatgtcggagacacggtcaaggccgagcagtcgctgatcacggtcgaatcggacaaggcctcgatggagattccgtcgtcggcggccggcgtggtgaagtcgcttgcggtcaaggtcggcgacaaggtgaaggagggctcggtggtgctgacgctggaggtcgacggtgccgcagcgcccgcgccggccgcggctgcacccgcgcccgcacccgccgcagcggcccccgcacccaaggcggcagccccggctccggccgccgcgcccgcggcgtccacctatggtggcaaggtcgacgtcgagtgcgacgtcatcgtgctcggcgccggccccggcggctactcggccgccttccgcgcggccgacctcggcctcaaggtggtgctgatcgaacgctacgccacgctcggcggcgtgtgcctgaacgtcggctgcatcccgtcgaaggcgctgctgcacgttgcctcggtgatggacgaagtgaagcatttcgccgacctcggcgtgagctttgccgcgcccacggtggaccgcgccaagctgctcggccacaagaacaaggtggtgggcaagctcaccggcggtctcacggccatggccaagatgcgcaaggtgacggtgctgcgaggcgtcggcaacttcatcgatccgtaccacctcgaggtggaggaaacctcgggcaccagctgggacacgaccggcaagaagcagaccgtcaagttccgcaacgcgatcatcgcggccggctcgcagtcggtgagcctgcccttcatgcccaaggacccgcgcgtggtcgattccaccggcgcgctcgagatgggcaccgaccccaagcgcatgctgatcctgggcggcggcatcatcggcctcgaaatgggcacggtgtattccacgctcggcgcgcgcctggacgtggtcgagatgctcgacggcctgatgcagggcgccgaccgcgacctggtgaaggtctggcagaagatgaacacgccgcgcttcgacaacatcatgctcaagaccaagacggtcggcgccgaagccacgaaggagggcatcaagatcaccttcgagggcgagcaggcgccgaaggaaccgcaggtgtacgacctggtgctgcaggccgtgggccgcagcccgaacggcaagaagatcggcgccgagaaggccggcgtggcggtgagcgaccgcggcttcattccggtcgacatccagatgcgcaccaacgtgccccacatctttgccattggtgacatcgtgggccagcccatgctggcgcacaaggcggtgcacgaggcgcacgtggcggccgaggtgatcgccggcgagcagaagggcgacaaggagctctcgagcgccgccttcaatgcccgcgtgattccgagcgtggcctacaccgaccccgaggtggcgtgggtgggcctcacggaagaccaggccaaggccgaaggcatcaagatcaagaagggccacttcccgtggaccgcttcgggccgcgccattgccaacggccgggatgagggcttcaccaagctgctgttcgatgccgagacgcatcgcatcctgggcggcggcattgtcggcacgcacgccggcgacatgatcggcgagatcgcgctggccatcgaaatgggtgccgacgagatcgacattggcaagaccatccatccgcatccgacgctgggcgaaagcatcggcatggcagccgaggtggcacacggtacctgtaccgatctgccgcctgcaaagaaggcctgatcgatcgggcggccgctcccttagccggagcggccacaaaaaatcccgccgcggcgggatttttttcgttctgcggaaactggcggctcagttgccggtgtgtgccgcggcggttgctgcagccttgacttcttcgtttggtgcgccaccgagcacgcggcgggcgccatcgaagcggcggctccagtagctgccgttcatgtcttccacgcgcacctgggcgccagtacgcggcgaatggatgaacttgccttcaccgacgtaaatgccgacatggctgaaggcacggcgcatggtattgaagaaaacgaggtcgccgggcttgagttggctgcggtcgatcttttcggtggcggccgcttgttcctcggcacggcggggcagcaaatggccgaccgtctggttgtacatggcgcgcacgaagccgctgcaatcgaaaccggattccgctgtgttgccgccgcggcggtatggcacgccgaggaagccgatggcggtcaccaccagatcggaagttcgctcggcgacggtttggcggacctgctggagttgtccgatcaggcctttgtcggcgagcaagcgggcaagttcgtcatcggttcggtcctgttgaggggcggcctggacggcgacggcaaacaggagggacgcgggtaggacgaaaaaacgcatggcgcgtaggatattgatgacgcccggttatgtcaacctcatccgaattaacgaatgtagccgcaacctgttgatttacaaactatttttcgattcggctgaagaaaaaatgtaacggtcaacctttatgaaccataagcgattgcctgcaagttaacttttgtattcatcttgaatgagctaacggcgtggatttgcatcgcaatacgcgtcaagatcggtccaattaccgggaaaagacatgaacctgcgcattcgcacgatcctccgcctgttgggaaacagtgttctcgtcgccggtttgggtttctggggcaccgcccttgcgcagatgcggccggagactgtttcttccggacttgagaatccgtggggcgtggcctttttgccgagcggccgttttctggttacagagcgtccgggccggttgcggctgatcagtgccgacggaaagatcggcgcacccatcaccggcctgcccgcgatcgccgcgggaggccagggcggcttgctcgacgtactggtcgattcaggcttcgaaaagaatcgcaccttgtatttctgcttttccgagccagcggccaacgggtcgaccaacagcacggcgctggtgcgcgcccaactgtccgaagacggcgcgaagatcgagaacctcaagatcgtcttcagccagcaacccaaggtggccagccgccaccatttcggatgccgcatcattgaggcgcgcgacggcacgctttttctcacgctgggcgatcggttcagccgcaaggaagatgcgcaaaagctcgacaaccatctggggaagatcgtgcgcattgccaaggacggcaccgcgcccaaggacaacccgttcgtcgacaaggccggcgcgctgccggaaatctggagctacggccaccgcaacgggcagggcgcggcgctcgcacccgacggccgcttgtggatgaccgagcacggcccgcaaggcggcgacgagatcaatgttccgcaagccggccgcaactacggctggccggtgatcacctatggcgaaaactacggcggcggcaagatcggcgatggcatcacggccaaggacggcatggagcagccgctgcactactgggtgccgtcgatcgcgccatcgggcatggcctttctcaccagcgaccgctatggcgcgggatggaaaggcaatctgttcgtcggttcgctgaagttcggctatctcgatcgcatcgagctgaaagacggcaaggtggttgccgaacacaaactgatggctgatggcagggcccgcatacgcgatgtgaagcaggggccggacggatggctctatgtgctgaccgacgagtcggatggcaagctgctgcggctgcgtccgaactgagcttttttcttcacccggggcagcccggcagcggaagcgttggcagcatgcggcgccagagccgcgtccattcgggccagtcgtggccgccttcggtcgtgaacacgcgctccttgggcagcgcggccgccagcaattggtggctgaaagcaaagcggtcctcggtgccgtagcccaggtagagcggcggccgagcaccgaacgttgcggtggtgcccacgtagccgcgcagccattgccagagctgtgtctcgttcggggctcgcgggtcgctgcccggcggatcgcccagcgggccggtccagcgcgtcacgccgccggcgttggcgatgtcggtgctgagcgtgcgctccccgaggtagggcgcaagggccacgaggccggcaagctcgcccggatgcgtttgcgcataaagcagtccgccgaaccccccgaccgagatgccgacgatccagatcgacttgtagcctttgccgcgggccggcaccatcacgtcctgctccaggcgatcgaggatggtcttgccgttgtagtagccaagatgcgcatcgacccgcatcacgtcgaccgcgagcctgttgtcgttcagtgccttgacgaagccctcgcgcgtgaattcgtccgggtgcgaatacgcgccggggagcatcaccagcagcgtgtcggcgttcggcgcgcagctgctcttttcgagcgtgctctccagcggcgccttggcggtgcgcaggccgccacatccggtcaccacgaacgccgcaccaagggccagaatcgacaagtggcgccgggtcgaaaagaagatctgcatcggcccggagtctagagagatgcgcgccttttcggtggtacggtcggccccatcaactccatttgaatgaaagaaccggttcatgctgctcgacgcctcgcaatcccaactcgtgctggtcgactatcaggcgcaactgatgcctgcgatcttcgaggccgatgccgtggcgcagaacgcagtgcgcctgggcaagatggcgcgcctgttcgaggtgccggtctgggggaccgagcagaacccctcgaagctcggcgaaaacgtgcccgacattcgcgcgctgtgccagcgcaccttgtccaagatgcatttcagcggcatggaggagggcctcggcgaatggctgcgcgtaccggccaaggcgccgcagggcaatgcccgcagcctgcccaagcacctgcagaaacccgccgccgcggccgaggagcgcaacacgatcgtgattgccggctgcgaagcgcacgtctgcctgctgcagacggcgctcgacctgctggaggacgagttcgaggtctgggtcgtgaccgacgcgtgcagttcgcgtaccgagcgcaaccgcgatgccgccttcgaccggctggccggtgcgggcgccgaactggtgaccaccgagatggtcggcttcgaatggctgcgtacggccgaacatccggcatttcccgagttgctgaagctcgttctctgacgtgaagccggctcgataggcgtctcgcaccccggggcaggcgcgggcggaacccgattgttcgggccgtcagcttgctgcaagatcggtctccataattatgaattcagttttggcgtggccgccggacgattcatataaggagacaacgcagatgagccgctacgaagagttctatcgccagtcggtcgatgcccccgaggctttctgggccgagcaggccaggctgatcgactggcagacgcctccggcccaggtgctggatgccagccggccgccattcgcgcgctggttcgtgggcggcaccaccaatctgtgccacaacgcggtcgaccggcacctggccgagcgggccgaccagccggcattgatcttcgtctcgacggaaaccggcaccgaaaggacctacagcttccgcgagctgcacgccgaggtgcagcgcaccgccgccagcctgatcgagctgggtgtgggcaagggcgaccgcgtgctcatctatatgccgatgattcccgaggccgcgttcgcgatgctggcctgcgcccggatcggtgccatccattgcgtggtgttcggcggttttgcaagcggctcgctggccacgcgcatcgaggatgccgagcccaaggtggtggtgagcgccgacgccggttcgcgcggcggcaaggtcatcgcatacaagccgctgctcgacgaggccatccggctttcgaagcacaagccctcggcggtgctcctgaccgaccgcggcctggcgccgatggacctgacggccgggcgcgaccacctggctgccgaactggcccggaagcaccacgatgccgaagtgccctgcacctggctggccgccaccgacatcagctacaccatctacaccagcggcaccaccggcaagcccaagggcgtgcagcgcgacgtgggcggctatgccgtggcactggccgccagcatggcgcacatcttcgacggccgcgccggcgaaacgtatttctcgaccagcgacatcggctgggtggtgggccacagctacatcgtctatggcccgctgatcgccggcatggcaaccctcatgtacgagggcctgccgacgcagggcatcgacaagcaacccgatggcggcatctggtggcgcctggtcgagaagtacaaggtgaccgtgatgttcagcgcgcccaccgcggtgcgcgtgctcaagaagcaggacccggcgctgctgaaaaagtacgacctgtccagcctgcgtgccctgttcctcgcgggcgaaccgctcgacgagcccactgcgcgctggatcagcgacgggttgggcgtgccgatcatcgacaactactggcagaccgagtcgggctggccgatgatcaccatcgccaacggcgtcgaggccaagccgagcaagttcggcagcccgggcgtcccgatgtacggctaccgcatcaagatcctgcacgaatcgaccggcgaggaattgaccgccccgaatgagaagggcgtggtcgtggtcgaggggccgaccccgcccggattcatgcagacggtgtggaaggacgacgagcgcttcgtcaacacctactggaagagcgtgcccggcaagatggtctattcgaccttcgactggggcattcgcgacgaggacggctacttctacatcctcggccgcaccgacgacgtgatcaacgtggcgggccaccgcctcggcacgcgcgagatcgaggaaagcatctcgggccacgccagcgtggccgaggtggcggtggtcggcgtggccgacgcgctcaagggccaggtggccatggccttcgtcgtgccgcggaatggccgcgccctgacagacgccgacgaggccctgaagctcgagggcgagatcatgaaagtggtggccgaccagcttggcgcactggcgcgccccgcacgggtgcgcttcgtgggcggcctgcccaagacccgcagcggcaagctgctgcggcgtgccatccaggccgtttgcgagcagcgcgatcccggcgacctgaccaccatcgacgaccccgccacgctgcagcagatcaaacagttggtttcttcggcctgaatgagcaaaagcgcgccttgcgaaggcgcgccggaacgccatatgtctgacgtggcacaatgcgaaggtactcaggcccttccccagccacagtcgcatccgccaatcggttcagccgtgtcgcggaaggtttcttaaccagctagtgcttccttcagggaagcgaaggtcagcggaatatgagcgattcttctacgccatcggcgtacaccgcctatcaaggcaacacctacctcttcggcggcaatgcgccctacgtcgaggagatgtacgaaaactaccttgccaaccccggcagcgtgcccgacaactggcgttcgtatttcgacgcgctgcagaatgtgcccgcggtcgacggcaccaacacccgcgatgtgccgcaccagccggtcatcaacgccttcgcagaacgcgccaagcaaggtacgaccaaggtcgtgcaggccagcggcgccgattccgaactcgggcgcaagcgcacctccgtccagcagctgattgccgcctaccgcaacgtcggcgcacgctgggccgatctcgaccccctcaagcgcgccgagcgcccggccatcccggaactcgagccctcgttctacggcttcaccgatgccgacctcgagacggtgttcaacaccagcaacaccttcttcggcaaagagaccatgtcgctgcgcgacctgctcaatgccttgcgtgagacgtactgcggcaccatgggcgccgagtacatgtacaccaccgaccagaaccacaagcgctggtggcagcagaagctcgaaagcgcgcgcaccaacccgcagctgacgaccgagcagaagaagcacgtgctcaaccgcctgacggccgccgaaggcctcgagcgcttcctgcataccaagtacgtcggccagaagcgcttctcgctcgaaggcggcgaaagcttcatcgtctcgatggacgagctcatcaaccaggccggcatcaagggcgtgcaggaaatcgtgatcggcatggcccaccgcggccgcctcaacgtgctggtcaactcgctcggcaagatgccggccgatctgttcgccgagttcgaccacaccgcacccgaagacctgccgagcggcgacgtcaagtaccaccagggcttcagctcggacgtgaccacgcccggcggcccggtgcacctgagcctcgcgttcaacccctcgcacctcgagatcgtgaaccccgtggtcgaaggctcggtgcgcgcccgcatggatcgccgcgccgacccgctgggcaagcaggtgctgcccgtcatcgtgcacggcgacgccgcctttgcaggccagggcgtcgtgatggaaacgctggcccttgccgaaacgcgcggctactccaccggcggcacggtgcatatcgtcatcaacaaccagatcggcttcaccaccagcgacccgcgggacagccgctcgacgctgtactgcaccgacatcgtcaagatggtcgacgcgccggtgctgcacgtgaacggcgacgaccctgaagccgtggtgcttgccacccaactcgcccttgaattccgcatggagttccagaaggacgtggtggtcgacatcatctgtttccgcaagctgggccacaacgagcaggacaccccctcgctcacccagccgctcatgtacaagaagattgccaagcaccccggcacgcgcaagctgtacgccgacaagctggccgctcagggcttgggcgagtcgctcggcgacgacatggtcaaggcgcagcgcgccgccttcgacgaaggcaggaacaccgtcgacccggtgctcaccaacttcaagagcaagtacgcggtcgactggaatccgtatctcaacaagaagtggaccgacgccggcgacaccgccatcccgtcgtccgaatggaagcgcctggccgaaaagatcaccacggtgccgaccggcttcacggtgcatccgctcgtgaagaaggtgctggacgaccgcgccgccatgggccgaggcgacgtcaatgtcgactggggcatgggcgagcacatggcctttgcctcgctggtggccagcggctatccggtgcgcctgtcgggcgaggacagcggccgtggcacgttcacgcaccgccacgccgtgctgcacgaccagaaccgcgagaagttcgacgaaggcacctacacgccgctgcagaacgtggctgaaaaccaggccccgttcgtcgtcatcgactcgatcctgtcggaagaagccgtgctcgcattcgaatacggctacgcctcgaacgaccccaacacgctcgtgatctgggaagcccagttcggcgacttcgtgaacggcgcccaagtggtgatcgaccagttcatcgcctcgggcgaagtgaagtggggccgcgtcaacggcctgaccatgatgctgccgcacggctacgagggccagggccccgagcacagctcggcacgcctggagcgcttcatgcagctgagcgccgacaccaacatgcaggtggtgcagccgaccacggccagccagatcttccacgtgctgcgccgccagatggtgcgcaacctgcgcaagccgctgatcatcatgacgccgaagtcgctgctgcgtaacaaggacgcgacctcgccgctgtccgagttcaccaaaggcagcttccagacggtcattccggacagcaagggcctcaaggcggagaaggtcaagcgcctggtcgcctgctcgggcaaggtctactacgacctggccaagaagcgcgaagaacgcggcgacgacgacgtggccatcatccgcgtcgagcagctctatccgttcccgcacaaggcgtttgccgccgagatcaagaagtaccccaatctcagcgacgtggtgtggtgccaggacgagccgcagaaccagggcgcctggttcttcgtgcagcactacatccacgaaaacatgcaggaaggccagaagctcggctactccggccgtgccgcttcggcatcgcctgcggtcggctactcccacctgcatcaggaacagcagaaggcgctcgtcgatggcgcatttggcaagctcaagggcttcgtgctgaccaagtaaaacaatctcttttcacacgaacaccctgaagaaaaaagcggagctcactccaaatgtctatcgtagaagtcaaagtcccccagctttccgaatccgtggccgaagccaccatgctcacctggaagaagaaggccggcgaagccgtcgccgtcgatgaaatcctgatcgagatcgagaccgacaaggtcgtgctggaagtgcctgcgccctcggctggcgtgctggccgaaatcgttcagcccgatggcgccaccgtggtggccgatcagctgatcgcgaagatcgacaccgaaggcaaggccgccgccgctgcccctgcggcagcacccgccgccgcaccggcaccggcaccggccgcagcagcgccggcagccgctgccgccgccaccggcggttcgaagtcggacgttgccatgcccgcagccgccaagctgctggccgacaacaacctcaagaccagcgacgtggccggcaccggcaaggacggccgcgtgaccaagggcgacgtgctcggcgcagtggcttcgggcgccaagcccgcggccaccattgcggcacccgctgccaagcccgcgctgccgcaagtcgccgcgcccgcccgcgcgcccgacctgggcgagcgtccggagcagcgcgtgccgatgagccgcctgcgcgcccgcatcgccgagcgcctgctgcaatcgcagtcgaccaacgccatcctgacgaccttcaacgaggtcaacatggcacccgtgatggaactgcgcaagcgcttccaggacagcttcaccaaggaacacggcgtgaagctcggcttcatgagcttcttcgtgaaggccgcggtgcacgcgctcaagaagtatccggtgatcaatgcctcggtggacggcaacgacatcctgtaccacggctacttcgacatcggtattgccgtcggttcgccgcgcggcctggtggtgcccatcctgcgcaacgccgaccagatgagctttgccgacatcgagaagaagatcgccgagtacggcaagaaggcccaggacggcaagctcggcatcgaagagatgaccggcggcacgttctccatctcgaacggaggcaccttcggctcgatgctctcgaccccgatcatcaacccgccccagtcggcgatcctcggcgtgcacgccaccaaggaccgcgccgtggtggagaacggccagatcgtcgtccgcccgatgaactaccttgccatgagctacgaccaccgcatcatcgacggccgcgaagccgtgctcggcctggtggccatgaaggaagcgctggaagacccgtcgcgtctgttgttcgacatctgaggcgaaagaatcagatggcaaacaaacaattcgacgtcatcgtcattgggggcggccccggcggctacatcgccgccatccgcgccgcgcaactcggcttcaacgtggcctgtatcgacgagtggaagaacggcaagggcggcccggcaccgggcggcacctgcaccaacgtcggctgcattccgtcgaaggcgctgctgcaatcgtcggagcatttcgagcaggccggccaccactttgccgaccacggcatcaaggtcgaaggcctggggctggacatcgacaagatgctggcccgcaaggaccaggtcgtgaagcagaacaacgacggcatcctgtacctgttcaagaagaacaagatcgccttcttccatggccgcggttcgttcgtgaagaccgacgcaaccggctacgagatcaaggtggcgggcgccgccgaagagtcgatcagcggcaagcacatcatcctggccacgggctccaatgcccgcgcgttgcccggcacgccgttcgacgaggaaaacatcctctcgaacgacggcgcactgcgcatcggcgcggtgccgaagaagctgggcctgatcggctcgggcgtcatcggccttgaaatgggctcggtgtggcgtcgcctgggcgccgaggtcacggtgctcgaagcgctgccgaccttcctcggcgcggtcgacgagcagatcgccaaggaagccaagaaggctttcgacaagcagaagctcaagatcgaactcggcgtcaaggtcggcgagatcaagtcgtccaagaagggcgtgagtgtcgcctggaccaatgccaagggcgaagcgcagaccctcgaggtcgacaagctgatcgtctcgatcggccgcgtgcccaacaccatcggcctgaacgccgaagccgtgggcctcaagctcgacgagcgcggtgccattgccgtggacgatgactgcaagaccagcctgcccaacgtctgggccatcggcgacgtggttcgcggcccgatgctcgcgcacaaggccgaggaagagggcgttgcggtggcggagcgcattgcgggccagcacggccacgtcaacttcaacaccgtgccgtgggtgatctacaccagccccgagatcgcatgggtcggccagaccgagcagcagctcaaggccgcgggccgcgcctacaaggccggcaccttcccgttccttgcgaacggccgcgcacgcgcgctgggcgacacgaccggcatggtcaagttcctggccgatgcggcaacggacgaaatcctcggcgtgcacatcgtgggcccgcaggccagcgagctgatctccgaagccgtggtggcgatggagttcaaggccagtgccgaagacatcgcacgcatctgccatgcacacccgtcgctgtcggaagccaccaaggaagcggcacttgccgtggacaagcgcacgctgaacttctgatcctttgaccagcgttaaagaggcctatgaggcggaactcgctgtgcgcgggttccagagcgatcccgcgcagctgcgtgccgtcgaggcgctggatcgctgcgcgcgggagtggggcgactacaaggcccagcgctccaacgcgctgaagaagttcatcaaccggcccgagctgccgcgcggcgtctacatgcatggtggcgtcgggcggggcaagagcttcctgatggacctgttcttcaacgcagtgccgctcaggcgcaagacgcgcctgcactttcacgagttcatgcgcgaggtgcaccgcgaactgcgcgaactgcagggcacggtcaatccgctcgacgagcttggattgcgtatttccaagcgctacaagctgatctgcttcgacgagttccacgtggcggacatcaccgacgcgatgattcttcatcgcttgctggtggcgctgttcgagaacggcgtgggctttgtcaccacgtccaatttcaagcccgacgacctgtatcccggcgggctgcaccgagaccgcatcctgcccgcgatcgcgctcctcaacgagaagctggaagtgctcagcgtggacaacggcaccgactaccgccgccgcacgctcgagcagttgcgcatgtatctcacgccgaacgatgcaggcgctgaaagggaaatgcgcaaggctttcgaaaagctggccgaaacggccgacgagagcccgatcctgcacatcgaggcgcgcgaaatccgcgcccggcgcaaggccggcggcgtggtctggttcgacttcaagacgctttgcggcgggccgcgctcgcaaaacgactatctggagatcgccagccagttccacaccgtgctgttgtccgacgtgccgcacatgccggtgcgcatggcctccgaagcacgccgtttcacctggctggtcgacgtcttgtacgaccggcgcgtgaagctcatcatgtcggccgaggtgccgccggaggcgttgtacaccgaggggccgcttgcgcacgagtttccgcgcacggtttccaggctcacagaaatgcaatcgagcgagtttctttcgctcgaacgccggatcgtcgacactcgactgacatgaaaaatatcgttctcgccgtgctgatgacattgggcagcctgccatcgtgggcgcagtccaccgcagccgcgggcaatgccaacttcgacgccgaacgcagcaggctggcggccgaacgcgcagccatcgacgcgcgcttcgaaaaggagcgcgccgcctgctaccagaagttcgcggtcgaagattgcctgcgcgacagccgcaggcgccgccgcgccgagaccgatcacatcaagcggcaggaaaccgccatcaacgacatcgagcgccagcggcgcggcgcggccgagctcgagaagctcgatcagaaggccgccacgcggcgcccgcaggatacgcccgagaagcaggacgagtcccgccaggcccagaaagatcgcgagcagcgcgcggccgaccatgcggcgagccgtgccgccaccgcggccgaggcggacgaacgccggcgccagctggaagaaaagcagaaagcgcacgccgacagccaggccaaggccgcgcagaagcgcaccgaagcgcctgcggccgtcgaacgcttcgagagcaagcagcaaaaggcggccgagcaccgcgccagccgcgagcgccagaacgccgagcgcaccaagccgcgcggagcacccttgcctccggcaccgccggcatcggcacccgcccgctgaagctctcgccgagccccttggcccgaggggcgccggcgcgccgttcaggcttctgccggcagcggctcgaacttcactaccgcaatggaaatgttgtcgcccgtgccgcgggcgcggcggcgcgcttctcccaccaggatttccaccgcgtcgcgcggcggctccgcgtacaggacgctggccagctcctcgggggtgaagtagtgccagagcccgtcgctgcaggccatcagcaggtcgccgggctgcatcatcggaatgtagtggggctcgacggggggcggcatcgtggtcatgccaaggcagccgagcaggatgttgcccttggggtggacattggcctcggcttcggtgatttcgccgcggtcgatgagcacctgcacataggagtggtcgcgcgtgcgcgtgacgagctggccatcgcgaaagtgatagatccgggagtcgccggcatgaatccaggcacagtcgcccttggggttcatcaggaaggccgccagcgtgctgtgcggttcctgctcgctcgacagggccgtgagcttgatgaccgtgtgcgcatcttccagcagctgctgcagcactgcggtggaactgtcgcgctcggggctgtagcgggagaacagctggcgcgccgtcatcagtacctggtcggaggccttgcgcccgccgctgcgcccgcccatgccgtcggcaatgacgcagagcatgcagccgggcacgcgtggatggctcatcatcaggacctggtcctgctgataggggcgatctcccttgtggagtccggtggcggcggcaagtcgaaagccttgggtcatgagcgcaaatgcgccagcggcgcgctttctatcttctcgggaggtcgaaccaggacgtattatcgagtgaacacgagctgcggcggaatacgtacgtcgcatcgccaccgttggactccaatctccattccctttcccgccaattgatcgagctgcgcatcgagcatgccgacctcgacgccaccatcgaccgcctggccgaggcttcgccgcaagacgaactgctgctgcggcgcttgaaaaaacgccgccttgcgctgcgcgaccagatcgcgcggctcgagaacgtgctcgatccaagagaacccgcgtgaccgaaacactcgaggacaaggtgcgcgacgccttcgcgcagggaggcgtcctgtcccgcgcggccgagcagttccgagaacgttcggggcaaaccgaaatggcgctggccgtcgcccgcaccatcgaagagggcggcgtgctggtggtcgaggccggcaccggcgtcggcaagaccttttcgtacctcgtgccggccttgctgagcggcgagcgcgtgctgttgtccacggccaccaagaccctgcaggaccaattgttcggccgcgacctgccgcgcctggtcgaggcgctcgaactgccggtgcgaacggcgctgctcaagggccgtgcgagctatctgtgcctgcacaggctcgacctggcgcgccacgatgcctcgctgcccgagcggggcagcctgcgaacgctcgccaagatcgagcaatggtccaaggccacccggaccggcgacctggccgagctgccggggctggacgaacgctcgccgctcattcccctcatcacgtccacgcgcgagaactgcctgggcgcgcaatgcccgcagttcaagccctgccacgtcaacctggcgcggcgcgaggcgctcgcggccgacgtggtggtcatcaaccaccacttgttcttcgcggatctcgcggtgcgcgaaacgggcatggcggagctgctgcccacggtgagcgtggtcgtgttcgacgaggcccatcagctgaacgaaaccggcgtgcagtttttgggtgcacagctcggcagcgggcaggcgctcgatttcgcgcgcgatctgctcggcgcgggcttgcagcatgcgcgcgggctggtcgactggcagcaactggtggcgggcgtcgagcgcgccgcgcgcgagctgcgccttgcggtcggcaagcagtggcccgggaccaagctgcgctgggtggggcctgcgcccgagggcatcgacccgcatatctggcagggggcgctcgacgccctgcagcatgcgttcgagatggcggcggaagggctcgacacggtcagcgagatctcgccggatttcgtgcgcctgcatgagcgggcgcagcagctcgccaagcgtgcggcgcgtttcgcgctgccctgcgaggtggagtccgtgcgctgggtcgacgtgggtacgcagctgcgcctggtcgaatcgccactggacatcgccgaggccatgcgcacgcgcgtgctcaagatcgatcgggacaaccggaatgcttacggcgaagaggaagacggccgtgcggcgccggaagacagcggccgcgcctgggtcttcacctccgccacgctgggcgacgaacccacgctgcgctggttcaccgagccgtgcggcctgggcgatgccgaggtgttgcgggtgcagagcccgttcgactatgcggcgcaggccgggctctacgtgccgcgcgtgtttcccaaacccaacgatgccgcgcacagcgtgcgcgtggcacaactggccgcgcgcggcgctgccgaactgggtggccgtacgctggtgctgacgaccacgctgcgtgccctgcgcgcgatcggcgacgagatgaagcagcagttcgagcggctcgaagcggacgtgcgccccgaggtgctggttcagggcgaactgcccaagcgcgtgctcatggaccgcttccgcgaaggcgcggacgcggggcgtgccggctgcgtgctggtcgcatccgcatcgttctgggaaggcttcgatgcgccgggcgatgcgctgcagctggtggtgatcgacaagctgccattccctccgcccaacgacccgctggtggaggcgcgctcgcagcgcctcgaagcccagggacgcagttcgttcagcgactattcgctgcccgaggcggccgtggcgctgaagcagggggcagggcggctgattcgccgcgaaacggactgcggggtgcttgcgatctgcgacacccgcctggttgccatgggctacggccggcggctgctggccgcgctgccgccgatgcggcggctggagagcgatgcggatttcgaggcagccatcgccgaactgaagaattcgctgtcggcctgaagaaggctggccgcggggtcgccgcacgcgcgcctgacccgatcgagacgaagaaaaagaaaaagccccgaagggctttgttctttttaccgggttaccagaccttccaccacggatcgtccttgcccttgaagccgcgcgccagatactcgctctgcgggtagttggtggtcagcacgcgctgggcgtcgtcccgcaggtccttcatgccgagcgcatcgtaggagcggacgatgatgtacagggcctcttcgagtgcgggcacttcgcggtagtcggacagggcaagctgcgctcgattgatggctgcgaggtaggcgccgcgcgagtagtagtagcgcgccacgtgcacttcgtactgggcgagcgagttcacgatgtagttcatgcgctggcgcgcgtcgggcgtgtagcgcgactcggggaagcgcgtcaccagctccttgaacgattcgaacgattccttggcggccttctggtcgcgttcggacaggtcctggcgcgtcaggaaggcgaacatgcccaggtcgtcgttgaagttgatcacgcccttgaggtagagcgcgtaatcgagcgccggactggccggatgcagcttcaggaagcgatcgatggtggcaatggcattggccttttcgcccgacttgtactgggcgtaggccttttcgagctgggcttgctgcgcgagcggcgtgcctgcggcgcggccttcgagcttctcgtacagcggcacggccttgtcgtaggcgcccgaaccggcctcgtccttggcttccgcgtagatgcggttggggctccagctcgcggtcttgtcgacgctggtggaggagcagccggctgcaagcagcgctaccgcgctgagcgcgatccaggcggggaccgataatttggcgcgaaacatcacatacggctttcgtgaaacagttgccctcaattatatcgaccgaccccctggacattgcccctgacacggccgaggtcgatgagggcgcggacccggtcgagcccagcgaactgcggcccttcgtcataggcgaggccgagcacggcctgcggctggaccgtgcgctggccgcgctggtgccggaattttctcgcaactatctgcaacagctgatcgaagccgccgccgtggagctgcaagggcgcacagtgcagaaggcttccgccaccgtgcgtgccggtcaggccgggcgcatcgagctgcgcccgacgccccagagccaggccttccggcccgaggccatggacatcgtcacggtgcacgaggacgagcacctgcgcatcgtcgacaagccggccggcctggtggtgcacccggccccggggcattggagcggcacgctgctgaacggcctgctggcgctcgatcccaaggcttcgctgctgccgcgcgcaggcatcgtgcaccggctcgaccgcgacaccagcgggctgatggtcgtggcgcggacccgggcggccatggatgccatggtggcgctgattgcggcgcgcgaggtcaagcgccagtacctcgcaatcggccacaaaccctggacaggagccgcggcccgccaggtggacgcgcccatcggccgcgatccgcgcaaccgtttgcgcatggccgtggtcgatctggagcgccacgcgggcaagacggcgcgcacgctcatcgagcggctggacagcaatgcagggggctgtgccgtgcggtgcaccctggaaaccggccgaacccaccagattcgcgtgcacatggcgtcgatcgggcatccgctggttggcgacgccctctacggaggcgcgccggccgcgggtctggagcggcaggcgctgcatgccttcaggcttgcgttcgtgcatcccgtcacgcaggcgccgatggagttccgctctcttccgcccgccgatctcgttcatgcgttgcgggcctgggggctggattacaatcgcgcctgacggcccgagggccgcgccggccaccccgatgccggccttgcgttgcactcgccgcgtgccggcagcgccttcttccatccttctgaacaagcgtccctgagacgccttttcccggataacgcgaaccatgaatacggcggatgccaagcgcattctcgaaaccgccttgatctgttcgagccagcctctgccagtgcgcgacatgcgcgtgctgttcgacgacgagctgggtgcggacaccatcaaggtgttgttgcttgaactgcaggaagactgggcgcaacgcggcctggagctggtgaacgtcgccagcggctggcgttttcagagccggcccgagatgcgcgaccacctcgatcgcctgcatcccgagaagccgccgcgctatacgcgtgctgccctcgaaacgctggccatcattgcctaccgccagccggtcacgcgcggagacatggaagacattcgcggcgtcaccatcaactccctcatcctgaagcagctcgaagaccgcggctgggtcgaggtgatcggccaccgcgaaaccgtcggccggcccgcgctctatgccaccacgcgccagtttctcgacgatctcggcctgggatccctcgaccagctgccgctgatcgagacgccggcgcagaaggcggcgctcgtcgatgcgctcgaccaagcctccggcaaccagccgggcctgccgatggaggtttccggtgactccgatgccgatgcttccgccatgacgcaagagggcctggaagcagacaccgaacttgcctcgcctgccgctgaagcccccgaagcggctgaggccgttgaagaagccgtcgaagccgtcgaagccgtcgaggctgccgccgcgcaattcgccgaggatgcggcttccaacgaagagcccgcagaaatccccgccgtcccggaagtcgagttgcccgctgaactcgaatccgaagtcccgtcgtccgacgaggccgatccccacgctgtttctcccggaaaaaaccaatgagctcctccgacatcgacgacgcggccatcgtgccggtcccgcccgaagccgagaaaaaagaggcggggacgacggaagcgtccggccagtcttcggacgctggcgcggatgccccatccacggcggccggcgagggcgaagctcccaagaaacggcgtccgcgccggaagaaggccgcggagcaggctgtcgagggcgaggccgcagcacccgcggctgccgagactcccgagactgccgaggtttccgagcctgtgacgcatgcggccccggctgctgctccggtctccgaggctccagtcgaggttgcagccaccgccgcagatgcagaacgccaggagcgccgcgtggaagaggctgcgcgcgacagcgcccatgacgacgaagatgaagaggaagaagagcccgacgaggaagaggacgacctcgaccgcgcacgccgggccgccgagcgcgagcagcgcaatgcgctgccgcctgagccgatccgtttcgcagacgtcatctccggccagttcgatgccgacgaagagagccccgaggtcccgccgctcaagcgggtgctgctgcccgaagccgactcgcccaagctgcacaaagtgctggcgcaagcgggcctgggctcgcgcctcgagatggaacagctgattcttcagggccgtatctcggtcaacaacgagccggcccacatcggccagcgcatccagtacggcgaccaggtcaagatcaacggcaagccgatccgctaccgcattgcgccgcctccgccgcgcgtcatcgcgtaccacaagcccgtcggcgaagtcgtcacgcatgacgacccgcagaaccggcccactgtgttccgcaagctgccgcgcctgcagcagggcaagtggcaatcggtcggccggctcgacctgaacaccgaaggcctgttgctgttcagcagctccggcgacctggccaaccagttgatgcacccccgcttcggcctggagcgcgaatacgcggtgcgcgtgctgggcgcgctcgatgccgaggaaaaaaagcgcttgctcgaaggcgttcggctcgacgacggcatggcccagttcggcaccatcgaagagggcggcggcgagggttccaaccactggtaccgcgtcaccatctccgaaggccgcaaccgcgaagtgcggcgcctgttcgaatcggtgggccatgcggtcagccgcctgatccgcatccgctacggtgccatggtgctgccgcgcggcctcaagcgcggcgcctggatggaactggacgagcgcgacatcaacgcgctgttccaggcgtcgggcggcggcgcaccgcgtcccccgcagcagcagcaacgcggccccggcggacaggatggcgcgggcggcggcaggaacggccgcaacaagaagcggcgcggcaaccgcaatgccggtggtggccagccgccgcgcgatgaaagccgcgacgcacccattccgaacccgctcggcgacggccggccgccgcgcggcgagcgcggagggcgcgccaaccgaggcggtggcggtggcggcaacgcaggcctgccgccgcaagggcaagggcgccgcggcaacaacaacagcaaccgcggcaaccgccagggcgatgaacgtcagccaagcggcgcgaaccagcccgatccgatgaagacctcgcttggctacatcggcgccgacagcttttcgcgccagcgcaaggaacagcgccagggaccggggcgccgtggcggcggtccgtcgggcggcggtttcggcggcggtggcggcgggccaggcggaaatcggcgccgcggacgctgaaacccagctctacagcgcagcctttcgcggggttttcaccaatcccgggggttgcgccggttaaaatcagaggctttgtcgacgcacgacgcaacaaattcgtcgcagttgtgacaaaacacttcaaaatcaaagctcaggaagcacttcaatggctatcgaacgtaccctctccatcatcaagcccgacgccgttgccaagaacgtcatcggcaagatcgtttcccgcttcgaagctgccggcctcaagatcgtcgccgccaagctggtgcatctgtcgcgcaacgaagccgagcagttctactcggtccacaaggaacgtcctttcttcaaggatctggtcgagttcatgatctccggccccgtgttcgtgcaagtgctcgaaggcgagaacgccatcgccaagaaccgcgacctgatgggcgccaccgaccccaagaaggcggcccccggcaccattcgcgccgacttcgccgacagcatcgacgccaacgccgtgcacggctcggacgctgctgaaaccgcagcgaacgaagtggccttcttcttcgccggcctcaacgtctacgcgcgctgaagccgcaccccggctgatttcatgaccacggccaacctgctcgaattcgatctcgaggggctggctgcgttctgcgaaaagctcggcgagaagcgcttccgcgccacgcagctgttccgctggatccaccagcgtggcgccaacgacttcgcccagatgaccgatctggccaagtcgctgcgcgaaaagctcgcgaccaccgctcgcgtcgaggctcttcctgtcctcacgcagcacgaatccaaggacggcacgatcaagtggctgttcgacgtcggcgacggcaatgccgtcgaagccgtattcattcccgaagacgaccgcggcacgctgtgcgtgtcgtctcaagccggctgcgcggtgggttgccgtttttgctccacggggcatcagggcttcagccgcaacctgagcacgggcgaaatcgtcgcccagctgtggtttgccgagcacttcctgcgcaagcacctgaagcgcgatgagcgcgtcatctccaacgtggtgatgatgggcatgggcgagccgctgcagaactacaccgcgctggtgcccgcgctgcgcaccatgctcgacgacaacgcctacggcctttcgcgccgccgcgtcacggtgtcgacctccggcgtggtgccgatgatcgaccgcctgggcaccgactgccccgtggccttggcagtgtcgctgcatgcgcccaacgatgcattgcgcgacgatctcgtgccgctcaaccgcaagtatccgatcgccgaattgatcgaggcctgcaagcgctacctggcgcatgcgccgcgcgacttcatcaccttcgagtactgcatgctcgacggcgtcaacgaccagcccgagcatgcgcggcagctggtggaactcgtccgcgcccatggcatctcgtgcaagttcaacctgattccattcaacccgtttccggcctcgggcctcctgcgttcgccgcagccacgcgtgctggcattcgccaggacgctgagcgaggcgggcctggtgaccaccgtgcgcaagacgcgcggcgacgacatcgatgccgcctgcggacagctggccggcgatgtcaaggaccgtacccgcgcggccgaacgcatggcccagcgccgtgtcgtttcggagcgccctgttgttttgcatccggttcgcaagaccgtcccccaggagcattgacccaatgagcatggcctttccgatggcaaccgcgagtgcacagcggctgctggccgcaagcgttgccggtgtcgccgtggcgtttctgctcgcaggctgcgtcaatacgcgcaccaccaccaccagcctggccgataccagttccggcaagggcaccgagatcgtcaccgagtccgacgagtccagccggcagcgccgcgcccggctgcgcatggaactggcgtcgggctatttcgagcacggccagaacaccgtggcgctcgacgagatcaagcaggcgctggccgccgaccccaacaacgccgatgcctacaacctgcgcggcctcgtctacatgcggctcgaggacgccggcttggccgaagacagtttccgccgcgccagtgccatcagcccgcgcgatcccaacgtgcggcacaactatggctggctgctgtgccagcagaaccgttttggcgatgccgcccagcagttcaccgccgcccttgcggtgccgagctacacggatcgagccaagacgctgatgacgcagggtgtctgccagctcagggcgggccagcgtccggaggcggagcgaagcctgatgcaggcctacgagatcgatgccggcaatccggtggtcgggctcaacctggcttcgttgctggcgcagcgcgaggaatggcagcgtgcgcagttctacatccgccgcgtcaacaacagtccttcggccaatgccgaaacgctctggcttggcgtcaagatcgaacgacggctcaacaaccgcgaagctgtggcgcagctgggagggcaactgcaacggcgcttcccgcaatcccgggaggcaatagcgtacgagcgcgggaatttcaatgactgaacgggtttcggagttcggcacttccgcggcactgccgctcgaggaaggcgacatcacgcacaagacggccggcgagatacttcgcgaggcacgcgaggcgcacgggctgcacatcgaaatggtggccgcggccctgaaggtgccgccgcaaaaactcatggcgctcgaggccgacgacatcggctcgctgcccgacccggtctttgcccgggccctggcaagcagcgtctgccgcgccttgcgcatcgatcccgctcccgtgctggcaaagctgccgggggcgcagcgcgcgccgctcgcaacggccgaccgcacgctcaagggcaacgtcgtttcaggcacgccgcgctggaacggcggccgctccagcgggcttccgtcgcgtccgctgttgatggtggtggcgctgcttctgctcggcgcggccgtgttgttctggctgccgcaatcggttttcgaccaggtcggcgccgccgtgtcgcgctggaccacgcgcagcgagggcgatgcaagctcggtggccggggcgcccacggctgcaccggcgccaggcgggccgggcgttgtcgtcgaaaacgcaccggtcacgccggtggcccctgtcacgcctgcaacgtccgcgacagctgccgcaccggcggctggcactgctccctcggcagccttgaccgtggccggcacgagcgccgccgccgcgtcggcagcgcccacatcggccaccgccgccactgcgggcggcaaccagccgcttgtcttcgtcgcgcgcgaagaatgctggatcacggtcacggaagccggcggcaagcagctgctgcgccgcagcctgaaggctggcgaaaccgtcggtttgtcgggcgcgctgccgctgtcggtggtggtgggccgggcctcggcggtcgatgtgcaagtgcgcggaaagccctacgatctgaagcctgtcacgcgcggcggcggcgtggcgcgtttcgaggtgacatcgtgaccgactgcactccgcaacccatcgaatcggcggcgcccaaggcgcgccgctcgcgccaggcccaggtggtctggggcgcgcgcaccgtcacggtcggcggcgacgcaccggtgcgggtgcagtccatgaccaacaccgacacggtcgatgccatcggcacggccatccaggtgaaggagctcgccactgcgggttccgagatggtgcgcatcaccgtcaacacgcccgaagccgcggcccaggtgccctacatccgcgagcagctcgaccgcatgggtatcgacgtgccgctgatcggcgactttcattacaacggccaccggctgctcaccgactatccggcctgcgccgaggcgctcagcaagtaccgcatcaatcccggcaacgtgggcaagggcgacaagcgcgaccgccagttcggccagatgatcgatgcggccatgcgctggaacaagcccgttcgcatcggcgtcaactggggcagcctcgaccaggaactgcttgccagcctgatggacatcaacagccagcgtgccgaaccctgggacgccaagcaggtgatgtacgaggcgctgatcacctcggccatcgaatccgccaagctggccgagtcgatgggcatggccggcaaccaggtcatcctgtcgtgcaaggtgagcggcgtgcaagacctgatctcggtctaccgcgagcttgccaaacgctgcgactacccgctgcacctcggcctcaccgaagccggcatgggcaccaagggcacggtggcatcggccacggcgctctccatcctgctgcaggagggcatcggcgacacgattcgcgtgtcgctcacgccgcagccgggcgagtcgcgcacgcaagaggtgctgatcgccaacgagattctccaggcgctgggcctgcgcgtgttcgtgccgagcgtcacggcctgcccgggctgcggccgcaccacgagcaccacgttccaggaactcgccaagcagatcgacgactacctgcgcatgcagatgccggtctggcgcaagaaatatccaggcgtcgagacgatgaaggtggccgtcatgggctgcatcgtcaacggccccggcgaaagcaagcatgccgacatcggcatcagcctgcccggcaccggtgaggcgcccgccgcaccggtcttcatcgacggcgaaaaggcccttacgctgcgcggcgacaatatcgccaacgagtttcaccagctcgtcgaaaactacatcgaaaagcgctttggcggcgagcacgctgccctggcctgaacctccgcagactcatggctgaaaaactgaatgccgtcaaaggcatgaacgacatattgccgcccgaatcggcgcgctgggagtggctcgaagccaccgtgcgcgacctgatgggccgctttgcataccgcaacgtgcgcacgccgatcctggaacacacggcgctgttcgtgcgcggcatcggcgaggtgaccgacatcgtcgagaaggagatgtactccttccaggaccgctccgacaaatacggcgacaacgaccacctgacgctgcggcccgagaacaccgccggcctcgtgcgcgcggtgatcgagcacaacatgctgtacgacggcggcaagcgcctctggtacaccggcccgatgttccggcgcgagaagccgcagcgcgggcgttttcgccagtttcaccagatcggcgccgaggcgctcggctttgccggacccgacgtcgatgccgagctgatcctgctggccaacgccctgtggaaggccatcgggctgaccgacgttcgcctggagctcaacagcctgggacagcccgccgagcgtgcgctgcaccgcgcccagctcattgcccacttcgagaagcacgccgacaagctcgacgaggacggcaagcgccgcctgcacagcaatccgctgcgcatcctcgacaccaagaatccggcgatgaaggatgtggtcgagtccgccccccggctgatcgactttctgggggcagaatcgctggctcacttcgacggcctcaaggccatcctcgatgccaacggcgtggcctacaccatcaacccacggctggtgcgcggcctcgactactacaacctgagcgtgttcgagttcgtcaccgatcgcctcggctcgcagggcacggtgtgcgccggcggccgctacgacgacctcattgcgcagatcggcggcaagccggcgccggccgtgggctgggccatcggcgtcgagcgcgtgctcgacctgatgaaagagcagggcgccgccattgaagcgccagtgcccgacgtctacgccgtggtgcccgatgcggcggccatgccggtcgtgctgcgcacgctgcagcaattgcgcgatgccggggtccgcgtgcagatgcatgcggccacggtcgacggcatgggaagcttcaagtcccagttcaagaaggccgacgccagtggcgccacctacgcactgattttcggcgccgatgaacttgcgcgcggcgaagtgactctcaagtcgctgcgcgacggcagcggcgcgcaaacctcccggccgctcgccgaagtggccacctgggccgccaccctacaatcgccggctcccaacacctgacaccatggcaacccatctcgatctcgacgaacaggaacagctcgaccagctcaagcatttctggaacacctacggcaccctgatcacctgggtggtgctgctcgtggccggtgccttcgtggcctggaacggctggcagtatttccagcgcaacaaggcggcacaggccgcggcgctctatgacgaggtcgaacgcagcacgcagtccggcgacgtggaacgcatccagcgcgtgctgggcgacatgaaggagcgctttgccggcacggcctatgcgcagcaagccggtttgctggccgccaagacgctgtacgaaaagggcaatctcgaagcctcgcgcgcggccctcggctgggtggcgcaaagcgctgtcgaccccggctaccaggcggttgccaagctgcggctcgcggccgagctgctggacaacaagtcccacgacgaagcgctcaagcagctgtcgggcaacgtgcccaaggaattcgaaccgctggtggccgaccgcaagggcgacatcctgatggcccagggcaagcgcgatgaagcccaggccgaataccgcaaggcctggaccggccttggcgcgacgtccgattaccgccgcctggtggaattcaagctcaatgcggccggtgtcgacccgaagagcctggcacccgtgatcaccgtcacgccagcagcccccaaaacttcctgatcgcaatatgaatttcaagcgtctcatgcctgaatcgaccgccctgcgtgcgggctcggccattctgctggcagcaatgctggccgcctgttccggcaccagcaagcccaagccggccgaactgcccgccaaccctgcgttgtttggcgtgcgccaggcatggagcgtgcgcattccggctgtgagcttcccgctcgccaccgacgtcagcggcgacatcgtcaccgtcgccggttccgacggcaccgtggtctccatcgacgcccgtgccggccgcgagacctggcgcgccaacgcgggcgccaagctggcggcgggcgtcggcagcgacggctcgctggctgcggttgtcaccaccaacaacgagctggtcgccatcgagggcggcaaggttttgtggaagcagcggctctcggcccaggccttcaccgcaccgctggtggccggccggcgcgtcttcgtgcagaccgccgaccgcagcatcagcgcctgggacggccagagcggccgccgcctgtggctgcagcagcgcaccgccgagaacctggtgctgaagaagtcgggtgtcctgattgcggtgggcgatacgctggtgtcgggcatcggcggccgcctggtcggcatcaaccctgccaacggcacctcccgctgggaagcgccgatttcggcaccgcgcggcaccaacgacgtggagcgcctggtcgatctgacgggcagcgtgagccgtgtcggcgacaccgtctgcgcccgggcctactacgccaatatcggctgcgtcgacaccgcgcgcggccaactgctctggagcaagcccgcggtgggcgccgagagcgtcagcggcgatgaaagctttgtctacggcaccgaaagcgatggcagcgttgtcgcctggcgccgcgccgacggcgagcgcgcctggcaatcgacccgcttcaagaaccgcgtcctgaccgggccgctggcagtggggcgttcgctggtcatcggcgaaagcactggaacgctgcacttcgtttcgcgcgaagacggcgcgctgctcaaccgcgtcacgcccgacggctctgccatcggcgtcactccggtgatggctggcaacacggttgtcgttgtgactgcgaacggcggtgtgtttggctatcgccctgaataactttttcttgcaaggcccgaccatgaaaaccgcgcccctgaaaggccggccatgaagccggtcgtggcactggtcgggcgtccgaacgtcggcaagtcgaccctgttcaaccgcctgacgcagacgcgcgacgccatcgtcgccgactttgccgggctcacgcgcgaccgccattacggcaacggccgcctgggcaagcacgaattcatcgtgatcgacaccggcggcttcgagcccgacgccggcagcggcatctacaaggaaatggccaagcagacgcgccaggccgtggccgaggccgacgtggtgatcttcgtggtcgatgcccgcgagggcctttcggcgcaagaccacgacattgccaacgagctgcgccggctcggcaagccctgcgtgctggcggccaacaaggccgaaggcatgcacgacggcaccaagctggtcgacttctacgaactcggcttcggcgacgtgcacggcgtgtccgccgcgcacgggcagggcatgcgcgacctggtcgaattggcgctcgctccgctgaacctgcccgatcccgatgacgagacggacgaagacgacgacgtcaacaagccgatcaagctggcggtggctggccggcccaatgtgggcaagtccaccctgatcaacacctggctcggcgaagaacgcctggtggccttcgacctgccgggcaccacgcgcgacgccatctcggtgccgttcgagcgcaacggccagcgcttcgagctcatcgacacggcgggcctgcgccgcaagggcaaggtgttcgaggcgatcgagaagttctccgtcgtcaagacgctgcaggccatcgagtcggccaacgtcgtgctgctgctgctcgatgccacgcagggcgtgaccgaccaggacgcgcacattgccggctacatcctcgaaagcggacgggcggtggtgattgccatcaacaagtgggacgcggtcgacagctatcagcgcgagcagatccagcgccagatcgaaacccggctgccgttcctcaagttcgcgtcgctgcacttcatctcggccatcaagcgccagggcctcggccccgtgtggcaggccattgcgcaggcccacaagtcggccacgcggaagatgtcgacgccggtgctgacccggctgctgctggaagccgtgcagttccagtcgcccaagcgcgcggggatgttccggcccaagctgcgctacgcgcaccagggcggcatgaatccgcccgtgatcatcatccacggcaattcgctggagcacgtgaccgaggcctacaagcgctttctcgaggggcgcttccgcaaggaattcgatctggtgggcacgcccttgcgcatccagttcaaaagctcgcaaaatccgtttgcggacaaggacgaataacgggcttggcggctgatggcagccaatgagctatggcttggccggaagttccgtcttttgagaaccgttatttttcaaaggcttttgaccccgattgctgcgacgcagaaaccctgtgttaaggtcatctctccaacaactactcttgaacacggagaatatcgtgagcaataaagggcaacttctacaagacccgtttctgaacaccctgcgtcgcgagcatgtgccggtctccatttatttggtgaacggtatcaagctgcagggccagatcgagtctttcgaccagtacgtcgtattgcttcgcaatacggtgacgcaaatggtctacaagcacgccatttccactatcgtgccgggtcgtgccgtcaacttctcggctgccgagaacgacgacgccgcagcctgatcgcgcggagcgcggcggcaaccccgccgcgctttttccatattgatcccgcttgtctgaactgaactctcgccaggaaggcgccgccgttctcgtcggcgtcgatttcgggctgccccatttcgacagcgaactcgaggaactcggcctgcttgcgcagaccgcgggcctggaacctgttgcgcgcctcatatgcaaacgcaaggcacccgatgcggcgctcttcgttggaagcggcaaggccgacgaaatcaaggaactggccgcgctgcaccaagccagcgaagtcatcttcgaccagtcgctgagtccggcgcagcagcgcaatctcgaacgccaactcgacgtggcggtctacgaccgcacgttcctcattctcgaaatattcgcgcagcgtgcacgttcccacgaaggcaagctgcaggtcgagcttgcccggttgcagtacctgagcacgcgcctggttcgccgctggtcccacctggagcgccagacaggcggcgccggtgtgcgcggcggcccgggtgaaaagcagatcgaactcgaccgccgcatgatcagcgaatcgatcaagcgcacgcgcgagcgcctggccaaggtgcagaagcagcgcggcacgcagcgccgccagcgcgagcgccgcgagaccttcaacatctcgctcgtcggctacaccaacgcgggcaagtcgtcgctgttcaatgcgctggtcaaggcgcgcgcctatgcggccgaccagctctttgccacgctcgacaccaccacgcgcaacctctacctgggcgatgcgcgccggcaagtctccatctcggacaccgtcggcttcattcgcgacctgccgcacggactggtcgatgcattcaaggccacgctgcaagaggccgtcgacgccgacttgctgctgcacgtggtggatgcctccaatccacatttccccgagcagatggccgaggtgcagtccgttcttcgcgacatcggcgccgatactgttccgcagcttttggtgttcaacaagctcgacgctcttgaaactgcgcagcatccgctgcatctgcaggacgatatggaaatcgatggcgtgcgggtcccgcgtatcttcctcagcgcccgcagcggcgagggcgtgcccttgctgcgcgccgagctggcccgtcggtcgggctccgtgggcgatacgatgaccccagaggccgacactgaattgcacgataccgccaattgattgggcacaatcccgccactgacaagagaacgaagcgaatgaatgcaaagccagcgtggagagggtttctgggcatgttcaatctgaacgatggccggtggggtcgcggcgatgagcccgcatccaacggcgaccgcccgaccggcaatcgcccccccgacgcagatccgccgggcgcaccggcgccaccgccttcgggcaacaacaacaacggcaaccgcccccgcggtcaaggcccgaaccaggggccaccggatctcgatgaactctggcgcgacctcaatcgcaagctcggcggctttttcggcggcaagggcggtggcaaccgacccagcggcggcaacaacggcggtggtggtggcaacggctacaggcccgacatgaagaacgcgggcttcggcctcgggctggttgcagcggtggctgttctcatctggctcggcaccggcttcttcatcgtgaacgaagggcagcaagccgtcgtgacccagttcggcaactacaaggcgaccgtgaacgccggcttcaactggcggctgccatatcccatccagcgccacgaagttgtggtgacttcgcagatccgctccacggatgtgggccgcgatgccatcgtgcgatccaccggccttcgcgaatcggccatgttgaccgaggacgagaacatcgtcgaaatcaagttcgcggtgcagtaccgcctgagcaacgcgcgagcttggctctaccagagcaagtcgcccgccgaaaccatcatccaggtggccgaaagctccgtgcgcgaagtggtcggcaagatgaagatggatgcggcactggccgaggagcgggatcagatcgccccgcgtgtgcggcaactgatgcagaccattctcgatcgctacgaaatcggcgtcgaagtcgtcggcatcaacctgcagcagggcggcgtgcgtccgcccgaacaggtgcaggccgcgttcgacgacgtgctcaaggccggccaggaacgcgaacgcgccaagaacgatgcgcaggcctacgccaacgacgtggtgccgcgtgcgacgggtacctcgtcgcgcctcaaggaagagtccgaagcctacaaggcgcgcatcgttgcgcaggcacaaggcgatgccggccgcttcagtgcagtgctggccgaataccagaaggcgccgcaggtcacgcgcgaccgcatgtacaccgatgccatgcagcagatctatgcaagtaccaccaaggtattggtcgacaccaagcaaggctccaacctgctgtacctgccgctcgacaagctcatgcagctgagcggcaacaatcccccggcgacgcccgtcgatgccgccagccccagcgtggccggtaccgcgccggctcagtcgtcggtgattccggtagcgccggccacgggcgaaacccgcgcccgcgatggccgctcgcgcgaccgtgacgtgcgctgatcaagggtaggaagaacatgaacagaatcggattcatcgcctcgtcgatccttgtcttgctggtgctgctgagctcgaccctcttcgtggtcgaccagcgccagttcggcgtggtctattcccttggccagatcaaggatgtgatcatcgagccggggctcaacttcaagctgccgcccccgttccagaacgtgtcgtacatcgacaagcgcctgctgacgctgtcgagcatcgacaccgagcccatgctgacggccgagaagcagcgcgtggtcatcgactggtatgtgcgctggcgcatcagcgatccgcgggcctacatccgcaacgtcgggctcgacgagaacgccggcgccatgcagctcaaccgcgtggtgcgcaacgccttccaggaaaacatcaacaagcgcaccgtgcgcgacctgatctcggtgcgccgcgaggcgctcatggccgacgtgcagcgcgaagtgctggctgtggtgaagggctccaagccatggggcgtggacgtggtcgacgtgcgcatcacgcgtgtcgactatgtggaggccatcaccgaatccgtctatcgccgcatggaggccgagcgcaagcgcgttgccaacgaattgcgttcgaccggctatgccgaaggcgaaaagatccgcgccgacgccgaccgccagcgcgaagtgatcgtggcgaacgcctaccgcgacgcccagaagatcaagggcgagggcgatgcccaggccgcttccgcctacagcgaagcctttggccgcgatccgcagtttgcgcagttctaccgcagcctcgaggcttacaagcagagcttcaacaagaagagcgacgtgatggtggtcgacccttcgtcggacttcttccgcgccatgcagggcgccggtacgccagcgggcagcgcggcacgccgctaaggctgcaggccgggctttcgtgagcgccgaaatattctggagcgcgcttgcgctggtcctggtgatcgaaggcatcctgcctttcgtgtcgccgggcggctggcggcgcggtttcggccagctgatgcagctgcgcgacggccagctgcgtttcttcggactttgcagcatcttgctgggtttgttcctcctttgggttttggggtaacgcggtcccggtagaatcccggtttaaccacgcccccgatccccatgtccgcctgggtcctcccggatcacattgccgatgtgctgccttccgaggcgcgccacatcgaagaacttcgacgccagctgctcgataccgcccgtggctatggctacgagctggtaatgccgccgctgctcgagcacctggagtcgttgctgtcgggcaccggcgaggcgctcgacctccaaaccttcaagctcgtggaccagctctccggccgcagcatgggcctgcgagccgacaccaccccccaggtggcgcggatcgacgcccacctgctgaaccgcgaaggcgtggcgcgcctgtgctactgcgggccggtgctgcatacccgccccgaccggccgcacgccacccgcgagccgctgcagttcggcgccgaaatctatggccacgccgggctcgaggccgacaccgaagtcctgctgctggcgctcgattgccttcatgcgtcggggatcggcgagggcctgatcgtcgacctggcagatgcgcgcatcgttcgggcgctgttcgccggcgtgccggtcgatgcctcggtgctggcgcgcgtgcatgcggcgctggttgccaaggacgcgagcgagttgcatgcgctcacgcgcgatttcccggcaccgtcgcgcgacgggctgcgcgcgctggtccagctgtacggcgatgcgtcggtcctcgacgaggcggccaaggccctcaagggcacgcccgccgtgagtgctgcgctggctggcctgaagcagcttgccaccagcctgcaggccgattccgcacggcagatcagcttcgacctggccgacctgcgcggctatgcctactacagcggcatgcgcttcggtatctacgtgccgggtgcggccgatgcgctggtgcgcggcggccgctacgacgaagtcggcgccgtgttcggccgcaaccgtccggcggtgggcttcagcctcgacgtgcgcgaactggtcggcgtgctgccggcacggccgctgcgcgcagccatccgcgcgccctggagcgacgcggccggcctgcgccaggccattgccgcattgcgcaagtccggcgagaccgtggtctgcgtgctgcctggccacggcagcgaaatcgatgaattccattgcgaccgcgagctcgtcgagcaagcagggcagtggcaagtccgagccatctgaatttttgaagtaatggaacgagcatgagcgtaaccaccggaagaaacgtggtcgtcgtcggcacccagtggggcgatgagggcaaaggcaagctggtcgactggctgaccgagagcgcccagggcgtggtccgcttccagggcggccacaacgcgggccacacgctggtcatcaacggcgtgaagaccgcgttgcacctgattcccagcggcatcatgcggccgggcgtcaagtgctacatcggcaacggcgtcgtgctgtcggccgccaagctgttcgaggaaatcgaagggctggagaaggcgggcgtcgaagtgcgctcgcgcctgcgcatcagcgaggcctgcccgctgatcctgccgttccacgccgcactcgacattgcgcgcgagacctaccgcgaaaagggtggcgtcgagaagatcggcaccaccggccgcggcatcggcccggcctacgaagacaagattgcccgccgcgcgctgcgcgtgcaggacctgaagcaccccgaccgctttgcgaccaagctgcgcgtgctgctcgatctgcacaaccacgtgctgacccaggtgctcggcgctcccgccatcgacttcgacacggtcttcgacgaggccatgcgccacgccgtgctgctcaagccgatgatggccgacgtgtcgcgcgaactgaacgacgcgcacaaggccggcgccaacctgctgttcgaaggcgcgcagggtacgctgctcgacgtggaccacggcacctacccgtacgtcacctccagcaactgcgtggccggcaacgccgccgccggttcgggcgtgggcccgggcatgctgcactacatcctcggcatcaccaaggcctactgcacgcgcgtgggcggcggcccgttcccgacggaactcgactgggccacgccgggcacgccgggctaccacatgagcaccgtgggcgccgaaaagggcgtgaccaccggccgcagccgccgttgcggctggttcgacgcggcgctgctcaagcgctcggcgcaggtcaacggcctgtcgggcctgtgcatcaccaagctcgacgtgctggacggactcgaaaagctcgagctgtgcaccggctacgagctcgacggcgaaaccaccgacatcctgccgatgggcgccgacgaaatcgagcgctgcacacccatctacgaaaccctcgaaggctggaccgaaagcacggtcggcgtcacgcagtacgacaagctgccggtcaatgcgcggctctacctgcagcgcatcgagcagatcacgggcgtgccgatccacatggtgtcgaccagccccgatcgcgaccacacgatcatgatgcgccacccttatcttgccgactgaacaggaacgaacccaaccatgttgaccgaagacggcaagcatctctacgtcagctacgacgagtaccacaacctgatcgagaagctcgcgatcaagatccaccagtcgggctggcagttcgacaccattctgtgcctggcgcgcggcggcatgcgccccggcgacgtgctgtcgcgcatcttcgacaagccgctggcgatcatgtcgaccagctcgtaccgcgccgacgccggcacggtgcagggccacctggacatcgcccgtttcatcaccacgcccaagggcgagatcgcgggcagggtgctgctggtggacgacctggcagattcgggccacacgctgcacgcggtcatggacatgctgcgcaacaactacaagcccatcagcgagctgcgcagcgcggtgctctggaccaaggcgctctcgaccttcacgcccgactactcggtcgagtacctggccaccaacccgtggatccaccagccgttcgaaggctacgacgcgctcggccccgagaagctgctggagaagtggtcggtctgacctgatccgcgtgcgccggttgcccgctcaaccggccgaatcgaacatcgcggtgtagcgccgctgcatttcttccggcgtcagcttctcgatgctgtggcccacgttccagcgatgcccgaaggggtcgcggaacacgccggaacgctcgccatagaactggtcttgcggcggcatgtccagcgtggcaccggctgcgacggcgcgggccaccaccgcatccgcatcgtccacatgcaggtgcagcgtcaccgcggtgccgccgagcgtcctggcgctgtggatgttgtactcggcaaattcgtccgaaagcatcaggatggcgccgttgtgaaaatcgagttccgcatggccgatgcgcccgctgggctcggtaagacggaagatctccttcacctcgaagaccttgcagtagaagtcgatggccgcgccggcatcgtcgacgcaaaggtacgggaacagctcgtggatcgccatgggggttgcctttccgaaaaaaagaacaagcagaggggcagggcgccattctgagcgctgcagcgccgctttcccaagcccttggccaagggatgccacagccccgctctgttcgtccggacgatggccgcgctagcatcggtgcatgagcaagccctccacgaccctgatccaccacccctacaccccacctgccaactttgcggcgccgcagcccggcatctacaaggcgtcgaccgtgttcttcgccgacgtggcggccatgcgcgcgcgcgactggaagaccaaggccggctacacctacggcctgcatggcacgccgaccaccttcacgctcgaggagcgcctggccacgctcgagggcgggaccgaatgcctcttggtgccgagcgggctcgcggccatttcgctggtgtcgttcgccttcctgaaaagcggcgacgaggtgctgattcccgacaacgcctacggccccaacaaggcgctggccaccggtgagctggccaacttcggcatcacgcaccgcatgtacgacgcaatggacccggccgacctggccgccaagctttcggaccgcacgcggctggtgtgggtggaggcggcgggctcggtgaccatggagtttcccgatctgccggcgctcgtgaacgtctgccgcgcgcgcggggtggtcaccgcgctggacaacacctggggcgcgggtctggccttcgcgcccttcgatttcaacggcagcgggcagggcgtggacatctcggtgcatgcgctcaccaagtacccgagcggtggcggcgacgtgctgatgggcagcgtcgtcacccgcgacgatcgcctgcatcgcgcgctcaagctcacccacatgcgcatgggcttcggcgtcggcgttggcgatgtggaaaccctgctgcgctcgctgcccagcatcggcctgcgctatgccgcgcacgaccggtcggcgcgcgaactggcgcgctggctcagcggccgcgaagagatcgcccaggtgctccatcccgcgctcgaggaatcgcccggccatgtcaactggcgtgcgctgtgcggcgcgtccgacctggccgccgggctcttctcgatcgtgttcgacgagcagttcagcaccgagcaggtcgaccgcttctgcgacagcctgaacctctttcgactcggctattcgtggggcggccccgtgagcctcgtggtgccttacgacatcggactgatgcgcgacgcgagcgtggcaccctggccctacaagggcacgctggtgcgcttctcggtgggcctggaggacgtggaagacctgcgggccgacctgcaacaggcgctggcgcggctgtaaggctcgcgcgcgccatggggagaaagcgccgccggcttcgtgccgctgcgttgcctgccgcgcgcggggcggtattgccgccagcgccaggccggttcgttccccgcgtgctggccgttcctgtgcccgtgcttgaggcgctcgcgcaagctgggccgctggaaggcgtgccggacctgagggcgacccggctcctcgtcggcgggttgatcgctgtttttgcgctggtcgcgctgtcgctcggcgcggcggtgatgctggagggcgaggggtccaacattcggggcaacgaagcggtcgtcgtgctcgtcggattggcgctggcagccggattgggcggcggtctctggcacctggtgcgccagttttcgcgggtcggccaggggatgttccgcatcgactcgacgggcctgcactggggcgacccggcctcgccgcggggcgtcgcctggcgcgagctgcggcgcgcgcccgccggcttctgcgacgtgaaaaccgagttcgcctcgggcgaggccatcgtcaaacgcctggtcttccagcagcaggttgcaggtggctccggcatcaccgaagtcaagctgcccctggcgctgaccgtggacgccgggcgcgtcctgcgctttcgcaaccgcgccgtgctgctgcgcgcgcttctgctctgcctcgcgacccggccagagccgcgcctgcgctttgcggccgaggtgttcatcgacgccggcatcgatccggcaacctgggaaccgatgctggctcccaggcgctggatgtggctgtcttccgttggcgcgctgctgccggtgctgcccgtgatttttctctggccgccgggtgtgcacgccggctggatggtggccgcaatggtcctcgccatggtggctggcgcgggggccatgggctggttcatgttccagcgctatccgggtttgcaaggtgtgttcgagttcgaaacgacccccggtccgccgccttgagaccgcaccgttatcgcttacagtagcctacgcacagtcaccgggactgtctcgcctcaaggagaagcagtggcaacaccaaattacggctacgagaagcgccagaaagagctggccaagaagaagaagaaggaagaaaagctccgcgagaaggccaatcggaagctctctcccagcagcgatggccttgcgccgggcgacccggagaccgacgtcgcttcgctggaacgcgatccgcccaccatccctgatctgcccaccaagaacggttgatttttcgaaaccgggctctcgactaaaaagccgctgccagccttcgggcctgcagcggctttttttgctttcggggccggcctatttggccgccagcagcttgcgcagttccggccagacgttgtcgagcagttgcggctgggccgcggcggtgggatggatgcggtcggcctggaacagcgcgagcgcatcgggcgcatcggccacgcccttgagcaggaacggaaccagcgcagccttggtcgcacccgccaccttgccgaacacggcctcgaagcgccgcgtgtagtcgccgccgtagttgggcggcacctggatgccgacgatcagcaccttggcgcccgcggcctgcgcggccttggtgatctgcagcaggttttcctcggtgttctggagcggcaggcctcgcagcgcgtcgttggcgccaagctcgaccaccacgtggctgggcttgtgctgcgccagcagcgaggcaaagcgggcccgcccgcccgaggtggtgtcgccgctgatgctggcattgaccaccgtggccgggatcttttgcgccgcaaggcgcttttcgagcaaaggcacccagccttcgccgcgcttcaggccgtattcggcgctcagcgagtcgccaagcaccagaatcaccggctggcggggtgccgcagcctgtgcggcctgggcgtgcgccactgccgatgtccctgcgctgccgaatgcggcggcggtcaagataaagtcacgtcgattcaaaacgaaaagccttttcatgtcccaaccctcgtctgatgccattgtcgctgtcgagcacgtgttcaaatccgtgaccgattcgaccggtacgctcgacattctgcagaacatcgatttcaccctgggcgcgcgggaaaccgccgccattgtcggcgcctcgggctcgggcaagagcaccttgctgtcgatcatcgcgggtctcgacacgcccacccgcggcacggtcaggctggcgggggacgacatcttcgccatcgacgaggacgagcgcgccgcgctgcgtgcccagcgcgtgggtttcgtgttccagagcttccagctgctgggcaacctgagcgcgctcgaaaacgtgatgctgccgctggagctagccgaccgcaaggacgcccgcaaggccgccaccgagatgctcgggcgcgtcgggctcggacagcgcctgggccactaccccaaggtgctttcgggcggcgaacagcagcgcgtggcgctggcccgcgccttcgtggtgcagccggcgctgctgctggccgacgagcccaccggcagcctcgactttgcgaccggcgagcaggtcatgcggctgatgttcgacctcaaccgcgagctcggcaccacgctcgtgctcgtcacccacgaccgcggcatcgcggcccagtgcgagcgccggatcaccatcgaggccgggcaaatggcgctcaatgagtcgaagcccgtgctggtggcttcgctcgaagcatgatcgtcccccggttctgggccgaaggccgcatccaggagcaggtggcgggcaagcagatcaccgtgcggcgctacggctggtcggacgacagcccgatcgccgcgcaggcgcatgccgaccagcgcacgcgagaggcgttcgagcgcatcgccagcggcgagaagctcaaccgccgcgagcgcaagcaggcctacaacggggccgaaggcgtgccgatccgcgaggagatcgtcgagcggcagggcgacaccgtcatcacgcgcaacagctatggcgcacgctgtctcaacacgcccgacgtgctgttcgtcgacatcgatttcgacgaacccctgcgcggcagcgtgttcggctttgcgctggcgcccgcgctgattgcgggcatcgtcggcggctggaccgccaagacctggctgggcgggctcatcgccgccgtcgtggtcttcatcgtcgcctaccgcatcggcctggccaagaagcgcggcgaggccagcgacaaccccgcgcccgagaagcgcgcggccgaccgcatcgggcgcttcgtccaccagcaccccgactggcacctgcgcctgtatcgcacgccagccggcttccgggtgctggcgatgcacgacgtcttcagcccggccgacatggcggtggccgactgctttcatgcgctgggcgtggacaagacctatgcgcgcatgtgccgcaaccagaactgctttcgcgcccgcctgagcgccaagccctggcgcatcggcatcggcgagcacatccggcctcggcccggtgtctggcccgtgtcgcccgagaagctccctgtgcgcgatgcctgggttgcgcactacgaaaaagccgccgagggccatgccgcctgccagtacctggaaagcgccggcaacagcgcgcgcgtgcatccgaacgcactggccgtgcaggaactgcacgacgaacggacccgggcgcacagcggattgccgattgcatgaaggagagggtgcgcagccctcgataatcgacagatgtcttctcccaaagtgatcttcggctttcatgccgtgggcgtgcgcatcaagaccgcgccgaactcggtgctcgaagtgatgttcgacaccagccggcgcgatgcgcgcatgaaacagttcatcgcacgcgcgcaggaagccggcgtgcggctggtcgaggccgacggcctccggcttgcaaagctcagcggcagccacggccaccagggcgtggtggcgcgggtcgaacccatcgcgcaggtccgctcgctcgacgaattgctcgaaggcctcgaggaggctggcaccgtgccccttctgctggtgctcgacggcgtgaccgatccgcacaacctcggcgcctgcctgcgcgtggccgatggtgcgggcgcgcatgcggtcattgcccccaaggatcatgcggccggcatcaacgccacggtggccaaggtggcgagcggcgccgccgagaccgtgccgtacttcatggtgaccaacctggcgcgcacgctgaacgagctcaaggagcgcagcatctggtgcgtcggcacgagcgacgatgcgcccggcaccctctaccagagcgacttcaagcggcccctggcgctggtgctcggcgccgaaggcgagggcatgcggcagctcacccgcaagacctgcgacgagctcgtgagcattccgatggcaggagccgtcgagagcctgaacgtttccgtggccagcggggtgtgcctctacgaggccatgcggcagcgcggcgcctgatgccgcaccgctagcccttggacaaggggctggccttgcggtggaagtacacgagttccgccatgcgccgcatctgcggcgtacccagcaggcggttgaacatccaatcgctctggaaatgatcgaaagcccagcgcaacgcgcgcttgagccggaagcgcggatagctgcgcacgaaccagcttgccgggtcctccacctcgccacggacgaaccgcgcaatcgcctcgccggcgcgctcgccgtgctggagcgccgtatgaatgccgccggccgtgaccggcgacaccatgccggccgcatcgcccaccagcagcgcgcgttcgcgtgccaccacgggcagcacgccgccgcacggaatcattcccgcgcgaatcgccacgggcggcgcatcgccgggcgagacgaccgaggcgatcttgcgcagcagcgggtcgatccgaagcgccgacgccgcctgcgtatccatccggcgcgcaaggccgatctggctcacgccgacgccgtcgagcgcccatccgatgtagcccggcgccagctggcggtcgacgaagcaatgcagaaagtcgggtgccaagcgtgcaccctggtattcatgctcgacaccgtagaggaagcgcgtgttgcgcgacagcccaagggccttggcaacgcgcgaatgcgggccgtctgcgcccacgatgtagcgggccgaaatgcaggtgccgcggcaagggccgtgggtcagcggaatctcccagcggtcattcatccacagtgcctgttcgaacagcgtgccaagctgcacgtcaaccccgctggcacgggctgaatcgaccatccagtcgagcagggcgggcgcgtcggtggcccagaaccaatagcccggcgcgtgcaggtccacgtggcgcatgtcgggcgaatagagccgcacgccgtcgatgcggcgcaccagggcgggcggcacttccgcgagccagggcaccgtgtcgaccgcgtccttgacgatgatcccggtggtatggagcttggcgccggcgctggactttttctccagcaccatcacgcggagccctgccaatgccgcggcgcgggcgcaggccagccctgcgaagctcgctccgaccacgagaaggtcgaccacggtgttcgaactgcgattcccggacgatggcggggcagggcaggcggcgaaaaagggaggggtgtcgaagcgagaaaaggaacttgaagcggacataggcgagctgacttgggcgttgtgcaccgcgacttgcggtgcgcacgcgaaagttagctacgccatgtgcgggcggcgtgaagcctgtgtgaactcgaagcgcggcaatttcaggaagggtccttggtgcgtgtgcgcgacactgcactgaagatcccgatgcccagaatgatcagcgcgccaatgccgatgtagagcgtgggcacgccggccaccgaggcgccccaggcgacgccggccaggaaaatcagaaaaccgatcatgtagagcacaaaggacatgcttgttcccccggaagctttggatgccttgcagtatcccgggcgatgcggtggccagcagaggccttcgtctccagtcgctgtgggaacttgcctactgcccgtgggccttcatgccggggaagcgaccagcaggtagcggcacccggtgcggccgagcgccttgaagaccagcggccgatcgacgccgaaatcaaggcaatcgccagtcgccagctcgaaccgctcgtcgccgtagtccacccgcagcgcgccttcgagcagccacaggcattgccgatacggcttgccgctccaccgcggatagccgacctgcgccgagcgcggcagctcgatctcgaccatctcgacgccgccggtggcaccgcgctccgcgacctggcgccgcaggtagccggcctcgggatcgcgccacacttctcctatattggacgatcttcacaacgtagtccgtcgcttgtcgaaaggaacacccatgcacctggtcccatgcaccgaggaagcccacgcgggcgccatcctcgccatcctcaatgaagccatcgccaactcgaccgcgctgtacgactacaaaccccgcacgcccgagagcatggccgcgtggttcgccaccaagcgcgccaacggatttcccgtgatcggcgcggaagacgacgacggcaagctgctgggctttgcgagctacggcacgttccgcgcctttcccgcctacaagtacacggtcgagcattcggtgtatgtcgaggccggccaccgcggcgcgggcctgggccgcacgctcatggaggcgatcgttgccgaggccgttgcgcgcgacgtgcacgtcatggtcggcgccatcgatgccgcgaatgccggcagcatcgggcttcacgagcggctgggcttcgaacatgccggcaccgtgcggcaggccggattcaagttcggacgctggctcgacgtggccttctaccagcgcattctctcgacgccgctgaatccggtcgacggttaggcgacgggttcaggccgggtcttcggcgctggcccggtccagcatctggatggtgccggcatcgagcttcagctgggtggccaccaccagctcctccaactgcgcgatggaggtggcgctggcgattggcgccgtgatcgagggccgcgcgatctgccatgcaatggccacctggcccggcttggcgttgtactgctgcgccaccttgtcgagcgcttcgaggatgcgcaggccccgtgggttcaggtacttcttggtggtgttggcgccgcgtgcgctcttggaggcgtcggcttcggtgcggtacttgccggtgaggaagcctgcggccagtgcatagaaattgatcacgcccacttcgcgcttcacgcacagcggctccagcgcatcttcgaacaccgcgcggtcatacaggttgtagagcggctgcaggctttcgtagcgcgcaatgccgagccgttccgacacgtcgagcgcctcggccagccggggcgcgctgtagttcgaggcgccgatggcgcgcaccttgccggccttgacgaggtcgtcgaaggcgcccagcgagtcttcgagcggcgtggcggcatcgtcgtcgtgcgactggtacaggtcgatgaagtcggtctgcaggcgcttgagcgaagcttccaccgcttcgcggatgtaggccggcgagaggcccgacttgccttcgcccatcggcttgcccaccttggtggccagcactacgcggttgcgcttgccgctctgcttgagccacttgccgatgatggtctcggactcgccgccggtgtggccgggcacccagctcgaatagacgtcggccgtgtcgacgaagttgaatccggcatcgagccaggcgtcgagcaggcggaacgaggtggcttcgtccaccgtccagccgaacacgttgccgccgaaggcgagcggagaaaccaggaggccggagcggccgagcgagcggagttgcgacatgagtttgtttccttcctgaaagagacgaggatcagacgaagcccacggcgccgagcagcgcacccgcgcccagcagccagagcaggtggacacgggtgcgccagacgataagcgcggccaccgcgctcagcagccacagatgccatgcgggcgcgtcgccggcatggttacccgccgccagcacccagccggtggcgatgagcaggccgaccaccaccggcgccatgccctgcttgaaggcgcgcacgccgcgccgctcgcggttgcggtgtccccagcgcgtggcaaggtaggtgagggtggtgctcggcagcatgatgccgaccatggtgaccaggagtccgaagaggccgagcagccatgcgcgcggcccggcgccgatgccgccgccggcgttgagcccgacgttccagcccatcagcgcgacgaagagcacgttcgggcccggcgcggcctgagcgatggcaaccgacgaactgaactgcgcgtcggtgagccagccatgctgcgcgaccaggtagcggtgcatgtcgggaacggtggtgatggcgccgctgatcgacagcagcgacagcagcgtgtattggccgaagagcgcaagccagtcgtgccactgcatggcgatcgtgatgtggctcatacgcctatcttccgccaggtccacgcgcaggccacgccgcccacggccagcagcacccagccgagcggcatcttgaagagggcaatggcgcagaacaccagcgcgacgaacgcgaggcaggtggcaaagcccagcggatgcctgcgcagttgcggaatcagcttgatgccggtggcggcgatcagcccgcccgacacggcgcccatgccgcgcagcgccgccgccacctgcggattggcggcgtagtgggcgtagagcacggccagcaccaggatgacgaccagcgggatcgcgagcatgccggccaccgcggcaatggcgccgcgcaggccgaagtagcggtcgccgatcatcaaggccaggttgatcacgttcgggcccggcatcacctgggctacggcccagtcttcgagaaactgctcgggcgtgagccagcgctttttctcgaccatctcgcgctggacgatggccagcacgccaccgaatccttgcagcgcaagccaggtgaatgaaataaaaaggtcgcgtggcgacgtcggttgcaaagggacggtcggcgctgccgcgcctggaggggacggatgcatgtgggagcgattatcgtagccatgcctgcaacgtgccgggcatcgggctgacatgcccctgcatcactcgacggaaaactccatggccatgcaaattcgcgcgctcttcgatctctgcaaggaggccgtcgcttcgtggtcgaacgactacgcccccagcatgggcgccgcgctggcctactacacggtgttctcgattgcgccgctgctgctgatcgtgatcgccgtggccgggctggtgttcgggcaggaggcggcgcgaggcgagatcttcctgcagctttcgggcctcatgggcgagcagggcgcggccgcggtgcagggcatgctgcaggcggtcaacaagccggccgagggcatcgtggccacggtggtcggcatcggcctgctggtggtcggcgcaaccacggtcttcggcgagttgcaggatgcgctcgaccgcatctggcgcgcgccggcgcgtaccaggaacaagggcctgttcacgctgctgcgcgtgcggctgctgtcgttcggcatgatcatgggcatcggcttcctgctcatggtgtcgctggtggccagcgcggcactggcggcgctcggcaaatggtggtcgccggtattcggcgcctgggccaccctggcgcaggcggtgaacttcgtcttcagctttgccatggtgacggtgatcttcgcgatgatctacaagatcatgccgcgtgccaaggtgcagtggcgcgacgtgtgggtgggcgccgcggtcacggcgctgctcttcacggtcggcaagcacctcatcggcctctacatcggcaagagcagcgtggcctcgggctacggggccgcgggctcgctggtggtggtgctggtgtgggtgtactactcggcgcagatatttctcttgggcgccgagttcacctgggtgtatgccaagacctacggctcgctcaagcatgccaaggacacgggcgaagccgccaacccctcgccgacgcgcgaggctgcgctgccccggaagggctagcccgcgaagccgccttcgtccaggaagcgctgttcctccgcgctgctggtgcgcccgagcagcttgttgcgatgcggaaaacggccgaagcgcgcaatgatgtcgcggtgcaataccgcgaagcgctgggtgttggcatcgagtgccgcgttcagctcgacggaacgctcctggtccgccagcgattcggaatgcatgaagggcaggtagaagaagcgccggagctcttcgtcgatccggaggtcgaggccggcctcgatcgcttcacgggcaaccgccagggccatcgggtcggtcgcgaatgcgcgcgcctggccgcgaaaggtgttgcgcggaaactggtcgagcagcaccagcagggccagcgcgccttcgggctccttcgcccagcggctgagctcgcctcgggctgccgcctcgtgcgcggcgagaaaacgcgtgccgaactcggcatcgaaagcatcgttcttggcaaaccagcgttcgggtccggcgtcgcgccagaaaccggcgacgtcgcgggcggtgggaaggtcgggagaagtcatcgccgcattctctttcagcccgcaaagtcgcggtggtggccgacaacgccctgcgcccagtctccctatgctggagcggttttcataactcaggagataaagctcatgaaccgatatggcacctttttgcgcgcaaccctcattgcgggcctggccaccgccgcgctcgccggttgcgggatgatgtccaagtcgaacaccgcgagcttcagcggcgcaatgaacgccgccagcgaagtgccgcccaacatgacgcgcggcagcggcatggcggaggcctggctcaacaaggacaccaacgtcctgaagtacaagatcacctacaccggcctgagcggccccgccacgggagcgcattttcacggtcccgccgccgcaggcgccaacgccggcgtggtgctgccgttcgccaatccggccagcccgatcgaaggccaggccacgctcacgccggcgcaggcggccgacctgatgtccggcaagtggtacgccaacatccacaccgccgccaaccccgcgggtgaaatccggggacagatgctgcccaagatgtaggcgccctggtcagcttgcggccgcggggctggtgtcaaatgacaccctatgacgacgaagccccagaagccccgcaccgcaagcaagaagacctccaacaatttcgaagcgcgccgcgacgacatgcgcgtcgcgcgcaaggccctggtgctgcagggaggaggcgctcttggcgcctaccaggccggcgtgtatgccgcgctcagcgaaaccgaactgcagccgcactggattgccggcgtctcgatcggcgcgatcaacgcggcgctgatcgcgggcaatgcgcccgagcagcgggtcgatcggctgcgcgagttctggcacctggtgtcctccgggccggcgcagcgcctgcctggctggctgggcgatcgcgccacgcagaaccagtggagcgccgtcatggcttcgctggtgggcattcccggcttcttcgagccgcgctactcgcctgcgctgctgctgggcgccgcggcgccgctcttgagctactacgacaccacgccgctcaagctcacgctcgagcggctgatcgacttcgaccgcatcaacgcgtgcgaggcacgcttcagcgtcggcgcggtcgacgtgcgcaccggcaactcggtgtacttcgacaacaccaggcagcgcatcgggccggagcacatcatggccagcggcgcgctgccgccgggctttgcgcccgttcacatcgacggcgacgattattgggacggcggcatcgtctcgaacacgccgctgcaatacgtgctcgacatccatccgcgctccgaaccgctggtggtgctgcaggtcgacctcttcaatgcgcgtggcgagatgccgggcacgctggcgggcgtgatggagcggcagaaagacatcacctactcgagccgcacccgcatgaacaccgatgcgctggccgccaacctgaaccttcagcaggcgatcgcggacctgatctccaagctgcccgcgcacctgcgcaacgatccctcggtgctcgcggtgcaggccgagctcacgcaccatcccatcgacatcttccacctgatctaccgcgacaagccctacgagctcgaatcgaaggactacgagttctcgcgcgccgcggtcgaagagcactgggaggccggcgcgcgcgacatgcgccggacgctggcgcatcccgaaaccctgcgcagcgatgccaccgtgaacggcgtgaccactttcgaccttggcgagccggggctggggcgcgtcaagcgtcccgggctgttgcgctgagtacaggctgcaacggcagccttgctcgcccggttcttgcaatcccgttttcttttgttctcccgtctttcccatccccaaggacattcaccatgcaactcaaggacaagatcgcgttcatcaccggttcggccagcggcatcggcaaggaaattgccattctgtttgcgcgcgagggtgccaaggtcgtcatcgccgacctcaacaagcaagccgccgatgccactgcggccgagttgcaggccacgggtgcgcaggcgatgggggtggccgtggacgtgaccagcgaagaccaggtcaacgcctcggtcgaagaggctgccaaggccttcggcggcatcgacatcctgatcagcaatgccggcgtgcagatcgttcatccggtcgaggagttcagctttgccgactggaagaagatgctggccattcacctggatggcgcctttctcaccaccaaggcctgtctcaagcacatgtatgcccagggtcgcggcggcagcgtgatctacatgggatcggtgcattcgaaagaggcttcgctgctgaaggcgccttacgtcaccgccaagcatggcctcatcggcctggccaagacggttgccaaggaaggcgcgaagcatggcgtgcgcgccaacgtgatctgcccgggcttcgtgcgcacgccgctggtcgagaagcagattccggagcaggcaaagacactcggcatcaccgaggagcaggtcatcaagaacgtgatgctcaaggagacggtcgatggcgaattcaccaccaccgacgacgtggcgcgcgtggcgctgctgttcgcggcctttccgaccaatgccctgaccggccaatcgctggtcgtgagccacggctggttcatgcagtagcgaaaagacgccgccgtgcgcggcgcacgatggttcaccctaatgtctctggcgagcgaactgtgagaaaaacctttcttgccgttcaatcgtcataccaatgactttcgccaggagacaaagaccatgcgtgtttcttcagcccgcttcttttcgcgacgctctttcgtggcccatgccgcaggtgtcgcggcagggctcgccatgtttgcggcggcggctcccgcggcagcccaggcgtatccgagccggcctgtcacgctgatcgttccctggggtgcgggcggtggcaccgatgccacggcgcgcatcatcggcagcctgctcgaaaaagagctcggccagccggtcacggtggtgaaccgcaccggcggcaacggcgtggtgggccacgcggccattgccgccgcaccgccggatggctacaccctcggcatggccacggtcgagatcggcatgatgcattggcagggcctgacaccgctgaccggcgcgtcgtacaccccgatcggccttaccaacctcgatccggcggccctccaggttcgcgccgatgcgccatacaagaccgccgccgagctgctggcggccgtcaaggccagcccgggcaagttgaaggcgtccggcacggggcagggcggcatctggcacctggcgctcgcgggcctgctgcgcgaccagaagatcgaccccgcggcagtgccgtgggtgcccagcaacggcgcggcaccgggtctgcaggacgtggtggcgggcggtgtcgacattgcgcccgtctcgctgcccgaggcgcgctcgctgatcgatgcgggcaagatcaagagccttgcgatcatgagcgacaagccttcggctctctatcccaatgtgcccacgctcaaggcggccatcggcagcgactggtctttggcggcctggcgcggcatcgtggcgcccaagggcctgcccgccgacgtacgcgacaagctcgcggccgcaatcaagaaggtggtggcaagcaaggactacaccgacttcatggcgtcgcgcggcttcggcgtgatctacgcgggtcccgacgaatttgcggcgtacatggcgaagtccgatgccgaactcggcgcaaccatgaaggccgtgggtatcgtcaagtgagggccgcgcggggcctgcgcgtcggggcgggaggcacggcgcgatgaagttcaacgacgcagtcttcggactggttctgctggcgctcggcggcctcgtgctggccgtggtgcgaggctatcccggcatgcccggccaacaggtgggaccggcgctgttcccggggctgatcgccgtggggttgtgcatcggcggcgccatgctgctggtcaagggctggcgcgagcggcagacggtggcctgggtccggctcggcgactgggcggcatcgccgcgccacgtgctggcggccgcgctggtcatcggcgcggtgctgttctacgtgttcgcatccgagtggctcgggttcctgcccaccgccgccatctcgctggtggcgctgatgctctccatgcgcgtgccgccgggccgcgcggtgctcatcgcgttgattgccacgctggtcatccatgccgcgttctacaagctgttgcgcgtgccgcttccctggggcctcctgacacccatcgcctggtaaccggaaacaccactcatgtcggcagcactcttgcaggctttctcgatggtcttcgagccctacaccatcctcgtgatggtgctggcctcgttctatggcctgttcgtcggcgcggtcccggggctgtcggccaccatggcggtggcgctgctggtgccggtcaccttcttcatgccgccgattcccgccatcgcggccatggtcacggccaccgcgatggccattttctcgggcgacattccaggctgcctgctgcgcattccgggcacgcccgcatccgccgcctataccgacgaagccttcgcaatgacgcgcaagggcatggccgaaactgccctgggcgcggggctggtgttctcggcggtcggcgggcttttcggcaccgtggtgctgatcgtggcggcgccggtgctggccgactttgcgctcaacttcagttccttcgagtacttctggctcgtgctgctgggcctgacctgcgcggtgttcatcacctccgaccggccgctcaagggcctcgtcacgctgctgctcggcctgctcgtggcctgcgtggggcttggcaacccggcgggctttccgcgcttcaccttcggaaatgccgagatgaccggcggcatcggcatgatcccgatgatgatcggcatgttcgccatctcggaggtgatccgcttcgccgtcgacacgctgccgccgggcgagatcgtggtcgagaaagtgggccgcgtgctggcgggccaatggacgctggcaaagaaatacccggtgcagatcttgcgcggcagcgtgctgggcacggccgtgggggcgctgccgggggcaggcgccgacatcgcggcgtggatgtcgtacgccatgagcaagaaattctcgaaggagcccgagaagttcggcacgggccatgtcgagggcatcgtcgaatcgggctcggccaacaacagcgcgctggccggtgcgtggataccggcgctggtgttcggcattccgggcgattcgatcaccgccatcgtgatcggcgtgctctacatgaagaacctcaacccggggccgacgctgttcaccacgaacccgcagaacatctatgcggtgttcatgctgttcatcatcgccaacatcatcatgattccgcttggcatcctgtgcatcaaggtgtccaagcgcatcctccgggtgccgcgcaacgtgctgatgccgttgatcctgctgttctgcgtggtgggtgcattcgccatcaacaactcgctgttcgacgtgggcgtgatgctggtggccggcatcgtggcctacctgctcgaggagaacgattttccgattgcgccggccatccttggcgtagtgctcggcggcatgctggaggaaaacttcatcacctcgatgatcaagtcggacggcaacctggccggcttcgtgtcgcggccgatcgccgccggcctggctgtcgtggtgctgctggtgtgggttgcgcccctcgtcaagaagctgtggcggaggggccggcgccccgcgtctaccgcagcttgagtgaccaggtttcgcccaccaactgctggccgaagccttcgtagggctcggccttgtcgagcttgaagccgcgcttggcgtagatggcgcgggcggcctccaggcagctgttggtccagagcgccatctttcgatagcccttggcgcgtgcgaaggcaatgcactcgtcggtcaggcgtgcgcccaatccgaggccgcgcgcggcgggcgagagcagcagcaggcgcaactgggccgtggtggccgacttgcgcaccacgaagatcgcacccacgcgttctccgtcgagctcggcgatccagcatttctcccacgcgggctgaaacttgcgcacgaactgggccacgatgtctgccaccagcgcttcgaactcgctgttccagccgtactcgcgcgcatacagctcgccgtgctgctgcaccacccagcccatgtcgcccggcagcggatcgcgcagcaccaccgtgcgggtgcgtgccgcgcgagcggtggccgggtcgagcagccgttcgatgcgcgccatggcatcgaccacctgctggcggtcgtgcggcggcagcggggagagcagggcggccgcttcgtcacgcgacttttgttgcaacggcgcaaacgcggcgtggccggcttcggtgagccgcagcacgctctggcgcgcgtcgcgggcgtggggctcccgcgtgagccagcccgcggcctcgaagcggcgcaggatgcggctcatgtagccggcgtcgagccgcaggtcgcggccgatctcgctggccaccggcgttttccggtgggccagctcgtacagcacgcgaacatcggtcagcgacatctcgctgccgagataggggtcgagcacgccgatgcggctcgtataaaagcggttgaattggcggatggccttgacggctgcggcgtcgggagtgggcgcagcgctggaaatagtagcttctgtcatatttatgattgactaaggcaaccatttaaaggccttgccgtcggcacgtcaacaagcgccgacgcgacaagactgatggaaaaccctaaaatcgcgggttgcccactgcagcgccgtgcccgccaagccgcgccgccaaactcccactgatgaacgcccccgtcgacgtctccttttttgcgcgtgccgccaagccgctgaccagctaccgcaagtactgggcggcccgtttcggcacggccagattcctgccgaccacgcgcaaggaaatggacgcgctcggctgggacagctgcgacatcatcgtggtgaccggcgacgcgtacgtcgaccatccgagcttcggcatggccgtgatcggccgcatgctcgaggcgcaaggctttcgcgtgggcatcatcgcccagcccgactggcagagcgccgagcctttcaaggcgctgggcaagccgaacctgttcttcggcgtgaccgccggcaacatggattcgatgatcaaccgctacacggcggaccgtaagatccgcagcgacgacgcctacacgcccggcgacgtgggtggtgcacggcccgaccgcgcggccatcgtctattcgcagcgctgcaaggaagcctggaacgacgtgccgatcatcctcggcggcatcgaagggtcgctgcgccgcattgcccactacgactactggcaggacaaggtccgccgctcgatcgtggtcgattcgaagtgcgacctgctgctgtacggcaacgccgagcgcgccatcgtcgaaatcgcgcaccggctggcggcgcgcgagccggtgcacgagatcaccgacgtgcgcggcacggcattcgtgtgccgcgaaacgccagaagagtggttcgagatcaactcgaccagcgtcgatgagccaggccgtgtcgaagcccacgtcaacccgtacctgatggtgtcggagcaggccaaggccaacggcgccacctgcgcgaaggaagacgaggcccaggccgtggcaaaggccgccgaagccggcgccgcagtgaacctcgtgaatccggccatcaagccgctgaccttcgtgccgaaccccgcgctccagcagcgcgcgaagatcaaggtcccgccgcgcgaccgcagcgtgattcgcctgccttcgtacgagcaggtgcgtgccgatccggttctgtacgcgcacgcgaaccgcgtgctgcacctcgagaccaaccccggcaacgcccgcgcgctggtgcaggcgcacggcgagggcaccacggcacgcgacgtgtggatcaacccgccgcccattccgctcaccacggccgagatggactacgtgttcgacctgccgtatgcgcgcagcccgcatccgcgctatgccgacgagaacggcagccacgacggcgccaccaagattcccgcctgggagatgatccgcttcagcgtgaacatcatgcgcggctgcttcggcggctgcaccttctgctccatcaccgagcacgagggccgcatcatccagagccgctcggaagaatcgatcatcaaggaggtcgaggccatccgcgacagcgtgagcggcttcaccggcaccatctccgacctgggcggccccacggccaacatgtaccgcctcggctgcaagagccccgagatcgaggctgcctgccgcaagcccagctgcgtgtacccgggcatctgccagaacctgggcaccaaccacgatccgctcatcaagatctaccgccgcgcacgcgcgctcaagggcatcaagaagatcctgatcggctcgggcctgcgctacgacctggccgtgcagtcgcccgagtacgtgaaggaactggtgcagcaccacgtcggcggctacctgaagatcgcgcccgagcacaccgagcagggcccgctcaccaagatgatgaagcccggcatcggcagctacgacaagttcaagcagatgttcgagaagttctcggccgaggctggcaagaagcagtacctcattccgtacttcattgccgcgcatccgggcaccagcgacgaggacatgatgaacctcgcgatctggctcaagaagaacggcttccgcgccgaccaggtgcagaccttctatccgagcccgatggccacggccaccacgatgtaccacaccaacaagaacccgctgcgcaagatcacgcgcgacagcgagacggtggacatcgtgcgcggcgacaagcgccgccggctgcacaaggcgttcctgcgctaccacgacgccaacaactggccgttgctgcgcgaggcgctcaagtcgatgggccgcgccgacctgatcggcaacggcaagcaccatctcattccgacctggcagccgctgaccgatggcgcctacacgagcgcacggcgcaagaactcgaccactgcgccggttgccgccaaggcatcggctccggtcaggctggcgccggtgaagccctccaagggccgcatcctcacgcagcacaccggtctgccgccgcgggacaacggcagcagcaagccgatcagcaagccttcgcgcaaggtgcgctgagcgagcgcgcggcgggcaggcgctacgcgtactgcatctcgccgttcccgaacgaccagttctccttcatcacctcgacgaggttgatgaagacgtcctcgcgccggatgtccagcttctggtgcaggtcgtcggccacgcgcttgtagaaggcctttttcatctcgatcgtgcgaccctggttcagcgtgatctgaatcagcacgaagcccggtgaatactcgatcccgagatagttcttcggatggaccaggtcttgcgcggcatgccgcgtgatgacttggaacttgtcgtccttcggcacattgatggtctcggtcatggcctggtagatcaggtcgccgatggcggggccgagcgtttccggcgaagcatcggacagttcgattcgaacgaatggcatggaggttccttgtgaacaggggcggagcctaacgccagaacgcaggcgaagcgcccgccagccagaaaacccaggccagcactgcggcgcagtgaagggcgaccgtgacgcgatacacggtcaggaagctccgcttgctcgacttgtggcgcagtaccctttgcgcggcccaggctcctggccagccgcccgtcagcgcgaacaggtgcaaggtgctctccttcgtgcgccagcggcccgtctgggccgcgttcttgtcgagcgcataggcgcagaaggtcagcaggctcaacgccggaacgacaccgagcgctagcggtggcaggcggccggaccagacggctgcgccgagcaacacaccgtaggccaggatgaaaagcacgccccacgaagcaggcgattcggacgcactcgcgcgacgcggcgttgcgcgaggtgcaggaggacggcggttgctgctgaccggcgcacgattcggtggcgttcgcgaggcaccggccagcgctgcctgcacggccatggcgcgtggtcccttgcccccgacgtggatctcttcgaagctcagttccatgccgacctgcggcttcagctgccgatcgctgaagtcgcgcaggtgcacgaacacatcggccgacatgtccggactgcgaatgaacccgaagccgcgctcggcctcccagcgtacgagtcggccttggcgtttcatggttgcgaacgggctggaagagggcacatggccgcgattctcccttgccgcggccgggcccggctcctatcatcggccgctcatgcatctgcaccactctccccctccgtcgacctgccgctgacgcgcgcctcgtgccgcgctcagacctgcaagtggtcgccgccgtccgccttcttcgtcaaggctggatgacggccggatggtcatgcccgccctctacaagagaggacggcgggcgtcatggagaactttcaacaatgaacgcaagaatgtctgccgccctggcctggggcggcgtgttgctggctggcgcgctctggggcgccggcgcgctggtggcgcaattcctcatcgatggcggcatcgcgccgcaaagcctctcgctggcgcgctttgcgctgggggtcccgcttctctggtatctgcactggcgcgcacgacggttgccgcaacccgcgatagccgcgacgcgctggagcgacctgtctcggccggagcagtggcaggtggtcggcaccggcgcagccatggcatcgaacgtgagctgctggttcgccggtattgcgcacctgggcgcggcgcttcccacggtcatctcgatctgctgcgccccggtgctcgttgcactggtgtccgtgctgcgcggctacgaacctttcggcctgcggctgctgggtggcctcgtgctggcgctggccggcgtggcactgctggtgatgccggccgacggttggagcgggaacggcctcgccgtcggacatgccgcgggcctcgcatggtcgttcggctcggcgctctgctatgcgctagtggtgctcggcaatgcgcgcatgccggtgcgcctgagcgccgtcaccgcctctgcctggggcatgaccgtggcaacgatctgcatgctcgcgattgcatggccggccggcatcacgtggcccgagggcagggtgcagtggctgggcgtgagctacaccggcgtggtgacgacgtctgtcgcgtacctggcctttgcgtggggcgcacggcgtctttcgcccacggccgctgtggtgggcacgctgatcgagccgctggtggctgcgttgctcgcggcgctggtgctcgcagagccgctggcgccacgccagtggttcggggcggtgctgcttgcgctggccatgctgctgctggtggggcgcgcggaaatcgcgaaaccaggcgcctgagcggaccgggggccgctcgttgtatggtgtggtcccatgagcagtccgttctttctgccggcttcatgggtgcgcatcctggcgggggctgccctgttcgcggtttcggcccatgcggcggcgttgccatccgattccgggggcgggtccgcttccgccgccgatgccttgcgcgccacgcatcaacgcatgagcggcaagctcgggcgcagcagtttcggacggccgatccagctcgattcgcaagaaacgccgagcgggctgcagggcgacatccatgcggtggtggaccattcgctgcctgcgatcagtgccgcactcaagcaatcgtcgcagtggtgcgaactgctcacgctgcacgtcaacaaccgccgctgccgcgcgggcacgacgccgcaaggccaagacatgctgacgctgttcgtcgtgcggcgttacgacaagccggtggagcaggcctttgagttgcctttcgtttatcgggtggccagtgcaacgccggagtacctgtcggtcgagatgaacgcggccagcgggccgctgggcaccagcaactaccgcgtcacgctcgaagcggtggcgctcgacgagcgaaggagcttccttcatttcagctacagctacgaccacaacatgatggttcgcatggccacgcaggcctacctcgccaccttcggccgcaacaaggtgggcttcaccgtggagggcaaaggcgcggacggccagcccgaatacatccgcggcctgcgcgggctggtggagcgcaatgcaatgcgctactttctcaccctggatgcctatctttcctcaggaaccggggcctccgccgagcggcgcgagcgccgctggtacgcagccgccgaacaatatccgcgacagctgcacgagatcgatctggaaacctatctcgcgatcaagcgcgaggaccggcagcgcgacggcgccggccgctgaattcacgggcttgtcacatgccgcggcgctaatcgccgggcctgtacctgttgtgcaggtgcacgacaaggacaagcaatgaaaagaagatcgaggatggggtggctggcgctggtgggtgccggcgctctggtcactgcctgcggtggcggcagcggcggtggagggggatgggcatttcccgtggtcggcagtggtggcggtggcggcacgaacccgccgccggtggcccagtccaagaccggcactttcctcgacgcggccgtcgaggggctcgactacacggcgggcggcagcgccaaggccagcaccaatgcgaacggcgaattcacctgcaccgacggcgagaccgtggccttcagtgccggcgcgctcgtgctgggcagcgctgcctgcgggacggcgatcacgccattgaacctggccggcggcaccgacgtgaaggccgatgcggtcgtcaatcggctgctcgcactgcagagcttcgacgaggaccgcgatccctcgaacggcattcgcctgacctcggcgctgaaggctgcgctcacggccggtgcgctcgatttcagcgccgcggccgacaacttcaacaccgctctcaatgcggtgctcgcggggctgcccgctccctacaatgcgcgcatggtcgattcgagccgccgcatgctggcgcgtgaacacttcgaaaacacgctggcttcgcgtctcgccgcaccggtggtcgaagcctcggcgcagaccaacgcccttggcaccatcggcatcggcgttacccgctaccaactgcaggccgatgccagcttcaacgtgccctatgagggcgacaacgagaagaccagggccgacttcctcaccggcttcctgccggcctacggctcgggcctggcgttcaagggcaaggccgacgacggcgcgctcgagttctacgcgatcaccgaccgcggcccgaacggcgacggcccgaccgcgcctgtgcccaacggcggcggcgccaccaacatcagcaaggtgtttccggcgccgtcgttcgcgccgagcttcggcatcgtgcgcatcggcaagaccggcgcggtgctcgcatcgagcctgccgctcaagctcgatgccaacaagaagatcacgggcctgccgccgcagtccggcgtgggatcgacgggcgaaacgccgctgaccgatcgctacgtgttcgatgccgccaaggcgaactacgacgccaatggcctcgaccccgagacgctggtgctcgacaaggcgcgcaacgtcctctggaccagcgacgagtacggccccttcatcgcacgcatcaacgtcgcaaccggcgtgatcgagaagaaatacgctcccggcagcggcgccgccgacctgccgctggtgctcgcgcagcgccgccccaaccgcggcatggagggcctgacgctcgatgctgccaatggcaagctgcacggcttcctgcaaagcccgatcgatccgaaggacggtgcgggcaagtcgatccaggcgacgccgccgggcggcagcaagaccgacgtgcgccacatcgcgaagttcacgcgctggctcgcgttcgatcccgccaccgagacatcgaagctctacgcctacccgatcgatggcagccagtacgacaagaaccgcaccggcaatgccaagctcggcgacgtggtgagcctgggcaacggccgtttcatcgtcatcgagcagggtgcgcgcaagagcgacgccaaggtgttcaacaagctgatgctggtcgagctgccggccgatgcgacggacatcgcggccttcgatcacaacctggagatcagcagcatcacgcaggcgccatcgggtgccgccgactactccaccgtggtgacgatgcgcaagaccgaactgctcgatctcaacgcactgggctggctggccgagaaggccgagggcctgaccgtggtggacgaccagacgctggcgctggtgaacgacaacgacttcggcgtcagcacgatcctgttcgatgccgacggcaagaccgtggccggcagcatcgaggactgcacggtggatgcggccggcgcgatcatcgccaagtgcccgatcggcgtgacgggcgcgcgcatcacgcgcggcagcgacctggagcggccgacgcgcatctggctcatcaagctcgatcgcaagctgagcgaactgcgcctttgatcagccggccagcgtgagcagcggcacgtcgcgctcgcggcccatggcctcgagttcggcgcgcgtgcgggccgccagccaggcggccagggccttgtgcgtggccgccgccatcatgtcgggcggcgccacgcccgccgcttcgcagaggcgggccgcgaaatgcggctccagtgccgccaccgccacgcggccatcggcacaagggtagacgcggtagcccgcatgggcgccgccgaccgcgcccgccggctgcgtcaggccccacgtgcgcggcagcgccagccagtcggccgaagcgttcagcgccacttcgaggtagacgccctcggccttgccgccagcgcgggcgcgcagcaacatggccttcagcaccgcctcgctcgcgagcagggcgccgcccatgtcggcatagagcgtgggcggcagctcggtgccggtcacgaggccgctttccgcgaggtaggtcaggtcgtggcccggttcctcggcgcgctcgcccggcgcaccgacgatggccacctgcgacagcaacggatggcgcgcctgcagcgcgggccagtcgaggcccagcttgcgcagcgccgaagggcggaatgaagtgagcagcacatccgccttcgcgagttcggcgtgcaactgctgctgtcccgcttcggtcttgaggtcggcggtctcgatggcgacgccttcgtgcagcgcggcgtaggcgggcttgttgtagagacccatggggtcgccgcccggcggctcgagcttcacgcaggtggctcccatttcgcggcagcgcaacaaggccgcagggccgggcaggttgagcgcgaggctcaggacgcgaacgcccgtgagcggctggaaggaggaggcagcgggacttggcatgggcgtagatccagagaacaggtcgacagccattttcaccttggcggggagccagatttcgcaagccatggcagccgctgcggcgtagcatgtgccacggcagaccgcctcctgccgctgttgcaacgatcaaggagacccaccatgtttgaagcgtccctcatgagcggccagcgcattctcgtgaccggcggcggcacaggcctcggccgcgccatggccgagcgttttctgggcctgggtgccgacgtggccatctgcggccggcgccaatcggtctgcgaagaaaccgcggccgagtggcgccagcagtttccggggcgccgcatcgacaccttcggcgtcgacatccgcattgcgcagaacgtcgacgagatggtggaaagcctgttccagagcggcgggctcacggggctcgtcaacaacgcggcaggcaacttcgtggcgccgaccgagagcctgtcgccgcgtgccttcgatgctgttgcgaacatcgtctttcacggcagtttctacgtcacgcaggccgtgggcaagcgctgggtggccgaggccaaggccggcaaatggaaggagggcgatgccttgcgcagcgtgatgagcatcatcgtcacgtgggtcgacaacggcagcccctacgtggtgccttcggccatgagcaaggccggcatcgaggtcatgaccaagtcgctggcggtggagtgggcgcgccatggcattcgcctgaacgccgtcgggccgggcgagattccgaccgagggcatgagcaagcggctgaatcccggcgaggaacccggcgcgcgcagcaagaagaccaatccgatggcgcgcaccggccgcatgagcgagctgcagaacctggcggcctttctcatggcgccggggcagtgcgactggctcaccggccagagcatcatgatggacggcggcaatgcgctggccacgggcggcaacttctatgagttgcgccaatggagcgacgacgactggcaggccgcgcgcgagcgcatcgaggcgcagaaccagaaggacaaggcgcagcgctgacgagcgggcgccgtccgccgccagggcatcggccacgcgggtatcgttgcgcatcaacagaatttcaggagaaaagaagatgcaactcgtcggcatgctcgattcgccctacgtgcgccgcgtggccatttcgctgcgcctcttggggcttccgttcgaacaccgctcggtctcggtcttcagcaccttcgaacagttccaggcgatcaatcccgtcgtcaaggcgccgacgctggtgtgcgacgacggcacgctgctgatggattcctcgctgatcatcgactacgcggagacgatcgcgggccgcagcctcatgccttccgatagcgcggcccggcagcatgcgctgcgggtgctggggctcgcgctcgcagcgtgcgagaagacggtccagatcgtctacgagcgcaaactgcgcccgctcgaaaagcagcatgccccgtgggtcgacagggtgcgcaaccagctggccgccgcctatgccgggctcgaggccgagatacggaaactgcccgcggtggccgatgaagcctccatggggcaggccgcgctgacgagcgccgtggcatggagcttcacgcaactggtgattcccgacgtcactgcgccggccgattacccgtcgcttgcagcctttgccgtggatgcggaaaagctgcctgccttcctggcgcttgcgcaggtgtgattcagttcgcgatgtccgccccgcgctcggccagcaggctgcgcagcagcgagcgatggcagcgcgattcttcttcgcaatagcagcccacggaaagcgccgcgctgtgtgaaagggcggccagcaggtcgaggctgcggctcgcgtcggcttcggccatctcggccttgtacttgcgcatgaaggcgttccattgcgcgggcgttgccgcgtcctggcccagcttcatggtctccgcggacggggcgagattcgggtaccacacgtcataccagttctgcgaggcgaactcggttttcgggaccccgcgcggcgggcgtcgcacggtgccgatgcgaaggccctcgccgccggcgcgcggcgtaccgaggcgaacgatgcggatgctcatgtgcggttccttctcttcttgcgacggcccaggggcctgagtccagggtgttgggtaggcgacagccgccatcatcgccgagtgcccgtgcggggcgatactggcgcgaagaaacccaaggagacatcgcatgctcgaccgaatcgaatggactcgccaccccgacggcgtggtgcaactgcagctcgcacgcgccgacaagatgaacgcgctcgatcccgcgatgttcgacgcgctgatcgacgcgggcagggccctgtgcggcgacgccacggtgcgcgcggtggtgatgtcgggccagggcaaggctttttgcgccggcctggacatggcctccttcgagcgcatggggcagggcgctgccagcgcggtgttgggcgcggccgcggatggtgccgatctgtccgcccgcacgcatggcatttcgaatgcggcccagttcgtggcgatggcttggcgcgaggtgccggtgcccgtcatagcggcggtgcatggcgtggctttcggcggcggccttcaagtggcgctgggcgccgacatccgcatcgtcgcgcccgacaccaagctgtcggtgatggaaatcaaatggggcctggtgccggacatgggcggcatggtgctgatgcgcgggctcgcccgcagcgatgtggtgcgcgaactcaccttcacgggacgcgtcttctctggcgaggaggcgctgcagctgggctttgccacccggctggcagccgacccgctggcggaagcgctgcaaatggcacacgacatcgccgccaagagccctgacgccatccgcgccggcaaacgtcttctcaatgcgtcgctgtcgcaggaggcgcgcgctttgttgattgccgaatcggtggagcagcaggcgctgatcgggagccgcaaccaggtcgaggccgtgcaggccaacatcgagcggcgtccgccgcgcttcgacccgccggcctgagggtggccccgggagggggcgtcacggcgggcgtttttcggcattttttggcgccttgcagccaaatagcacgggaatcgggctcgatctcctgcaatatgtaagaattaagtatctttatttcaggcgtctgaccatcgccacaaaagagttgttctttatgtgatgaaggtcacgtctgccttgaattaagggtaggggaggggtggtggctgctgtcacattccttaacaattaattcttttgtctgcgacggcgttcctgcatgtcgaccacgttttcctgcaacctcaatgtgcccatcctggtgggcgaggatcgctacaagtacgtccccgtcgtcggggtctttcgcagcattccgttcgaccaggtcgatgagtgggtgatgcatcccggcggcggcccgcgcagcgatcgcgagctggcggccgaagttcttgtcgaaatccgcaagccgcttggcacgagcgggcgcaccgtgccgcactccttcgaagtggcagacattcttcagctggaccgtgcggctgccatcgtcgtgtccacgttccttgccgcattgccccgcgtctgagggcaagcaggccccatcacccggccgcgcgcgcctagtgcctgccgcgggcgtccaccggccagatcgcaaccagggtatcgccgtcgaccacgtggtaggcgtcgtgcagattgacggtcgggtcgcagtggggcgtgacgaactcgatgcgatcgcccagcgcggggcgctccgccgcgaacatcaacttgccgtgttcgtcgccgaagaaggcgtagcggctcgccggatcggcgccacgcgccaccaccggaacgccgcagtcggtggcaaagcacttggtgccgccgtcgacggtgacccagcccgccgcatgggtgctcaccaccgccgtctgcacgaacagtgacacctcgaagggcgaaggctgcgccgggccagcgagcacctgcgtgtattccgcgtccatgaagacataggagccggcctgcagttcggtgaacgcgtcgcgctctgcgtcgaggtcatgggtgccggtacccgcgccggtgacgatctcgaaatgaatgccgccgcgcttggcttcggccacgatgtgcgcgatggtttcgcgcagactggctgccgcggcactgcgctgttgccggtcgggtatgtgctgcagattgccggcataggcctgcaggccgcgcagcttcaggcgcggctcggccgcaatgcggcgtgcgagctcgagcacctgcgcctcggtggcggcgccggtgcggttgtagccggcgccgtagtcgaccagcacatcgagcgggtgcgtcagcccgagcgtggcttcggcaaggtcggccgcgttgcgcgggtcgtccaccaccaccatcattccgccggggcctgcgagcctggcgagcttgaccacgcgtgcgatcttgctcggggtgacggcgggcgaggtgatcagcacgcccggaatgccagccttgaccatcacctccgcctcgcccagcgtgacgcagctcacgccgatggcgcccgcagccacctggcgccgcgcaatctccacggacttgtgcgtcttgacgtgcggccggagccccacgccccgcgcgttggcaaacgcggccatgcgctcgatgttgcgcgcgagggcgccaaggtcgagcaggagcgccggcgtatcgagcgactgccgcccgccggcaatgccgatcagcggtgtattgacttgcgtgtcaggaagcatgagcaactttcaaatgcgggaagggcgtctgcgttggggaagaggacgaggaacgcggaatcgaacggcgaaatgatcgcaccgaaaggcattctcattctgattgacggcaccttgcgtctgccgcgccggcgcaagagaaagccgtcagtcgccccgcgatggtgttcggcgcggggtgcgcctgagcgccaaccaccacagcagcgccgcattgacggcccatcctcccgcaagaacgatgagtgcggtttgcgcgacgcccggcgccagatcgagcgtcaccaacgccagcgaccacggcaacgcccccgcgatggccgccagcatggccgtctcgctctcggggaaagccgcggacgaaaccacgcacaccgcgcccgcggccgtataggcgagcgcgcccaggcgccaccacgaagggaagagcggtcgagggtccggttctgcggtgtgcatgtgctgaagattgcagatggcagcatcatgccgcgacagccgctcgcgcgcagcggtgtaggccttcaggcgacgagtggcatcaaccgtacggttgcgagcaggcagcggaccggcaggcccgtacgtggatgtgtgggtagaattcggccttcccggcggaagcagaagcggccaagccgctgatttgcctggtgtggcccctgcttggggccgcgggtgcgaaggttcaagaccttgtgtgccagccaagcttctttcttcttctgtccggcccggaatctgcccgtagctcagttggatagagcacctgccttctaagcaggttgtcgggggttcgatcccctccgggcaggccatctcgcaccttcacccagccttacctctgccgcagccctgcctgcggcgaaagtcgttcatcccggaaactgcaccaccgggccgccaggcttggtacccggcggaacatacgcgggcgccggatcgccgccgcggccgagcgagcgggtgtaggtgtagatggccttcaagtctgcgtcggtcatcgcgcgcacgttgaaccatggcatgggcgggcggggcgtcatgacgcgcgcatgcttcacccactgctgctggctcatgtcagccatgaacaagcgcagattgaccgcgtatgtggtgccccacgggccggaccagcccaaggcgtcaccggtcaaccacagcttctcgtccacctcgccgttctttggcgcgtagccgggcgtgtggcaatcgttgcagcccgcgatcatcaccaggtagcggccgcgctggatctcgcccttgttcgccttctggcttccacctgtttgcgccccagctaaggctgaagacaggaggatggtcaacacggcggtggagcgcgcaacgcggcgaatcaggtgggcagtcggggcggcatggggattgatgcgatccttcattggctggctcctgggcttggcgttcatgtcgaagtagacatggcaccacggtagccctgggtgccgggccgcgcatgggcgcttcagccatttctgcctggtcgttttgtcatgggcaccgcggcgttgtagcgatcgatggccactgtggcgagatgcaacggtcacagctcccgcaacgttcgaccttgtagcagtgcagcgggaaaacccgcgaccgaaagccccgacgacgccctggatggcgcctgaaaggcggcttggcgcgtggcacagacattgcccccaatcctcgtgaaggcatgcctgcaggcacgcccgagccgctatccacacccacgaggagacaccccatgcaattgaagctcttgaacgcgctcatggccatcggcctggccgcggccggcagtgccggcgcgcaagtcacggacaagatgatccagtccgaagccaccaccaacggcaacgtcctgacctggggtgtgaacacccagggccagcgctactcgccgctgaagcaggtcaacaccggcaccgtgtcccggctggcgccggcatgggccttttccttcggaggggagaagcagcgcggccaggaggcgcagcccgtgatccacaagggcaagatgttcgtcaccgcttcctactcgcgcatctacgctctcgacgcgaccaccggcaagaagctgtggaagtacgagcaccgcctgcccgagggcatcatgccttgctgcgacgtcgtcaaccgcggcgcggcgctgtacgacaacctggtgatcttcgccacgctcgacgcccagctggtggcgctcgaccagaacaccggcgacgtggcctggaaggagaagatcgacgactacgcggccggctactcggccaccgccgcgccgatcatcgccaacggcctgatcctcaccggcgtgtcgggtggcgagttcggcatcgtcggccgcgtcgaggcgcgcgacgccaagacgggccgcatggtgtggtcgcgccccacggtggaaggccacatgggctacacctacgacaaggacggcaacaagcaggaggcgggcatctcgggcaccgtcaacaacagctggccgggcgacctctggaagaccggaggcgccgccacctggctgggcggcaccttcgatgccaagaccggcctggcctacttcggcaccggcaacccggcgccgtggaacagccacttgcgcaagggcgacaacctgttttcatgcgcgaccgtggccatcgacgtgaagacgggccagatcaagtggcactaccagaacacgcccagcgacagctgggacttcgacggcgtgaacgagttcgtcaccttcgacatggacggccggcgcgtgggcggcaaggccgaccgcaacggctacttctacgtcaacgatgccaccaccggccagctcctcaatgcctttcccttcgtcaggaagacgacctgggccgacggcatcgacctgaagaccggccggccgaacttcgtggccgcgaaccgtccgggcaacccggtcgacggcgacggtggcaagaagggcagttcggttttcgcggccccgggcttcctgggcggcaagaaccagatgccgatggcctacagccccgacacgaagatgttctacgtgcccgccaacgaatggggcatggacatctggaacgaaccggtggcctacaagaagggcgcggcctacctgggctcgggcttcaccatcaagccgctcaacgaggactacatcggcgcgctgcgcgcggtcgatcccaagaccggcaagatcgcctgggaggtcaagaacggcgcgccgctgtggggcggggtgctcaccaccggcggcaacctggtgttctggggcacgccagagggctacctgaaggcggccgacgccaagaccggcaaggtgctgtgggagttccagaccggctcgggcgtggttgcgccgccggtcacctggcagcagggcggcgagcagtacgtggccgtggtctccggctggggtggcgcggtgccgctgtggggcggcgaggtggccaagaaggtcaacctgctggagcagggcggcatggtgtgggtcttcaagatcccctccaccggcagcacgcgcaccgcacgggcgggcgatgtccgcaccgcatccaactgaggaggcgccatgacgaatcgcaacagcgaagggagccgcgatgcctcccgccgggatttcgtcggccgcgcggtcggcggcgcctgcctgctggcggcagtgccggtgcgcgtgctggccgcgccgccgcgggccgaggagaacgacgagacgtcggtgcagctcggctacaagcacgacacgaagaacgtcgacaagaagaagtacccccgccatgcggccacgcaggaatgcgtgaactgcgcgatgtggcagggcacacccacggatgggtgggcgggctgcgcgatgttcgggcgcaagcaggtcgcggccaagggctggtgcatggcctgggcgcccaagcccgcgtgagcggcggagcgcgtctccgtgcccttcagcgcggggacgcacggtggcaggcgggcattgcgccctgcctgccggcgcagcgcaacgacgggtcggccgccttcacagcgagatctccatgccgtcgtaggccacctcgatgccatggctttcgagcacctggcgctgcgcgctggcggcatcgaggatcgggttgctgttgttgatgtggatcaacaccttgcgccgcgccgacgtggccagcatcgcgtccaccatgccgccgcgcgagccggcgccagtctgcggcagatgccccatgtcgctggcggacctggtgccgaggcctgcgtggcgcatttcgtcctcggcccagaaggtgccgtcgagcagcaggcagtcggcgtcgtgcatccagcgcagttcctccgggcccacctctgcaaggcccggcgcgtagaagaggcggcggccgccctgcaggtcctcgatcaggagggcgatgttgtcgcccaccgtctgttcgcggcggtgcggcgaatagggtggagccttgccgggtatggccacggcggtgaagcgcagcgaggggaagcccgcgacgctgaagtcgacgagggtctgggtgccggccacggccagcatgtgccagcgcgtgccgcagtagtgctccagcacgctgagcacgggaaaggaagtggtcaggtcctcgaacacgcagggcgtggcatagaggtcgatgcagggcccttcacgcaggccgagcaagccggcgacgtggtcgatctgcgcatccatcagcaccaccgccttgatcggcgtgtcgcgcagtccgtggcgcggatgcagctgggcgtggctgcggatctgctggccgatgtcgggcgatgcattgagcagcacccacgattcgccgtccgcggagacggcgatcgagctttgcgtgcgcgcgcaggcatcgagcacgccctggcgctggcctgcgcacagcgggcagttgcagttccattgaggaaagccgccgcccgcgccggagccgaggacaaggattttcatgaggcctcaaaaaacgcgggggtcgaccattgcatgaagtctccttgtgtgggctgtgccggtccgggcggaattgccgggcggcggaattccgcaaatcgcatgcccacgcggcgcgatgcgcgaggcgcgccgaaatacaggtggtttcccttgggagcgcgcgcgaaatgctccaggctggtacagcgccgtgcggcgctggcacaggggtttacccgaggcttcgcacgcgccccgtcaatcgcccttgttccagcgcagcttgcgatagatggtgttgcggctgatgcccaggcgcttggaggcgacggagatgttgccgtcggccgccgcgagggcgctgcgaatcatgtcgatcccggcttcccccagggtgcgcggaacgtctggtggagcgtcgggcgagggctcggcgtcgcgcgaggggagcatcgtgtgctcgggtacggcagcagctggcgctgcctccggcagggcgggcgctccagggggaagcggcgccgctgcctgtgctgctgcagcgggcgcggcctggggccgcacgcgccggacatcctccaggaagtcgtccgacaagtggtgttcgcagatgtgcctttcgcccgcgcccatcacggcggcggtgcgaagcacgttggcgagctggcgcaggttgcccggccaggcataggccttgaagagcgccagcaccgaggcgtcgatctcgggcgtgtcctgcgggcattcggccagcaggatgcgccgcgccaccacgtcgaggtcgctgcgctcgcgcagcgccggcagccgcaccaccaggccgttgaggcggtagtacaggtcttcccggaaggtgcctgcgtcgatcatctcgcgcaggttgcggtgcgtggcgccgatgacggcaatgtccaccgggatcgacttgaggctgcccagagggctgacgttgcgctcctgcagcacccgcagcagccgcgcctgcagggacagcggcatgtcgccgatctcgtccaggaacagcgtgccgccgttggcctgcacgatgcgccccaccgcgcccttgcggcgcgcgccggtgaaggcgccatcctcgtagccgaacagctcggcctcgatcaacgattcgggaatggaggcgcaattcaccgccacgaagggctgccgggcgcgattcgaatcctggtgcacggcgcgcgcgagcagctccttgcccgtgccggtctcgccgaggacgagcagcggaatgtcgcggttgatgacgcgccgcaccttctgcagcgtggccgcgatctgggcgtcgccggtgtccaggtagtgcaggccggagaaaggaggctgcgaggaagggcaggggttccgtgtcgccgcggcggcgccatcacccgccgcgtgcgcccgaggagcactcgcctcgccgggcatgcgcggctccaccgaggtcacgggcatgtccagcaccaccccacgctgcggcccgttgaatcgggcgctgacatggaactgctgcccattggccgcatgcagcatcatcggcgtgggcagcggcgcgcggaaatggtcgaacacggccgaggccgtgatgccgaacaggctggtcaggctctgcatgcgcagcgcggcgatgctcatgtccagctggtccagtgcgccgcggttggcgcccaggatcttgccgtcgacgccgacgacgatgatcccctcgagcagcgtgccgatgaactccgcacggccatggaagtgcagccgcaggcggttgccgtagtcgtccgacaaccactggttctcgatcatgcgtgccgacatgcgcaccaggcccatggtgtgctggtggtaggagcgctggtcgccggtgacgtcgagcacgcccagcatctcgccgcggggatcgaagatcggcgcggccgaacaggtgaggaagttgttggcgtggatgaagtgctcgccgccatgcacgaccgtcggcgtttcctcgaccagcgtggtgccgatggcgttcgtgcccttggaatgctcggcccagctcacccccggcgtgagcgccaccttgttggcgcgctgcaggaacttgtcgtcgccgacggagtggaggatggtgccggtggtgtcggccagcacgatcatgctgtcggtgtcgacgatctgctcgagcagcatctccatcaccggcgccgcgtgcgtgaacagccgctggttgcgctcgcgcgccaccacgaggtcgctgcgccgcagcggatcgaagtccggccgctcgatgcgcgacaggcccagcgcggcgcagcgctggtgccactgctcgatcagctcggtgcggcctgctcggggtggcgtgacggccagcgtcgatggcttggtccagccctgtggagggctggctggggcatgaaaggcgtcaaccatctgctgtctcctgtcctgcttctttgagcgggcaacttgtctctggccagtttgaggaatgctctcactgggttgcttcattctggaacacccccagggagcgcggtgttccgagccgacgctgcagaggcaaggatgccacagcaaccggcccttgtgggcactgtcccggtgtcgggacggtacagggaaggcaatttgtgttcccgcttgcagcaacagaccgttggcacagcgattgcaaatttgtgggggttcccaatcaccacaacggagacccgacatgatgaatcccgatccaagaatcctgcggcccctggtccgtccgccgaggctgcgcaaagcggtgcttgcggcggtgctgagcgtggccgcttccggcgctgcctgggcccacggcgacgtcacgccgcaggccgtggacacgtcgtcgctgccgaagctgggcgatcagtggcgcgcagagaacccgtttcgcggcaacagcggggccatgcagatcggcacctccgcctataaccagaactgcgcgcgctgccacggcatcgacgccatctccggcggcatcgcacccgacctgcgcaagctcgacaacgattgcgccgccctcaaggacgccgcgcgcaaggcggcctgcgtgaaggagatcgacgacttcttcctcaccaccgtgcggcgtggccgcacgcgcaacggtgccgtctacatgccgccgttcgaaggagcgatgaaccaggaggcgatctgggcgatcaagacctacctggagacgcggcgcgacaagccgatgtgaggcggctgcgatgcacacacttccttccttcttgtcgcgccgcgaatgcctgcgatgggccgcggccgccggcgtggccgtgctctctggcacggcacgcgcgggcacgctcgacaggatccgcgcacgcggcacgctgagcgtcgcgatctaccaagacatgcccccgttccacgtggccggccagggcatcgacatcgaactggcgcgcgcgttggccggcgcgctggacgtgaagctctcgctgctgccgttcctggccgacgagaacatgggcgacgacctgcgcaacatggtgtggcgcggccactacctgggcttcggcccggccgacgtgatgctgcacgttccagtggaccgcccgctgatgaacgaaacgccgcaggcgctcatcttcgcgccgtactaccgcgagcgcgtggtgctggcgcggcggctcgaccgcttgccccaactggacacgctctccgcgctgggcgatgcgaaggtggcggtgtccggcaagacactggcgggctggctcatgatcggcgccgacaacggcgcctaccgcgaccagctcgacacccagccgaaggacggtgccgaggccgcccgcgccctgcagcgcggcgaggtggccgccgccgcggggctcgcctccgagatcgagtcggtgttgcgcggcgacgctcgctttgctattgcgccgctgccttcgccacgcattcagggcaacggctgggcggtgggcatggcggtcaggaaggacgcgaccgacctggcccaggcgctgcaggccagcgtcaatgccctcgttcaaggcgggcggctgcgcacgatgttcgaggggggaaacgtcgactggcaggcgccgtgagtcgacgagcgatggcagcgatcctgcgcattccagcggataccaacgagcaacaccaacgacggaccacgcgtccgaagaccccatgaacatgcccaattccatcgaatccgtccttgtcgagaaccgcgtattcccacccgacgcccgcgccagctctggtgcgcgcatctccggcatggccgcctacgaggccctgtgccgggaagccgagcaggacttcgaaggcttctggacccgcctggcccaggacaacctcacctggaccaagcccttcaccaagaccctggacgaatccaacgcccccttctaccaatggttcggcgacggcgaactcaacgccagcgccaactgcctggaccggcacatcggcacccccgtcgaacacaagaccgccatcgtcttcgaggccgacgacggcgccgtcacccgcgtcagctacaaggaactgctcgcccgcgtgagccagttcgccaacgccctgaaggccgccggcatccaaaagggcgaccgcgtcatcgtctacatgcccatgaccgtcgaaggcgtcgtcgccatgcaggcctgcgcgcgcatcggcgccacccacagcgtcgtgttcggcggcttctcggccaaggccctgcaagagcgcatcatcgacgccggcgccgtggccgtcatcaccgccaactaccagctgcgcggcggcaaggagctgcccctcaaagccatcgtggacgacggcatcgccatgggcggctgcgagtcgatccgggccgtgttcgtctacgagcgcacccccaccgcctggaatcgcgtcgaaggccgcgaccagagcttcgccgaggccctccagggccagagcaccgactgcccgcccgtgcccgtgaacgccgagcaccccctcttcatcctctacacctccggctccaccggcaagcccaagggcgtgcagcacgccaccggcggctacctgctgtgggcccggctcaccatggactggaccttcgacatccggcccgaagacgtgttctggtgcaccgccgacatcggctggatcaccggccacacctacgtggcctacggcccgctggccgccggcgccacccaggtggtgttcgaaggcatccccaccttcccgcacgccgggcgcttctggcagatgatcgagaagcacaaggtcagcgtcttctacaccgcccccaccgccatccgctcgctcatcaaggccgccgaaggcgacgagaaagtgcatccgaagaactgggacctttcgagcctgcgcatcctcggctcggtgggcgagcccatcaaccccgaggcctggatgtggtaccaccgccatatcggccgcgagcaatgtccgatcgtggacaccttctggcagaccgagaccggcggccacgtgatcacgccgctgcccggggccacgccgctggtgcccggctcctgcaccctgccgctgccgggcatcatggccgccatcgtggacgagaccggcaaggacctgccccacggcgcgggcggcatgctggtcatcaagcggccctggccctcgatgatccgcaccatctggaacgaccccgagcgcttcaggaagagctacttccccgaggagatgggcggcaccatctacctggccggcgatggggccgtacgcagtgccgaccgcggctacttccgcatcaccgggcgcatcgacgacgtgctgaacgtctcgggccaccggctgggcacgatggagatcgaatcggcgctggtgtccaagaccgacctggtggccgaggcggccgtggtgggccggcccgacgacgtgacgggcgaggcggtgtgcgcctttgtcgtgctcaagcgcagccgcccgaccggcgaggaggccaagcagatcgccaacgagctgcgcgcctgggtggccaaggagatcgggccgattgccaagcccaaggacatccgcttcggggacaacctgcccaagacgcgcagcggcaagatcatgcggcgcctgctgcgcagcattgccaagggggaggcgatcacgcaggacacgtccacgctggagaatccggccattctggagcagttgtcacaacggatttgaaaagcaaaacgcctgcaacaacttacgttattgcaggcgttcactttttttggtcggggcgaaaggattcgaaccttcgaccctctggtcccaaaacagaccgagaatccataaaaatcaacgacttggcgccattttgtctaacgcaagttcggcgctttggagttgtttttccctctgacgagtaaacgccgttagacggatttcagcgcgtcgcgctggtcttttttgcccgcttgtggcgcacgtaatcggcggtctgggtctgggtgctgtggccgcccatggtctgggcttggccgatgccgcggtcggtcacaccgtcgatgtccgtgagcgccttggcgcgcaggtcgtggaagtgggcgttcttgaccttggcccgctctcgagcgcgagtccaggcggtcgaggcgccgtcgtaggtgtagggctcgccctttagcgtggagaacacgtagcgcatgctgaccggcttcgcctttccggccttgccctgttggccgggcactggcggcgggtgcttcagccgctcgatgaccgccttcagctttggcgtccactcgatgagaattcgcacggccgtcgagtccgcggtcttcgccggttcgaagagaatcccttccttccgaatctgcgcccactccagcgtcaacaagtcgctgatgcgctggcccgtcaggtaggccatgtcgatcaggcagcagatcgtgtggcccgacctcgtgcggttgccatcgtccccatagcaggctgccaccttgatgcgccgcaactcgctgtccgtgatgtagcgcgtgcgcgccttcaccttcttcgtcttgaccgggtcgacggggttgcttcctgccggtcggaaccctttcacttcggcgaatcgaaggcgctcgcgcagcgcggccctgtaggcgttgtaactgcgcggctgcgcgtcccaggtctccaggaagtcgatcacgatgggcggcgtgatgtcgcgggcccggaactcggcgaacgcctccgagatcgccttgttgtgcgtcctgtcgtcggcttgggtcttctcggtgtgcttgctcccgatttccttcatccacgcggcgcagagcttcggcatcatgtcgtcgagcgacttgtcggtctcgatcttggccagcgccaggtacatggccgaaaggccttccttgattcggcagagcttcgtccacttccgctcatcgccaactgcagcgacgtgaaagtagcttccgtgtttctcgtagaccctcggcgggaggtcgcgtttcatgctctcttccttgtgaccggtcgaagtctgggctcgttcgccggcatgctggcgccggcgctgaccgcatcgtagtgcggccgctcgaggatgacactaccgtcaacccgcgaccggcgcgcccggtagaagccctggcgcagcagctcggccatctgctcggctgaccgcttgtagcctgtgagctgcttcagttcggcgcgggtcaggatcgcgctcgcctgctgcgcctcggcactcgacgccaggggagtttcggccgtggtcattgaatctccttcagcgcgtcgtcgcgcgctcggttcaattcggacatcttgccgaggtcgccgccgcggtcggggtggtaggccgaggcgaggcgccgatagatctcggacagctgcgcacggttcgtcacaccggtgccgaacacgtcccgccatgagcgcgggcccatcgcagtctgctgctggggcggtggtagcgccgagaagccggtgaacgcagcttccagcatgtcgccggtaccccagcgggcgatgccgcgcagcgcctcgatggtcttggcgatggcctgcatgttgtgctcgatcttctcccaccggtcgcacgcgaaggacatctgccgcttcttgtaggtgaagtagaccgagacgcccggatcgtccggctggcgctggttggcgagcggcagcccatcccgccggagcgcggtgttcgtgctgatgacaatggccggatccgggtagcggccggccaggcggccgatctcggcaacgatgttgtctcgagcgcgagcgaaggtcacatcgaacttggcgcgctctcggcgccagcgttcggtgcgcggccggccgacgggccattgcagtggataggcttcggcgctcacctggcgtctccttcaccggtttcgagcggcgcgtcgtcgggtttcgacgcagctgcgcggcgcaacatgccatcgcacccacacactgaccagtcgccgccgcagacgccgcaacggccgtcatccattcggatactcgcttggctgctggcgtttctccggctgtcgtcacgttttgccatctcgaccgccttgtcgagggtgctggcgctgaagtgaacggggccaaccggcggaaacacgacccaatgacccggagcccacaggttcgcgtatcggcgcagcgcaacaccagcgttcatgcggtcgcgctgctccggggtcatcttgtggtgatccatgcccgcccagcgccacagctgctcatggtcgatgcggtcggccaggtcaagcaaccgctgttgcttcgcgctaggggacatttcgccttgtgcttgttcggcggggtcgcgtggggtgtcgttcatgttcagtccgtccatttgatgcagccggcgctcgagcagcggccagaggtccggccatcgacagccgagaccacgaaggtgagaagcccgcggcacttcgtacagcggatggagccgcgctgcgtctcggcagggcgaaagtgagggggctggcagtgctgcttgcgcacctcggccattgcgcgcgccaccgcgctggcgaaggcgccgaagccgggggtggtcatggcggatctccagcatcgatggcgacgcttgagcagtccgggcagcggttgcccttcggcagcgtgcaagcgaagccgttggacttccggccgcagacaggcgcggtcgacagcgcgtgcgccagatgccgcgcataggtgctgacggcgcgccagtacgcggccatcggacccttgcgcttcagccaagacttttcggcctcggtgttggcctggtcacgcagttcccgtagcaccgcctcgaggggggcgcgttgctcggccggcagctcaagcagtttgcggccggccggcaggctcagcagagggttgatgtagcccatcagcgagcgtcctcagcgggctgggcgcgcaacggttgccattcgaccggccgcacctcgtagaagcccgagccgccgccggagtacggtacgaaccagcccttgaagggaggctgctcttctccgccgccatcggcgaagtgcatgggctcgaagacgtttcccttctcgtcgcggccgcggacgtgcaggatcttggagccgcggctcggcgcattggccaacgggtcccaacggccgggacgccactcgatcccttcggaccagtgcggcacgcgttccgagtgatgcgtgtccggcacctggtgcacagggaacggcgtagtgctgaccacttcaggcggcgccatggggcacctcgttccattcgcggccgtcgagcagacggccggcgagcttcttgccgaagcgttgaatcggttcgtcgagcgacttcggcgacgcaaacaccgctccgtctgcgcggcttcggtcgtacggtgcccactctccccactgcttgaacagaaacggcacgtggtgtgcctcgcactggtcgcgcagatctcgcgcccagtcgggatgcatcggccgcgcgccggggccactttcaccgccaatgatgacccaatcgatcccggggcggatgagcgccttctcgtctttcgacagaggttcactgatctcccagatgccgcgcccctcgcacacaggacacttcccatcggcatccagttcgcccggatggcgctcgcagtgcggagcgatgacgcgccacaggttcaccggccccagcagcggctccatgctgagaaagcgcttcgcagcgggaacagccagcagcctcgggatgtcgcggtccgcttcgggctggtcgaccacagtggcgccgacccaaacgttggcgggtacatcgccggccagccagcgttcgatccagcgcagcagcgcgacggctgcctcggatgcgcgttcgagccggccgcggagtgtcgccgcggcggcttcgagccggctgcgccagatgccgatgcgcttcgacagcatgagccagtcgatgtcgggcgtgagccgcaccagcgcgagcaggtcgatcagccattcgatgtcgacggcgttgtcgagccagtcagcgaggctcgcgcagaacacgcgttggcggcggccgtgctgcgcgaagaatgccgtagcctgagcattccagcgcttcggcaaagcccagtttgcggcgctcgtgcggtgccggggctcatgcgcgccccagcccaccttcatcgttcgggccggcgtactcaccgcggcgtagcagccatcgcacccgcgcgagatctgcgtgcagccgatccagggattgaaggtggaatcggtccattcgatcttggtgtcagctgccatggcgtgcctccctgatgtcgatgacgggcaggtagttgcccatggccagcggaggctggggcttgaggtcgatggtcaccaccaagccgtgctggcgcgcgtagtcgaccagttgctgggcgtgcatctgcaccgcctggatctctttggcgcggatgcggtcgggggaggtgtcgaggaggctggcttccatcattcgtctcccgagtgctgcagggccttctgcgcgtcggcgcagagcacctcgtctttcacgctggcaaacagtcggccgtagttccagctggtgtcgcggaaaacgcggccgtcctcgaagtcttcgaggcacgacagcacgtcgttcgcgatgtccttgtcctcggtcgtttcgatctggaagcgatcgagggcattgcgcacgcggtacgggccttcgctccagtcgccgcgcgtgagctgcatcgctatggcgaggtccagccgctgatccttggagcgcagcgcttcgagcacatccgaccagctggagtcgatcggtagctcgtagcgcagcagcacggccgccagctccatgtcggccttgcgcttttcgaccagggccgcggcttcgcgttccttcttggcgtcggactgcttggcttcttcctcggcgcgtgcggcgtaggcgtcgtagtccttcttcaggcgctcataggtgtgggtggcggcctcgaaaccatcggttgtcaggcagtgccggcgcaggtcgcccaggtagccggcgtcgtgccggatggtcttcgggtaccgggcgcgcgacttggtgtcgcgctcgctgtacgacttcggcatgccgatctcggccatgagggcttcgatgcgcgcggccacggccttgttcgcctcgatggcgggcaggttcttctcgtgcgtggagatgtcgcgtgcacgggccgattcgagctcgcgcagcgcatgcgccgccaccgcgcgcggattctcctgctggtaccggcccacgtaactggcgtagctcgaagggctggccatgcacttcccgatggaggcacacagctcgacgggctggatggtgattgggttcaaaatgcgactcctaacaaccggaggcagagatggataaacccgaaccgaatgagcttcgaatcgagctggagaagggggtgcaccgcgcagtggcggtgctgtatcagtacgccgcggacgccatcaccattcacgcgatcgagcgacacggcctgccgcctctttccgacgacgacaacacctacaacgaggtttcgaaggccgtggaggcggcaaagaagatttggtacggaacgctctgagcgaggatgtccaagcccacccgcaccgccgagcagctgcagcaacttctgcttgagcgcatagaagccatctcggacctgcgcggccaggtcaccgacgtgcaccgcggcggtgtggttggcatcccggccgaggagggtggcccgaactggaccgtccgcgtggtcagtgaccgcggcacgcaccgcgccgacatcgcgcggatcattcgccaactgcaggggcagttcgacctggaggactgaagcgcgcgatactccgaccccaaacaattggaggtgggaatgagcggactgaggatgctgagtctgtggacgctggctggatgcgtcatcgccgtaatcgctggctgggctccgctgtcggactggcttaaaacgcatgctgagctcgcagcttgggtgcaggcggttgggtcggtcgccgcaatcatcgcgacgggcatctacgtgcaatggcagcaccagctcgaagtcgagcgaaaagggatcgaagaccttcaggcgcgacgaagaaggctcgaagtcatagtcgagctctcgcgagcgaccaagtcgagcgtgcgatgggtccaacagcagctgatggatagggaaacggtgcacgacactgccgaaggaaggctgtaccttgatcgtcgggtcgtcgcagaacttggaacactgttgtctgcgatcccgttgcatgagcttgaggatccgacggttgccaatgaagttctttcccttcttcatagcgcgcgaaagatgagtggcttggtagacgacctcctccggttgcatcgagtgttggatgcgcaaatgtttgagaacgctttcattgccttggcgcaagccgcagacgcatgcgaggttcactacgtgaacttgcgtcagcgcgttgacttggttgcgcccaaatagcccatctgcttcgtcgtgcatgggaaacatcaagcgaccctcccgtaaatctgcgcttcgtgcacgaagttcgcgcgggccagtgcctcggcgagcggcgggcacacgctgttcccgcacatgcgcacctgggccgtgattgagagcgggatgcgcggcactgacagcgggtcttctgcctgcacgccacccttgaacagcagagccggatccggaatctcgtggatgatgtaggtggcagggaagccctgagcgcggaacagttccagcggcttgagcatgcgcagtgtgatgtcgaccaggacccaccactgcccggcttcccagaccagcaccatgtcgctttcctcggggaagtgctcgggcaggtgctcgtgcagtagcgcggcgcacagacgcgccttctcgcgatgttccagcgccaggcagtcagtgggaacttgcatcgtctcgaccagcgcgatgcggtccttgctggtgacggtggatacgggatccagcatggaccggctgttttcgccgacaccgaagtacttgacgcaataggccatcacgagccgctggttgctgccggcggcggtgatggtggacaccggcgcgtcggcactgcggccctcgccgtcgtagaaaccgccgttggcctgctcgaggcaggctgccaccagaacctgctcgccgcgatgcgcgccagtgatggcaggcagcggctcgtcgggaatccgaccaggtcgatcgccgtgatgcgtgaggtgcgtcaggtggcaggcgaccacggcgctcccaacgccgctcgctgtggccgtgggcaagggctgctccatgctgcggttgccatggctccagcggaccgcgccgctggcactcgactcgccgtggcccatgtcgaccagatgcgcggcgaccagcgcctgcttaatgccgcctgccaccgccgtgccagcgggaccttggatgtcttgggtccgtgcatcctggccgggccgctcgccataaccgatcgtgatgaggtgagccgccgcgagcgcgtgatgcgtgccgctggcggaaatcgtcgaaacaggttcggtgacggcgtcgccgttcaggtgggcttcactggtgccgcgcaacggagcgagcgcgggcgcgaccagcgagaaatgaccacccttcacctgggcgcattgggtgcgcaacggttcgttggcagccatattgcgttggttgctggcgttggcgtgctcgctgacgaagggagccagaaccggctgcgcgacggctcggtggttttcggtcgtgagggttcccaggggctgctcggcggaagccggtttgccggagtaggcaggaccgcccgcgccaacgatgaagcgcttgtcggtgttcaggacgtgacgccacaggcccttcgccacgcggcgctgggtgttcttcgccaggtccttcttccgcccgaagatggagttcgccttgatcgtgaagtcgatgacctcagcagccgtgcgccatggcaacacctggccgccgctgacagccttgctgatcggcgcgccgtgtgtcgggtcagggcgggtcaccacgggcaggccatcacggcgacccaccatgaagaagcgcttgcgaatggtgggcgtgttgtagtcgcaggcccgcaactcgtcccattccaggtcgtacttcatgccgtcgagcagctgtgccacctcggcttcagtgagcgccagcgggtcgccctcggcgcacagaaccgcgcgcatctcggcgatggcttcgttgccttcgcgctcttccaaggggatgccctgacgcagcatctgcacgaaggcacgaaaggtttctccgcgacgcgcaggattcggataccacttgccgtcggtgctcagcatcagagggccccaggtctggaattcctcgacgttctccaacatcattgcccgcggcttgcaccgcacgacccagcgcagcgcgacccaagcgaggcctcgaatgaactggctgaccggcgtgccgcccttggccttggagaagtgcttgcagtcgggcgacagccacacgagggccaccggctgattgcgggtgaccttgatcgggtccacgtcccacacgctctcgcacaggtgcagggtgcgagggtgattgatggcgtgcatcgccagcgccaccgggtcgtggttgatcgcaatgtcgactgggcggccgaatgcccgctcgaggccttcactggtgccgccaccaccggcgaagttgtcgatgatcagctcatcggcgaagccaatagggatcgtgaagtcgtcgcgcctcatgcatcgatctccgtgcgttccctgagggggcgcgcgaagccggcgcacgggggcgactcgtacatcatccgcacctcgtcgacctgccaatcgatgattggcttgagcggttgcggtgccacggcggcgagcgcatcggcagcaggcgcgtcgtcgctgatgaccatgacctcgcgcaccgcctcgacggtgatgccgagggcctgcgctgcggcgcgggcggctgcctcgcggtcgggattcagtgcaagggcgcgcgcgaacgcggccttcaccttctcgatggggatgacggtgaagtccatgcgtcaggcgtccttgccttcgccgtccgcatctgcgtcgggcgcgctgtccggattggtgtcgccgtcggggccgccgtgctgcgcggcgaagatgttgccagcgtcggggccaggtgctgcgctgccgtcagcgtcaggtgcagtcggcgtgtcgggcttgcccgcgcggtagcccttcttcaccgggatcagttcggccggcgccagcagcgtcaccgagatctcgccttcggaagccaggccggagagctcgccgtagacgtcgttgtcctgcagctcttcgccgttgtactggatggtccccatgatggtgacgctgccgccttcgctgacctcgtagtgcaggttggccaggaccacgtcggtgaagtcgacatgcgcgtcgtcggtgccccagtcccagatgaagcggtagccgcgccatttctcgcccttggcgtagtggtagctggtgggcagcttggagtgacgcaggttgggcagcggaatcgcaacgcctggcagcagctcttggcctgcctttagcgcgttgttgcagtagtggtgctcgcgcaggccgggctcgatcatgtcgagcagggtgttttcgccggtgagcgagaaggcaatgtcgatcgcgcgcaccttctcctcgccgtgcagctcgcggcgcgggttggcattggtgatggcgatctgcgtgggcttttcgagctggaaagacatggggtcggtgctccgatgagtgaggaaagaaagagggcggccgctctcacggcgctggctgggaattgagggagggaggaggagggttcagcccggccagcagcgcccgaaaaatggtcaggccgcagccggagcgggagcgcggaacttctcgaagggcagctgcttgatgtgctgcccgaagtacttgccgatcgactcggcgccgacgaactcggcatgcaccttcgcgtcgacgttcgggtagtggtagatcgagccattgccgcgggcgaaggtgacggccagcgtcttgcgggcagcgtcgtagccgacggccgcgacctggttggactcgaccggcgtcatgggaatggcgacgtactcggcttcggagaaggcttggggttcggcaaaggtcttgggcatggtggtggtcctctggtggttgatggatcaggcggcctgcttggcctggatggcttgcacgtgcgccacgagagcggcgcagatgtgagggaagtcggcttcgtgaaagagcaccgagccacgctccttgaggccgacgaagcccagcgtggcgaggccttcggccgagatcagcagcggggcgatccgctccttgatctggccgaggctcagcgtcgggtgtgcgctcgacgcggcggccgcacgcacgggcatggggattacggtgggcgctggtgctgcggcggaggcgccacttggcgttgccgctagcgccgcgacagcggcaggcgtcgtagttggggaagccgcgggcgccggcgcggcggcggtacgtatctcggccttggtgagcagcgcgcggatctcggtgacggccgtttccttggcctgctgcgccatgtccgcgagagagccgaagcgctcggcgtcgataggccaggcctcggtttcagccagcgtttcgcggatgcagtcgatggtgccgccagtgcgcacgccggcgcggccgagcgtggcgatcatcacctgctgctggatgccccgaatttcggataacgcaaggtccttgcggatcttctcgcgctgctcttcttccttcttcgcctcggccgcgcggtgctcggccacgcgggtcttcacgagcgaggtcaggtcttcgggtgccttgagcacgatctgcgcggtgtcggggaacagctgctgcaggccggccgcgagttcgcgcaaggtgcccaggttgatctggatgcggtcggccgccgcgctggccgcgatcttggcgttggccagcgcggtgtcgacggcgttttgcatgctgtcgaacgtgcgcaggcccttgatcgcaccgccgaagtccgcgggaatggcgggcatgtagggcttgccgaagcgggcgttgagcgccgccatgtgatcggccagcgctttgacgccaccggcgacgatttcgccccggcgcgcttccttccgtgccttgaccagcttgtccagttcgagccgcgtggagcgtgcctcggccgtgatgtcgtcgatggtcttgaacagcacgtcgatgctctcggtctggctgagcgcgtgctgcttggcggcggccagtcggctctcgacctcgccgcaccacttcaccgtcttgtcggcattggcgaagtcctggtcggtcttcaggtcgcgattgatgccggcgaacacggccagcgcgtgctcgcggtactgcgcgaggttgctggccgtcaccatgcccgtgacctcgatgcgcagcgcgggcagcgactcgggcgtgcgacccaccgcctcgacgaccggatcggtcggaacgtaggtttcgaggtcttgctcgaactgcgcccagcctgcgctgaggcgcgcgaaccatgccgggtcaggaaacacccacacgtagaccatcttctcgggcgtgccgtcggacacaacgaagatcagcttctcggcgcccgtcaccttcaggacctgctggcactgcggcatgtgctcatcgggcacctggccggcggtcacgatcgcggcaagcgcttcgttccactgcttgtgctccatggcgatgcggtcatccatcgacagaccgtcgcaagatgccgactcctttccgtcggagcaggtgactgcgtagagctcctcgccgatcagcttctcgatgtgcggccgcgccagcgcttccacttcgtggccgtggtccagcacgttgacctgaagccattcgctgaaggtcttcgcgatgcccgtcttcttcatgcgcagcagctcgttgcgcgtggtcttcttcgacaggcccagcatggcggctgcctcgctggcgccgaagtgctcgaggcggaactggtcccaggcgtcggtgccctgcaccaggtcgtgtgtttgcttcatggtggtggtccttcaggcgttgagttcggcgcggcgcttgtcgaagagcgcgttgagttcggtgcggtgggccgggtcggccacgtccttgatgaggtcggcggcaactgccagcgcgtcgtcgttcgccgccttgttcagctggtcggcgacgtgggcgtaggtcggacccgtggccgaagccggagagcggatggcggcgatctgttcgtcgctcagcgggaacttggtgcgcgctttgttgatgacctggtcggccttggcgcgaccctccgcgatggcggcacgccactcggggagacgctgcgcgaagaggtcggctggccagcaggttggcgcggccggaggtggcggcgcgccggcgcgcttctgttcgtcggcgccatcgctgccaccaccgccgcgcccgtcatcgtcggcatcgtccttggtggccagcccagtcgcggccagcagcgtgtagcgctgcaggtaggtgatcgtcgaggcaacctgctggatgctgttcttcttgccgcttgcgtcgggtgagccgtccatcgaaacggattcggcgtgcccgaggcggtgcgtgatcgtgcaaatgaccacgatacggccgcccgtctgctgcaggtcccaacgatgcgacaggccgtggcgcgccatcgcgggcaccacgacatcggcgatgtgggagagctcggcgtgcttgtagccgacgaagtcgccgtccttcgtggtgtagccgacgtgcttgcgcttgaagatttccagcggttcggccttgaagtcggccatggcctgcacgaaggccttgcgcgcttcgttcgcttcccagcgctgctgcagctccatcatcttctcgaactgctcgagcgtggcgccgctattgatggcggccatcatgatgccgacgggcgacttgtccacgaggccgccgccagcgcgcgcggcaggcgtcgggtgttctacacgtggggcgagttcgagcacttggctctcttcgacagtggttgcgttcacggttggtctttcaggggaagaaggtgagaaggaagtcggggcgcaggaaggcgatcgcagcggccacgacgcagcacccggccgcgacctgcagccagaccacgatcagctgcagcagctcgtcgatggcgccgtagggctctgccacgggctccggcgtgtcgtcgggaaagccatggggatgtgcgcggctcatggactgcctcactggaagttgttgaagacgagggccgcggcgatgccgatcacggcgacgatgtaaagggtgagatctgccgcgcggtgcgggtgggccggctccggaagcggcacgatcacgccgccgactgcggcagggccgaaggcctgttccagcgtgcgagggcagggcgtggtgcgctcgtgcgtggcatcgaccttgccgacgaacagggcgggcgcagagagcggggtgtggaagagcgcgctcacgaggccgactccggatcgcacagggcgaagtgctgcgcgagaaggcgtgctgcgtgctcgccgtcgacgatctgcacgtcgaggtcttgcttcgggaatatgggcagcacgtgctccgcatcgaagaggaagtgcgggccgttcacgaggcgctcccgcgaatcttggcggcggcatcggcgatggcagcgttgaccgtcatgcccttgccgaattgaaagagctgctttgcagcgcggtctgcttcgctgagggcgagccaatccttcgtgccggccgcatcgcgcatgagcatcacggtgccgagctgcgtagggtcggccgattgcagcgcgaagtcggcgctgtagaacacccagcctgccggcacgaggtcggcgcagcgggtgcgatccatcgaagccagctcctcgcgcgtcaccggcggcaggcgccgctcgaaccggctgttgtggatcggcacgaggtcgagattcacgtcgtgcctgctcaccacgcccgtccgttctgctgctcgagcgcgaagtggtcggagagggcgaagtacgccggcgtgcccttggcttcgttgacagccagatcggtagccagcgcttggtcttccgtcggcacgaacaccgcttcggggtggtgcttggcttcgacgcgctcgcggcgcacgctgcgtcggctggcgaggttggagcgggtgagggcgctcatcacgcggccgccatcaggttggtgacttctgcggcgtgcgcggcgctggccgaggccttcgtgatcgcggcggcggccccctgctcagcaacgcggcggccttcagcaaccagtttgcgcgcttcgtgcgcttcgatcttgttcaggccgttgtgcggcacgaattcgtagaaggtgcccttcgtggcgctggccagcacgtaggcgtccggcttgaagtcgccgtgcgtcgggaccttggccacgaccgtcagcgacaggaagccgaccttgacggtggcgccgactgaccagtcttgctttgctttggtttgcatgcccatctcctgtgttgatgggctcgattaaacgtggtgtttatctgattgtcaacaccatgtttaatcgtggtgtgtaaatttctcggagcggttgccgaagggcgcaaaaaagcccgcgcgaggcgggcttggtggtggtgcccccagtggggatttttgtttggtgtttgcgggcgtaggctaggcaatcattcaagctgaaggagagcgcgatgctggaacttctaccgcaacggaccggggggcgggaggcaaccatcaatggctacgcagtgccgcgcattgaagtcctcgaagacccggcaaccggccattggcgcatcacctacgacaggcgatttgccatcgtcgccgaaagcctcgaagaactgcaacgctggctatggatcgtcgccaacgcgcaagccgtgggcgaggggtattcctgccatggggagaattccgtctttagaccgaaccctcaccagagacgggtcatgcagatcggatcgatagaagctgcccctatgggcactctggaagactgagcagattgttgggctgctccccgtcgttctcggtcttgaggtacttgttgcctctggcgctgatagcaattacgacccagacggatgtcccgcggacgctcacataaaaattccacttgccctgctcgatacccgcgatagccgcctccagcggcagcttccatggggtcccatccgcgttgacacctccaacgaaagcgatcctctcgtgcgcatcttggcgcggtgtcttgttgatgcactgaatttgcacattttgtgccatggcttctcctctgtacaacccacgaaccgcatgggcgcggccttctcatggtgttgctgtagctgccgtccaatcagttgcagctgaaggtattgccgttggcacggcagaacttgccgtccgcccgccagaagtttcgcccgtcgcccgtccggttgtatcgattgccagcgctgtcccagcacccactggcgttgcagttcgtgatggtggtgggtgcgccgctgccggcttggcgagcttcgtcggcgcgcgcgtcgcgttcggctcgcctggcgcggtccgcatccatcgtcgccatgcgacgctgcatgttgcgttcgtcctgggctcggattcgttcattgggatcgctttgaatgatcccgccacctgcgtcacccacggcatcacttgtgggctccctcaggagtcgcgcggcgttctcaatgctctccatgttgcgctgcctgccgtagacctcgttctcccagcgtctatcggtcgcatcagctccgagtactcgagccgcctgctttgcagtggtggggcatgcggtgtcgctgaacgacaccttgcctgcagcatcagtgcagcggtggacctgggcgcaggcggcaaaggacgctgcgagcaaagttgtggcaaccagcgcttttgagcagctcatattgcggtcccctcacagtttttttccgttccacgcccagaccactcgcccgcggacttccaccggacgggagccgtcgagcacgtcgactgttttcaccgtagggttgtcactgctgatctcgaacgtgccgtcgatgcgctgacgcacgcgcttgatgtagatccggtcgttggcttccatgacatacacgccatcgatcttgggtgcggtcacgccgatgtcgaccagcaggacgtcgccatcggcaaaggtggggtccatcgaatcgccgtagccgtggatgaaccgtaggttctccatcttcgtgagcggcttgatggttcggctcacccactggggcgacacggtgaggcggccgacgaccacttcatcgtgcaactgatcctcacctggccccatcgaagcaagctgcgccagcacgggaatgctcagtgcctcgaagccagggagatagagctcgctagtttctggggtgccgcccgacttcgcggctggtggccggtgcttcgctgctgcatcttcgtcgccctcgccggtaagtagccagttcgcggagcagcccagctctctttcagcgcggatcgcaccttccttggacatgccgcggcttttccagttcgtcagcgtggccgaactgacttgcagcaatacctggagagcagcgaagtcgctgacctgatgcgctgcaccctttgtcttttttcttgcgtagtcgaggaggcggctcacggaggggtgcatccgggaattctgaggcactaaacagggcgttgataaacgtggtgttgacactttaataaacaccatgtttaatcccgcccatgactgatatcgaactgatcaaggctctcggcgggccaaccaaggtagccgagctgttgggttacgacaagtccaacggtggggtgcaacgtgttcagaactggctgacccgcggcattcctgctcaggtgaagctcgacaaccagctgctctttctcaaggcgcagcgagaagcggagcgcaagtcggagccggccggggagggcgcctgatatgcgcagtacgccatcggaatggcagcgcataagggcgatctctcgagacagctccaggaagcgcgcttgcggtgcgcctcccgccgcactgagggccgaagcagttgcctcgacctcacaacccgtcaggtctcctgcttcttcaactcctcgacaagctgaagtcgcgctgcagcaatgtacttcgcgatctcctgggatgctcgctccgagcgcatcgggtgcgctccaaacaggccggggtgattcgtgattagcagcgccaacaaggtatcggccttcgatgctgcgatatctgcgtccattttgtctgcccctcgcggggtccgtgttgaggaactcggactctaccccgcgggtgggcagacacccgatgcaatcgagcctctggccaacaccctcgctctggtgctcgcctacgccttgttcctggtgaccgctgcgctcgccctgggcgctttcttcgtcggccgcccggccgccgcactcatcgcaatcgccgccggcgcgatcgctctctggctggttctggagggtgagcgcgcgctcgatgcgcaggcgctcgacgagttcaacggctagttcgtgaaggctttgaaacatgggaccgatggtcttttttatgtgcccggaggggatagtcaagtgaagtcaaatgaattgagccaggctgaagcacagcgcgaactggaccttttccggcagccggcgccgaacgaggttcctctcgagctggtccgcaagcaggccaacgccggcgcggctttcaccctggcgtgcacgtcctccgggttgcacgaccagagcatctacagcttcatcggcatcgacgctggcaccttctccaagatcaagaagggcatcgcgacgctgcaggccgaccagctggccaagttctgctacgcggtgaacaaccggatctatcccgagtggtgcgcttttcagctcggctgcacgctggtcgaactcaagactgaggccgagcgccgggccgaggccgccgagaagcgagcggccgaagcagagctcaaggtccgcgtgctgatggaaaccttccacgggagggcgaccgcatgaatgccgacagcaagatgatgcggacgctcggcgcgatcggtcagtccaccacctacagcgagatggcagcagccaccggcatcgacgccaagctgctgatgaccaacgtggcgcacctcaagcgccgcggctacgtcgagcgcatcaacgagggcgcaccgaagtgcgagatcgcgtacttccgccgcactgcgacgggagacggcctgatggacgccgaacctgagccggaactcgaaccgttcccggtggtggtcatgacgacggtgcagcgtgccatccaggcgcggccgccgctggccaccgtgtggagtgccgcgtgatggagtacgccgacttcctgcgcgcgaagattcggatggctcagttcaagggcttcgacgttccgctcgagcagatcaaccgccacctgaagccgcacacccgcgacatcgtgaagtgggcagtgcagggcggccagcgcgccatcttcgcgagcttcggcctgcacaagaccgccactcagctggaaatcttccggcagatcggccgggcccggcccgagctgtaccgcctgcaggttgcgccgctcggcgtgcggcaggagttccgcgacgagatcgaagcacgctttcaaggcgagcacgcgatcgacatgcgcttcgtgcgccgcgacagcgagatcgatgacccggccacgctgtacctgactaactacgaggcggtgcgcgagggcaacatcacggtgccgcgcttcggcgccaccagcctggatgaagccagcgtgctgcgcagctacggcagcaagacctatcaggagttcctgccggcctttgcacccgtcgagttcaagttcgtggccacggccacgccgagcccgaaccgcttcaaggagctgatccactacgccggctacctcggcgtgatggacactggccaggcgctcacacgcttcttccagcgtgacagcgaaaaggccggcaacctgaccctctacccgcacaaggaagaggagttctggctctgggtggccagctgggcggtgttcatccagcgccccagcgacctcggccattccgacgaaggctacgtgctccccgagctggacgtgcggtaccacgaggtgccgagcgactatgccgcagccggcaccgagaagaacggccagggcctgctgatccctgacgtggccatgggcctctcggcggcggccagcgagaagcgcggcagcatggccgcgcgcgtggccaaggtgcaggaaatcgtcagcgcggatcctgctgatcactttgtggtctggcacgacctcgaagacgagcgccacgccatccagcaggcgatccccgcggccgtcagtgtctggggttccctcgacctcgacgaacgtgaagaccgcatcgtcgccttcggcaagggcaagtaccgcgtgctgtccaccaagccggtgatcgccggcagcggctgcaactttcagcgccactgccaccgcgaggtcttcgcgggcatcggcttcaagttcaacgacttcatccagagcatccatcgggtccagcgcttcggccaggcccaccgggtgcgcatcgacatcgtgcacaccgaggccgagcgggaggtgctgcgcaccctgcttgcgaagtgggcacaacacgaagaaatgagtcagaagatgaccgacatcattcgcaagtacggactgagccagctcgccatgcaggacgcgctcgcgcgctccatcggcgtgaagcgcatcgaggtgcgcagcgacctgttcacggtggcgcaaaacgattgcgtcgaagaggcgaggctgcagccggagaactcggtcgaccagatcatcacaagcatcccgttcgcgaaccattacgaatacacaccgagctacaacgacttcggccacacccaggacaacgagcatttctgggagcagatggactttctgacgcccgagctgctgcggatcctgcggcccggccgcatctactgctgccacgtcaaggaccggatcaacttcggcaacgtcaccggcgccggcgtgcccacggtcagcccattccatgccgaagcgctgttccacggtctgaagcacggcttcgactacctggggatgatcacggtcgtgaccgacgtggtgcgggagaacaaccaaacctaccgcctcggctacacggaaatgtgcaaggacggcacgaagatgggtgtcggctcgccggaatacgtcctgctgttccacaagccgcagtccgaccgctcgcgcggctacgccgatgtaccggtggtgaagtcgaaggccgaatacagcctggcgcgctggcaggttgatgcgcacgccttctggcgctccagcggcgaccgcctgctgacggccgaggaaatggccagctacgggcccgccaagctggccaagctgtttaccgagcacagcctgcgcaacgtctacgacttcgatttccacgtgcgcatcggcgaggaactgctcgagcgccaggcgctgcccagcaccttcatgagcttggctccgggcagccatcacagcgaggtctggcacgacgtggtgcgcatgctgacgctgaatggggagcaatcgagccgcgcggtcgagaagcacgtctgcccgctgcagttcgacatcgtcgaccgcctgatcgagcgctacagcaacaagggcgacctgatctatgacccgttctgcgggctcggcacggtgcctgtacgcgcgatcaaggccggccgccgcggtggtggctccgaactcaacccagcctatttccttgaccagttgcactacctgcgggccgccgagcgcgacgccagcatgccgagcctgttcgacttcgaagcgctccaaaccgaaccggaggctgcatgacgcctgtccagatgctggttcaccgccagcgcgcgcatctgatcctcgccgagggcttgggcatcgagatctgcatggcactgggtgaccgcgatggcgcccaccggcaccgccgtgagatggaggcgcagatcgcggcgcgcgatgccgcaatccagcaagccgaggaagagggcgagagctacttcgccatctccggcacggtggccagcattcaggctgaagcgcggagggcggtgagcgcgtgaccgactcagctgaaaagacaaagcggccggcgtcccagtactactggggcgactggttcaaggacgtggccctgcagacctgttcgctgccggcccgcggcctctggcacgagatgaactgcctgatgcatcagggcgagccctacggtcatctgaccatgccgaacggcaagccgatggaacccctgcagctgggcaacctctgcaagattgggccttccctgtgccgcaagctgattgccgagctggaggagaacggcgtgttgtcacgagcggacaacggcgccatctacagccgccgcatggtccgcgacgaagacctccgcaaccgccgggcagcgggcggaaaagagggtgccgagcatggcatcaagggtgcagaggcgggttccaaggggggtaggccgaagcatggcaaggggggttctgaaacccccctcccggggttcgagaaaccccccccttcttcttcatcttcatcttcaccttcggggttatttccggaagctgacgcttcctcgtcgacagcgaggctgccgacctgccggcccgagcaggtcgtggcgatttaccacgaggtattgcctgaactgccgggcgttcgagtcatggacaaggcccgtgagaaggccatccgtgaccgctggcaatgggtgctgacctccgagaagccggatggctcgcgtcgcgcgacgacgagcgacgaagcgctggagtggttccgccgctatttcgatctagcccgcagcaacgacttcctgatggggcgcacgccccgcaatggcgagcacgcgaactggaaacccgacatcgagtacctgatgaagtcgcaagggctgaagcaggtgctggagaaaaccaatcttgaggccacagcatgaacgaccgtgtcgatgaatccctcctggcgcccgtggtgctgtggagccctgaggctgaaacctcgctgctcggcgcgctgctgctggacaacggcctgtgggaccgggtgggcgacatggttgccgaggctgatttcttcaagaccgagcacaagctgatcttcggtgccgtcagcagcatggtgaacgccggccagccggtcgacgtgttcacggccttcgaccagttgcagcgcgaccgcaaggccgacctggtggggctgacctacctgaacagcctcacgcagtacgtgcccagcgcagccagcgtgcggcagtacgcggtcatcgtgcgcgacttcgcgctgcgccggaagctgatgacggccagcagcgacattcacgagctggcctgtcagcgcggcatcggcttcgaagagacgctcgagcaggccacgtcgctgctgacaggcctgttcgatggcggcaagggcggcgagtggcagggcatggacgatggcgtcgtgctgctgctggaccgcatcaacgcccaggccgagggcaccgcggtcgacgactttaccgccacgggcctgtacgacctggacgctcggctcgacggcggcccccgcgatggcgagctgatcgtgatcggcgcgcgccccggcatgggcaagagcgcgctggccctgtcggccggcatgcacatggcgatggagagcgggaagacggtcggcatgttctcgatggagatgccgaaggcgcaggtcgtgagccgtgccatgtcgctgctgtcgcgcatccatctgagccgcatcaagcgcggcgaacggctcaaagactacgactggccggccatcaccgcggccgtggaccggctgcgcaaggtcaacttccaggtgaacgaccgcagcggcctgaacatcaaccagctgcgcgccgccgcgcgtggcctgcgccggcgccacggcaagctggcatgcctcatcgtcgactacctcggtctgatggctggcaccgatccgaagatgccgcgggtctaccagatcgaggagatcaccaagggcctgaagagcctggccaaggagctcggctgcccgatcttcctgctgtgccagctgaaccggaaggtcgaggagcgaatcgaccagatgcccgtgctttccgacctgcgcgactcgggctccgttgagcaggacgccgacatcgtgatcttcgtgcaccggccgcacaaggccaagccggatctgtccgacgagtggaagtactacgccaagctgtcggtggccaagctgcgcgacggcgagccgggcttcgtcgacctgatgtacgtcggggagaacacccggtttcagaactggccagccgagacgccgatcccgaccagccaggtgcgcaccgcgcgcgcggcgaaaggcggtgacctgtgatctacatcggcatcgacccgggcctcagcggcgcaatctcgttcgtgaccgaacgctcgtgcgtcgtcgaagaccttcccaccatgccgctgcccggcaatggcctcatcacgcggaagatcgacggccgcacgctggtcaaggtgatccgcgccaacgtgcccatcggcgagaccgccgaggcctacctcgagcaggtcagcaccatgggcggcaagaacaacgccgtccagacgcagggctcgctgatgcgctctctcggtgccatcgaaacggtgctggagtgcctgggctacaagcccacgatgctgggcccgcagaagtggaagcggttctacgggctcgacgcggacaagaaaaaggcgctggccaccgcgcgcggcctgtaccccgcggcaccgctaagcctggtgaagcatcacaaccgcgccgaagcggtccttatcgcccactggggcctgaggaacaaagcatgagggcgaacacctgtcatctacgccagcactcgccggaaagttcgctcgccggcacggaaacggttgtcatcaatgcgggcggcgatttcaccgtcggccagttcaagtcgaccaccaatttcgccggcagtctccatgccgggatgcggatgacggacttcgaacttcttcaggtgggtcagggtttggcggttgcctgttgcctcgtcttccacttgaaaactggcgactgcgcggtactcggtctgcatgatggcatctcgtttgttgaaaagctccgattgttctgcaggtcgatcaacggactgagggcagctttcccgaatcgaaatcggaggcacgcatgaccatctgtgcccgctgccatcgcgcgctgctgcgccagccggtttatctcgccggctcggcgtacggcccgaagtgcgccaccgccatctcgggctcgaagccgcgccgcggcgccgggcgcacgcccagcgtcgatgcccgccagccagaccttttcaccgaggccgcaccatgaagaccgtgaccatcaccagttcggagcaatacaaggcggtcgtgcgcgcatggtatgcgtccgacgtgtccgaggacctgcaggccggccactccatcgagctcactctgaagcgccggaaagacacgaagagccggctgcaggaggagaagtaccacgcgatgctcaacgacatcgccaggcagtgccggctgttcggcaagcagctgccgcctatctcgtggaagcgcgtgctggtcgatgccttcaagcatgagacgaaggacgatccgcagttccgtgaccactgggccaggttcggcgacatcgaactggtaccggcgctgaaccatccgggcttcgtgatggtgggcgagcagacgcgcagcttcaacacgacgcttgcggccggcttcatcgaatggctgctggcgtatggcgctgagaacagcgtgcagtggacgccatcgcgcgcgcagcgggcccagtacgaggagatgcagcgatgaaacgctcgcccatgtcccgcggcaccggcttcgcccgccgcgcgtacagcgcgccgccggtagcaccgcagcgccgcgtagagcgcgccggcgtcatcgtgcgggtctccgccgcgcccgcggcccggccgaaatcggaagcgcaccgcaacccgtacctcctcagcatggcgcgcggccgctactgcctgctgcgcgtgcccggcgtgtgcatcggcggcaccgagacgaccgtggcctgccactcgaacctgtcgattcacggcaaggctggcgcgcgcaaagcgaacgacgagtaccacgccccgggctgcttcgcctgccaccgttggctcgaccagggccccgccgatggcgtgctgaaggcgatgaccttcatgcgtgcacacctcgagcaggtcgactactggcgcgccgtggtcgccgacaccgcccagccgcccaaggaccgcgccgcggcccagtgggcgctcgaccacctcaatgcaacacccgtgggccaaccatgaccgctgaactcactgccaagcaggccggagtgctcgccttcatgcgcgggttcttcgctgagaacgaccacctacccggtgggccagatatcgcccgccacttcggtttccgaagccccaacgcaggcgccgagtacatctccgcgctcgagcggaagggctacgtcgagcgcaatgcggtcggcaggtaccgtttcaccaggagctcggaatgcgcaagcgcacccgccgccagcactacgcgctgaccaacccggtggccctggccatcgccggcgcacgcatcaccgaagactgcttgctcgaccagctgcgcacgcgcgaactgtcggctatccattccttcgctacgggcgccgccaccgtcgacgactggcgcaccgtcgccgatctgtgcaatctcgcgcagaccatgtgcggcatgggtatcggtcccgaggtgctggagccggcgctgaaggtcgagagcgtgctcggcgaagcgcacgagcgctacctggccaccaaccgcatgggcaccaccggtgtcggcctggacgccatgcgccaccttcaggaatggcaccacctccagcgcacgagcgtcgcgcgctcggtctacgaagccgccatcgtgcgcaccagcaatcggatccgcagtgcacacccgagcgtcaaggtgtgcatcggcacccccagtcacacaggagcccaatgacccctacgcagcctcaacccgtccgccgaggtgccggcgacctggtcttccagacgatccaggacctgcataacgccggccgcatcgccacgcggcccgtcgtcgtggcgatgaccggccagagctacagcgtcgtcgatgaccacgtgaagcggatgctggaagacggccggctgcggcgcgtcgcgcccggtgtcttcgaacccgtcgaggagatgccgccggcgcaggcgatctcgctcaccgtgctgccgagcggcatggccaagctggaagtcggcgatgtgtgcctggacctcaacccggccgactgccgccggatcggcagcctgtttcgtggcagttgcgaagagctgacgggcctgcagggcgcgcgcgaactcgccgacggcgtggccgagctcaagcgccagttgaccgcggcgcatcgccgcgccgaccagcaagacgaagtgatccgccggctgcagcgccagcccaagcaagacgaaatgccattcgcataaccggccgcgaggccacaacccgggcgagagcccatttcccaaggaaaaccatgagcaccaacgcatccatcgaacaggaaatccagaccaagggcaagaccgctccgcgcgtcacgccatcagatctcgccgcgaacatcgtcggcgaaacctacttcaccgcagccgacggcgtgctcggtgcgtacaagcggcacggggacgtgtaccaagggacggacgctcacagcccggcctacggcctgctgaccttctgcgtgctggtgctgcgcaacggcttcaccgtcaccggcgagagcgcttgcgccagcccggagaactttgacgccgagatcggccgaaaaatcgcccacgagaacgcggtgcagaaggtctggccgctcatgggatacgagctgaagtgccgcctggcgcggccggctgcctgatccagaccatcaccatccacgtcacaccaccaccatgatcccaaccatcgaagaaatcctcgccatgttcgccaagggcgactgcacccaggagcaagcctttcagtggatcggctcgcacattgacgcggccacgcgcgacgccgcgctgctcgatcacttcgccagcaccgcagccatcggtcgcgactcgaccggcaacatctcgacgctcagcgccacggcggtgatgggtgaagacccgccggactggccggcgaatcccggcaaggccatccagtggtggtgtgacgccgaggcccggatccgctacctcaaggccgagtcgatgatgaaggcgcgcatcctgtgatcttcaggcgcatcaacccggtgggcgcgccggcgttgctcatcgatgaaccgtcgccgttcgtcgttggagcggggcccgaccctcgcgacgcggacccggcgtaccagcgttgggtgctggcctgcctgcaggtgcggctcagcatccaggctgaccagacctttccgcacccgccggaccgacgcgcccaggtggcgcgcatcatccgcgcgtctcttgttgcagaatgatcattcggatactggagaatcaaccagcatgaagaccgcagagcctcccgctgcaccgttgtcgcagttgctcgcccttctcgaacaggtcgagttcgtgctcgccgccacggcgccggcaactgctcagcagatcgaggtgtggccggagttgcggcagcgtgcgaaggaagccagagccgctgtcaaggcgaccctgcgaggaccgaaaacgtgaagacttccgacctcattggagcgcaactggactactgggtggcgatggccgagggcttcatgcgcccgcggatcgagtggggcgtctgcatgatcgaccagccggacagccgtcccatgaacccgtcgacggattgggctcacggcggcccgatcatcgaacgcaagaagatcatgatttcctggaacgtggatcattggatctctggcgcgaacgatgcctctgataatcccaacagccgcatctggtctggacgcaccgcattgatcgctgcgatgcgtgcccacgtggcgtcgaagttcggtgatgaggtgcctgattgaaggcgtcggagctggtgggcaagcagcttgaggcctgggtggcgaaagccttgggagagcagcccgggacggcctacaccagcgcctggccaaacttcgaccaggtgcttgagcgcgatgcaatccacgtcgcgcccatggccggcaagaacttcacgtggtgcgccatcgtcgtcggccggcccaacggccggttgccggaaggccgcggtgggtggatcgaaggcgccacgccgcgcatcgccgtcgcgcgggccatcgtggccgcgcgcttcggcaacaccattgaggacgaccgatgaacgccttgatcgcagccgtagatcaacacgggaatcgcatatcggcggtggttccatgcacctgggagttccgagcaggaggggttcggctcgtcggcatagcggaaatccccatcattgccgagggcgtcgccaccagcgtggagatcttcacgccggacggtgagcacgtctacacgacgaagcgtgtcggcttgccacgcgcccgattgcggaaaggggacatcatcgtcctgcgcgttggcgaaatcgacatgctcgaaagcacttccggcaagcgctaggcaccccagtagggattggacgcccagcagggcgatcagaagatgcgggctccttcactccatcccctgaggacccgcatgaaatccacccgttccggcttcctggccttcgccgtcgctgcgcttgcgatcgcgtcaaccgctgtgaccttcacggtcgatcgcgtcagtgccgcgtgcacctacgctttccatgtggccaccgacttcctagccagcgccgtcgagaagttcgagcagccagtgctgcgcctcgctgcccgcccggtcgagatgctccaggcatgcgcctacgcgctcactctggccaagcgcgaacgcccccgcgtgacgcccggctggcgcatgtgcccctccacctgacctgattaaccctctccaagggcaagccgctgccgcaagagcagcgccggaggcaaccggcaccgtcagcagatctatgacaagcgcagcgttgctcctccacgcctaggtcggactgatggcccgaacaggcagcgccagcggaccttccatttcgcgcgccagcgcgcggcccagggtgtagtgggccggagaatttcggccgtgaacctgcggtctggcgaaaggggaatggcagggatattgatcccttggggcgcggccagcagcgcccaccagcctcgcatcgtcgaggaccatcacgcatgcggaacgcagggtttgagaaagcagcaacctcggttgccaagccaaaccggagcagtccgcagccgtgatggtgaatgcgcaggctgatgcgcgcacgttggacaaaggtgtccccgcgacaaccgaagcccgttcgactcgggaagccctggcgcaacgataagcagtcaggcaagccggagatcagcaccggccaccatcgacccacacggcctgaaataacggcccctgcagggaagcgctgcacttcagacggacctttcggggtccgtttgtcgttgcggggcgtttagatgaagccgatacgccgggcttccggctgcagcttcttggcggccttgagaagaaagctcaactgggtgtagtgctggaccagctgcacgcgttctccctcatcggtcacgccgatgaaggtcacgagatcgggcttggcgaagccgatggtctctgcgtggaagaggatgaccccaccgaatgacgcaatccgcagcgcaacctcgtggtccgcatcgagctgcgcctcgaagtcctctatgtactttcggatgttctccgctgtgcggatcaccgggttggacttccggtgctcgtgctccatgacgcctttcaaaacgtcatcaatttctgagtgacgtggaaccatttgagcaggaaaaggggtgtttggaggtgtggccatgcagcgattctgaccgccatcaggcgtccccccccgtagggtttgtcggtatccaagcccccggtaaccatccgggcccatgagtgaagacacccccgcaaagaaacccgactgggccgtcatcgaggccgagtaccgcgccggcatcaaacccctgcgcctcattggggaagagcaggggatcagccacgccgcaatcaacaagcgggccaagcgtgacgagtggtcccgagacctcggagccaagatccaggccaaggccgatgcactggtttccaaggcggcggttaccaaggaggttgccagcgccaagaaggtgaccgaacaggccatcgtcgaggctgccgcgaccatccagtacacggtgcgcatggagcaccgggcggacatcaagcgctcgcgcgtgctgttccagaacttgctcggcgagctggaggcggtgggcacccctgacgggcagcacctggtcgaccagctgatagagagcttgaacggtcccgaggaaggcgagaccgaagacgcggcccgccggcgccagacccgcaaccgcaagctgctcagcgagattcaggccctgcccacccgcatcgactcaggcaagcgcctggtcgagatgctggagaagctggtgcgcatggagcgcgaggccttcgggatcagcaccgatgaaggtggcgacaaccgcggcggcgccaagaccgtgatcgtgccggcgaaggacatcgcgtgaagctgcccgacgtcggcgaggacatcctctggaagcccgcccccaagcaggccatgctgctgtcggccatcgacctcgaggtgctgtacggcggtgccgcgggcgccggcaagtccgactgcctgctgatcgacgccctgggcctgcagcagaacgcgatccagaaccggaactaccaggccatcctgttccggcgcacgttccctgacctgcgcgacttgatcgaccgctcgcaggacctctacccggcgttcggcggcaagtacgacaagacccaccacatctggaccttcccgagcggcgcgcgcgtcgaattcgggcacatgcagtacgactcggaccgcttcaaataccgcggccgggccttccagtacatcggctgggacgagctgacgctgttcccgaccgacatcccgtaccggtacatgctctcgcgcctgcggtcgaaggacccggcgatcatctgctacgtgcgggcgaccacgaaccccgacgggcccggcttccgctgggtgaaggagtacttcaggatccagaccgagggcctgtcgacccgcttcaaggtctcagtcaccgaccccgagaccggcgaggtgcacgagcacggccgccgcttcatctcggcgcgcctgagcgacaacccccacctggcggacagtggctaccgccagaccctgctgctgctctcggccgaggaacagcgtgcgctgctgatgggccgctgggagacgccgaacatccgcggcgcctactacgccgagcagatggaagccgcgcgcctcgaggggcgcatccgcaagatcccgcgcctgccgcacgtgcccgtgaacaccttctgggacctgggctggaacgacactaccgcggtgtggttccaccagcgtgtcggcatggagcatcgcttcatcgactacatggaggccagcggcaaggacctgcagttcttcgccgccgagatccagggccgcagctacacctacgcgcgccactacctgccgcacgacgccgacaacaagaccctggccagcggcggcaagagtgtccgcatgctgctgcagggcctgctgcccgcccacaagttcgaggtggtgccgcgcaccgacagcctggtgtcggcgatcaaccagacgcgcgccgtcatcccgtcctgctacttcgacgaagaccgcacggccgacggcatcgccggcctggaagcctaccgccgcgagtgggacgagaagctcggcgacttcaagcaggagccgctccacgactgggcctcgaacccgtccgacgccttccggcagttcgcgcagggctaccgcgaaatctacaagggtggcaagaagccaaccagctggcgcgaccggctgaagacgcacgccgcccgcaaccgatcggcgcaagccgcataaaccatggcctctgctgtctacccctcgaagaacacccccgagcccaagggcgacgccatcgcgcgcgaaaactggtaccgctacctgtacggccgcgaccagggccacctcgactacatggcgcaggcgcagaagtgcgagggcatgtacctgggcggcggcgagcagtggagcgaagacgacaaggcgatcctgcgagaggagggccggccgttctacgagttcaacgagatcatgccgagcatcaacagtgcgatcggctaccagatccacaaccgcatggacattgccttcaagccgcgcggcaacaagggcgacctccagacggccggcatcctgtccaaggtggccatgcagatcgccgaccaggcgcagctgcactggaaggagacgcaggtgtttggcgatggcgtcatccagcagcgcggctacttcaacctgcggatgaacttcgacaccaacatgaagggcgaggtcgaagtcgagacgctcgatccgctcgacgtggtgccggatccggatgcgaagtcctacgaccccgactcgtggggcgacgtcatcatcacccgctggctcaccctcgacgagatcgagcagctgtacggaaaggacgctcgcaccaaggccgaggcctccggcgacgacggctccgactggggcgagatggatgacgagacgcggcgcaaccgcttcggcgaccgcctgcgcagcagcagcggcaccttcgacgcctacaacacgctggaaggcaagctcctgcgccggtaccgcatcgtcgaccggcagaagtgggtctacatgaacacgaagtgcatggtgttcccggacaccggcgacatcgaagcgatcgacgacatgaccgcggaacaggtcgcggccgccaccgagaagggcgcgatcagggccagccgcatgcgccggcgcatcaagtggacggtcagcacctactgcgcgctgatcttcgatcagtacagcccgcaccagcacttcacggtagtgccgtacttcgcctacttccgccgcggcaagacccggggcatggtggacaacgccatcggcccgcaggaggcactaaacaagggcgtgagccagttcgtggccatcgtgaacacggcggccaacagcgggtggatcaccgaagaggagtccatcaccaatatggaagatggcgagctcgagacggtcggcggccagacgggcctccatatcgagttcaagaagggttccacgccccccaagaagatcgagccgaaccaggtgccgaccggcatcgatcgcctgatcgaccgcgccacccaagcgctcaaggacgtgaccgtgcccgaggccatgcgcggtgcccagggcgccgaggtgtcgggcgtggccatccagtccaagcagttcgccagccagcagcagctcgcagtgcctctcgacaacctcagctacacccgcgcgctgctggccatccgcctggccaagatgatccagcgctactacgacagccaccgcatcttccgcatcaccgagaccgacgagttcggcaacgaaaaggaggaggtgctggagatcaacaagccgatgcccgacggcagctacttcaacgacatcacgatcggtgaatacgacgtggtggtcagtgagcagccgatgcagatcaccttcaacaacagccagttcacgcaggcgatggagatgaagaaggcgggcatcgccatccccgatcagatcccggtgcgctactccaacctgcaggacaagcaggaaatcatcgaaggcatgtcggctgccaaggcgccgcccgtcgatccggtggccgaggccaaagccaagctcgctctggcccaagccacgaagaccgacgccgagaccgtcgagtccaagggccgcacgatgtacagcgccatccagacggcgcaggtcatcgccgccacgcctgagaccagcgcgcttgccgatgcgctgctgggctcccagggcttccaggacatggacggcggcccgctggtgcccgaagccgcacccggcatggccgtggcgccggagggcctcatcccgaacaacaccaacccgctcacgccggccagccccgagctaggcgtgaaccgaggcatcgagacaccggaggccgacggcgtgcggccgaacccgatggcgcagatgcccgcttgatcaccaccaccgcaaccaccaccaaggagcatccatgaaccacatccattcgccccgaaccgacgacggcgccatcgagcaggagattcaggccaagggcaagaccgcaccgcgcgtcacgcccgcggacatcgccgcgaacatcagcgcagagacgtacttcacggcctacaacggtttcatgaccgacgccggccgcgacatgtcgatgtgcgatgccgatgcactcaagctgctcaccttctgcgtgctggtgctgcgcaacggcttcaccgtaaccggcgagagcgcatgcgccagcccggagaacttcgacgccgagatcggccgaaagatcgcccgtgagaacgcagtgcagaagatctggccgctcatgggctacgcgctgaagcagcagctgcacgccgccgcctgatcccccaatccaccaccaccagagagaaccaccatggctaccgaagaactcgtgaacgtcaccaacgtccccgtgaccgttgatcccaagaccgctgaagaccgcggcgacaacttcacccccactgacgacgagccgctgctcgacaacgacggcaacagcatcgacgcggccgatgctccgacccctgcgcccgcgccggcagccgctccgacggccgcgcctgtcgcggcacctgctgcagctgccgacgacctcgacggcgacgagatcgaacgccagaacggcggccagatcccgaagtcgcgcttcaacgaggtgaacgagcgtcgcaaggccgagaagctgcgggccgacgagctggcggccgagaacgcgcggctcaaggcagccgctgcagctcctgcagctgcaaccccgacacctgcgcctgcacctgcggccgcgccggcggtaccgtcgttcgacatcaacgcccaggagcgtgcgtacaccgaagccctgctcgatggcgacaccgacaaggcgctcaagatccgcggcgagatcaacgaccacatcctggccacggccgagcagcgcgccagcgtgcgggtgcgcggcgagctgtcgcaggcgcagcaggccaccgcgctcgaggaagcctcggatcaggccatcgccgacttcccgtacctgaatacggcggagggtgccaccgcgctgcgcatcatcgtggccacgcgcgacgcctacatcgccgacggcatgaagccgcacctcgccttgaagaaagccgcctcggaggtcgccccgcgctttgcaccggctcctgcgactgctgcagcacctggtgtgccccccagtagggaattgcccacggctacaccgccaattgatactcgcaccgccgacgcactgaagcgaggtgcagcagattcaaacctgcagcctcccgccatcgtgaacggcatcggcaaccgggccacccagggccgcatcgacgtcaccaccatgaccgaggcgcagttcgaagctctcccggaagccgagaagaagaagctgcgcggcgactagttccgcagcgaccgggcctgagggagttcaccgcccctcaggcgccacctggtgacctcgtccacacggcaggacggaaaagcagcccggcgccttgaccgcctccaacgtcatgttcccgcattggcagcgcaacgcctcaaccgacgttccaaccaaagcaaaaggagcatgccaaatggctgcaaccaatttcgcggcactcacgccgcaacaaaagatcgtttggtcccgcgacgtgtggcaagccgcacgcgaccagatgttcatcaagcgcttcctgggcaccggtgacaactcggtgatccagcgcatcaccgagctgacgaagaccgagaagggcgagcaggtgctcatgcatctggtggccgacctggtcgaagacggcggtgtcggcgacaacgagcgcgaaggcaacgaagaagagatgaagagctacagccaggtgctcaacatcgacctgatcaaccacggcgtgaagaacaagggcaagctggccgaccagaagacggtcatcaacttccgcgagatgggcaagagccgcctgagctactggctggccaaccgtgtcgaccagctggcgctgctgaccatgtcgggcatctcgtatgccttcatgaacaacggtgcgccgcgcgtgggctcagccttcccgacgctctcattcgctgccgacgtgtcggccccgaccgccaagcgcgccctgatgtgggacggcacggcgctggccacgtcgaacacggcttcgatcaccaccgccttcaccgtcagctacaagatgatcgtggacctcatcgcctacgcgaaggagaactacgtcaagccgctgatgtcggagggcaaggagtactacgtgctcttcgtccagccgggcactctggcgcagctcaagaaggatccggactaccagcgcgccgtcgtgggcgtggccacgaagtcgggcctcgacagcccgtggttcaccggtgcgacgatcaccgtcgacggcgccgtgatccacgagcaccgcctggtctacaacaccaagggcgcggcttcgggctcgaagtggggcgccgccggcctggtgaacggcacccgcacgttgctgtgcggttcgcaagcgctgggcatggccgacatcggtgtgccggaatgggacgagaagtccttccagtacggcagccagcagggcatcaacgtcgacaagatgttcggcctgctcaagccgaagttctattcgatctacgccaagacggtcgaagacttcggcatcgtcaccgtcgaccactacctgcagtaagcaggcgagggcggggcttcggctccgccctccacatctccccgaacaccctccgcacaccctgtcactgaaaggacagaatcatgtcgctccaacgcaaatccgatcgccagccgcgcctggtggcgatcctcgacatcggctttgccgaccccgccgcgtacggcacggccgagaacgcgatcagcctgccgggcaatgccatcgtggtgggcggtgcgctcaccgtgctgaccgcctggaactcggccacgaccgcgaccctgtcgctcggcgatgccacgctggccacgcgctacgccaacgccgtcgacctgaagacggcagcgcgcacggcgctcaccctcactggctacaagcacaccgtcggcgaatggctcaaggccctcatcgcccagaccggtgccgctgccacggccggtgccgcacgactcgaggtcgagtacatcgtcgccggccgcggcctgacgaaccaaggctgagccacggctttctcctggtgaagtggacgggcccgcgagggctctttaacccccggcggcttgatctccgccgggttttttgcacaaaggaaaactgaccatgaagctctatgcacccaccgaagaggccgtctcgatcggcctcaccagcggccacatgctcgttatcgagcgcgccggtaccgaagtcccgccgatgttccgccgcgaagccattgcccgcggctgcctgacgtcgcccgacgaggtggtcgagaccgacgacgaagccaacttcgatcgcaagaaggtcatcggcgacgccatccgcctgatgctcgacggtgacaacgaaggcgacttcaaaaacgatggcacgccgaacctcaacgcgctgcagaagcgtgtcggcttcgccgttcagcgcgaggaagccgacgcgatcttcaccgagatcagccaggaaggcgcaggcgactgatggacgtcgagcagttcatcgccacgttccgcagcgtcctcgacgacaaggccggcagcttcggcggcgggagcgaggacgtcttgtggtccgacgaggagatcgtcggctacctgacggaggcggtgaacgaggtggccgagcgtgcgctgctgatcgaggatcacaccacgccggccgtctgctccatcaccctgctggcgggcgtcggcgaatacacgctgcacccgtccgtgctccgcatcaagcgcctgacctggaacggccggccgctcgacgtcaccagcaccgaggcactcgacgaagagcacgtggcctgggagaccctggccgggcggccgtgccgctacgtgcactcgggctccgacaccctgcggctctaccggatcccgcgggccgaagacatcgcggtggcgccaaccctcgcgctcaccgtctaccgcacgccgctggcaccgtacagcgtgaacgacctcaccgaagtgccggagctcaagacgttctatcacgaccggctgatgcagtggatgtaccgctgtgcctacctgaagaaggactccgagaccttcgacgcgaacgccgccgccaagcacgaggccgccttcacggccagcttcggccagcgccccgatgccaacgtgcagcgcaagcgccgcgacaagcggccgcctgtggtgcggatgcggttctgatcatggtgcgcaccgtcaaagtcggctctctcgcccccggcatcaacaaccggctggagcccacgcagctgcagacggtcctgcccgaccgcagcaaggcgaccttcctctacggtgccgacaacgtcgacatcaacaagaagggctatctcaagcgccgccgcggcaccgccagcaccatcgccgggcagtcccattcgatctggagcgacaagcagggcgccttcgcggtgatcaacggctcgctcacggcgctggccgccagcggcgcggccctggccagctcggcggtgcgcgcaggcctgccggcgctcccgatctcctattcgcgcggcgccgacggtgacgtgtattggtccaacggccaggtcatccgccgcgtggctgagggcgtggaccgccccatcgccacggagccgctcgccgccgtgcctgccttcactctgacggccggtgcgctgcgcgaaggccgctacctgatcgcactcaccgtgcgcaccgtcgacggcgaatcgcctgccacaccggtcgcgcagctcgaggtgcccgatggcggcggcatcgccttcaccgcgcccacggcggtcgaggtctacatgtccggcccgaacggcgacatcctgacgcggcaggccaccggtgccgcaggcaacgtcgccatcgtcacccacgccgaagacggccgccgctgcgagacgctgaacatggcgctgatgcccgcgggcacggtcgtgcgccaccaccgcggccgcatgctggtggccagcggcaacaccctgtgcgtctcggagccctacagctacggcatcaccgacccgtcgaagtcctatttcccgttcccggcaccggtgaccgtcgtcgagcccaccgagggcggcgtgtacatctgcgccgacaagacctactggatcgacgacctgttcaacgagtcgctgcagacggtgctcccgtacggcgcgatccccggcaccagcgggagctcgccgaacgacctgcaggtgttctggcaggcacctggcggcctcgtcatcggcgatgcgaccggcgcagccaagaacgtgcaggaagacgcgctggagctttcgaatgccgccacgggcgcctcgctgtaccgcgagcgcgacggcatgcaccacatcgtttccacccgcttcggcgtggagccctccgtcgcagccgcgaccagcttcatggacgctgagatcgtccggaaaggcaccatcctatgaacagcctcgcatccaaagccgagagcggcttcacctacgtggtcgaggtcgtctcgcccgacggccggcgctcgcagcgcgaggtcgtgcacaacctcatccccacggaaggcctcaaccacatgatgggcgtgaccttcaagggcgccacgcaggtcgcgacctggttcatcggactgttcgagggcaactacacgccggtgccgacgaccagcgcggccaccatcgccgcggccgccaccgagtgcacggcgtacaccccgggcgcgcgtgtcgagttcgttgaaggtgccgtggccgcgggcgccgtcgataactcggccagcaaggccgaattcaccttcacggccgacaagaccatctacggcggcttcatcggctcggcctcgccgaagggggccaccacgggcgtgctcatcagcgccgtgcgtttcgcttcgcccaaggtactcacgaccggcgacgtcctcagcgtgaccgccggcaactctctcgtctctgcgtaaggaaccaccatgactctcaaagcctccaccggcctgcgcaatgcagttctcagcggcagctcgctgaagacggcgctcgcgctgggcaaaatcatgatctacggcggcgccgtgccagccgatgccgacgcggccgtgactggcacgctgctgaccacgatcaccttgaacagcacggccacgggcctcagcctgggcacggccgccaacggcacgctgccaaaggcggtcgaggtctggagcggggtcaacgcggccaccggcaccgcgacctacttccgcttcgtggccgcgggcgacaccggcgtgctcagcaccacgcaatcgcgtctgcagggcacctgcggcaccgccggtgctgacctgaacatgtcgagcgtcaatctgaccgccacggccgtgcagaccatcgacgccgccaatatcacgttgccgaccttctaagccatgcccacgctgaacatcgtcacgagcacgctgcccggcaactgcgcaactggcggctattccacgcacatcgcgggcaacggaacggtgttcgtggtgatgccggacaacggcagcacctactatcgctcgggcgacggcggtgcgacctggacgtcctacacgcatcccctacctgcgggtcagcggtaccacaatgctgtggcgtggaacggctcgtacttcctcgtcgtttacaacacacgctgggctaagagcacggacggcatcacgtggacgaacggcacgattgcgggcggctcctcgcactcgatgctggcctggagcggcacgcgctgggtgctcggcatgaccgcgtacaacaccaaccagcagctgtggagcacggatggcgagaactggaacgcggtcacggtgctgggcgtcaactggctctgtactgacgtcatctgggacggtgcgcggttctgcatggatgtggagcagcaattcgccacgccctacgataactatttcatgaccagccccgatggggtgacatggacccagcgcggcaagatgaacgtgtcgtcgggcgatggcgcagaccggatgttctacaacggcgcgctctacctcgtcatcaaccgctacccaaacccagctttcagtccggacggcatcacctggagcaactcgacaacttccgggggcgtcatcggcacttgcggcagcgacttcgtatcgcaggacacggcctcgaccttctcgaccagtactgacgcgacggtcttcacctcgattcccgtgaacctcggcggcacgggcgcttccggcttcttctgggattggaagccctgccaatatgcgccgggcaagttcgcctgcattggaaacagcaacaagttcgccaccttcgaggtgatcagcgcgatcccaccgttctggacttccttgaccggtacccgcgaggctgtctgatggcctacggcaagttccgcaacggcccgacctcacaggggcgccaggccgccaactgggtgcagggcgacagcgcggacttcacgacgcgccgccgcggcaatgcgctggtgcggaaagcgggcgaattcaccaacatcttccagaagccagatctcgcgctggacggctactacgttctcggcgacctggtgggcgccggcactcatgtgctcggctcggccacggcgcgcggcaccttctcggatcgcggcctggcacccgacaacggcggcttcgtgctgtcggaggtcggcttctacggcaagggctgggggtcgatcctcaagaatgggccgtccaccgtctacacggatttcgacggcgatccggccacggtctttgccaacacccttgcgcgcacccgcaacggtcgggtgctggcggatctgtacgactacaaccccgcggtgccgcaggaggcctcgggcaccctgtcgttcatcgtgcgcggcggctaccgctacgtcggcaccacgccgaccttctacaccggcttgaccttcaccgggctcgacggcggcggccagtacctgcaggccttcgtgcatgacgacggcaccacgcgcacgctcggcgggaccgaatacctgcccgggcagatcggctggtacgcgacccccagcgtgctcgcaccaggcgtgattctgaagatggaccgctacctgcggccgacggacgtggtgaccaccatcgatccccttgcatgccctggcctgcgcttcaactacacgaccgatggcggcctcggctgggccagcgccacggacagcatgttcgcggccgagctgctgaccatcaccgggttggacattgggcaccccggctatttcaacgacgcgatcgccgaagcgaacctccgcacggcgccgctgtcgcgcacgctgtcggtggccatcgggcacgtgccctacatcgagatggacggcaccacgcccgtggtgaaggtgaaggtgaagatgggcctcatcaacacaggcgccggttgcgcgctgtcggcgagcaccaccctgtatgacggcctgccgatcggcgccgcacgcttcctgagccgcgacctgctggccgtccccgagggcgtgctggtcttcacgcgagacgatgccggcggcgccgagtggaacgcgccggcacggatccggttcacgaacaacggcacagggttcgacgagcgcggctacatgccactgcccgagtactgcaccggcgtgccctcgggcatcgacaccaagaccctcatctgcccgatgttcgacggtgcctacaacctctaccagtcgaaggactggggcgcgacctggacgttgcgggccgccatcacggagaacggcgtaccgcccgccaccgggctgccggtgatggggaacttctccctcgtgaccatgctgcgcaaggacgatctgccagccaatgccgctcccgccacgccgtggctgtacgactgccgggccgccgaaccatgacgaactccctcatcaagaacaccaccatcgacaccacggtcgaggtgatggagattcccgcgattccgtatgtgccggcgcagcccgcgcgcacggtgtacgagacacgccgcgtctgcggcttccagcagaccggctcgggccactacacctacgtgaccgaggcctcgggcgcgatcacggccatttgggtgcctgatcctggcacgccgattcaggtcggcacctggggctgctgggaccagctggtgcctgtcacctatcccgccactgcggagcaactcgcggtgccgggctcgccagggtcgggcggcaccgtctcctcgaactacaaccttggctggaacgccggcggccgctcgatcgccatgttcacggccaacggctacgtgcagttccaagcgcgcgccagcgccgtgggcatcatcgccggcctcaacgtctatgacggcgtggacgcgcactacagcggcaacaccaccgactacgccttcctgttgtcccacggcgtggcgcgcgtcattcagaacggagtgcagggcgcctacctgggcacctacaccgatgcgacggtctttaagatcgaccgcaccggcacgaccatcacctactacatggccggcgtgtcggtggcgaccgccacgagcgcgccgaccgcgccggcctggctcgaggtgtcgctgtattcgggcgacgacgaggtgttcaacccgtcgctggtgcaggtcagcgcgcctgacctgaccgcgcagactgccaccctggatggcgtgctgctgccgctgaccttcttcggcacgcagggtccctttgcggaactgtcgggcgtgctgccggccctgaccgcacagatggaatcgggcgtggtgctgccgaactacgcagtaggcgattggcagctgccgccgctggcgatgagcctgaatggcctgacgggcgaaaccgctacgctcgcgggcacgctgttgggcctgcgcatgctggccgccgaccatccgtatgcggagatgttcgcgacgctgccgccgctgacggcgaacctgtcggcctacgaaggcaacttcaatgcctcgatcggctcggtggccgtggccggggcgtcgatgaccctggccagcttcctcgtggtgtcgatgctgtcgacgggcaccgtggcctcgacgctcgtggtgcacaccgcggtctctgccgagatgctctccgaagccgccctcggctcgaccttcgccgcaaatgccgtggtcgatgctgtgatgttgagcctggccagcagcggcaccgtgctgggcgtgcccgagagcgacaacgagacctgggtgatcaatctcgacagcggcggcaacaccagctactcgaactacgccttcaacagcttcgcgcgcatcggcagcaagtactacggcgccagcgccgccggcatcttcgaactcgacggcgacaccgacgacggcgcgctgatccgctcccgcatcagcctgggtgagctggacttcggcaatccgatgctcaagacggtcagcgagtgctatgtcggcatgtccggtactggccacttgttcgtcaagctgatcgccgagggccgcgagttcgtctacaagacccgcggctacagcgacaagctgaggcagcagcgcgtgacgtttggcaagggcctgcgcacgaactatgtggagctcgagctcttcaacgaagacggcgcggacttcgaactcgacaccgtcgaattccacgtcgccgacctttcacggaggatctgatggcaactattccccccggtggcatcgtcaccatccccgatccgacgagcggcggcgccggcgcgccggtcaccacgacccagatcatcaacgcgatgtgggcgaacgcgcagagcaagtccgaatctggggacctgcgcatcggccaggccatcggcttcgccgatccggcgccgcacgtgctcacgccaacgctggacacgacctacctgccgccgctgaagcccgacctgccgccggacagtccgaacgacgcggaggcgatgtacaacacccagcgcgaccagatgatcaacctgatcaccgactcgtgggcggacttcatcagcacctacttcccgaacccgggcttctacaacgatgcgctggcttggtgccataccgcgttcacctcgggcggttccgggctgagccctgtggtcgagcagcagctgtgggagcgtgcccgggcccggatcctggccgacagccagcgcgcggaagacgaggcgacggcgacctgggcgaatcgccgctggccggtgccgccaggcgcgctgaccaaccagatcaaccagatccgcctggacgccggccgcaagctggccgagcagagccgcgacatctcgatcaagtccttcgacaccgagatcgagaacgtgcgctttgccgtgaagcaggtgctcgaccagcgcaaggtcgcgctcgacgccacgggcgactacatcaagaccatcatgctcggcccgcagaccgccatgtcgctggccacgggtctcgcgaacatccgttcggaggcctcgcgcgcgctggtcgccctgtacagcgcggagtccgcggcgcttcagccgcgggtgcagctggccatcgctgatgcggacctgaagatgcgcggcgagcaggcgaacctgcaggcgcagatgaactcgctggagtcgaaggtgcgggcggccatcgccggcgcgcagctcgtcggccagcaggcagccgcaggcctcaacgcgatcaattcgagcgcttcgatcagcgggtcggacaccacgaacacctgatcgaaccggggggcggcgtcccccctgtagggttcgccccgggctccttgggccggcacgatgccggcaattcaaggagcctcccatgaccattcagatgggcgtcgatcgatgagcgacgaaccgaacaccgaacgcaccacgcggatcatcgatctgcgcatccccttgccatgggtgctcactggactgatcaccgtcggcttcacgctggtcagcatgtacttcaacgtgaaccagctcgtgcgcgacgtgggcgagctgcagatcaccgtgaaggccggcaatacccaagtcaccaccctggcgggcgaacaggccctcctgcgctttcgcatggagaacatcgagggcgagatgcgagcgatgaagtcgagccaaggcgcgcctgtggccccgaactaccccccaccgaggaagatcccatgaccacgctcaagcaacgtctcgtcgattggtacaacgcgcacgtcgtggcggcctggtaccgcagtgtcgcgctctacgtcggcatgtcggccaccatcgtgccgtacatccccgattggctgcagctggctctcgaccattgggacctggccagcgtgctgatcccgaagctctcgcccgatggcaaggcagtgctgcaagcgttcatcttgctggtgctgctgccgatcgcgaaggcatggcagcagaaggcgatgcgcgccgcggcgcttgaacaggcggtgcgcacggggcaggtcagcacggtcgccggctccgaggaggtgcagatcaacgtgggaaagggctgaccgtggacgcgcagcttctggcgcgctgcactggcgcccagctttcccgagcgcagcgattcgcggatgtgctgtcggccggcatggccttctacaacatcaccacgccgctgcggcaagcgatgttcctgcccaacatcgggcacgagtccggccggttggtctacacgaccgagctctgggggccgacgtcggcgcagcggcgctacgagggtcgcgtcgacctcggcaacacccaaccgggcgacggcaagcggtacgctggccacggcctgatccagacgaccgggcgggccaatcacgccgccgcgcgcgaccggctccgcgaacgctttcccgatgttcccgatttcgaagccgaaccggagaaactggcggagccgcagtgggccgcgctgtcggcgtgcgactactgggacatgcgtaagctcaacacctgggctgatgccggcgacttcgacaaggtatgcgacatcatcaaccgcggccgcgccaccccaggggtgggggattccaacggatgggccgagcgcctcgagctctacaacggcgcacgcaaggcgctggggctcgcctgagacgcgccacccagtagggtttggccgtgcagagggtcatcgattcaatgcctcccattgaagcgaatcaggaccaacgaccatgccaaccgaacttctcgcgcccggcactgctgcggccatctctgcggaaaccgttcttgctgatggtcagaccgcgaccgtcttcctgacgtccgacagcggctcgggcattccgaatgacagcccgttgttcatccagctgcagcgctccaccagcgcatggaacgatctggtcatcctgagcggcccgaacaagctgaaagcggaagttcatgggccggtgaccttccgcgtctcccggcgtgcgcctggcgtgtatgcgagcccgctgggcgccgaagtgacgatctcgactgctgcgggtagtggtagcagcagcgcggtcacagtcgctgatggcgccgatgcgacgcagggcgacaaggacgatgcgcccgcagcctccgacatcggttccttcagcatcgtcgcgttcatcaagcgcgggatgcagaactggaccacgctgctggcgcgcatccctgcgctgtccactggcgcggttccggtggagaacatcaagcagccgctcgtggcgcgccagctggccgctggtgccgccagcgtgaacacgccgctcaccaccacctgccgccgcatttccatctacgctcgcgccggcgacgggcgctatgccatcggaagcaccgcgcagaccgcctcggccacggcccacttcatcgctcagggcgagcgactggacgtcgccgtgcccgccacgccgaatatcgccgtgatgcgcggcggcgtgtcggactgcacgctggaactgacggagcttgcgtaatgcaggcacgcgcgacccggatgggtggccaccgcgcgcctacggcgcttgcggacgtgatcgcgggcatctttgcttcgacccctgcgagcgcttggtacgacccgagcgacctgtccacgatgtaccaggacaactttgctcagaccgccgtgacagcggtggagcagcctgtcgggttcatgatggacaagtcgaagggcggtgcgcctcgtggcgctgaggtcgtgctcaacggcggcttcgactctggcctcacgagctggacgacacccaacgcggcacccggcacgactaccttggttggctctcgcgtcgtgctcgacagcggcgcggccggcagcggtggcacggcgcgcttgcgtcaggctctgaccgtcccaatcggctggtacgaggtgacgttcgacattagcgccttcagcggtctcgccgggaatgcacagctggcgctcggctccgacctgtcgggcggctcgcagtacctcgcaatcagcgcatccactgtgggcaccgcgcgccgggttatctatgtctcaagcacgacgctcggcatcgcgtttttctgcggctccacgaccacgcagaccacgttcactgttgacaacctcacgatcaagccaatcagcggcgcgaacctttggacaggtgcccccactgtcaacaatggcagttgggttgacaacgccgatggcagctacaccaatgcaggtaacaccggcacgattgggtacaccaacaggttggttatcggaaaaacctacgaagcattcgttcgtgtcacagcccgcactgccggaaccttctatgtgccttatgacggggtggggccgaacgcgatcatcgtttccacggtcagcacgtatcggcgcgtcttcacagctacgaccaccagtctctacatctacagcaacgccttcaatggtacggtcgcttctgtctatgtgcaggaattgccaacagtcatcccattgacgcaagccacgagcactgcacgtccggtgttgtcggcgcgtgtgaacctgtttacgaaaagtgaaaagctggatgacgctgcgtgggcgaaagctgcgacggggactgctacggcacccgtagtaactgcggacacagcggttgcgcctgatggaacctcgactgctgatcgcgtcgtcttcgctttgaacggtggcaccacttcgaatgacttgtcgcaattctcgtttgcggccagtatcacaggtgtagtgggtggctcctacaccagttcgatttggatgaagaccaacgatggaactaccaaggtattcatgttggttggagtggcaggcggactgcatttgatttctgtcacaccgacatggcaaaggttctcgtgcacggaagtggccgtcggtacgtcccttagcccgatccgggttcgtcttcgcggcaatgaagctaccgctgatagtgctgacgtgtcgatgtggggcgctcaatttgaggccgaccctgtgctcggtgcgtatcaacgcatcgacacggccacggactacgactggctcggctggccgctgtatctgcgcaccgatggcacagatgacggcatggctactggcggcgcaggaggtacggtcaacttcgatctgtcgggaactgacaaggtcagcgtgttcgctggtgtccacaaggcgagtgatgctgttgccggcgtgatcgccgaactcagcgcgtctgaagcgtcgaacgcaggaacgttcttgcttcaagctccggcagacacgaccaccgcaaactaccgcttcgacgtggcaggagacgcaccgcccggcaccggataccgggcaactacattcaccgcacctatctcgaatgtgctgagcatgtattgcgacatcgcgggcgccaaccggacctcggaaatcttcccgcggatcaatggcgccctgcctaccctggccgctgcgggcaacagcacggctggtgcaggcaacttcggcagctatccgctgtacgtcggcagccgcgccggcacgtcactgcgcttcaacggccgcctctacagtctgatggtcatcggtcgcgcgctcacccccgacgagttgttcgtgtccgagcgctatgtgggccaaaaaatggggatcgcgctatgagctacgtccatcgctgcatgatcgtgccggccgcgcaggcgcccctggccagagagcttgtcgtcacgctggcaggcgcccccgctgccaacatgttcaccaccggcctctcggcaaccggcgacattcccttcacccactacgtcagcaccgggatgatcgaggagcagttcgccgctgtgctcgcagatcccgcgctgatggcgatgctgtgcaacagcgtgggccgggccatcaccgagcccgagtgcaccgcgctgctgaccgcctgcgacgtcagcaccgaagagccgcatgtggccttggcgcgcatcgggctcaagatgctgttcgtcgagcagctgcaagagctccaagcgcaacgcgatgcggccgccgcccaggaggcgcagcatggtgctacctgacctccgcaactgggcgctgctggcgctgtcggtgctcgtagtggcgctgggcctatcgacctggcagtacaagcgcatgtatgccgccaccgatttcgcgctggccgtccaaaacaacgccatcaaggcgcagaacaaagtcgctgagcagctgctcgccaagcgcaccatcgagcgcgatgcgctgcagaagaaactggaggaacgcgccgcggcgcaggggaagaccgatgaaaaagctgtggctcagattggcgctgacgacaagcagcagcgtgctgctcctgtgcgcgtccgggtgcacgactgcacccgtgatgccgggagtggtggtggacgcgccccaggtgaagccgccgctgccgccggagctggtgcagaagacaccggcgcggccagtggggtactttcgaaagaaggtgctcgacgccttgcagacgccctgaccgaggttgagacgatgagcgcggcgtatgcgtcgtgccgggcagaattgattgcacagtaagtgaggtattcgaagctacccggcagcggcagcctcgaatatctctaccgctgggaacagcagatcccaaagaccctgatcgagagccaccctatccaggaactcttccatgccttttcgggtgcagacgtgaagatggcttatttggtaagaaattcctcctgcacgccaataatcgcggccgacaaataacgtcgtgtgcgtgcattgcaccggatctcccatcaatagtccgtcgctggagtagtcggctgtccagagggtgccatctgcgacgacaagaaagggaaggacgaccgtgctaaatgtgccctcgctcgcttcctcatagtacgcagcgtcctgaaccaggcttgctgctgagccgagcgcttgcgtccatttttcgtagacctcggagtctccagcggtgaagtcgcccttttcggtcatgcctacttgagaagtcgacttgccgaccatcgctccaatcgggtacatgccgtccgtctgccttagcgtcaatgttttggaaggcggcccaatttctctgaagggaaaatcagcactacgggtgtatgaccaaatgacctggtggtagctctcctcgtcgatcctgggaatttgagataggacaagtggataggcgctctttaggctcttgcattcgattgccagatcaatgcgacattcgttttgtatggcgaatgccctcacgtcgtattgtcgcgacttgctggttaccgaatcttcgtaggtgccaccgtgggtcgctggcaatccgagcgcccgtgctttggcgtagatggccaactccaatccgaaatcgtcttggctctccaagtacttgcgcaaatcggctgcgctcatagggtcttcgcgatatttcgccatgaatgctccgtcctctttctgctattggacaacatttgagcgccccccactggggtttcgcgaccaccgccgtcgcgcgaagaatgccgtctcagtactctgagaggcctccatgaccgacaccccgcaaggcagcgcagccgccatgctggcgcgcacgaagcgcaccgagatccagcacttcgccgacggcggctcggtgcggtgcaccaccgttcgacacttcgccaagccgagtggggcggccgcgaagatggcgcaaatgccgccttcgcacgccagcgccgaatcgatcgagcacggcggcgaggtccgcgggcccggcggtcccacctccgactcggtgccgctctggggctccgccggcgagttcatgctgccggccgacaccaccgcagcgatcggcaaggaaaagctcgaggcgctggtcgaagccacgcacaagccgacgaacaagtccgccgagaagatgggccgcctggcgcgtgccgacggcggcgtgatcgacgatccaggagccgtcatccgcgtgggcaatgcgtactctggcggcaatgtcagcggcccgatctcggtgaacgggcaggccccgggcggtaccgtgagcgttgccgatgcgttccgcgcgccgcccccgccggcgaagccaccagtcctcggcgcgcccgccgcgcaaatgccggtgttcgcgaagcctgcagctccaactgcggtgccagcggctgcagccgttccaacgccggcagcagcacccactgcagcggcaccggcaccgctcgactacgcgaatcgcaacgctggcttcaatgccgcggccgacgcgcgcacagccctttcctcgcagaacttcggcacccggcgcccggctgcagccgctccccccgctgcagcgcctcccgcacccgctgcggcacccgtgaagcccctcgagccggttcagtccgtggtgggctatgccgatggcggagagatcgaagacccccgcaagccggtgccgaccttcgcttctcccgatgcagcggcacaggccctcgctggcatggccggcaacgcacgagacgatatgcagcgtgccgcggcggttcagtttgcatccctctcgcccaaggctgccgcagcttcgtcggccccagcgtcctacgtggcggagatcccgcgcggccgctatgaatcggcggcgccgtggccggagcctgcgacgaccggcccagcaccggctgctgcacccgcggccgctcccgcagcaccactgaccccagcgccggcaccggccgctgtgcaggctcccgcaccagctcagatgcagctggcagccatgccggctgccgcgcccgagcgcgctaatccgctgggcagcctggccgacacgaacgcgcagctggccaatctgcaggcctcgaacgctgcggtgccccaaggtggctccccgatcatcgacagcgctgcgaccgaagccgatcggcgggcccagttcaacgagcaggcgaacctcggcaatgcactcgcgcgcacctcgtggtcgccgcgccgcggcacccaggcgaacgaggctgcggtggctgccgcgatggcgcctatcgatgcccgtgcacgcatggcgcaggtcgctgcgaaggaggccggcgacacccagcgcgccagcattcaggagcgcggcgccgatgcgcgcgccaggctggcggacacccgcgcccagcaagccctcggcgttgatcagcagcgcctggccctcgacagcaagaaggtcacgctggacgcgaaccgcgatgaccgtgccgcggcttccgccgaggtcgagcaggcgcagaaagcgcgcacggccaagctgcaggacctggtgctcaatggcacgccggcgcagcagaagatggcgacaggacagctggcggcgctgcaagggcgcgaggtcagcggcaatgcgccaccggcgaactatcgctggtctgccgatggaacccgcgcggaacccatcccgggaggcccggcagatccagggattaaggcgaacaaggcgctgaccgaagatcaggcgaaatccgctggctatgcgatccgcatggaggacgcgctgaagaccatcagcgaggtggcgaagaccaacccgggcgccacgcggccaggtgtcggcactgcagcgatcaacatgctgccggagggcatcgccaatgcgcttcgccccgaagaccgccagcgcgtcgaagccgcgcagctcgatgcgctcgatgcagcgctcactctggcgacgggcgcggcctacaccaaggagcagttgcacgggctgagccgctcgtatttcgcgcagccaaacgacggcgacaccaccgtcgcggagaaacaggcgcgcctcaacaagatcatcgagaccgcccgcctgagagctgggcccaccggctccgcaatggcagaccagatcgctcgcaccagcggcacgcggactgcgcagccggccgccgtcgcgagcccagccgatcacgccaatctgcccgcaggcgccacctacatcgcgccggacggcagcacgcggaggaagcagtaatggccgagttctgggagagcgacgaaatcatcgcgccggcacccgcggcagcgccggcagcgcccgccgctgccagcgtcgccgtgccggcaccagctgctgctgccacgtcggcgccggccgctgccgcggattcgttctgggcaaaggacgagatcgtttcgcctgctcctgtgccggccgctgcggtgccgaacgtgccggcgcccgagcccggcaagcccgagcggtcggtgctgggcgagatcggccaccaggtgggtctgacggcacgtgcggcggtgcagggggcagccgcgctgccaggcgtggtttccgatgccatcacgggcccgatcaatgcgggcttggacactgtcgcaggggagggcaacggcttccgcttccagaagctctccagcgcgctcggcaacatcatggaccagacgggcgtggccaagccggagaacgccaccgagcgcgtcgtgcaggatgcagccacgggcgccgccaccgcgctgactggcgtgggggcagggcaggtcgtcgccaaggcggcggggccaatcaccaaagccgtgggcaatgcgctggcggccgctccgaccgcacaggccgtcagcggcgcaacgggcggcggtgccgcgggcgtcacgcgcgaaagcggcggcggtgcggtggcgcagaccgtggccggccttgctggcgcgctggcgccgacggccgtgccctatgcagcgcaggcgggcgtgcgcggtgcgctgcgaggcggtgaagccactcgccagcgcatggtcgacaacatcgccacctttgaggaagccgcgggcaccacgcctacgctcggccaggccacgcagagccgcgcggcccagggcgccgagaccggcctgtccaacgtcatcggcggatccggcgtcatgatccgcaagggagagcagcaggccaaggccttgcaggacagcgtgcagaagatcaccgagtcgctctcgcccaacgccagcggcgtggacgccggcgaggccatctcgcgcggcgtgaacaccttccgcgacaacgtgcgggccacgcagcagcgcctgtacaacgcgctcgacaagcacatcgcgcccgatgcgcccatcacggtgagcaacacgcgcaccgccatgcaggaactcaatgcggggatcgacggcgccgagaacctgtcagcgtggtttcgcaatgcgcggctcaacgacctcgaaaagtcgctggtggcggaccttgagaaggccgcagctgcgcaggcgcaggccggcgcgcgcagcgggctgacgaacgcgcaaggccccaatctcaacaccgccgcgctgccctacgagagcatcaagaagatgcgcacgctggtcgggcgcgaaatgtcggatgcgaacttcacgtccgagatcaaccgcgacaagtggtccaagctctatgccgcgctgagcgaagacctcggcgccacggcgaaggcggccggcccgcaggccgagcaagcatggtcgcgtgcgaacaccttcacgcggctggccagcgagcgcatggagcagatctcgtccatcgtgaaccgcgacgcgcccgagaagatcttcaaagccgcgaccaccgggctcgccgatggcggcacccagatcaaccggctgatgaagagcatgcccgtggagaaccgccgagaggtcgccgcagccgtgctgcagcgcctcggccgcgcacgcccgggccagcagaacgagatcggcgatgcgttctccagcgagaccttcctgaccaacctggccaacctgtcggcgccggcgcgcaaggcgctgttcaacacgtcgggcttcccagggctggagcagcgcattgcgcaaatggggcgcatggcttcggttcgccgcgaaggctctcaggttttcgcgaacccgagtggcaccgcacgccaagcgggcctgttcgggtgggtcgccgcgctgggcagcgcgattgccacaggaaacgccgctggtattgctggtgccatcgccgtgccggtgggcgcgaaactcgcggcaaaggtggccacaagcccgcaggtggttcgcttcgcagctggcaagtctgaagttcctcaaggactcgcagcctcaaccatcgcagctgcctcgcgaactgctcaaccgacggacaacggcaagggagcgatcatggacggcggcaagcccttccagaaccgcctcaaggctggccgcgtcgcgcgagagcagggcggtaccgtcatgccggcgcccaacggcggcttcgtggtgctgcgaggtgccgcgcgatgagcaatgtcgacagcggtgcgcacgaggccgccacctcgccgctcagcgcgctgccccttcccaccgatgcacagatcgccgcgggcaacttccagatgggacacgtgaccatcgcgggcctcgacgtcaccatcgaatggccccagggctcgacgcgcaagggcgtcagcaaggacggtaggccgtggcaacgccagatgagcgcgcactacggctatgtgctgcgcaccgaaggcgcagacggcgagcacgtcgacgtctacatcggcccgcaccatcgctcgctgcgcgccttcatcgtcgatcaggtggatgcgaaagggcgctttgacgaacacaaactgctgctgggttttgcgagccgcgaggaggccaaggccgcctatgcgaaacacttcccgcagggtttccgggtcggaccggtgaaagagatggcgctgccccgcttgcgcgaatggctgaagagcggagacctgaagcagccgatcaatcggctcgtgcccacggatcagcgaaagaggctgtagacgaagaggcccaggcctccaaggatgagcacggccgctccgagcagagcggcaattacttgcaccgatatcttggtgtcttcccagaaccggagtcggtgctcctcagccttgagcaggagtctgaagtcctcgccggtgaagttcttggggtccttggccatgtgcggaatgtatcagggcgcgaggccagccgctaatcctcgtcgggaggtgtcaggtggagcgtctccaatgaagcagtatgtcgcttgcggaaaggcttcacgaccgagcggaaggtgaagtacgccgccgctatcgaaagcagccatacaagcagcacagagtccttgtagtgaatctggccaaagagcaagccggccatcaacacggccaccgccattgctcccccagcgagttccgcggcttcagctttcgccgcctccaggcgctcgtgaatgcaggcccattcgtacttagaaattgccacagtgctcctttggtcgcggccatcgcgaaatgtagccgaccaatggaaaaagggccggtgagatcgctcccgccggccccgttcagctgctatgcagctcaggcgacagcaaactccagccgcttcccaagcgcgtgcagcgcttgctgcacggtgtcgaccttcgtcacgtggtgaaggtcggtgagccggttcacttcctgggcggtcgtgttcagcttgcgcgcgagttctgcgggacgcaccttctgccggatcatctcgttgagcagcagcaccttcgcgcacaggctggccggcagctcgatcgcttccttgcccttcggcaccttgcgcggggctggaacctcgcgcttatcttcgaagtagaactcgagcgcggtgaccagtgcatcgcgcgccatatcgagcgcttcctcgcgcgttgcaccgcccgtcaacgcctccgggatatcggggaacgaggccataaagccgtccccatctttctcaatttcaaccaagtaacgcatacgagactcctttctaggtagccgcggaaaatctttgaagctgcgagagacccctttcggggcctctctcacaaacctagctgtttcagaatcgctttccggagaccttcgccaatttcgtggctcggatgccggggcatcactgtttgctttccgttgagcctgaccttcaagtggcgcttgccattctcgaaggtggcccctaggtcagcgagctgtctcttgaactcgctttgcttcatcgaccctccatgttttgaacatgggtgattataaacaaaattgttgaatacttgcaagtgtttctaaacaaaaatgttgagaaatcagagggttcgattgcaggttcaatgggaagcttcgcgctgcgccttgcgccagtcccatggcgccacgggctcttcatcgcgccacagcccgacgtgcttggccttggcctcggcttcggcgaattcgtactgcccgcgctcttcggcactctgctcgcgcgcataggcgcgataccaccaggccatgccgaccgtgaccatggccagacccgcgtcgagcgtcttgggcccgcgtggcgcggaggcgggcgccaccatcaccttgcagacgctgcggccgtagcggtcgaccttcgggcagtcgagcgcggcttctttcatgtagaccagatcggacagcgcctccttagcgcgctggccgaacggctggcgcttctcgggcgcatcgatgccgttgaagcgcaccttgatctgttcgtagtcacccgcggtgccgcagcgcgcggtgagggtgtcgccgtcgctgacacccaccaccaggcacgtgcggggctcggcggcctgggccagcaccggcagtgcgagcaaaccggccagaagaagagggtggagcgccttcactgcagcgagacctcggtgccgtcggcattgaccatcacgccgggcgtgctctcggcgatctcgatcggcacgcccatgtgcacgctgccgtcgatgttgggaccgccgatgcccgtgcggcgggtctccacgtattccctgtgctgggccggcgtgaggatgaacttttgagggtaggcgttgccgtttgcgcgccagtgcttgatcagcgcgtcggtcatcggtagatacagagttgccatcgtcgcgactcaggcggtggcgcgctcgcgcaggatctcgacggggccgatgccgctatagatcgtcgcgtcggtcttcaggcaggtgatggtccagcggtcgccgggcgtcaccttgtagtcgccgggcgccagcggcagctcgcggtcttcgtgcacctggctacccagccatgacggcacgcggaggatggtggcgggctcgataaaaaattcagattggctcatgctgagattgtcgggcgaggctccgctcaaattggccgcacgtcgaagaaggcttgacaccctgaatgccccacgtgtcggtatgttaaaagttcgcatttctgcgattgcctctactattgccttatcggttatctgcaaaacggcctctaggccagcagcctgcgaggaggaacgatgaagcagcagaaatctcctttcgatgtgctcggcacgcatccatatccgcaagaacagtggcgatgtgcctttgtggcggagtgggcgcgactggcggaaggatgcgccgatgcggctcaaacggccgaagccgccgcggagctttatgcccggtacggcgcgcgaaacccgactgaagttgcccgcgaagagtggggcggcccgacatagttaccccgtcggtgccccagggcgctgcggtgccccttttgcaggcacaacgtcgcggcgcaggcaggacaacgctctctggcgatgcgcacatgcttatccaccgtcttatccaccgcaatggtgcagaactcgccctctgtgattgatccattctggggcggcatcgagcaaagttgcacacaattggtaatacctgtcagcgacaactggcaggcagccggaaagacatcgagattccagcgggctcgctcacgctactccatctctcggcgctctaccggtacgcatagccaagcctgtcggaactccctgaccagcaactggccgtctatggtctcggcttcgatctcagtgccggcaaacagcacgcccagccctttgtacggcacgatcacggggtcaatcatccgcccgcgacccgacatcctggcggttccgtaagcttcatacaaactggcctcgaccgtgttgcgccctacgttgttgtggtcgcggtcggattcgagaacggtcaccatgaggcggcgcggcgcatcgcgctcgcctttgcgaaggcgcaggccttgacgcctcaacagggtgacttcagcgaaaaacatactgtacaaatatacagcattcgtactaccatgcgcgcatggaaaacgtgcccgcaacccggcggattgccgcctgtgtgccccgaattcgaagctggccgagtcacaaacaacaaagccttcaggctttgggcactgcaggctttgaggggtcttctcggcgggcttggatggtcggctagcaccgcgctgtcgtgcgtcgcagtcgagaaaacctaccgatcctgttgggacacggtggtccgatcttcgtccaactctggaagcccgaacagcgtcgcggggtagcctagagccgcactggtcgagaaaaaatgctgctacaaatgcaacaaatcagaagacggctccagcaccgaatgcgaaaggtgaagaagccctagctttcgccatcgctcgaaagttgaaacttgagcgtggcgaacgcaatctgggccgcctcccgcggcgcacagttggcactcagcgggaagagcgctgcaaaaagtttctccacccattcgcgatcgaccgcgccgttgcaacgatcgcacaactcgctgatgaactcgtgacgccaagcttcggcaggaggcaacgtcatgtcggcgaccgtgatcggcttgtcgggtttccacatgtgagaaatgctactccagcgctggagcggtatcaatcggcagaagagctattcggcccgcgcaggtttgcctgagtgggctttttatcgcttctccggccaggccatcaacttgcctgcggccgtcaggcggtagtcgaagcgccgcttgggatcaacgacgatctgatgggtgataacgtcgaatgcttcgatcagaccgttttccagaagcacccgcagctccgcatcggggacgcccctccaagcacccgcgtcgatctgcaacaaacgacctcgcaccaaggcatcgttttccaacatgtgcttctcctcgtgatagatcggcttattctggcccctatacggtgcagttcagagggtagaccgtcggccttgcgcgggccctttcaatgaaaccctatttcattgacctggtgctttgtgcacagatgcaggaactgggctaccgcagtggggcccgagatgggtactcatgaggtagttccattgccacggggcggggcgtatgcttttgcaatcatgaccatggccgacgtgtcgatggattttgatctgccggagggctggagctgctcggttgagctcgaacgcgccgttgacggggtctacgccggacgagccgagttgcgactcgaatccacttggcgctgcgtgctggtggtgacccagcagccgagccgagaagcggcattggagtgcatgaagtaccgtgccgttcgcttcatcgaggaatggagcacgagagcaggtcaagccgcagagcgaaggctggcacaccccgcgtgatccgaaggtcacatcaatcgcaaccctccggcgaatcgcatcgaagtcttcgcgaacctgggcgcgtcgcccatcttggcaatctctgcgaggccctcgtcggtgatgccctccaccgtcgccatcgaagccttggcgtacagcccggccggctgaagcgctgaaattttggcctcgatcaaccccgtggccatgagcacggacacatctcttatttcctctggttcaacgacctgtaccggtagttgggtgcgcagaagcctcatcaagaacaagagcggcattcgatcctccggtcgccggcgctagctgtgcccaaaaatgccggctcttttgggctaaaaaatgtagtgttaagtacgatatttcgcatagggagtcaaatattcccttgggagtgacaacaaatgcacaaaattggccgtccgctttctcagggggcgctcaatccagaaccgccgcgcagaccaacccaaaaaagctcaagcgtcggccactgccgagcattcatgccctttgcgaaacgctcgacaagcggaggcctcacggcaagaatcgtccgatgtgcacccgctacatcagccccgaagagcgtgagatggaagctttctggaagatcgaccggaagtccaaccagcgcaaggactgggagaacctgctcacggtgtttccgctgtcgctggccagcttcattcggcgggtcgacgaggtggaattcgcacgcgaactcgtagtcgggcagtggggaatgattccgccgtggtcgaagacccatgtgccgacaaccgcacggggcacgcgcttgagcacggtcaacgcgcgcaccgagggcatggagaaatcgccgacgtacaaggatgcctgggcccgcggcaagcgctgcatcatcccggccgccagcttcgacgagccgaactgggagaccggcaagaacgtgtggtggcgcttccggcgcggggacggtgcgccttggggcttggccgggctctggaacacctggaccgacaaggaaaccggcgcggtctgggacaactacacgatgctgacgctgaacgccgacggccacgcactgatggggcgcatgcacaagccggatccgaagttgccccccgaccagcaggacaagcgcagcctcatcccactcgaggcgcacgacttcgaccgttggctgacctgcactgtcgaggaggcgaaaacgatgctgaaggtgccaccggtcgagctgttcgaagcggggccgctcgtcgccgcgtgagcgcatcccgttagacaagtgccgcaccgttagacacgcggcccagaaacgaaaatgcggacagccacctaagtgactgtccgcattacgattttttggtcggggcgaaaggattcgaaccttcgaccctctggtcccaaaccagatgcgctaccaggctgcgctacaccccgacaagccttctattctagcccggatatcgggcctctcagcgtttctcgtattgagtcctgccgaaaaggatctcgcgctccttgtcgccggtgatcggctggcgcaggtcggccagcactttcacgccgcgctgcacggcggggcgcgcggcgatggcgtcgaaccaggccttcaggtgcagatagtcggtgagggtgatgccctggttttcccagctgcgcagccatgggaagatggcgatgtcggcaatcgaataggtcttgccggcgatgaacttgttcttcgacagctgcttgtcgatcacgccatagaggcgcctggcctcgttgctgtagcgctcgatcgcgtagccgatcttctcgggggcatacatgcgaaagtgatgcgcttgaccgagcatggggccgacgccgcccatctggaacatgagccactgcaggacgtcgtagcgctcgcgatcggtcttgggtagcagcttgccggtcttgcctgccaggtacaccaggatggcgcccgattcgaaaagcgagatcggcttgccgtccggaccgtcggggtcggtgatggccggaatcttgttgttggggctgatctgcaggaagtcgggagcgaactggtcacccttgccgatgttgatcggccgggcgttgtacggcaggccgcactcctccagcatgatgtgaatcttgtggccgttgggcgtgggccatgaatagacctcgatgggcgatgcgggcatgtcgcggggctccaatgtggtgggggtgggaattcgagggaggcagcatatacgcggccattcaaacgcgcgcagcgccgggcattcgccgctcaggcaacaagcggcgcgcctcccgtcaggccacggccgagctggatgaaagatgctggtggatcagcgccaccacggcagcgccttcgccgatggctccacccacgcgcttgaccgagcccgagcgcacgtcacccacggcaaacacaccctgcacgctggattcgagcgccgcggcggcgcgtgccggaaagccgctgctcgccgcgccgcccgtcagcacgaagccgtgcttgtcgaccgagacaccgcagccttcgagccagctggtctcgggctcggccccgacgaaaagaaagatgttgcgcgccgcgcagtcgtgctcgttgcccgtggcctggcagcgccaggtcgcacccatgaggccttgctcggaaccgccgttcagcttcaccagctgggtgtgtggatgcagttcgatgttgggcgtggcctcgatgcgatcgatcaggtagcgcgacatgctggccgcgagagaggggccgcgcaccagcacgttgaccttggccgcatggtgcgacaggaacaccgccgcctggcccgccgagttgccgccgccgaccagcgcaacttcttgctgcgagcagagcttggcttcgatggccgacgcccagtaccagatgccgcgcccctcgaattcggcgagcctcggcacgtcgggccggcggtagcgtgcgccgctggcaatcaccaccgtgcgtgcgttgatggtgcggccgtcggcaagggcgatgcgcaggctgccgatggggttgttgcgcgtgcagtccagcgacttgaccttggccgggatcagcatctccacgccgaacttctgcgcctgcacgaaggcccggccggccagcgcctgccccgagataccggtgggaaagcccaggtagttctcgatgcgcgcgctcgcgccggcctggccgccaaaggcgcggcagtcgagcacgatcacgcgcaggccctcggaggccgcatacaccgcggtcgccagcccggccgggccggcgccgaccacggccacgtcgaacagctcgttgcgctccgccgtgtcgaccatgcccaggcagcgcgccagcgcatcttcggccgggttgaccagcaccgagccgtcgggacacacggccagcagcttgcaggtgccgtactgttgcagcagtgccgcggcatccgggtcttccgccgcatcgaccaggtgataggggtgcccgttgcgacgaagaaagttctccagccgggccatgtcgggtgactgcggctggccgatcagcaccggcccgctggcgccggattcgatcagcgccacgcgccgaaggatcagcgcccgggtgatgcgctcgcccagatcggcctccgccacgagaagcgcgcgcaactgcgcgggcggcacgatcagcgcttcgacttcttcttcggcatggccgtcgaccagggcagggcggccgctcagctggcccacttcggcaagaaattcgcccgggccctggcgcacgatgggcaccacgtgccccaggccgtcgcgttgcgtgaccgccaccacgcccttgagcagaacgaacatgcccgggctcgtttccccggcggtaaacaggcgctctccgcatgcaaagcgctgcaccgttccgaagtgcgcaatgcgcgcgatttcggtgtcgctgagaacgggaaaggtctggtggagacggttgtccaaattgctgtttgcggctgtggccatttgcagaagctccttgtcgcggacccatcgcattagacaaccaagcggcccttcctgcggcccgaacacgctgtaaccgccgtcatgcaaatgcaatgccactgacatgcccgtttcaccgcaggtgctgagactccatcggcagaaagggttccccatgaaagaactgcccaacccgacatttccgctgtcgcagatcggactgcgcgccgccctgtggccggcccccgcagctgcgcgcccaacgctgcccgaggcgccagctgccgtgctggtgccgccggtcgtcgatgccaggcaaggcatcaccgtgagctgggcgcgccacctggacgaggtgcgcgccgcgcagcgcctgcgctaccaggtgttcgtcggcgaaatgggggcgcgcgtgagcacgccgctggcgggccacgacatcgacctgttcgacgacttctgcgaacacctgctggtgcgcgaagaactgacgcagcaagtgatcggtacctaccgcgtgctcacgccggcccaggcccggcgcgtgggcagcacctacagcgacaccgagttcgacctgacccgcctgcgagacctgcgcgagcgcatggtcgagctgggccgcagctgcgtgcatccggaccatcgccagggcggcgtgatcctcgcgctgtggggtgccctggccgggttcatgcatcgcaacaagctcgacaccatgatcggctgcgcgagcatccccatgtcgcacaacggcgtgaccagcggcgatgcggcggccagcatctggcgccagctgtcggccagccacatggcgccgatccagtaccaggtgcagccgcgcctgccgctgccggtcgaaaggctcgacggcgcgctcgacgtcgagccgcccgcgctcatcaagggttacctgcgcctgggcgccaaggtgctgggtgcgccggcctgggacccggacttcaacaccgcggacctgccgatgctgatgcgcatcgacgacctgccgtcgcgctaccgcaagcactttctgggcgcatgaaaccggcggttgcccggcccgctgccaggccatccgcctcgtcgcccagcgcgggggagccgggcgcggaggagtcggcgtcacaggatcgtcacggaaacgtcacaaacgagggcgacactgtcatatttcagcctacgtgtgctcccgtgccccttgctccagaatcagtgcccatgcaatctgctcccgctgaccggacgctcacggtcgcggcatcggcgcttccgctgctcgaccgcgatcacagcatcctgtctttcaatgagcgcgtgctcgactgggcccatcggcccgaggtcccgctgatcgagcggcttcggtacctgtgcatcgtttcttccaatctcgacgagttcttcgaagtgcgtgcggcgccgcacctgattgccagcagcgccggagaccagaagggcagctacacgatcgagtcgttcgagcgcctggccgaggcggcccacacgctggtggcgcgccagtacgcgctctacaacgacgagctgatgccgacctttgcaaagcacggcatccacatcatttcgcacggcgaacggaatgcggcccagcgcaaatgggtcagcgaatatttcgagcgcgaagtgcgcccgctgctgattcccgttggcctggatccggcgcacccgtttccgcaggtggccaacaagtcgctcaatttcattgtgcgactcggtggtaaggacgccttcgggcgcgaaaacccgatccagatcgtcaaggtgccgcgtgtgctgccgcgcgtgatccgcatgccggccaaggtgtccgacggcaagacgctgttcgtggcgctttcgagcgtggtgcgcgcgcacctctcgagcatgttcccgggccgcgaagtgggcgacttctctcagttccgcgtcacccggcactccgaccttgcagtggacgaggaagacgtcaagaacctgcgcacggccctgcgccaggggctgcagcatcggcactacggacaggccgttcggctcgaggtgtctgccagctgcgccgaatcgctcgcgagttttctgctggcgcagttcaacctgcccgcagaagcgctttaccgcgtgcatggcccggtcaacctggcccggctgacccaactgatcgatctgctggaggagccgcagttgctctttccgccgtactccgcctcgtatcccgtcacgctgtctcctgtgcagtcgttcttcgagcggctgcagcgcggcgacgtgctgatccaccagcccttcgagagcttcgacggcgtgctcgctttcttgcgcgaagcggtgctagacccgcaggtgctggccatcaagcagaccatctaccgcacgggcaccgactcggagctgatggacctgctgcgcgaagccgtgcgccgcggcaaggaagtgacggtggtggtggagctcaaggcgcgcttcgacgaagaggccaacatcaactgggctgaaatgctcgagtcgatcggcgcgcaagtggtgtatggcgtggtcggcctgaagacgcacgccaagatgctgctggtgacgcgccgcgaaggcaagcagatgcgccgctacggccatctctccaccggcaactacaacccgcgcaccgccaggctctacacggacatcagccacctgacggccgacccgctgctgacggccgacatggaagcggtgttcgtgcaccttgccagccagagccggctgcccaagctcaaccgcatgtggctggcgccgttcgatctgcacaagaacctcgtctcgcagatcgatgcgctgggcctggccgcttccaccggcgagcccacgcgcatcgtggccaagatgaatgcgctgaccgacgagcaactggtcgccgcgctcatgcgtgcgggccagagcggcgtgaagatcgacctcatcgtgcgcggcgcctgcaccttgccggcgcaggtgccggggttgaccgacaacatccgcgtgcgttcggtgatcggacgttttctcgagcactcgcgggtcttctattttcggagcggggaggaagagtcgctctacctctcgagcgccgactggatgaaccgcaacatgatgcggcgcatcgaactggcctggccggtgaccgaccccggcctgcgccagcggctgatcgacgaatgcctggtggcctacctgcacgacggccgcgatgcctgggacctgggaggcgacgggatctacacgcgcgtcgaccacgacacccaccgcggcgaggcgggagagtcgcccatcgtcgaagcgcacggcgcacaagccgcactgatgaaccgatatgcatcgcgaggccatcaccccgatgcatccagcaactgacgatcgaaagacgacgagcatggacttgatcttctggcgccatgccgaagccgaggactggaccgagggctgcgacgacctgcagcgttccctgaccgcgcgtggcgaaaagcaggccaagcgcatggccagctggctcgaccggcaactgcccgacggcacacgcatcatctgcagccccgcgcggcgctgcgagcagaccgtgctcgcgctcggccgcaaatacaagctgcgctccgaactcgcgccagacaccacgccagaggccatgctgggcgcggccggctggccgaatggcaagtcggtggtgctgatggtcggtcaccagccatcggtggggcaggccatttcgctgcttcttggcttgaagcaggacagctgcccggttcgcaagggttccctctggtggatccgaacccgcgaacgcgacggcgacgtgcagaccgtggtagtcacggtgcagtcgcccgagcttctctagctgctggagccgccttcagggcggttttccataccggcgctccaagacaggcgctttgtcatggcggggggcagaggtggcggggcgcttgtctcccgggaaaaggtgcgcaccgctcatgtgcgcatgcggtgcaatttctacagtgactccacggcaaaaacgccctgacccgatgacgggaaagaagcggtgccggtcggccacctcactggggaacacgcatgaaactgctccacccgctatcaagaagcttcatgagcatgctgcgcgaagacgccagcatgtcattgaaaacgctgactcctctgcttgttgccgcagccctcctgtcggggtgcgcgacgaacaccgcccagcctgcgctgcaggcccgccacgaagccacccgggcgatcgagaaggtcgagctcatctacaacgtggaggaccagctgatcgtcacggacggcggcgggtccgggctgacgggcttcgcggggctcctggggcccattggcgcgatattggccctcaccatcgataccaacagccgaatgacgatggccgaccggaccgaccggcgcagcaaggagttcacggccgccgtaaggaacagcggagcggccatggcactcaacaggaagttcgctgaacggctggcggcgcgcctgcgggaaagcggccgcgaggtgaaggtgacgcctttcatgcgcgcgaccggacagctcgccgagatgcaggtgcccgaactccggcccactccgggctacagcacgttgatcctgcggatcaccacggcgtatggggcctccgatgcgacatcgagcttcaagccgttcgttctggtggagcagttgctccggaacgagcagcagtccgtcgttcaccagacatccagcttcgccgacgtgaccgagccgacctattttctgtatgagggcctgctcaaggacaccgcaggtgcccatgaagggctgaagcagggtctcgaccgggtcgtgcagccggcctatgcaggcatgttcggggatgacgagccgcgcacggcccgctcggccaacacccagaccgctgccctcggtgcgaattgacgcgccccgcgcccgctgaatgccacccgtctcagctgcgccgcagtgcggtgccagtggcatacttgccggcgagtgatgcatttggtcacaaatttcatatataacttacaaacccacagcgattgcgcagcaggcgccttccaagtacccatgaaaacgtttcttcctctgttcgttgccgcggccctcctggcggggtgtgcgacgaatgcaccgcaggccgcacgccccgataccacccggtcgcttgccaagatcgaactcttctacaacgaggaagaccagttcactgtcgtggatggcggcggttccgccatagtgggcttcgccgggcttctggggccggtcggcacgctggtggcgctcggtttcgaagtcggcagccgggcgaccctggctggccggacggagcggcgcagcaaggagttcatggcggcagtcaagagcgacggcacggcggccacgtctcccaccctcagccggcagttcgcggaacaattcgcagcgcgcctgcgggagagcggccgcgaggtgaagctgacgcccgccttccgcgtcaacgggccactcgccgagatgcaggcactgggacatcggcccacgcccggctacagcacgttgacgatgcggatcaccgcggcgtacggcgcacccgatgccacgtcgagtttcaagccgttcgtcgcggtcgagcaattgctgagaaacgagcagcaggccgtcgtgtaccactcgacccacaccgccgacctggaggagcctgcctacttcatgtatgacggcctgctccaggacgtcaaaggggcccgggaagggctgaggcagggcttcgcccaggctgtgcggcccgcctattccgtcatgttcggcgaagacgagccgcacctggccggcgctgccgagcccacgcggacggccggcctcgacgcagcctcggcgcaacgtgaagtgaagtgaagtgaagcgcctcagcagccgctgagttccacgcgccagctgctggtcttctgccaggccagcacctcttcccgcagcaggtgcgcggactgcggataggcgtcggcccagtcgggcgcgcaagcgatcgtgaaagccctggcacccagcgccgcgagatgcagcgcctgcgggtcgggatcgcggcgcgcgtggcacaggatcaccgcaaggcgcagcgacagcagctgcatcacgaaggtctcgtcttccagcgcgacgtcgagcttgcgcagctttccgcgctgccccagcaccagctggccgagcgcatgcaactcgttgacggcaaagccgggcgcgtcggtgttgtcgaggatgtaggcgccgtgcttgtgatagtcgctgtgggaaaccagcgtgccgatctcgtgcagctgggccgcccagccgagcttgcgcagcgcgcggccggcgcggcttccggcgctgccgccacgcgcggcaggtgcgagctgcacgaacaatcccgcggccgtttcgcccacccgcctggcctgggccgtatcgaccgagaaccgggtggccagccgcgccacggtggcggtgcgcatgtcggccacgctttcgtcgcgctccagcaattcgtagagcacgccgtggcgcagcgcgccctgggccaccttcatttcgtcgatgtcgagcagttcgaacaccgcgcgcagcacgctcacgccgccgccgatcaccggcttgcggtcttcgcgcatgccgtcgatgcgcagcttgtcggtgctgccggccttgagcaggcggtcgaccagccagttgaggccgtcgcgcgtgatcaggcccggctcgccgccggccgctgccagcacgtcgcccaccgcgccgatggtgccggatgcgccataggccacgtcccactggtcgcgggtgtagcttgagagggcgtcgtcgagcaccgccttggcggccacctcggcggcccggaatgcggccggggtgaagaggccttccgcgaagtgcttcatcgaccaggcgacgctgccgacgcggtaggactccatcagctcggcgtccagcgcgcggccgatgatcatttcggtggagcgaccgccgatgtccaccaccagccggcgttcccggtcggaggcgtcggtgtgcggcagcatgtgcgccacgccctggtagatgaggcgggcttcttcccggcctggaatcacgtcgatgccaaagcccaggatggtgcgcgcgcgcaacaggaattcttcgcggttgcgggcctcgcgcaaggtctgggtggccacggcgcgcacctgcgagcgcttgaagccggccagccgctcgccaaaacgggcaagcgcgtcccagccgcgctgcatggcttccggcgtgaggtttcgggcgctgtccaggccgttgccctggcgcaccgtctccttgaggtattcggtgcggtggatctggccgtggtcgacctgtccgatctcgagcctgaagctgttggagccgagatcgactgcggcgaggcgggtgccgttttgcatgtagttgtagtgaagagggcggtgtctctgatcgtagcgccgtgacaggcgcgccactcccggatcgtcggcggcgagggtccagaggctaggcgcgggaaatgacgattgtgtgacagcgtcacacaagccgcaggggaaacggcgccattttccctctatggcggggtgtcacaccgatgtcacacaagcttcctagagtccgttccaagcccgaaaagggactacttcttacttctaatggaagctctatgaaaacgacgctcaaatttgcagccgccggcctcgtggcctcggtcttcgcccatgttcccgcatacgcacaagacgtgaccggcgccggcgccagctttccggcgccgctgtatgccaagtgggcctccgatttcaacaaggccaccggcgtcaagatcaactaccagtcggtcggttcgggcgcgggcttgaagcagatcgaagccaagacggtcgatttcggcgcttccgatgcaccactgaaggacgacgaactccaggccaagggcctgatgcagttccccaccgtcatcggcggcgtgatccccgtggtcaacatcgccggcatcaagccgggtgaactgaagctcaacggccaggtgctgggcgatatctacctgggcaagatcaccaagtggaacgaccccgccatcaaggcgctgaacggctcgctggccctgcctgacgccgccatcgcgccggttcgccgcgccgacggctcgggcaccagcttcctgttcaccaactacctgagcaaggtcaacgccgagtggaagaccaaggtcggcgaaggcacggccgtgaactggcccaccggtgcgggcggcaagggcaatgaaggcgtcgccgctttcgtgaaccgcctgcccaattcgatcggctatgtcgaatacgcctacgtcaagcagaacaagatgacctatgcccagctgcagaacgcagccggcaacttcgtctcgcccgacgacagcgccttcaaggccgccgccgccgccgccgactggaacaagagcttctaccaggtgctgaccaaccaggccgacaagggcgcatggcccatcaccggcgcaaccttcatcctgatgcacaaggtgcaggacaagcccgccaacgcgaccaccgtgctcaagttcttcgactgggcctacaagggtggcgacaagacggccgacgatctcgactacgtgccgatgcccgatgccgtgaaggccaccatcgccaaggcatggggtgaagtgaaggacgcgtcgggcaagccggtcgctttcaagtaagcccatcaactttcaagtcaagaacggcgcatccatgagcagctcttcgctccaggatgcgccgcattcgtcattgccggagcgacccgtgtcatccacttttcctgcttccgcatcctcgctcgacctcgcggccgaacgcggccgcgccaccgccccgccgcccgccaaggcgccgcgctcgggccccatggccgatcgcctgttcggctgggccgccaagggcgccgcgctgctcacgctcgcaatgctgatcggcatcctgctgtcattgatcgccggcgcctggcccgccatctcgaagtacggcctcggctttctcaccagcagcgtgtgggacccggtgcagaacgagtacggcggcctggtcatgatctacggcacgctggccacgtcgatcatcgcgctggtgatcgcggtgccggtgagcttcggcattgcgctgttcctcaccgagctgtcgcccaactggctcaagcgcccgctgggcacggccatcgaattgctcgccgccgtgccttcgatcgtgtacggcatgtggggcctcctggtgttcggcccgatcctgtcgacctgggtgcagcagccgctgcagaagctgcttgccggcgtgccgtacctcggcgcgctggtgtcgggtccgcccgtgggcatcggcattctttcggccggcatcatcctcgcgatcatgatcatcccgttcatcgcctcggtgatgcgcgacgtgttcgaagtgacgccgccgctgctcaaggagtcggcttatggtctgggctccacgacctgggaagtggtctcgaaagtggtgctgccctacaccaaggccggcgtgatcggcggcatcatgctcggcctcggccgggcgctgggtgaaacgatggcggtcactttcgtgatcggcaacatgaaccagctcaattcgctttccgtgttcgaggctgccaacagcatcacctcggcacttgccaacgagtttgccgaagccggcgcgggcctgcaccaggctgcgctgatgtatctcggcctggtgctgttcttcatcaccttcgtcgtgctgacgctctcgaaggtgctgctggcccagatgaagaagagcgaagggacgaagtcgtgagcactgctgaaagcctcttgagcgcgaaggcgctcgccgaaacccgccaggccaagtttgccgcgcgcaaccgcgtcaacaagatcgcgctcacgctgtcgctcgcggcgatggtgttcggcgtgttctggctgatctggatcctgtgggagacactgcgcctcggcctcggcggcctggcgcttgccacgttcaccgagatgacgccgccaccgaacgaggcgggcggcatcgccaacgcgatcttcggctcgttcgtgatggtggggcttgccaccttcgtgggcacgccaatcggcatcatggccggcatctacctggccgaatacaacaccaagggctggctcgcctcggtcacgcgcttcgtcaacgacattctgttgtcggcaccgtcgatcgtgatcggcctgttcgtctacgccgtggtggtggcctatttcaagaccttctcgggtcttgcgggcgcactgtcgctggcgctgatcgtgattccggtggtaattcgcaccaccgagaacatgctgcagctggtgccgccgggcctgcgcgaagcggcctacgccctcggcgcgccgaagtggaaagtgatcctgagcattacgctgcgcgctgcacgtgccggtgtggtcacaggcgtgctgcttgccgtggcgcgcatcgccggcgaaaccgcgccgctgctcttcaccgcgttgaacaaccagttctggaccgccgacgtgagccagccgatggccagcctgccggtgacgatcttcaagttcgcgatgagcccgtacgagaactggcaacagctggcctgggccggtgtgttcctgatcaccgtggccgtgctcgccctcaacatcctggcgcgggtcctcacgcgcaacaaacactgattcaagaaaagcaaccatgccaaataccgtcgcacaaccgtcgcgctcgaagatctcggtcaaggacctgaacttctattacggcaagttccacgcgctcaagggcatcaacctcgagattcccgaaaacaaggtcacggccttcatcggcccgtcgggctgcggcaagtcgaccctgctgcgcaccttcaaccgcatgttcgagctctaccccgagcagcgcgccgagggcaccattgcgctggacggcgagaacctgctcacctccaagcaggacgtggcgctgatccgcgccaaggtcggcatggtgttccagaagcccacgccgttcccgatgtcgatctacgacaacatcgccttcggcgtgaagctgttcgagaatctgagcgcgagcgaaatggacgaccgcgtggagtgggcgctcaagaaggctgctctctggaccgaagtgcgcgacaagctgcagcaaagcggctcaggcctttccggcggccagcagcagcgcctgtgcattgcccgcggcattgccatcaagcccgaagtgctgctgctcgacgaaccttgctccgcactcgacccgatctcgaccgcgaaaatcgaagagttgatcgccgagctcaaaaacgagtacaccgtggtcatcgtgacgcacaacatgcagcaggccgcacgctgcagcgactacaccgcctacatgtacctgggcgacctgatcgagttcggcgcgacggaacagatgttcttcaagccgcagcgcaaggagaccgaggactacatcaccggccgtttcggctgatgccaaggaggcacacatgactgaaaaacatctctccagccagttcgacagcgaactcaacggggtttcgtcgcgcgtgatggagctcggcggcatggtcgaggcgcagatccaccaggcggtgtatgcgctgctgcagttcgaccccgacgcggccgaccgcgtgatggaaaccgagcagcgcgtcaacgcgatggagatcgagatcgaccgcgagctgtcgtcgatcattgcgcggcgccagccgaccgcgcgcgacctgcgcctcctgatcgccatctccaagaccaccgccaacctggagcgcgtgggcgacgaggccaacaagatcgcgcgcatggtcaagtcgatcatcgagagcggctcggcccgcgcattgccctcgaacgaactgcgcattgccgccgacctggcttcgggcctgctgcgtacggcgctcgacgcgttcgcgcgcctggacacggccgccgcgctgtcgatcctgaaggacgacgacctgatcgacaaggagttcgacggcttcgtgcgcaagctggtcacctacatgatggaagacccgcgcacgatctcggccagcctcgacctgctgttcctggccaaggccatcgagcgcatcggcgaccacgccaagaacatcgccgaattcatcatctacatcgtcaagggtgccgatgtgcggcacacttcgatgcaggaaatcgagtccgcgctgcagtaacccgcgcggcaagactcacaggaaagcatgaagaaaccccgagtcctgatcgtcgaagacgagtcgtcgatcgccgagctgatcgccgtcaacctgcgccataacggcttcgagccgatctggtcggaagatggcgccgcagcgcagcgcgagatcgacgccttcctgccggacctgatcctgctcgactggatgctgccgggccaaagcggcctgcagctcgcgcgccagtggcgcaaggacgcgcgcaccaaggccgttcccatcctgatgctgaccgcgcgcggtgacgagcccgacaaggtggccggcctcgacgcgggcgccgacgactacatcaccaagccgttctccacgcaggaaatgctcgcgcgcatccgcgcggtgctgcgccggcgcgcgcccgaggtggtcaccgaacgcgtggaaatcggcgagctcgcgctcgacaccgccacgcaccgtgtcacctggcagggcaacgcgctcaaggtggggccgaccgaattcaagctgctcgcctacctgatgcaacacgccgagcgcgtgcacagccgtgcgcaattgctcgacaaggtctggggcgaccatgtctacatcgaggagcgcacggtcgacgtgcacgtcaagcgcctgcgcgaatcgctgggtgccgcgtcgcccatggtcgagacggtgcgcggagccggctatcgcctgaccgcccaagtcacggtttgaccagcgccgtgtccatcggccgcgggcgcggataatcgcccgccatgccttttcgtattgctacttttctcatagcgtcccttgcaatgggagcgggcgctgtagccatttttggctggagattcggatggctgggcgcctggttgggcgcggtgctctggctcgtgctcgatgcgtggcgggccgagcgcctgctgcaggtgctgcgcaacaacgccgccggcctgccgacgcgtggagccggcgtgtggggcgaactctcggagcgcatccgcaagctgctgcgcgagcgcgagcaacagacgcggcaggccgaagaccggctgcaggagttcctggcggccatccaggcgtctcccaacggcgtgatcctgctggacgagcagggccgcatcgaatggtgcaaccagacggcggcaagccagttcggcatcgacgccgagcgggatcttctgcagcatcttgcgaacctcgtgcgcgacccggctttcgtggcctatctggcgtcgtggaactacagccgcgacgtcgtcatcgacgcctccggcctgcgccaggcgcagcagcgcagccacccggtgcgtctgtcggtgcaggtgcatccgtatgcgggcaaccgccgcatgctgctgacgcgcgacatcacggcgctggaacaggcggaggccatgcggcgcgacttcgtcgccaacgtttcgcacgaaattcgcacgccgctcaccgtgctggcgggttttgtcgaaactctgcagaacctgcccctcgacgcggaggagcgcgcccgttatctctcgctgatgggccagcagtcgcaccgcatggaaacgctggtgaacgacctgctgacgctctcgcgcctcgagggcagtgcggggccgacgggcaaccagtggatccgcatccgcgcattgctcgcgcagtgcgaggacgaggcccgcgggttgtcgggccgactggcgccgcagggccatcgcctttctttcagcgtcgaggccgagtccgaaatctcgggcgcgccgaccgaactgcaaagcgccatgtcgaacctgctgagcaatgccatccgctacacgccaggcggcggcgaggtggtggtgagctggcggctgctgcccgacgggcgcggtgaattcgcggtgcgcgataccggccccggcattgccgccgagcacattccacggctgaccgagcgcttctatcgcatcgatcgcagccgctcgcgcgagaccggcggcacggggctgggcctggcgatcgtgaagcacatcgcgcagcggcatggcgccgagctgcgcatccagagtacggtgagcaagggctcgcgctttgcgctggtgttcccggcaacccgggtgcgtgaagcgcgggtgctagcgaagtgaacgccgcatcgtccaccgcagcagcgcgccgaacaacagggccgtgacggcgagcgcgcccgcgctcatgagccagaacgccaagggcgactgcattgcgggccagggcccgaggccccggtaggccagcaggtagctcccgccgagcccgaagccccagagcagggtgcaatagatgaccagcggcacgagcgtgacgcggtagcagcgcagcacgaacacgcacagcgtctgcagcgcatcggcgaagtggtagaccgcgaccaccagcagcagcgccgcggccagcgctatcacggtcgggttgtccgaatacacatgggccagcttgaagcgcagcgccaccatcgcgccggcaaaaaacagtgcgcagagggcggtgagctcgaagcccaggcggcaagcgcggcgggcccttgccgcttgcccggcaccgagccagaagctcacgcgcgcgctggtggcaatgccgagcgagagcggcaccatgtaggccaccgccagcaggttcgaggcaatctggtgcgcggccgccgccgccgtgcccaggcgagcgatgaacagcgccatcagcgtgaacgaggtcacctccaccagcaccgccagcccgcccggaatgcccaggtttgcgaactgccggatctgccgccaatcaggagcctcgatgcgctcccagagccggtagtccttgtagaaggaactgccgcgcaggagccagaccgcgcaggccagcatggcccagttcacgcacagcgtggcccaggcgcagcccaccagtcccatggccggcaggccggcgccaccgaaggtgaaccagatcgacagcggcagtttcacgaacagcgaacccagctgcagccaggtcacgacctgcggtttgccgaggctctggttcagtgtgctgaacaagcggaagagcagggcgggcgggagcgcgaaggcgagcaccgccaggtatgcctccacgccggcgcgcatctcaggaggcacctgggtccaccgcagcacggcaccggggaacagcagcacgaccatgccgatggcgatggtgatggcgctcaggtagagcgactgccgcacggagcggcccaattcgcttcggcggtcggcgccgtgcagttcggcccacaccggcagcagcgcctgcagcacgcccatcagcgagacgaacacgctgatgaagatggccgcgcccaccgacagcgcggccagcgcgctctcggcatagcgcccggccacgatggtgtcggtcacgccgaacgccatcacggccagttggccgaccagcaccgtgccggcgtgccgtgcgatcaggcctcgttcgccaatcacttgctacggcacgatcttctggtagagcagcaggtcgtcggttgcgctgctcggccggcggagcgtgccgctgaaacgccaccgatccagcggaatgatggtgtgcagccgctcgatggtttccgggctgaccagcagccaggggcagttggtgccaagcagcagcggctgcaggttgaaacggccgtgatgctgcagggccgcaatgtgcgcccggctgagcgccagttcggcgatgcagctcggctggccgacccgttcggccaccgcgcgcacctgcggaacatagctgcgcgcgtagtcgatggagggcagccagagggtcatcagcagcatccagcacagggccgtgccgccggccggaagcaccagcgttttccagagtgccgcgcggtggcgcccggtgcgccagcgcaccagccagcaccaggcgaggcttgcggccagcgccaggacgaacgcaatggccgagaactccggcacgaagccgggcaccagccgcgccacgctggccgccggcttgggcggaacgccggtctgcatggcgacccagtagatccagcccagcacggccaatccgctgaagaacagcacgttgaaccagtcgatcagcgccgccacgctgcgccggaacgtgggcagcgcgaaggccgccagcgtggcgagggcgggcagcgccagcagcagcgaacggtcggaatagtcggtggtccaggtggcggccagcggcaccagcgcgaaccagaacggcagcgccacgtggcgcgcagtgagctgccggcgccagcgccagagcgtccagatggcaaggggccagacgggccaggtgaaccacaccagcagcttggcctggctgcgcacgtcgcccagcacggaggtgctgttcggatgatggcccggcagctggatcttccactgcagcagccccagccctgcggccagcgccgcggccaccagcgccgccgcaatcatcgtggccagcgcgcctttgctgtagcccgggctctcatcggccgtggtgtgggtgtcggcgttggcgttggcccgggcggtgcgccgttcgtaggccatgaagagcgcgctgcccactgccagcgccagcccgaccgtggggccgccgctcagcgtcatgccgacggtgccgaccaagagcgcgatgaccggcccgacccggcggtacggcagcgcagccacgccgtagaagagatgcgaggcgaaatacagttgcgccagggccggcgtggtttcatggccgagttgcgcgagtccgaggcaggcgatcagcgccagcagcccgccgtcggcgatggcgcgcgcatagtcggtcggccgggcctcgccaccgaaggcgaaggccaccggctgggcccgcgaggtgcgggcgaggtaatagacggcgtaccaggtggcggtgaacgtgccccagagcagcagcgcaaagacgatgcgcactgccaggtcggggtgcagccacgagggcgcgatcttgatcgcccaggcaccgatccagtatggaatgagcgccggggtttcgggcctgaggcccaggagcatggggtcgaaccagcgagcgatgccttcggtgttgcgcgccagctcggccatgtagccgaaggaggtgatgtccgcgctcttccaggggccgcgccccacgaggcccggcagaaggtaggcggcgcacaacaacagcaatgcgatgcgcggcaaccggcgcacggcgctctgggcaacgattgctggagtgggctggttcacgaggaagttcgggcgggcagtcttgggaaagaaaaagggcagcgcggtaaaccgggctgccctcgatgcgaaagcgcgtgctttacttggaagcagcgccggtggtcttgccgaagcggttgcggaacttctcgacgcgaccgcccatgttgtcgacagacttttgcgtgccggtgtagaacgggtgcgattcgctcgtggtgtcgagcttgaacagcggcagttcgcggccgtcgtcggtcttgcccatttccttggtgttcgcgcacgaacgggtcacgaacttgaagccgttcgacatgtcgacgaacagaatttcgcggtaattcgggtggatgccttcttttgccatggtatttcctttggggtcgatgcgagagccacaagcgtgcctacagagggcaagccattccggggagggaatcgccgggcaaaacgcccagccgcacttttcgcggagccagcgattatcgcatactggccgttttgagcgaaaggcggcctctcagatgacctccagaacgttgcgtgccggcctcgtcggctacggctttgccggccagactttccacgcgccggtgctttcggccgttccagggctcgaattggcggcggtggcaagctcgcagccgcacaaggtccacgccgaatggcccggcgtggcggtggtgcccgacgtggcagcgctcgtcgcccgggaagacatcgacctggtggtggtggccacgcccaatgcccagcattgccccgttgccaaggtggccctggaagccggcaagcacgtggtggtggacaagcctttcacgctcgatgccgccgaagctcgcgaactcgagttgttggccgagcgcaacaatcgcgtgctctcggtttaccagaaccgccgtttcgacgccgactacctcaccctccaggacgtgctggcgggcggcgaactgggccggccggtgtacctggagtcgcatttcgaccgcttccgccccgaggtgcgcgaccgctggcgtgagcagaaagtgcccgggtccggtctttgggtcgacctgggggcccatctggtcgaccaggcggtccagttgttcggcaagccggacacgctgcagctcgacaccgcggtcctgcgagagggcgcgcaggtcgaggactattttcatgccgtgctgcgctacgaaagcggtccccatgcgccgctgcgcgtggtgctgcacgccaccacgctagccgcccatgccgcgccgcgctacatcctgcacggcacacgcggcagttacgtcaagcatggggtcgatccgcaggaagacgcgctgcgcgccggtggtcgcccgggcggcgacgactggggcatggacccgttgccgggtgagctgaagacggtggcggtcgagaactgggtacgcgagagcacggtgcccaaccgccgcggcaactacgtcgattactacgccgcggtgcgcgacgcgatcctgggcatcggactcaacccagtgccgccgtcggaggcggtggcgctcatggaactgctcgacctgggcgctcgcagcgcacgcgagggccaggccttggtgccatgaaaaaagcgcgtcgccccaatgggacgacgcgctttcgggcgacgatcgcgagggggctcagccgcctcggcgcatcatgtcgaagaactcgacattggtcttcgtcgccttcatgttcttgagcatcagctccatcgactcgatctcgtccatgttgtacatgagctggcgcaggatgcgggtcttttgcaggatctcgggggcgagcagcagctcttcgcggcgggtgccactgcggttgagctggatcgacgggaacacgcgcttttcgtacaggcggcggtccaggtggatttcggagttgccggtgcccttgaactcttcgaagatcacttcgtccatgcggctgccggtgtcgatcagcgcggtgccgatgatggtcagtgagccgccttcttccacgttgcgcgccgcgcccaggaagcgcttggggcgctgcagcgcgttggagtcgacaccgccggtcagcaccttgcccgacgagggcacgacgttgttgtaggcgcgggcgaggcgggtgatcgagtccagcaggatcaccacgtccttcttgagctcgaccaggcgcttggcgcgctcgatcaccatttcggccacgtgcacgtggcgcgccgccggttcgtcgaaggtcgaggcaatgacctcgcccttcacggtgcgctgcatttcggtcacttcttcaggccgctcgtccaccagcagcaccatcatgtgcacttcggggtagttggcgctgatggcgtgggcgatgtgctgcatcatcaccgtcttgccgctcttgggcggcgccaccagcagggcgcgctggcccttgccgatgggggcgatgatgtcgatgatccggcccgtgatgttctcgtcgctcttgatgccgtcgcgttccagcttcatctgttccttggggaacagcggcgtcaggttctcgaacatcaccttgtgcttgttctgctcgggcggaccgtcgttgaccttgtcgagcttggtcagcgcgaagtagcgctcgccgtccttgggcgtgcgcacttcgccttcgatcatgtcgccggtgtgcaggttgaagcggcgcacctggctcggcgagatgtagatgtcgtcggtgctggccgtgaagctggtgtcggggctgcgcagaaagccgaagccgtcgggcaggatttcgagcacgccgtcggcaaagacctgctcgccggccttggcgcgcttcttgatgatcgcgaacatcagctcctgcttgcgcatgcggccgacgttttcgatctcaagcgcttcagcctgcttgaggacttcagacacgtggagtgccttgagttcgtttaagtgcatggaatgaccccttgcggggcaatcgatcggaaaaacggggggaggtttgatgtgaagcgagagctgcctcacaaaccggggaactcgaaccggctacctcgaagggaccggtgatctgtgggagattatgacagcaaaaaaccgtccggccaacgcattgcgcgctggccggttgaaatgtctcaggcgagctgctggtcgatgaaggccgtgagttgcgccttgctcatggcgccgaccttggtggcggccagctggccgtccttgaacagcatgagcgtgggaatgccgcggatgccgaatttggccgggatgtcgcggttctcgtcgacattgagcttggcgatctgcagcttgccttcgtaggcggtcgacacttcatcgaggatgggcgcaatcatcttgcagggaccgcaccattcggcccagtagtcgaccagcacgggctggctggacttgagcacgtcggcttcgaaggaagaatcggagatgtgtttgatcaggtcgctggccatgagatgtgtccttgtgcgcggagagtttcggtgcagctaaagtgctggtcattgtgacagaaaccaaggggtggggtgccatgcgggaacgctatgacaccgatagcaaaagccctttgcgcgtcgcgcctccatgctcccaaacccctcgatagatcatgaacgaaggccaccccgtccaggccctgtggtgcgaccccgccgacggcgtggtggcgcgcattgccggggccattgcacagcgcgggctgcacgcggcgcgcaccgtggtgctggtgccgtatgcgcaattgatgggcgtggcgcgcagcatgtgggcgcgctgcgggagcccgggcttcgtgccgcgcttcgaaaccacgcgcaactgggcgcgcagcgcgggtgggttcctgccctcgggctacgacatcgcattcgacatggcgcaagacctggtcacggcccaggcgctgctttcgcaggccggttttgccgccgagcgctttgcgctggccgggcgcgtggtcgagctggcctaccagctggccccgttggcagcggcagcgctgcccgaagagcggggcagcgaatgggcgcagcgggcggcccaggtggccgaggcgggcagcgagtcggaatggtttcgcatcgaaagcgcgctgatccgcgtcgcggtggcctgggtcgccaactcgggctacgccaccgacgtgctgctgcgcgagaacgtgcgcgcgcaggtcgatgcgctcatcgtgctcgagggcttccagaccgatccgctcacgcagacactttgcaccttgtggggcgaccgcgcgattcatctctcgctggtgcccacggctcggccagccgcggccgccagcgcgcatgtggccgccgaccccgaagacgaggcggagctcgcggccgcctgcgtgctgcggcacctggccgaaggccgtgcgccggtcgcgctgatcaccaccgaccgagcgctcacccggcgcatcggtgcgcagctccaggccgagggcatcgcggcgcacgacgaaaccggctggaagctttccaccacacgcgccgccgccacgctgatgagcgggctgcgcgcctgtgcgcacgacgcgggcagcgaccaggtgctcgattggctcaagagcggcgccgacggcgatgccatggccgtccaggcgctcgagtcccgactgcggcgcgaaggcgtgcgcgagtggtccgcctggtgcggccaggtggcgcgcagcgagaagccgcaggacatcgcgctgctgccgttcaccgaagccatcgaaggccgccgcatggccatggccaagtcgcggcccctggccgattggctgcgcgcgctgcgcgagctgctggaggccggtgcccaatgggagtcgctcgccgccgacatggccggcgccaaggtgatcggcgcgctgtggctcgatgccgatgcgcacggcggcggcgacgactttcccggcggacgccacacgctggccgaattcacggcctgggtgcgtgacgtgctggaagacgccagctttgtaccgcccgccggcagcgacacgccccaggtggtggtgctgccgctgcaccagttgttgggccgcgcgttcggcgccgtggtcattcccggctgcgacgaccggcgcctgccggcttctcccgagccgccaggcaactggagcgccgcccagcgcgccgagctgggcctgcccgcgcgcgagaccctcgaggccgcgcaacgcgcagcctgggccgcggccctgtgcaacccctgctgcgaaattctgtggcggcagtccgatgccagcggcgagcccgttcgcccgagcccgctggtgcaggcgctgcagctcgaccacgccctgcagccggcggcagacccgcgcacgccgcgcgaagtggcgttgcagccgacgccgtatcccatgccctccggggcgctgctgccgctgcggaacatctcgaccagcgtctatgaagacctgcgccgctgcccgtaccgcttctttgcgctgcggcaactcggcctgcgcagtgccgatgagctcgacgccgaagtcgacaagcgcgacttcggcaattggctgcatgccgtgctgggccacttccacgatgcgctgagagagacgccgaccaacgatgttgccgagcgcgtgtcgctcatcggcgcggcggcagagcacgccacgcgcgaattcgggctgtccgatgccgagttcctgccgttcgccgcggcgtggccggccgtgcgggacggctaccttcagtggcttgccggacacgaggccagcggcgccgtcttcatggaatcagagccctggaaggagcagccgctgggcggcctgcaactggtcggccggctcgaccgcatcgaccgcatgcccgacggccagtccttcgtgatcgactacaagaccgagtccgccgcggtgaccaaggagcgcgtcaaggacccgaccgaggacacgcagttggccttctatgccgcgctggtggccgacgacacgctgcgcgcggcctacgtcaacgtcggcgagaagtcgtccggcacgcagaccgtcgaacagcccgtggtggtggaagcgcgcgatgcgttggtggcgggcatcctcgacgactttgcccgcattgcgcaaggcgcggcgctgccgccgttgggcgaaggcgccatttgcgactactgtgcggcgcgtggcctctgccgcaaggatttctgggaagtcgaacaacctccgctttctccggtggccggaggattggccaaatgaacggcgccgcctacgaacacaacggccggcacgtcacgcgcgaggccttctacaccgtcgcctgcgatccgcggagatcggttgccgtcgaggcctgcgcaggcgcgggcaagacctggatgctggtgtcccgcatcttgcgcgccttgctagaagagggtgaatccgcctgcgagccgcacgagatcctggccatcaccttcaccaagaaagccgccggcgagatgcgcgagcggctcgaccagtggctcgagcaattcgccgagcgcagccccgaagagctggtgcgcgaactcgtgattcgcggcgtgaggcccgataccgcgcttgctgccgtaccgcgcctgcaaggcctctaccggcgcttgctcgaaggcggccggccggtgcagtttcgcaccttccatgcctggtttgcgggcctgctgcgcaacgcgccgctggcagtgctgcgcgaactcggcctgcctgcgaactacgaactgctcgaggacgatgccgaggcgcgcgcacgcacctggcggcccttcttcgaagccgtgacctccgacaaggaggccctggccgactactacgctgtcgtcgccacctatggccggtcgcagaccgccaaggcgctgggcgaagcgctcacgcgccgcgtcgagttctttctgtccgatccggcctccgccgtgcagcacttcagcgccatgcatcccgcgctcgaaggcatggacgatccgaccgatgccttgaggggagaggcggtcaggcaccgctggctcgaccgtgctgccgcgctcggccgcgaagccaacaagacgccgcagaaggccgccgaggcgatcatcgacgtgttcggcaccggtgagccgccgcgcgagtcgcgctcggccgcactggcgcacctgcgcaagaacttcttcgtcgccgctgaagacaggcttaccaagaacctgcagaaataccctgcagcgcaagaggccgaggccgaactccaaaccttgtgcgccgcgcaggcacagcacgcggcctggctctaccagcagcgcatgacgcggctcacgcgcatcctcatctccgcctttgccgaggtcaagcgcgcgcatgggtgggtcgacatgaacgacgtcgaacaggccgcgcagctgctgctcggccagtcggcgttgtcgggatgggtgcaggagcggctcgacgcgcgcatcgcgcacctgctgatcgacgaattccaggacaccaacccgctgcagtggcaggcgctctacggctggctcagcgcctacaccggcgcgggcggcagcgcgccgcgcgtcttcatcgtgggcgacccgaagcagagcatctaccgcttccgccgcgccgagccgcaggtgtttattgccgcgaagaagttcgtgcgcgaaggcctgggtggcgagctgctcaactgcgaccatacccatcgcaatgcgcgtgcggtggtcgggctggtcaacagcgccatgctggcggcgcaagaagccggcgagttcgacggctatcgcgcccacaccaccgagcgcaacgacgatggcgaattgctcaagctgccgcccatcgaccgcgacgccctcaatacgggagcggaggctgcgccggccgacgacggcatgctgcactggcgcgacagccttgttactccgcgcgtgttgcccgaagaacaattgctgcaaaaggaatgcgagcaggccgcgcgctgggtcgcgcagcgcattgccgatggcacgccgccgcggcagatcatggtgctggcgcgccggcgcaaccggctggccgccatgcaggacgcgctgcgccagcgccatattcccgtgcagcagcccgaaaagaacgaactgcacgacgcaccagaggtgcaggacgtggtggcgctgatcgatgcgctggtgtcgcccgcgcacgatctttcgctggcgcgcgcgctcaagtcgccgctgttcggcattggcgacgatgcgctggtgcaactggcgctgcgccagcgcgagcaacccgccctgagctggttcgggttgatccagaaaggagaaggcttgccgccgcagttggtcgaagccggcgccaagctcaagcaatggcagcggtggctctccgcgctgccgccgcacgacgcgctggacgcgatttttcatgatggcgatgtgctggccaggttcggcgccgccgtgcctgcccccatgcggcagagcgcgctggccaatctgcgcgggctggtcgcggcatcgctcgacatcgagggtgcgcgctttgccacgccctacgcgctggtgcgcgcattgcgcgccgggggcgtacgggcgccctcggtcgccgtacccgatgcggtgcagctcctgaccgtgcatggcgccaagggtctcgaggccgacaccgtgctcatgctcgattgcgatgctccgccgccgcgcgcgcagaccatgggcgtgctggtcgaatggaaaggcagcgacagcgcgcccacgcgcttcgtgttcctggccagcgagaaaacgccgccgggctgcgcggccacgctactcgaagaagagcagcgggcgcgccatcgcgaagagctcaacgggctctatgtcgcgaccacgcgggcgcgcgagcgtctcgtgctgtcgtcggtgcagccggcccgcgccaacgagggcagttggtggtcgcggctcgagtcgatgtgcgaaccggcgcaagccgacgaaccgctgctcgcgctgcccctgggaacagcggctggcagtttttcgatgaagaagatgcccgtcgcgcccgccgccgaactgcccgccgtcaagaaagccgctggcggcactgtcgatgcccgggctgccgcgttcggccaagcgatgcaccggctgctcgaatgggccgtgccgggcgaggcgctgccacccgcgcacgtgcgtgccgccgcccgcgagttcatgctcgacgcgcaacaggcccgcggcgccgcggtgctggccgagcgcatccgcgcgggtgctggcgcatgggcgtgggacgagcgcatgatcgactggcacggcaacgaagtgaccctggtccacgaaggcgaaacgctgcgcatcgaccggctggtgcgcgagcgcgccagcggtgcctggtggatcctcgactacaaatctgccgcgcgccctgaacgggacgcggagttgatcgcacagatgcagcgctaccgcgcggcagtgcaacatgcctatcccggtacctcggtacgcgtcgcgttcctgaccgggcagggcgaactggtaaatctcgaatgactctttcccataccgtcgccgtgatcggcggcggacccgccggcctgatggcggctgaagtcctgagcgcgtccggcgcacaggtgcacgtttacgacgccatgccctcagtggggcgcaagttcctgctggccggccgcggcgggctcaacctcacgcattccgagcccttcgatgtgttcatgagccgcttcggcgagcgccgcgcgcagctcgaacccatgctcgcgcagttcgggccgcagcaggtgcgcgaatgggtggccggccttggcatcgagaccttcgtgggcacctcgggccgtgtgtttccgaccgacatgaaggccgcgcctttgctgcgtgcctggctgcaccgcctgcgcgcggcgggcgcgcagtttcacatgcgccatcgctggcttggagatggggcattcgacgcggctgcattgcggttcgcaactccggccggcgagatcgccgtgaaggccgatgcggtggtgctcgcacttggcggtgcgagctgggcgcggctgggctccgatggcgcatgggcgccatggatgcaagagcgtggtgtcgatatcgcgccgctgctgcctgccaattgcggattcgacggggcagggtggagcgagcatttttccagccgttttgcgggccagcccttcaagtcggtcgcgatctctttcaccgacagccaggggcgccgctttgcgcgcaagggcgagttcgttgcaacggccacaggcatcgagggcagcctgatctacgcggcgtcggcactgctgcgcgacgaaatcgccgcgcacggcagcgcgacgctgctgctcgatctgttgcccgaccgcagcgccgagcaggtgctggctgccgtcaagcatccgcgcggcgcacggtcgctcagcagtcatctcaaaagcaggctcggcctggaaggcatcaaggccggtgtgctgcacgaagtgctgagccgcgacgcaatgcaagatcctgagcagttggcggcaaccatcaaggccgtgccgctgcggctggtcgcaacccggcccatcgacgaagccatcagcacggcgggcggcgtgcgcttcgaggcgctcgacgaacggctcatggccagcgcggtgccgggcgtcttcgtggcgggagaaatgctcgactgggaggcgccgaccggcggctacctgctgacggcgtcgatggccagcggggcggccgcggcgcgcggagcgatcaagcagctgggcctttgagggtataactgaatacttttgtattgtttattgcacgtacaaggaataagctgcaatcagacaaaataaaggagcagcgatgaccagcgttccatcgccgcgcgccgcgcgcgggcttgcttatgcatccctggtgttcctggtttggtccggcggtgacgcaggaggtggcgcccgcgcgcagggcgcgaatccgacgctggcgggcacgtccgcatcggcaagcaggccggcgccaccagacggacagccggcgtccctcaccagtccgtcccccggcaccaagttcgccagccgcagcgcgaccttcgtctggaacaacacgggtgccaaccagtacggcttgacgatcctgtcggcctcttcggcgacacccgtggtggacacatcgacaaatgcgacaacgctgacggtgacaaaccttcccatagacggcgcggggctcgtggtccggctgcgctcccgattcaaggggaagtggctgccggccaacgaatacctgttcacggcagccggatacaccgcggcgcaatcgaccgccgcggtgaagccctggtccgatctgatcgcgctgccactcgtgcccgcatcggccgccaacctccccgacggcaagctgctgctgtgggcagcccgctcgcccaccagcttcagcacgagcagcagcgaggcgtacacctacacctcggtgttcgaccccgtcacgcgaacagccagcccgctggttgtcacggccaccggccaccagatgttctgccctggcctgagcatgctggacgatgggagcgtgctggtcagcggcggcagcgatgcgacgaagacctcgatctacgacccggcgctgggcggctgggtgacgggtgcgcaactcggcattgcacgtgcctaccagtcgagcacgacgatgtccgacggctccgtgttcacagtcggcgggtcgtggaacggcgggcagggcggcaagtacggcgaggtgtggtcggccgccaccaagacctggcgcacgctgtccggcgtaccggccaacatgcccgatgcgagcaatgtctcgaacccgccgctggccggccctgacgcggccggggtctaccggggcgacaaccacatgtggctgttcggcgctgccaacggttgggtattccacgccgggcctgctgccgcaatgcattggatcgacacgcgcggcagcggcgccatcctgcaggccgggctacgcagcgacgacccctatgccatgaccgccagcgccgtgatgtacgacatcggcaagatcctcaagcttggcggcgcgcccaaccacgacagcggcaacgccttcaagaccgcctacatcatcgacatcagcgcgggcgcgccgacggcgcccacggtgcgcaagctttcgccgatggcctatggccgaacctttgtcaacagcgtggtgctgcctaacggcgaggtgttcgtgataggcggacagacgcagcccgttccgttttccgattcctacagtgtgctggcggccgagctgtggagcccggcgctggagagcttcatcacggtgccgccgatgcagaaaccgcgcaactatcacagcgtggccctgctgctgccggacggacgcgtgctggcgggcggcggcgggctgtgcgactgtgcgggcgaccacccggatgcggagatctacacgccaccgtacctgctggcgagcgacggttcgccggcgtcccgcccggccatcacggccgcgccggccagcgccacatgggggagccagatcgccgtgacaaccgaccgcgcggcggcccgctttgcgctggtgcgcatggcatcggccactcactcggtcaacaccgatcagcgccgcatcccgctgtcattcacgggcacggcaggcaactaccagttgggcattccgaccgatcgcgggacggtgctgccgggcaactacatgctgttcgcactcgacagcagcggcgtgccgagcgtggcgcgcaccatcaacatccggtagcggccggcgcgcttcgcgaagccgatgctttcgatgatgatgctggcgctggcgctcggaaccgcactggccgttggcccggcgtggtccggaacgcctgaagccgccatgccttcctcggtggcgcatggcgcgcgcctgttcgatggcaccgagccactcgccggcacgctgtccggccacagcgcgccgctgccgggcgcagcgactcgctgcatccagtgccacgcgggccccggcaagtccactgccgctgtctccggtttcgcgccgccgctcgaccggcgccaattgcgcgaagtcctcccgcgccgcggcggcccgcccgtcgcgtacgagcgcgcatccttctgccgcacgctgcgcaccggcatcgacccggcccatgtcgcgctgccccgagccatgccgcgcttcgatgccgacgaaggccagtgcgcggcgttgtgggactacctgacgcaagccctttctcaatgaacccaatgaacgcgcggggctccttcataccctcgcgggttgcatcccgcgggcgccggcgcctgcttgccgccggtgcactggcgtggctgggtgtgcctccggcccgcgcaaacaccagcatcggcccggtgctgccggcggtgtcggctccggccctgccgctgcggcgccacgacggcgccacaccgatgctcgctgcgcagttgcgaggcgccccaaccgcggttcaattgatgtttaccggatgcagcacggtctgcccgattcagggggccttgttctcgacgctgcaggcggcattgctgtcggagcgctacacggcggtgcgcctgctgtcgctgagcatcgacccactgtccgacgaccctgttgcactgagcgcctggttgcggcgcttcggcgcaaggccaacgtggagcgcggcggcgccagcccccgaggcacttgagtcgatgctctcgctgttcacgggaggcgcggcagcgggcgaccgccataccggccaggtttatctgttcgatcgtcacgcccggctggtctggcgaaccagcgagttgccgccgaccgaagaggtcatggccggactacggcagcttggttagttggatgcagcggctgcggattcagcgccggtgaggggccgcctgccatggccagcggcgcagccgcggcgcgcggggctggggatttcctcaaccaggatgcggcaaaaccgagccagtagaggatggcaagaatcagcaacttctgagtcaggccccgcggtacgtcccgccatagcgtctgcacccagagcgcaatgaaacagaacgccgccagggcaaatgcggcgacgaagcgaggccgccacagcgggtcttcgcgcagccgccaggactgcaacagcatcgccgtggtcgtgcaaagaaacgccgtttgggccgcaacgccgtgaatgaagccttcaagagtcggcggcgacagatacgtgttcgtttcggccaaggccgtgaccacaagcccgagactcccgcatgcgaacataagcaggggggcggcgctgcgggcgcggggcgacagggcgcggtagtagccaacgcccaaggccagaagtgcggtagccaaagcgaagtacgcaccgcgcacccacaaggcgtgcgggccgatcagataaaagctcaaaggcgcgcgaagccagtcaaggtcggtgcgcagcatctgtgccgacgcacacaccagcaagaatgcgcaaaccccagtgccacccgccaatccgaattgacggctccttgcgctacaggttccgaacgtcatccgcgcttgacctctaccacgcgtccattgacgatgctcaacgtgcggcggttttcaaggtaatccatggttccgggaaaccgctttccgtctcgcatcccgatgcgccatgggcagcccgccagcaggtccaccgcttcgcgctcgggtttgccgatcagcgcgttgtctccgaggcggtcggccttgcagccctccgccgtgcccggtgcgccttgaggccccggcgcggcgacggatgcgggtggggtgttcaccgcagcgcagcccaccacacccatggtgagtattgccgccactgccattcgaccggcggcctggtttttcttgatcgttgtcatgcaatttcctttcgttggttgatgggggcgactgtggctattctgaagcgcgggttctcggacgagaccatcggcgccggtgggctgttgctggggcgctcgggccgacggccgtggcggctgcggcattcatgctgctttgaattgcccgagccgggcgtgttcgttgcgggagagatgctcgattgggaagcaccgaccggcggctacctgctaaaggcatccatggccagcgctgcggccacagcgcgtggcgctgtcaagcggctgggcctctgacggcttcgcgcggctgcggcggggaaggcctcagagccgcgctgcgacccgggtgtcggcgaaaacgctgcgcccgagccagcgccagaggttgcgggtatcggattccgtgccgatgacgcgcaggcgccgctcgcgcaacgcagcctcggcgtcgaggtcgccggtccagatctcggtcagggttcgcacggtcgattcgacaatcagcgtcggttcgtcgccggggttgtcgcggcagaggtcggcgctgccctggtcgacaaccagccaccagcgccgctcgccctcggctgcgtcggtgaagcggaagtggatcacgatgcagcgcgcgcgcgggcactcgtcgatccgcacgaagcggcggacgtcccacatcaggaagccggcgtccagctggtcgcgcttgagccggctgccgatccagcgcgcaccccaatggcccagggccatcacgatcgggcgcagctcctcgcccgctgcggtcaggtgatattcggccgtgctgccgtcgccctgaacccgcttgacgacacccacttcctccagcttgcgcaggcgctgtgccaacagcgagcccgacatgcgcggcacaccgcgccggatgtcgttgaagcgcgtgctgccgcacagcagctcgcgcaccaccagcggcgtccagcgctcgcacagcacctcggcgccgcgcgccacggtacaaaactggccgtagtcgatcatggcgccaatttagtcgctgcggcgatccgaggccagtacagattctggactggagaacttccggccgcgctgccatccttgagactccctcactcgatggagatccatcatgaccaccgtcacagccccgccggcattcaacgccgccgccttcaagaccaccacccgcgctcaatggcaggctgccgccgaggcctggcatcgctgggggccgtttctcggccgctggctgggcgacgcgacggaaacgatgttcgatctggcccgcatcgagcccggcagccgggtgctcgacgtcgcggccggcgcgggcgagcagtcgatcggtgcggcgcggcgcgcaggccccagtggccgcgtgctcgctaccgacatcgcgccggccttgctcgagcgcgcggctgcggatgccaaggccgcgggactgtcgaacctcgagacccttgaactcgatggcgaggcgctcgacaccctgcccgccggaagcttcgacgccgcgatcagccgcgtgggcctgatctactttcccgaccagcagcgcgcgctcgccggcatgcggcgggccttgcgtccgggcgggcgggtgtcggcggtcgtctactcgacccccgagcgcaatgcatttttctcgatccccgtgaagatcattcgcgaacgcgcgcggcttcccgcgccgctgccgggacagcccgggccgttttcgcttggtgccgaaggcgcgctcgaagccgcgtttgccaaagccggtttgcacgacatcgaggtacgccgggtgccgtcgccggtgcggctggcaagcgcagccgaatgcgtgcgcttcgaacgcgagtccttcggagcgctgcaccagatgatggtcgggctcgacgaggccgagcgtgcgagcacctgggatgccattgaagaggcgctgcgacagttcgaaggcagcgaaggcttcgtcgggccatgcgagatgctcgttggcggcggaagcacgtgagggtgggagtggggggcttgccgcccccatttcagcgcgcaagtccttgagaactcacggctttttgatgttaggttgacgagccttacccctggcactgactacgcagttagggctgcttggttccccacctgacccggttggccacttcaccatgcagggaggcccgtcagcacgcattgtaacccggtggcccggcaaagccgggtcaccggtgtccctcgggaagacgggtcttttttgatttgcgggacggggccgaggaccggcgcggcgccttttagaatgcccgcaatgtcttatctagtgctcgctcgcaagttccgtccgaaaacctttggtgagatggttggccaggggcacgtggtgcaggcgctcgagaacgcgttgaccacgcagcggctgcatcacgcctatcttttcaccggcacccggggcgtgggcaagaccacggtttcgcgcattctggccaagtcgctcaattgccagggcccggacgggcagggcggtatcacggccacgccttgcggggtgtgccaggcttgcaaggacatcgattcgggccgcttcgtcgactacaccgagctggacgcggcatcgaaccgcggggtggacgaggtgcagtcgctgctcgagcaggcggtgtacaagccggtgcaggggcgcttcaaggtcttcatgatcgacgaagtgcacatgctcaccaacaccgcgttcaacgcgatgctgaagacgctcgaggagccgccggaatacctcaagttcgtgctcgccaccaccgatccgcagaaggtgccggtcacggtgctgtcgcgctgcctgcagttcaacctgcggccgatggcacccgagacggtgctggagcatctgaccggcgtgctgcagaccgaacaggtgccggccgagccgcaggcgctgcgtctgctcgcccgtgccgcacgtggctcgatgcgcgatgcgctgtcgctcaccgaccaggccatcgctttcggcaacggcgaactgctggaaaccggcgtgcgccagatgctcggcagcgtggaccgcggccatgtgttcaagctgatcgaggcgctggcagagggcgacggcaagacggtggtcgacacctccgaggcgctgcggcgcgacggcatgtccgccgcctccacgctggaagaaatgacggcggtgctgcaggccatggccgtgctgcaggcggtgccttcgcgggccgagtcggccgattcggccaccgaccccgatgcggccgacacggcacggcttgcggcgctgatgccggccgacgaaacacaattgctctacagcctgtgcctgcacggccgcggagaactgggcctggcgcccgacgagtacgcggcgctcacgatggtgctgttgcggctgttggccttcaagccttccaacgcggctgcttcctcggcctccacggaaaaaaaaactctgaatgaagcccggaaggcggtttcggcccctgcggccgtagcgccggcccgggcggtagaagttgccgcggcgcccgttgcggctgccgcaccggtggccccgcaggcccctgcggcgccagcgggacagcgccttgccgtggtcagcgagccccttcggcagggcgaggccaggccacccgccacggcagaggttccgccgtgggagacgggcgccaaggtgcttgccgtcccgatgcgcgtccagccgcctccgagccagcgcgacgtgccgcgccccgacgagcagcgcagcccggcaccacctattccgcccagcgaagacggcgatttctggcacgccacggtcacgcagatggtcgcggccgagagcatcaatgccctggcgcgcgaactcgcgctgcagtcgcagctggtggcgcgcgacgtcgaccagtggatacttcgggtggagcgcgagttgctcaaccagccttcggcccgtgagaagctcaccgacgcgctcgctgcgctcggccacggcgtgaagcttgccatcgagatcggcggcgtggtcgacagccccgcgcgccgcaacaagcaggccgcggacgaacgccagcgcgtggccgaggaagccattcgcagcgatcccgaagtgcagatgctgatgcgtgaattcgatgcgaagatcgtgcccggaaccctcaagccggcctgacagaacgctactgaaaactcgtgccggcacttgcggcattccggttcgaccgccatctctcttatccttcccccattccaaccaatcaggaccaacgatgttcaacaaaggacaactggccggcctcatgaagcaggcgcaggcaatgcaggacaacctcaagaaggcccaggaagagctggccaccatcgaggtcgaaggtgaatcgggcgccggcctcgtcaaggtcgtgatgacctgcaagcacgacgtgaagcgcatcaccatcgacccgagcctcctggccgacgacaaggacatgctcgaagacctcgtggctgccgccttcaacgccgcggtgcgcaaggccgaggaaaccagcgagcagaagatgggcaagctcacggccggcatgcctggccttccgcccggcatgaagctgccgttctgagccattgatggccgacgccagttcgctcgacgcactggtcgatgcattgcgccgcctgcccggggtcggcgtcaagtcggcctcgcgcatggcgtttcatttgctgcagcacgaccgcgaaggcgcgcagctgctttcgcgcgcgttgcagcaggcggcgggcaacgtgcggcattgcgagcgctgcaacaccttcactgaggcgcctgtgtgcaacgtgtgcctcgatgcgcgccgcgacgcgaccaagctctgcgtggtcgagacgcccgccgaccaggccgcgctcgagcgcacgggggcctttcgcggctactacttcgtgctgatgggcaagctcagcccgctcgacggcatcggccccaaggacatcgggctgcagaagctcttcgaccgtgcgctcgacggcacggtgagcgaggtcatcctggccaccaacttcacggcggagggggaggccaccgcgcacgtgatcggcgaggcgctcaggcagcgcggcctcagcgtgacgcgccttgcgcgcggcgtgccggccggcagcgaactcgaatacgtggatctcggcaccatcgcgcatgctttggtggaccgtcgataacgtgccgcggccgttgcagccgctggcgaacgcagacaacaaacccaaatgactctttcactgctcaccgttgcctactggtgcgtgttcatcgcctgcgggctgccgtatctcgcggcatggatcgcgaaagccggcagcttcggtccgcgcgacaacacgcatccgcgcgactgggccgcgaagcagagcggctggcgcgcgcgcgccaacagcgcgcagtccaacagcttcgaggggctgccgttcttcattggcgcggtgatcattgcgcaccagctcggcgccaaccaggcgcggctcgacgtgctggcggtggcctatgtcgtattgcgcctgatctacatcgcggcctacatcacgggcatcggcagcgtacgcagcgcggtctgggcgctcggatttctcgtcaacatcgcgattcttttcctcgcgcgataagccgtttggcacaggccgaagaggccttcatgcttacgtgaaaacccgcacgggatgaccccgatgcagccgacaggggcgcacccctaagctcgattcggtctaaagaatcaatgagcccgcaggtccgttccatgctccctcgcagaaccctcatcacagcctccgcagtcgctgccgcatcgatcgcgctgccgcgggtttttgcgcaagccaagctcgagaagacaaaaatttccattgcggtcggtggcaaggccgccttctactacctgccgctcaccatctccgagcagctcggctatttcaaggccgagggcctcgatgtcgagatctccgactttgccggcggtgcgcgcgcattgcaggcggtggtcggcggttcggcggacgtgtgctcgggcgcttacgaacacaccatcaacctgcaggccaagaaccagttcttccaggctttcgtgctgcaggggcgtgcgccgcagatcgcggtgggcgtgtcgaccaagaacatggcgggctacaccggcatccaggatttgaagggcaagaagatcggtgtgtcggcgccgggctcctcgaccaacatggtggccaacctcgtgctgtcgcgcggaggcctcaaggccagcgacgtgagctacatcggcgtgggcgtggcagcgggcgcgctcacggcgctgcgctcgggccagatcgacgccatcagcaacaccgacccggtcatgaccatgctcgagcagaagggcgacgtgaagatcatcagcgacacgcgcacgctcaagggcacgcagcaggtgttcggcgggccgatgcccgcagcctgcctctatgcgccgacggacttcatccagaagaaccccaacacctgccaggcacttgccaacgccatcgtccacggcctcaagtggctgcagacggcggggcccggcgacatcatcaagacggtgccggagacctatctgctcggtgaccgtgcgctgtaccttgcgtctttcgacaaggtgcgcgaatcgatcgccaccgacggcctcgtgccggccgaaggccccaagaccgcgctcgcggccatcgccagcttcgacacctccgtgaagcccgacaagatcgacctcacgaaaacctacaccaacgattttgctaggcgcgcgaaagacaggttcaaagcctgactccgaacgtccccgcgacccggcctcggccgggttttttcttgtggcggccgatgccagaattcctgccagacatgtccgactacgcactcgaacttctctccatcagctgtacttttcactcgaaggatgatccgggccagcgctacaccgcggtggccgacaccacgctgcgcgtgcgggccggggagttcgtatcggttgtgggccccacgggatgcggcaagtccaccttgctgaacgtcggcgccggtttgctcgaaccgtcgtcgggcaccatcaaggtcttcggccaggcgctgcaaggagtcaatgcgcgcgcgggctacatgttccagaccgaggcattgatgccgtggcgcagcgccattcacaacgtgatggtggggctgcaataccgcggcgtgcccgacgccgaagcccgcgagcaggccgaggcctggctgtcgcgcgtgggtctttcgggcttcggcgaccgctatccgcaccagctctcgggcggcatgcgcaagcgggtggcattggcgcagacgctggtgctcgatcccgacatcatcctcatggacgagcccttcagcgcactcgacatccagacgcggcagctgatggaaaacgaagtgctcgagctgtggagcgcaaagaaaaaggcggtgctcttcatcacgcacgacctcgacgaggccattgccatgagcgaccgcgtggtggtgctgtcggcggggccggccacgcatccgatcggcgagtttgccatcgacctcgcgcgcccgcgcgacgtggccgaggtgcgcacgcagccgcgcttcgtcgagctgcatacgcagatctgggaggtgctgcgcgacgaggtgctcaagggctacgcgcagcaactccggaaggccgcatgatgcccagcctcaacgaacgcaatgcgcgcttctggcagctggtgctgctggcggtcatcctggtgggctggcatgtggcgtcgcgcaaccagcagatcgctttttttcttggcgaaccgatccaggtggcagggcgcatctggagctggtttctgccgttcgaggtgccgccgaacctgctgtttcccgagggtctcaagggcaatgcagacatctatcgtcacctgggcaccacgctgctggaaacggtgctggccttcggcattggcaccgtgctcggcctggcgtgcgggctctggctggcgctggcgcccacggcgagcctgatcctcgacccctacatcaaggccgccaattcgatgccgcgtgtgatcctcgcgccgatcttcgcgctgtggttcggcctgggcatctggagcaaggtggccctggccgtcacgctggtgttcttcatcgtgttcttcaacgtctaccagggcgtgcgcgaggtgagcccggtggtgctggccaacgcgaagatgctcggcgccaaccagcggcagttgctgcgcaccgtgtatctgcccagcgccaccagctgggtgttctcgagcctgcacacctcggtggggctggctttcgtcggagcggtggtcggtgaatacctgggctcggcgcgcggcgtgggctacctgatcctccaggccgaaggcaccttcgacgtcaataccgtgtttgccggcatcgtggtgctgacggccttcgcgctgctgctcgacggcctcgtcggcctgatcgaaaaacgcctgatgaagtggcagccgcgcagcggagaaaccgagaagctctagcgctcctcggctcagcgcttcttagcgcttcttctttaccggcgtgccgccgcgcttttcgcgtaccacctgctgttgcttgccggccggcgacttcacgatgttggtgccgcgcgcggccacggcctttgccgtactgccgcctccgcgcttgccggcaacagccgcgtgtccgcgcgccggcgccgcgcccgagcctacgcgagccgcgggtgccgcacgaacaggcaggtacaccaccacgctgtagccgcgcttgaacgagtggttgagattgacgtcgttccactcggccacgctgtccggcttgagcttgtagcggcgcgcgatgctggccacgctgtcgttgcgccccgccttgacggtggtgcggcggttgacgatctcgggttggaagctcaggtggccactgtcggccacgagcgccgtcacgtcctccttgacgcgggcgccgcgcggcacgatgagcgtggagccagccttgatgagcatgcgcggcggaatgctgttgagcgcgcgcagatcggtttcgctcatgcccgagcgttgggccgcatcggccaccgtcatggtgttgggaacgacccatgccgtccagcttgcgtactggccttgcgagtaggcgtcgaagttgcgctggaacacggccgcgttgtcccagggcagcaggatttgcggcgtgccggcggccagcagcacgggcttgtgcgcagcagggttcagggcgcggaaatcttcgagccggatgtcggccagcttggccgccagttcgacgtcgaggtcgcgcgtcagcgtgacggtctggaagtacgggtgattggcgatcagcggcaactcggtgttgaacgcctgcgggttcgcgacgatgttcttcacggcctgcagcttgggcacgtacagccgcgtttcggccggcatggaaagatcgctgtaggtggtgggcaggccgagccgctggttcttggcgatggcgcggctcacgctgccttcaccccagttgtaggccgccagggcaagctgccagtcgccgaacatgccgtagagcttttgcaggtagtcgagcgcggcgcgggtcgaggccaccacgtcgcgcctgtcgtcgcggaagatgttctgcttcaggtcgaagtcggtgccggtggccggcatgaactgccacatgcccgcggcacgcgcgctggagatggcctgcgggttgaacgcgctctcgatgtacggcagcagcgcgagttcggtcggcatgttgcgccgctcgagctcttcgacgatgtggaagatgtatttgttcgagcgctcggtcatgcgctggatgtagtcgggccggctggcataccactgctcgcggtcgcgcaccaggtcgctttggaggttcggcatcttgaagccgcggcggatgcggtcccacatgtcggcgggcggcgccagcgtgaccacgctctgcgagtgggcctcgctgctggtgatgggggtgagggggccgcctggatagaccggcgcggcgctgctcgaagtcttggagccggtgcctcccgcggtaggctgctgcgaggcgggagtcgaagaggaggaagaggacgaagaggggccgctcgtggtgctcgcgcagcccgcgagcaacagtgagccagcaaggcagacagcagcgataagtttcatcggaagtcgtttttccattggcgcagcgcagcaaacacgtcggcttcggccgcattggcggaaagctcggcgtgctcgcgcaccgctctaaggacagtggcttcgcggctgcgaagaaaggggttgattcggcgttcggttgccagttgcgagggcagcgtgggctgcccctgtgcgcgcaggctttcgcagcgcgcggtgtagtgagtcagatcggcattgccgggttccaccgcgtgggcgaaacgcaggttagcaagtgtgtattcgtgggcacagcatacgcgggtgtcgcccggcagcgctgcgagcgcgtcgagcgaggccagcatttgcgcgggcgtgccttcgaacagccggccgcagccgccggagaacagcgtatcgccacagaagagcagtggcgcctggccttcgcctgcaggaagaaagtaggcgatgtggcccgccgtgtggccgggcacgtcgatgaccgcgaagcgcttgccgagcacttcggcgctgtcgccgtgcgagagcggggtgaagggttcgggaatgcgctcgcgcgccgggccgaagaccggtgcaccggtggccgcatgaagcgcagcgacgccgcccgtgtgatcgtgatggtggtgcgtgactagaatcgcggcgagctgcagcttgtcgcgcgtcaacgcgtcgaacaccggttgagcgtcgcccgggtccaccacgatcgcgttggagccgtcctgcagcatccagatgtagttgtcagcgaaggcgggcagcggaacgagggtcatgagcggtcaaattataggtttgcaggattggttcgcgacccctcccggacggtacctcctggggtgggagcaagcccagttcgaccaggcggttgcggacatcttcggctatcacgccttgcagctgggcgccgccggggtcgacgggctgcgtaccaaccgcatgccgcaccgctggctggcgctgcctgagcttgtgcagggcagcaaggctgcgctcttcaccgattttgcggcgctgccgtttgcagccaacagcctggatctggtggtgctgccgcacgcgctggaactgagcgacgacccccatgccacgctgcgggaagtggagcgggttctggtgcccgagggccgcgtggtgatctgcgggctcaacccggccagcctgtggggcatgcggcagcgccgcgcgcacctgtaccgcaagctcgggttcggcgatctctttctgcccgaaggcggcgagttcatcggctactggcgcatgcgggactggctgcggctcctgagcttcgaggtggagtcggggcgctttggcgtctatcggcccgcggtgcgcagcgaagcctggctggagcgctgccgctggatggataccgccggcgagcgctggtggccgattttcggcgccgtgtatttcgtggtggcggtcaagcgggtgcgtggcatgcgcctgttgagcgccgactggcgccgcgccgcggcgcgcgcgacggctccggtgtcgattgcgggcaagatgcacaaggccgaccgcagcgactgaatgaacgaatgatcgatggatcgagagagaaggaaaagatagttttgaacgaagtcgtgatctacaccgatggcgcctgcaaaggcaatcccggccctggcggctggggcgcctggctcaagtcgggtgccactgagaaggaactgttcggtggcgagctagccaccaccaacaaccgcatggaactgacggccgtgatcgagggcctggccgctctcaagcggccctgcaaggtcattctctacctcgacagccagtacgtgcgcatgggcatcaccgagtggatccgcggctggaaagccaagggctggcgcacctcgaccaagcagccggtgaagaacgtcgaactctggcagaaactcgacaagctggtggcggagggcggccacgtcatcgaatggcgatgggtcaagggccactccggcgaccccggcaacgaacgcgcggacatgctcgcgaacaaaggcgtggacaaggcgctgggccgaatctgagcccttgaggagcgcgaagactgggggcgagctaaatgaccccttcgaacatcatcacattgacctcgtcgcccgcagcgacgttgccgtggtcgtgatgcagcaccacgagcccgttggcctcgaccatcgaactcagcacgcccgatccctggttgcccgcaatgcgaacctcgggcagcgcgccggacacggcctgcacgaagccgcgctggtattcggtacggccggccttcttgcggatggcgctcacgctgcgcgcgcgcagcaagggcggcggcgccgcggcgatgtcgtggcatcccatcatgcgcagcagcgccggtcgcacgaaggccagaaaagtcaccatcacggccaccggattgcccggcaggccgaagagcaccgcagagcccggcggcgacgaagaagccggatcgcgcggaaccagcccgaccgccatcggccgccccggacgcatggcgatgcgccagaaggccatgtcgccgagttgctgcatcacggcgcgtgtgtggtccgcggcgccgacgctcacgccgccgctggtgatgatggcgtcagcctggcttgcggcacgctgcagcgtggcggcgagcgtggccgggtcgtcgcgcaccaggcccaggtcgatgacctcgcagcccagccgcgtgagcaggccgaacacggtatagcggttgctgtcgtacacggcgccttcgcgcggcgcctcgccgaggctcaggatctcgtcgccggtcgaaaagtaggccacgcgcagacgccgcagcgcggacaccgcgggcagccccaggcttgcgaccatgccgagcgcggcgggcgacaggcgctcgccgcaccgcaaggccggttgcccctgcatcaggtcctcgcccgcaaagcggcggttgtcgccgcggcgaagcaccttggcgggaaagctcacccggtcgccgtcgaccttgcagaactcttgcggaaccacggtgtcgagcccgtcgggcatgacggcgcccgtcatgatgcgaaccgcttcgccgccagccagggtgccgcgccacgccgccccggccagggccgtgcccaccacgcggaggtcgatggactcgtcggtgcgcgcatcattccgcaggatggcgccgtcgaaggcaaagccgtccatcgcggaattgtcgtgcggcggcacgctgacgggcgagatgatgtcttcggccagcacgcggcccagtgcttcgcgcaccccgacttcctcgcgttccgaaacgatggccggggccgccagctgcgccagaaaagcctggacgccgccgacgctcagggcctgggggtcatagcccgcaagggcggcggcaatgtcggcgatgcggctcatcggttttcgagggcgtgcagttcggccagcgtgttggcgttgaaaaaggcgtcgggcgcatcgccgggccggtcgaaggggacgagcaccgtgcggtgctgcgctgtccaggcgtcgatcttgcggccgccggactgggtgaaggtcaccaggctttcgagcagcgcggtgcgcagcaggcagaacaccggctgaggccgcagcaccggcgccgcgccgggttcgtcagcggcctcgggcgcgctgaccatggcgatctccgcgttgtcggccaccatggcctcggccagacggctggccagatcgagcggaaacagcggggtgtcgcagggcacggtgaggagatagggtgtttcgcagcgttcgaggccggtcagaaagcctgccagcggacccgcgtagtcggccaggctgtcgggccagaccggcacgccgaaggattcgtaggcggccaggttgcggttggcgttgatcatcacctcgcccacctgcatacccaggcgcaacacggcatgcatggccagtggcgagccgttgaagttctgcaggcccttgtcgatgccgcccatgcgcgagcctcgtcctccggccagcagcagcccggtgatctcgctgggggaaatggattcttgtgtggaggtcatccgccgatatagctcatttcgacgcggcgcggcgccttgttgttgtcgttggcgtcgtgctcggcgctgtcggggccgcgaagcgcgcgcagttcggaataacggtcggcgcggccttgccagatgtggccgatggccgaggcaatgtcttcgtcggtggcggtgccgcgcagcaggggccgcaggtcgtggcccgcgctggcaaaaaggcagaggtagagcttgccctcggtagacaggcgagcgcggctgcagtcgtggcagaaggcctgcgtgacgctgctgatcacgccgatttcgccgccgccgtcggcataggcccatctttgggcggtttcgcccggcgcgctgggctcgagcggcacgagcggatactcggcgccgatgcgcgcaatgacctcggccgagggcaatacctcgtccatgcgccagccgttggtggcgcccacgtccatgtattcgatgaagcgcagcaccaccttgccgccatggttgtcgcgaaagtagcgcgccatcggcaggatttcctgctcgttggtgccgcgcttgacgaccatgttcaccttgagcggcccaaggcccgcggccaaggccgcgtcgatcccggcgagcacgtcggccaccggaaaatcgacgtcgttcatgtggcggaacaccgcgtcgtccaggctgtcgaggctcacggtcacgcgctgcaggccggcggcccgcagcgccgccgccttgcgctgcagcagcgagccgttggtggtgagcgtgagcgccagcggttcgccggccggggtgcggagctcggacaactgctcgatcagcccctcgatgttcttgcgcagcaatggctcgccgcctgtgagccggatcttgcgcacgccatgggccgcgaacaggcgcgcgagccgcgtcatttcctcgaagctcagcagcgcgctgtgcggcaggtattggtagtccttgtcgaacacgtccttcggcatgcagtagctgcagcggaagttgcagcggtccgtcacgctgatgcgcaggtcggtcagcgggcggcccaggcggtcgagcaggcgccccgtggcgggcacggcgatctccggcaccgacacggtgggtcgcgcgcggccgatttcggagaccgggatgacggtggtgcttttgcttttcatggggcaacggccaatttactccatggagcaagggccgatccggaaagggctactcgacgggaccgcactttcgacgtctgtctcctgaaaaggggctgcgggcagtgtatcggggcccggcgccgaacgcccccgaagcggccgccgatacggcttcagccgtgcttgatggcgacggtcttgagggtggtgaaaccgtaaagcgcttcgaagcccttttcgcgcccgtagccggacgacttgacgccaccgaacggcagttccacgccgccgcccgcgccgtagttgttgatgaacacctggccgcttcgcacccgcttggccatgcggaactggcgcgccccgtcggccgtccacaccccggcgacgagaccgaactgcgtggcattggcgagcgccaccgcttcgtcttcgtcggcgaactgcattgctgcaagcaccggcccgaacacttcttcttgcgcaagacgatggttgaagggcacgtcgcgcagcagggtgggggcctggtagaagccggtttcgggcgcttcgtcgaccacgacgccgtgggccaccatcgggatcccggccacctgggcgtcgctcaggaaatcccacacgcgctgctgctgcgtctggcggatcagcgggccgacgtcgaggtccatggctgccggcccgacgcgcagggccgtgaaggcgtggcccaggcgctcgagcagcggctcgtagatgccgcgctggatcagcacgcgcgagccggccgagcaggtctggccggcgttctgcacgatggcgttgatgatcaccggaatggccgcgtcgaggtcggcgtcggcaaagatgatctgcgggctcttgccgccgagttcgagcgtgaccgggcaatgccgctcggccgccacctgctggatcaacgtgccgatcttggggctgccggtgaagctgatgtggtcgatgccggggtgccgcgccagcgcgtcgcccacttcatggccgtagcccgtcacgatgttgagtgcgccgggcggaaagccgacttcggccgccagctgcgccacgcggatcagggacaggcaggcgtcttcggccggcttcaccacgcacacattgccggccgccagggcgccgcccacgctgcgcccgaagatctgcatcgggtagttccagggaatgatgtgccccgtgacgccgtgcggctcgcgccaggtgaacacgctgtagccgtcctggtagggaatggtctcgccgtgcagcttgtcgcaggcgccggcatagaactcgaaatagcgcaccagcgccaccgcatcggcgcgcgcctgcttcaccggcttgccgcaatcgcgctgctcgatcagtgcaagctcgtcgacgtgttcggcgatcttctgcgacagcctgtaaagcaggcggccgcggtcggccgcgctcaccttgtgccacacgccatcgaagcaatcgcgcgccgcgcgcacggccgaatcgatgtcggcggcattgctgcgctggatgtcgtcgaaaggctggccgtcggacggatcgagcacttgcagggtgcggccggaggaagacgggacgtcggcgttggcaatgaagttgagttgcatggaacggattttgcgcgaagcggggcagccacgccgcgcgcgctcctgctcctacctgggcgaacgcgttcgcggcagcgcccgcaccgcattcagcatgcgctccacatgcttgtccggattcaggttctggtagtagtacgccaccttgccgtccggggaaatcacgtacgagagacggttggcgaagtccggccgggtttgcatcagggcgtcgaaaccgttgatcaccgccttcgattcgtccgacgccacgggaaaccggctttggcaggacttgaccgaaaacttcgcgagggtttcgatgtcgtcggccgacacgccgatgacggtggcacccagcgcggcgaactggtcgatggcttcggcgaaggcatgggcttcgatcgaacagtcgttggagtcggctgccggaaagaagtacaacaccaccgggcccttggccagcgcatcggccagcgaatagcggaaggtcttgccggcgagcgcggcattggcggtgaacttgggcaccggatcgccgatgtccagggcggccgaggcggggagtgccagcccggctgtgaccagcatcggtgcgatgcgtgagaggatcggtcttgccatggtgtaactccggacaggtgtagaacgaattctaggacggtgagccagttttttggattgcagtccggatgaaaccgaaaccgacatgtactggcgcgcgtacccatggcagggagcccaaaaacaagcaggtctgcgagatcgatccatcatgaatgcctggacacaacttctgcgaatctgcctggccggcgccatgctcgcggcgctggcggcctgcggctcgctacccccagcgcgcgaacgggcggcggtgaatgcgaccgcggtcgatccgaccaccacgctcgcaaagatcgcagcggcctcgacgccgcccggcgagcactccggcttccggctgatgccgctcggcgtctattcgctggacgcgcgcgtgcagcttgcgcaacgcgcccagcgctcgctggtggtgcagtattaccagttcgaaaacgacgccaccggacgccttttgatgcgcacgctgcgcgaggctggcgcgcgcggggtgcaggtgcggctgctggtggacgatctctacaccgccaagagccagcagctgctgttggcgctttcgcagacgcccaacgtggacgtgcggctgttcaatcccttctgttgtgggcgcaatggtttcctgtcgcgctttgcggcgtcgccgcacgagatcgggcggctcaaccaccggatgcacaacaagctcttcatcgccgatggggtgatggcggtggtcggcgggcgcaacattgcagacgaatattttgtgctgagcgaggcgcagaacttcatcgacatggacgcgctggtggttggcaaggtgctgccgcagctcgagtcgattttcgatgcctactggaacagcgagcaggtctggcccgttgccgacatcgtccgcggcgagggcggccgcacgcccacggccgccgacttcgacgccacgatcggcatggcggcagcgccgccgaagatcgtgcttccgccttccgacgtcctgggctatggcccgattgcggaagaactcgacggtggccgcatggggcttttgtggggcgaggcccacgccatcgccgatccgccgaccaagccgaccaccatgacggcggacgaggccattgccaccagcgtgacgatgaaggtctggacgctgttgatggatgccaagttcgaagtcgacctgacttctccctacctggtgccgggcgagcgcggcatggcggcgttcgaagatctggccaagcgcaaggtcaagctcacgctgctgaccaattcgctggcggccaacgacgagccgttggtgcataccggctatgcgcgctaccgcgagcggatgctcaggagcggggccgacctgtacgagctgagcccgcagcgcaccaccgcgggcgagcgcttcggcatgttcggcaaatcgctgggacggctgcactccaagaccgctgccatcgacaagacgcgcattttcatcggctcgatgaacctcgatccgcgctcggcgagccagaacaccgagatgggcgtggtggtcgacagtccgcagctggcgcgggagatgctgcgcgtcatcaacatcagcaagctgcagaactcgtatcgtctgcgcctcgccaaggaaaccggcacgctgcagtggctcacgaacgatggcgagaaagaagtcatcctgacgtcggagccggaatcgagcttcttccaacgtctccacaacctgctcattgcgccgctggttcccgaaatgctgctgtagcctcgggggatggcgcaaacctttacttcgttgtccgccctccaggtgatgttgtgggggttggtctttttcggcggcatctatctggggttcggcgctctcaattggctgctgacccatcgcgtgctgccggcgctcggcatcgggcgcgtgctcgacccgcggccgctgcagccggggcaggtgcgccgcgaattggcgcagtcgggggtgtcggtgctcgtattcgggctgggcatggtgttcccctggggcctgcttcaactgggctgggcgcggctcgacgccgacgcgggttggcgccagatcggggccgaagtcctggtgctcgcgatctggaacgacgttcacttctggctcaaccatcgcctgctgcacacgcgctggctgcggcgctttcacgggccgcatcaccgctcggtcgtgaccacgccctgggcgacgtacagctttcatccgatcgaggcggcgatgctcggcaacgtgatcctgctgccgatgctgctgcacgatttcagcttctggtcgcttgcctcggtgccgcttttcagcctgttcttcaacagcgtcgggcattcgaactacgacttctttccccgggtctcttacagccattggtttgctgccagccgccgccaccatttgcaccatgcctgccacggcggcaactacggattccagttcacgttcatggaccggctgttcggcacgcgcattgccgccgatgcggcggagccgcagttccaggcatttcgctcaaaacggcaaccccagcaagagcatggcacgccggcctgaggggccccgtcggctggcacggctgcgccatgggcgcgactggcagagccttgcgtatctggcggcgctcccggcattggcggcatggcaatggatgcatggcttctccgtgctgctttatgggccgatgctgttcctcacgcttggcgtgggtgtgatccaccacaaccacgtgcatctgcgcatgtggcgggggcggcgcatgaaccggctcaccgacttctggatcacgctgctgcagggacacccgaccttcgttttctggcctgcgcacgtggccaatcaccatcgccaccggcacgggccgcgggacgtggcgcgcacctaccgctttggtggcgacaccaatcatttgcggggttacctgctgcatccgttccaggccgtgtgggtgctggtgccggtgttctgcggttggctcgggcggcttcgcaggcaccggccgggcccgtggcgctactgcatggcgcagtacgcgctgtggctcggcagctggagcgcgctgctgatgctcgactggcgcaaggccctgctgttggtgatcttgccgcagttgcacgggttgcactggctgctggcgaccaactatctgcagcacgcgcacgccgacggacgccggtccgcggcggatgcggaggcgccgcgcgataccgcaggtacccgcctgaactacgcacgtaatttcgaggggctggtgaacccgttgctgttcaacatcggcctgcacaccgcacatcacgagaacccgcatgtccattggtccgagctcacgcaattgcaccgcacgcgctaccgcgcgcgggtcgatcccgcgctcaacgagcaagggctggtgccctacatggttcgcgtgttcgtgctgggcgccctgtggccgcgttttcgcagccgctcgctgatgtcacccgtgccgtccgtgtcgccggagtcttcaacccactgaaccatgcctgttccatttcaacgcgtctacatcgagagcgccggctatttcatgcctggcgagcccattcccaacgagcgcatggacgcctacatcgcgccgctcaaccgcatgtcggagcgcatcaagcggcgcatcctggccgagaacggcatcctcacgcggcactatgcgatcgacgaagagggcgtgacgcgccacaccaatgcgcaactggccgcaggcgcgattcgcgattgcctgcagcgcggcggagccgagctgtcgcgcgtgtcgctgctggccagcggatcttcgggcggcgatacgctgatgccgggctttgccaacatgatccagggcgagctggcggcgccgccaatggaaacgctgtcggtgcacggcatctgcgccgcgggcgtgtcggccatccagtcggccgcgcagggcatcgaactgggcgcgcaccgcactgcgctcgcggtggccagcgaaatgccgtcgcgccttttcaagcgctcgcgctttgcggcgcgcggttacgaaaccgacttcgattcgcactttcttcgctggatgctttccgacggcgcgggcgcactgctgctgtccgacggcaggcccgcgctggctggcaacccggggctgcgcctgaggctgaaatgggtgcaccagcgcgcgttctcgggcgactaccccgtgtgcatgcagttggggctgaccgaggaccgcgcccgcggccatctcgatttcggctcctgggccgaggcggaggcggccggcgccctgtcgctgcggcaggacattcgcctgctgccgcatctgttcgacatcggcatccatgaatacgcgacgctggtgcgagacggatgggtcgatccgaagcgggtcgaccatttcctgtgccactactcgtcggaaaaattcattccggtggtcgaagacctgatgaccaaggccgatctcgcaattccccgcgagcggtggtggagcaatctggcctggcgcggcaataccggtgcggcgtcgatcctgatcatgctgtcggaatttctgcattccaagacgctgaagcctggagagcagatcttctgctacgtaccggaatcggggcgcttcatggccgcctacatgctgctggaggtcgaggcatccgatgcgcctgctcgggcggtggccgtatctcacaagacggccgaggcagcgcccgaagacgagacagcaattgcgccgccgcacgatccggccgccgcgcctgaaggcctgggcgcactgctgaccgaactggccggcatctggcacgactaccgctcgaacgtctggcgcacgccgctgatccgccagatccgcgagcgccgttttgcagcgcccgactacctgaactggatggagcaatgggttccgcaggtgcgcgaaggcagccgctggatgcgcgaaggcgccgcttcgctgaccggtccatacaagacgctcgccgcactgatcgacgtgcatgcgggcgaggagcaggacgacttcaacattctcttcagcgactacaggaaagcgggcggcaccgtggcgcggatcgacgacctgcgccgcaaccccggcggggaggcgctcaatgcctacctgcacgggctggcggccacgcgcgaccccatcggcctgctgggtgccatctacatcatcgaaggaacgggccagcgcatcgtgcccgcgctgctgccactcatcaaggccggcctgaagctgccgcccgatgcattccgctttctcgagtaccacggccacaacgacgagaaccacctgaatcgctggctcgccgcggtcgagatggtgatggcggtggaggcaggcaaagaaggtcaagacgccaccggacggggcagggcggcccgccagatcatcgatacagcgcgccatacggcggcgctgtacctgatgcagtttcagcacatcacggagcgaatgccacatgagccgaatgcctgatttcctcacgcaggggcacgacgagcgcgatcccagtccctggctcgcgctctatctcgaccagagcacgccgctgccggacgaggtcaaggcggcatggctcgccgattccagttcgggttcgcgccagtacctgctgccgttcctgcggccggtggcgcggctgacgatcgtcctgatccaggtggtcaaggtgttcgtgccgcgcaactggtcgcattcgaagctgctgcaccggctgctggcctgggggctgaaacgctttgtgtcgccagaggccaactggctgatcctgcggcactttcacctggggtcgcaggtcctgggcttcatcggtcgcaattcgcccgcgccggtgggcacctcgccgctggagccggccgacatcgatgcgctcaaggacgagatgttcctgaagcacgacctgaacctcttcaacttcgtgattcgcctcaaccaggcgctgcgcgacaaggggctggtgctgggcaaggcgccggctgtcgacttttcgatgatcaaggaccctgggttgcggctatcggacatgccgcacggccggctcaactttctggacctgcagagcgccatcgaattgttcacgccgctgtaccagctgatgttgacggacaacgacttctggcgcgccgccaattccctgcaactggatgaaaccatcggcatctacgcggccaccctgctcggtgccccggagcacctgatcctggtgaacaacaagcatccgctggtaccgctgtcgaccctgcgcgccggccaccggctggtgattcacgggctgtcgacagaaatgctccacagcctgcttcagcgcatgcggactgcccaggagacggccccacggccggagcagccacttgcataggcgtatgctgcccccagatgcaaaccatgaacacgaccgaccatccgtctcccaagaccgatctggcagtgacccacgtgctggctcagctgctggaacggctcgagcacagcgccgttcccgtcagcgccgagcaataccgctcggtggtcgagcacctggtgcacgaattcagcgacgtcgaaccgggcgccgacctgggccgcctgctcgatgcgtacccggccgcggccgaggtgtacgaaaatctcaattaccagcatgccggcctgtgccgctcggcgctcgatgcggcacttgcagccgaagtcagcgccaggaaagccattgaacgcgcgatgcgcaataccgaacccaaaaaggataaagccgatggccaaagctgaggtcaagaccgccgttgtggccgacggcctgcgttacaagtcaaaaacacccggttcgccgttccgcgcttcggcgtcgttcagcggcgcgaccatgtcctgcttcatgtgcggaaaacaccgggtgcgctcgcaactgcgtacccgccaggtgcttggcaagtcgcagacggtgtgcgcgccttcgtgcaaggcgctcgacgaatcgctcgaataaatcgaacttcgtccctcgacaggtcccgcgtcgcttttgcgacatgccctgcgcgcgcattgcagattttctttccaaagcgcctgaaatcgatatacagttagaaacatatgatgcatttaattgcatagataaatagttctaatttgtagtcgacgacaaatgattttgtacacaggcaatgacgtccagcgccggacgatctgcggaaggacttgcaatgagtaagccgcgtcatgtcgtgatgcaggtggtcaagcgctcctctggcagcgcaacgcaccacgtcgaattcctcatggacgacaactttgccgagcgcctgcgccaactgcgctcgctggttccgcctctcggcagcctcaacaaacagcgcgacctggtgatcgacaaggtgcgtgtgaggcttccgaacgccatttggcgcaccgggagccaagtcgacaatggcgtggaaggctcctgtatcgtcattgcctctgagggctctttcaattgcggcggcaaagaccgcaacacgcgcgaaaagctcgtgacctacaacttctcaatttcgcgcctcgtcgaccttcataccgagcgcccggagggcgagaccctctatatccgtgatggcaccttcgccaacgacgagcctgccgattcgcctgcaggcctgtgggtggcctcgttgaccgaggaggaggtggtgatgcgcgtgccggatgcgccgtccgacttcgacaccctgcacgaactgacgctgcggcccgagcagcgcgccggcgccggcgcgtccacgcaccgagccaccttttactgaagcgcggcggctgcctcggtagccgagcccacgggcgtgtactgcgcacggttgtcctcgagccagcgggccgaaaggctgctgtcctgctgcgccggatggaaatcggcgcggaaatagctgcgccaagcgctccagttgccttgaaagaggccgccccggccgagcagaatgcgcgcggcactcctccaggtcgcccatttccacaactgcccttcatggcgcaggttggcggctgtctgccgcatcaaatcgcccaggaacatgagcgtcacgcggcgaaaccatcggttgcgccatgggtccgagccccctgcggccttgtagaggtcgaaggcgacggccttgtgctccagctcctcggcgctgtgccaaagccacatggtccgcagccgcggttcggcgccttcgagcacttgggggtgggccagcagccattcggcgaacatggccgtgaagtgctccgtggccgcggtcactgccagtgcgtggcgagggtcggcgccttccatgagttgcatgcgcctggccgcccgtggcgaccagccatccttcaagccctggttctcgagatgcccgttgaaaagcgaatggatgcggcgatgcgtggcttcctggccgatgaagccgcgtacgtcggcgcggtatttttcctgcgcctccggcggcagcgtggccatgacgtcgcgcaccgcgtcgatgaagaactgctcgccgaacggaaagctcatcgacagcgcattgaagaaggcagtcgagaatgaatcgccgccgcaccagttgcggccgaacggcgtttgcagatcgatcagaaggcggcgcacgacaaggtcggtcatgaaagaagtcctcgaggaactgagttggtacacattcgtaccgattgacggcatggtgcgcacaacactcggtaccgtcaagtaccaatgcgtaggaaaatgtgccatccatgaacacagcaactgaaaacccggcagtggccagctcttccgcaccaccggcgcacgagcactattcccgactgctggaaggcatggcgcgcgcggtggcggccaagggctacgcggacacgaccatcgccgatatcgtgcgcgaggcggccgtttcgcggcgcaccttctacgagcatttcacgaccaaggccgaatgcctggtttcgctttacgaggctgccagcaagcgggcgctgcgggctgttgccgaggccttcgatccggcgcaaccctggcaccggcaagtggagcaggccatgacggcgtacctcgactatctggcgcaggatccggtgctcctgcgtacgctcttcgtcgagatactgggcctcggaatgcccgggcttgtggcgcggcgccgggtgaacgccgaaatcgccagcttcatccaggtggccatcaacagcagcagcaacaacggtgcgcagggccccgccgcgcacctgacaagcgaaatggccctgacggtcgtgggcggcatcaacgaactggtgctccaggccatcgagcaggaccgcatgggcgatctgcgccagctggtatctccggccacgcgcctggtgcgcgcggtggcggccgaaagcctcgggtagcgcgccgggtggcgcagggcagggcggtcttcgaacccgcgcttccgatcaggccggtttgctttgcgcgggatcgtagaagaactcttcctgggcgatgcggtctcccgcccagcgctgccacgcgagctcttccatgcgcatggccttgccgcccttgaaccggaaatcgaaaacccagcggatcaccacgtggtccccgttcacgaacacggggcgcacgcaggtcgagacgacagattcgacgcggtcgagcaccgcctgctcgtgggcgaccagggtgccgcggccgcgccggggctcggcctggttttcgcgcatggtcgcgtcttcggtgtagtagttctcgatggccttggcatgcgcgccgctttccaccgcggcgatgaaggcctcgagtctttccgcggaaggcatcagctcttgaccttcacttcgacccggcgggcttcgctcgccggccctgcggcctgggtttgttcgggcttggcaagctcgaccttgtcagcgggtgcaccggcggccttgagcgcatcgccgaccgcgactgcgcgctgcttggccagctcggcgttcgccgccgcatcgccgctggcatcgtgatagccgctcacgagcaccgtgctgccgctctgcacggccttgatcacgtcggccagcgcctctttggcattgggcgcgacctcggccttgccgctctcgaaatagaacttcaccacgccgttctcgaccttcacggccgcgccttcggccgccgccacggggcctgaagccaccgatgccgcgggtgggaccggggtggaggcctgtaccggggccggcgccggcgcgacggaggccgccggtgcggtggcggccgggggcgtctcgatcttgtgcggtacggctgcgcccgcgtcgccggcgtggaacttgaccaccagcggcacgatcagcagcgccacgatgttgatgatcttgatgagcgggttcacggccgggccggccgtgtccttgtaggggtcgcccacggtgtcgccggtgacggcggccttgtgcgcctcggagcccttgccgccgtggtggccgtcctcgatgaacttcttggcgttgtcccatgcgccgccgccggtgcacatcgaaatggcgacgaacaggccggtgacgatggtgcccatcagcaggccgcccagcgccttgggtccgagcacgaggccgacgacgatcggcaccaccaccggcagcagcgacggaatcatcatttccttgatggccgcgcctgtcagcatgctcacggccttgccgtactccggcttgccggtgccttccatgatgccggggatctcgcggaactgtcggcgcacttcctcgaccacggcaccggccgcgcggcccacggcttccatggccatggcgccgaacaggtaggggatcagcccgccgatgaagaggccgacgatcaccatcgggtcgctcaggttgaagctgatgttcaacccgaagctctccagcttgtgggtgtagtctgcaaagagcaccagcgaggcgaggccggccgagccgatggcgtagcccttggtcacggccttggtggtgttgccgactgcgtcgagcgggtcggtgatgtcgcgcacgctggcgggcatctcgctcatctcggcgatgccgccggcgttgtcggtgatggggccgtaggcgtcgagcgccaccacgatgcccgccatgctgagcatggccgtcgcagccaccgcaatgccgaacaggcccgccagcgtgtacgaggccatgatggcgatgcagacgaagatcaccggccaggctgtagagcgcatcgagacgccgaggcccgcgatgatgttggtgccgtggcccgtggtcgaggcctgcgcaatgtgctgcaccggcttgtactgggtgccggtgtagtactcggtgatccacaccagggcggccgtgagcgcaaggcccacgaagcaggcgccgaacagcttgagctggctgccgctcggggcaatggcgttgtcggggatgagccagctcgtgacgaaccagaacgcgatcagcgacaggatgcccgccaccgccaggcccttgtagagcgccggcatcacgttgaccatgccgggcgaggccttgacgaagaagcagccgatgatcgaggcgatgatcgacacgccgcccagagccagcgggtagagcaccgcgttgactggcgccgccgtgaccatcagcgcacccagcaccatggtggcgatgagcgtgaccgcgtaggtctcgaacaggtcggccgccatgccggcgcagtcgccgacgttgtcgcccacgttgtccgcgatcacggcggggttgcgcggatcgtcttcgggaatgcccgcttcgaccttgcccaccaggtcggcgcccacgtcggcgcccttggtgaagataccgccgcccagccgcgcgaagatcgagatcagcgaggagccgaaggcaaagccgatcagcgggttgaggatgttcgaaaggctgcggtccggcgtgaggttgccgttgcccgccaggaaccagtagaagaccgaaacgcccaggagccccaggcccaccaccagcatgccggtgatggcgccgccgcgaaacgcgacgtcgagcgccgggccgatgccttgcgtggccgcctgcgcggtgcgcacgttggcgcgcaccgacacgttcatgccgatgaacccgcaggcgcccgagagcaccgcacccaccacgaagccgacggccgtggtcacgtcgagaaagatggcaatgaggatggccagcaccaggccgaccaccgcgatggtggtgtattgcttggcgaggtaggcggaggcgccggcctggatggccgccgcgatttcctgcattcgcggattgccggggtccttggcgagaatccaacttcgtgcccagaaaccgtagccgacggccacgaggccgcagacgatggcgagtatcaggggggtgttgccgatcatgctttgcttctccattcgttcgttgtgacttgtggagacggacagcatggatcctgcgcgcaacgcgtacgggacccaggttttccgtcgcgttgcttcctcgaagctcgctgcaccgaagtgcggagccgattggccaacggttgcaatttacaggcaaaagcgcgggcgtgtgcgaccgcgccatgacacggaaagtaaactccgggtttgtccccatctcccctcatacttttcaactactcgaaaacgtcatgtccttcgacaaagtctcccccggtaaaaacatccccgacgccttcaatgtcgtgatcgaaatcccgatgaacgccgacccgatcaagtacgaagtcgacaaggaatcgggcgcgatcttcgtggaccgcttcatgacgactgcgatgtactacccggccaactacggctatgtgccgcagacgctgtctggcgacggcgacccggtcgacgtgctggtgatcgcgccgtatccgctcttgcccggcgtcgtggtgccgtgccgcccgctcggcatcctgatgatggaagacgaagccggcgtggacggcaaggtgctggccgtgcccaccgacaaggtgctgccgatctacagccactggaagtcggtcgacgacgtgaacccgatgcgcctgaaggccatcagccacttcttcgagcactacaaggacctggaagcgggcaagtgggtcaaggtgctgggctgggaaggcatcgacgcggccaagaaggaagtcatcgacggcatcgctgcctacaagaagtaaaaaacagttccgtgcgaaacatgggccaggggcagcggtgcctcagccctgaaccgcatcgcccgccagccgcatccactcgcggttgacggagcgggcgtgcgagttccagtggcgcgcggcctgctggagttcgctccactggcgctgtgcgccggcggcgtcgccttgctgggcgagccaggcaatgtagcgggcacgggtctcgaccgtgttgtactggcttagcgccgcctcgaaggcctcccgcgcctccccgtggcgcccatcggcggcgagtgctcgggcggtgagcacggccacctcgtccctgcggtagtcgccgcgcgtggcgcgcagggcctggagcgcttgcagcgcttcgcggccagaagccgggccacccgccgccagcagtgcgctggccaggccaaactgcagttcaggatcggacgcgagcgggcccttcagggcgtcgcggtagtgcccagccgcgtcggcggcctggcccttgtcgagcgcggccttggcgaggcgcagcttgttctgggccgtcggtgcgaggtcgtaggcttcggtggccgcgcggtattcgcgctcggggtcgatgaagccgatggctgcactcgccaccttgcccgcggtgcgctgcatgcgcgaggcgggcaggtactcgaccacgaaatacacgatgctgcccaacagggggaagctgaaaagaatgatgagccagtacatctgcttgccatggcgcatcgcgtgtaccgcgaagaacagcgcaatgaggatgtgcagccccaatccgacgaatggcatcgacttctttctgttgttggatgttgggcgcgtttatagcagcccctgatggcgccaaaccgactgcgatccgcctctcaaccggccttgaaggggctgcgttcgcccaggtggtccaggtagttttcgataccttcgccttcgcgctccagaaagcgctcgaccgcgtcggcgaacgcggggtgcgcgagccaatgggcactggtggtcttcaccggcatcaatgcgcgggccatcttgtgctcgccctgcgcgccaccctcgaatcgcttggcgccgtgcgcaatgcaccaggcaaggggctggtagtagcacgcgtcgaaatgcaggcagtcgacgcgttcaatggcgccccagtagcggccgtaggcgaccagcgcgtcgtccgcgtgcgtggacagcgcgatcaggctcgtggcaatgggcttgcccgcgcgttcggcgacgaacagcagccaggcttcgggcatggtgtcggccatgcgctggaagaaatcgcgcgaaagatagggcggattgccatgctcgcgataggtgcgtgcatagcagcggtagaaaaaatcccagtccgtcggcgtgatgtcggcaccgcgggaccagcgaaaagtcacgccggcctcggccaccttgcggcgctcctggcggatcttcttgcgcttgtcgtgggacaggctggcaaggaacgattcgaagtccgcgtaaccggtggttccgcccggcgcctgctggaccgcgttcatccagtgaaactgcaccgtgttgcgcagcatcaggcccgcttcggtgcaggcggcgatgtcggcgtctgcaccgaacagcaggtgcagcgatgaaagttcttcctgcttgcaccaggccaccaatgcttgcaccagcagtgtgcgggcctgcgcgtcgcgtgccagcaatcgcgcgccgggcaccggcgtgaacggcactgccaccaccgccttgggatagtaggcaagcccatgctgctcgtaagcattggcccaggcccagtcgaagacgtattcgccataggagtgggtcttgatgtacgccggacaggcggcctgcagctcttcgccgcgccacagggtgatgaattgcggggtccatccgctctcgggcgaggcgctgccgctctcctgcattgccgcgaggtattcgtagcgcatgaaaggcgacggctcggcttcggccgagagcagcgcgttccatgctttcgggctcaggtccgacagcgacgccatcacccgaatgacataatcgttcaagtctttttcttccttccgtatgacgctcacgctcgccatggcgcaactcgattttgtggtgggcgactcggccggcaccttcaccggagcctccgatgatgccgtgaaagccgagacccccggcggcgtgctggcacgctacatgcaggacgatgagggcatcgacgagatcatcgccgcgggctacaaacgcgcggtggtcgagcgggttgcgcggctcatcaagatcaatgaatacaaacggcgccatgcgccagtgggcatccgggtcacccatcggagcttcggcaaggattggcgttaccctatcaccagcaaattcaacgaaaccgccggagcgcaaaaaccatgaagcagatcaccgccatcgtcaaacccttcaagctcgaggacgtgcgcgaagccttggccgaagtgggcgttaccggtctcactgtgaccgaagtgaaaggtttcggccgccagaaaggccacacggagctctatcgcggtgccgagtacgtggtcgacttcctgccgaagatgaaggtcgaagtggtcgtcaacgaggacgacgtggaacgctgcatcgaggccatcgtcaattccgcgcgcaccggcaagatcggcgacggaaagatcttcgtcaccagcgtggaccgcatcgtgcgcatccgcaccggcgaagagaacgaaaacgccgtctgacggctcgcccccagtcttcgcgcacttcgtgtcgcttcgccaaccccctaccaggggcaacatcagcggcccggcaaagccggttccgcggtgtttccggaaagaggcaggtctgcctgactgccgggctacaggttttcggccagtttgttgccgcggggatggagcggcacttcggcgcgcagcgcactgagcagttcggtggggtcggtgccggtacggaccaactccatctgccattcacccatgaagccttcgcgcacgctgtgcgcgaggaagcccagcaaaccgtcgtagtagccggcggtgttcaggatgccggtgggcttgtcgtggtagccgagctggcgccaggtccagatctcgaacaattcctcgaaggtgcctatgccgcccggtaaagcaatgaaagcatcggcgcgttcgcccatcatggccttgcgctcatgcatggtgtcgaccacgtggagttcgtcgcacagcgggttggccagctcccggtcgaccagggccttgggaatgatgccgacgacgcggccgccggcattgcgcgtggcctcggccacggtacccatcagcccggtgcgtccgccgccgtagaccagctggccgcggtgcgcgccgatccactggccgaccgcttccgcggccttggaaaactcggcccgctcgccggggcgcgagccgcaatacacacagatcgaaaattcaggattcatgccgccatcatgcctcgtgcggcgggcgtcttcatgacgcgaagtgctgccacagagccgccagccagatgccgccgcacagggtgagcgacaacaagacggcggcgctgcccatgtccttggcgcgcttggagagatcgtgccattcgggcccgatgcggtcgatggcggcttcgaccgcggtgttgagcagctcgacgatcatcaccaggatggcgctgccggcgagcagggccacttcgacccagctgcggccgagccagaacgacgccggaatcatcacgatcgccatcacggcttcctggcggaaggccggctcgctccagcccgcgcgaagcccatgcagggaaatcagcgtggcatgccacacgcgctccaggcctttgcgggccttttgcgggttgacggcgggatctggaagcttgggcaaggcactcattggcggctcatgggcttggaggtgatgagccgcgtaccggcccaggcgtcgtgccagaactggcgctcggggtggaagcgcgccagcaatgcccagatggcgacccatccgaagatcagcaccgccgattctcctcccgacagcttgaaaggtgcgatggccgccaagggcggcaggaaccagatccagctcagcaggtagcgcgccagggcgcggcgctgggtgagcgggcgtccgtgcaggtcgacgatgcggatgttccaggtcttcatggccagcgtctgtccccgggtccagaaccagacgaagtagacgccgaaaaccacgaagagaaacgcctggagcaggtgccggcgggagtccatggcatcgcgcatctgcccaagcgtgctgaacagccagcccgcgacaaacaccacggcgaacagcagcatgccttcatacagccagcacgccattcggcgccacaggccgggcactatcgaaagaggagcgtcgcctgaagattctgcggacgaagaaggaggattcgattccgaactctcggaagcatttgaaaccatcgaaaccttgggaatcaggggggcgaaggctgctcggcgcggcctgcaggattggaaggcgatgggccggcggcagacggtggtaccagcacctgagcctcggccgggggagccggctgcggcgccacgctggaggcggcaggtgccgacacaatggccggaacccgctccggcggcgacgccaccatgacggcggccgcaggcgccgttgcgggcacagccgaagggggcggggccagcatgatgcggggcgtgtgctgccccgcaggcgtcacggccggcaccgtcacgagcttctgggagggaatggggcgcaccggaatggcggccccgcgcggcttggcgggcgcgcgctctgcgagacggcgcttttcttcctcgctcaatgcctggtattgctcccacttggccttgcgctcgtcggcaggaacgcgcttgacctcggcaaagttgaggcgagcctgggcgcgctgctggttgctgagggcggcccattcgatcatgcggctgtgcaaagtggttcggtcatcggccgacatgttcgcgtagttgcgtgacagtgccagccatttgcgcttgtggcccgcattcagggtgtgccaatgcgatgcgagcgggtgcagcgcctgctgctgctccgcggtgagctcgctccagtagggtttggttgcctttggcacggaggggttggaggcggccaccggcgcaggctgggcagtctcggccggcttggctgacaaggattgggtctgggcgctggccagcgtcaggccgaacgccgcagcagcgagcgcgaacgcccaaatgactgcgcccgacgtttgcgggcgcagcaggcgggacgcgtcggtgcgggaaacggaagtgcgtcgcatgcgttcggcgggatttcagtcggaggcgccgtcagccttaaccttgaggaactgcgcgaaccccgggtccgtgtaggcggcgggcgggaggtcgtccgtcagaagggccgagtcgacttccgccaactcgctggcacggtcttcgtcctgcatcacgctgatggtgatgaggcccgcgaccagcgcgatcagaggcaccaccgagccgatgcgcgtccaccagccgccgcccatggtggccacatgcccggactgcatgatgaccgtggccgcccgcaactgaggggcttgcttgcgcatggcgacggcttgcgcccgcgccacgcgcagccgctcgccgatgtcgtgcggcagctcctgggtgccggcggaaagccgcgcagccacccgctggccgaattgatcttcgacggcgaaagaagaggttggaaccttagtgttcatagcgaaattcccttggctttgagcgccttgctcagggcgtgtacggcccgcgaacaatgggttttgacgctgccttcggagcagcccattgcagcggccgtctccgccacatccatttcttcccaataacgcatcaggaaagcctcgcgttgacgtcccggcaaagcggcgatctgttcttcgatctcgtggaacacctgggcgcgtcgggtcgtgtcttccgcgctctccgtttccctagagtcggttggcgagacgaagttctccagaagatcgaaatcgccttcgtcgccagcggcctcgaagtcgccaaggttcgagaacagggcgcggcgggttttctgccggcggaaccagtcgagcgtgcaattcgaaagaatgcgctggaacagcatcggcagctcttccggcggtttgtcgccgtagtgctgcgccagtttcatcatgctgtcctgcacgatgtcgagtgccgcttcctcgtcccgcacgtgatagaccgagcgcttgaaagcgcgccgttcgacgctcttcagaaagtcggaaagttcttgttcagtggccaagcgagagggggcgccacaggcgccgcgtgggaaatggtgtctgggtagcgcttgtgtttttctgccgcggattatgccccggtgccttttcgcggggatttcggcgcggcggccgccgcatcaatgtcataattcgcgctgcaagtcaaaaggcaaacgggtcacggtccggcggaacatcagtccgctcatggctttggcctcaagtcctggcgcggccccacaagggctggcaaggggcacccaaggtttttcgttcccgaaaaaactccaaaggttgatcatggaaatctctaaggcggaactcgcttccgcagcagccgcgtcctctggcgccggcaacccaacgcaagaactcatgggcgctgaagtgctggtcaaggcactgcaggccgaaggcgtccagtacgtctggggctaccctggcggcgcggttctgtacatctacgacgcgttctacaagcaggacaccatccagcacgtgctggtgcgccacgagcaggcggccgtccacgcggccgacggctatgcgcgcgccaccggcgacgtcggcgtggcgctggtcacgtccggacctggcctgaccaatgcggtcaccggcatcgccacggcgtacatggactcgatcccgatggtgatcatctcgggccaggtacccactgcggcgatcggccttgatgccttccaggaatgcgacaccgtgggcatcacgcgccccatcgtgaagcacaacttcctcgtcaaggatcccaaggatctggccatgacgatgaaaaaggccttccacatcgcacgcagcggccggccgggcccggtggtggtggacgtgcccaaggacgtctccttcaagaagacgccgtacgccggctatcccgacaaggtcgagatgcgttcgtacaacccggtgcgcaaaggccatggcgggcagatccgcaaggcgttgcaactgttgctcaacgccaagcgtccttacatctacacgggcggcggcgtgctgctcggcaacgcctgcaacgaactgcgcacgctggtcgacatgctaggctacccggtcaccaacacgctgatgggcctgggcgcctatccggcgagcgaccgcaagttcctgggcatgctgggcatgcacggcaccatcgaggccaacaacgcgatgcagaactgcgacgtgctgctggccgtgggcgcgcgcttcgacgaccgcgtgatcggcaacccgaagcacttcgcgctgaacgaccgcaagatcatccacgtcgacatcgacccgtcgagcatttccaagcgcgtgaaggtcgacattccgatcgtcggcgacgtgaaggacgtgctgaccgagctgatctcgatgatccgcgagagcaccaccaagcccgatgccggcgcgctggccgactggtggaagaccatcgaggcctggcgctcgcgcgactgcctcaagtacgaccgcggcaacaaggacgtgatcaagccgcagtacgtggtcgagaccctctggaacatgaccaaggacgccgacgtgtacatcacgtcggacgtgggccagcaccagatgtgggccgcgcagtactaccgcttcgacgagccgcgccgctggatcaactcgggcggcctgggcaccatgggcgtgggcattccctacgccatgggcatcaagctcgcgaagcccgattcggaagtgttcaccatcacgggcgaaggttcggtgcagatgtgcatccaggaactctccacctgcctgcagtacaacacgccgatcaagatctgctcgctcaacaaccgctacctgggcatggtgcgccagtggcaggagatcgaatactccggccgctacagccacagctacatggatgcgctccccaatttcgtgaagctcgccgaggcctatggccacgtgggcatgctgatcgagcgtccacaagacgtggagccggcgctgcgcgaagcacgcaagctcaaggaccgcacggtgttcatggatttccgtaccgatcccaccgagaacgtgttcccgatggtcaaggccggcatgggcatcaccgagatgctgttgggtgccgaagatctctgatccgcggcgcattcgcttaactctttactgacgaatctattgaccgccaagcccgcgcattaccgtgcacgggggagggcggcgaaaagaggagtcacgcaaacatgaaacacatcattgcagtgctgctggaaaacgagccgggtgctctttcccgcgtggtgggccttttttcggcccgcggctacaacatcgaatcgctgaccgtcgcgccgaccgaggacccgagcctctcgcgcatgaccatcgtcaccgccggctcggacgacgtgatcgaacagatcaccaagcacctcaaccgtctgatcgaagtggtcaaggtcgtcgacctgaccgaaggcgcctacaccgagcgcgaactcatgatggtgaaggtgcgcgcggtcggcaaggagcgcgaagaaatgatgcgcatggcggagatcttccgcggccgcatcatcgacgtcacggacaagagctacaccatcgaactgaccggcgaccacggaaagaacgacgcgtttctcgaggccatcgagcgcagcgcaattctcgagacagtacgcaccggcgccagcggcatcggccgcggcgagcgcattctgcgcgtctagtttttttcagcaatcaccaccccccgaatcaacgaaggagcatcgacatgaaggtttattacgacaaggacgcggatctgagcctgatcaagggcaagacggtcgcaatcatcggttatgggtcgcaaggtcacgcacacgcgcagaacctgaacgacagcggcgtcaaggtcgtggtcggcctgcgcaagggcggcgcttcgtggcccaaggtcgagaaggccggcctccaggtcgccgaagtggccgacgcagtgaaggccgccgacgtggtcatgatcctgctgcccgacgagcagatcgccaacgtctacaagaacgacgtggctccgaacatcaaggaaggcgcttcgctcgtcttcgcgcacggcttcaacgtgcactacggcttcgtgcagccccgcgccgacctcgacgtctggatggtggctcccaaggccccgggccacaccgtgcgcagcacctacacgcaaggcggcggcgtgccccacctcgtggccgtgcaccaggacaagaccggcaaggcgcgtgacctcgcgctgagctacgccaccgccaacggcggcggcaaggccggcatcatcgagaccaacttccgcgaagaaaccgagaccgacctgttcggcgaacaagcggttctgtgcggcggcacggtcgagctgatcaaggccggtttcgaaacgctggtggaagccggctacgcgcccgaaatggcgtacttcgaatgcctgcacgagctcaagctgatcgtcgacctgatctatgaaggcggcatcgccaacatgaactactcgatctcgaacaacgccgaatacggcgagtacgtcaccggcccgcgcgtcgtgaccgaagagaccaagaaggtcatgaagcaagtgctcaaggacatccagaccggcgaatacgccaagagcttcgtgctcgagaacgctgccggcgcaccgacgctgatcagccgccgccgcctgaactccgagcaccagatcgaagtggtcggcgaaaagctgcgcgcgatgatgccctggatcaagaagaacaagctggtcgaccagacccgcaactgatccaccacgaaggggcgccgcggcgcccgtttcacgagggccacccgctggggtggcctttttcatgatggggacgaaccacccctgaactacactgcgaacccatgcgatttacagatcaagacgctatcgaacggatagccgttcgcgcagtgtccacgagggacggaggcaaactcaatgcatgacgacacggttcccgacgaggtgccgccccgcaagcgccgcaagggcatctacatactgccgaacctgttcacgctcgctgcgctgttcggcggcttctattcggtcgtgatggccatgaatgcgcgcttcgatctcgcggcgctcggcgtctttgccgccatgattctcgacagcctcgacggccgcgtggcccgcatgaccaacacgcaaagcgcgttcggcgagcagatggattcgctgtccgacatggtgtcgttcggcgccgcgccggcactcatcgcgtacgagtggtcgctcaagggcctgggccgctggggctggattgcggcgttcgtgtactgcgcctgcgcggcactgcggctcgcgcgcttcaacgtcaataccggcgtggtcgacaagcgctggttccagggccttccgtcgccggccgcggccgcgctggtggctggcttcatctggctcatgaccgagtggggcaagcggggcggcgaggtgctgtatctctcgtggacccagatcacgtggatcaccttcgggttcacgctctatgccggtctttcgatggtcaccaatgcgccgttctacagcttcaaggacgtgcagatgaaaaagagcgtgcctttcgtggtgatcgtgctgatcgcgctgggcatcgcggtcatcaacatccatccgcccacggtgctgttcggcctcttcgtggcctacggcctgagcgggtacgtggtgtatgcgtggcgcaaggccaaggggcagcaggccagtgtgatcagcacctcgaccgaggagccggacgagcgcggcttgcataactgaacgcggcttgtgctacattcgcaatcctcatgaccaagatttcgctgctggccctactagccctccctcacgggcggagacggtagcgcacgcgcaaatccctcaccacggcccgttcgcaccagcaacgggccgtttgtttttggggttgctggttgattaccaaccatccagagaaatcgacatgctcaagcaacctcaagccaaataccgcgcattcgccccgatcggcctcaaggaccgtacctggcccgatgccgtgctgaccaaggccccgatctggctgtcgaccgacctgcgtgatggcaaccaggcgctggtcgagccgatggacatcgcccgcaagatgcggatgttcgagacgctcgtggccatcggcttcaaggagatcgaagtcggctttccctccgcttcgcaaatcgaattcgatttcgtgcgcaagctgatcgaggaagaccgcattcccgacgacgtgacgatccaggtgctgacgcaggcgcgcgaccacctcattgcccgtaccttcgaatcgctgcagggcgcgccgcgcgccatcgttcacctctacaacgccgtggccccggtgatgcgccgcgtggtgctcggcatggacgaagaccagatcgtcgagcttgccagcagccatgcgcgcatgttcaacgactttgccgccaagcagccggccacgcagtggaccttccagtactcgcccgaaatgttctcgggcaccgacgtcgtgttctccaagcgcgtggtcgatgcggtcaccgaagtctgggcgccgacgccggagcgcaagtgcatcgtcaacctgcccaccacggtcgagcattccacgccgaacatctttgccgacatgatcgagtggatgcaccgcaacctcgcgcgccgcgattccatcgtgctgtgcgtgcatccgcacaacgaccgcggcaccggcacggccgccggcgaactggccttgatggccggcgccgagcgtatcgaaggctgcctcttcggcaacggcgagcgcaccggcaacctcgacctcgtgaacgtcgcgctcaatctctacacgcagggcgtctcgccggaactcgacttctcgaacatcgacgagatccgcgcgacggtcgagcactgcaaccagatcccggtgcatccgcgccacccgtatgtcggagacctggtctacacctcgttctccggctcgcaccaggacgcgatcaagaaggcctttgcagcccgcaaggacggcgatatctgggacatgccgtacctgcccatcgatccgaaggacgtgggccgcagctatgaagccgtgattcgcgtcaacagccagtcgggcaagggcggcatggcctacctgctcgagagcgaatacggcatcgaaatgccgcgccgcctgcaaatggagttcatgcagaccgtgcagcgcgtgatggacgtggccggcaaggaactcaccgccgccgacctctggcagctgttcgtgcgcgaatacggcctcgaagccgcgcacgcgttgcagcaccgcgtgctccaggaagaaggcgagggcgccaatgcttccgtggtgctgcgcggcgacctgccctgggacggcgaaattcgcgccatcgagggccgcggcaacggcccgatcgacgccttcacgcaggcgctgagccaagccaccggccacacggtgcgcgtgatggactatcaccagcacgccatcggcgcgggcgccgatgccaggtcggtcgcgtacctcgaactgcgcgtggacgaggcccagacattgttcggcgtcggcatcgacgcggacgtgatctcggcgtcgctcaaggccattgtctcgggcgtgcagcgtgcgcggacccgcggcgcgcacagcgcacaatcggtggttgagctcgcctgacgcagtccgccgccgtccgcgcaaggtgcgaaacgattaaaggaacaaaggagtccacgatgaccgaccaactcattattttcgacacaaccttgcgcgacggcgagcaatcgcccggtgcttcgatgacgcgagacgaaaagatgcgcatcgccaagcagctcgaacggctcaaggtcgacgtcatcgaggccggttttccagccagctcgaacggcgacttcgaggccgtcagggccattgccgatgccatcaaggattcgaccgtgtgcggcctgtcgcgcgcgaacgaccgcgatatttcgcgagcggccgaggccctcaagggcgcggcgcgcggccgcatccacacattcattgccacctcgccgctgcacatggaaaagaagctgcgcatgtcgccggacgaggtgcatgagcaggcgaggctcgccgtgcgctttgcgcgcaacctcgtggccgacgtcgagttcagcccagaagacggctaccgcagcgaccccgattttctctgccgggtgctcgagaccgtgatcaacgagggcgcgaccaccatcaacgttcccgacaccgtgggctatgccattccggagctctacggcaacttcatcaagatgctgcgcgagcgcgtgcccaacagcgacaaggcgatctggtcggtgcattgccacaacgaccttggcatggcggtggccaactcgctcgccggcgtgaagatcggcggcgcgcgccaggtcgagtgcacgatcaacggcctgggcgagcgtgcgggcaattgttcgctcgaggaggtcgtgatggccgtgaagacccgcagggactacttcggcctcgacctcaacatcgacacccagcacatcgtggccgcgagccgcatggtgagccagaccacgggcttcgtggtgcagcccaacaaggccgtggtgggcgccaacgccttcgcgcacgcatccggcattcaccaggacggcgtgctcaaggcgcgcgacacctacgagatcatgcgggccgaagacgtgggctggagcgccaacaagatcgtgctgggcaagctcagcggccgcaacgccttcaagcagcgcctgcaggaattgggcgtgacgatggagagcgagggcgacgtcaacgccgccttcctgcgcttcaaggaactggccgatcgcaagtccgaaattttcgacgaagacatccttgcgctcgtcagcgcggaagagcattcgcacgttaacgaacagtttgcttttgtttctctttcacagcacagcgaaaccggcgaacgcccccacgcaaagattgttttcaccgtccagggcaaggaagtcactggcgagtccgacggcaatggcccggttgatgcttccctgaaggcgatcgagtcgctcgtcaagagcggcgccgaaatggttctttactcggtcaatgcgatcagtggctcgacagaaagccaaggagaagttacagttcggttacaaaatgcagggcgggtggtgaatggagtaggtgcggacccggacatcgtggtcgcgtcggccaaggcttatttgagtgcgctcaacaagctccagagccaagctgagagagtggcggcacagggttaggtttactgaccatcctaagttaagaaagggatgcaagtaactgatattgcgtgccttttttgatttggatacactgcggttctcattttcgccgctggagatttataaatgcctgaagcccgtctccgccgagtttccagccagcggttcctgcccgcagtcaaatttgtcgccgtcgcgttctgcgccacggcgtttttgctgtccggagcccaggccgccaagaaggaacaaaaaccaagcgtcgccaagacctcgctggccaagaaggccgcgggtcctgtgccggtggaagtcaaacggcgtactgccaaggccgaccgcagcgagaaagtcgttcgcggtggccgcaatgtcgtggcttccatccgccaaaaaaacggccggaccgtggtcgccgtgcaacgccgttcggtggttcgcgtcgaaacgcccgcgcgccagtccttcggccagttggccggcctgcacggaaccgacgacgtgctcgacctgaagtcgagcgttgcactggtcatcgaccaggacacgcacgaagtgctgttcagcaagaacgaccatgcggtgctcccgattgcatcgctcaccaagctcatgaccggcctcttgatcagcgaagcgcgtcttccgaacgacgagctgatcaccatcacccaggacgacgtcgacaccgagaagggcagccgctcgcgcctgacggttggtaccacgctgccccgcggcgagctcttgcatcttgcgttgatgtcgagcgaaaaccgcgcggcgcacgccctgggccgcacctatcccggtggccttgcaaccttcgtgagcatcatgaacgccaaggccaagatgctcggcatgaaggacacgcgctacgtggagcccacgggcctgtcgagccgcaaccagtcgagcgcgcaagacctggcgctgctcgtcaacgccgcctacgccgacgccacggtgcgctcgctttcgacttcgcctgaataccaggtcgaggtaggcaaccgcgtgctgcagttcaacaccaccaaccgtctcgtgaagagcccggattgggaaatcggcgtgcagaagacgggctacatctccgaagccggccagtgcctcgtgatgcaggccaaggtggcggggcgcaagctgatcatggtgttcctggattcggccggcaagttcagccgtatcgccgatgcggagcgcgtgcgccgctgggtcgaggccacgcacgcctcgacgggctcgccggccgccgcgtcgcgcgcgcccagctaccaagtcgctggctgatctgacaccagccctgaaagggctggtctgatctgacgccggccctgaaaagggctggcagaccgcacgcggcgcaggccttgggtcaggccgtggctgacgaagaagatccgccgccgtccgccgcagatgctctggacgccgccgcggcggcgtccttgtagccgagcgctcccgagatttcgttggccgtggcctgcagcttgggcagccatccttcgtccagccggtcggcgggcgcggaaatcgacaatcccgccaccagcttgccctggtcgtcgtagatgccggcggccatgcagcgcacccccagctccagttcttcgttgtcgcgcgcaatgccgtactggcgtgccttcgacaattcgcgctccagcgccggcagctgcgtgatgctgttgcgcgtgtgtcccgccaagccggttcgggtggcatagctgcgcacgcgctgcggatcgtccgccgccaggaagagcttgccggtggaggtcaggtgcagtgctgcgcggccgccgatggcgcgcaccacctgcatgcccgaacgctcgctgtacgagcgctcgatatagacgatttcgtcaccctgccgcatgctgaggttgaccggctgctgcgtgagcttgtgcagctctcgcatgggccccagcgcggcgtcgcgcacgttgagccgccccttgacgaggttgccgagctccagcagccgcatgccgagccggtagctgccggcttcgggccggtcgacaaagcggccgaccgccaggtcgttgaggatacggtgcgtggtggaggggtgcaggccggtcttctcgctgatttccttcagcgaaatggcttcctcgcgcgaggcgagcacgtcgatcagcgcgaacatgcgctcgatcacctggatgactggaacggcaggaacgtcggattgggtttttctcatggcgcgatgcggtgtggaccgggcgccattttaccttgtgaaatcagccggtgcttgccagcgtccgtcgatcagcagttcatgggggctgaagcgcgccttgtagttcatcttggcgctgccttcgatccagtagcccagatagacgtgcggcaagcccagcttgcgggcttgttcgatctgccagagcacgctgtaggtgccatagccagcgccgctctcgggctcgtagaaggtgtagaccgccgaaatgccatcgttcagcacgtcgagtatcgacaccatccgcagcgcaccggcgctgccgtcgggcagtgtctcgcggaactcgaccagcctggagttgacccggctctgcagcaggaactgggtgtattggtcgatgctgtcgtggtccatgccgccgccggcgtggcggccgttctggtagcgcagatagagctggtagtgctcgggtacgaagcacagcttgagcacgcgtgcctgcagttccttgtgctgcttcacggcgcggcgctggctgcggctgggccggaagccgttgaccagcacgcgcagcgggatgcaggcgcggcacccgtcgcagtagggcctgtaggtgaacattccgctgcgccggaacccgctgagcacgaggtcggaatacgcgtcgttgtgaatcaggtggctgggcgtggccacctgcgaccgggcctggcgatcgggcaggtagctgcaggggtagggcgccgtcgcgtagaactgcagcgtgtgaagcgggagatccttgaggtgcgtcacgtcgattcagaaggccgcgtggaaaggagttctgtccagtatacgggctcgaaatgccactgtgggccctgctgttcgcgtgccttggccacatgcgccacaaagcttgcgcgcgacatctcccgggctcccaggctcgccaggtgggaggtgttctgctggcagtcgatcatccgcacctgaaagcgccggcacaggcagaccagggccgccagcgcgatcttcgaggcgtccggacggcgcgtgaacatcgattcgccaaacaccgcacggccgagcccgacgcagtagagaccgcccgcaagcttgccgtcgatccaggtttccacgctgtgcgcgtggccggcccgatgcagcgccatgtaggcgttcaccatgtccgggacgatccaggtgcccgactggccggtgcgcggcgattgggagcaggccttgatgaccgccgaaaaatcgcggtcgatgcgcacttcgcagccgggggtctgcgcgaagcgggcgagggtcttgcgcagcgacctgtggagcttgaattcggccacctggagcaccatgcgcgggtccgggctccaccagaggatcggctggtcttcgctgaaccacgggaacacgcagtggctgtaggcctgcaccagggtgtccacatcgagggccccgccggcggcaaggaggccgggtacggggtcggcgtcgccccaggcggatgcggggtcgggcagcgcgtcgccgggttcgagccaaggcagttgttgcatggccgtaggtatacacggcttcgcggtgcgcttcatccacgttgcacaaaatggccgttctccagcgggacggcaagcgactgacgcggctgcacgccatcggctccgcctgcgaaacacacaggaatacccaagagcccatatagtgctgcttccatttgctctccatcggacccgcaaggcgagcgttgccttgcggatggccagcccaagaggaccacgttgactactgaatccaatcccacgcgtttcggcagcggccatgcagtgcgccgcctcgaggacgagagcctgcttgccggccgaggccgctacacggacgacgtcacgcttgccggccagacacatctggtgttcctccggtctccctacccgcacgcgcgcatcgtctcgatcgacgtctctgccgcggcagccatgcctggcgtgctgcgcgtggtcaccggcgccgaaatggccgaggccggcgtcaagccgatgccgggcgccgcgggcttcaggcgggccgacggcagcgatgccgcgagccccccgcggcttgccatggcgcacgaaagaacccgcttcgtgggcgaagcggtggccgcggtagtggccgaaacggtccagcaggcccgcgatgccgccgaagccgtggtgatcgactacgaagaacttcccatggtggtcgatcttgcaagcgccaccgccgacggcgcgccgctgctgtgcgacgaggccacgggcaacatcgctgccgaaatgcgccatggcagcagcgacgccgcaacggccgcctttgccaaggccaaacacgtggtggcgctcgacgtgatcaaccagcgcgtcgtggcgctcaccatcgagccgcgctcggtgctcgccgcgcatgaggacgggtccgatcgcctcaccatccgcatgagcacccagatgccctcgggcgtgcgcgactcgatctgcgccgccatcggcctcgcaaaggaaaaggtgcgcgtgttggtgggcgacgtgggcggcggattcggtatgaagaccggtgcctatcccgaagacattgccgtggcctatgccgcactgcaagtgaagcgtcctgtgaaatgggtcgccgaccgcagcgaggagtttctttcgagcgcacatggccgggacatcgaggccaaggccgagctcgcgctcgatgccgacggaaagattcttgcgctgcgcatcaagacgctcgccaacgtgggcgcctatgccaccggcaccggcgtcgcgatccagctcctgatcggcccctgggtgcagaccagcgtctacgacatccagaccatcgactttcatttcaaggcggtgctcaccaacaccgcgcctacgggtgcctaccgcggcgcgggccggcccgaggcgattttcaccatcgagcggctgatggacgaggccgcgcgccagaccggtatcgaccgcgtcgcgctgcgccgccgcaacttcatccgccccgaacagatgccctacaccaacccgatggcgcagacctacgacacgggcaagttcgagtcggtgatggaccaggcactggcgctggccgactggaacggcttcgagggccgcgcggccgagtccgcccggcagggcaagcaccgtggcctgggcattgccacctttctcgagtggaccggcggcaatgtgttcgaggagcgtgtcacggtctcggtgcaggcggacggcgtcatcgaggtgttctccgccgtcaacgcaatggggcagggcattgccacctcgctcgcccagctggcggtcgatgccttcggcgtgccgatcgagaaggtgcgcgtggtgctcggcgacacggaccgcggcgacggcttcggcagcgccggttcccgctcgctgttcaccggcggctcggcggttcgcatcggcgccgaacgcaccatcgacaaggcacgcgaactcgcggccgaggagttcgaggcggcccccgacgacgtgacctacagccgcggcgtgttctccgtggccggcaccgacctcgagctcgacctgttcgacctggcgggcaagcagcccgagcgtgaaatcttcgtcgactccaccagcaccgtggcgggcccgacctggcccaacggctgccacatctgcgagatcgaactcgatccgccgacgggcgagatcagcgtggtggcctacagctcggtcaacgacgtgggccgcgtggtcaacccgatgatcgtgcgcggccagctcgaaggcggcgcggtgcagggcatcgggcaggcgctgtacgagcaggtggtgtacgacaacgaaacaggccagcccctcaccggcagcctgatggactacgccgcgccgcgcgcggacatcgtcgagaccatgttccacatggagatggacgagtcgacgccgtgcaccaacaatccgctgggcgtgaagggcgtgggcgaactgggcaccatcggagccacgccgaccatcgtcaacgcggtggccgatgccttcgcgcgcaacggccttgcgaacggcacgccgcgcctgcacatgccgctgagcccgtctcgggtatggcaggccatgcacactgtggactgaggcttggggcgctcgtcgcgggtgaattcgaatgctcgtcaccaccgaactgcagaccgaacctatccgcgtgtcgagctaccgctgcgacgcgggtcccgatgcgcagccgttcaccgagatgcacgtcgactactccgtgtcgtacgtgcgaaaggggagcttcggcttgcgcacgcgtggcaacgcctatgaattggtggccggttcggtactggtgggctgccccggcgacgaatacatctgcacccacgaccaccatgtctgcggcgacgaatgcctggcgttccacctgtcgcccggcttcgtcgacctgataggcggcgaccagcggacctggcgcaccgcggggctgccgccgctgcccgaactcatggtgctcggcgagctcgcgcaggttgcgaccgagggccaggccgacatcggcctggacgagctcggcatgtggtttgccggccgtttcgtccaagtggcgagcggacgcggcaagccggcaccgcagccggccgcgccgcgcgacaggcgccgcgcggtggatgccgccctatggatcgatgcgcactcgcacgacgacatcggtcttgaaggcgcagcgtccgaggccggcctgagcgccttccacttcctgcgcctgttctcgcaggtgctcggcgtcacgccgcaccagtacctggttcgctcccggctgcgccacgcggcgcgcctgctggcggacgacgaccgccccgtgaccgacgtggccttcgacgtgggctttgccgacctgagcaacttcgttcgcacctttcaccgcgcggcaggcgtgtcgccgcgcagctttcgccaggccgccaggggcgatcgcaagattttccaagaccgattggcagccctgctcaatgatgaccgcctgattcattcatcgagcagaaagtcatcgccatgtacgaccacatcggactgaaagtcaaagacctcgccgcgagccggcgcttccacgaagccgcgctggcgcagctcccctgaggcgcacggccatggcaacgatctacaaagaattcatcgtcgaagccgatgccgacgcagtctgggatgcgctgcgcgatttcggcgccgttcgcacgcgcctcgcgcccggttttctgaccgactgcaagctggacgggcagggcgcccgcatcgtgagttttgccaacggcctggtggcgcgcgagctgctcgtgggcatcgatgaggccaaccgccgcctggcctacaccgtcaccgacggccaggccagccaccaccatgcctcagcccaggtgttcgcccacggcgaagggcgttcgcgcttcgtctggatcaccgatgtgctgcccgacaagttcgccgcctacatcggatcgatgatggacgagggcggcgtcgcgatgaagaagacgctcgagcaaaaaagcccggcgccgccggccggctagaaatcctcgagcggcaggcccacgtagttctccgccagcgaggtggaggcggcctgcgaatgcacgaggtagtcgagttcggcttcctggatcttctggccgaacgcgccggtctccgggaagcggtgcatcagtgaggtaaaccaccacgagaagcgctcggccttccagacccggcgcaggcagaggtctgagtaccgatcgagtgcggagggcgatttttcgccatagaagatctcgaacgcgcgcgacaggtagcccacgtcggccgttgcgaggttgagccccttggcgccggtcggcggcacgatgtgcgccgcgtcgccagccaggaacagcgaaccgaaacgcatcggctcggcgacgaagctgcgcagcggtgcaatgcttttttcgagcgaagggccggtcacgagccgctcgcgtgcctcggggtcgagccgcgcgcgcagttcgttccagaacgcctcgtcgctccagttttccacccgttcttcggtcggcacctgcacgtagtagcggctgcgcgtggcgctgcgcatgctgcacagcgcaaagccgcgctcggtgttggcgtagatgagttcgtgcgacaccggcggcacgtcggcgagcacgcccagccagccgaaggggtagattttctcgtaggtctggatggcgccttcgggcacgctggcgcggctcacgccgtggtagccgtcgcagccggcgatgaagtcgcactcgatctcgtgcgtctggccgtctttttcgtagcgcacgcgagggcgcgccgagtcgaagccgtgaaggctgacgttggccgcgctgtagatggtcgtgaggccttcggccgagcgcgcctccatcaggtcgcgcgtcacctcggtctggccatacacggtgacctgcttcccgcccgtgaggccatgcaggtcgatgcggtgccgcgctcccttgaacagcagctcgatgccttcgtgcggcagcccttcggccttggcgcgcgcatcgacgccggcacgcgccagcagatccatggtgacttgctcgagcacgcccgcgcggatgcgccccagcacgtagtcgccgctctggcgctccacgatgatgttgtcgatgcccgccttgaaaagcagctgcccgagaagcaggccggccgggcccgcgccgatgatcgcgacctgtgttcgcatgttcatgtctccgttgaggttttcgcaagcgtaggtcgttcggggcagcctggcgcggcgctttgcgaggcactgtgcgatcatgcgagtggctgcgcgatgatcgcgcaacacttcgtaccttgaccggatgaccatcgccaaagccgacttcatcgagggcattgccaagggaatggccgtgctcgaaagcttcgacaccgagcgccagcgcctcaacgccaccctggcggccgagcgcgccggactcacgcgcgccgccgcccgccggcacctgctcacgctggcccacctgggctacctggagaccgatggcagctatttctggatggcgcccaaggtgctgcgcttctcgggcagctacctggcgtcgtcacgcctgccgcgtgcgctgcagcccacgctcaaccggctcgcggcacaaaccggggagtctttctcggccgtggtgctcgacggcgaagaggtggtcatcattgcgcgcagcggcagctacggcacgccgacccgcgtgctggcgtacggcctgcaccttggcgcccgcctgccggcgcacgccacgtcgaccgggcgggtgctgctcgcggccatggcgccggcccagctcacgcagtggctcaaggggcgccacctcgcgcggctcacgcccaacaccaccacccaggcgcgcagcctgcgccagctggtttcccgtgtgcgcaagaacgactactgctttgccagcgaagagcacgagctcggcgtgcaggcgctcgcggtgccgctgcgcgacatgcagggccacacggtggccgcgctgaacgtggtgctttcgggcacgcgctaccaggaagagacgctgcagcgcgagatgctgccgctgctcttcgaggcggcgcgcgaggtcaggtcgctgctgtgatctgaacttccgcgctgccgctgcctcgaatcccgaaaacgcacaccacaaccatgcgactcctgcttctcgaagacgacgtgatgatcggcgaagccgtgctcgacctgctgcgcgccgagcaatacgccgtggactgggtgaaagacggcgatgcggccgagtccgccttgcgcacccagcagtacgacctggtgctgctcgacctgggcgtgccgcgccgcgacggcctcgaggtgctgcgcagcctgcgtgcccgcaagcagcgcatgcccgtgctgattgccaccgcgcgcgactcggtgcagcagcgcatcgaagggctcgatgcgggcgccgacgattacgtgctcaagccctacgacctggacgaactgctggcccgcatccgcgccttgttgcgccgcgccgcggggcgcgccgagccggtgtacgagcacatgggcgtgagcatcaaccccgccacccgcgaggtcatggtgggcggtcagccggtggtgctgtcggcgcgcgaatgggccgtgctcgagccgctgatcgcgcggcccggcatggtgctgtcgcgtgcccagctcgaggaaaagctctacagctggaaggacgaaatcagcagcaacgccgtcgaggtctacgtgcacggcctgcgcaagaagctcggggccgaactgatccgcaacgtgcgcggcgtgggctacatggtgccgaaggcatgatgcgcgcgctgaccgggtcgctgcgcgcgcgcttgctgtggttcctgcttgcggccatcgtgcttgctgccggcgcgcaggcgctggtggcctaccgcacggtgttgaaagaggccgacgacatcttcgactatcacatgcagcagatggcgctctcgctgcgcgccggcctgccgccgagcgcggcggtcggcggcatcggcagcggggagcagaacttcgatttcgtggtgcaggtgtggaccgccgacggcgtgcgcatcttcgaatccgccgagcaggcggcgttgccgcaactggcggtgctgggctttgccgacgtgcgtgcgcgcggcaccacctaccgcgtgttctcgatgcagacgagcgggctggtcattcaagtggcgcaggacatggcggcgcggcgcaacatggccggggcgctggccctgcgaaccattgcgccggtggcgttgatggcgccgctgctcatgctggtcgtctggtgggtggtgagccggtctcttgcgcccgtggcacgcgtgcgcaagcaggttgcctcccggcaggccgacgatctttctgccgtgagcgaggaagacctgcccgatgaggtgcgcccgctggtgcaggagctcaacctgttgttcgaccgggtgcgccacgccttcgatgcgcagaagcacttcgtggccgatgcggcgcacgagctacgctccccgctcgccgcgctgaaactccaggtgcagggcttgcagcgcgcgcccgatgccgcagcgcgcgatctggccgtgagccggctggtcgcgggcatcgaccgcgccacgcggctggtcgaacagatgctggcgctggcccggcacgaggccagcatggccgccggtgccaagtcccagccggtcgaccttgccgaagtggcgcgcctggccatctcggatgcggtcgcagccgcgcaggcccggggcatcgacgtcggggtttcgcatgccgacgccggcgccgtggtgaacggccagcccgaggcgctgcgcatgctgctgcgcaacctgatcgacaacgccgtcaagtacacgccggaacaagggcgcgtcgacgtcgctattgcgatgaacggtgcggcggtggacctcagcgtggacgacagcgggccgggcctccccgaggaagagcgcgcgcgcgtgctcgaccgcttctatcgctcgggcgagccgcaggcgcccggaagcgggctcggcctcgcgatcgtcaagtcgattgccgacctgcacggcgccacggtggtgctcgctgcctcgccgagcctgggcgggttgcgggtgctggtgcgctttccctccaaggcctgaaggccttcgagcaccgggccgcggtttaagccgcgcttaagccagtgcaccgacattcctttcatcgtgttgcgcacagacgcattgaaaggaaaaccagaaatgaacacccgcctcacttctccccatgccctggtcatcgccttggcgaccgccggggtgatcggtgccgtcggtgccggcgcctacaccagtgcccgcgcggtgaatgcgccgaccaacaccgcgagcgtggcgccggccgcgatggtgacgctgcccgacttctcgaccatcacttcgcgcgatggccccgcggtggtcaacatcagcgtgaccggcaccgcgaaggcgtccgacgccgaagccgcggccgagatgcagggcatcgacccggacgatccgatgctccagttcttccgccgcttccagggccagatgggcccgcgcgcccagcagcgcgaagtgccggtgcgttcgcagggttcgggtttcatcgtgagccccgacggcatcatcatgaccaacgcgcacgtggtcaaagacgccaaggaggtcacggtcaagctgaccgaccggcgcgaattccgcgccaaggtgctcggcgccgacgccaagaccgacatcgcggtgctcaagatcgatgccaagaacctgcccaccctggcgctcggcaacaccaaggacctgaaggtcggcgaatgggtgctggccatcggctccccgttcggattcgagagcacggtcaccgccggcgtggtgagcgccaagggtcgttcgctgcccgacgacagctacgtgccgttcatccagaccgacgtagcggtgaaccccggcaactccggcgggccgctgctcaacacgcgcggcgaggtggtcggcatcaactcgcagatctacagccgcagcggcggctaccagggcgtgtcgttcgccattccgatcgacgtggcggtgcaggtgaaggaccagatcgtcgcgaccggcaaggccacgcacgcgcgccttggcgtggcggtgcaggaggtgaaccaggcctttgccgactccttcaagctcgacaagcccgagggcgcgctggtctcgaacatcgagaagggcggccctggcgacaaggccggcctgaaggcgggcgacgtgatccgcaaggtcgacagcgagcccatcgtctcgtcgggcgatctgcccgcggtgatcggccagcaggcgccgggcaagaaggtgacgctcgaagtgtggcgccagggcgagcgccaggagatttccgccaggctgggcgatgcgagcgacaagcccgcgcaggtcgcgaagaacgacagtgcggcgggccagggcaagctcggcctcgcgctacggcccctgcagccgcaggaaaagcgcgaagccgcgatcgagaacggcctgctgatcgaagacgttgcgggaccgtcggccctggccggggtgcaggcgggcgacgtgctgctggccatcaacggcacgcccgccaagaccctggagcaggtgcgcgaggtggtggccaaggccgacaagtccgtggcgctcctgatccagcgcggcgaagacaagatcttcgtgccggtgcgaattggatgacgccccgtcccaggcgccaggacgaagaaacgtgagctcatcgaccggcggcctttcggcgcacatcctgcccacgtcggccaccatgatcggcgtgtgcatgacggtgatgtcgatcggccacctgggcccgcgcgacgatctgcggctgctcatcgaccgcatgctggccatcgatgcactggtcttcctggccagcgcgctcttgtccttcatctcgatgcggtcgcgcagatcgggtgttcggctggaggcctggggcgagatggtcttcatcgccgggctcgcactgctggcgctgggcgccgtcacgctggcgtttgccttgcgctgaggctaacgccgcgcggccttgtcgagccgcgccgccaccagcgcgagatgcccgaccagttctctgggcgactcgatctcgaaatcgtgtcccaggcaggccagccacacggccagcgcgtcgagcgaattggcgccggtctcgatgcgtgtgcggctgtcgtccacggcctttggcattccgccgacccaggccatgtgcgcctccagcgcctcgatgggcgcgtgcaccaccacgcgcgcatggtgcagaaagggcgacaccgcgagcgcatgctgcatgtaggcctcgacgtcgccatggggcagccttcgggccgtgaatcgggcacccgtaggggcggggtcgacgatgcggtcgaggcggaaagtgcgccagtcctggcgcgccgtgtcccaggccagcaggtaccagcgctgccccgtctgcaccacgcgatgcggctccaccgtgcgggcgctggcggcgtcgtgatggtcgcggtagtcgaagcgcagctccagcctttcggtgcaggcctcggccaggagcgacacggccttcagccggacagccggcttgccgcgcatcacgggcaccaccgatgcgcgcacgctttccagccgccgccgaagccgcggcggcatcagttgctccagcttggccagcgcgcgcatcgacgcggtttcgatgtcgcccaacgccccgccggccgtgccgcccagtcccagcgccactgcaatggcctcttcgtcttcgagcagcagcggcggtagcgacgtgccggcacccaggcggtagccgccggcgacgccggaggtcgagtcgaccgtgtagcccaggctgcgcagccggtcgacgtcgcggcgcagcgtgcgctcggtgatctcgagccgggtggccaattcggcgccggtccatgaacgttgggcctggaacagcgacaggagccggatcaggcgtgcggaggcagacaacatgggttgaatgatgcctctgatcgaggacagaatctgtccgcaatggggcttagcctcggatcttctccactcacacgggacacgacccatgaagaagatatacagcggaagctgccactgcggcaaagtccggtttcaggcggacatcgacctgggcgaaggcaccggcaagtgcaactgttccatctgcaccaaggccagggcgtggggcgccatcgtcaagcccgaggcctttcggctcgtgtcaggcgagcgggagctttcggtctatcagttcaacacgcacagcaccgagcatttgttctgccggcattgcggcatccggccgttcggccgcggcaatgtgccggagatcggtggtgcctacgtcagcgtgaacgtcgcttgcctggatgacgccacagccgatgaactggctagcgcgccggttcgctacatggacgggcgcaacaacaactggtttgaggcgccagccgagacgaggtatttctaggcggcaaccgaatcggcgtgcgggcctgccgatggcggcgcccgcatgcgacgcgggttgggttcgagaggggaggccggctgcgcctacagctccttgctgccggcgtcgttgtcaggaacctgcgcatcgagttcgtccttgatcgtcctgtctccgcggatggccagatacaacacggcacccaggccaagcacgacgacgaagatcacggcgaaaaagccgctccccaagatccaccaccaaaacaaaccgctcgcaagaagcagaagcgcaaccaagagtaaagagttcaagtgcatgcaccgcgctgataggacgttggcggtaatgtacgcggcgttggctgctccatgcctgactttgggtctgggacataccctcttttcgggttttcgtgatgtccactacacgcgatgcactaggcggatccaaagtagcgggcggcgacgcggcccaggttggtgatttcactcaccgttgcgcagagaggcatggggctgtgtggcggtgagaacgcgaccttgatgtacccggcgtctcgcagatccttgagccggtctatttcggacggactggagaactgcactggcaaccgcgatgccaggatctgggtgaaaagcgcatacgccaagttgcatctcccgagtcaaggggaaattgggcgacacgccgtcgcccgggcttcgacctggatcggtgcgagcctgtaacccgttcacccatccggtccggaagataccctggtcgatgcgtcctatcgattccacgtccggcataggcctcggccaggccgatgcccgccgcagaaggctcaaagagggtactcatgagggatttcttccgcgcggactgcggcctatgctttcgcgaccatgaccgcatccctgatggatttcgatctgccggagggctggagctgcgcggtggaactcgagctcacgcctgagggcgtctatgctggacgggccgaacttcggcacgaattcacgcagtgctgcgtgctggtggtgacccagcagccgacccgtgaagccgcactcgaatgcatgaagtttcgcgccgctcgtttcgtggaggaatggaactccaggttggcgcagcccatgtagacgatgtgccccaaaaggaaatgccccgtcaccttttgagtgacggggcatccagaggccttgcggcttgtagtggctcctcgacctgggctcgaaccagggacctacggattaacagtccggcgctctaccaactgagctatcgaggaacaagcctcagattatagcgtgattttttgagcctttcgagtgcacccatacggccgcaataaatttccgaaaaatttttgagcgcgtgttcagagcgacacgctcaacccgaggcgcagcgtgcgcggtgcgccgggaaagaggtagacatggccgaactggtagggcgattctttccagtagcggcggtcgaacaggttgtcgatggcgaggctccagcttgtctgaacgccgcgcaacttggtgtcgtagcgcagcacggcatcgacgcgcgtccatgagggcagcgtgatcgaaccatcggccaacacgttgcgccggccctcatgcgacagctgtcccagcagttcgagaccgggcaccgaggccacgcgatagccggcctgcgcgcgcagcacttgcttgggcacgttggtgggcgactggccattgatggcaggctcggcggtgctaccgcggcgcttggcatcgatcagcgtgacgctgccgcctagacgccaaggccccgtgttccattgcgcgcccgcctcgagtccgcggtgcaccgcgctgccatcgtagcggccatcgcagggcgtgatgaagagccggttgcaggcgtcgagattggtcatcggccgcttgatgtcgaaccacgcgagctgccagttgaatgcatcgccgccgcccttgagtcccagttcccattggcgcgacgtcagcgcgggcaacgcctggcccgcgttgctgtactggtcgcccctgttcggcacgacctgcgattcgacgcccttgccccagctcgcgtaggcgagcaatccgggccggatcgcatagctggcggcgacccatggcgtggtcacgccttgcttgtagccggtggggttggagccgtcgttgctgatgctgcttcggtcgagccgcgtatgacgcacgccgagccaggtggtgaagcggtcgttccagcggatcgcatcctgcaccgacagttctgtcgaacgctcgtcgcggttggtctgcggtgtgatggcgtcggagtttggcggcaccacggccgtggcccagacgttgccggtgccgacgtagttgtaggcctggttctggaagcggttgcgcacgcggctcgcgagaaggccgaagcccagctcgtgcttcacgctgccggtcatcacgttgcccttgaggttgaggctgcctgcagtttgcgtgcgccgctcgttctcgctgcgaaagtcgtagaagtcgaaggtgccgtcggagcaatagcggtcgaagttgccttcggcgccgcagccgaaggcgtaggccaggcggtcatcggacttgagcctttgctgcccgatctgcgcgctccagcgccagtcggcattgagtgcctggctgaagcgcacgctgccggtcagtgcattgaactccgagggctgcgaccacggctggttgttgatgttgatttttggatcgaccggcgggggcagcgtgttgcccagcaggctgaagccgttctggctcggctgcgtcttgtggctgcgctcgatctcgaactcgagcaccgaatcgcgcgtgatgcgccagtcgcccgcaagcgagaacatgttgcggttgccgtcgaggttgtgcgtcagcggcttgaggttttcgttcgccacgttgaggcgatagccgaattcgcggttggcgccgaagcggccacccaggtcgatcgcgccgagcacgctgccgcggctggtggtttcgaggcgcagcgtgcgcaggtcctgctcggtcggccgcttcacgacgtagttgaccagcccgcccggcgcgctggtgccggcctggatgccgctggtgccgcgcaggatctcgatgcgctccttgttgtcgagcgggatcgatgtctcggcgctgatcggcaatccctcgcgccggtagttgaagcggttgtccagcacgaagccgcgcaccgtcaggtagtcccaatagccggccgagttgtaggcatcggtcaccgaagaatcgaattgcgtgaggtccgcaagccggcgcgcgccgctcgcgcgaagctgcgtgctgtcgatcaccgtggccgacagcggcagttcgcgcagcggcacgtcgccgaagccgctcacctcggcttgcggtgccgcattgctttcgttcaccgtgacggcgggcaattcggtgggctgttgggcctgcgcgccgcaggcggccagaaggagggcggcagccactgcgtgcgagatgggcgacagcggccgtgcgggaaaggggatttgtttttttgtcatcttgtcttgttcatgcggaggccgcgcccatggcggtcatccattgcgcggccgtggcctcgggatcttctgcggtgaccagcgcgcgcaccacggccaccgagcccacgcccgtggcaagcacctcgggcagtcgcaccgcgtcgatgccgccgatgcccacctgcggatagccgcgcaacaggcgcgcataggcggcgagccgcgcaacgccctgcggggccgtggccatcttcttgagggtggtcggatagaccgcgcccatggcgatgtagctcgggctcaccgcatcggcgcgcaccatctcggcatagccatgggtgctgacgccgagccggaggcccgcatcgcggatctgccgaacctgctcggtcgcgagcgcatcgaggtcttcctggcccaggtgaacgccgtaggcgccggcggcgatcgccgtctgccagtggtcgttgatgaacagcagggcacctgtgccacggacggcatcgactgccgcatgcacttcgcgctcgacggccgccgcgtcgtcagacttgaagcgcagctgcaccgtgggaacgcccgcgcgtgccatgcggccgacccattgcgcatcgggcagcaccgcgtagaggccgagccgttgggggcagggcgcaaaggcgtcgtcgcgcgccgtgggtggaaacgcgcgcatgccgaaatcggccggagtctcgggccactggttcgcatcgaacgcgccggttcgcgctgtctgcgcctgccacgctcgtgccaggcattcggcatcgatctcgatgaagcccagcgcgatgcaggcctgcttcgcgccgcgatacacggggtcgtcggacgaaaagctgccggccgagatagccgcggccgtgatggcgccgaagcgcagcccgtgggccgcaacgattgcatgtgccacggcgcgggcgtcgtttgaagcgatcatggtgcgtgatgccagaagggcgtgccgagcaccggcgtgctcggttgagcggagtcttgcgcggccatggcgccggcacgatgagcggagcggccggcctgaacggcatctgcgaaggcgccggccatcgccactgggtcttgcgcgagcgcgacggccgtgttgagcaacacgccgtcgtagccccattccatgacctggcaggcatgcgagggcagtcccagtcccgcatcgaccagcatcggcacgctcagccgctcgcgcagcaactgcagcgcgtagggattgaccgggccgcggccggtgccgatgggtgcggcccatggcatgacggcctggcagcccacatcgaccagccgctggcacagcacgaggtcttcggtgcagtagggcagcacctggaacccgtcgcgaatcagctgcgacgcggcgtcgacgaggttcagcgtgtcgggctgcagcgtgtagtcgtcgccgatcagttcgagcttgatccacggcgtgtcgaagagctcgcgtgccatctgcgccgtggcgatcacttcctgcacgctgtggcagccggcggtgttgggaagcacgggcacggcgaggcggcgcagcagttcccagaaaccgttgccgctgtcgctcgcacccgggctcgcggcctggcggcgcagcgaggccgtgagcatggcgggcctggcgcgcttcactgcggcttcgagcaggtccggcgaggggtagcgcgcggtgcccagcagcaggcggctctggaaggtctggccgtagagaaccagcggatcgttgtccggcacggaagatgtggttgtcatggtgtgtgttgtctccatctctgtgggtcgtctggatcagccaccagtcacggggcggatcacttcgatgcggtcttcgggctgcagcgcgcggcccgcatgggccgagcgcggcacgaactcccggttcacggccaccgcgaacggcggcacggcatccagtgcggcgagcgcgtcggccaccgtggcgccgtccggcagcgtgaatggcttgttgttgatcaggacgttcatcgtcatgcttgggatgtctccaggccaagggtctgcgcaagcgccgagcggccgtgcacgagcagctccatggcggcgtcgagcacggcgggcgcgatcatgaaaccgtggcggtacaggccgttgatctgcagcacgcgcgggtgcggctggcgaatggcgggcaggttgtcgggcagcgtgggtcggcactgcgttgcaatctcgaggatgcgagcctccgcgaagccgctgtgcaccgcgtaggccgcgctcagcagttcgagcgtggagcgcacgctggcgggcgacatgtcgtccgactcgatctcggtcgcgccgatcacgaacacgccgccgggcttgggtgcgatgtagagcggatagcgtggatgcaccagccgcgtgggccgctgcaacgtcacctcgggcgcatgcacgcgaacgacttcgccgcgcacgccgcgcagtgcattccactgcgggcgggcgccaaggccgcggcagtcgatcacccagtcgggctggcccggcgtgcccggagaaaaatcgcccggttcccgtggcgacttccagtgcagcgtgacctcgggattggcccgcagcgtcgcgagcaatgacgagagcagggcgcgattgtcgagctggccttcacccggaagaaacaagccttgtgcgaagcgctggccgagcgaaggctccagcgcggcaacgccggcaccatcgagcgtttgcatggcggcgagttcgggcacctctgcaccggtgcgggccagcacgcgcgcgagccgcgcggcttcggcggcgtcctgccggtgccacagcaccagcgttccttcgcgttgaaagaacaccggctgtgccaagggcgccagcagttcgggccaacgcaacagcccgtactgccccatgcgcacgacaggcaccggagccacggccgattcggccagcggcgcgagcatggcagccgccacgcgtgcggccgcgccttcggcttccgggctgccggcttcgaacagctcgaccttgcagccggcctgtgcgagcttgaccgcaagcagccggcccatgaggcccgcgccgaggatggcggcggattgaaatggcaggctcatggcattgctccttccccctctgggggaaggccgggatgggggtagccagagcgcacaacggatacgccgcttgcccccaccccaaccctcccccgggaggggagggagcaagacaacgccagtcgccgataattttcggcatgacccaagcactttccgacgacgcggcgcaagcgcccctgcgctatgtgcgcgtgctctcgatcgccggctccgacagcggcggcggcgccggtatccaggctgacctgaagaccttcgcggcgctgggctgctacggcatgacggccatcaccgcgctcactgcccagaacacgctcggcgtgtcgggcattcacagcgtgccggcggcttttctcaaggcgcagatccaggccgtggtcgaggacatcggcgtcgatgcggtcaagctcggcatgctgcatgcgcccgaggtggtcgaggtggtggcctgggccatcgatcactaccggctgcccaacgtggtgctcgacccggtgatggtcgccaccagcggcgaccgcctgatcgcttcggaaaccgtgcaggtcctggtgcgcgaattgttcccgcgcgccgtggtcgtgacgcccaatctcgacgaagccgccttgctcatcggccatgccatcgacggcattgatgcgctcgacggtgcggccgacgaattgctggcgctcggtgcgaaggccgtgctgctcaagggcgggcacctgcctggcgatgacgtggtcgacgtgctgctgcaggcaggcggcacgcgcaagcgcctggcctcgcagcgcatcgcaagccgcaacctgcacggcacgggctgcacgctgtcgtccgccgttgcggcgcatctggcgctgggcttcgggttgcccgaggccgtcgaacgcgcgcgtgcttacgtcatcggcgccatggcggccggggcggatgtgcatgtcggcgcaggccatggtccgctcaaccacggctttgcgccagtgccgacgcaccgcctgccgtcgtagacgtgggcttgggccggctgatccaggccaggaggaatgtggccgccagcgtcggcagcgccgagccgaactgcggcgcccacttggcgcaggcgtgataggccgcgatgcccgcaatccagatcagcgccgcgcccaggtcaacccggcgtgtgccgctcgatgaaatggcttggcccgtgcccagccgccccaggatcacgccgtagagcggcacgaacaccgaactcagcatcagcaagaacggctcgagcgtgtgcatcggcagcaccagcgccagcgcggtgcacagcgccgccagcagcaggccccagcgccgcacgctccagcgcggcagcaggctgtgggtcgataccgagcccgagtacacgtcgccataggcgttgtcgagttcgtcgatgaggatcaggccgagcgccaccaggccgccttgggcgagcagcagggcggtgaccagaccggtgcccggctccgccacgctcacgaccatcacgccgagcgaatagcaccagatgttggccagcgcgtagccgagccaggtgccggtgaatgcgctgccgaggccgcgttgcccgctggcgttgcgtttgccgtgacgcgcatagtcggccaccagtggcagccacgacaccggcatcgcaatcaccaggtcgagcgcgctgaacatgcccatgccgccggctcccggccgcgcccagaaggcgtccagccccttggcctgaagccgcgtcgcgaactgccaggtgagccacagcagagacagcaccaccagcggcaggccgaagcggctgacgaaacgccgcaccagcttgaccatggaacccgcgagcagcgccagcagcaccgcgccccagagcagcgtggtgagggcgtcgcccagtggtccggtgagcgtcaaatcgaacgcctgctggccgatggcctgcgtgccctcgcgcatgatgacgagctcgaaggtggtccagcccaccagctgcacgatgttgagcagcaccggcagccgcgcaaaggcgctgccgtaggtggcgtgcatcagcccggcgcttgccaggccgctttcgcagcccagccgcgcggtccaggccagcaggccggcgcccagcagggagcccagcacgatggcgatggccgcgtcgcgcgtgccgacggccggcaccaggtaggcgccgatctgcatcaccagcagccctacgcccaggctgaaccagagcgaggcgtggtcgtgccagccgaacacgcgctgcgacgcgggcagcggcgtcagcgcctcgttggcggaagaaaagtcgtcgtgtgccatccagttgctccaatgcaaaaggtttggcaggtgggcgaggctccggcagcggagccatcgcgcgagacaacgcgacaggccgccggaccagcttccctgcgcgaggattacctcggacctcctaagtaaacaaaggagatgcaatcaggttcaaagggactttctcagcagggacggcaagccgccctagcacccctagcgaacgagtattttaggctcccacgccgcgagcggctcgaaaagttgcggcacacgacagaatttggcggcggattcacccgttaaccgccgctcgctgaagcggtcgcctgagacacccccctttgccgcccctggttcgtcggcatcgggcgggccctggaactaggctgcgcctgtgcgcgggcctaaaatgttcgtccctgtaatcagcgggagcggcagtgttgaatgcctttgccgacgcgcagctcgctcgtgcacggcgcgatcgccggctggtgggggcgtgcctggtgctgctcgttgctcttgcgtggctgtatctggcaatcttggccgaagcgacggcagcgatggacagcccactgcacagctcgcgcgcgatgtggctgatgccgatgggagagtggggcgcgcgggagttcgcgctcggcttggccatgtggacggtgatgatggtcggcatgatggtgccgagtgcggcgccgatgctgttcgcgtatctgaacgtgagccgctcgcggcctgcaggactttcgccaatcgcagcgacggctgctttcctgctcggctacctgctggtgtggggcggcttcagcgtgattgcgaccgccgcgcaatgggcgctgcacgcaaccgagctgctcggacccacgatgcgcagttccagcgcctcgttgaacgcgctgctgttgatcgtggcgggcgtctaccaatttcttcccatcaagaacgtctgcctgtcgaagtgccggcttcccctcggctttctgctcaccgagtggcgcgacgggtggaccggcgcggtgaggatgggcctgcggcacggcgctttctgtgtcggctgctgctggctgctgatggcgctgcttttcgtcgcgggtgtgatgaacctgctgtggatcgcgctgctgtctgccgctgtgctggtggagaaggcgctccccttcgggcgtcaggccgcgcgcgttgtcggcgcgttgatggtcgcggcgggcctggggatcttggtgctgggctgaggccaggctcgtgcctggaaattcgactcgccgttgcctatactttgtgtgaggctgggttgcgtgggcgttggctgtttcaggcggccgaaggagacgacgatgacttggcagatggatgcgacgatgctcgagatgtgcaactgcaaggcgatgtgcccgtgctggctcggcccggataccgtcccggaccagggttggtgcgccggcgcgttgctgatcgacatcgagaagggcgcgatcgatggccaggacgtgggtggctgccgcgccgcgctcgcggcctggtggcccggtaatttctttgctggcaacggcacggcccgcttgtacctggacagcagcgccagcgacgcgcagcgcagcgcgctcgaagctgtgttttcgggcaagaagggcggcatgttcggtgccgtgctcgggccagcggtcacgaagtggctgcccgcgaagagcgtgccgatcgacattcaaggcggcgacgtgccgtctttctcggtgggcgacgtcgccaaaggcacgctcacccgctacaaggacggcgcgggcaagaccgcaacggtgcagggcacggcggcgcagggggccttccagagcacctcgatggagattgcgagtgcgaagggtacgcgctggaccgagcccgatgtgcgcgactgggagggcgactccggcacgctgcacaaggtccactgggccggctgaacggcgcggcgcgttgtcgctcgacgtgccgaaaattgcaacacagccccgggggcggacctgtccgcgtcttacgtctttgcgagcctgcgcgcaaaagcttccaaaccatcgatgacgatctggatatggcgctcgaagctgctgtccagcggcacggtgctgccgttgtcccagcgcacgatgaaggcctggttggcaagcagcggcaggttgcgcgtgagcaccgggtggtcgagcgggcggatggtgtggacgcgctcgcgcagttcctcggcccaggcctgggtgttgtccgagggcaagggggaaaactccatcgtcacgaagcccagcatggccgcgatcacgcagttgtaggcctccagcagcggcagtccctcgaatccggcctcgaccagggccgcgagcacgccttccaccagctcggtgggcaggctgccgttcgacaccagttgcgcgcccagcagctgcgccacgttcgggtggcggcgcaccgcggcgcggcagcggcggaacagttgcgcgatccattcctgccagccctctttgccgggcggcggcgtgacgtcggccatcaccatggcggccacttcggcgagcagcgcttcgcgcgtgctcacgtgccagtgcaccgtggccggatagacgccgagccgcgccgcgatctcccgcatgctgaaagcgccaaggccgaactcgtcgatgtgcgccagggcggcctcggcgatgcgccgcttcgacagcgcgccgccgccggcgggccggccggcggtcttgggtttgggctcggcggcggttttcttcatggatgctgccattgtgcggtggggaaattgattgtataaataatattaattgagcgatgatcaattaattgattgaaactgaaagccccatcggctctttcgaggacaccctatgaccgacgccatcgacctcgccctcgcagaggcgcatcaacgcttcaccgacggcaaccccgcgagccggcgccagttcgaggagcaggtgcgctacatgcccggcgccaacacgcgctcggtgctgttctatgcgccgtttccgctcaccattgccaagggcgagggagcagcgctctgggatgccgacggccaccgctacgccgacttcatcgccgagtacacggctggcgtctacggccactcggcgcccgagatccgcgacgcggtgatcgaggcgatgaagagcggcatcaacctcacgggtcacaacctgctcgaaggacggttggcaaagaccatctgcgagcgctttccgcagatcgagcaattgcgcttcaccaactcgggcaccgaggccaacctgatggcgctcacggccgcgctgcacttcacggggaggcgaaagatcgtggtgttctcgggtggctatcacggcggcgtgctcggcttcggtgccggccccttgccgacgaccgtgcccttcgacttcctggtgctgccctacaacgacgttcagcttgcgagcgaacagatcgcgaagcacgggccggaaatcgcggccatcctggtcgaaccgatgcagggcgcgagtggctgcattccggggcgactcgacttcctgcaggcgcttcgcgatggcgccacgcagaccggcgcgctgctggtcttcgacgaggtcatgacctcgcgccttgcgccgcagggccttgccaacaagctgggcatccggtccgacctcaccacgctgggcaagtacatcggtggtggcatgtccttcggcgccttcggcgggcgggcggacgtgatggcgcagttcgatccgcgcaccggttcgcttgcgcattcgggcaccttcaacaacaacgtcatgaccatggccgccgggtacgcgggcctcacgaagctgttcacgcccgaggcggcgggagccttggccgagcgcggcgaggcgatgcgggcgcggctcaatgcgctgtgtgcgaaggagggcgtggccatgcagttcaccggcgtggggtcgctgatgaatgcgcacttcctgagaggtgaggtgcgtcgcgtggacgatctggctgtggtcgacgggcgcttgcgccagctgctgttcttccacctgctgggccagggcatctacgcgtcgccgcgcggcttcgtcgtgctgtcgctgccgctgacggaggcggacatcgcccgcttcgtcgccgccatcggcagcttcatcggcgagtaccggacgctgttgcctagcgcgaagtagccacgcccagcagttcgtgcagccgcgtgctggtggtcgtgtactgcagcggcaccgccttgcccgggaacacgatggcggtggcgccccaggccgccagcgtggcttcgtggaagccgcagacgatgagtttcttcttgcccgggtaggtgttgatgtcgcccaccgcgaacacgccgcgttcgcgggtttcgtatttctcggtgtcgaccggcacctgcttgcgctcaagctcgaggccccagtcggcgatggggccgaggcgcggcgagatgcccaggcaggcgaccagcgcgtcgagcggcaggtcgatggtggttgcgtcgggcgtggtgatctgcagttgcttgccgtcgaaagcggcgggctggccgaccttgaaggccagcttgcccgcggccacgagggcgcgcatcgcggcgatattcgcctcatcggcctggaaaccatcgcgccggtggaccagcgtgacctgcttcgcgatgctcgtgagcgcaaccgcggtttcgagtgcgacatcatcgcccccgttcaccaccaccgcctgacccacaaagcgatctagcgattcggggtgatagaaaagcgagctgccttcgaactgcgcaatgccttcgattgcaatgcgcttgggcacgaaggcgccgacgccggccgcgatgaacacggtcttggccaggaaggccgtgcctgccgaagtcgtgagcaacaggcgctcatcggcctggcgggcgagcgtggcgacctgttcatcgaaatggaactgcggcttgaacggcgccacctgctccagcagcgattgcgcgaggccgcgtccgctggtgaccggcgtgccgggaatgtcgtagatcggcttgtcgccgtagagcgccacgcactggccgcccacggcgggcagcgcatcgacgatgtggcaggagatctcgagcaggcccagctgaaaggcctggaacaggccgacagggccggcaccgacgatcagcgcgtcggtttcagtggggactgccgaggcgctcagcgcaccagctccccgatcttgtcggtcttgtctttccactcttcggcgtcggggagagccggcttgcgcttggtgatgctcttccagccgtcggccagcgcgagctccgcgttgagcttgatgaaggcgatctggttggccgggaggtcttcctcggcgtagattgcattgaccgggcactcggggatgcagaccgcgcagtcgatgcattcgtccgggtcgatcaccagcatgttggggccttcgcggaagcaatccacggggcatacgtccacgcagtcggtgtatttgcaacggatgcaggcttcggagacgacgtgggtcatttgtcttctaacgtcagtgtgaggtcggggaaaaccccagattttaggcctttgcggcggcaggctgcacgagcacggccgcagcggtcttgtgggaggccgtatcgaccagcaccagggagcccaatgcacgcgattgcgtgaagggcagcacggccagcggctgctgcagcgccagcaccacgtcgccgatggaattggcttccagctgcgttgcgggctccgattcgagcgtcgtgatgttcacgcgatcgacgatgcgcgccaccttggccttgacccagcggtggccctgcagcgcccaatacacgcggcccgcgaccagcggttcgtcgtcgagccaggccacggtggcggtgatttcgcgcaccggctcgaaggcgccgggcgccagcagccagtcgccgcgcgacacgtcgagttcgcggtcgagcacgatgccggcactgtggcccgcatgcaccaccttcggttgccgcgtgtggctcagcacctgcgcaaccgtggcggtctggttgctcggcagcaccgtcacgcgctggccgggttccacatggccggcagccacgcggccccagaacacgcggcggccctgcgaggtgtcggccgaggaagagaacttctcgacccactgcaccggaaaggcgaagggcacagcctcgtcctgcgcggtgaccggcagctcctcgagcagctcgagcaggctcgggccctcgtagccgacccagtcggcatgtcgcgtggccacgttccagcccttgagggccgagatgggcacgatgccggcaacttcgacgcccgccgcttcggcaaaagcgttcagcgcggtcgagatgcgctcgaaggccagggcggcatcgtcgatggcgtcgagcttgttgatcgcgaacacgatcgactgcacgcgcagcagatgggccagcagcgtgtggcggcgcgtctgcggcagcagctcgcgcttgacgacggtgccgtcttccacttcggcggcccaggccagcttggtggcatcgaccagcaccacggcggcatcggcggccgaggcggcggtgaccatgttgcgggtgtactgctcatggcccggcgcgtcgccgatgatgaacttgcgcttggcggtcgagaagtagcggtaggccacgtcgatcgtgatgccctgttcgcgctcggccgagaggccgtcggtcaacagcgccagatcggtttcgccgccgcgctgcacgccggcaagctggtcttgcagcacggtcttgctgtcgaccagcaggcggccgatgagcgtgctcttgccgtcgtccaccgagccgcaggtgatgaagcgcagggcggtgccggtgtcaccgtggagggcggtgttgtcgagggttgccgtcgtcgtgctcatcagaaatacccgtctttcttgcgcttctccatcgaagcttccgaagtcatgtcatccatgcgtgtcgcgccgcgttcgctcacgtcgaccgacagcgtctccagcaccacgtcgccggcatcggccgcgaggctttcgaccgggcaggtggtcgtgatgtcgcccacggtgcgaaagcgcacgtcgcgcacctgcacggtttcgccatcgcgcgccggggtgagttcggtcaccgggaccagcaggccgcgtcgctcgaccacttcgcgcttgtgcgtgtagtagatcgacggcaggccgacgtgctcgcgctcgatgtattgccaaacgtcgagttcggtccagttcgagatcgggaacacgcgaaagtgctcgcccggtgccaggcgcgtgttgaacagcgtccagagctcggggcgctggtccttgggctgccattggccgaagctgtcgcggtgcgaaaagatgcgctccttggcacgcgccttttcttcgtcgcggcgggcgccgccgatcagcgcgtcgaagcggaattcttcgatggcttcgagcagcgtgaccgactggtgcgcgttgcgcgattcgccaggatgcgccaggcgcacggtaccgcgcgccatcgaatcctcgacgctgcgcacgatgagttcggcgcccagttccgtggcgcgctggtcgcgataggccgtcacttcggggaagttgtggcccgtgtcgatcatcagcagcggatacggaatgcggcccgcgccgaaagccttttctgcgcacttcaggagcaccagcgaatccttgccgcccgagaacaacagggtggggcgctcgaaggcggctgccacttcgcgcaggatgaaaatggtttcttcctcgagcgcgtcgaggtgggtgttggacaggtgcgcgggagagtgcatgggcggcaccagcagttcggtttcggtacgggcgttcatcggatggggtgctgaatacgaagattcggtgcggcggcgttggcgctcaatgcgcaagatgcaatccgcactcgcggttgtcttcgcccttggtcgggtccacgtagtcgaagttgttgggcaggccatgcgcctcgcagtaggcgtacagctccttggacgaccagtgcagcagcggcgcaaccttgatcaggccgtccggattgacgctgaccgggtccatctgcgcacgcacggcggtgtcggtggcgcgcagtgcggtgaaccagaccttcggcgccgtctcgcgcagcgcgcgtgcaaagggctccagcttcacctcttccgtgaaagcggcatggcgcggatcgtcgagcgccggggtcgggccctccaccgcttcacgatgcgcacgcgagcggcgcggcaggtagatgtgtagatgaaggcccagcagtttcgtcacctcgtcggcaaagcggtaggtggcttcggtgttgtagccgttgtccatccagaccacgggaacatcccgctttgcgcgcgtgaccatgtgcaggatcacggcctcgaaagggcggaaattggtggtgatgatcgaaggctggccgaggccgatcgcccagtccaccaggccctccgagttgcggccgagttcggcgttgatgcgtgcgaagtcgatgtccgtggcgatgctcatgtctaaggtttccaatcgggctcaggtgccagccgcaaagtgcggcgcggtcttcaccgcatcgccctggtagaaggcggaaaaacgatcgaactggcgctgcgcgtcggtggcatccacgccttccttgagcacggcgctggagaagccggtgcgttccatctgcaccagctggtcgatcagcacgtcgccggtggcgcggatgtcgcccttgaagccgaggcggcggcgcagcaaaaatgcctggctgtaggcgcggccatcggtgaacttcggaaagctcaggtcgatgcgctcgatgtcttccaggcacacctcgatggcgagcgggtcggcatcgttcggcagttgcaggaccttcggatcgccgtcgtcgatatgctcttcggcggccaggatgttgagatgcctgttcatgctgcttcctccaccttgaaccgcgcgccgttggcggcggccttgaacgggtcgtggccgacgcggcgcaaggtgtcgatgaaggtttcgccgccctcgcgggtgtcgcggtacgtggtgagcacggcctcgatcacgcccggtacttcggccgccgagaaagaggggccgaccgccttgcccgcctgcggggtgccgctgagtgcggagccgtcggagccgcccagcgacacctggtaccactccttcccgtccttgtcgacgcccaggatgccgatgtggccgctgtggtggtggccgcacgaattgatgcagccgctgatgtgcaggtcgatctcgcccaggtcgtcgagctcgtcgaggtcttgatagcgctcggtgatcgcttcggcaattggaatggaacgtgcgttcgccagcgagcagaaatcgccgccggggcaggcgatcatgtcggtcaagaggtgcacgttggcgctggcaaagccggcggcgcgggcggcaagccacagtgcatgcaggtcttcggcatgcacccagggcagcacgatgttctggtcgtgcgtgacgcgggcttcgccggccgagaagcggtcggccagcacggcgagcgtgtcgagctggtcggccgaggcatcgccgggcgcctgcttcaggcgcttgaacgacaacgtgacagcgcgcagcgcggggttcttgtgcggggccacgttgcgggccagccagcgggcgaactgcacgtcgtccgcggcgtgggcgcgcagctcggcgtcggtcttctcggcgctttgcagcacgcgggtggcgagcgtcggcggcacgaaggaggcggccacgcggtcgtactcttcctgcgtgatggtgtgcggtgcgccgtcgtgctcgaggatctgcttgtactcggcctcgacgtcgtcgatgtagcgctggccttcggccttcaccaggatcttgatgcgcgccttgtagatgttgtcgcggcggccatagcggttgtagacccggatcaccgcttcgaggtaattcatgatctgctgccagggcaggaactcgcgcagcacggtgccgatgatgggcgtgcggcccatgccgccgcccacctgcacgcggaagcccacatcgccaggggcgatgttttgtgatgcatcgccagcctcgtgtttcaccacgtgcaggcccacgtcgtgccagccggtggcggcgcggtcttcggtggcgccggtgatggcgatcttgaacttgcgcggcaaaaaggcgaactcaggatgcagcgtgctccactggcgcatgatttccgcgaacgggcgcggatcggcgatctcgtcgatcgcgatgccggcgcgctcgtcgctcgtgatgttgcgaatgcaattgccgctggtctggatgccgtgcatgtcgaccgaagccaggaggtccatcacgtcggccgactttgaaagcggaatccagttgtactgaacgttctggcgcgtcgagaagtgggcgtagtgcgtgggcagcttgtgcgtgccgagcaggccctgggtttccagcgccttcttgtagacctcggcctcgggctcgtcgtactcgcgggcaatgcgggccagcacgcgcagttggcggctcgaaagctcgccatagggcacggccacgcgcagcatcggtgcgtagcgctgcacgtaccagccgttttgcaggcgcagggggcgaaactcgtcttcgtggagacggcctttttgccagcgctcgagctggtcccggaactgggcagcccgttgatgaacgaactggcgatcgaattctgtgtattggtacatcgtgcgtgtgtcttgaagaagtgcggtgccgcacgtacaacggggcgccccagcaagaagccgagattctgaaagctggccttatggaagcaaactattttttggttcgcgctttatgcggataagcttattctccagcgcccatgcgggtttccgggcggttgaatgcttattctggataaggcgagagtgctctcaccaggcaaggataacgcccgcgggagatccgcgtttgtccactctctcgctggggagagagcagttgggcaaggtcaccgttgccggccctcaccccagccctctcccggagggagagggagtaatactttcagcgcagcatcgacgacatcgccgaacagcagttcagcatgcgcaccgcagcttccacggtttcggcggtgaagcgcagggtcacgccgtcgacgcgctcgaaggctggccactggcagaacagatcggccatgcccggcgactgggtgcgcagcgtgaccacctgcgggcccttcaacaccagcggacttgcgttggcgcgcccggccagcgcctccgccacgccggcccggatcgcctcgcgcgactgctcgggcgacagcgacacgccgctgttgaaccccgtggcgcgtttggtctggacgaaggtcgcatgcggaaagagcggccggttctcgtcgatgaacacgtcgtcgccgctggccatgaccaccggcgcgccgtattcgccggccagcgccccatagagcccggcctcgcccagctcctggtcgccgagccagatgcctgcaaaggcaaagctgttgatcgtgtgcgccaggatgccgcgcccctgcgcgcgcgagtggtagccgaccatgcagaccgcgtccacgccttcctcgacgccggccaccatgctgaggtagcgcggcttgccctgcaccacgcgcgcgcgcgcatcgagcacgtcgggcggcatgttgcgaaagccgccgtgcgagtcgttgaccagcacttcggcggcgccggcatcgaaggcgcccgcaatggccgcgttggcctcctctgccatcagcaggcgggcgcgctcgaattcggggttgccggagcgcacctgctccgagtggtaaacgccggcaacgccttcgatgtcggtggagatcagaactttcatggggcgtgtggcggtgcaagagaagaagaaacggaggagggcagcagctcggccagcgtcggccggtggttgccgtcgcgcccggtcacggccgtggcgtgccacagcgcatgaagaatggcctgctcggtgctgtcggccgcggcctcgaacaggccgtcgagcaggctctcgtgcaccatcgcgatggccggcatcgggcgttcggcgcggtcgggcagcgtgcaggcggtcgagaaggccagcacgatgtcaccgctgccatggccgaagaccgagccggtgcgtgccaggccggcgcccgcgcgcaaggccagccggcgcagttggcgcgcgtccagcggcgcgtcagtggccaccacgatgatgatcgagcctttttcgggctccctcgatgtccggctgccttctgcggccagcctggacaccagttgctcgccgattgcctggccggccagcaccaattgcgatgggcggccgtagttggccagcaccagcgtgccgaccgtgtgcacgccgccatcctgcgcggacacccggcgcgaggcgctgccgatgccgcccttgagctggaagcacgacatgccgcgcccggcccccacggagccttgcgcgaagtcgctgccggcgtcttcaagcgcacgcaggtagtcggcctcgctcacggccaggcgctgaatgtcgttgagaaaaccgtcgttgcactcgaacaccagcggattgaccgtgggcagcgaccggccgctctcggggttggcggccacgcagtggcggatctgcgcggtggccaccgtgcccaccgagtaggtgttggtgagcgcgatcggcgtctcgagcacgccgagctcggccatctgcaccagccccacgctcttgccgaagccgttgagcaccacggcagcggccggcaccttgtcgcggaacgggtcgccggcatggggccggatcaccgtcacaccggtttgcacagggccgtcatcgagcgtccggtggcccaccgtcacgccttccacgtcggtgatcgcgttgcgcggaccctggagcaggttgccgatgcggggaggattcgatgtcattgaagaaaggagggcaggctactcgcggtcgatcttcgggtcgagcgcgtcgcgcagcgcatcgcccagcaggttgaaggccagcacagtgaagaagatggccaggctggggaacagcgccacgtgcggcgaggtcaccatgtcggcgcgggcttcgctgagcattgcgccccattcgggcgttggcggctgcgcgcccatgcccaggaacgaaaggctggccgccgtgatgatcgaagtgccgacgcgcatcgaaaagtacacgacgatcgacgagatcgtgcctggcaggatgtgccgcacgatgatggtccagtccgatgcgccgatgctgcgctcggcctcgatgtaggtctgctgcttgagcaccagcgtgttgccgcgcaccaggcgcgcgaaggccggcacgctgaacaccgacaccgccaccaccacgttggtcatgctgctgccgaggatggcgaccacgcccagcgccagcaggatgccggggaaggcgaacagcacgtcggagattcgcatcacgatgcggtcccaccagccttcgtagtagcccgcgagcaggccgaaggccgtgccgatgaagccacccaccagcaccgaaagaaagccggccatcagcgagatgcgcgcacccatcaagatgcggctgaagatgtcccggcccagcgggtcgacaccgaaccagtgcgtggccgaaggcccggtgttcagcatgtcgtagtcgaagaagttctccgcgtcgaagggcacgatccacggcgcgaacaccgcgacgaacaccagcagcagcacgaagagcgcggccacgatgcccaccggctgtttcttgaagcggcgccagcattcgccccacggcgtgcggaccttgcccgcggtttgaaccgccactacgggcgggacgatgatttcggcagacaggccggtagcttgcgtcatggctgcttgctcacttgtagcggatggtggggttgatgaagccatacagcacatcgaccaccagattgatcaggatgaattcgagcgagaacagcagcaccagcgtctggatcactgggtagtcgcgcatctgcacagcatcgaccaagaggcggccgaggccgggccagttgaagaccgcctcgaccaggatcgagccgcccagcaaaaagccgaactgcaggcccatcatcgtgacgaccgggatcagcgcgttgcgcaggcagtgcttgatgatgacggtgcgctcccgcacgcccttggcgcgcgcggtgcgaacaaagtcttcctggatcacctcgacgaaagacgcgcgcgtgaagcgcgccatcacggccgccacggcggcgcccagcgtgatcgagggcaggatgtagtgcttccaggtggcggcgcccacggtgggcagccagccgagctggaccgaaaagatctgcatcagcagcatgccgagtgcaaatgcgggaaaggagatgcccgataccgccagcgtcatgccgagccggtcgggccattggttgcggaacaccgcggagacgatgccgatgcccatgccgaagaacacggcccacaccatgctggtgatggtcagcatcaccgtggggaaaaagcgctcgccgatctccgtcgacaccggccgccgggtgcggatcgatgtgccgaagtcgccttgcagcatgtgggtgaagaagctcacgaactgctgcggcatcggcttgtccaggcccagctcctggcgcaccatggccacggtctgctcgtcggcgtcctggccggcggcaaggcgcgccggatcgccgggcagcatgtgcacgaacaggaacaccagcaccgccacgatgagcagtgtcgggatcaggcccaacagtcgtttgagaaagtaattcagcatggcatacagacaatcaaccctcgtcaaggcctcggggccaatcgggagacaccgcggaaccggctccgccgggccgcaggtgtcgcccccttgagggggaggcggctacacgaagtgagccgcttcgggggtgggtcaattaattgaaatcgcgtcgatgttgatgttgccgtcaggcatcacgaacacacccgacaggcgcttggaatgcgccgacaggttctgctcggtaatcagcggcacgcgcggcaggtccttgcggatctcttcctgcgcggtcttgtagagcgcggccttttccttgtcgtccacggtaatcagagccttggccagcgcgttgtccaccacttcgctcttgtagaacgacatgttgttcagcttcggcgaccaggcttcggaggcgaacagcgggcgcaggccccagtcggcctcgccggtcgacgacgaccagcccgtgtagtacatgcggaccttggccgtcttcggatcgggccatgcatcgacctgctcggtgcgctggcccacttcgagcgcctgcacctgcagcttgatgcccacttgcgcgagctgctgctgcacgaactggatggtcttctggctggtcgtgttgttgtaggcgctccacagcaccgactcgaagccgttcgggtagccggcttccgccagcagttccttggccttcttcacgtcatagggaatcggcgccatcttctcggcgtacttcacgccctgcggcagcacgccctgcgcggggaaggcatagccgccgaacgcgaccttggccagtgcctccttgttgatggcatagccgatggcttcgcgcaccttcgggttgtcatagggcttctgcagcatgttgaaagccaggaagcgcgtgatgatcgaaggaatggccaccacttcgagcttgtcgctcttcttcagcagctcggcttgttcgtagggaatcgggaacgcgaaatcggcttcgccggtctgcagcatggcggcgcgcgtgttgttctcgagcaccggcttccactggaggttgtcgatcttcggatagcccttcttccagtagccgtcgaacttcttggccttgaccgcttcggtctgcttccactcgacgaactcgaaggggccggtgcccacggggtggaaggcgatgtccttgttgccccacttcttcagcgcggtgggcgaaatcattgcggccgaggcgtgggccagcgagttgatgaaggggccgaagggctccttcagcgtgatgcgcacggtggtggggttgagtgcctcgaccttgcccacgcggttgaactggttgtagcgcagcagcttgttttcctgattcagcacacggtcgagcgtgaacttgacggcttcggcgttgaagtcggtgccgtcatggaacttgacgccctggcgcagcttgatggtgtagaccagaccgtccttcgacacctcgtagccttcggccagaacgttctggaccttcaggtccttgtcgaactggaacaggccttcatagaaggtcttggtcacggccgtggtgatggtcgtgttggtgttgtacgggtcgagtgtttcgggctggtagccgatcgacagcacggcgtctttcgcggccattgccgtgccggtcatcgccagagcggccaggcccagcagtgccgatgcccatcgcagggaggaagaagattgcttcatggaaagaactccggtggttcgagaaaaaagcaggagggcctgcgggttgaaaaaatcggtcgatcaatcagaaggcgccgccaatggcgtgccgcgcgacaaagtgcccgggcgccacctgcaccagcggcggcacgtcgggctcgtcgcccacggcgcggatcgggctcggaatctcgccttcgagcagcgcgcgcggcttgtggcggcgcgacgggtcggccaccggcaccgcggccatcagcttgcgggtataggcgtgctgcggcgcctcgaagacggcgcggcgcgggccgatctcgacgatctggccgaggtacatcacggccacgcggtggctgatgcgctcgaccaccgccatgtcgtgcgagatgaagagaaaggccacgcccagttcgcgctgcaggtcgagcatcaggttgacgatctgcgcctgaatggacacgtccagcgccgataccgattcgtcggccaccaccaccttgggattgagtgcgagcgcgcgcgcaatcgcgatgcgctggcgctggccgcccgagaactcgtgcggatagcgctgcgccacctcgggcggaaggcccaccttctgcagcagccagtcgacgcgctgctgtgcttcggcgcccttggcaatgccgtggatcaagagcggctccatgatcgagaacccgaccgtcacgcgcggatcgagcgaggcgaacgggtcctggaagatgaactggatgttgcggcgcagagcctgcaactcgcgcgtgggcagctcgcggatgttttttccgccgaactcgatggcgccgctctggctttcgaccagccgcagcagcgagcggccggtggtcgacttgccgcagcccgattcgcccaccagcgccagcgtttcgccggggtacaggtcgaagctgatcttctcgaccgcgtgcacgcggcgcttcacgcggccgaaaagaccgctgcgcacgtcgaagcgcgtcaccaggtcgcgcacccgcaggatgggacctgcgtcttcacgcacggtggtttgcggcgtggtgttggtgcacggcacggtgtccgggctgccctcggcgcgcagcagctcgaacttggccggcaggtcggtgccctgcatcgcgcccagcttgggcacggccgacagcagcgccttggtgtaggggtgctgcggcgcggcaaacacggtgtcggacgtgccggcttccaccttgtcgccgcggtacatcacgagcacgcggtcggcaatctcggccaccacgcccatgtcgtgcgtgatgaagagcacgcccatgcgcatctctttctgcagctcgcggatgagctggaggatctgcgcctggatcgtcacgtcgagcgcggtggtgggctcgtcggcgatcagcagctgcggcttgcacgacagcgccatcgcgatcatcacgcgctggcgcatgccgcccgagagctggtgcggaaagcggtcgagcacgttgcgcgcttcgggaatgcgcaccagctccagcatgcgcaatgcctcggcgcgcgcggccgcattgttcttgccctggtggatgcgaatggcctcggcaatctggtcgccggcggtgaacaccgggttgagagacgtcatcggctcctggaagatcatcgcgatgtcagcgccgcgaatgccgcgcatcgtggtgtcgcgtgcctgcgccaggtcgagcacctcgccattgcggcggcgaaacgccatgcgcccgccgaggatgcggccgccgccatgctcgaccagacgcatcagtgcaagcgaagtgactgacttgcccgaacccgattcacccaccaccgcgagcgtttcgccatggtcgacgtggaacgagagattcttgacggcgtcgacggtgcgctcggaagtcgagaagcgcacggtgagatcgtcgacggcgaggacgcggccgtccggcagggcgaggggaggggtggacatgggagtgcgaaggaaggagggcgtcaggcgaagatggccgtgaccggcgtttcatcgccgcgggcatggccgcggtacatgccttcggtgttgaaggcgaggctcaggttgccgtggcggtcgacggcaatcagcccgccggtgccgccaatggccggcagcgactgctgcacgacggcatgcgtggctgcttcgagcgtggcgccgccgtaggccatgcgggcgcaaacgtcgtaggccgccgcgacgcggatgaacatctcgccgctgccggtgcaagagacggcggcggtgcggtcgtcggcataggtgccggcaccgatcaggggcgaatcgccgatgcggccgacgcgcttgttggtcatgccgccggtcgaggtggctgcggcgaggtggccgtgcatgtcgagcgcgacggcacccacggtgccgagcttcttgtcttcgtcgagcggcggcgtcgtcatggccgcgccttcatggtccgtcaccacgcggccggtgccgcgcacgcggtagagctgctggcggcgcgcgtcggtggagaagaaggagggctcgaccatctccagcccgtgttcgcgcgcgaaggcttcggcgccggggccggcgagcagcacgtgggcgccgtcttcgagcacggcgcgcgcggcgcgcaccgggcggcggatatggcacacgccggcaatcgcaccggcggccagggtggcgccgtccatcacggcggcatcgagctcgtgcgtttcgtcgtgcgtgaaaaccgagccatggcctgcgttgaagagcgggcagtcttcgagcagctcgaccgcgaggcaggtggcatcgagcgcggaggcgcccttccggagcagtgcctgagcggccagcacgaagcttcgcaaggcatcgtgataggcctctgcctgggctgcatcggtcgtggcggcgctgatggtgccggcaccgccatgaatggcgatgacgggcatgacgttgttcatcgggaaactttcttctttttcttgcgggcgtcggccgtggcggcggcgccggcgagttgtgtggcggcatcggctcgcggcaggccttgggcgccatgcagccagggccgcacggcctgcaggatgcggctcgcggactggaccgcgcgcggcgcccgcagcgccaccgcgctggtcagcgcctcgatcaacgccagcacgctggtctcgcagttcggccggtagctggtttcggtctggcaatagagcaccacgtcggccagcggcgccagcggcgaactcgggcggtcggtcagcgccagcacggcgcagccctggcccttggcaatctgggccagcgccaccgtgtccgtgaggtagcgcggaaaggtcaggccgatgaacaggtcctgcggcccggcgtgcatcagcgagcgtgccgcatgcgtcacgccgctgacgctggagagcatccgcacgtcattgcagctgccgtccaggccgtgctgcagcagccccgccagccacgcgctggcgccgaagccggcaatgtagacagagcgcgccttgccgatgcgctgcaccgcggcttcgcaggcggcgtagtcgagcgactggcgcgtggcttcgatgttgcggcggctttcgtcgagcgcggtggcgaacacttcggccacggtggtcggatgctcgaggttgccgcgcaggcgctccaccggcgccaccagcgattcgaacccgcgaacgagttcggcgcgaaaggtggcgtagccgtcgaaatcgagtgcccgggcaaagcggttggccgtggcgacggacacgccgacggcggctgcaagctcgtcgatcggcaaggtcgcaacctgcagcggatgctccagcacgaagtcggccacctggcggtgcgaacgcgtcagccgcggcagggcctgcgcaatgcgctgggccacggtggtgccagtgttgtcgacgttggtgctcatgcgtgggttcgtgcacccgaaacggggcatccgatgaaaacgagtttacaaatataagacaaaaaagaaaattttctgtcatttttgatcgaaggagcaaattgcaggccagcaatgggccgcagtcgagcgcttcgacgatcctgtcagccgggcgtgagcccaagcacccagcgcttgaagtgctccagcgccccggaagccgggcggccttcgggatgggcgaagtagtagccctggcgcacgtccaggtggcggtcgatcgggatcacgagttcgccggttcgcagttcgcgctcgatcaggatgcgcggcgcaaggcccacgcccatgccggcggccgcagcggccgtcaccatggtgaagagttcgtagcgcggcccgcgcgaggcgtgcacggtgtagtcccagccttgctgcgcataccagtcgcgccaggcgtgcgcgcgcgtgcccaggtgaacgtggcggcagcgttcgaaggccgattcgtcccacggcccgttggcatcgcgaaacgcggggctgcagaccggcaccatttcgccctcggaaaagatcagcccgccctgggtgttgggccagaactggtcgccgaagtaaatggcggcgtcgtaggcgttctcctggaacgagaagggctgcgaccgcgccgagagattgacggtgatgttcggatgccgacggctgaaatcgggcaggcgcggaatcagccattgcgtggcgaatgtgggcaccacggccacttcgagcacaaaacccatgtcgtggccggcgctgatctccagcgtgtcgcggcggatctggtcgaggtggcggcggatgcgtgccgcgtattcgcgccccgtatcggtgagggtgaggcgccggcgcacgcgcgagaaaagcggcacccccagccgctgctcgagcgcggccacctgccggccgacggcgctctgcgtcagtgccagctcggccgccgcacgggtgaaactccccagccgcgccgaggcctcgaaggcttgcagcgcacccaggttgggaatgtcttttctcatcgttgctattctgcgggcggggctcgcggtttttcgcggcgcttgggacaatggcatgtcggcgagcagcaagaaaggtatttcatgcgtcgtgtggtgatcatcggcggcggcgcgatcggctccgccatcgcttatttcttgaaccgggatccagaggaggaaccgttcgaggtgaccgtggtcgagcgcgatttttcgtacacgcaggcgtcgtcggccctgtcggccagttcgatccggcagcagttctccaccgccgtcaacatcgagatgtcgctctacggcatcgagttctttcgcgcccttggcgaaaccctgcgcgtgggcgacaacgtgcccgacatcggcctggtcgagcccggctatctgtacctggcgcccacggacggcgtcgaagtgctgcgcgagaaccacgcgctgcagaagacgcatgatgtcgacgtgatcttgatgacgccggatcagctggaggcgcgcttcccctggatgtcgaaagaggacatcgcgctcgcgtcgctgggcctttcgggcgagggctggtatgacggctacagcctgttgcaggcctttcgcaagaaggcggtttcgcaaggcgcgctgtatgtgcaggccaaggcgaccgggttgcagcgcgacggccatcgggtgaagggcgtcgaactcgatatcggcaacgtgctccaggccgacgtcgtggtcaatgccgccggtgcctgggccgccaaggtggcgggcatggccggcatcgacctgccggtgcgcggccggcgccgcatggtgttcagcttctcgtgccccgacaccctgccgggctgtccgttggtgatcgacacgtcgggcatctggtttcgccccgagggccgccgcttcatctgcggttttgcgccgccccaggatcgggaccgcgacgatgcgccgctcgaagtcgactaccgggtgttcgacgatttcatctggcccgcgctggccaagcgcgtgcccgtcttcgaggccatccgcatgaccggcgcatgggccggctactacgagatgaacctgttcgatcacaacccgatcctgggcctgcatccggactgcgagaacctgtactttgcgaatggcttctcggggcacgggcttcagcactgcccggcaacggggcgcggaatcgccgaactcatccgctacggcgagtaccgcagcctcgatctgtcgccggtttcgtttgcgcggatcctggaggaccggccgctgctcgaaaagaacgtgatctagccggaggccaggcacaggcgtacgatcgttgcaagcgagggtcacatcatcatgacttcacaggcattgatcgataccgcacaggcactggtcgcaggagacaaggggctgctcgccatggacgagagcaacgccacctgccacaagcgcttcgccaaactgaacattccccagaccgaagacgcgcggcgcgactggcgcgagctgatcgtcaccgcaccgggcctgggcgcatgcatcagcggcgcgattcttttcgacgaaaccatccggcagcgaaccagcgcgggcgtgtccttcgtctcggcgctgggcgccgtgggcatcattcccggcatcaaggtcgacaccggcgcgaagccgctggcgggccatccgggcgaaacggtcaccgaaggcctggacggcctgcgcgagcggctggccgagtacgctggcatgggcgcgcgttttgccaaatggcgcggcgtcatcacgccggggcccggcttgcccagccgcgcatgcatcgaggtcaatgcccacgcgctggcccgctacgcggccctgtgccaggaggcgggactcgttcccgtcgtcgagcccgaagtgctgatggaaggcgaccattccctggctcgctgcgcggaaatcacggaagacacgctgcacacggtcttcgcccagctgcatctgcagggcgtgttgctcgaaggcatgctcctgaagccgaacatggtgctgcccgggcaggcctgtccgcagcaagagagcgtggaagaagttgccgatgctacggtggcgtgcctgctgcgcaccgtgcctgccgcagtgccggggatcgcttttctctcgggcggccaatcggcgcagctcgcttccgcgcggctgaatgcaatgaaccagcgattcaagtcgcggctgccctgggcattggcattttcatactcgcgcgccgtccagcaaccggcgctggatgcctggaaaggcgactccgccaatatggaggtggcgcagaaggcgctcgtgcgtcgcgcacgctgcaaccaggcggcacgccgcggcggctacgacgcgctggcggatgcaccggaagcgggttgaagttcagccgccctttgccgggttcaccagcacaggcgtcgcccggtagctctcgggaaacagcttcttgaggttatcgagcttcggcatgtcgtaaatcacgacgtagccgtatctcggattgcgcgtgagaaagtcctggtggtaggcctcggccgcatagaagggcttcgacatttcgatcgtggtggccaatggcttgccgaaggtcttggcctggttcagctgcgcgatgtagtccctcgccacgcgggcctgctcgatgttctcggcaaacacggtggagcggtattgagggcccgtgtccggcccctgccggttcagctcggtcgggtcgtgcaccaccgaaaaaaagatctgcagcagcttgccgtagctgacctgctgcgggtcgtagttgatgcgcaccgtttcggcgtggccggttcggccggaacccaccttgtcatagcgtgcggtcttcgcgtcgccgccggcatagcccgacacggcgttgttcacacccttgacgcgctggaatatgccttgcacgccccagaagcagccgccggcgaacacggcggtctcgtatttcgcggtgggcggggtcatcaagtcgaacctgggcggcggcacgcgccgggccggctcggcggcgaacgagggcgctgcgtgccaggccagggctgcggccaccagcgtgccggcggcaagtgcgaggagtctcatgcgtcgtccttcaaggcatcttcggtgccaagccgatggtgcgacattgccgccgtttgcaacgggcgtcaatgtcgcttccccgcctcttgccgcgcgagactcggcccgccggtcacatgccggtcacacgccgatcagggcgggcaggggcgagcggcggctgcgcccggccgggttgccttgctggtggcgccttcgtccaccgtgcccagcgggcgcgtgaacgtgcagccataggccgggtccgccaccgtggccgcggtgaccacgtcgtcgcccgccggcttcacgccgtcgcgctcccacttgaccatggcgtcgaaggcttcgacctgttcggcgagcgtgaagtcgcagtgcgagatgccccgaaccgcgcgctgcaccagccagccgccgttgcccttggccgccgcgcgctgctggtagatctgctccatgctgaagggcacgtagaggtcgcccagcgtgtgcagcgtgaccacgggaatcttgaattcgccgttggccttggggatccagcgcaggccgtcggtacggaggcggttggcgtcggccgccgccgtcagcttgagcaccgaggcgttcagggccgtggtccccggcacgtcgccgtcgatggtgtaggtgaagcggttggtgtcgagggtgctcctgttcaggatgccgttgaccgtgccgtcgctgccgaacacaccccacaccgccgcgaacgagccgccctgcgtaaagccgaggtcgaacatcggccgttcgcccccggtgaggttcttcactactgaggcgaacttcaatccggtggccgtcggcgtgcccgggaaggcggtgtacagcgtgccagtgacttgcgccttgatgtccaaccagttgacggtggggtacttgggcaacccggccagcgcctgcgcggcgacctgcgcgcccgagaaatagtcgaacagctcggtgtcgccgagcacgccgcacatcggcactgcgccgttgtacttcaccttgtggttggccgtggcgtaggcctcgtcctcgatggccgccgcggtgatgtggccgcccatcgagtggcccgtgatgtagagcctcgacggtgccgcgagctcgcggccgttggccttggcgatggcgttgaactgcagggccagcgcattggtgtcttcaacgcccgcgcgcacgtcgtagaagttcttgctgtagctcgaggcggcccaggcgtagccgttctggatcaggtagcggcggatggacgggtcgttcaccttcagcaggttgacgtcgccggcatagccgtgcgcgtacatcacgagcttgccgttccagttggcgggcacttcgacgcggtattgcgcgccgcccagcatgccggcccaacggctggtggtggcgttgtcgatggtgtcgccggcatcggccgcgagcgccgcaaaagtggtggcggcgggatcggcgggcgcgaaggaattgcggctgtcctgcaggcgcgtttcttcgggtggaggcgggggagggggcggcgccggtggcgcgggagccggagccggaggcagtggcgtgaaggcaaaaccgttgccgccgccgcccccgccgcaggatgcgacggcaaggctggctgcgagggcaagaaatgtcaggcgcgctgaatgcatgggtgtctctctccgttttcttggtgttgggaagaagcccggcgcagcggagcctcaaccgaccgtagagaacgaccgtgctatttcgctgaaccggcggggcagcgtaggggcgttgccgggcgcgtcggtccgggctttcccgtagctgctatctcctgcgcgacaccgcgagacacctgcgcgcggagggcttcagccttccttgcgccgcgtcaccaccacggtggcatcgaggccgtcgtaggcctcggcatcgccataccagctgccggagatcggcgcggcctgcgccggatcgcgcgtgacgccgacgcgaataagttgcccgctgcccatgaggttgttggtgggatcgaaggcgagccagccgatgcccggcaggtaggcttgcagccaggcatgcgtggtgccggcgccggtcatcgattcgccgggcgcctgggccgcgcggtcgagcgcggcgtcatagagatagcctgagacgaaccgggtggcgatgcccaggcgccgcgcggcctccatcatcaggagcgcgtagtcgcggcagctgccgctgccgagcgccagcgtctgcagcggcgtctgcgtgccttcctcatcgcgcgccttgtattcgaggctctggccgatgtgcgcgttcatgcgcgcgagcacttcgcgcgtgctgttgggctggtcggtgtgcaggaactggtgggcccagcggatcagggttccacccgcatcgtcgtcgtggtgcggccgcaggtaatgctccaggtcgaggcgctcctgcaccgtataggcaaagggcaggaactcggccgccggatcgagcgcgagctggtcttgctgcgccggcacgtgctcgatggtgaaggagcacacgatgcgcagctccgtggcctcgcccatgggctgcaccagcgcaaccgaattcgaatgcgggtcctggatcagccgcgtgaacgactgcgggctcacctgcaggtcggtggccagcacccgcaggtcgtggctgtcgcgtggccggaacatgacgcggtgcagcccgaaggtcaccggtttcttgtagcggtagacggtggtgtgcgtgatgtcgtattggatggccatgcggagcattctcacgtgttggcgtgcgccgtggtggctgcgggcggtcagatgccgccgattgccaggaaatgtgggcctaagcctgcgtgcgctgcgtgcccagcgccttcgccaggttggccggcaatggcagcggttccccatgccattgcgcggccagcagctccgcgcacagggccgcgaagctgagcccgcgcgagcccagtgcggtgcatgcccacaggccgtcctcgtccagcgggccgaccagcgggcggcggtcgcccgatgcgcagcgcacgccgacccaggcgttggcctcgccgcgatcgaagctggcggccaaccccgcggcggcggcggggtgcagccgcttcaggcgctcgcggtttgcttcggcatcggcgtcgttcggcgcgagctcggtgctgtcccggtcgaaggtggcgccggcgagccagagcagggcgccttcgccttcgggcacgtgggcgatcaggtggccgtcgccgttgagcggcgtggcgggcagcgcgagttcgtccgtcacgcggccccacgcgacctgcccgcgcaccggctgcagtggaagctggggagcgaagcggcccgattggtagcctgccgcaacgacgatgcggtcggcttcggccagcaaccggccgtcgtcgccgaacagctgccaccccgccgcgctgtgtgaaacgcgcgcaaccgccgcattgccgcgaaactcgacgcccggctcgcgcagccacgcctcgatcaaacgcgaagggcgcacccagcccgcacgtgcgtgccagagcgcgggcgcatcggcaggcagccccgtctctgccaattgcgccgtgcttgcgggccacgactcattggggccgctgtcgctccatccggcgggcacccgcgcgtcgccctcgggtcggcgctccagcacgccgccagcacgccagtcgcggccttcttccagcaggcgttccagctcgagccacgtgcctcgaatgccggcgcgcgtgagccgcgacagcagggcgtcgtcgggcgagacatgcggcgccatcacgccgaccggcaggcccgaagcgccggcggccgggcgatcggccgcatcgagcaccgtcacctgccatccgcgccgtgccaggctcgccgccacggccgcccccgccagcccggcaccgatgactgcgcagcgcccgggggcctcgacgtgttcgggtgcagggccgcggcggcgcaccgtccacgcaggcgcgaacacgccggcaaggcagtcgcgcttgggtggcaggccctcgcgtctttcaagctgaaagccgttctgagagagcacgtcccgcaccgcgcgggcataggtccaggtggcaaggccggtgccctggcgggcaaagcgtgacacggctttcagcgtgtcgggcgaccacattgcggggttctgctgcgggctgaagccgtcgagaaagatgctgtcggcctcgaaacgctgcgcgcgcagcatggcctgcacgtcgccgatgcacagcgtgagcaagacccggccctggtcgaaggccaaccggtgaaatcccggcagcagcccctgccactgggcggccagttccttggccaacgaggccagctcgggatacgcctcggcagcgcgcagcaggtcttcggcacccacgggatgcgcttcgaccgagacgaaatgcagcagccttggccggttggcgtcctcgcgccaggcctgccaggttgtcagaaaattgaggcccaggccgaatccggtttcgagaatccgccattgcggccgtccgtgccaggcttcgggcaggccgcaaccgcccaggaacacatggcgcgactgcgccagggctccggtttcggtgtggtagatgtcgtcgaagcgctcgctgtacggcacgccgtcggcgcgccaggcgacgggctcggcggccaagacgggctcagttcgaggggggaacgtagccctgggcaacgtcggcgccttcgccgaagaagtgcttttccatctgacgggccaggtactggcgggcgcgcagatcggccagattcagccggttttcattcaccagcatggtttgctgcttgagccaggcggcccaggcttccttgctgacgttctcccacaggcgcttgcccagttccccgggatagggcgggaagtcgagcccttcggcctctttgccgagcttgatgcactgaaccatgcgtgccattttttgatgcctctggtggggaaagcggttgcttagttgattttgctatttagaactgagaactcggtcgttccagtttctatatgtcgtattcagaatacgtggcttcatcgatatgcctttttgagccagacaccatgagccttcgccgcgactttatcaagctttccctgggggccggcgtggccggtgccatggccctgacggcgttgccgtcgtttgcgcagggcgccgcccccgtgacgctgctcaacgtgtcctatgacccgacgcgcgagctttacgtcgactacaaccgcgcgttcgcgaaatactggaaggccaagaccggccaggacgtcagcatcaagcagtcgcacggcggctcgggcaagcaggcccggtcgatcatcgacggcatcgatgccgacgtggccacgctggcgctgggcggcgacatcgacgcgctggtcacgcacggcggcgtggtcaaggccgactggcagaagcgcctgccgcagaactcggccccctacacctcgaccatcgtgttcctggtgaagaagggcaaccccaagggcctgaaggactgggacgacctcgtcaagccgggcgtgcaggtgatcacgcccaaccccaagacctcgggcggcgcccgctggaactacctggccgcctgggagttcgccaagcgcaagtacggcagcgacgccaaggccaaggaatacatcggcagcctgttcaagaacgtgcccgtgctggacaccggcgcgcgcggttccaccatcaccttcgtgcaacgcggcgtgggcgacgtgctgctggcctgggagaacgaagccttcctggcgctgaaggaattcggcactgagaagttcgagatcgtggtgccttccatttccatcctggccgagcccacggtggcggtggtcgacaaggtggtcgacaagaagggcacccgcgccgtggccgaggaatacctcaagtacctgtattccgacgaaggccaggacattgcgggccgcaacttctaccgcccgacctcggagaaggccaaggccaagtacgacaagcagtttcccaagctgacgctggtgaccatcgaccaggccttcggcggctgggcgaaggccgacaaggcgcacttcgcggacggcggctcgttcgaccagatctacacgaagtagggctcacagcccgctccgggctgcacccctgtggctgtcgcttcgcccctctcctgagggggggcggggagaccgcttcccgcatcgaagcctcccggctgtcgattgcgccctaaccaacgaaagccatctgtgtccgttctcctgattgctggcagcccttcggcaccgtcgcgctccaccgccttgctcgaggccgtggccgagcggctggccggccgcaatgcgcagatcgagcggctcgcgatccgtgatctgccggcagcggcgctgctcttggccgactggaaccatccggccatcgagcgcgccatcgcgcaggtggcgcgtgcgcgtgtggtggtcgtggccacgccggtctacaaggcggcttacagcggcgtgctgaaggtcttcctcgatttgctggcgcagaacgcgctcaagggcaagacggtgctgccgctggccaccggcggcagcccacaccacatgctcgcgctcgactatgcattgcggccggtgctgcacgcgctctcggcgcgccacatcctgccgggcgtgtacgcgaccgattcgcagatcacgctgacgcccgagaacgcctaccaggtgcatgccgatctggccgagcggctcaacgaggccgtcgaggtgctcgcgaccgaagggctgaagctgcccgcgacacacggcttcgagccggtcccattttcccgcgtgcgatgtagcgtctgacgggttcttcgtcgaaccctcgctcagccaatctcattttcgttccccattttgaagtcgcccgtacgcggcgaggggacagctttgcccaaaggaatccacccatgaaccccgtagccaccgaagactccgcgctcgaaacgccgcctcgctccatctggcgcgcgctgcgagaccttgccatcagcacgatcgtggtgaccgccgttgcgctcatcgtcggtttcatctcggcctgaaaggacacgccttcatgacttcgatctccattccgcgccgacgcctgctgcagggcacggccgccgcgcttgcgctgccttcgttcgcggcgctggcccaggcgcaggggcgccagcttcgtatcggccaccagaagggggccctcagcatcctcaagggccgcggcacgctcgagaagcgcttggcgccgctcggcgtgtcggtgaagtggaccgagttcacggccggtccggtgcagctcgaagcactgaacgtcggttccatcgacttcggcgacgtgggcgaagcgccgccgatcttcgcgcaggccgcgggggcgccgttggcctacgtggcaaccacgcttccgcggccccagtcggaagccgtgctggtgcccaagggctccgccatcaggaccgtggccgacctgaagggaaagaagatcgctctcaacaagggctcgaacgtccactacttcatcgtcaagctggccgagaagcacggcctcgcgtacagcgacctgaacctcgtctacctgccgccggccgacgcgcgtgccgcattcgagaagggctcggtcgatgcatgggtgatctgggatccgttccttgccgccgccgagaagttgctggaggcccgcatcctggctgatgcgaccggcgtggtgggcaaccgcggctattacttctcgtcgcttggctatgtggcgaagaacgccgacgtgctggccattgcgatcgaggagatcaacaaggtcgacgtctggggcgccgcccacaagaacgagctggcagccgagttcgccgcgctgtgggggctgccccaaccggtggccgaactgaccgtggcgcgcgcggcctatggcaccacccccatcagcaaggccgtgctcgccgagcagcagaagatcgccgacaccttcttcgacctgaagctgatcccccgaaagatcagcgtgctcgaggccgccgcggcgggcacgttgtgacgcagccgttgcaggaccgcgccgcacgcgtggtggccaccaccacgcgcgcctggggcattgccggacagcaacggcgcacacgtgccggctttccgcgcctgcgcttcgcactgccccgcgtgcgcggctttttcttcgccatctgaggggccgcctggcccgaaccgacggaagacgacatgcagatattctggtttctccccacccacggcgacagccgctacctcggcacgagcgagggcgcgcggcccgtcgatctggcttacctgcagcagatcgcaggggccgccgacaacctcggctacgaaggcgtgctcattcccaccggtcgctcgtgcgaagacccctgggtgatcgcctcgagcctgatcggcgcgacgaagaagctcaagttcctggttgcggtgcggcccgggctgcaccagcccagcctcgctgcgcgcatggccgcgaccttcgatcggctctcgggcggccgcctgctggtgaacctggtgaccggcggtgaccaggccgagctcgaaggcgacggcgtgtacctggaccatgcggcgcgctacgagcagtcggccgagttcatccgcatctggcgcgagattcttgcgcgcagccatgacggcctgggcttcgactacgagggccgccacctgagcgtcaagggcgccaagctgctctatccgccggtgcagaccccctatccgccggtgtggttcggcggctcgtcggtcgccgcgcacgagctcgcggccgagcaggtcgatgcctacctcacgtggggcgagccgcccgccgaggtggccaagaagattgccgacgtgcgcaaccgcgcggcgcgcaagggccgcaaggtcgagttcggcatccggctgcacgtgatcgtgcgcgaaaccgaagacgccgcatggaaagccgccgaagaactgatcagccgtgtcgacgacgagaccgtgatccgtgcccaggccgccttcgcgcgcatggattccgaaggccagcgccgcatggcggcgctgcatgcgggcggcgccaggcgctcgcgcgccgaactcgagatttcgcccaacctctgggccggcgtggggctggtgcgcggcggcgcgggcaccgcgctggtgggcgaccccaagaccgtggcggcgcgcatcgaggaatacgccgcgctaggcctcgacaaattcattctctcgggctacccgcatctcgaagaggcctaccgcttcgccgagcttgtgtttccgctgctctcgcgcaaggcgcagacacggcttgcgggcggctcgctcagcgggccgttcggcgaagtggtcgccaatctcgacgcgccttcgcgtctcgcttcccaaagctgaggacccccatgacggaacaagtgcaagaactgccggcggtcgcgccttcagaagaaaacgccggccgggcactccgggccttcggtgccaacgtggcgggccggctggtgccgtggctcgtgccggtggggctgatcgtcttctggcagattgcttcatcgctgggctggctctccacgcgggtgctgccggcgccggttgacgtggtcaaggcggcgtgggggctggcggtgtcgggcgagctctggacgcacgtcaaggtgagcgcgggccgtgcgctcgcgggcctcgccatcggcggcggaaccgggctggtgctgggccttttgacaggatcggtgaagttcttcgagacgctgctcgactcgaccatccagatggtgcgcaacattcccgcgctggcgctcatcccgctcgtgatcctgtggttcggcatcgacgagtcggccaagctgtttctgatctcggtgtcggtgttctttccgatctacctcaacacctttcacggcattcggaacgtcgatccgcaactgatcgagatgggccgaacctatggcctctcgcgctggcagctgtaccgcgaggtgatcttgccgggcgcgctgtcgtccatcctggtgggcctgcgcttttcgctcgggctgatgtgggtgatcctgatcgtggccgaaaccatctcggcgcaggccggcatcggctacctcacgatgaacgcccgcgagttcctgcagaccgacatcgtgctggttggcatcctgctgtatgcgctgctcggcaagctggccgacctgttcgcgcgcgggctggagcaatggtggctgcgctggcatcccggctaccagaagaagccgaagtgagggcagggcgcatgacgacctcttccacaatttcgcgccgcacggccatcgcaacgctgggcgcactgggtgccggtgcggtgctggcccagggcgcaacggcgcggcctgccacggtgcggctcggctaccagaagtcttcgacactgaccgcggtgctcaaggcgcagggtacgctcgagaagcagttggccccactcaatgtcacgctgagctggcacgagttcaccagtgggctgccgctactcgaggcgctgaacctcggcaatctcgacatcagcgccgacgtggccgacaccgtgccggtgttcgcacaggccgccggtgccgacctgacctttgtcgcacaggaggcaccttcgcccgccgcgcaggccatcctcgtgcgcgaagactcgccgctcaagtcggtcgccgacctgaagggaaagaaggtcggtttcgccaaggcggccggcgcacactatctgctgatcgcggcgctggagaaatccggcctgtccttcaaggacatcgagcccgcctacctgacaccggccgacggccgcgccgccttcgagcgcggtgccatcgacgcctgggtggtgtgggacccgttccttgccgcggcccagcgccaggccagggtgcgcgtgctcgccgacggcaccggcatcgcctcgtaccagcgctactatcttgccgggaccccgttcgcaaaggctcgcccggacgtacttcgcgtggtgtacgccgagcttgagagaaccggccagtgggtcaaacagaacccgaaggaagcggcggcgctgctgtcgcctgtgtggggcctcgatgcggcgacgatcgagcaggccaatgcacgccgaagctacgcggtgcgccccgtcgtggccgaggcgctgaccgaacagcagcgcatcgccgatgccttcttcgcggagaagctgcttcccagaaagatcaacgcgctcgacgtggtgctcttccaaccgaggctgaaatcatgagtgccgttctgaaagacatccagcaaccggccatcgccggcggtgttcgcctcgaggcgcgcgggctgcacaagcgctatggcgaccgcgaggtgctgcgcaacacgcagctcggcatcgagccggggcagttcattgccatcgtcgggcgcagcggctgcggtaagagcacgctgctgcggctcatcgccggactcgaggaggccagctccggcggtctctacaccgacggcaaggcgatcgacggcctgcacgacgacacccggatcatgtttcaggaagcgcgcctcttgccatggcgacgcgtgctcgacaacgtgacgctcggcttgcccggcgacgccaaggcacgcggcaaggaagtgctcgcgcaggtgggcctggccgaccgcgagaacgaatggccggcgcgcctgtcgggcgggcagcgccagcgggtgtcgctcgcacgcgcattggtgcatcacccgcgcctgctgctgctcgacgagcccctgggtgcactcgacgccttgacccgcatcgagatgcaccgcctcatcgaaaacctctggctgcgccaccgcttcaccgcgctgctggtgacgcacgacgtgcaggaggccgtggcgctggcggaccgcgtgatcctgatcgaggacggccgcattgcgctcgacgagaacatcgcgctcgccaggccgcggtcgcagggcgatccggcttttgcggccattgagaaacgcattctcgaccgcgtgctgcagaaggccggagaggcagagcccgccgagacggacgcaagctggcttcagccctcggcgcacacgctgcgctgggcgatctgaactcgttcatccacaaaaacagaaaggcagttgaatgtcgcagaactggaaattcgaaaccctgtcggtacacgccggctactcgcccgaaccgaccacgcgcgccgtggcgccgcccatctatcaaacggtggcctatgccttcgacagcgcccagcacggtgccgacctgttcgacctgaaggtgccgggcaacatctacacccgcatcaacaacccgacacaagacgtgctcgagcagcgcgtggccgcgctggagggcggcatcgcggcgctggcgctggcttcgggccaggcggccgtgacctatgcgatccagaccattgcggaggcgggcgacaacatcgtcagcagcaccgcgctctatggcggcacctataacctgtttgcgcacacgctgccgcagttcggcatcaccacgcgctttgcggaccatcgcgatctcggaagcttcgagaagctcttcgacgagaagaccaaggcggtgttcgtcgaatcgcttggcaacccggcgggcaacgtgaccgacatcgcggccattgccgagattgcgcaccgccacggcgtgccgctgattgtggacaacaccgtgccttctccctacctgagccggcccatcgagcatggcgccgacatcgtggtgcactcgctcaccaagtacctgggtggccatggcaccagcatcggcggcgccatcgtcgattcgggcaagttcccatgggcccagcacaaggagcgcttcaagcgcctgaacgaacccgatgtgagctaccacggggtggtctacaccgaggcgctgggcccggccgcctacatcggccgcgcgcgggtggtgccgctgcgcaacacgggtgcggccatctcgccgttcaacgccttcctgatcctgcagggcatcgagacgctggcgctgcgcatggaccgcatcagcagcaacgcgctgtcggtggcgcagcacctgaagacgcacaaggccgtgaagtgggtcaactatgcggcgctcgaagaccaccccgaccatgcgctcgcgaagaagtacttcggcggcaagtccagcggcgtgctgactttcggcatcggcagcggccgcgagggtggcgcgaagttcctcgatgcgctgaagctcttcacgcggctcgtgaacatcggcgacgtgcgctcgctggccacgcacccggcctcgaccacgcaccgccagctctcgccgcaagagctggcgaaggccggcgtgacggaagacaccgttcggctgtcggtcggcatcgagcacatcgacgacctgattgccgacctcgaccaggcgctggccgcggcagccggctgatccgcatcgcttccatttcccttcactcccattcgaaccattcttcaacccgaaaagagaaacatcatgtccattcaagccatcaacgtccgcaaccagttcaagggcaaggtccgcgaaatcatccgcggcgacgtcgtctccgaagtcgatgtcgaaaccgcctggggcatcgtgacctcggtcatcaccacgcgctcggtcgacgaactgcagctcaaggtgggctccgacgtggtcgcgctcgtcaagtcgacggaggtttcgatcgccaagctctgacggaccctcgagctcgcgaacaacccggcaccgccttggtgccgggtttttttcgatttcgcagtcgggttttccgttcttggcacatggatcgcgggcttctacagtgtcggttacaacgcccggagagaacaccatggtcaacttcgaagtgagcgacatcgtccgcgcactgcacgatgcgcgtaacgagtggcgcgattcgcagcgccgctcgcgtgaacccggcgcgacgcgcgaatttccctcgcgggaggcgctagcgcagatcgtggagctgctcaagggcgcgctctttccgatgcggctcggaccccccgagctgcgccacgacagtgaagatttctacgtcggccatacactgaacaccgccctggagtcgctgcgggtgcaggcgcggctggagctgaacttcaatgcgcgccaccagccgcgtcccgcgagcgagatcgaccaggcagcgaccgacgccgttcgccagttcgcgagtgcgctgccgggcctgcgccggctgctcgacagcgacgtgctcgcggcgtaccagggggacccggcggcgcgcagcgtcgacgaggtgctgctgtgctaccccggcgtgctcgcgatgatccaccaccgctttgcgcaccggctctacgaactcggcctgccgctcttggcacgcatcgtggccgaactggcgcacgcgcagaccggcatcgacatccatcccggcgcgcagatcgacgcgggctttttcatggaccacggcacgggcgtcgtgatcggcgagacggcggtcatcggcaagcgcgtgcgcctgtaccaggccgtgacgctgggcgccaagcgctttccgaccgacgccgagggctacttgcagaaaggcctgccgcggcatccggtggtggaggacgacgtggtgatctacgcaggcgcaaccatccttggccgcgtgacgctggggaagggcgcggtcatcggcggcaacgtgtggatcaccgaggacgtgaagccgggtgcaagcgtaacgcaggccagcctgcagaacgcaccgaagggccacgcgccataaggggtgagccgaaggtccgggcgtcgtcggccacgctatgcttcgccattgttaacaatgttgcttgcatccgcatgtccttgcctcaagccacttcctccgcttcttcttccatgcccccggccgccgacgagtcctgcgatgtgctcgtgatcggcggcggtcccgcgggggccacgatttcggcgctgctcgcgcagcagggccgcaaggtggtgctgctcgaaaaagcgcatcacccccgttttcacatcggcgaatcgctgctgccggcgaacgtggagcttttcgacaagctcggcgtgcgcgaccaggtcgagaaaatcggtatgcccaagttcggcatcgagttcgtctcgccggagcatgagcaccgcagctatgtggactttgccgagggctgggacaagtcgctcgactctgcctggcaggtgcgccgctcggaactcgacgaactgctgttccgcaacgccgccacgcgcggcgcgcagacgctcgaaggctgcaaggtgcgcgacgtcgccttcgatgccgatggtgccacggtgcaggctgaaatggacgacggtgccaagcgcagctggcgcgcccgcttcgtggtcgatgccacggggcgcgacacgctgctggccaacaaattccgctgcaaggaaaagaaccccgaccacaacagcaccgcgctgttcggccacttcaccaatgccgagcggctcgaaggcaagaaggaaggcaacatcagcatctgctggtttccgcacggctggttctggttcattccgctggccgatggcaccaccagcgtgggcgcggtctgctggccctattacctgaagacgcgcgacaagccgctgaaagactttttctacgacaccatcgggctgtgcccagtgctcgtggagcggctcaagaacgccacgcttgtcgacgatgccgtgcacgccaccggcaacttctcgtattcgagcacccatgccacgggcgaccgctacctgatgctgggcgacgccttcaccttcatcgacccgatgttctcgtcgggcgtgtaccttgccatgcacagtgccttcgacggcgcccagctggtggccacggcgctcgacaagcccgccgagttggcgcccgcgcgcaaggatttcgaggccatgatgcgcaagggaccgcgcgaatattcatggttcatctaccgcgtgaccaacccgacgatccgcgacatgttcatgcatcccggcaatccattccgcgtgaaggaggggctgatgtcgctgctggccggcgacatctaccgcggcacgccgatgtggcgggcgctcggcatgttcaagtttctttactacttcatctcgatcacccacatgcgccgcacgtgggaggggtggaagcgccatcgcttcaacatccgcgacatgggcgcgttgaagggcgagacgattctcaagtcggagtagcgtcgcggctggccagtgcggcccgcgcctcgtaggccttgagatgcacgtaggccgtgcgcagcactgaaggcgccggcgattcggcgcgcgctgcgcggttcaacaggtcgccgatgatgtggtcggcctcgaccggcgcgccgcgcacgatgtccttgtacatggacgccgtcatcggcgagcccggcgcggtcatcatcttgcggccgcgctcgatggccgccggccgcggggcgaagccgttgtgcgcggcaatggcgcagcattcgtcgaagatcgcgagcgctacgtcctggccgcctgccgccacgacatcgccgatggatgcgcgcatcaggctcgtgaggcctgccgccgaggcgatgaagatccatttctcccacatgtcctgcgagatggtttcgctcgctgtagcgtcgaacttcgctccggcgaactgcgcctcgatggcatcgatacgcgctgatcggccgcccgcgcgctcgccgaaactcaagccgtgcatgtcgttgaggtgcagcacgcggccttcgtcgtccaaggtggcggagatcatgcaaaggccgcccagcacgcgctcgtcgccgaatcgctcgatcagccgatcgatgtgcttcatgccgttcagcagcggaagaatgaccgtctccggcccgaccgccgacgcgaacgaatccatggtcgagtcgaggtcgtaggccttgcttccgacgaggatcacgtcgaaaggcgcctcgatgttttcggccaccacgtagggcggcgagggcaaattcaagttgccgaaggggctttggacctccagcccgcttttcgcgatctgtgccgcgcgccgcgggcgcagcagaaaggtcacgtcgcgtcccgcctcgagcagtcggccaccgaaataaccaccgagtgcgccggcacccaccacgagaaatctcattgcgattcgctcctgagtcgaaagaacccgagcgatgatgcccgcgatttcgcaagcctgcatcgcgtgccgaaaaggcggatccaaagcgaagagcttttctggaaaaggtcatgggtgcttcgcataatggttttcgccatcccgtctttcactcaatcactcaaggagcttcattcatgagccagacccgaattgccgtgatcgttggcagccttcgcaaggattcatacaaccagaagctggccctcgcgctggcacaccttgcgccctcggacttcacgttcgaacatgtgcgcatcgacgatctgccgctgtacaaccaggacgacgacggcaaccaggcaccctcggtgaagcggctcaagaccgaaatcgcagcggcccagggtttgttgttcgtcacgcccgaatacaaccgctcgattcccggcctgatgaagaacgccatcgaccatgcttcgcgcccttatgggcaaagcgcctgggcgggcaagcccgcggcggtcgtgggcatttcggtgggcgccaccggcaccgcgatggcgcagcagcatctgcgcaacgtgctggcctacctcgacgttgcgacgatgggctcgcccgaaatcttcctgcaattcaaggatggctttttcgacgatcgcggccacatcggcaacgatggcacgaagaagttcctgctgggatggatggacaagtacgtcgcgtggatcaaacgccactcagcagtctgatggaacctgccatcggcaccatctaacgtgaaaaagccgccccgagggcggctttccttcgcgcgcaggccgggctcaggcggcctgggccacgttcttctggttggcggcttcggccgttgccaccaggatctcggcacgcgccccggccaccgcggcggccttgggtgcgtcacccatcgagaggccttcggcgcgcacgaagcgcacgtcggtgatgccgaagaagccgaagaccaccttcaggtagctctcctggtgttccgcggcctggccgccttcggtggtcgagtagatgccgccgcgggtggacgcgacgatcacggtcttgccgccggccaggcccacggggcccttctcggtgtacttgaaggtgcggccggcttgcgcgaggcggtcgatccaggccttgagctgggtcggaaccgaaaagttgtacagcggcgcaccaaccacgatgacgtcggaggcgaggaactggttcacgagcttttccgagagggcgttttcgcgctgttgggcttcggtgggctgggcctgcacgccggtcttgatgccgagggcgtcggggccgaagtgcgacggggcgtcagcggcaaggtcgaggtactcgaccgcggtgtcggtgtgcgcggttttccatgccgccacgatctccgccgtgagaaggcgggaggtcgaatgggcactcaggatgctggagtcgatgtggagcagcttcatggtcaatcactttcgtgtggtggtcggcgctcaagagtggccggcgttggaagaattctatttttgatgcgagtgattgataagtagtcaaaatttgacttcattgttctgctggcgggacaataaacccatgcaggacctcaacgacatggttttcttcgccgaagtggcagagcgcggcggctttgccgcggccagccgcgcgctcggcattcccaagtcgcgcttgtcgcggcgcgtagcggacctcgaggatcggctcggcgtacagctgatgcagcgcagcacgcggcggctgtcgctcacgccggcgggcgagatctatctgcgccactcggccgccatgcgcgatgcagcccaggccgcggccgaagcggtggcgcaggtgcagacggaacccagcggcacggtgcgcttgagctgtccgatctccattgcccacagtggtctggggcaattgctgccccggttcgtggcgctatacccggccgtgcgggtcgacctgcgggtgatgaacaggccggtcgacctgatcgaagagggcatcgacgtcgccttgcgtgtgcgtccggccatcgaggacagcacgacgctcgtggccaaggtgcttggaacgagccgcgcggtgctggtggccaggccggacttgctggagcgccagggcccggtgaacaagccggccgatctcgcacggctccagaccgcggccatgtcggccaacagcgaggggcgcagcgaatggcggctcgaaggccccaagggcgagattcacgtgcacgttcatacgccgcgctacgtggcggacgatcttgcaacgctgcagctggccgccctcgagggcgtgggcgcgaccctgctgcccggctacatgtgccgcgacgacgtggaggcgggccggctcgcaagggtgctgcccgactggggcccggcgccggtcgtcgcgcacatggtatttccggcgcggcgggcactggtcccggcggtccggcgattgatcgatttcctggccgagcacctgcacggaagcgaaaccggcatgtactaacctcgctaaataagccggggtgatgctccttatgcgaaaaacgccataaccaaacaagtagatattcgtttggcattgaagcagcccttcgcacaatcccaggtcccatccatccaaggagcgaccatggcgaccctgcgactcggcgatacagcccccaatttcacccaggattcgagcgaaggctcgctcgacttctaccagtggggcggcgattcgtggatcgtgttcttctcgcacccggccgatttcacgcccgtgtgcaccactgaactcggcaagaccgcggcgctgtcgggcgaattcgccaagcgcggcgtgaagcccatcgcgctgagcgtcgatccggccaccaagcacaaggagtggatcggcgacatcaacgagacgcagaacaccaccgtgaacttcccgatcattgcggaccacgaccgcaaggtggccgacctgtacgacctgatccacccgaacgcctcggccacggccacggtgcgcagcgtgttcatcatcgatccgaagaaggtgatccgcacgaccatcacctacccggcatccactggccgcaatttcgacgaaatcctgcgcgtgatcgattcgctgcagctcaccgacagccacaaggtggcgacgccggtgaactggaaggacggcgacgacgtggtcatcatcccgagcatccaggacccggccgaactcgccgagcgctttcccaagggtttcaaggccgtgaagccttatctgcgcatcacgccgcagcccaacaagtaagcgggcagggcagcgtcgccatgcagacttccgtgatcatcgtgcccggctggcgcgactccgggcccggccattggcagagcctgtgggaagagcgcattccgggcgcggcgcgggtggtgcaggacgactgggcttcgcccaagcgcgaggcctgggtgtccacgctggcccggctggtgctcgagagccccggcccggtggtgattgccgcgcacagcctgggctgcatcgccacggcacacctgccggcagaggctgccgcgcgcatccgcggggcgcttctggtggcaccggccgaccccgagcgccgcgccgtgctgtccgactttgcgcccgtgccgtatgcggccttgccctatcgcagcatcgtggtggcgagcagcaacgacccgtattgcccaatccgcctggccggcgcatattcccgcgcctggggcagtgagtttgtccgcatgcagaatgcgggccatatcaacatcgattcgggacatggagactggccgctcggcctcgccttgctccagtcgttgaccgacgagcccgccgcctggccggcgggccgtgaattttcagaaaccttggcaacctcatgacttccagactcaagaccttcgtcgccgtgctcgcgttggcatcttccgcattcgcaggcagcagcgccttcgcacagggcagcacgctgctgaacgcctcgtacgacgtggcgcgcgagttctacaaggactacaacgcggcgttcgtggcccactacaagaagaccaccggcaaggacgtgaagatcgaccagtcgcatggcggctccagcgcccaggcgcgcgccgtggccgacggcctcgatgccgacgtggtgaccatgaacacctcgaccgacatcgactttctggccaataccggcgtggtcgcgaaggactggaacaagcagttccccgagaacgcatcgccgaccacttcgaccatgctgttcctggtgcgcaacggcaatcccaagggcatcaaggactgggaagacctggtcaagcccggcgtgcaggtggtgatcgtcaaccccaagaccggcggcaacgggcgctacgcctaccttgcggcctggggctacgtgaagaagaagggcggcaccgacgcgcaagcggccgagttcgtcggcaagctgttcaagaacgtgccggtgctggcgcgcggcggccgcgacgcgaccaccgccttcctgcaacgcaacatcggcgatgcgctgatcaccttcgaatccgaagtggtgtcgatcgaccgcgagttcggctcgggcaaggtggattccgtttacccgtcgatcagcatcgtggccgagaacccggtggccgtggtcgagcgcacgaccaagaagaagggcaccggcgagctggccaaggcttatctcgactggctctactccgaagaagcccaggaaatcgcggccaagcatgcgctgcgtccgcgctcggcggccgtgctgaagaagtacgccgctacgttcaagccgctgcagctcttcacggtgcaggaactcttcggcagcctcggcgatgcacaaaaggtgcacttcaacgacggcggccagttcgacaagctctacacgcccggcggcaagtaaatgagcggcgctgtttcttcggcgctcccgtcagcgggagcgccgctttcgcgtgtgaataatcgggcggggggcgccaggcgggtgctgccgggctttcacatcacgctcggtttttcgattttctatctctgcctgatcgtgctgatcccgctgtcggcgctggttttcaagaccttcgcgctgagctgggagcagttctgggtggccgtgacctcaccgcgcgtgatggcctcgtaccggctgaccttcggcgcctcgctgatcgcggcgctggtgaatgccgtattcggcctgctcgtggcctgggtgctggtgcgctacaagtttccgggcaagcgcatcgtcgatgcgctggtcgacctgccgttcgcgctgcccacggcggtggccggcatctcgctgaccgcactgctcgcgggcaacggctggatcggacagctgctcgagccgcatggcatcaagctggcgttcacgccggccggcatcgtgattgcactgatcttcatcgggctgcccttcgtggtgcgcacggtgcagccggtgctcgaagacgccgaaaaagagcttgaagaagccgccacctcgctcggtgcaacgcgcctgcagactttcacgaaagtgatcttcccgtcgatcgcacccgcactgctcacaggctttgcgatggctttcgcgcgggccatcggcgagtacggctcggtgatcttcatcgccggcaacatgccgatgatctcggagatcacgccgctcatcatcatcggcaagctggagcaatacgactttgccggtgccacggcggtcgcgctcgtgatgctggtgatttcgttcatcctgctgctcgtcatcaacggcctgcaagcctggcagcgccgccgcgcgggagcatgacatgagtgccccttccaaaatcattcgccgcgcgcaggccggcaccaccgagtcgccctgggtgcgctggctgctgatcggccttgcgctcgcgttcatgttcctgttcctggtgctgccgctggcggccgtggcgaccgaggccttgcgcaaaggcgtcggcgcctacctcgaagcgctgaaggagcccgacgcctggagcgcgatccgcctcacgctgatcactgccgccatcgcggtgccgctgaacctggtgttcggcgttgccgcggcctgggccatcgccaagttcgagttccgcggcaaggcctttctgaccacgctggtcgacctgccgtttgcggtgtcgccggtggtggcgggcctgatctacgtgctggtgttcggtgcgcagggctggttcggcccctggcttgccgagcacgacatcaagatcatcttcgccgtgccgggcatcgtgctcgcgaccgtgttcgtcaccttcccgttcatcgcgcgcgagctcattccgctgatgcaggcgcagggcaccgacgaggagcaggccgccatcgtgctgggcgcgaccgggtggcagaccttctggcgggtgacgctgcccaacatcaagtggggtctgctgtacggcgtgattctttgcaacgcgcgtgccatgggcgagttcggcgcggtgtcggtggtgtcgggccacatccgcggccagaccaacaccatgccgctgcacgtggaagtgctctacaacgaataccagtcggtggcggcgtttgccgtggcatcgctgctggccatcctggcgctggtcacgctggtgatcaagtcggtcatcgagtggcgccacgaacgcgagatgaaggcgattgccgatctgccgcccgagcggccgacggcggcttgaacagtcccgcggtgaggggagatccctcaccccgaccctctccccaaggggagagggagtaatcagaagaaggcagaggaagagattccatgagtatcgaaatccgcaacatcagcaagcagttcggcgacttccgggcgttgaacaacgtgaacctcgacgtcgagtcgggcgagctcgtcgcgctgctcggcccctcgggctgcggcaagaccacgctgctgcgcatcatcgcggggctggaaacggccgacaccggcagcatccttttttcgggcgaagacactaccgacgtccacgtgcgcgaacgccaggtcggcttcgtgtttcagcactacgcgctgttccgccacatgacggtgttcgagaacgtggccttcggcctgcgcgtcaagccgcgcaaggagcgcccgagcgatgcgcagatcaagcagaaggtgaccgacctgctcaagctggtgcagctcgactggctggccgaccgctacccgtcgcagctctccggcggccagcggcagcgcatcgcgctggcgcgtgcgctggcggtggagcccaaggtgctgctgctcgacgagcccttcggcgcgctcgacgccaaggtgcgcaaggagttgcgccgctggctgcgtcggctgcacgacgaactgcacgtcacctccatcttcgtcacgcacgaccaggaagaggcgctcgaggtggccgaccgcgtggtggtcatcaacaagggccgcatcgaacaggtgggttccccgcaagaagtgtgggaccagcccgccagcccgttcgtctacggctttttgggtgacgtgaacctgttccatggccgggccgacaacggcgcggtgcaactggacggcatgcgcctcgactcgccggaacacagcggtgcgcgcgacgccaaggccatggcctatgtgcgtccgcacgacctcaccgtggagcgctacaccgccggcgcgaccggcatcgtcgccaccttgtcgcgggccatcgtggtcggccccatcgctcggctggaacttgagcccaccgaaacgaatccagataatccgggctccggaaccatcatcgaagcgcaactccctgcgcaacagttccgggaactgggcttgcaagagggcgacaccgtcgtcgccacgccgcgcaaggccagggtgttcgtagaagaagattgggtttccccttgatcgattggtatttcggcgcgccgcgccgcgcctatgggctgatctgccttgcctgcgtcctgatgctggccttcgggctctatctgcagcatgtagtgggcctggagccttgccccatgtgcatcgtgcagcggtatgcgctggtgctggtggcactcttcaccggcctggcgggcgtgttccgcagccgcggcctgcaggccacgggcggtgtgctggcgctgctgtcggccattggcggcgcctacacggccgcatcgcagagttggctccagtggaatccgcccgaggtcgtctcgtgcggacgcgatctgtacggaatgatcgagacctttccgctcaagcgggcgctgccgatgatcttccgcggcggtggcgattgttcgaaggtcgactggtcgctgttcgggctgacgctggcgaactggtcgtttgtcgccttcgtcgttctcgcgatcctgctgctggtgctgcttttccgcgggcgcgcggcgcgctgagcaagtgctgagtccgcgctccacccattaggaggagcgcgcgaactgcggctacagcggcagggtgtcgaaagccgcgtagccggtcgccagccaggacttcacgcgctggcgctccagcaagccgagcgcatggggcccttcgcggtcgttcacggccttccagaaactcgtgttctgcgcatcgatcttgcgcatgctggcctcgtgcagacgcggcagggtgatcacgcgggcgccgttcgccgttgccttggagagcgactgcgacgccagcagcatgccgaagtcgctgccgcggccgtagttctgcaccacgatgtagttgggccggttgccgaaggtgtcgatcagcgcgccgagcaggtcggtggagtccttgccgtcgtccagcacatgccagaaattgacggccacgcccagttcgtcgaacacgtcgaacagatcggattccttgatccagcgcgacagcggtgccagcgtctgggcggcaaggtcgacgatgacgctttgctgcggattggtttcgaagccgttcaccacggtgtcgagcccctcgaagctgtcgaccacgatgggcgacgcaaagccttcgtagaagcgcgtgaacgagctgtgcgaacggtcggtgtcgaagccgatgaaaggcttgctgtagtcgatgaagtactgcgccagcacgcgcgcggtgaccgacttgccgaccccgcctttttcgccgccgatgaaattgatggagctcatgagttgctgctgcctcgaatgggttgaggagtgaagggctgattcattctagggggcgcgttttctttctcttctatttgccgcgcctcgccaagccttgcagcaagggatgtgcctgcaagcgctgctgcagccgttttttccatgcggcgggcagcgtcgatgcctcgatcatcggcggccattggctgcgcgccagccgcgccgtgtcggcaatgacgcgccggaccagtggctcgtgcagcccggccgagaagcagaaggcgcgcacgttggcgggcgtgaacaggaccgtgcgtttggtggcggcaccggcgggcgctgcgggcagaagagggagagcgtggccgtcgacgccctggagcgcggcatacgccacgatgtcgtaggccggcgccagccgcggtgcgatgccgtccggatagagcacgccaaagttcttcaaatgcgcgtcggggttgccgagcaagtcgttcaccgcaaggcgccgcatcagttcgagcacggcttcttcgcccagcgacgggaaggcctgcatcgcaagcgccatgtccagatagctcgcgctgtacttgtgcatcgggtcgactgcgagcacctgcgcaaaatcctcgaaatgaatgcggcgcgcaccttcgcggtcgaaacgcgtgacggccagaaagtcgggctcgtcgggcaatgcgtagctgtgttcggccgcaatggccgagagcggtgccagctcggcatggcagacctcaacaccggccgcacccgccaattgaagcgacagcatttccagctgcggcatgtgggggcgtccggccacgggcagcttggcgatcacgcgcgtgctcgcgccggcccgggtgcgcgccacgtagcggccgccctggcggcgcaggccgagcttgggttgcacgcccgacaccgagatgccttgcggcatgggcagttcgaccaccgacatctcgagcgcgtcctggtcctgcgtgatgagccgctgcagcgtctggcggtccaccgcgaccggcttggcgctcactgcgccgggcaggtcgccgccgcaggccgcgaggagctcgaaatggtcgttttcgcggcagccgcgcagctgcgcgatatggctgcgcaacacgccttcgggcagaagattctggaaaaagcgcggcagctggccgccttgcgcattgaacaacgggtttttcacgtcggcccagagcgcggactgcgtggcggcatcgctggccaccatcgacagcgaaagcacctccgccggtggtgcggcgaccagctcccgctcggccacgaagcggcacaggtcggcgtactggaagagcttgccgaagcgccgcgtgccgagcgagatctcgaggatcttgacgttcatggcggtcggcgcttgttgacgtacggcggaggcggagcctgcgccacggcatggcccacgcgggtggcgacggggcggtagtcgggatcggtggccgcgctctggccgaagcccttgggcgccagctgcagttcaagtccgagcgcatcgaccagcgcgagcagcgaagacagctgcgggttgcccttcaggctcagcgcattgcgcaccgagcgctcggtcaggccggagcgctgcgcaatttcagcatgggtgatgcccgtggcatcacgccgggctgcgagggcggtgatgagttcctgcttggtcacggaaagatattaccgcaaagctcgctttcggaaatatatttccttggtactaatgcttctatcttggcaacagcgtgaagaagggcatgaccacgcccatgacccagttctgcccgaagtcgagcgcggcccgtcggtatttctcgtccgcctgcgcggccagcaggtcgagccgcgccaccaccttggacagctcgcggtcggccacgaggttgcggccgcgctcgctgatctcggtggccagcagcaggggctggccgtcggggccggtcttggacgagatcagccagagcgatatttcgaagttgcgcgccgcacggtagctgttctcggcattgacaccgtcgagcaaggtctggtcccaggtgtcgccgttggcctgcttgagcatggtggcccagccgaccaccagcgccgcgacccggtctccctggtaaccctgcggcccggtgtcgaatgcgaggcggatcgcgtcgatgccggtggcgccgcgcagttcgggcagggcggggcctgtgagcaccgcgtcccaggcgcgttgggcggccgcctcgacactggccgcggatttgcgccattcgcgcgggttgcgccggtacagcgtggtctgcacgcgccggatcgattgcaggttgtcgcgcaaggacaggttggcaatgcggttggcgctggattgcagccattcctgattggcatagggttcggcgcgctcggtggaacgcacggccgcgcagccgccaagacccagcaaggcggcagcgccagccagcaggcagccgcggcgcgcggcgaagggtgatgaaagcagggaatcgctcatgccctgacgttatcatccacggctggggcggcggcctgcctggagcggcaggcccgtgcaattttccttacaaatcaataccttggcgctacgccaaggcaggccgacaagtcgtgcgtcttaattccatcaagctttcgggcttcaagtcgttcgccgaacccaccaacttcctgctgccaggccaattggtcggcgttgtcgggcccaacggttgcggcaagtcgaacatcatggatgcggtgcgctgggtgctgggcgagtcgcgcgcgtcggaactgcgcggcgagtcgatgcaggacgtgatcttcaacggcacgaccacgcgcaagcaggccagccgttcgagcgtggaactggtgttcgacaacgccgaccatcgcgcgggcggccaatggaaccagttcggtgaaattgcggtgcggcgcgtgctcacgcgcgacggcaccagcagctactacatcaacaaccagccggtgcgccgccgcgacgtgcaggacgtgttcctgggcacgggcctcggcccgcgcgcctacgccatcatcggccagggcacgatcagccggatcatcgaatccaaacccgaggaactgcgcctgttcctcgaagaggcggcgggtgtctccaagtacaaggagcgccggcgcgaaaccgagaaccgcctgggcgacacgcgcgagaaccttacgcgcgtcgaagacattcttcgcgaactgaacgccaatctcgaaaagctcgagaagcaggccgaggtggccgcgcgctacaacatgctgcagggcgatgccacgaaaaagcagcaccagctgtggttcctgaagcgcagtgaaagcgacgccgaccaggccaagatcaaggccgattccgaaaaggcgatcaacgacctcgaatcgcgtaccgccgacctgcgccgcatcgaggccgaactcgaaaccgtgcgccaggctcactacgccgccggcgaccaggtcaaccaggcccagggcaagctctacgaggccagcgccgaagtcggccgcctcgaaggcgagatccgcttcgtggtcgaaggccgccagcgcgttgagcagcggctcgttcagttgcgcgagcagatgggccagtggggccgccgccgtgaagaggccgaggcagagatcgaaaccctggccggccagggcgtcgatgccgaagagcaggccgtgctgctagccgcacaactcgaagagcacgacgcgcgcatgcccgagctcgaggaagccgtgcagcgggcccagaacgaagccaacacgcagcgcgccgctgtcggccaggtccagcagcagatccaggtgctggccgctgaccagcgcaacatcgaagaccagagccggcagctcacgcagcgcagcgaacgcctgcgtgccgaccagaacgcgctggccgcgcccgacgaagcccgcctgcagtccatgcaggaggagcatgcggccgcacaggaagctgcgagcgaagccgacgcccgcctgcacgaactgcaggaatcggtgccgcagctcgacgacgatcgccgctcgaagcagcaggccgtcaacaccgaaggcgcgcgccatgccgaactttcggcacggctcgaggcgctgcgtgcgctgcaggaaaaggtcaagaccgacggcaagctcacgccctggctcgccaagcacgggctcgaaggcatgcagggcctgtggagccgcatccacatcgagcaaggctgggaaaacgcgctcgaagcggcgttgcgcgagcgcctgggcgcgctcgaagtcagccggctcgacatggtgcgcgccttcggcaacgacgcgccgcccgccaagctggcgttctacagccccccggccgccggcgtatcgcaggacggcggcacgctgccccgcctgtcgagcctgctgcggctgaacgacgcgggcctgcaggccctgatgaccgactggctccatggctgctacacggcgcagagcttcgaagaggcgcttgcgcagcgcgccacgctgaagccgggcgaagtcatctacgtgcagagcggccacgccgtgttctcgcacagcgtgaacttctacgcccccgattccgaacaggccggcctgctggcgcgccagcaggaaatggaaaacctcgagcgccagctgcgcgcgcagacgctcatcaacgaagaggcgcgcgcggccctggtccgtgccgaagccgcctatgccgaggccgcacagcgcctggtgacggcgcgccgtgaagcggcggaaacgcaatcccgcgcgcatgaactgcaggtggaaacgctgcgcatgacgcagctggccgaacagacgcgtgcgcgcagcgagcaactggccaccgacctggccgaagtcgacgcgcaactggaagagctgcaagaaaagcgcatggccgccgaaggccgcttcgaagagctcgacatgcagctcgccgacagccaggaacgccatgcggaactcgacgaacgcgtgatcgaagccggccgcgcattgaccgcgagccgcgagcagcaccgcagcctcgaacggcaggcgcaggaagccaccttctcgcagcgcacgctggaagcgcgccgcggcgaactgaaccgcgcaatcgaaaccgcatcgcagcaggtggtggccctcactgacgaagacgagcgcgccagggccgagttgggccgcctgtccgatgcggcggcccaggccggcctgcaggatgcgttggcgctcaagctcgagcgcgaagcagccctgggtgccgcgcgcagccagtacgacgacctcacgatgaagctgcgtgccagcgacgaacgccggctgcagctcgagcgcgaactcgatccgctgcgccagcgcatcaccgaattccagctcaaggagcaggccgcccgcctcggtgtcgagcagtaccagcagttgcttgacgatgccggcgccgacctcgaagccgttgcgctgtcgatcgaaaccgacaaggttcgcctcgcgggcctgcaaggcgagatcgaccgcctgaaccgcgaagtggtggcattgggtgcggtgaacctggcggcgctcgacgagcttgccgtggccagcgagcgcaagactttcctcgatgcgcagtccgccgacctgaacgaagccatcggcacgctcgaagacgccatccgcaagatcgatggcgaaacgcgcgagcttctcggcggcaccttcaagatcgtgaacgagcacttcagccgcatgttccccgagctgttcggcggcggcaatgcgcggttggtgatgacgggcgacgaaatcctggatgccggcgtgcaggtgctggcacagccgcccggcaagaagaaccagaccatccacctgctgtcgggcggggaaaaagcgctcacggccatcgcgctggtgttcgcgatcttccagctcaacccggcgcctttctgcctgctcgacgaagtggacgcgccgctggacgacgcgaacaccgaacgctatgccaaactcgtgaccgccatgagccgcgaaacccagttcctcttcatcagccacaacaagatcgccatggaaatggccgagcagctgatcggcgtcaccatgcaggagcagggcgtctcgcgcatcgtcgcggtcgacatggaagcggccgtcacgatggtcgaagctgcttaagccgagcagcatccatgagcaatctcactctcgccctggccatcctcggcggcctcgttctcgcggctgtcgttgccttcaacacagtcacctcgcgccgcaatgcgccgcggcagcccgacgcacgggaccttgatctgtccgacgccgagcggccctccgcatcgtccggcggcgtggagccgatgctgcacgtcgatccgcaccaggtgccgggccaggagcgccacgagcccctgttcgatcccgatctgcccgcgccgggcgccagcccggtcccgaccgccgagcggcgcggtggactcgatccgctgatcgacgtgattgcgccggtctcgctcgacgggcttgcctcgggcgacgccgcgattgcggccatgccctccacgcgccgtgcgggcagcaagcccgtggccatcgaaggcctgaacgagcacaccggccagtgggagccgcccgtgccgggccagcgctacagcgcgttccaggtaggcgtgcagctggccaatcgcaccggtgcgctcaacgagatcgaatactccgaattcgtcgtcaaggcacaggcctttgcggatgccgtgaacggcgcgctcgagtttcccgagatgctcgacgaagtggcccgcgcccgcgagctcgaccagttcgccagcgcgcacgatgcccaactgggcttcgtgctgcgcgcgctgcatgccgcctggagccccggctacgtgcagcagaacgcggcccggctggggttcgtggcgggcatcatccccggccgcatggtgctgccgaccagcgaagccgggctgccgccgatcctcgggctgtcgttcgacacccaggccgcactggccgacgatcccgcgcaatcggccatccgcgaactcagcctcagcctggacgtgccgcaggtcgatcgcgccgagcagccgttccgccgcatgcgcgaggccgccgccacgctggcgcgcgagatggacggcgtggtgaccgacagcgacgggcagctgctgcgcgacgagaccatggatgccatcggcgccgacctcgagcagctctacgacacactcgagtcgcgcgacctggccgccggctcgccactggcgcgccgcctcttcagctgatccgatcgttcgggagacacccatgacaacgcgcgacgaagcggcacgcgaagccgccgcactgagcgaacagcttcaccgccacgctcacctctattacgtgctcgacgcgcccgaactgcccgacgcggagtacgacaggctgttccagcggctgcaggccctcgaggcagaatttcccgatttgcgcacccccgattcgccgacgcagcgcgtgggcggcaaggtgctcgacggcttcaccaaggtgcgccacagggtgcccatgctgtcgattcgcaccgagaccgacatcacgcctggtggcgccagcgccttcgacgcccgcgtgcgcaaggagctcggcctggccgaagacggaccgcaggtcgagtacgtctgcgagctcaagttcgacggcctggccatgaacctgcgttacgagcacggcgtgctggtgcaggccgccacgcgcggtgacggcgaagtcggcgaagaggtcacgcagaacatccgcacggtgcgcgagattccgctgcggctcgaaggcaaggcaccgcccgtggtcgaagtacgcggcgagatctacatgaagcgcgccgacttcgaatcactcaacgagcgccagcgcgaaaagatcgcggccgggcagaagaacgagaaagtgttcgtcaacccgcgcaacgcagcggccggcgcggtgcgccagctcgatccggccattgcggcggcgcgcccgctgagcttttttgcctatggcctgggcgaagtcacgcccgccagcgaaggcgggccggaattctcgacccagttcgattggctgcagcagttcgacgcgtggggattcccggtggcgaagcagactgcgcgggcaagaggtgctattgagttgatagcgttccacgagaacatcgggcgccagcgcgacgccttgccctacgacatcgacggcgtggtctacaaggtcgacagcctcgagttgcagcgtcggctgggcttcgtctcgcgcgagccgcgctgggccgtggcgcacaagtacccggcgcaggagcagatcaccgacgtgctcggcatcgaggtgcaggttggccgcaccggcaagctcacaccggtggccaagctcgcgccggtcttcgtcggtggcgtgaccgtgaccaacgccacgctgcacaacgaagacgaagcgcgccgcaaggatgtgcgcgtgggcgacaaggtcatcgtgcgccgcgccggcgacgtgattcccgaagtggtcggcgtggtgccggagagcctggccaggcccgacaccgagcgcggtccgctgttcaccatgccgcaccagtgcccggtgtgcggctcggaggcgctgcgcgaagaaggggaggtcgactaccgctgcaccggtggcctgttctgcggggcccagcgcaaggaagccatcctgcactttgcggcccgccgcgcggtcgacatcgacgggctcggcgacaagctggtcgagcaactggtcgatgccaacctgatccgcaccttgcccgacctctacaggctcggcttcacgacgctggcgggcctggaccgcatggccgaaaagtcggccaggaacatcgtcgatgcgctcgaggcctccaagaagaccaccctgccgcgcttcctgttcggccttggcatccggcatgtgggcgagagcaccgcaaaagacctggccaagcatttcggcaagctcgacgcgatcatggacgcgaccgaggagcagttgctcgaggtcaacgacgtcggcccggtggtcgcgcagagcctgcgaaccttcttcgaccagccgcacaaccgcgaagtggtcgagcagctgcgggcctgcgggctgacgtgggaagagggcgaacccgctgcgcgcgctcccaagccgctggcgggcttgaccttcgtgatcaccggcacccttcctacgctcagcagggacgaggcgaaggataaattggaagccgccggtgccaaggtggcaggctcggtcagcaagaagacaagctacctggtggccggggaggaggcaggcagcaagctcgacaaggctcgtgagattggcgtcaatgtgatcgacgaggcggggatgctggacatactcgccaatggcgtcccgggttgaaaagagggcgccggcgcggtgttcttaccgctcgttacgtgacttcacaccggcgcagtcaacagggtctacaagctggcgttgataaaacagaaggctgacaaggagtcccttatgcaaaagattcgtgttctcggtacttgcgtcgccatcggcggctttgcgctgctcggcggctgcgtgggcgttcctgccgaaccctattacagcgggggctactcgcagccgtattacgacaatccggtggtcgttcagccggcgcccgtctacatcgaaggcggcggctactacgaaggccgccgtccttactacggcgggcggccatactacgacggcgggcggccttactacggcaggccgggctatcctgtcgcgcggccagtgcctgtgccggtgcccgtgccgtcgcgtccgggttggggcggcggtggccgccattccggtggtgcggccgtggcgccgtcgggcggttcgccgttgccgcagtaccggtcgcagccgccgcgcggcgatcagaagctgtatacgtcgcccgactccaagggtcaaaccccaccctgattctcgaaaggtgggccggtgagcggccctggcggtcgcgataatcccgccatggccatccgcgaaatcctgaaaatgggcgatccccggctgctgcgcattgcgcagccggtggccgccttcgataccgacgaactgcacctgctggtgcgcgacatgttcgagacgatgcttgcggtcaacggcgctgggttggccgcgccgcagatcggcgtcgaccagcagctcgtgatcttcggcaccgatgtcgtcaatccccgctaccccgacgcccccccggtgcctcgcaccgtgcttctgaacccggtcatcaccccgatcggcgaagaggaagaagagggctgggaagggtgcctgtcggtgccgggccttcgcggcgtggtgccgcgctttgcgaacatccgctacaccggcttcgacccctatggcgatcccatcgaccgcgtcgccagcggttttcatgcgcgcgtggttcagcacgaggtcgatcacctgctgggcaagctctacccgatgagggtgcgcgatttctcacgcttcggctacaccgacgtcctgtttccaggactcgacgccaacgacgacgactgaaaagaaaaagccggcgcgcgggccggctcatgagcttagttgtacctgccgcccaggccgaagcggccgccgccgaacaggctgatggcaatagcggagaacaggtacatgccctgcagctccagcgcccagccgccctggccgttcagcgcgcccaggtccttctggtgcaccagccagatcgccaccaccatgttgatcgcgacgatcaacgccgccggccgcgtgaacagccccacgatgagcaacaccggcgcgacgatttctccgacataggtgaggtatgccaaggccgccggcagcccatgggacgccagcatgccgccaatgccgtcgacgcccttgccgccgaccttcgcaatgccatgcaacaggatgaggatgccgagtgcaacgcgcagaacgagcttgccggtgtcgtcggatttggtcatgaacagtttcctggtgagagagtgattgaagggccatatgttagtgaatgcagcgaccgagaaaagcctgccgcgagcgacgtggggcatatgcatccaaccgtccgttctttggcagagtggcgcgcagccccgtacactgccttttgcctactgttgaggagaacacaccaatgaaaagccgattccgtcccgcgctggccgcggccgcatccgtcgtggcgcttgccgcggccgctcccgcctttgccggcaagaccctcgatgccgtcaagcagcgcggtaccgtcaagtgcggcgtgaccaatggcgtggccggtttttccgcgcccgacacacagggcaactggtccggcctggacgtcgatacctgccgtgcgattgcggcggccgtgctgggcgacccgaagaaggtcgacttcgtgccgctcaattcgcagcagcgcttctcggccctgcaggccggcgagatcgacatcctcgcgcgcaacaccacctggacgctcacgcgcgacgcgtcgctgggcttcaacttcaccaccatcacctactacgacggccagggcttcctggtgccgaagaagctcaaggtgacgagcgccaagcagctcaagaatgccaccatctgcacgcagtcgggcaccaccaacgagaagaacgtgtccgactactttcgtgcacagaacatcccggtcaagaccgtcgtcttcgaaagcttcgaggcttcgttcaaggccttcttctccggccgctgccaggctttcaccaccgacgcctcggcgctggcgggcctgcgcaacaaggaagcgccgaaccccgacgactacgtcatcctgcccgagctgatttcgaaggagccgctcgcgccgctggtgcgccgcggcgacgacgaatggtttgccattgccaagtgggtgcccaatgcgctcatcgaggccgaagagttcggcgtcacgcaggccaatgccgacgagctcaaggccaacagcaaggacccggggcagcagcgcctggtcggctccggtgaagacctgggcaagctgctgggcctcgacaaggactggtcgttccgcgccatcaaggccgtgggcaactacggcgaaatgttcgaacgcaacgtcgggccgaagtcggtgctcaagctgccgcgcggctccaacaacctctggaacaagggcggcctgatctacgcacccccggttcgatgagcggcggggcctcgcgccgcggcgcctggctggcctggatcgtccaggcgctgctggtgctggccgtcgtggccggcgccttctgggtggtgcaccatgcgctcgaagtgctgcgctcgcgcggcgttcgttccggattcgacttcttgacggagcccgcgggcttctcgatcagcgaaggctggctcgatttcgacgccagccagccgttctggcgcgcctttgtcgcgggcctgatcaacacggtgcgcgcctcggtgcccgccgccattttttcggttgtgctcggcaccttgatcggcatcggccggctggcgccgcacgtgctgttgcgcggcatctgcaccgcgtacgtcgaactgctgcgcaacgtgccgctgctggtgcagttgctgatgctggcttttgccatggccaacctgctgcccgacccgaccgagcccgtgcgcctgctccccggcgtgtggctcagcaagggcgggctcagcgtgccttggcccgcgtcgggcgaaggcggctggtggcccacgcacttcgaatggcccgagaagggcgacttcggcgtgagcggcggcgcggcactgagcccggaatacgtgaccatcgttgcggggctttccttctactccgcggctttcgtggccgagatcgtgcgcgccggcatcctctccgtatcgcaagggcaggtgctggccgggcaggcgttgggcctgacgtcggtgcagcagcttcgcatcgtgatcctgccgcaggcgctgcgggtgatcgtgccttcgctcaccaaccagctgctgagcctcaccaagaattcgtcgcttgcggtggccgtgggctacccggaactggtgtcggtagccaacaccaccatcggctcgaacggccgtgccttcgagtgcatcgcgatcatcatggcggtctacctgctgctgtcgctcgtcatctccttcggcatgaaccgctacaacgcgcgcgttgcgctgcgaggctggcgatgagaaacgtcgcgcaagggcccatcgcctggcgcagtgaactctggggttcgccgctgcgcgcactggccaccgtggtgctgctcgcgctgctcgcatggggcggcttccatgccgtcgaatggggcgtggtgcacgcggtgttccggcccgatgccgaagcctgccgcgcgctgcagcacggcgcttgctggggcgtcgtggctgagaaatggcggccgatgctgttcggccgcttcccctatgaagagcaatggcgcccggccgtcgcagtggtcgtgctgtcggccgtcacggtgctgagcgcctggccgcgcagctggcgctggtggctgctgccgctctgggcggtggcgctgctgctcttcgtgctgctgatgcgcggcggcgcgctcggcctccacgccgtgccgacgagccgctggggcggactgccgctcaccatcggcctcgcggtggtgggcctggcgctggcctttccgctggcactgctgctggcgctcgggcgccgctcgggctggccggtggtccgcacgctgagcgcgagctacatcgagctggtgcgcggcgtgccgttgatctcggtgctgttcatggcctcgttcctgctgccgctgctgtggcccgccggctggcaacccgacgtgctggtgcgcgtgctcgcgggcttggcgctgttcgtggcggcctacctggccgagatcatccgcggcggcctgcaggccgtgccgcgcgggcagaccgaggtggcgatggcgctgggcttcggacgctggcccgtgcagcgggacatcgtgctgccgcaggcgttgcggctcgtggtgcctgcgctgaccaacaacgtggtcggcacgctgaaagacacttcgctggtcacggtggtcggcctgttcgaactcaccggcgcgctgggcctggcgctcggcggcgacccgacctggcggccgttctacctcgagggctacctcttcattgcggcggtgtactgggtgctgtgcttcgggctctcgcgctacagcgtgtggctggagcggcggctgggagagggcacccgctgaccggttgcccttcttcgggttgtcagcccgccgacagcgccttgtccaccagttgctgcgcttcctcgaggatgcggcccaggtgctccgcacccttgaagctttcgccgtagatcttgtagatgttctcggtgccggagggccgcgcggcgaaccagccgttgccggtgacgaccttcacgccgccgatggccgcgccgttgcccggcgcatggctcagcacggcctcgatcttgtcgcccgcgagttcagtcgagctgacctgctgcggcgacagattcgacagcttctttttctgttcgacggtggccgccgcatcgacgcggtcggacaccggctggcccagcgcctgcgtcaactcggcgtagcgttcgcccgggtcgcgcccggtgcgtgcggcaatctcggccgagagcaacgcgggcacgatgccgtccttgtcggtggtccatgccgagccgtcgaaacgcaggaaggttgcccccgcgctttcctcgccgccgaagcccagcgagccgtccaccagcccgtcgacgaaccacttgaagcccaccggcacctcgtggagcttgcggccgagccgggccgtgacgcggtcgatcatctggctgctcaccaccgtcttgccgacggccgcttgcgccggccactgcggacggtgcgtgaagaggtagtcgatcatcaccgcgagatagctgttcggctgcatcaggcccgcgctgcgcgcgaccacgccgtggcggtcgtggtcggtgtcgcaggcaaaggcgatgccgaagcggtctttcagcgcgatcagcttgtgcatcgcgtcgggcgaggacgggtccatgcggatgcggccgtcccagtcgagcgacatgaagcggaaggtggggtcgacctcctggctgagaacttcaagacgctcgagcttgtagcgctcggcgatggcgggccagtagtgcacgccggcgccgcccaggggatccacgcccaggtcgatctccacgccacggatggcgtccatgtcgagcacctgcgccaggtcttcgacataggtgttgacgtagtcgtgccggtgcgtggtcgaagcgcgcagcgcctgcgcgagcggcatgcgcttcacaccctgcagcccgcctgcaagaaagccattggccgcggcctcgaccgcggaggtaatgtcggtgcccgccggtccgccgttgggcgggttgtacttgaagccgccgctttcgggtggattgtgcgaaggcgtgatcacgatgccgtctgccagcccggtcgtgcgcccgcggttgtagaccaggatggcatgcgagatggccggcgtgggcgtgtactcgtcgtccttcgacagcatcagctcgacgccgttggccgcgagcacttccaccgcgctgttgaatgccggcgtggagagcgcatgcgtgtcgatgccgaggaacaacgggccgtcgattcctttctggcgccgatggtcggcaatggcctggctcatcgccagcacatgccattcgttgaatgcgttgtcgaaggaggagccgcgatgccccgaggttccgaaggccacgcgctgcgcggcgaccgagggatcgggccggcccgtgtaataggcggagataaggcgcggaacattgaccagcaggtccagcggtgcgggctggcctgcgaggggattggttttctggctcatgtcgggtgttgccgttcgagttgaatcaagtcgacaacatcatgccgcaggatgcgcctgcgaatgaaacaagcggaaagcggcctggcgctaacagccctaagacgccagcgcttccatcagctcggtctcgatcgccagctgcgtcttctggccctgcagttcgggcccgctgatcaggaaggtgtcttccacgcgctcgcccagggtcgtgatcttggcgagctgcaggttcaggtggtgccgtgcgagcacgcgcgccaccgaatacaaaagccccgcgcggtcgctggccgagatgttgagcagccagcgctgcgccttgtcgtcgggcagcaggctgatgcgcggcttgatcgggaaactgcgcacgcggcgcgacacgcgtcccacgctcggcgagggcagggggccggcttcggtcagcgtgtgcgcaaggcccgactcgaccatgctgatgaggtcgcggtaatggtcgggctggaaagtggtcaccacctggaaggtgtcgagcgcgtagccgttgctcgtggtgtgtactttcgcgtcaagaatgttgaacgacgactggtcgaaataaccgcagatgcgcgcgaacaggtcgggctggtcgggcgtgtagaccaccacttgcaggccttcgcccaccggtgaaagatgagcccgcactactggcgccgccttgggatcgacgggcacgttgggcggcggcacgaagcgcgagagctgcttggcgtgccaggcgatctcggtggcgtcgtggcgcatgaagtagcccacgtcgagcgtgtcccacagcgccttgtgggcctcgaagcgctgggcatgcagcgccagctgcaccagtgcttcgcgcttgcgcaattccacctcggcgtcggggtcgggcatgcgcccgcccagtgcgcgcagggtgtagcggtacaggtcttcgagcagcttgcccttccaggcattccacacgcgcggcgatgtgccccggatgtcggccaccgtcagcaggtagagcgctgtgaggtaacgctcgttgcccacgcgcttggcgaaggcaccgatcacctcggggtcgctcaggtcctgcttctgcgccacctggctcatcaccaggtgttcggcgacgaggaattcgatcagcttcgcgtcttcgcgcgcaatgccgtgctgcttgcagaagcgctgcacgtcgcgcgcgccgagcgtggaatggtcgccgccgcggcccttggcaatgtcgtggaagagcgcggccacgtagaggatccacggcttgtcccagccggccgcgagctgcgagcagaacgggtattcgtgcgcgtgctcggcaatgaagaagcgccgtacgttgcgcagcaccatcaggatgtgctggtccaccgtgtagacgtggaacaggtcgtgctgcatctgtcccacgatgctgcggaacactcgcaggtagcgccccagcaccgaggtctgattcatgagcctgaacgcatgcgtgatgccgtagggctgcagcaggatgcgcatgaaggtctgatggttgaccggatcgttgcggaacttgctgtccatcacgtggcgcgcgttgtagagcgcgcgcagcgtgcgggccgacaggccctgcacgccgatggtcttctggtagagaagaaaggtctcgagaatggcgtgcggctcgcgctcgtagagatcgtcgctcgcaatctcgatcaggccggcgcgctcgaagaagcgctcgttgatgggcgtgtgctgctcgtccaccggctgcagccgctccgcgatgttgagcagcaggatctggttgagctgcgacaccgccttggccgcccagtagtagcgccgcatcagcgcctcgctcgacttgcgctgcgattcgccttcatagccgaagctcgcggccacggccgtctgcaggtcgaacaccaggcggtcttcgcgccgcttggcaatcacgtgcaggcgcgcgcggatcagcgagagcagggcttcgttgcgcttgatctgctgcgcctcgaaggaggttgccaggccgttcttggccaagtcgtcccagcggttgccgaagcccgcggccttggtcatccagagaatggtctgcaggtcgcgcaggccgcccggcgattccttgcagttgggctccagcgcgtaaggtgtgctgtcgtacttctggtggcgatgccgcatttcctgcgacttggcgacaaagaaagcctgaggatcgatggcccgcgcaaagcgcctgcggaacgccacgaacagcttcttgttgcccgcgacgaagcgcgattcgagcagcgaggtctggaccgtgacgtccttctcggcttcagccaggcactcttcgaccgtgcgcacgctggagccgatttcaagcccggcgtcccagcattggccgatgaaggcctcgatgcgcgctggatcgatttcgctggcgtggccctcgggcggcagcagcagcagcacgtcgacgtcggaatacggaaacagctcgccgcggccgaagccgcccacggccgccagcgtgagcgagtcgccgaagtcggcgtcccgccagagcgcgcacagtgtctggtcggccagcgccgacagctggcgcagcacggtgtgcacgctgcgcgtgggcgcgcgcgcaaagcgcagggtatcgaacagcgccagcttcttcgcgcgataggcttcgcgaagcgcggcgacgtcgatcttggctggttcgatcacgacggctttgtccggggccgtgcgccgctcgcgcggctcacgttttcgtggaagtgacgaacgagggcaggggtgggctgccttcggacagcgtgagcacctcgtagcccgtttcggtgaccagcaccgtgtgttcccattgcgccgacagcgaatggtcgcgtgtgacgatggtccagccgtcgtactggccgcccctgaagtcttccttcacctcgcgcttgccggcattgatcatcggctcgatggtgaagatcatgccgggcttgagttcttcgagcgtgcccgggcggccgtagtgcagcacctgcggctcttcatggaagcgctggcccacgccgtggccgcaaaactcgcgcaccaccgaatagccctggccttcggcgaacttctggatggcgtagcccacgtcgcccaaatgcgcgcccgggcgcacctgcatgatgccgtgccacatggcttcgaaagtgatgtggcacaggcgcttggcggcaatggaagcgtcgccgatgatgtacatgcggctgttgtcgccgaaccagccgtccttgatgacggtcacgtcgacgttcatgatgtcgcccttcttcaagggcttgtcattcggaatgccgtggcacaccacgtggttgaccgaggtgcagagcgacttcgggaacgggacgctgctggcgcccatgtagcccacggtggccgaggtggtgccctgcttgaccatgtattcggccgccagccggtcgacgtcgttcgtggtgatgccgggcttgatgaggggcgtgaggtagtccagcacctcggaagccaggcggcaggcgacgcgcatggcttcgatgcccgcagcgtctttgtaggtaatgctcatcccggaattatcccattggaagaatgagcctgcccccaacgcggggcacttcgtgtccccgctgcccccaagggggcggccgactcgggacggcccggcgttggcctaaaatcccgggttaacgcggatggccccagtcagcggccgtccgcctcgattttcttgattcccaacgcggcccccgaggccccatcgaccgtgacgcagcccgcacctcaagcccttcctgtcgtaaccatgttcgagggcggcagcgcactcagcgatttccgcgcacggcagctgctgcccaagctgcaggccatcgagccccgcatcgaaggcattgccgcccgcttcgtgcacctggtggtcaccgatgccgccctggacgcagccgaccgcgaccgcttcgctgcgctcctgacctatggcgagcccttcgaggcactggccaaggccggtacctccgtggtcgtcaccccccgcctgggcaccgtgtcgccctgggcttccaaggccaccgacattgcccacaactgcgggcttgcgctgcgccgcgtcgagcgggtcacgcaataccacctgaggctcaaggcgccgctgatcggcaaggcgcccgtgctcgaaggcgacctgctcgccgccgtggccgggccgctgcacgaccgcatgaccgaatcggtgctggccacggcggagcaggccgcgagcctcttcagcgagttgccggcccagccgatggcgctggtcgacgtgcagggcggcggccgcgccgcgctggtggcggccaacacgggtttcggcctggcactggccgaggacgagatcgactacttggtcgaggcctttacccggctcgggcgcaacccgagcgacgtcgaactgatgatgttcgcgcaggccaacagcgagcactgccgccacaagatcttcaatgccgccttcaccatcgacggcgtggcccagccgcagagcctgttctcgatgatccgccacaccgagaaacagaacccgcagcacacggtcattgcctatgcggacaacgcctcggtgatggagggctcgacgatcgagcgctttgtcgcccgctcggattcgcagggctatcaaaaagatagcgccctgagccatgtgctcatgaaggtggagacgcacaaccacccgaccgccatctctccgtttccgggcgcctcgaccggtgcgggcggcgagatccgcgacgaaggcgccaccggccgcggctccaagcccaaggccggcctgaccggcttcaccgtgtccaggctctggccggaagagggccactacggcaagcccgaacacattgcgagcccgctgcagatcatgaccgagggcccgctgggcggcgccgcgttcaacaacgaattcggccggcccaacctgctgggctacttccgcgaatacgagcagacggtggccagcgacctcgacaccgtgcagcgcggctatcacaagcccatcatgatcgcgggcggcctcggcagcatcgacgccacccagacgaagaagatccagttcccggccggctcgctgctgatccagctcggcggccccggcatgcgcatcggcatgggcggcagcgccgccagctcgatggcgaccggcgccaacgcggccgagctcgacttcgactcggtgcagcgcggcaaccccgaaatcgagcgccgcgcgcaagaggtcatcaaccattgctggcagcagggcgcgaccaacccgatcctggcgatccacgacgtgggcgcgggcggcctgagcaatgctttccccgagctgaccaacgacgccggccgcggcgcgcgcttcgacctgcgcgccgtgcccctcgaagaatcgggcatggcacccaaggaaatctggtgcaacgagagccaggagcgctacgtgctggccattgcgccggaatcgctcgaacagttcaaggccttctgcgagcgcgagcgctgcccgttctcggtggtgggcgtggcgaccgaggagcgccagctgctggtggctgatgaaggggccgccgtgcagcctgttgacatgcccatggacgtgcttctgggcaagccgcccaagatgcaccgcgacgtgaagaccgtcgcccgcagtttcaagccgctcgacctcaccggcgtcgatctgcaaaaggccgccatcgacgtgctctcgcacccgaccgtggcctccaagcgcttcctgatcaccatcggcgaccgcaccgtgggcggcctgagccaccgggaccagatggtcggcccgtggcaggtgcccgtggccgattgcgccgtgacgatggccgactacaagggctttgcgggcgaggcgatgagcatgggcgaacgcacgccgctggccgcgctcgacgcgccggcttcgggccgtatggccgtggccgaggccatcaccaacctgctggccgcgccgatcgagctttcgcgcgtgaagctctcggccaactggatggccgcctgcggcgagcccggcgaagacgccgcgctgtacgaaaccgtcaaggccgtgggcctggagctgtgcccggcgctgggggtgtcgatcccggtcggcaaggattcgctgtcgatgcgcacgcagtggaaggacggcggcgaggcgaagaaggtcacctcgcccgtcagcctgatcgtcaccgcattcgcgacgctcgccgacgtgcgcggcacgctcaccccgcagctcgacgccgaagaggccgacaccaccctcgtgctcatcgacctgggccggggccagcaccgcatggccggcagcatcctggcgcagacgctcggccagagcggcgatgtggtgcccgacctcgacgaccccgcgcagctcgtggcgctggtcgatgccgtgaacgcgctgcgcgccgacggcaagatcctggccatgcacgaccgcagcgacggcggcctgttcgccaccgcctgcgaaatggcctttgcgggccatgtgggcgtggccctcaacgtcgacatgctggtcaccgaaggcgacggcatctccgacagccgcatggaaaccggcgacgccaagaactgggcgcagcaggtcagcgcgcggcgcgaagagctcacgctcaaggcgctgttcaacgaagaactcggcatggtgttgcaggtgcgcacggcagagcgcaacgacgtgatgcaggtgctgcgcgcccacggcctcagcgcccacagccatttcgtcggcaagacccggccggccagctcgacgatggacgcgggcaagggcaagctcgaagtctggcgcgatgccaagtcggtgttcagcgccacgctgcacgacctgcaccaggtgtgggattcggtcagctggaagatcgcccgcgagcgcgacaacccggcctgcgccgacgccgagcacgccgccgccggcgagccttcggaccccggcatgcatgtatttctccctctccctcagggagagggcaggggtgagggcaacggcctcaacgctcccgccatcctccaatcccgccccaaggtcgcgatcctgcgcgagcagggcgtcaactcgcacgtcgagatggcctacgccttcaccgaagccggcttcgaggcctacgacgtgcacatgaccgacctgcagacgggcagggcggacctcgccaacttcaagggcgtggtcgcctgcggcggcttcagctatggcgacacgctgggcgccggcatcggctgggcgcgcagcatcaccttcaacccgaagctcgccgaacagttcaaggccttcttcggccgcgaagacaccttcggcctgggcgtgtgcaacggctgccagatgttcgccgaactggccgacatcatcccgggcgccgaagcctggccgcgcttcaccaccaaccagagcgaacgcttcgaggcgcgcctgtcgatggtcgaagtgctcgaatcgccgagcctcttctttgcaggcatggccggcagccggctgccgatcgcggtggcgcacggcgagggctatgccaacttcaagcaccgcggcgaccaagccaaggccatcgcggccatgcgcttcgtggacaaccacggcaaggccaccgagcagtacccgttcaacccgaacggcagtgcaggcggcctgacttcggtgaccacgccggacggtcgtttcaccgccgtgatgccgcacccggagcgtgtgttccgcaacatccagatgagctggacgccgggtgaccgcagcgaactgagcccgtggatgcagatctggcgcaacgcgcgccgctgggtgggctgaccggcgcatgctcgacctcgatcacccgcgaagccggcatgtgctggaagccgcgcggatcgaggacgcgatccgccgacagttgctcgcatggcgcgaggatgcggccgccgcttcgcttcggcacctgggcggcctgaaaccgaggcgcgtggcaatcaacgcgtcagcattgcccgcatcagatagcccgcgatttgcgggttctccttgatgcgccttgtgctgtagccgtaccagtccttgccatagggcacgtagatacgtaccccgtagccagccagcagcagctggtcccgcaacggctcgcaaacgccgagcagcatctggaattcaaagcgcgagcgatcgatatctcggctgcgtgccagcctcgtcacgccatcgatcaactccgcgtcgtgcgtggcgacaccgacgaaggtgccggtatcgaagcaacggcccacgtggtgcaggaagtgtgcgttgatggcgcttctgtctcgccatgcgtcgtccaccagatgctgccggtcttcgacatagatgcctttgcacagccgcagatttcggccctggccgagcagcggctcgatatcgcgataggtgcgcttgaggtacgcttgaagcacaagaccgacgttcgtatgtcgtggcctcaggcggccgagcagatcgatctctttttgcgtgcagcttgcgtcttccatgtcgatgcgaacgaagttgccgtggcgcgccgccgcatcgacgatgcgcaggaggtagtgttcgcaatgcgcttcgtcgagcaaaagccccagtgcggagggtttgaccgacacgttggcgtcgagtccatgggcatgaacagcgtcgagcacctcgatgtattcatcggcagtgcgctcggcctcgcgcatgtctgccacgacttcgccgagtacgtcgacggtcgcggcgcatcccagtgcattgagtttgcgaatgcgtgcgacggcctcgccgacagtgctgccggcgatgtagcgacgggatgccttttgaacgaggacgcgcggaaccagggggatggcgtgcgccatcagtgcattgaatgtgagcacaggaatttcccaaaacgaaagaacgacgacggccccgccggttgcggcggggcagggcgacgcccgagggccgtgcatcccatgagggagcgcggcgccggaggggcgttcagttctttgcggagggaggccaggctgcggcttgcattcgtgtgggcttggagctggatgtgcgtggaggtcgcgagtgtcgcagatggcgcggtcgccattgcccaaaagaaaagcgacccgaaggtcgctattctttttgccgtgtcgacttactcgaccttggccttggcgcgcagttcctcttggtacttctgcaggcgctgctgctgcagctgctgcgtgatctgcggcttcacttcttccagcttcggaagctgggcctggcggatgtcgtcgacgcggatgatgtgaaagccgaactgcgtcttgatcggggcaggggtggtttcacccttcttgagcttgatcatcgcttccgagaattcgggcacgaagctcgccgggttggcccagtcgaggtcgccgccgttggcgcccgatcccgggtccttgctctgcttcttggcgatgtcctcgaacttggcgcccttcttcaggtcggccatgatcttcttggcctggtcttcggtttcgaccaggatgtggcgggccttgtattccttgccgccgttggctgccacgaacttgtcgtactcggccttcacgtcggcgtccgagaccgggctggtcttgcggtagttctcgaacagcgcgcggatcaggatcgcctggcgggcaagttcgagctggttcttgtagtcgtcggtggcgtcgaggccctgtttctgcgcttcctgcatgaacacttcgcgcgcaacgacttcctcgcgcagctggccctgcatttccggcgtaaccggccggccggctgccgccagctgctgggccagcacgtccatgcgcgccttgggcacgggcttgccgttgacgatggctgcgttctgcgccatggccgccataggaatcgcaccgagcagcgctgcggccgcaacggcctgcaagatttgttttttcatggaatgaatatcaggctgggggaaatgcgcgtatgggaaaaagcgcgtggaagaaagcggatgagacgacggatcgaagaagaagggagggcgggccgccgcggccatgtggacggatggcggcatgcaactgatcgaacgactcagagcacctcgatggcgatggcgtgcagaccctgcgcgataaaaacttggagggcatcatacacaaggcgatggcgcgccacgcggggcttcccttcgaacagtggggaagcaacgcgaacccggaaatgcgtgccgcgcccctccgcgttggcgccggcatggcccgcatgggcgctgctctcgtcgatcacttccagcacggtgggctggagcgcctgacgcagcgccgcttcgaggtcgcgcgccgtcggcaaggggtggttcacgttcatgcggcaggcttgtcgtcgcccttgaggtgcggcgaaatgtaaagcccctgtgccaccaggaagacgaccggaaacacatagccccagagcttgaagttgacccaggcctcggtggtgaagtacgccgccacgtagccgttgatgatcgccatgaagaggcagtagccgatccaggccacgttgaggcggccccacacgcggtcgggcagctgcagttgcgaacccagcagcatcttgaggaagttctttttcagcgcccagagcgcaaccgccagggcgatggccatggcgccatagagcaccgtgggcttccacttgatgaagcggtcgtcgtgcagcaccagcgtgagcgtgccgaacaagaggatcagcaccagcgtggccttctgcatggcctgcagcttgcgctccatggcgtagatgatgcccatctgcaccacggtggcggccatgagcacgccggtggcggtgtagatgtcggccagcttgtaggcgccgaagaacagcaggatcggaaagaagtcgaggatcagtttcatgcgctggggagggctggttggttatttcttctggaagtccagcgaggcggaattcatgcaatagcgaaggccggtttcggtggggccgtcggggaacacgtggcccaagtgggcgccgcagttcgcgcagacgttttcggtgcgcaccatgccgtgcgagcggtcgacgatgttcttgatggcacccggcacggcttcttccgagaagctgggccagccgcaacccgcgtcgaacttggccgaggcctcgaacagcttggcgccgcagcagatgcaatggtaggtgccgtcttcccagtgggcctcgtacttgccggtgaaggggcgctcggtggcggcatggcgcgtgacctcgaaggccgcgggctcggcgcctttttcagcgagcagggctttccattcggcgtcggttttctgtgcgggagtggtcatgatgagcagctgattgcgatcgtggaggcccagtcgggcgggaacccggcataggcatcggcaccgggatgttcttcagatggggtttggagcagtgtcagcaaggttgccacacccgagaagtccttttggcctgccgcttcgatggcttgctgccccaggtggttcctcaacacgtacttcggattggatttgagcatcaaatccgcggcttccgggtgcgacgactgcgcgtggcgctccgaaaataatagcagccaggcgtcgaaaccggcacgatccaggaacaggtcgcgcaccggctcggcgttgccgccggccatgtgctgcgagaggcggcgccagaagatcgtgtagtcgaccttttccgcggccaggagcttcagcacgccctcgatgagcgtgcggtcgccctcggccgaatcggtgagtccgagcttggcccgcatgcgcccctcgaactcgcgcggaaacaccgtcttgtaggactccagcgccgccaccgcgatttcctggtcgccgatcagcggcagcagtgcctgcgccaggcagaacaggttccagtaggccacgttgggctgctggttgaaggcgtagcggccgctggtgtcgctgtgattgcagatgtggcgcggatcgaaaccgtccaggaactggaacggcccgtagtcgatggtgagcccgaggatgctcatgttgtcggtgttcatcacgccgtggcaaaagcccacggcctgccattgggcgagcagggcggcggtgcgctcgctcacggtttccaggaaggccgcataggcgttgccgttgaagcgctccgtggtgcggcaggtcgggtaatggcggtcgatcacgtagtcggccaatgcacgcagttcggcgtcgcgctggttcgccgcaaagtgctcgaagtggccgaagcgaatgaagctgggcgccacgcgggtcaccacggccgcgctttccggttcttcgcggtacacgggggcgtccgagccggtgacgcagagcgcgcgggtggtgggtatgccaaggccgtgcatggcctcgctgcagaggaattcgcgaatgctggaacgcagcacggcgcggccgtcgccgccgcgcgaatagggcgtgcggcccgcgcccttgagctgcacttcgaggccgcccgccgtttcgcccagcatgatcgcgcggccgtcgccgagctggccggcccagacgccgaactggtggccgctgtagaccgtggcaaagggccgggttcccgccaccaacaggttgccggtcagggctgccagcgtgctgtccgattgccgccagccggccggcaagccaagctcgcgcgccatcgcttcgctatggcccacccagtagggatcgggtagcggcgtcggccgcaattcggtgagaaacgcgggccccaacgccaggaatccgggtttccattgcagtcccaggtcggcggcgaccgtgtcttcggcaagcaagctcatgcccggattgtccggcagagcgcgtaaccccttgctgcgcgggccatcgagggcccggcgcggtcagtgggcgagtgccggggccgcccagatccgcgcccggtattgcgcgggcggcaggccgaaccaccgcttgcaggcccggaagaaattgctgctgtcgacgaagccgagcatgtccgccacgtcggtgagcgtgtggcggtcttcggccaggtactgctgcgcgagttcgcggcgggtgcggtcgagcagcgactggaacgacaccgactcttcctgcagccgccgctgcagcgtgcgctccgccagcccgaggccggcggccacgtcctgccggcgcggctcgccccgcggcagccggcgcgcgatctcggcgcacaccaggctgctggtcgtggtctggcccaggaggcccagttggtcgtccagcaggtgctcctgcatttcgccgagggcggggtgatgcgtgggcagcggcatggccaggtcggtgttcgacagcagcatgcggttcgcggcggcgttgaagcgcacgtcgcagccgaaggcctcgcggtgcagccggtcgctggccggcgcggggtagacgaactccatggccagcggctgcagttcgcgccgcgtgagccattggcattgcatgagcgtggtcaggagggcgtattcgacgcgctggcggggtatcggcaagctgccgccgttgtgctccatcaccatccagcaaccgcgtgggtcgggttgcagcgagaaagccgtcgcgtccgagatcacggccatgtagcgcgccagccgcgcgagggccgagccgagatcggggctgcaggccatggcgtggccgaccgtgcccagcttgctgtgcgtggcggccaggtcgcgatgcaggcccagcgaaggcttgccggcgcgcgccacggccagttgccagagcatggtgatttcgtcgaccggaatgcgcgcgttctggcggcgcagcgaatcgggatcgaacccagcgtcccgcagcagcgaaggcacgtcgagcccttcggcctcgaacatcgagagcacgccttcgagccacgcggccgagctggtccgcagctcgggctgctgcgcgcagcccggtcggcgttggggcctgcgctgggcgtgtggcatggaggttcctgaagtcattgaattggctcgcttgcgatagcgggggaaacgcggtccgttcctagaattttctggcgggttcggccggccggagtatggccaccgggcaccgatgcaggaattccgattaacccggtgtggagacaaaaaatggatacggcactgacagcagtacaggcacggccagaagaccagcgggcggcaggaacgacggtggcggttgcacgggccatcgccatgacggcgtgtctggctttgacggcctgcgggggaggcggttcttcgggctcgtcgtttgcgttccttcctgtcgcgccacccgcgcctccaccgcccgctgcgccgcccccggccgccgacggccccatggtgcgccagaccaccgccggcaagatcgagggcgtggacgacagcgccaggacgggcacctggttctggaagggtgttccgttcgcgcaaccgccggtcggcgcgctgcgctggcgtgcaccggccgagcccgcggcctggagcggcattcgcccggccacgaagttcggcaacgcctgcctgcagatcggccggcttttcagtcccggcaccaacaacacctacgacgccaccatcggcaccaacctgggcaagccggtcggcagcgaagactgcctgttcgtcaacatctggcgcccggccaccaccgacgcgaacctgccggtgctgctgttcgtccatggcggaagcaacatatcgggctacacggccgacccgctgtatgacggcgccgcgctggcgaagaacgccaacgcggtggtcatcaccgccagctaccgcctgggcatcctgggcttcctgaacctgccgcaattgcggccgggcggcaccgcgggcgacgactcgggcaacttcgcgctgctcgacaacatggcggcgctgcgcttcatcaggaacaacgtcgcgggcttcggcggcgatccgaacaacgtcacgctgtcgggcgaatcggccggcgccaccaacctgctggcggtgatgacttcgccgatggccaagggcctgttccacaaggccttcgagatgagtggcggcatttcgcttgcaagcaacctgccgcccggcacgctgccttcgctccagccggccgcggtttcgctcgcgcagggccaggccatcctggagaaactgctcgtggccgacggcaccgtcgccgacgcggcggccgccaaggcctacatcggcacgcgcaccccggcacagattgccgactacctgcgcgcacaggaaggcggcgccatgctggccacggtggtcgccgccggcctgggggccgtcgggcccattcccgacggcacggtgatccccaccgacccgatcggcgccatcgcggccgaccagtacgtgaaggtgcccttgctcgcgggcaacacgcgcgacgagggcaagctcttcgcgtcgctgctgccggccatcggttttccgaagtccggctggatcgtcaacgacgcccagcgcttttcgatgatgttcaacttcgaccccgacgcggcgccctcgctcacggtggccgacatcatcgatccgttctacctgccggtagacacccccgtcacgggctacaacgcggcgacggggctcatcacgaagcatcttttcgaggccaatcgcgacaacctcctcaatacgatgaagacgcgccagtccaacatctggcactaccgcctcgattgggcgcaggaaccgtcaccgtggaacgacgtctatggcgcctcgcacgccttcgacctgccgttcgtattcggcaacttcggcccctcgctgctcagcggcgtgatggccgccaaggccaaccagccgggccggctcgccttgtccaacgccgtcatggccagcgtcggcgcgttcatgcgaaagggcgatccgaacgccgccgaactcggcacaaactggacgccctggccttcgagcctgctgctcgacgccacgccgatggcggcgaagatcagcgtgcagtaggcgccgtgtccctcgagttccacgtgcgggtttctgtcattgtgcgaatggccgaagattgagtgaatccgttgtccgcaaagttttagcagccatttcacaaatgacaggagtctctagatgctgggtttgatgcaagaccaaccgcttttgatctcatcgctgatcgagttcgccgagcgccaccacggcgacgccgagatcgtctcgcgccgcgtcgagggcgatatccaccgaagcacctggggcaagatcgcatcgcgctcccggcaggtggccaatgcgctggacggcgagcaactgctgttcagcgaccgcatcgccaccctggcctggaacggctaccgccacctggagctgtactacggcgtgagcggcacgggccgcgtgctccacaccatcaatccgcgcctgcaccccgaccagatcgcatggatcgccaaccacgccgaagaccagatcctgtgcttcgacctgagctttctgccgctggtgcaggcggtgcatgccaggtgcagcaccatcagaaagtggatcgccttgtgcgatgccgacaagctgcctgccgacagcggcattcccaacctcgtgagctacgaggcctggatgagcgggcaatcgacggactacgactggcccactttcgacgagaactccgcttcgagcatgtgctacacgagcggcactaccggcaaccccaaggcggcgctctacagccaccgctcgacgctgctgcacgcctacgctgcggcgctgcccgacgtgatgtgcatctcggcgcgcgattcggtgctgccggtggtgccgatgttccacgtcaacgcctggggcatcccgtattcggccgcactggtgggcgcgaagatcgtgttcccgggcccggcgctcgatggcaagtcggtgttcgagctcatcgagtccgaaggcgtgaccttcgcggccggcgtgcccaccgtgtggcagatgatgctgggccacatgcaggccaacgagctgaagttctccacgctcaaccgcaccgtcattggcggctcggcctgcccgccggccatgatccgcgcgttccaggacatctacaaggtcgaggtgctgcacgcctggggcatgaccgagatgagcccgctgggcacgctgtgcacgctcaagaacaagcatctcgccatgccggccgatgcccaactcgcgatccgcctgaagcagggccgcgcgatcttcggcgtcgacatgaagatcgtcgacggcgacggcaaggcgctgccctgggacggcaaggcctacggcgacctgctggtcaaggggccgtgggtcgtgaaggaatacttcaagggcgaaggcggcgatccgctcgttcccgacgagcaggggcgcggctggtttcccaccggcgacgttgccaccatcgaccccgacggctatctgcagatcaccgaccgcagcaaggacgtgatcaagtccggcggcgaatggatcagctcgatcgagatcgaaaacatcgccgtctcgcatccggccgtggccatggcagcctgcatcggcgtggcgcatcccaagtgggacgagcggcccatcgtcgtggtggtgaagaagcccagtgccgaggtcacgcgcgaagagctgctcaagttctacgaaggcaagacagccaagtggcagattcccgatgacgtggtcttcgtcgaggcgattccgctcggcgccaccgggaagattctcaagacaaagttgcgcgaactgttgaaggactacaagttgcccaccgcgtagccgcactgtcgcgcacgcgatagccaggccgccttggcggccctgcttgcgggcattccctgtgcggcgaaaaaaagggcgcttgtacgctgcgatctcggcccatcatccctggagactcctcatgtcccgtgctatcaagtcagtagctttctgcgcaatgctgctcagcgccacagcctctttcgcccagaagggcgagaccgtcaaggtcgcctggctcgacccgctgtccggcctgatggcggcggtggggaccaaccagctcaagaccacgcagttcatggtcgaggagttcaacaagaagaacacctccggggtgaagttcgaactcatcgccatcgacaacaagctgagcccgcaggaaaccaccagcgccttgcgctccgccatggaccagggtgcgcgctacgtgatgcagggcaacggctccgggcccgccttggccatcatcgatgcgctcgaaaagcacaacgcgcgcaacccgggcaaggaactcgtttacatcaactatgccgcggtcgaccccgatctcaccaacagcaagtgcagctactggcacttccgcctcgatgctgacacctccatgaagatggaggcgctgaccaccttcatgaaggacctacctgaagtcaagaaggtctacctgctcaaccagaactacgcgcacggccagcaggtctccaagttcgccaagcagaacctgaaagacaagcgccccgacatcgagatcgtcggcgacgacctgcatcccctggcgcaggtgcgcgacttcgcgccctacatcgccaagatcaaggcctccggcgccgattcggtcattaccggcaactggggttccgacctcgcgctgctcatcaagtcggccaacgactcgggcctgaacgtcaagttctatacctactacgcctacggcaccggggcgccaaccgccatgggttccggcgccgacgggcgtgtgttcgtggtgggctacggccactacaacatgggcggcgacatccagcggatcatgggcgaatacaagaagaagatgaacgacgacatggtgcagacgtcgatctatcacgccttcgcgatgctcgacaccgccttcgtcagggcccgctccaccgatcccgtgaaggtggcggccaccatggaaggcatgaagttcaagagcttcaatggcgaaatcgaaatgcgcaaggccgaccaccagctgcagcagggcctgtggatcaccaagtggcaaaaggcgggtggcaagttcccctatgacgccgagaacacgggctacacgatggcgccggtgaagtattacgaatcgtatgtggccagcacgcccaccacctgccagatgaagcgcccgtagggcattttgcaaacggattttctacccttgggtagcaccggttcagccgccggtagcaccttggagaaatgcagtgtcgcctgcgcgatagaaacggcctttgcagccgccctcttacgggcattccctgaggggaggggctgcaaacgcttgtactctcgtgcggccttttgaacggtttgaccaggagatatagatcgtgaagttcgctctgaaaatcgctacagcagccatcctttccgcagccgccaccggcgcgctggcgcagaagggtgaaaccgtgaagattgcctggctcgacccgctgtccggcctgatggcggcggtcggcaccaaccagctcaagacttaccagttcctggccgaggagttcaacaagaagaacgccgccggggtcaagttcgagatcatcggcatcgacaacaagctgagtccgcaagagaccaccagcgcgctgcgctcggcgcaggaccagggcgcccgctacgtgctccagggcaacggttcaggcgcggcgctggccatcatcgatgcggtcgagaagaacaatgcccgcaaccccggcaaggaactgctctacatcaactacgccgcagtcgaccccgacctgaccaacagcaaatgcagctattggcacttccgcctcgatgccgatacctccatgaagatggaagcgctgaccaccttcatgaaggaccagccggacgtcaagaaggtctacctgctcaaccagaactatgcgcatggcgttcaggtggccaagttcgccaaggaaaacctcgcacggaagcggcccgacgtgcagatcgtcggcgaggatctccacccgctggcccaggtgcgcgacttcgctccctacatcgccaagatcaaggcgtcgggtgccgacaccgtcatcaccggcaactggggttccgacctcgccttgctgatcaagtcggccaacgatgcgggcctgaacaacgtcaatttctacacctactacgggagcgtgagcggcacgccgaccgcgatgggcacagcgtcagccggcaaggtgtaccaagtgagctacggccactacaacatgggtggcgacatccagcgcctggcggtcgagttcaacaagaagttcaaggaagacctgtacacctcgtcagcctatacggcactgctgatgctgagcgaggccttcgccaaggtgaaatcgaccgatcccgtcaaggtggctgccgcgctggaaggcatgaagttcaagagcttcaacggcgaagtcgaaatgcgcaaggccgatcaccagttgcagcagggcctgtacatcgccaagtgggagaaggcgggaggcaaattcccgatcgacgcggaaggaacgggtcacaccttcgtccccgtgaagtactacgagccatacgtcgcgagcacgcccacctcgtgccagatgaagcgacccaacaattcctgattgcctgatcgcgcgctgaccggtcgaggcccgacttcaccactcgggcctttttctttttcaaccgacacgaaagaccgatgaacgtcgaattcttcgtcatctcgctgctcaacggcgtcagctacgggctgttgctgttcatgctgagctctggccttacgctgatcttcagcatgatgggtgtgctcaattttgcgcatgccagcttctacatgctcggtgcgtacattgcgtacacactgtcgggcatcatcggcttctggccggcgctcttcatcgcgccgctcctggtgggcctcttgggcgctgccttcgagcgctacagcctgcgccgggtccacaagttcggccacgtgcccgagctcctggtgaccttcggcctttcgtacctgattctcgagctggtgcagcttgcctggggccgctcgacggtgccttacggcctgccgccgcagctgcaggggccgctgttctcgctttacggcacgcagtttcccaagtcgcgctcgttcatcatgctggtggcggtgctgatgctcatctcggtgtggctgctgctcacgcgcacgcgcatcggcctggtgatccaggcggcgctcaagcaccccgacatggtcgaggcgctgggccacaacgtgccgcgcgtcttcatgctggtgttcggcggcggtgccgcgctcgcgggcctcgccggcgtggtgggcggcaacacctacgtcaccgaaccggccatggccgcgtcggtgggctcgatcatcttcgtggtggtggtggtcggcggcatgggttcgctggccggcgcgttcctcgcgtcgctcctgatcggcatcatccagaccttcgcggtggccatggaccagtcgtttgccggcggcctgcagatgctgggcgttgccgtgacagaccagaccttcggctacgagctgctcaagctcacgatctcgcaggtcgcgccgatcctgccgtacctgttcctggtgctgatcctcatcttcaggcccaagggcttgttgggcactcgggaggattgaatgacacaagcacagtcccccaccatcgccgccgaccctcgcgccaaccctcttgcgacagcagagggcacaagaaagggtggaaccgaaatgacatcgacgaccgcagccccgaccacgcagtactaccgcttcaagccctggaacatcgggcgcttcctgatctggtcgctgttcgcagtcgtgctgatcatctcgccgctggtgttcaagagcagcctcgccctcaccatgctctcgcagatgggctatctcatcatcatctgcctgagctacaacatcctgctggggcagggcggcatgctgagcttcggccatgcggtgtacgttggtcttggctccttccttgccattcatgcgatgaacatgggcagcaagggcggactgcagattccgctcgtggccattccgctggtaggcggcctggccggcatgttctttgccatcctgctgggcttcgtcaccaccaagaagtcgggcaccaccttcgcgatgatcaccatgggcataggcgaactggtggcctccatggcgctgatgttcccgagcttcttcggcggcgagggcggcatcaccaccgaccgggtctacggcccaaccttcttcggcttcaacttcggctcgcagatccaggtgtactacctgatcgccgcatattgtttcgtgtgcaccgcgctcatgtttgccttcaccggcacgccgctcggccgcatgctcaacgctgtgcgcgacaacccggagcgcgtggagttcatcggctacaacacgcagcgcgtgcgctacttcgcattcatcatcgccggcttcttcgccggcatcggtggcgggctggcgtcgatcaacttcgagatcgtgaacgcggccgacagcctgagcgccatccgctcgggcggctacctgctgttcaccttcctgggtggcgcggtgttcttcttcggcccgatcatcggcgcggtgctgctggtgttcgcgtcgatcctgctgtcggagctttccaaggcctggcagctctacttcggcctggtgttcgtgttcatggtgatgttcgcgcccggcggcatcgccagcctggtgatgatgaacctgcgggtcgccaagttcggcaagttcaaccgcttctggctgctgtacatcgcactcgcggtggcactggtgccggtcgtcgtcggcgccgctgcgctcatcgagatgatctatcacatccagctcaacgcggcgatgggcccgaacctgaacttcttcggcgtgacgctggatacgtcgggcatggcaagctggctggtcgcggcggccatcctggcggtcggcctcggcgcactcgaggtggcgcgccgccgcttcgtgcgtgtctggggccgggcacaggaagaaatcgaagcagaaatcaaacgtcgggaggcggcgtaatgagcgcgcaacacgcactggaactgaaggcgctgcgcaagaatttcggcaagaccgaaatcatccgcggcgtggacctggcggtgaacgccggggaacgcgtggccatcatcggcccgaacggggcgggcaagtcgacgctgttcaatctcatcagcggacgtctggcgcccaccagcggcgaagtgctgctgaacggcgagcgcatcgacggcaagaagcccttcgagatcaaccggctgggcctgtcgcgcagcttccagatcaccaacatcttccccaagctcagcgtgttcgagaacctgcgctgcggggtgctgtggagcctgggctaccgctacaccttcttgcgctttctctcgaacctggacgacgccaatgcgcgcaccgaggagctcatcaagcagatcggcctggagcgcaagcgcgacgtgcacgcggtgaacctcacctacgccgagcagcgcgcactcgaaattggcgtgaccatcgcgggcggcgccggcgtcattctcctggacgagcccacggccggcatgagcaagaccgagacctcgcacttcatctcgctcatcaagcacgtcacggtcggcaagacgctgctcacggtcgagcacgacatgggcgtggtcttcgggctggccgacaagatcgcggtggtggtgtatggcgaagtcatcgccttcgacacgccggcggctgttcgcgccaatgcgcgggtgcaggaggcctacctgggctcttcggtcgctgatgcacaaagccagggccagggacactgacatgctgaagcttcacgacatccacgcctactacggcaagagccatgtgctgcatggcgtttccttcaacgtcggggcgggcgagatcgtcgcgctgctgggccgcaatggctccggccgctcgaccaccgccaaggccatcatgggcctggtgcatgccgagggcacgctgcgctggaaagaccaggacatcctgcgcaggaaagcctacgagatcgcccacctgggcatcggctacgtgcccgagaaccgcgacatctttcccaagctcacggtacaccagaacctgctgctggggcagaagggctcgggcaagggcagccgctggtcgttcgacgacatgtacggcatgttcccgcgcctgaaggagcgccagcacaccgaggccggcgtgctctctggcggcgagcagcagatgctcacgctgtgccgcacgctcatgggcgaccctgacctgatcatcatcgacgagccgaccgagggcctcgcgcccaagatcgtcgagctggtggggcagtacctgaagacgctcaagaacaagggtatttcggtgctgctgatcgagcagaagctgaccattgcgatgcagatctccgaccgtgcgctggtaatggggcacggcagcatcgtgttcgacggcacacccgacagcctgcgtgccgatgcgaccactcgcaaggagtggctcgaagtctagggctcgcccccaggcttcgcgcacgctttttccacccccttgcgggggcagcaccagcggtccggcagagccggttccgcggtgttcctggaacgggctgtaacctttaatgagtcttgtctcggcagcgactgcgtgccattgtgaggccacgcgaaacgcctagaatccctcgaaaaagaacactcgtgctttttcttctttttcttcacacaccaaggaatgcagcatgacggctgaatacaaagtgctcggcgatgtcgccgtgatcacactgaccaacccgccggtcaacggtctcggtttttcgacccgcatcggcatcaccgatgggttgtcgaaggccaatgccgacgacgccgtcaaggccatcgtcatcacgggcgccggcaaggccttctcgggcggtgcggacatcaaggaattcggcacgcccaaggcgctgcaggaacccaacctgctgagcgtcatcctcgcgctcgaagcttcgccgaagcccatcgtcgcggccattcactcggtgtgcatgggcggcggcctcgagctggccctgggctgccactaccgcgtggccgctcccggcaccagcatcgcgctgcccgaggtcaagctgggcctcatccccggcgccggcggcacgcagcgcctgccgcgcgtgcttggcgtggaaaccgcactcaacatgatcgtgagcggcgagcccgtcaagagcgaactgctggccagcctgccgggccagaagcttttcgacaagctcaccgtctcgcccgaatcggtgttcgaggaagccgtggccttcgccaagagcgtggccggcaagagcggcgacgcattgccgctggtgcgcaacctgccgtgcaagcacccgcagggcgatgcctacttccagttcgccaagaacatggtcggcggcatgtcgaagaactaccccgcgccgctgcagtgcgtggaggccgtacaagccgcaacgaagatgaagttcgacgccggcatggccgaggagcgccgcatcttcacatcgctgatgttcacgcccgaatcgctggcgctgcgccacctgttcatggccgaacgtgcggcctccaagattcccgacgtggcggacgacacgtccaagcgcgagatcaagtcgatcggcgtgatcggcgccggcaccatgggcggcggcatttcgatgaacttcctgaacgcgggcatccccgtcaagattctcgagatgaagcaggaagcgctcgaccgcggcattgccaccatcaggaagaactacgaatcgcaggtcaagaagggcaagctcaagcaggacaagtacgagcagcgcatggcgctgttgagcaccacgctgagctacgacgacctgaaggacgccgacctgatcatcgaagccgtgttcgaggaactcggcgtcaaggagaaggtgttcaaggaactcgatcgcgtcgccaagaagggcgcgatcctggcttccaacacctcgacgctcgacgtcgacaagatcgcctcgttcaccgaacgtccgcaggacgtggtcggcatgcacttcttcagcccggccaacgtgatgaagctgctcgaagtggtgcgcggcaaggaaacggccaaggacgtgctcgccaccgtcatggacatcggcaagaagatcaagaagacggccgtggtctcgggcgtttgcgacggcttcatcggcaaccgcatgatcgagcagtactcgcgccaggcgggcttcctgctggacgagggcgccacgccgcagcaggtcgacaaggccatcgagaagttcggctttgccatgggcccattccgcatgggcgacctggccggcaacgacatcggctgggcgattcgcaagcgccgcgccgtcgagtatcccgacatgaagtacagccgcacggccgacaagctgtgcgagctgggccgcttcggccagaagaccggggcagggtggtacgactaccaggccggcaagcgcgacgcgattccgtcggacctcgtcaacaagatgatcgaggaccaccgcaaggagcttgggatcacgccgcgcaagatttccgatgaagagatcgtgcagcgcctggtgtatgcgctggtgaacgaaggcgcgcacatcctcgaggacggcattgcctcgaagtcgggcgacatcgacatggtgtacctcaccggctacggcttcccgatctggcgcggcggcccgatgcactacgcatcgcaggtcggcctgtacaacgtggccgaaaccatgaagcgctttgccaagaacccgcgcgacgacgccgagttctggcagcccgcgccgctgatccagaagctggtggccgaaggcaagcagttcagctgacagcagacccggagccctgaccgcctatgttgaaacgcatctttctcgggctgctgctggtgcttgtggcactggtggcggccgtggcggtcaagacctggaccacgccgtcgcagcagctggcggtggcgccggcacccaaactcgagatggacctgcaggccgccgccaagcgactggccggcgcgattccgatccgcacggtgtccagcctcgacgatccggccaccaatctggccgagttcgacaagctgcacgcttacctcgaacagcagttccccaaggtccacgccaccctcaagaaggaagtggtgggccagcgggcgctgctctacacatggatcggtaccgacgcctcggccaagccgatcgcgctcatggcgcaccaggacatggtgcccattgcgcccggcaccgagaaggcgtggacggtcgaccccttcgcgggcgaaatcaaggacggctacgtctggggccgcggcacgctcgacaacaagggcaacctgtttgcgcagatggaggccatcgatctgctgatcggcagcggcttcaagcccaagcagaccgtgtatctcgtgatgggcgacgacgaagaggtgggcggcctgcgcggtgcgcggcccattgccgagctgctgaagtcgcgcaacgtgcgcctcgactgggtgctcgacgaaggcctgctgattctcgacggcgtgctgcccggcctttcgaagccggctgcgctcatcggcctggccgagaagggctatggcaccttctttctttcgctcgacaccgcccccggccactcgtcgatgccgccgcagcgcagcgccatcggcagcatgagcgccgcgcttgcacggcttgaagccaaccagatgcccggcggtatcaaaggcgtggcggcccagatgttcggtgccctcgcgccggagatgagcagcatgaatcgcgtgatgctctccaacctgtggctcaccgaaccactggtgcgcagccaactccagaagagcccgagcagcaacgccatgcttcgcacgaccaccgcattgaccatcgtgcgcgccggcaacaaggacaacgtgctgcccggccgcgccgaggctgccgtcaacttccgcatcctgccgggcgacaccatcgacagcgtggaggcgcacctgcgcaaggcgctcggcaacgacgagatcaagatcaagcgctaccccggcaactccgagccttcgcccgtgtcaccgacggacagcactggctatcgcgccattcaacaggcggtgcgccagtcgtttccggatgtggtggtggcccccggcctcatgaccgccgccaccgactcgcgccacttcagtctggtgagcgatgccgtctaccgcttttcgccgttccgcatgaagagcgaagacctggcccgtttccatggcaacaacgaacgcctggccatctccaactacggcgagatgatcggcttctatcaccagctcctgcgcaacaccaacgctgcgccggcgcaatgacgacaacaaacctctttcccttccatcttcaaaggacctcaccatgaccagcgccgtcattgtttccaccgcccgcacgccgctcgcgaagagctggaagggtgccttcaacatgacgcacggcgccacgctcggcggccacgcggtgcagcacgccatcgcgcgcgccggtatcgaagccgccgaagtcgatgacgtgatcatgggttgcgccacgcccgagggcgccaccggctccaacatcgcgcgccaggtcgcactgcgcgccggctgccccgtcaccacctcgggcatgacgatcaaccgtttctgctcctcgggcctgcagaccatcgccaccgccgcgcagcgcatcatcgcgggcgaaggcgaggtgtacgtggccggcggcgtcgagagcatctcgtgcgtgcagaacgaagccaacaagcacatgctggccgacccctggctggtaaagcacaagcccgagatctactggaacatgctgcagacggccgagcaggtcgccaagcgctacaacatcggtcgcgacgccatggacgaatacggcgccgccagccagcagaaggccaccgccgcgctcgaagccggccgcttcaaggacgagatcgcacccatcaccgtgctggccggcgtggccgaccccgtgatgggcctgcgcaccaaggaagtcacgatcgagaacgacgaaggcatccgcgccggcaccaccaaggaaggcatcagcggcatccgaccggcgctgcccggcggcctgatctcggccggcaatgccagccagttctccgacggcggcggcgcctgcgtggtggtcgacgagaagtacgcagagcaaaagggcctgaagccgctcggccgcttcctcggctttgccgtggccggctgcgagcccgacgaaatgggcatcggccccgtcttcgcgattccgaaggtgctcaagcgcctgggcctcacggtcaacgacatcgacctgtgggaactgaacgaagccttcgcggtgcaggtgatctactgccgcgacaagctcggcatcccggctgaccgcctgaacgtggacggcggcgccatcgccgtgggccacccctacggcgtgagcggccagcgcctcacgggccacgcgctcatcgaaggcaagcgccgcggcgcgaagaaggtgctggtcacgatgtgcatcggcggcggtatgggtgccgcaggcgtgtttgaagttctttaactctcgcccagccggcggcgcatagcgcgccgccgccttcgccaaccccgttcaggggggacaccagcgggccggctgagccgcttccgcggtgttccaggcacaggacccgcgcatccattcacaccgagatcgatcatgagcctgcgtcccaccctcgacttcctgctctacgactggctcgacgcggaatcgctgagccagcgcgagcgttttgccgaccactcccgcgagactttcgacgcggtgctcgacacctgcgaacgcatcgcacgcgaaaagtatgcgccggccaatcgcatcgtcgatacgcaggagccgcacttcgacggcgagaaggtcgtattgccgcaggccacgcacgatgcgcacaaggccttcgtcgaatccggaatgatgagcgcggcgcaggactacgacatcggcggcatgcagctgccctacacgctgcaggccgcggccaacggcttcttcgcgatggcctcggtgagcatcggctcgaacatgctcaccagcggcaacgccaacctgctgatggtgcatggcaccgagatgcagaaggaggtgttcgccaagaacgaattttcgggccgctgggccggcaccatgtgtctctccgagccgcaggccggatcgtcgctgagcgacgtggccacgcgcgccgtacccgacggcgcggaccatcagaacgatccgctcgggccgcgctatcggctcacgggcaacaagatgtggatctcggccggcgaccacgagctgaccgagaacatcgtgcacatcgtgctcgccaagattcccgacgccagcggcaagctggtgccgggcacgcgcggcatctcgctgttcatcgtgccgaagtggctggtgaacgtggagaaccctcaccccggccctctcccgcaagcgggagagggggacggcagcgtgaaggtcacgctgggcagcaggaacgacgtggccctcgcgggcctcaaccacaagctgggctggcgcggcaccaccaacacgctcctgaacttcggtgaaggcaagtacccggtcgatggcaaggcgggcgcggtgggctacctcgtcggcgagcccggcaagggcctgcactgcatgttccacatgatgaacgaggcgcgcatcggcgtcggcacggccgccaccatgctgggcatggccggctactacgcctcgctcgactatgcaaaggcgcggccgcagggccggctcctgaagaaacccgagacgggcgccggcagccaggtcgtgaaggactcggccagcccgcaggtgcgcatcatcgaacacgccgacgtgcggcgcatgctgctcgcgcagaaggcgtactgcgaaggtgcgctggcgctggagctgtactgcgcccggctggtcgacgagcaaaaaaccggcggtgcgcaggccgcggacgacgcgcgcctgctgctggaggtgctcacgcccatcgccaagagctggcccagcgagtggtgcctggaagccaattcgctggccatccaggtgcatggcggctatggctacacgcgcgactttccggtggagcagtattggcgcgacaaccgcctgaacatgatccacgagggcacccacggcatccaggccgccgacctgctgggccgcaaggtgctgatggaaaagggccgcggcctgcaattgctggccggccgcatcaccgacaccatcggccgcgcggccacggtgcccgcgctcgcggggcatgcccaggcgctgggcgccgccctgcagcgcatcggtactgccaccgaggccgcctggtccaccggcgacccggccgacgcactggccaacgccgtgccctacatgcaggcattcggccataccgtgctggcctggatctggctggacgtggcgcggcgagcgctggaaatcgacgcagagaaggccagggccgtaacagctggcaagattggcgccacggactatttcttccactacgagctgccgaaaatcggcgcctggctcaatgtggtcgagagccgcgaccccacctgtacagcattgcccgaggacgctttctgataatggccaacgccgctcccaacaacaccccgaaccccgtcaagcccccgaagccgcacgcccggctcgagaagtggatctggatcctgatctacggcggcctgtttctcgtgatcctcggcattgccacgggccgcaccgagcccgccatcggctggtcgatggccgtgccaggcggggtgatcgccctggtgggctttgcgctcatctacgtgcgctctcgcctcaatgacaaataaggaaggcgtgaccatgctgaatccggaacatcggcgcagtcgcgaagcgcggcaatgcttggactatgaaacctgaaccccgtgtgcccgacgcaaaggccacttcggcggatcggcgggcgtacggtcgcgcacagcgcgcgcactttccgctcgaacagtgggcacaggcgcccaagcccgatgcggcaggccgcagcccgctcggctggctgaaggcgtccaaccgcggccgggtgcccgaactggtgccggtccgccatggccgcatgctggccacgccgttcaccttctaccgcggtgccgccagcctgatggcgaacgacctggccaggttgccgcacagcggcattgcgacgcaactgtgcggcgatgcgcaccttgcgaacttcggcttcttcgccagccccgagcgctcgctggtcttcgacatcaacgacttcgacgaaaccctgcaggggcccttcgactgggatgtgcgccggctcgccacctcgtttgtcgtggccgcgcgcgatctgggcttcaagccgcgcaccgggcgcgacgcggtccggcaactggccgaggcgtaccgtgaccgcatgcgccgcttcgcgcgaatggacacgctggaggcctggtacgcgcgcctcacgtcccaaacgctgctgaaactcggtgccgaggatgcgaccgagcttgcggtcatcaagaaggcccggcgcagcacctcgcgcgtgtttgccgaagaggcgaccgagatggtggagggccgcctcatggtgcgcgaccggccgccgttcgtctatcacgacgccaaggccaccgcgcgcgagatcggccgctttcgctccggattgccggcgttcctggcgcagtaccgcgccagccttccgcccgaacgccagcggctgttcgatcgctatgagctgcacgacgttgcggtgctgacgcctggcgtcggctcggtgggccggcgctgtttcctgctgctgatggtggccgaccaggcccatcctctgttcctgcagtgcaaggaagccggcgaatcggtgctggaggcccatctgggcccggcgccgggatcgaactctcccggccagcgcgtggtgcaggggcagcggttggcgcaggccgccagcgacgttttcctcggctgggccgaggcgtccggcggacgcggcttctatgtgcgccagctgcgcgacatgaaggcgtcctacaagctcgaagacttcaagccggtcgatctcgtcgagtttgccgaggcctgcggctacagcctggcgcgcgcgcatgccaagggcggcgacgcctgggccattgccggttacctcgggcgctccaagacgttcaacaccgcgctcgcagactttgccgaggcctatgccgacgtcaaccaggccgactggcgccagctgaaaaaagcagtggcgtcgggcaagctcgccgccgtcaaggccgtcggcgacgcttcgtagcggcggcaggcaagccacgaatccttctttcacatgttccggagacaacagacatgacaccccgcaccaccaagcaactcttcgacctcaccggcaagacggccctcatcactggcggctcgcgcggcctgggcctccagatggcgcattcgctgggagaagccggcgcgaagatcatgctgagttcacgcaaggccgacgacctggaacaggccgcagccgagctgcagtcggccggcatcgacgcgcgctggatcgccgccgactgctcgaaggaagaagacacgcgccgtctggccgacgaaacgctgcagcgcatgggcgcgatcgacatcctcgtcaacaacgcgggcgccagctggggcgcgccggccgagagccatccggtcgaggcctgggacaaggtgatgaacctcaacgtgcgcggctacttcatcctgtcgcagcacgtcgccaacggctacatgattcccaggaagaccggccgcatcatcaacatcgcctcgattgccggcctcaacggcaatccgcccgagatgcagacgctggcctacaacacctccaaaaccgcggtgatcggcttcacgcgcacgctcgcggccgaatggggccgctacaacatcaacgtgaacgcgatctgcccgggcttcttcatgacgaagatggccgccggcctgatcaagtcgctcggcgaggaaaaaatggcctcgcatgcgccgctcggccgcctgggcgacgaggaagacctgaagggcatcgcgctgctgtacgccagcgatgccggcaagcacatcaccggccagtggctggcggtcgatggtggcgtcagcgtggtgctcggtgcttgaaatggccgaaaaagattccaccgacatcaacatccgctcgtacacgagccagatcccgtttgcgcgccacctgggtttcgagctcaccaagttcgagggcggcgagtccgagatcatctacacggccaagcccgagcacctgaacaccttcgacgtgacgcacggcggcgcctgtatgacgctgctcgacatcaccatggcggccgccgcacgcagcgtggcacccgagatgggcgtggtcaccatcgagatgaagaccagcttcatgcagccttcggtcggtccgctgcacgcacgcggcacgctcatccaccgcaccgcaacgctggccttcacggaagccaaaatctacgacgagctggagcgcgtgtgcgcgcatgccaccggcaccttcaagtacgtgaagcgccgcctgcccaccggccccgcgagcgccaacgcgatgcgcccgccttccaccgattaattgcattcccccggagacactcatgcctacgaacaaacagatccacctcgacaaccgccccgatggcgaggccgttgccggcaacttcaagctggtaaccgccgagacgcccgcgctggccgacaaccaggtgctggtgcgccaccacttcatgagcctcgacccgtacatgcgcggccgcatgaacgattcgaagagctatgcgcagccgcagccgctcggccaggtgatgcagggcggcacggccggcgaagtggtcgaaagcaggcaccccaggttcgccgccggtgacaaggtggtgggcttcggcggctggcaggaatacagcgtggtcgatgcctcgcagcccggcgcactgaagaaggtcgacaccacgcacgtgccgctgtcgcactacctgggcgcggtgggcatgccgggcgtcaccgcctggtacggcctggtgaagatcattgcgcccaaggccggcgagacgatggtcgtcacggccgccagcggcgcggtcggcagcgccttcggcgcgctggccaaggcgcgcggctgccgcgtggtgggcatcgcgggcggcccggacaagtgcaagtacgtgaccgacgagctgggcttcgacgcctgcatcgactaccgccagcatcccgacgtgaagagcatgagcgccgcgctcaaggaagcctgcccgaacggcatcgatggctacttcgagaacgtgggcggctacatcttcgacgccgtgctgctgcgcgccaacgccttctcgcgcgtggcgctgtgcgggatgatcgcgggctacgacggccagccgctgccgcttgcgaacccggcgctgatcctcatcaaccgcatgaagatcgaaggcttcatcgtcagcgagcacatggaagtgtggcccgaggcgctgacggagctcggcaccctggtgggcaccggcaagctcaagccgcgagaatcggtggcacaaggcatcgaatccgcccctgaggccttcctgggtttgctcaagggcaagaatttcggcaagcaactggtcaagctgatctgatgaactgaacgcacggcagaaagtccggtcatgcgcgccgggccggtccaagcaggtgtgcaccgcagtgcgaagcacggaggtattcgaatgaattcgacgcacgaggtcttcaaccagcccgaaccgctggtggactacaacctcttcgaaaccaaccggccccttcgcgatgcgctgaagttcaacgcgccgcagttgcatgtggcgcagttgcaagagctcggggtcaccctcggctcggccgagatgcaggcgcatgcgcggctcgccaacacccacacgccagagttgcacacgcacgaccgcttcgggcggcgcatcgacgaggtggagtttcatccgagctatcacctgctcatggcggccgcggtcggcgcgggcctgcatggcaccccgtggaccggcatctcggaatcgccgcacgtacagcgtgccgccggcttcatgctcttcaccgagctggagccgtcggtcctttgccccgtctcgatgacctatgcggccacgccagccctgcgcggcaatgccgccgtctacgctgactggggtccgaagctcggcagcctctggtacgacccggcgcttgccttcgtcaaggagaagcccggcgtgaccatgggcatgggcatgaccgagaagcagggcggctccgacgtacgggccaacaccaccaaggccgtgcgcgacggcagcgacgactggggcgagcgctatgcgatcaccggccacaagtggttcttctcggcgcccatgtgcgatgccttcctggtgctggcccaggcgccggccggcctgagctgcttcttcctgccccgcgtattgcccgacggcacccgcaacgccctccacatccagcgcctgaaggacaagctgggcaacaaggccaatgccagttccgaggtcgagttccacggcgccagcgcatggctggtgggcgaagaggggcgcggcattccgcagattctcgagatgggcaccatgacccggctcgactgcgcgctgggcaccagcggcctgatgcggcaggctttgagcattgcgctcaaccacgccagccagcgcaatgccttcggcaagccgttgatcgaccagccgctcatgaagaacgtgctggccgacctcgccctcgaaagcgaagcctcgacggcgctggccattcgcctggcccgtgccttcgaccaccaggacgacgagcacgaacggctgatcgcccgcctgctcacgccggtcgccaagttctggatctgcaagcgcggcagccactttgcccaggaagccatggaatgcctcggcggcaacggctatgtggaagagggcggcgaaggcatcatggcgcgcatctaccgcgagatgccgctcaattcgatctgggaaggagccggcaacatcatggcgctcgacctgctgcgcggcctgcgcaagggcgatgcggtggccgcgctcgccgaagaactggcgccggcgcgcggccagcatgcggcgctcgaccggctggccgacgccctgccggcccgcatcgaggccatggcctccgaagccgaggctcgccgcctggcgcaggacgtggccctggcggtgcaggcttcgctgctcgcgcagaccgcaccggcggccgttgccgacgccttctgcgcatcgcgccttggcggcgactggggcaacgccttcggcacactgggcgcgggcacccatttcgatccgatcatcgagcgcgcgcagccgctctgaacgcagcaatatccaagcactccacgggaacaacaacatggccgacctcatcctgcatcactacaacacctcgccgttctcggaaaaagtgcgcctcatcctcggcgccaagaagctgccctggaagtcggtcctcattccgcccatcatgcccaagcccgaggtggaggtgctcaccggcggctaccgcaagacgccgttcctgcagatcggcgccgacatgtactgcgacagcgcgctcatcgccgacgtgctcgagcacctgcagcccgagtccacgctctatcccgagcccgaaaagggcatgtcccgcatcctcgcgcagtgggccgacaccacgttgttctgggctgccatggcgtggaacctgcagcccaggggcgcagccgaggtgttcgccaaggcgccgcccgaaatggccaaggccttcggcgaagaccgcggcaagatgagcgcggccaacatgacgcggctgcgcccggcggacgccaccagcgcctacaagtcatacctgcgccggctgtcggacatgctcgacgacaagccctacctgctgggcgaggtgccgtgcatcgccgatttctccgcctaccacccgctctggtacacacgccgcatcgactcggtgcggggcatcctcgacctcacgcccgcggtcaccgactggatggaccgcatggccgccatcggccatggcacgatcgagaaattcagtccggaagaagccattgccgtcgccaaggccgccaccccgcacacgctgctgaccgacagcaccttccaggacgaccacggcattccgctcgggagcgccgtcaccgtgcgcgccgagagcttcggcctcgaggaaacccccggcacgctggtggccgccacgcgcacgcactacacgctggagcgcagcagcgagcgcatcggcacggtgcatgtgcactttccgcgcatcggctacgtgctcaagaaagcggaggcctgacggccttcaagcggggaaccttcgtgactgcgcgggcgcgcgttccgtatttcaatagcggctccaacgtcagagacagacattcaacgcagaaggacaccggcaaatgattcaggacttcaagggcaagacggccgtactcaccggcgcgggttcgggcttcggcctcgaatgcgcgcgcatcggagcggcgcgcggcatgaacctcgtgctcgtcgacgtgcagcaggatgcgctcgacaaggcccaggccgagatggaagccgccggcgcgcaagtgctcgcgcgcaaggtcgatgtgtcggacgccgcgcagatggaggccctggcccttgccgtgaaggagcacttcggcgcgccgcacttcgtgttcaacaacgccggcgtgggtgccggcggcctggtctgggagaacaccgtggccgactgggagtgggtgctcggcgtcgacctgtggggcgtgatccacggcgtgcgcctgttcacgcccatgatgctcgaagccgccgccaaagaccccgcctaccgtggccacatcaccaacaccgccagcatggccgggctgctcacgccgcccaacatgggcatctacaacgccgccaaggccgcggtggtgagcctgaccgaaaccttgtaccaggacctgaacctggtcaccgaccagatcggcgcgagcctcttgtgcccgtacttcgtgcccaccggcatcaccagcagcgagcgcaaccgtcccaacgcgcccaaggaggccgaactcaccaagagccagctcatcggccaggccatgagcaacaaggccgtgagcagcggcaagatcaccgcggccgaagtcgcggccaaggtgttcgaagccatcagcgacaaccagttctacgttttcagccaccccaaggcgctgggcaatgtgcagagccgcatggagaacatcgtcgcggtcaagaacccggcagacccgttcctcgagcggcccgagatcgggcagaagctgcgggagcagttgcgggcggcctgaacggcccgcagccgcacatcacttcgctccccagacacccgtcggggccgtgcgtgcaacgtaggcggcaaagctgcgcggcgggcggccgagggcctgctccacgccgtgggcgacgggcgtgttgcggccgtccagaacggtgttgaacaggtagaccacgagcccggcaacatcgggcggcaggccggcttcggccagtgcctgggcataggcttccttcgagatgatctggcaggcgatctcgcggtccgtggcctggccgatctgcgcgatggcgtcggcaaagctgagcgcctgcgggcccgtcacttcatagagcttgcggctgtggcggccatcgaccagcgcttcggcggcgatgtcggcaatgtcgtcggcatcgacgaagggctccggtgccagcccttcgggcagggtgatggcgcccgcgacgatctcgtcgagaaagtagttctcgctgaagttctggaagaaccagctggcgcgcacgatggtccagtcgagcgaggtggcttgcagtgctttctcggcatccagggcctccggttcgccccggcccgagaggagcacgatcttctcgacgccggcctcggcggccgcatcgaagaacgcggtcaccgtctcgacggcgcccggcacgcacaggtccggctggtaggccacgtagacggcgcggacgtcctgcagggcggatttccaggttgcgggctcctcccaatcgaagcgcggctctgcggagcgcgagccgacgcgcaccgcgtgcccggcggcgcggaggcgcgccagaacgcggcctccggtcttgccgttggcgccgagtaccagaatgggatgcgcatcatcccgggtgctgctgattgccattttcgaactccttgagataatgtgagaaatgctcatataaaaaatgatagttactcacattttgaatgtcaaccccagggtgcagccatgagccgcaccgcatcgccgcgctctcgggtagcagccgcggaaccgcccacggcaagaaagagccccatccaggagcggagcaaggcgcgcgtggagcgcatcctcgaagcggctgccgagctgatcgtgcgaggcggaagcgaccagttgaagatgagcgaggtcgccacctcggccggtatttcgatcggatcgctctatcagtactttcctgaaaaatccgcgctgatccgcatgctggcggagcgcatcaacgcacgcagccgggagtgcatccgggacggcctgaaggacgtgaccgacctcgccagcctgcagtcgtcgttcgccgggctggtggacgtgtactacgcgatcgtcaacgagcggcccgtcatgcgcgacatctggagcggcatgcaggccgacaggcaattgctgacgctgcagattgccgagagccgcgtctgcggacagatgctggccgacgccatgcacaaggtgcacggccgcgccaacgcgaagcggatcgggcaggccgcctttctgatctgggaaatgggcgaggccaccatccgcctggccatcgcggtcgatcccgcggaaggcgctgccctggtggaggcgttcaagcgcatggcgctgcgggaaatcacaacccctctggcgtgagtttcggcggccgggtcacgccgcggcctgcgacgcgatccactcccacacggcgcgaatcgcggcttcgtcttcccgcccattcgccaccgcgagaaagtagctcccggtatcgagcgcaggcccgaagggctgcacgagcgcgccgctgcgcagttcttccgccgcgagcgtgaggctcagcaacgccacgccatggcccgcgagcgcggccaggatggcgtgggtttcgtccgagaacgacaggccggcggccttcatcgaccggcccctgggcggcgcaacgcccgcttcgcggaaccagctcgaccacggcgcggacgccaccgcgccaggctgccagtcggaatggatcagctggtgcttcggcaggtcgcccgcgcgcttgaggcccagcatcgggctgcacagcggcgcgtagcgctcggacatcaactcgcgcaccaccaggcccggccagttgccgctgccggagcgcaccgcaatgtcggcgtcgccgcgcgccaggtcgaccagcgtgtcgctggcatgcagccgcagttcgatgccggggcaggccttgcgaaaagccgccatgcgcggcagcacccagcgtgcggcaaaggcggtgttggtggtgagcgtgacggcctgcgatgcgacgggttgacgcagcctttccacgccagcctcgagcgcatcgaagccggcgcgcagatcgtcgaagagccgttcacccgcgggcgtcaacgcaagctgccgcgtgagccggcgaaacagcggccggccgagcgtgtcttcgagcgcgcgcacctggtggctgatggcagagggcgtgaccgagagttcgagcgcggcgcgctgaaagctcaggtgcgcggcagccgcttcgaaggcgcgcagcgagagcagcggcggcaggcggcgaggccggcggatggatgagccagtttcgttcatcgatggagaaatgatcgtttgtcgctgaatgggttcatctctagattaaagacccgtgcagccattctggcagcgcaagacagaatagatcaactcatccatgaagaccatgaacctgaaccttcttcatatcgacgccagcgcccgtccgggccggtcggacatcgacgcccacggctcgcacacgcgcaggctctctgcgcgctttgtcgagcgctggcgcaaggtccggccgaacgaccgcatcgaccatctcgacgtgggccagcatccgcccgcacacgtcaacggacgctggatccacgccgccttcactccgcccgccgaacgcgaaccctggatggcggacgtactggccgaaagcgaccggctcgtcgaccagctggttgccgccgacgtgatcgtggtgggcctgccgatgtacaacttcagcgtgcccgcgcagttcaaggcctacatcgacaacatcgtgcgcgtgggccgtaccttcggcttcgaccgtgcgcgcggcgcggtgccgtattggccgatgctcgcggacgcgggcaagcgcatggtgctgctcggcgcgcgcggcgaccacggctacgaccccggcggccgcattgcgcacctgaaccacaccgagagcagcgtgcgctcggtgttcggctacatcggcatcaccgaggtggtcgaggcggcggtggagtgcgacgagttcggcggcgagcagctggcgcagtcgctgcggcgcgccgaggaggccgtcgatcgcctggtggatcagctcatcggtacgacagcaccagcccgtgcaccagccgcgtccagccgtccagcatcacgaacagcagcagcttgaagggcagtgaaatggtggtgggcgcgatcatcgacatgccgagcgccagcagcgccgtggcgacgatcaggtccaccaccacgaacaccaggtagatgatgaagccgatctggaaggcacgcgtcagctcgctgagcgtgaagctgggcaccagcaccatgaagtcgtcgtcccgcaattgttcggcgcgcgccttcggccagatgttggaggccgacttcaggaagaactggcgctcgcgttcgtgcgtgtgcttctgcaggaactccttcacgggcaccttggcggcgtcgatcaccgccatgatgtcgcccatgctttcgcccttgatgccgaagttgcggttgcgcagggtgtcgccaatgtccatgccgaccggcgccatgatgtagaccgtcaggatgatcgcgatgccgttcagcaccatgttcggcggcgtctgctgcaggcccagcgcggtgcgcagcaggccgaacacgatgaccagcttggtgtagctcgtcaccatcagcgccgcgaaggtcgcgaagccgaacgcgaccatcaccgcgacgagtgtgagaggctccggtattccgccttgcatggggagcccgctcagacttcgccgggagcgaactccgacacgcgcacgcccaggcggtcgcccacggcgaccaggtagcccttgcccagcacgttgccgtgcgccaggatgcgcaccgggctgcggttgagcggttcggccaggtcgaacacgtggccggcacggatgctcttcagctcgccgagcgacagcgacagctcgcccacctcgaagcgcagcgtcacctccagcgcatcgagccggtcgatcggcaggttgacgttgtctgcggcgggcgcaggatcggcgggcgtatctggcttcatggcactgtctctcgattgctgaacggtgatgcgcgagccctcggcaacggccgagagatgtatcccactggggcctcccaactcggcggtaacgacgatcgcggcacccgaagaactccattgctcgatgccgacgatgtcgccggggcggatgctgctgatctcgcgaagctggatcggcgtgctgccgagccggaagctcaccggcatgcgcaatgcgtggaaggcctcgctcgttcgcacggcatggcgaggtccggtggccgcgggcacgagggcgtcgagcgtggcggcatcgtcgaactgcacgcagccgcgcagcatcgcgccaccgtccgatggcgtggcaacgaagaaggccgcgcgctcggggtcgcaatgcatgagcggctgttcgcgctgttcgcgccactcgcgggtgtcgcgggtgtcgtggccatcacgcgcggagcgcgcctcggccgccgaaggttgccattcgaaatgcaggcgcagcgctttctcgagcgcgtcgatcaccgggtgaagcgcgtcggccaggaggatgtagcgcaggtcgcgcggcagcaggtcgatgcggcgctcgccgagcagcgcctgcatgctcggcgcatccatggcgagatggccgatgtgcgcgccaagcttgaagctgtagctctcgcgggtggtgtgggcaaaggcttcgtcgtgctgccacgcgagccggtagctcacgcccttggccgccacgccgtgccaaggcgccgccgcatggaggcggttgagcgcacgcacattcgctgcatcggcgcgaggcaaggtgcgagcctcgccgagctcggtcaccgcttcagcaggcccggtccgcatgcatgctttcgttcgaacaacttctgcgtcttgtcactatctacgtactttcaagcaacgcgaacaccttcgcatcgggtcggcgcagcttagcgaaaggggcagggcgcaggtagtacgcaaaagcgtagtgccgcgcacgccacaggtccttcgtacttacgagaactcgtggttgccgtggacggagggcggcgcttagagtccaccgcgacgtgaggttcttcacgctcgatgtgcgtcgcgatgcgatgcgcatccaacaaaaactccaagagtttcaatagagcaaggacgcaatggcgagtccctcgcgatcattccaaccgtaccgcggcagctttcgcgacctgctgggcaatgccggccgctacaacgatctgctgctcgcgggcctgctcgtggtggtggtggcgttgttcgtgctgccgctgcccacgccgctgctcgaccttctgattgcgagcaacctggccatcagcctggtgctgttgatcgtcgcgatgtacgtgccttcggcgctgtcgctgtcgacctttccgtcgctgcttctgttcaccaccttgttccggcttgcgctcaacatcgcgtcgaccaagctgatcctgctgcaagccaatgccggccacatcatcgagaccttcggcaagctgatcgtcggcaacaacgtggtggtgggcggcgtggtgtttctcatcatcgccatcgtgcagttcattgtgattgccaagggctcggagcgcgtggccgaggtggcggcgcgcttcgcgctcgatgccatgcccggcaagcagatgagcatcgatgccgacgtgcgcgccggcgtgctttcttccgccaaggcgcagaagcagcgccgcttgctggagcaggagtgccagctgcacggtgcgatggacggcgcgatgaagttcgtgaaaggcgatgccattgccagcatcgtgatcgcgctggtcaacattcttgcgggcatggccatcggcacgctgatgcacgacatgaccctgggcggtgcgctgcagcgctacgccatcctcacggtgggcgacggcatggtgtcgcagatcccgtcgctgctggtgtcgattgcggcgggcatcgtcatcacgcgcgtgagcaccggcgaccgccgcgattcgcagctcgcgcagcagatcggcgagcagatgatggcgcatccgcgcgcgctcatcatcgcgggcctcgcggtggccagcttcctcatcgttcccggttttccgaaatgggtgttcggcctgctggctgccctcctgatcggactgggccttgcaatgcgcatgctgcgccggcaacgcaacacgccgggctggatctcccacggcgacggcgtggcgtccgaagagaccgacaccgaccacgccattgccgcgccgctggcggtgcgcctgtcttcgggcctgcgcagttcggtcgaccgcttcgtgctcgatcagcacctgtcgctggtcaagaactcggtcgaatccgacctcgggccgatctttccgcggctgcagctgaactacgcagagggcatggccgacaacgagtaccaggtgctggtgcacgacgtggcggtggcccgcggcatgctcaaacccgggtggctgctgctcgacccggcgcaggcggtctcgaccccgccgggcgcggaagtcgccgagcctttcggccccttcgcgcgggttgtctgggtgccggacccggagcccggcatgacggcgtggaccggtgcgcaagtggtgagcctgcatgtcgaccacaccgtgcgccgccacgtgaaggacctgatcggcctgcaggaagtgcagcgcctcttgcattcggtgcagcgcgatgcgcccgagcttgctgccgaggtgctgcgcgtggcctcggcgcagcgcattgccgaggtgctgcgccggcttctgcaggaaggcattccgattcgcaacctgcacgccatcttcgagagcctgaccatgtgggccgccaaggagcaggacggcattgcgctgaccgagctggtgcgcatccatctcgggcgctacatcacgagccgctatgtcggcgcgaaccgccagctcgaggcgatcctgttcgagtccagcctgctcgaccgcgtgcagaacgccattgagcgttcgccgcgcggcaacctgctgctcttgagcccggccgtcacgcaggacatccgcgagcagctgcgccgcattctgggatccacggccaaccgcgtggtggccatcgcgtcgtcggacgtgcgccgctacatcaagaacctgatcgaaccggtggcaccgcacatggcggtgctgtcctaccaggaaatagacgacgacgtggccctgcaacccgtgggctggatcaccaatccccaagcgcattgatgaacgacaacaacgacctgtttcccgagggagccgaagcccaccatgacaccgcagaacattctggacatcacgcgcgagggcctgctgctcgtgctgtggatctcgctgccggtggtggtggtggccacgctgtcgtcgctcatcgtggcggtgctgcaggccgtgacgcaggtgcaggaccagagcatcggccagtcggtgcggctcatcgcggtgatggtggcgatcatcgtcacggccggctggctggggcgcgacgtgatgcgcttcgcggagcgcgccttcctgtcgctgacaacgctctcatgactgccgcgatgcggatcgttgcgcgccttgttctcgtccgccggcaggccttcatgatgcttggcggcgcagtgctcatgctgctgcttgtgcagcacagtctggctgcggagttccgctggcagaacaggcctttccagatcgtcgccaacgagaagccgcttggcgacttcctgcgcgaactggcctcctcgcagggcatcacggcggtgatcgatcccaaggtcaacggcgtcatcagcggcaagttcgacgggcccgcgaagaacatcctgaacagcgtgtgcgcggtcaacgggctcacctggtatttcgacggtgcctttctgttcatagacctggccgccgatgcgaagagcgaggtgctgccgatcgcggcggagaacgccgggcgcattgccgagacgctggtgcggctgcacatctccgacgagcgctatccgctcagcatcagcgagcgcgacgccagcgtctacgtgaccggcccgcgtcgctatgtggagatggtgcgccaggcggtgaagctcgcggaccagaagacggcgatggccgagggtgccgaaatccgcctgttcccgctcaagtacgcctgggcctccgacttccgcatcaaccggtcgggcaaggagacggtgatcccgggcgtggccaacgtgctgcgcagcctgtacggccgcaacggcagccagtcctccagcggcggtgggggcgggcgcggaaccggcgggcccctctcggtggggccgaaccggcagatcaagctgcgcagcggcgagaccatcaacgcacccaagatcgacattgccggcgcgggcttgggcggcgatgcggccacgctgggcggcatgtcgagcatcgtcggcaacgagctgccgcagttccaggccgacacgcgcatgaacgccgtgctggtgcgcgacatgcccgacaagatggcgcaatacgcgcggctgatcgaatcgatggacacgcgcccgcggctggtggagatcgaggtgaccatcatggacatcagctccgacacgctcagcagcctgggcgtcgactggcgcctgcacgggcggcacgccgacttccagaccggccgcggcgaccgcgggccgctgacctggggcggcaccggcagcgaagccggccagatcgggagcttcgacaccacgggcaatccgctcaccccgctgggcggcatgttcaccgcggccatcggcaacagcgcgcgcaactacctgctcgcccgcgtgacggcgctggccaccaacggcagcgccaacttcgtggcccgccccaaggtcatgacgctggacaacaccgaggcggtgctggagaacctgagcgagttctacgtgcgcgtggacggcttccaggacgcgggcctgttcagcatcaccgccggtaccgcggtgcgcgtgacgccgcttatcatcgaagagaaggccgggcgcggcgtgatgatgtcgatcgacatcgtcgatggcgacctgagcccgcaatccgtcgacaagattccgatcgtgcgccgccgcacggtcaacacgcaggcgctggtcgacgagggcgcgagcctgctgatcgccggctactcgtcggaagagaagagcaatgcgatcaccggcgttccgctgctgaaggacattcccggcgtgggcggactcttcaggtacaccgacaagaagcaggccaacatggagcgcttctatctgctgacgccgcgcctcgtgacgccaggctccacggcctcggtgccgatgctgcccctgcccgagcccggaggttgacgatgaatggcgaagttccgttcgacgacgacgcccgtgccgagccggcggccccgcaaggcgcgcaggccacaggctggtgcctgcgcttcctgagcggcgcggtgaagggccgcaccatcgtgctcaagcccggcatcaacgtgctgggctcgggcggcgaatgcgaggtgatgctgccgggcggcgatgtgctgccgcgccacctcgcgttcaccgtcggcgagctggtggtgtcgatgcagcgcctgggcaccgcctcggcgcgcctcaacggcgaggagatgcagcagccgcgcaagagcgtggtggccggcgacatcgtgagcgtcggccagatcgactttcagctcgaccgcacctatcccgccagtgcgcaggaagaccgcatgttcgcgccggtgcacggcgcactgtccgaaggcgaggcgctggcgcagcagccgggcgcgggggcgcagcggctgggcctgtgggtgggcggcgtggtggcgctcctggccgtgctcgggctcgcggccatggcgctggtcggcgatggcggcgccgcgatgaacggcggcagcgtgaacctggcagaagtggaaaaggcgctcgtgccattccccgaggtcgaggtgatcgcggcgccgggcggacagttcggcgtcaaggggtacgtggaatcgaagcagcgccgcaagacgctggaagacgccatggcgcgcttcggcagcaaggtcagcgtcaacgtgcattcggccgaggacatggtcgagcaggcgcgccgctatgtcgacgatcccggcgtggccgtgacctacaccgggcagggccggctggcgctgaccggcacggtggaagacgcggccgtgcggcagaagatccgccgcctcagcgaagacctgcatccctcggtgctggtttccgacaaggtgcagtaccgcgagaaacccaaggccgagaccaaggacgacgacatgcgcgcccagtgggacagctggcagagcgtgctgccggcccgcatggtgagcatcaccgaagacggcgagggcctgcgccacatccagctctcgaacggcaaccgctactacgagggttcggtgctgcgctccggcgccgaactgaagcgcatcgacgccgacgggctggtcctgagcggcggcgtgcccaacaagaaacccgcgaggtgaaggacatgttttccttcatcccgcgccccccgatttcatgcgcagatgcaccgcggtgcgccgcatggaatggcttcgccgaatggcggagcgccttcatccgcaacggaaaaaaacctcaacctttgacaggagtttcaccatgagcgcagtcgacacctcgatccagcaaatgcagcaagccgcggccgaccaggctcgcctgatgagcgtcagcatggctgcgggcgccaccatctcgggcgcagccgccacgacgcagacggtgaacggcgccaacgccgccggcaccgaagtggcgaagtccaccggcaacgacatccgccagtccgccaagcagaactgacggtgaggcccgcgcggagccgcgaggcttcgcgcggccctttttcttttccgaggagagtgaaacatgaccgatcccattgcgtcggctgccgttggcgcaccgccaccggaagccgcggcctccgcctcatcacaggctgcgcagcagtccaccgccagcccgtcgcgcttcgagccgggcgagacgcacatgttcgccaacatgatgcagggcgtgcaggcaccgggcggaacggccgcgcccagcgcgataggcgacgccgccaagtcgctggccgcgcagttgtcgggcaacgtgcgctccatcgaggacatgcgcaagagcatgctcgagtccatcgatttcgcagaccccatcaagaccatgttcgtgatgaccgaccacgccatggaagccaacatgatgtttgcgcgaatgcatatttccaccgggctggccagcgccgcgaccagcctgttcggcagcctgctgaagaaccagcaatgaagacactcccacgcccgcgctggctggccgcgctcgtgctgttgctggcattggccggttgcaaggtcgcgctttattccaacctcaaggagcaggaggccaacgagatcgtcgcggccctgtcggctgaaggcatcggcgcggccaagaccaagctcgaaggcagcaactggcaggtcgaggtcgaggaagaccggctgagccaggcgctggacgtgctgcgggtgcagggcctgccggccgagcgctacgtcagcatgggcgaggtgttccagaagcagggcctggtgtccacgccttcggaggaacgcatgcgctacatctatgccatgtcgcaggagttgtcgcagaccttgcgcaacgtcgacggcgtggtgtccgcacgggtgcacgtggtcatcccggccaacgatccgctcagcgagaagatccggccttcgtccgcggcggtgttcatcaagcaccgtcccgatgtggacctgcgcctgctggcaccggccgtgaaagacatggtggcgcacagcatcgaaggcctcacgcacgaccaggtctcgctgtcgctgttcgaggcgcgccgcaccaccggcgccgcggccgcgggccatgcggccggcgcgcccatggtgctgggcattctgtcgacgcagaccgccatggtgctgctgggcctgctgttgctggccgccgtctgcctcatggtgctgcccacgctgctgcggcgccaaggccaggactggcgcacctggatgcggcgccaggtgctcaacaagcgctgagcgcacgcccatgcccggatcgaccgcagcgccgcaacccgttgttccagccatgcccggcccgatggacctggtgcgcctggtgatgcgcttcaacctgcatcccgaagccgacctgcatccgagctggctgccgccggattggccggcgcggcaccggtcggtggcgcgcatggggcccgccggccgcgccgtgctggccgagctgctgcgccggcggcaggccccggaacccgtgcaatcgcgcaccgtggccgactacaacttcgactcgcggctcaagcgcctcgcgctgctcgacgccgcctcgctgcgccgtctctcggcgtacttgggcttctgcgcgcacctgccgcttttcaggctgcgcggcggtgccggcctggagatccgccgccaggcgcgccgtttcgaccgcgacgccgtcgacttcgtgctcgaccgcgtgccccagctcaccgaactgcgcatggacggcaccgtgctccagcagcgccccctggccacgggccgcgtggtgctcgaccgcggctaccgcctgctgctgggcgccgccgcgtccgaaggggcgctcgtgcagggtcgcctgaagcacaagctgccgcgccgcatctccgccctgagcgtgccggccttggagccgcgccaggcctcgcaactcaatgaactgatgctctcctgcatcgttcccgaaagactgccgcaatgggactggcttttctgatcaccaccgacaacctgcagctgctgagcgagcgcaaggtactgaaggagaacgaatacgcggcgctgctcgatgcggcggcggtggtggacaccgcacgccgggaggcgcaccgcatcacccggcaggcacttcaggatgccgaagccagccgccgccagggctatgaagagggactggagcgcgccaaggccgagtacgcgcggcaactggtgtccgagaccattgccgccgagcggcaactgcattcgctgcgcagcgcaatggcgcagatcgtggtcaaggccgtgggaaagttcattgccaacgcccggcccgaagcgttgttcgaagccgcattgctgcgcgtcgatacgctgatccgcagcgaacccttcatcagcgtgcgcgtggcgcccgcgcaggaagctgccatgcgcgaggtgctctcccggctgcgcgacgaagcgcagtggaacatgacggtcagcgtcgtcgccgacccggcgctgcctgtcggcgcctgcgtggtgcagaccgcttcgggcacgctcgagctcggcgtcgatgcgcaactcgaagccttccggcgtgcggtcgaacgcggcggcacggccgacggcgcggaggcaaggcggtgagcatgcccggatccatcacccccgatgcggcgctgggcatcgtcgccgacctggagcaagtcttcggccgcgtgatgccggtgggcatgcgcgggcgcgtgagcaaggcggtcggcatgctgatcgacgccaccggcatccaggcccacgtgggcgagctgtgcgagctggtcacgcccggcgagccgccgctgctggccgaagtggtgggctttcgcggcaacacggccatcctcacgccgatgggcccgatcaccggcatctcggcgctgaccgaggtggtgcccaccggccgcggccacgcatgcccggtcggtgcaaacctgctgggccgcgtgctcgacgcactgggccagcccatcgacgatctcggcccgcttgccacgcacacgcgcctgccggtgcaccgcgagccggtgagcccattggcgcggcgcatgatcgacgcgccgctggccaccggcatccgcgccgtcgacacgctgctgacactgggcgaaggccagcgcatcggcgtgttcgcgccgcccggcgtgggcaagagcaccttgctcggcatgctggcgcgcggctcgacggccgaggtgaacgtgatcgcgctgatcggcgagcgcggacgcgaggtgaaggagttcatcgagcacaacctcggcccagagggactggccaggaccgtgatggtggtctccacctccgaccggccgccgatggagcgcatcaagtcggcctatgcggcaaccaccatcgccgagcactttcgcgatcaaggcaagaaggtgctgctgctggtcgattcgctcacgcgctttgcgcgcgcgcagcgcgagatcggcctcgcgagcggcgagccgccgacgcggcgcagctatccgccgtcgatcttctcgatgctgccgcagctgctggagcgggcggggcagggcaagaccggctccatcaccgcggtgtactcggtgctcaccgaaggcgacgaagagaacgacccgatcgccgaagaagtgcgctccattctcgacgggcacatcgtgctgtcgcgcaagatcgcggcagccaaccgctacccggccatcgacgtgctggccagcatcagccgcgtgatgccgctggtggcttcgcgcgagcactgcgcggcggccgcgcactttcgcagcctgctggccaagtaccaggagatggagctgctggtgcagatcggcgaatacaggccgggcaccgatgcgctggccgacgaggcgatacgggcgcggcccgcgatgctcgacttcctgtcgcagccgccgaagaccagcctgcctttcgagcaatcgctggcagcgttgctgcgcggcgcaccgcgaacggagcacgccggatgagcagcgactggaagctcctggccgacgtgcgcgagcggcagaagaccgtcgccatgggcgtggttgcgcgcgaccgcgcggccgccgaggagagccaggcccgactgaggcaggccgaggccttgcggcagcagcaagtgcagaacaagctgcagcactgggaggccacccggggtgcgctgtcgggcggccggttcagcgtggcggagttccggcatgcgggcgcatggagcggtgcgctcgatgcgcagatcgcagaggccggcgaggccgcggcgcaggccgggcgggcacacaccgagcgcgaacaggtgctggagcaaagccggcgccagctgcgcgccgcccacggcgaggtcgagaaggcccgccagatgcagcagcgcgcgcgcgccgagcacctgcacctgcaggagctgcggatcgaagacacgaatgaagagagcaccgcgcaggcctgggccatgcgccggccggcctaagtgtggagcattcgatggaaagcttcgaactcggtcacatggagcagtttttctcggcggtggtgctcacgctgccgaggctgttcgcgatcttcgcggtggtgcctttcctgtcgggcggcatgatcaccggtaccgtgcgcaacggcatcctgctgatgctcgcgatcttcatgtcgccggtggcgggcgaggtgccggccgcatcgatggccacctgggtgttcattgccggcaaggaggcgctgatcggcgtgttgctcggcctgggcttcggcatcttcatctgggccatccagagcgtgggcgacctgatcgacttccagaccggttccagcaacgcctctttcttcgacccggtggcggggcacgagaacggcgcgaccagcgaattcctgggctggatggtcatcacgctcttcgtgtcggccggcggcctgctcgcgatgctcggcgtgatcgtcgactcctaccgcatctggccggtcggctccttctttcccaacctgggcctggtgctcgagcagttcgcgatccgccagggcgacacgctgtttctctggatcgtgaagctggcctcgcccgtcatcgtggtgctgctgctggtggaactgggcgtgggcctggtgggccgggtggcgccgcagctcaacgtgttcgtgtttgcgcagcccctcaagagcctgctggcgcatttgatgatgctgctgttcctgttcttcgtgtacgagtcgctgcaggatttcctgcggcccgagaacggcgtgctcgatttcctgcggtccaccctgtagcggcgaagcatggcagagaaagaccaggaccccaccgccaagcgcctgcgcgatgcgcgcaagcgcggcgaggtggtgttcagcaccgacgtggcctcgaccgtggtgttcgtggtggtcgtggtgtccctgtggctgggcgggcaactcatctacaacctgctgcgcgaactgtggctgcatgcgaccagcaccaccttgctgacggcgcccgacgaccgttttgccgaactgctgctgcacaccggcgagacgctggtgtggggcacgctgccgatcatggccattgccgccgcggcgggcatcgtgggctcgctgttccaggtggggggcgtcgcggcctgggagcgcctgaagcccgacgtgaaccgcatgaacccggccgagggcctggcgcgcatcttctcgacgcgcagcctcatcaaccttctgaagatgtgcaccaagaccgcgttgcttgccgtgctgatgttcgtggtggtgcgcggcttcgtcgacacggcgctcaagctgggctatgcgcggcccgaggggatcatgacggccgcggcgcacatggtgctggttgccttcggctgggcggtggtgatctacgtcgtgatggccatggtcgactacgcgcacgagcaccacgagttcatgaagcagcaccggatgtccatcgaggagatccgccaggaacacaaagagatggagggcgaccccatcaatcgctcgcgccgccgctcggcccatttcgaggcggtgtacgcgagcctcaacgaccgggtgcgcgcggcgtcggcggtgatccattcgccgcgcgtggccgtcgccctgcaatacctcggcgagaccgacctgccgcgcgtgatcgcgcgcggcgagggcgaggtcgccgcacagatccggcgcttcgcgagcgaaggattgataccgaccgaattcgagcccgcgctggccgagcgcatctacgacgaagtgcccgaagaccagccgatcccgcgcgcgctgtatgcgccggtggccaagctgctgcgctgggcgcagggcagcgaatgaatctcgagaaaccgacgatcgaaaggaaccagccatgttgattgccgatggtggaggcagcgtacgcgtgccggtgaacgtacccaaccccgtgaacacggcgcagcagcctgcgagttcggccgagtcggacgccgcggcccgcgcacgggagttgcagcgccagctggaagagctgctcgcaaagatccaggaggcacagcggcaggccgaagaggcccgcgagcgcgccatcaaggcgcagcgcaaggcccaggaggccaaggaccatgccctggccatggaggtgcaggcgcaaaaatccaaggacctggccgacgccaacaaggccaggaaggcgcagcaggacgccgggctcgaagacgcacgcgccaaggccgcgagcgcggaagccaacctgaacgacaaggacctgacgctgctcaaggccaagatcgaccagaagaaggaacagcagaaaagccccgaagccaaggcctccgcggacaccgacgagaaagtgaagagcgcccagaccgaccgcgacggtgcacagaagaccaacgaactttcgaagctctctctcgacgcgcaggagaaggagagcaaggcgcaggacgccgaggccaaggtcgtcgagttgacgcccacgccgggtcgcccgtcggccaccatcaccgacaaggagcgcacggcgctcgacaaggccgaggaaaaggccaagacactgcgcggcgaggcggacgccgcgacgaagaagttcggcagcgagatcggcgaagaggcgaacaccgagttctggggcaatccgcccgcgccgacaggcaccgaggggccgcccgcgccggccgccgacgatccgctgcaaacgccgctcacgcaactgctgcaggtctcgccgaaggccaccaccaacccggccgccagcaacggactgctgttcaccccgacgctgaccgttggcaacacgggaaccaccagcggcagcctgctcgtgccgccgtccaccttgtcgtccggcaccggcacgaacgcgacgtcgccattcaacaccttcctcaagtcgccagagccggtcgtcacgccgcaggtgaagaagacgctgacggacattgcggacggaaagagcgtggagcagatcgcgagcgaccgcaagatgcgcgtcgaccaggtgatgtccgaggccaacgcggcgggcgtcaagatcaccacggccgcgccgaaggacggcgtgcaggccaccaccatccagcgcggcgacgcctcgctgacctacagccgcgacgcgaagcaggacaccctttcggtcaagggcagcatcaccgacccgaaggcacccggcggtcagaaggccatcgacgcgaaggaagacggcagcgggcgctacagccagacgacgaaggacgccaagaccggcgacacgaccaccacaaccctcgacagcagcgccggcacgcgcaccgtgagcgtggtcgacgagaacggcctgcgcaccgacaccaccacgtcgctgaccggcgcagaggtcacgcgcccggtgggcgactacgagggctaccgggaggtcgccaaggccgccgacctgacgctcgagcagctgctggcactgaaccccgacgtggactacggcaagccgctcaagcccggccaggagatggtcgtgacgggcgtgcccacgaccgtgaagaccttcggcaaggatggctcggcactcgagaagaccaccgcgagcgacggcacgctgcaggtggtggccacgagcgcggacggccggcgcacggtgctgatgggtgagcccgatgccaggaacggcccgggcgaagcggcgcgcaagtcgatcttcgacgacaagaaatccgtggcggataccgcgaagaaactcggcatgaccgaagccgaagtgctcgcggccctgcccgagggcacggtcgacgtgagagagcccaccaccgacaacggcgacgtcgagatacgcacgctgtacgacccgggcaccaaccgcgtggtggtcgagacgacggactggcagcacggcgacgtgagccgcaaggatatcggcgagaaggcgaagttcaccgtcacgcagaaggaccccaagaccgaaaagtccgagaaggtcgaggtcgaagggggcgtcggctacctgcagaacgaggccgagaacaaggcggcccaggccgatggctatggccgcgagatcagcgacctggacaaggacatccgactctacaagcgcatgggcgagccggtgaccgacctggtcgagcagcgcaaacagctggtgtcacagcagaaggacgcacagggcgaagccaagatcgccgaaagcaaggccaccgcggccttcaccaggcgccagcaggtgttggtcgacgaagacgcgcgcgtggcctaccagaacctggcctatgcgcggcccggcagcaaggaccagtcgaaggcagccaaggtgctggacgaccagctcgagcggctggaccacatcgaccggctcgtcgatgcggccgacaaggaggtggacctggccaaggccgatctcgacaaggcccagaagcaggacgacaaggcgcaggccgacgccgacctgcagacggagttccagaaatggaagcgcacctggctctggaacggcctcgacgagaaggagatccagaagcgcgaggccgagggcgcaacgcccgtcgggcactcgtaccgcaacgacgaggaggaaaacaaggcggcgtggaaggccttcgtccagcagcaggaaatgatggacgagcatggcgacaaatacctcaccgatgcggggcggcccgcgcgcgacgcctggctgaaccgcaacaaggccagcgacgcggcgctggattccggcatccgctacgacaaggcctcgatcgcgagcgccacggccaatggccacgtggccaaaggcgaggtcgaccggttgcagtacaaaaaggatctgtgggtcgatgccaacccgaactcgttcaaggagagctttgcacagcaggacaagctcgacaacgccaccgacaggcttgccaagagcaagatcggcgtcctgctggacgacgggcacaagaagtacaccgagttccttgcgaagtcgcccgtgtccgaacgcgaggacccggaagggctcaagaagctgcagcagcagtacaacaacgacaacgaggaatctgcagaaaagatcagccagcagatccaggatctgaagctggggcgcacgggccagcaggcgaagtctgcggaggccttcatcgcacagtgggcggcgcgaaaccccgaactgcaaaggcagatcgaagccttcgacgcgcgtcccatccccggcagcgtgcgcgccgccgaggcccgcatgcaggagaaggaagaccttctcgcgtcgtccgagcaggggcagcagctgcagaaggcgaaaagcatcaagatcagggccgagaatgaactgacccagctcagctgggacgacgaagagcgggtgcagaatgactacgacacgtccaagaaagcgcaagaaggccacacctggctgcgcgacatcttcgacgattccgccgacgagtcgctcgactacacgaaggaccagctcgatgcggtgaagcggctcaaggacaagctggcctcgggagagatctcgctcacggagtacgtggatcaggaagacgagctcatggacgcctatgggctcaaggccgtcgaccttacccgcgaggccagggagaacgacgaatactggagcgtggtggacgaagccgcgcgcataggcacctcgacgctcgcgggcatcggcgccaccatcctctcgggcggcaacgtggcggcgggcatcgccgtcggcttcgccgtcagcgagctctgggacacgacgggcgacgtggtggccgcggcccagggccgcaacatccaggccgacggccacacttccttgttcacgttcggctacaaggcggccacgggggacgtcacctgggacgacgccaagttcatgttcaaggacgaagtggtcgacctcgcctcggccgccgtcacgccgaccggcgtgggcgcaggcatgcgcaccagcgcggccctgaccgcgaagttcgcggccaaggagggcgtgcagctcggcgccaacaccacgctcaagttcaccaaccgggtggctatcggcacgcgcgccggtttgaaatcgcaggtcgtcgacggggtcggccgcgtgggcgtggacaccctgcatgtcggcctcgacggccagctcgcctcggaggagggtaacaggcgcatcggggcggccatcgtcagctcggccgcaggtttgctgaccgcgccgatcaccggggggatctcgggtgctgcgccgttgccgaacgccatgaaaggcatggccgcaaaggcgaagttcggtggcgcggtaaccgcgcagtttgcgaacgacgccgccggcagctggggcaccggccatctgatttcgctgaccaacaacggccgcttgatgaacgacgccgaaaccaccgcggcgtggatccaggcgttcccgggtacggtgaacaacatcgcgctgcatccgcacatggcgcgcaagatggcagcagcagcggcggcggcggcggagcagaagcaacaacagcagcagaacgcaggcaatcctgcgaatgtggtcgctgcagcgaatgctgccaacgtgggggacgcgggcagtcctgcggtcccggtggccggtgacccgcaggcgcatgtgccgcaggtgcatgcgccgcaaaaccctggcggcggcactggcgttgcgccgcgcccgatcaacgtcaagacggatcatctcccgggtcttgcaggccgtgacgtcgaccacctcgtggtggtgaacgcgagctcccgggatcttgcgacagggctcggcacacacacccgtgccgccgaggcgctcgcgccgggcggcgtggtcgagttccgcgtggcgctggacacgcagaaggtcgtcgcctcggccgcggacccgaaggcgccgggcagcggcggcaaggtcaaggccggcaaggacggcgccgacgaaggcggcgtgacgcgcaagggcgacgaggcgcaacagcagaaggagcaccaggcagcgcaggacaacgccattcgcgtgcggctgcgcggcgtgggcctggagaacgtcaggatcacacgcaacgcgaatcccggcgcgggccggcccgagatcgtcgtgcaggcaagcaggccggcgatggcccgcgcgcccgagagcgtcttcgcgaagcccgcctacgacggctacgaccagcgcatgtcctacctgcgcggtgacgaaatggtgggcatctacggcgcgggcacgcggcccgaccccgtcgcgctcgaggctgcgcgcaacgaggcgcgcgccgcccggcgcgacatgcgcgtcggcctgacggtgcgcaaccgcctgaacgtgaacgaagcccagccctggctcgcttcgcccacgatgcaatcggtgagcaccggcatcggcacgcgcaccaactttcgcgagatcgcccggggcgcctacgacagcttccagctgcgctccacggcgccgttgaagaacgcgctgggcaaggagctgtcggtcgcggtgcggcccgacgaataccggcgcaccagcatgctgcaatggggtgtgctgccgttttcgcgcgacaccatcttcaccgtgttcgcgaaagacctgatcggcatcgcgaagaaggagatgttcggcgagggaacaccaggctatggcgtgaacatgcgctcggccaaggtcgtcgggccggctgccgacggctcgggccaggtggtggaggtgacgctcagcgtcaagctcgacggcgagcacgtcacgctggccgaaggccagaaggacttcctgggcggcaaggccggcaacacgccgggcgaccatgtgaaggtgtcgagcagcctgctgttcgaccgcgtgatcgaggatcgccggttcgcaccgttcattcccgcgctgaagaagatcacgggctacaacggcgtgttctcggcgtcggtggagcggcgctggcagatgctgctgaaggacgtgatcggcaaggacgacatcgtgcccgcgcgcttcttcgagcagttccagaagactttcgccgatgcgaagtacaagatgcaggtcgtggtgccgcacgcggacgccgcgaaactgtacgacgcgacggcgatcgatgtgcgcgacttcgtcgccgggccgaacgtgcgggccctcaaggacctggtcgccaaaggccatgtggaccccgcgaaggcgctggtcttcgttcccgagcgcggcggcaaccatcaccgcaccgcggtgccgggcaaaccggtgcagaacgagctcgtcgacctgaccggcaagctgcggcgggtgccgcacgaatcgaccagcaacgtctgggtgatctttgccgacaacaagctggagcgcggcttcgagcgcgggatgtaccgggtcaagagcttcgcctacaacatgctgcccgaatcggcgcagcgctcgcagccttcgccgcaccacgtggcgggccgcggcaacctgatcgacggaatgacgggtggccggggccggcccgactccaacggatcgctgcggctcaccgccgtgtttccggtgcccagggtcttccatgcgggcctgctcgcgggcagcaccgagttccgcctgcagatgggcgtggacgcgccgggcgtctccaggtcggtggcaaaggggggcacgagcagcgtcagggtctcgccggacggcacggccgcggtggatgtgccgaactggttcccgcgcctgctcgaacagtcgctcaccggctcgacgccgctcgtgccgacgggcggcacgaagcagctgggcaagttcttcgacgatctgcaaacggttctcggccccgagcagcgtgccaccgtggccgcgctgcgcgaaaagcacacgggcggcgacaagccgacgatcggcgatgcgaagttcctgcgcgccgacgtggcgcaggacatcgtggacgtgctgacgggcctgcagcccggcaatggacgcaaaccccaggcgctggtggcggggcagcggcccgacgaggcggtgcccgcgaggtccgcggccgcgacgcgtccctcggggctgcgccgcgcggacctgaactacgtcgacggcgaggtcacagtcaaggggcggccggtgcaggccagcgacatcgagctcgccgtgccggcggacagcatcctgatcatcgcgaacagggccaacccgccgagtgccgagcgcatcgcggcggacgtgcgcgccgcgggacaccccgaaggcaaggacgtggtgatcttcctctgcgacgcaggaacgccggcgcggcccgatgcgccggtgcccgcatcgctggcacgggacgtgagcaacaagctcggcgcgcgcgtgcatgcggtggatggcgacgtggtgctgggcgagcaagtcgcactcggcggcagcgccgtcacgcagcggccgaacctgccgctgaccgatgtgtcgcagaacgcgccgcaccgcacggccgatgcgaacctcgacgcgcagaagcgcttctggctcgagccgggcggccgcacgcaggaggctgaggcgccgttcgcgcagaacgtgctcgacaagggcgcgtgggtgggcgacaagaccatcgatccgctgcacctgggcatcgaagagcgtgcggtcgagctggtgcccttcgatgcgcagcatgcgcgcgacgtgctgccttacctggcgaaggagttgaagtacagccccgactacatgcggctcaaggccgacggcatgacggaaaaatgggtcgcagaaatcgaggccggcacgcgcatggccttcgtgatctatcccgcgcccggctccgcggcgcagcgccggccgctcggcatcattgccgtgcacaaggaaccgctgatcggcgacaactacattggcacgcgcgattccgccgactacaagggcgaggcgccggcgggccggctggggaggcaggagctgctcgaccgtggcgaagtgtggcagttctccacctacctcagcgccgaccgtgcttcatcccggaaccgcaagtcgccgttccccggcggggtggtcaactcggccgcgaagaagcaggtgatggatctggcggtggcggagctgacacgccggggcgaacctatcgacgccttctatgcgcgcgtgcatgccggcgcgcccgaggccgtgcccgcactcggctggccggagaccgtcaacgccaagagcctcgtcagccaggagcgcatggccggcggcggaccgctggccgtggtgcacgagaagggcccgcacgcaccgggtgaaacagcgccgacgcgctatgtcgccatcttcgaaacgccggtgagccgctatgccgaagacggtcccggcacggcggcataccgctcgctgatcgatacccagatcggcaatgacccgcgctcgcaccgatggctcgggccacaggagtggcaaggccagccgctggtgcatcgcccggccgacctcaactacctggagggcaatgccacggtgaacggccgcccggtgccggtgcgcgacgtcgaggtggcggtgccggagaaagctttcctcgtgatggccgacgaggcgaatgtgccgagccccgcgcgcatggccgccgacatgcgcgcggccggctatgccgacgggcaggaggtggcgctctacatctgccgcgccggcgagatggcgaacccggccgcgccggtacccgagtctctcgcattgcagctcggcgacaagctgggcgcacgcgtgcatgccgtggaaggcaccatcaagctgggcgagaagatagaactcggcgaaggcgacttcgtcagcgcccagccgaagctgccgctgatggacgtctcgaccggccgcccccacgccaacgagaacttcgacgcgcagaagcgctactggctcgcacccaacggccggggcgaacgcgtcgacgcgccgcttggcgccgatgtgcgcaacatgggcgcgcgggtcggcgacaactggatcgacccgttcgtgctgggcatcgaggacagggtggtgcggctggagcagttcagcgaccgcaatgcgtccacggtgctgccgtcgctgaaaaagcagctggccgtcagtcccgacttcaagaatctcgggccggaaggcatggcgcgcaagtggcagcaggaaatggaggacgggacccggatggcctatgtcgtctatccggccgaaggctcgccgctgggccagaagccgctcggcattatcgcggtgcatcgcgaggcgctggtcgacggcaagtatgtgaagacgctgcccgcgtcttactaccgcgacggcaagtttcccgcgggcgaggtgtcgcgcgaagagctggttgcgcgcggcgatgtctggcagttttcgacctatctcaacgccgatgcgaagcaggtgccgggcaccaacaaggccggcaagatgctgaccatcgaggaggccgccgccgagggcaagcggcgaggggaagaggtcctggccttctacgcacgcgtgcacggcggtggcccgctcgtgctgatggagccgcacgtcaacgccaacacaagtttgttcggccaggagtcgatggcacgccgaggccccattgccgtgggcctggagcagggctcgccagtgaccggcggtgccgaccgctacgtgctgatcttcgagacggatcgcgggttgtacctgccggacggcgccggcaggaagaagtggaccgccgatatccagaacctgatcgacagccatccggatccggcctcgtggctcggtgcggcccaggacaccggagcgtccggcccggcagcgagcaacgccgcgagccgagatgcgaccgcgaacgtgaccccggggcggggcgcatcggcaatcgatccggacagcgtcgcccgccagacctatgacgccctggcgaacgagttgggcctgaccgccacgcaggccgacgccatgcgcggctggaccgtggcgcatcgcgatgcggtgaccgggttctacgatgcccggctgtccagcctgaaggccgacaccgtcgcgcgcgcgcaagcgcacgtcgcgcagagcggcgacgaggcgcactacgtgtcggcggacatcggcaacctgggcgggctgaatgcggcgatgaacaatgtggcggaggccgccaacgttcacttccgcggacttgccgagatcctctccacgcgtctgggcgcgaccgatgccacggtggtgccgatgcgcaccggcggcgacgaactcggcgtggtggtcgtgggcatcgacgaacccacgctcgcaaatgccgtcgaggcgacgcagcggcaggtttcacgctacgcggaagaccacggcctggccgacattccgcatcccaagcacgaagaccaggccggcgtcggcctgcacatcgggtatacatcggtatcgcccgacaagaccctggaccacatctttaccgaggccgaccaaggcgtcgacaggagcaagcagcatgtcacaacagacaagggacgaacggctgggactgaccggcctgagcccggagcaacgaaagcaacgcctgcagcaactgcagcaggaagtggacgaggagcgccagcgcgcgaagaccgcgctggaggcccagcgcgcggcgcgccggaatcaggccaacccgaagtcctgacgccggcccatccgacacgcttcgcaacgggctcgcacgatcacgcgaggatcgatccggacgcggtcaggctgcaggagttttccgatgcggcccgcgccgccggcctcgacacgcggcagttcacaggcctgctgcactacgcgaatgctgccaaggacagcgtgacgggcttctatgacgcgcgtcaatccggcgtgaaggccgataccgtgctccggctgcaggacctggtggccagttcggacgacaacggcttctacgtatcggctgacatcgcgaatcttggcggcctcaaccacgcgatgggcaacgtggccgaacacgccaacgttcatttcaaggccatggccacgctgttcgcggatgaactggcggccaccggcgccaccgtcgttccgctgcgaaccggcggcgacgaactgtctgctgcagtcgtgggccagatcgacgaagcggggctgcgtgccgcgctcggtgcggccgaccagcgcattgcgcgctatgcgcaagagcaggggctggccgacattccgcaccccaagcgcaagggcgagaaaggcgtcggcatgcacatgggctatgccgaggccatgcccggccgaacgctggaccgcatcttcaccgaggcggacatgggcgtggatgcgagcaagaatgcggcgcggcatcccaggatcgatttcgaggatgggcagcccgtggcgctgaggacgagtgacggagaccaaatctcggcccaccggttgacgatgatcgagtccgacggcacgcggcggccgatgaccggggccgaggtggtcgccatgatggggccgcagatcggcgtgggcgggaacggcactgtgtacgagttcggcactggccaggcgatcaagatcctgcgcaccgacagcgatatccgtgacggtcgcttcagcatggctctggacgagttgcaagtcgatctgccggacggcgcgacgatccacagcagcatgaagcgggcggtcgaggaggtggcggccttgcggaaactggccgatgccgcgggcgcggagaacgtgatcgacgtcaaggggccttacctggtgggcaaccgcctcgtcacggtgatgccccgctacgaagagtcgagcacggcgatgagggccaccgccacccgcacgcttacgggaccgggcaccgatcttctcaacgaacgcaccgcgacgggggttgcggcgatctcggagggtcttcatcgtgccgggaaggacccttgggatccgcagttcatggtcgactcgacggggcggccggttctgcatgaccctgccggggtccatgaagggttgactccctccgatttattcaacaacgtggtcacgcggatggcgcgcaccggccggcaaaacgccgcgcttcgcgccgcacccgaaactgcggacaaggcgttgttcgcgctggggccggcgcccgacgaagtgggccggatgggcgggttgaagttgcccgccggttccggcgaaacaccgggcggcctgtaccccacggtggcggcggccaagtgggcggctatgcgcgatgtgccgccgcccgatggcagcccggcgaagccggtgccgcacatctacaccgtggatgcgggcatggcgcgcgatgcgctggcggcgcgcccggcgccggacggcacgcgcgccattcccggcgacgcgctgattgccgcgcgcacgatcgacaggttcggcaggttcgcggcgtcgacggacatgcgtccgggagcgccgatcgatatcgactgggaaggccggcccgtcacgatgagggacgcggacaccggcgccgagttgcccgtgcgtcgcttgatggtccgcgaagcggatgggactcggcgaccgatgacgggggccgaggtggtcgccatgacggggcaagacatgctcggccgcggcagctccgccgatgtgtacccgttcggcgaagggcaggtgatcaagatcttccgccaaactcgcgcgcccgatccggaccaatcacatctgctggtggacttgcccgacggcgcaacgcttcatccccgcatggccgcggcggtaggagaagtggccgcggtgcgggagcttcgcgaagcggctggtgggtcggggttcgtcgacgtcaaggggcctttcctggtgggcgaccgcctggccctggtcatgccgcggcacccgttcgcgggcaagaggctggaactggacctggagatgcggacctattccggcgagggcagcgagctgctcaacgaacgcaccgcgcgcaccgcaggcgtccttactgatcggctgaatgctgcggacaagttccctggcgacccacagcacctggtcgagcaagacggttcggtgaccggcttcgatccgctggaggtttccagtggggagctggcgcagaactatcacgagggccaggcgctgaagctggctcgcacggggcgccacaacgccgcgcaacgcccggcgccagagacgccgaatgccggcaaggtgcagttcgtggtcgggtcgtcgcccgaacgcgtgatcgcagcaggcgggctggagataccggcccccgatggcgtgcacaccacggtggccggcgccaagtgggccgcgatcgaacccatgccggccccatttgatcgcgacggaagcgaggaagccgcctacgtctacaccaccgaccgtgacagcgtgcaggttgccgcggatgggatgcatgcgattcccctggaagccattctttcggggcgccaagtggacgcgttcggccgcttcgttcccgatcagaccgtgcgtttccgtgccaccggcggcaccgtcggcaggcagatccccgaagggctcatcgatctgagcaagctcgggcagagaaaggacggcccggaccggggcgcgagcacctaggccgaggtgacggaggagtccggcgccgccgcctgcgccagcacccagtccctgaacacccgcatgccccgcgtctcgcgccgtcccttcggcgcgcagacgtagtagccgcgcggcgtcagcgcggcctggtcgatcgggatcgcgatgcgccccgcggcgagctcgtcctcgatcaggcagcgctgcaccacagcgaggccgaggcccgagatcacgccctgcaccagcatcacgacctggtcgaagtcggcggcggggcgtgggtttgcgtcgggtacgccttgcgtgtcgaaccacaggcgccagttgtcggggtagttggcgtgaaacagcagtgggcgctgcaacaggtcttgcggctggcgcaatgcgagcgggccgcgcaggtcttcgggccggcagatcggcacgatctcgcggcccacgagatagtcggactggatgtcggccgaatgccacggcgcgctgccggtgcgcacgcggatccagccgtcgatgtcaggcttgtccagtgcatcgtcgcggcgatagggcgcgaacgaaatggccacctcgggatggcgcttgcgaaaatcgggcagccgcggaatcagccacttggtggccagcgttggcggtaccgagaggcgcagcgtgtgcggtccgtgtggcgcaccggcggcttcggcggcggcctcgagttgccgcagcgcaggtcccacgttgtccaggtaggcgcggcccgcgtcggtcaatgtgctgagccggccatgccgatccagcaggcgcacacccaactcttcttcgagccgcgccaccgcgcggctcaccgcgccctgcgtgacgcacagttcgtcggctgctttggagaagctgcccagacgcgcggtgctggcaaaagcgtgcaactcgtgcagagacggtgaacggatgcgcatgggtggagtgggtggcccgctatgagcgggagtcatagcaagcggcgcaattgtcaccccaaacatgcggggacgattcacataatcgccgcactccagggcaccttgcccgtgtgttgtctccctgttatttctttcgacttaatcgcaatgaacaaccgccgcgaactcctgctggccatcagcgccgttgctttcgggctaccgctcgctgctgccgatgcccgcgcttcgacctatccggacaagccggtcaagctgatcgtgccgttttcgcccggcggttcgaccgacctcgtcgcgcggctcctggccgagaagatgtctgtcatcctcgggcagcaggtggtggtcgacaaccgcgcgggagcgggtggcaccatcggcatttcggcggtggcgcgggccgagccggacggctacacgatcggcatggccaccgtgagcacgcatggcgccaacccggccgtctacaccaagctgagctacgacccggtgaaggactttcagccgatcaccaacgtgatgtcggtgcccagcgtgttcgtggtcaaccccaagctgccggctaaaagcatgaaggagttcatcgcactggccaagtccgagcccggcaagatcaccttcgcgtcgcccggcaacggctcgctcggacatgtgaacgtcgagcagttcatggaccttgcgggcatccggctcacgcacgtgccgtacaagggcgcgggccaggcggcggccgatgcgctggccggcacggtcgacgccatgaccgacaacctgccgtcgtcgctgccgcacatcaagtcgggcaagctgcgcgcactggcggtgctgtcgccgcaacgctcgccactgctgcccgatgtgccgacctaccgcgagctcggcttcgaagccatgagcgagggtggctggttcggcctggtcgcgcctgccggtacgccgcctgccgtggtcgagaagctgatggccagcgcgcaccaggccatgcaggaccccgctttcaagcagcgcacggtcgacatctcgggcgtgccgatggccaatacaccggcacagttcgcgcagcagatccgcgaaatgatggacaaatacgcgcgcatcgccaaggtggcgaacatcaagctgtgagcgcgcgcagcatggagagcagcgatccggccgtcgttgtcgccgatccgccgcccggcgtggcccggctgccgctggtgtgcgattcgccgcacagcggcacgcggtacccggcggactttgtcacccgcgttccgttcgcgcagctgcgccaggccgaggacacccacgtcgacacgctctgggccgccgcgccgagacacggcgccacgttgctggccgcacagtttccgcgcgcctacatcgaccccaaccgggccatcgacgacctggaccccgaactgctcgatggaccatggccgctgccgctgaacccgggcgagaaatctcgcctgggctacggcctggtctggagccgcatcgcggccgacgagcccttgtacgaccggccgctgcagaccgccgcggtgcagtcgcgcatcgagaaatactggaagccctatcacgtggcgctgttcgccgcggtcaagcgcgcggtaaccgacttcggcgccctgtggcacctcaacctgcactcgatgcccggcaacgcctacgagaagctgcgcatccaatcgacccgtccgcttgcggacttcgtgcttggcgaccgcgaagggaccacctgcggccccgagctgctggaggtggtggaagccaccgtgcgagcccacggctatacggtggcgcgcaacgatccgtacaagggcgtggcactgatcgccgaaatcggcaaccccgccaggaagcgccacagcctgcagatcgaaatccgccggccgctgtacatgaacgaagcaacgcgcgaaccgaacgatggattcgctgcgctgcagcgctgcatcgaagccaccatcggcgcggtggcggcgcacgtgcagttgcagttgaggagggagtagccggcaatgccgcagcgccgataccttctacccggcaatgccgttcctggccgagggcggctgcagggcgtcgaatgccgaaagcctgcggtagtcgccgggcaacaccgcataggtgccaagaaaggtcttgtgcagatggctctggtcggtgaagccggcggcatgcgccgcgtaggtgacgcgcgcgccgccggcaatgaggtcgcgtgcgtattcgatgcggtggcccaccaccatttcgtgcggtgtgaatcccatcgcgcccttgaagcgccgctgcacgtgtaccggatgcaggcccgccgcatcggccaggctgtccagcgtcatgcgctgatgaaagccggacgcgatcagttcatacagcctgttcatccggtcgtcgccgctgtcgacaacgcgcgcgggcggcgcgcgcaacggaatccaccgggccaggcgttggcgcagcagggcgcggcccacggcgttgtcttcttcattgcccaggcccgtgctcgtgggttcatacaggagccgatggcactcgataaaatcgaaggcctcggatgcgtcgagaaaaaccgagacgcctgcatcgtcttccacgcgggccaaccgtgtgctctcgtgcgccgcgctgatgcagcgggcgacggcggagctgcagtacatcgcgtcctcgcgccacggaacgccgcatgctcgcaccgagtgccagacctgcggcgcgatacgcagcagggcgcccggcggtaccaccgtcacgcggttgcaggtacgcacgtgcagttcggtgttggacaccgagagcgtgaatccgacgtgcctgtgcggccggatctcgtgatgcagcagcatgttggcggtcagttgaagacctgtgagatcagcatctcgccagtagcgggaagccaggagttccatcgaaaagcagggctccctgaacgtcttggttttgttgaaaaagagcaatcggcatgccagccctcggcctgcctccgcgggcattcacccgaaggtattcagttgcgcgccagcgcgagatgccatcgcccgccggcgccggcgaatgtgctcgaggctaagaatttacaaggcggcattgccgcgctttggtagtttggctccaaccccgcagcgtccaccgatgcatgcggcacttccatcaggcctctcatgattgttggtactttcttgcaacacgccggagcgatagcgctgccggatccgcgcgaattcgattcaccgccgccgtcgaatgcatatggaaacggcgccgagccaccgctcgaagggccgtttccacagctctattcggaagaccagctctacctgccgcaatcggcggaccggcgtgcggacggcgtgcccggcatcgtcggcgatctgctgaatgcttcaggcagcaaggagtgccgtgatcttgtccaggcgatgttgaatgcgctgggcttcgattggcttggctacggcacgatcactttcctgcgcggccgctggtggcccttgagcttcttcaccgcgcacgcaaaccccgagtggacgcagcgctacttttcgcatcgcctctacgaaactgatttgcggcagccgggcgtaccggcttccagtctcccgctggtgtgggacatcgagcagatcgaggcctcgccattgtccgcagctacatccgtgaccgaggacgcggagggacggcggcagcgctttatcgacgacctgcgcgccagcggcattcgcagcgggttgatgttccgcctcgcgctgccgacgcaggtgaaccagtacaccgtcatcagcctgcagtcgagcgagccgggccgccgctggatcaccgacgaggtcgtcggccaggccctgacgctgggcttgagcgttcacgagtacctgctgcgccattcgcgcatgccgagcgaagcgagcgcggcggcgcgcatcgagatctcgcccacgcagcagtacatcctccagcacctgctgcaggggcgcagcgacaaggagatcgccaaccgcctcgacatgtcggcccacaccgtggactaccacatgcgccagttgcgccgccgctttgccgcgcgcaaccgcgtgcagctggtcaacgcggtgcagcagggcgacagcgactttggtgtgcacaacgagagctaaggcagcacggccaccgggctgcgctcggcgaactgcccgttccagtacgggtagtaggggtagggcggggtcacggcgctggcggcatcgagccgcttgacctgatctgcgctgagttgccagccgagcgcgccgaggttctgcttcagttgctcttcgttgcgcgcgccgatcagcacgctcgacacggtgggccgctgcagcagccagttgagcgcgatctgcggcagcgtcttgccggtttcctcggccacctggtccatggcatcgatcacgcggtacaggcgctcgtcatccacgggcggcgcgaagccggcggtttcgtgcagccggcttccggcgggcagcggctggccgcggcgcaccttgccggtcaggcggccccagcccagcgggctccatacgatggcgcccacgccttggtccatgcccagtggcatcagttcgaattcgtagtcacggccgatcagcgagtagtaggtctggttggccacgaagcgctgcagcccgagccggtcggaggccgcgagcgacttcatcagctgccagcccgagaagttggacgcgccgatgagccgcaccttaccggcgcgcaccaggtcatcgagcgtgtcgagcaccatctcgaccggggtcatcgcatcgaaggcatgcagctgcaggatgtcgatgtagtcggtgcccaggcgcttcagcgcggcgtcggtcgcggcgatcaggtggtggcgggaggcgccgacgtcgttcggcccgtcgccggcgcgcagcgccagcttggtcgagatgatggccttgtcgcgccggcccttgagcgccgcaccaaggatcgattccgaagcgccgttcgaatacacgtcggccgtatcgaacagggtcacgccggcattcagcgccaggtcgacgatgctgcgtgcgccttcgacgtcggtgttgccccaggcgctgaagagcgggccctgcccgccgaaggtgccggcgccgaagccgagggcggggaccttgaagccggagcggccgagaaagcgttgttccatgatgttgtccttgtcgtcaatgaaagaggtggaggctcaggcttgcactgaggcgcaatcggccggggaggcgcgcccttcgcgccggtcgagcgaacggctccagagtgcgatggccagccccgcgagcgtgagcagcgccgccacccagccgagtgcgcgcaggcccgggccatggtcgatgaccacgccgcccgcccacgcgccgagcgcattgccgaggttgaaggccgcgatgttgaggctcgacgccaggttctggcccgcgccggaagccttctccagcacgcgcagctgcatcggtgccacggtcgcgaaagacgcgatgccgagcaggccgacgaacaccacggcggtgaacggcgttccgatggtgaactgcatcgcgccgagcacggcggcgagcgccaccagcgtgccgagcaccgcgggcatggtcgacttgtcggccagcctgccgccaagaatgttgcccacggccaggccgccgccgaacaccagcaggatcggcgacacggccgactccggcaagccggtgacctgcgtcagcaggggctggatgtaggtgaacaccacgaacacgcctgcaaagccgagcaccgtcatcgccaagccgagcagcacctgcggccgtgcgagcaccgcgagctcgtcgcgcagcggcgcggccttggcctcggcccggacgcgcggcacgaacagtgcgagcaccgcaaaagccagcacgccgatcagcgtcaccgcccagaaggtggcgcgccagccgtactgcagcccgagccaggcgccggccggcacgcccagcagcgtggcagcggtgagcccggtgaacatgatcgcgatggccgacgcgcggcgttccggtgccacgaggcccgtggccacgaccgaacccacgccgaagaaggtgccgtgcgcgagcgaggtgatcacgcgcgcggccatcagcagctcgtagttgggcgcgagcgcgcaggccaggttgccgagcgtgaagatcgccatcagcgcgagcagcacggtcttgcgcggcagcttgcgggtggcgatggtgagcagcggcgccccgaccgcgaccccgagcgcatagcccgagatcagcaggccggccgccgtgatggagaccttgagatccatcgagacctgcatcagcaggcccatgatgacgaattcggtggtgcctattccgaaggcaccggcggtgagggcgagtagagcgattggcatgatggctctactgtgcgggttattttcaatgatgactagaatgccgcatggatatggacttgtgagttgaattcacaataaaaggcacaaggaaccgacatgccacgcatcgacgtcaaccgctccggcgaaatggaagcctttgtgcaggtggtcgagtccggcggcttttccgctgcggcgcgcctgctggacatgacgccttcggcggtcagcaagctggtcgcgcgcctcgagctgcggctgggcatccagctggtgcaccgctccacgcgcaagctgcagctcacgccagagggcctgcacttctacgaacgcagcacgcgcgtgctggccgacatggatgaggcggagcgctgcgccgccgcgggtgctgcgccgcgggggcgcgtgagcatcaatgcgagcgtgtccttcgggcatcacaagctggtgccgctggtgccgcgcctcctggagctgcacccacagatcacgctcgacattgcgctgaccgaccgcgtcgtcgatttgatggacgagcgcgccgacatcgccatccgatggggccagctgccttcgtccgacctggtggcgcggcgcctgggcgaaaccagccaggccatcgtggcctcgcccgactaccttgccaagtacggcacgccgcatacgccgcaggaactggaggcgcacaaccgcctgggctggagctaccggcgcagcgcgcccgactggccgttgcgcgtggaggggcgaatgatctctctgcccgtggccgggccggtgcgcgcggccgacggcgaaaccctgcggcagctggccattgcgggtgcgggtgtggcgcggctgtcgctgtatcacatccagcacgacatcgatgcggggcggctcgtgccgctgctcgaagaattcaaccccggcgaggtggagccgattcacgccgtgtacatcggcaaggccggtaccttgccggcgcgcgtgcgcgcggtgctcgactttctggtggcgtgctcgggcgtgggaggagggcgctacacgatcaagcgcacggcgccgatgccggcaaattccgcggtcacctgatcgccgcggcggcagggcagcacgccgacccacgagccggtggtcacgaccgtgccggccggcgcggtctggccgtggcgtgtgacgtggcgcagccagatgggcagcagccacgccggatcggccagcggatgggtgccttcgcgcaccacggtttccgcattgccgaccttcgtttcgcagcgctgcgaagcccagtcgacggccgcatagggctgccattcgccaagaaccagcgcgccgtgcacctgcgagtcggccagccgaagcaatgcgggcgtggcagccaggtcttgccagcgcgaatcgacgatctctaccgagaccgccatcgcgtcgatcagcgaagccgcatcgttgtggtcaagcttcgcggccgtggcgggtgtcacgtccttgccgagccgcagcgcaatttcggcctcgatgccgggcgcgtgaaacgccaggtcgtcgaaattggccgagctctggcgaacgccagccgggggcaacggcgcatgcgtgagcgtcacgtctcgggagccgccgccggatttccagcagcccgggacagtgccgccttgaaaccagccgagcgcggtcgccacggcgtcctgcacttcgtaggcctgagttgcgtcctgcagcgcgtcggtccagagcgcggcgtcgagggtgcgattgctgcggcgcgctgcgatcagcgcgtcggctagggctgtgatggagggggtcatttttgggattttgtcagttgccgtttttcggggtgcgtgcaaaggacaccgggtactcccctccgcgaatgtcccccgccttcggctcctcctttatttcgctgcggggagcacccggcgccctgtgcaccagggcacgctgctggtgtaccgccgatcaacaaccgctctgaataacgatcccgtcgatggggtgccttgcgcagcgaaataaaggaggaggccgcaggccgggggacatccgcggagcaaggcaccccgtcggcgggagcgccgccctgaacaacactgaccagcaaaggcgcggcgtcaagtttcaacgtgcaccttgccgtccttcaccaccttcgcccacttggcaatttcagtcgagatgaactgcctgaacttgtcctgcgaaccaccaccgtcctcggcgccgtaggtatcgagacgctcctgcacatcgggcatcgcaagcaccgcgttgacgtcgcgattcaccttctcggcaatgcccgcgggcagcttgcccggccctgcaaggccgtaccaggtggtggcctcgaagcccgcaaagccctgctcctgcatcgtgggtacgttggggtggcccttggcgcgcttggtgcgcgtttgcgccacggccagcacgcggccgctcttcacgtgcggcgtggccgcggtcatggtctcgaagctgtactggatctggccacccatcaggtcggccaagagcgggccactgcccttgtacggtacatgcattgcatcgacgccggcttgcagcttgaacatttccagcgccaggtgctgcgccgagcccgcgcccgcggagccgaagctcaccgtgccgggcgaagccttgcaggccgccacgatgtctttcaccgtgaccgccttttgcgccgggctggcgatcaggaggttgggcgtgacgcccaccagcacgatcggcacgaagtcgcgctccacgctgtagcgcagcttgggctgcaggctgggtgcgagcgcgtggctgttgatgtgcgccatgagcagcgtgctgccgtcgctgggctgctgcgacacatactcggccgccagcacgcccgccacgccgcccttgttctcgacgatgacctgctggttccacatcgtcgtgagcttctgggccaccacacgcgccagcgcatcggtgcccccgccgggtggaaagcccaccacgatgcgcaccggccccgaaggccactcctgcgcgaagagccggggcacgcccagcgtggcggctgcggcgcctgcggcttgaatcagcgaacgtctctgcatcatctttgtctccagtgtggtggatccgatgcgtgccggaccgacaagtccggcaaggtgacggccgccgcgccgttcgagcgacgcgctgcggccggtgtcgagtaggtccgtgtgctacgcggccttctgcagtgccgcggatgcggcgtggcttgcgaaatggtccatggccgcgtgcacgccgctgcctgccagcttgatgccggagagcttcatgcccatttccacacccgccaccatggccaccagcgtcaggtcgttgctgtcgcccaggtgccccatgcggaacatgcggcccttgagcttgccgaggccggtgcccagcgagaggtcgaagcgctggtggatgaggcggcgcagcgcatcggcatcgacgccttcaggcgtgatcacgccggtgagcacgggcgagtacacggccgggtcggcgcactggatcggcaggccccaggcattgaccgcggcgcgcacgccggcggcccagcgcaggtggcgcgcaaagacgttgtccaggccctcgccgagcaacatgtcgagcgactccgacaggccgtagagcaggttggtgttgggcgtgtacggccagtagccgtccttgttcatctccacgatctcgtcccaggcccagaacgcacgcggcagcgtcgcgctcttggaggcttcgagcgcgcgcggcgagagcgcgttgaagctgatgcccggcggcagcatcaggcccttctgcgagccgctgatggtgacgtccacgccccattcgtcgtgccggaaatcggcgctcgcgaggcccgagatgctgtcgaccatcagcagcgcggggtggcccgccgcatcgatggcgcggcgcaccgaggcgatgtccgaggtgacgccggtggaggtttcgttgtgcaccacgcacacggcctggatcttcttttcggtgtctttgcgcaggcgcgcctcgatgaggtcggcctgcacgccgcggcgccagctgggcgcggcgggcagctgctcgtccttgccggaccaggcgaggaattcggtggtgaggccgaggcgcgtggccatcttctgccacagcgatgcgaagtggccggtctcgtacatcagcacgtggtcgcctgggctgagcgtgttggcgagcgcagcctcccatgcgcccgtgccggaagcgggatagatcgcaaccggatgacgggtcttgaagatctgcttgatgccgccgagcaccttgagccccagcgtgccgaactccggcccgcggtggtcgatggtcggcaggctcatggcccgcaggatgcggtcgggcaccgggctcgggccgggaatctgcaggaagtggcggccggtgggatggatgtcgagttgaagcatggactgtcctttcgctttcagttttgcattcaaaaatgaaatgagcatgatggtttaccctggtattcggggattgttgatgcaggtttttgcattcaaaatgcattcaagggaaacagagacatgactgcagaaatcatcgaaatctcgcgccttgcgctgcatgaccaagtggccgcgcgcctgcgcacgatgctggtcgaagggcacattgccccgggcgccaagctcaacgaacgggagttgtgccttcagctgcgcgtgtcgcgcacgccgctgcgcgaggccatcaagctgctcgcggccgaagggctggtcgacctgctgcccaaccgcggcgcggtggcggtgaagctcaccgaggccgacgtggtcgacaccttcgaggtgctggccatgctcgaaggcatgtcgggcgaactggcggccaagcgcatcaccgacgaagaactggccgaggtgcgcgcgctgcactacgaaatgatggcctgcttcacgcggcgcgatctctcgggctactaccgcctcaacgcgcgcattcacaccgccatcaacgaggccgcgggcaatccggtgctgtccagcacctaccgctcgatcaatgcgcgcgtgcagtcgctgcgctttcgcaccaaccaggacgaggccaagtggaagcacgcggtcgaagagcacgagcagatgatccaggcgctggccgcgcgcgacgcgccggccatgcgcaaggtgctggtcgcgcacctgatacgcaagcgggacaccgtgctggcactgcttcaggccggcgaaatctatccccaagcccacaaggcgagctgagcccacacaccatgcgcgtcgatcccgccagccacatccagcccgccggaactgttcttccgcccaacgacacctgcgaggcgctggcgcggcggctgcgcgcggaaacgcaaggcgaggtgctgttcgacgacggctcgcgcgggcgctacgccaccgatgcatcgatctaccagatcacgccggtgggcgctttcgtgcccaccaacgatggcgacattgccaccgccatcgacattgcgcgcgacctgaaggtgccggtgctcgcgcgcggcggcggcaccagccagtgcggccagaccacgggcgccgcgctggtgatcgacaacagcaagcatttccgccgcgtgctcgacgtgaatctggaggagggcaccgccaccgtcgagcccggcctggtgctcgaccacctgaacgcgcaactcaagccgcacggcctctggtttccggtcgacgtgtcgaccagcgcgcaggccacgctgggcggcatggcgggcaacaactcttgcggctcgcgctccattgcctacggcaacatggtgcacaacgtgctgggtgcgagtgcctggctctcgagcggagagctggtggcgttcggtccgcaggccacgctggacgcgcgtgcggccggcatcgcgaagttcgtgcacgggctcgcgctggcgcatcgcgagcagatccatgccaactggcccaaggtgctgcgccgcgtggccggctacaacctcgacatcttcgacaaccagagcgagaagccgtacaccgccgacggcagcgtgaacctcgcgcacctcctggtcggggccgaaggcacgctggcctacacccggagcctcacgctcaagctcgcgccgctgccgcgcgccaaggtgctgggcatcgtgaactttccgaccttccattcggccatggacgcggcgcagcacatcgtgaagctcggccccacggcggtggaactggtcgaccgcacgatgatcgagctgagccttgccaacccggccttcaagccgaccgtggaaactgcgctgatcggcaagccggcagccatcctgctggtcgagtttgccggcgccgacaaggccgcactgctgccgcagctgaagcaactggtcgagctgatgggcgatctcggcctgcccggcagcgtggtcgaaatgcccgacgacgggcgccagaagaacctgtgggaggtgcgcaaggccggcctcaacatcatgatgagcctgaagggcgacggcaagccggtgagcttcatcgaagattgcgccgtgccgctcgagcacctggccgaatacaccgatgcgctgaccgaggtgttcgcccgatacggcagccgcggcacctggtatgcgcatgcctcggtcggcacgctgcatgtgcggccgattctcgacatgcgcgcggacggcggcgccaagatgcgcgccatcgcggaagaagcctcggcactggtgcgcaagtacaagggcgccttcagcggcgagcacggcgacggcctgtgccgcggcgaatggatcgaatggcagttcggcccggccatcaacaaggcgtttcgcgccatcaagcagaagctcgatccggccaacctgttcaaccccggcaagatcgtcgatacgccgcgcatggacgacgcctcgctgttccgttttgcgccgcccacggcacccaggccctaccggcgcatcgaactcaagcccgtgctcgactggtccgcctggaacgtcaacgccgaccccgtcacggagcagaccaccgccccgggcaccggcggcgacagcaccggcggcctcgccaaggccgtggagatgtgcaacaacaatggccactgccgcaagttcgacgccggcaccatgtgcccgagctaccgcgtgacgcgcgatgagcagcacttgacgcgcgggcgtgccaacacgctgcggctcgcgctctccggccagctcggagccgatgccttcaccggcgaagaaatgcacgagaccatggacctgtgcgtcggctgcaagggctgcaagcgcgactgcccgaccggcgtcgacatggcgaagatgaagatcgagtttctcgaccactacaagaagcgccatggccacacgctcaaggacaagctggtggcctacatgcccgactatgcgcacagggcgagccgcgtgtcgtggctcatgaacctgcgcaacaccttgcccggcgcggcatggctgggcgaaaagctgctggggttttccgcacggcggtctctgcccgaatggcgctcggacaccttctggcgtgccaaggccgacatgcatggcatgttcgcaagccgcgagggggtgctttcggtgcaggccagcggcggcaaggccgcggtgcttttcgtcgacaccttcaacggcaccttcgaaagcgagaacgcgctggcggcggcccgcgtgctcaaggccgcgggctacacgctgcacacggtcgagaaaagcggcggccaccattgctgtggccgcaccttcctggccagcggcatggtggacgaggccaagcgccgcgccgaggcgctgatcgatgcgctccggcccctggccgaggccggcgttcccatcgtcgggctcgagccctcgtgcctgctcacgctgcgcgacgagaccctggtgatgggcttcggcaagaaggccgagtccgtggccaggcaggccctgctgttcgaggagttcattgcgcgcgagctgaaagccggccgcttcaagctcgcgctcacgccggccacggcgccgatcctgctgcatggccactgccaccagaaagcctttggcgccgtcagcccggtgctggacgtgctgcggctcattcccggtgccgagcccgagctgatcgaaagctcctgctgcggcatggcgggcagcttcggctacgaggcgcgccacatcgacgtctcgatgcagatggccgaggccagcctgctgccggcgatccgcgccaggcccaatgccatcgtggtggccgacggcaccagctgccgccaccagatcggcgacggcgcgcagcgcgaggcggtgcacgtggccgtgctgctcgaacgccatcttgcgccgcagaccccgccgaccgaggagatttagcggctggcacacaatggcgcgatgaatgcagcaaccacggaggaatccggcttcgcgctgttcgacaccgccataggcacctgcgccttggcctggggtccgcgcgggctcatcggcgtgcaactgcccgaggacaacggcgaagccgccacgcgcgcccgcatgcgccgccgcttcgcagacctgtccgagtcggccccgcccgagagcgcacgtcaggcgatcgcggccatccagggcctgctgaacggcgcgtccgacgacctccaccacatcgtgctcgacatgagccgcgtgtcggaatttcaccagcgcatctatgcgattgcgcggcgcattccgcccggccagacgcgcacctatggcgacatcgcggccgagctcggcgacaaaggcttgtcgcgtgcggtgggccaagccatgggccacaaccccttcgcgcccgtggtgccatgccaccgcgtgctggccgcgggcaacaagcccggcggcttttcagccggcggcggcgcgctgacgaaactgcgcatgctcgacatcgaaggcgcccggccgaacgggatggcttcgcttttctaggctgcctgcggaatcgcagcgcgaggtgagcgcgctcggccccctcagcctgaatacggccccttgacttcgccccagccccatcgcggcatgggtgcctccgcgtccacggccgcgccaggctgcgagttgatgaccgcgagccgcgatccccactcgagatagccgaccagcgccgaacgaaactcgggatcgtccggcatcgcgagttcgtccgccgtttccagcagcagcccgacccagcggcgccgctgttcctgctgcaggtggcggttcaggtgctgccggatcatgtgcggatgcccaccgtgatgcttcgaatagtcggccgggccgcccagcacttcggccaggaaggcggcaacatgggccgggtgatcggcgtccatgtgggcgaagaccggtgccagcaatgcatcgcccttgacgttttcatagaagcgcgtcgtcaggcgaagcagcgcctcgctgccgccgagccattggtacagagtgggaacgctttgggaatcggtcatggctgtgacgacgcttgttcctgttgctgctgcgcgcgcatgatctggtgccgctgccaatagcggccgaccgcagccttgaagttttctttctgcttgccgatgccgcccaccttcaccttggtggtgcgcgaacccagcatgcccttgtcatggtgcgtgacgaccagcatgtcactgaaggcattgtcctggtacgtcaggttcttgacttcgtcccatccgatcgtcgagccgccatcgacgctctgatgcaggcccgtgtagctcacttcgacgctctcgtcgttcttcagcgcaaacgccaccggcggaaagtggcgcagcaccacggcgcgctcttcttcggtggccggctcgtagcggtaggcaaggctcagttcgtggttctggacgaagcgctgttcgtagtcgctccacagccgctgctcgatggcggcggcggtctcgatgtcgtcggcccacgaagcctccggcgcggtcgcgacgatggcgccataggcgctttcgggcacgtggtggcccacgttgcgcatgcgttcgagcagcggcggatgggtgtcgtagggatgcggcacgtcggcggtcttcatggtttcgatgaaggcctccgagttggcatagggcggcaggccggccgccacgaagccggcgatgcccagcgcaccgtcgtgctcctggttctgcgcaaagagttttctctcgacgtcgttgcggtagcttgcgtaggccgagatcttgatgagcgactgaacgatggcgccgggcgcggtgaggctcgcggaaacgcggtcggccttgtattcgcgctcgcggctgtcgcgcgccagggcaaaggcgaagatcattcggtacaggcgcagcaggtagtgcgcgacgatggtcaggccgccgctgcgcatcttccaggtgtactggtcgaactgctgcagcttggggccgagcgcggcgctgctgcgggtgtcgccgccacccaggtgggccagctcgtgcgccagcaccgcgtcggcttcggactggtcgagcacgcgcagcaatggaatgctgacgaacaacgtgcggccgtccagcgtgcgtccgcccacctgacagggcgcttcggtgacgaagaagttggtatcgatgccggcaacgatctggtcgggcggcgcggtcttcacgcgggtggcgagctggcggatgcgctcccacaggcgcggcgcatcggcctcggcgaccacttcgccttcgatctcgttgcccgagggcagcttcttgaacagcgtgtagatcgcatagaacaccgctgcggcggccgcgatgcccgcaatggcaataagcttgacgtagtagctctgccagaagtacgccgtgagccagaacgacagccacaccagcatcgcgctctgcagcacgacctcgaccgcgctcgacaccgtcatgagccgccagccggcgacaaagctggcgtagcgcaagccgcggttggcgaaggccagggcgcccagcaccagggccgccgcgagcagcgccgccccgagcgccagtgtccagagggcggcgcggtcggcccagtggaagtgccagtacatcgaattgggactgcacaccttgtcgtggaactccctgtcttcctcggcggtggcttcgcaggccttggagagcggatggctgcggtagaactcgctggtttgcgccttctcttcggccgacaggcgggtgtcggaagcgatgcgtttctcgattgcctgcaggaactccgcgtcttccgtgcgcagcacgtattccgtaaaaaccagcgtcgccgccggaatggcgaagagcgacaccagggtcaacagaaacacgcgtaaaaggtcggcatggatcgttcgggcgagggccatggggtgctgctcctggaagcggttgttgtgattcgttgtgtcggacagtccgggacaggcgatagcgtagcgaccgtttgcatgcttgcgaatctccgatggcgtccatgcgaaaggcgtgaataccaaggtcgtactctttgtgcagaattagcaacggccgcccggcgaccccacgccagcaccggatgccggccttcgcgacaatcggtccaatgcgttcttctccgttcttcaagggggccctgttgccgggcgccgaggcctcggcatccgaagacaccgccgccatgcagccggtcgacgggctcgagcccactgcgcgccgccgagcgatgctggtcatcatcctcggcatcatggtggccgtgctcgatggcaccatcgtgaacctggcgctgccgggcatcgcgcgcgagctgcaggccagcccgtcgcatgcgatctgggtggtcaacgcctaccagatcgccacattggtcatgctgctgccgctggcgtcgctgggcgacctggtgggttaccggcgcgtctacctggtgggcatggcggtgttcaccgtgtcgtcggtcggcgccacctttgccgattcgctcggcaccctgatcgtcgcgcgcaccttccagggcctgggcgcggccggcatcatgagcgtgaatgcggcgctggtgcggctgacctttccctcggcgctgctgggacgcggcatggccatcaactcgatggtggtggccacgtcgtcggtggcggggccgtcggtggcggcagccatcctctcggtggcttcgtggccgtggctcttcgcgatcaacgtgccgctcgggttgctcgtcttcacgctgggcatgaaggcgctgccgttcaaccgcttgccgcccgcggcggggctgcgcttctcaccggtcgacgtggcgctgaacgtgctgatgttctcgctggtgtttctcggcgtcgaccggctcggcgtgcgcgagggcggcgcgccatcgtcgtccgcctgggcgatcctgctggccggcgtggccgtgggcttcgtctacctgcagcggcaacgcaggctggcggtgccgctctttccgatcgacctgctgcgcattccggtgttcgcactgtcgatgggcacgtcggtggccgcgttctgcgcgcagatgctggcctatatcgcgctgccttttctgctgctcgaggtgtatggccgcagccacatcgaggccgggctgctcatcaccgcctggccactggccatcgtggccatggcgcccattgcgggacggctgatcgggcgctaccccgacgggctgctcggcggcatcgggctgggcctgctcgctgtcggcctggggttgctggccgcgctgccggcgcaaccgggcaatgccgacatcgcctggcgcatggcgctgtgcggcctcggattcgggctgttccagtcgcccaacaaccacaccatcgtgacctcgccgccggcgcaccgcagcggcgcggccagcggcatgctcggcaccgcgcggctcacggggcaaacgctgggagcggtggtgctggcgggcgttttcagcgtctggagcccgcacggcggccacgggccggtggtggcactggtgctggcggcctgttgcgcgggcgtggcggcggttttcagcagcctgcggctgaaaacggcggggccccacggctgaataggttagggtacggccccatgacggaagtacctgaaaccgtggtttgccctggctgcgatgcggtcttcagccgtgcgcccctgcagccgcgcgaggtgtcgcgctgcgcccgctgcggcaccgagctctaccgccatccgggcgaccagcaccgccgcatcctgccgctcaccgtggcgtgcctgatcatgttcgccattgccaacctgtttccgatcgtcgagatcgagctccagggcctgcgcagccagaccacgctggccggcgccgtggtggttctgagcacggagggcatgtcgatcgtggcgttgctggtgctggcgacgacgcttctttttccgctgctgcagctgtgcatcctggcctacctgctggttccgctccagcgcgagcaccggccggcaggctttgccattctggtgcgcgccatgcagatgctgcggccctggggaatgatcgaggtgttcctgctcggcgtgctggtggccatcgtgaagctgtcgagcatggccacggtggtggccgggccggcgctctgggccttcatggccttgacggtcatgctcaccgccgtgctctcgttcaatcccaatgccttctgggaaatgaccttccgcccgcccggcgagcccgaggaggagacggggtgatcggccccttccgcccggttgaagatgaccaagacgaagcgccggttgcaacggccgcctcgctcggcctcctggcctgtccgcattgcgatgccgtctggcgcgacgcgcaggagggcgaagcctgcggccgctgcggcacgcgcctgtacacgcgcaagccctacagcctgaaccgcacctgggcctttctcatcgcggcctgcatcatgtacataccggccaacctgctgccggtgatgatcacgcgcacgctgttcggcgcgcagtacgacaccatcctgagcggcgtgatctatttctgggtgtcgggcgcctacgggctcgcggccatcatcttcatcgcgagcttcctggtgcccctgttcaagctcacggtcttgatcctgcttgccttgctggcgcagcgcggcagcggctggcggcggcccgagcgggccaagctctatcacatcatcgagatcatcggccgctggtcgatgctcgacgtgttcgtggtgtcgctcctcgccgggctggtgcagatccagggttttgcggtcatcaacgcgggcgtgggcattgcggcattcggctcggtggtggtgctgaccatgctggcctcgctgagtttcgatccgcggctctcgtgggacagcaggcagcagcagcaagccgaacatgaacgtgaacgcgagcagccgctgctcgacaacagggaagaaaagccagcatgagtgacgaagaagccagacccgacgacaaaccggccccgacgggccttcctccgccgcgcgtggtacggcggcgcgaatggctgccctcgctgatctggctgattcccatcgtggccgcgctggtcggcgtgatgctgatcgtcaggattttgatggagcgcgggcccgagatcgtgctcaccttcgagaccgcggaggggctggaggccaacaagacggccgtcaagtacaaggacgtgcagatcggcacggtgcagagcctgcggcttgcgcgcgaccgctcgcacgtgcgcgtgcaggtgcagctcaacaaggaagccgagggcttcaccgccgaagactcgcgcttctgggtggtgcggccccggctcgacacctccggcatttccggcctgggcaccctgctgtcgggcgcctacattggcgccgatgccggtgtgtcgaaggaaaccgcgggcgagttcaaggggctggaggtgccgcccatcgtcacgcgcgatgcctcgggccagcagttcttgctgcgcgccaccgacatcggctcgctcgacgtcgggtcgccggtgtatttccggcgcatcaaggtcggccaggtggcggcctaccagctcgacggcgacggccgcggcgtgacgctgcgcgtcttcgtcaacgcgccgtacgacaagttcgtgggcgtcaacacgcgcttctggcaggccagcggcatcgatgcgcagttgagcgccagcggcttcacgctgcgcacgcaatcgctggccaccatcctgctcggcggcattgccttcaaggcgccggacgatgccatggggccgctcgccaaggagaacacggccttcacgctggccgaagacgagaccacggccatgaaggagcccgatggtccgccgcaaacgctgctgatgtacttcaaccagtcgctgcgcggcctctcgccgggtgcgccggtcgacttccgcggcgtggtgatcggcgaggtcaaatcgatcggcgtggagttcgaccgcgccgagcgcgagttccgcatgccggtgctggtgcaggtgtaccccgaccggctgcgccgccgcgcgggcgaatccggagaagagtcgcgtgccacgcagcaggagcgcctgcggttcctgaccgagaaggggctgcgcgcccagctgcgcaacggcaatctgctcaccggctccgtctatgttgcgctcgacttcttcccgaaggcgccgccggcgaagatcaacatggacaggaacccgatcgagctgcccaccgttgccaacagcctcgacgagatccagtcgcaggtgcaggaaattgcgagcaagctcaacaaggtgccttacgagcagattgcgggcgacctgcgcaccacgctcgccgcgctcaacaagacgctggccagcacggagcaggcggtgacccgcatcaacaccgacgtgacgcccgagctcaccgccgccatgaaggacgtgcgcaagaccgtcaacaacgccgaacgcacgctggccgacgattcgccgctacagcaggacatgcgccagacgctgcgggaactcacccgtgccgcgggttcggtgcgcgtgctgacggactatctcgaacgccatcccgagtcgctgctgcgcggcaaaccggacgacaagaaatgaagaagagaaaaccgttcctgctcgctgcagctgccgctgcagcagcgctgatcgttctggcaggctgcgcgagcaagcccgacaactactacacgctggcaagcacggtgccggctgcggaggcggcaccttcgaccatcggcagcgcggcgcccctgtacatcgagctggcaccggtggccgtgcccgagcggcttgcaaggccgcagatggtggtgggccgaccgaatggcggcgtacaggtcgacgtgctcgagcagcaccgctgggccgcgtcgttcgagaacgaattgcaggacgcgcttgccagcggcatcgcggcgcgccttggtgcgctcgacgtcaccaagggcggcaggcaaacggcgcagcccgtgtggcgcatcgcggtgcaggtgcgccagttcgatgcggtcgatggcggccgcgtggacgcgggcttcaactggacgctgcggcgctccgacgagacccgcacgatggcgtgccagctgaacgtgggcgagccggttgcaagcggcatcgatgcggtggcgcaaggcgcgcagcgcgtgaccgcggcagcggcggcggccatcgcgcgcagcgtggctgcggcgcgagcgaacgcggcagcgaccgcatgcacgccctgattctttctccctccccctctgggcgagggcaggggtgggggcacggcggcggtcacacaagcatggcgcccagttgaaggctgcccccatcccaaccttcccccagagggggaaggagcaaaacaggaatcgcatggatcggagatcaccatggcacagatcggaaaggcgccctgcgacgaaacgctgatcctgcatggcgcgaaggcacaggagggcgcctgcccggatgcctccaagccttgggtgctggccgcggccatcgtggggtcgagcatggccttcatcgacggcacggtcgtcaacgtggcgctgccggccattcaggccgacctgcgcgccacggcgttccaggcgcaatgggtggtcgagagttatgccttgctgctcgcggcgctgctgctggtgggcggcgcactcggcgacaatttcggccggcgccgcatattcgcgatcggcgtggggatcttcgccatcgcctcggtggcctgcggtctctcgagcaacgtgcagcagctgattgccgcgcgcgcggcgcagggcatcggcggggccttgctggtgcccggcagccttgcgctcatcagcgccgcatttcccgagaaggaacgcggcaaggccatcggcacctggtcgggcttcagcggtatcacggcggccgcggggccggtgctcggcggcttcctggtcgatcatttctcgtgggcgtgggcctttctcatcaacgtgccgatggcgctgctcgtgatgtggatcgtgtggcgccacgtgcccgaaagccatggctcgtcggccagcggcgggctcgactttttcggcgcgctgctggccaccgccggcctcggcggcatcgtctacgcgttcatcgaggcgcccacgcagcactggaactcacccgcggtgctggcggcgctggccatcggcattgccggcagcgcgggcttcattgccgcggagcgcaaggcacgcacgccgatgctgccgctggcgctgctgcgcatcggcaacttcagcggtgccaacctgctgaccttgctgctctacgcggcgctgggtggcgggttgtacttcttcccgctcaacctgatccaggtgcagggctactcggccacggtggcgggcgccgcgctgctgccgttcatcctcatcatgttcgcgctctcgcgctgggccggccagctggtcgaccgcttcggcccgcggctgccgctggtgatcggccccgcgattgccgccgtgggttttgcgctgttcgcggtgcccggtgtcggcgcgagctactggagcggcttctttcccgccgtggtggtgctgggcctcggcatgaccgtgaccgtggcgccgctcacgaccaccgtgatgaatgcggtgggacccgagcaggccggcgtggcgtcaggcgtcaacaacgcagtgtcgcgcgcggctgcggtgctggccattgcggtgttcggcgcggtgatggcctgggccttcgacggcgccttgtccgagagcctgcgcggcatgggcgcctcggcgcaggtgtcgtcgtttctcgaaggcgagcgcagcaagctggccggcgccgccctgccgccgggcgtggatgcggccaccgccgcggccctgaagcgcgccgtggccgaatccttcgtggcgggctttcgctgggtgatgctgctgagcgccgggctggctgtgctcagtgcgctgagtgcctggctgatgatcggcggcgggcctgccaaggagcgcaggaacggcggctgaaaggatggcgccttctcggggaaggcgcccattctcagttcacgtctgcatcgttgccggtcttccgtttcaccagcaggcgctgcgggccttgtccctcggcaccgagcttgtcgagcggattgcgcagacggcatcggtcgattgacaggcagccgcagccgatgcagtcgtccagcgtgtcgcgcagcttcttgagctgcgccatgcggtcgtcgaggtcggcgcgccagttggcggaaagccgtgcccagtcggcacggctgggcgccgcgtgggcgggcaagttggagagcgccgcggcaatgtcggcgagcgcaatgcccacccgctgggaaacccggatgaaggccacgcggcgcagcgtctctcgcgcgtagcgccgctggttgcccgctgtccgcgtgctggcgatgagcccctgcgactcatagaagtgaagcgtcgataccgtcacgccgctgcggcgcgcgacttcgccgacgctcagcacgggagcgatgccagcttgttccagagcgttgttcatgaatacctcttgacctcaactttacttgaggtttgagaatgctttccggcgggcagttcgtgcccgcgatctcaaggaaaaagcatgaccaacgatcaaacccccaacgttccgacacccgtttttcgcgtcgacaagttcatcgttccggccgaggtgctgcccgctttcgtcgcgcagatgcagcgcattcagcaaaccttgcgcagcttgccgggatgcgtgcgcaaccaggtgctcacccagaccggcgggccgggcgagttcaacgtgttgaccgtggtcgagtgggccagtgagcaggccgtggccacggccacgagcttcgtgcagaagaagttcgcagaggaggggttcgatccggccgacttcgtgcggcgcaatggcgtgcgcgctgacttggggttctaccgcgccgagtgagggattggccccggctcactgccgcggcatcagctcatagaagtcgaatccgttgctgcggccgccgaggcacaccgccagggtgtcttcgatcttgcgccattgcgcgagccggttgcgccatttgcgcacgctgtggccctcatcgggaaagctcatgtattcgaccggccggccgagcttctggagcgtggccaccacctcgtccgaatcctgccgcagcacgcgcacgtcgttggcgccgtggatcacgagcagcggcgccgtgatgcggtcgatctgcgagatgggcgaatcccgcagcatgcgctcgcgctcctccggcttgccgacgtcgccgaagaacgccgcgaagtagtggcggttgcgccagaacggcggccagttctcgatcacgcggggccagttggcaacgcccaccacgtcgatgccgcagcggtagtcgtgcggcttctggatgagctgcgtgagcaccgaaaagccgccgaagctcccgccgagcacggccatgcgcttcgggtcggccacgccctggtcgatggcccattgcacggcttcggcaatgtcgcgctgaagccggccgctggtttcgtgggcgccggccatcatgaaggcgcgcccgtagccggcggagccgcggtagttcacgtagaggaccgcatagccccggttcgccagcatctgcgtgggcgtcaagctcgcggattgccacgagtcgcgggtccacgggccgccgtgaatgttgaccacgagcggcgcgggcccctgcacgccgcgcggacgcacgaggtagccgtggatcacgagaccgtcggacgccttgaacgagaagggctccatgggcgagaagagatcggtggtcggctcgcgcggcggcgtaagccgcgtgagttgcccgctcgcgcggtcgagcagcagctccacggttccgttctcggtggtcgaacgcagcaccatgcggcgctggtcgttggccatgcccgcggggcgcgtgatgacgggctcggcgttcagccagccgcgctcccgggccgtcttcacggcagcggccacttcgttgcccagcgcggcatcgagataggcgatgcgggggcggccaggttcagatatgtacgcgagcggcgctccctgctgaggcgggaacacgccgtagtcgaggtcgaccgccgcatcttccgccagcagccgctccgcgcccgtggccaggtcgacttcgaccagggcgagcttgtcgcggccgacattcgtcatcgtccagagccgcccggcgccgaggtcgatgcgctggggccagaaggaatcgaaagccttcaccgttttgaaggcgcgccagccgccgtcgggctggcgcagttccagcagccggtcggagccgtcggcgctgccaagctgccgcatgcggcccgcgagctcgcgccgggtgtcgatgaaccacgagatcacgcggctgtcgggttcgctgcgcgcaatttcgcgcacggtgcgcgtgcgggcatcgccttcgaaaaggtccatgctggagcggtcgcgctggttgttcgcgaagtagaaggtggcgctgccgggcgcgccccatcccagcatggccgagcgcacgccgggccagggcgtcacggcccagggcttggcgcctggcgcctcggtgtcgagcacgaagatctgcgtgttctcgtcgcccgtgaagtccttgaggtaggccagatggcggctgtcgggcagccacgagtaggttggcccggacacgaagggccgcgccagcgtgccggtcgcaaaggtgcgggtgctggcgctattgaccgtggcggcgtcggccgtcttgcgcacgccgaggcccacgtcggtgccgaccgcctgaaaccatacgagctgctgcccgtcgggcgagagcacatggccgttgaccgcatcgatgttggcgacgaagcggcgcatgggaacgagcggcggcagcgtgttgtcctgccgcgcggcaaccagcgccgggtgcgtgggcccggtggcgcagccggaaagaagcgccagcgtgccgcaggcggcagccagggcgatgcgccagcggctgggggttctgctgtatctcatgttcctcgtccctcttggatgtcttgatgcgcggtcttgtccgcgcatggattctgccggtggcacgaacaagggtgtggctttccgcgtcgtcctgccggtggtcccgagggattgacaagcacctcatgctgcctggatactgaaccttcaggttcatcattcaagactcaggagattcccatgcagaagatcgttccctgcctctggttcgacggcaacggcgaagacgcggtgaagttctacaccggcatctttccgaactcacgcatgaccgaaaagcagctctggggcgatgagaaccccagcttgaaggggtcgctgctgaccgcgatgttcgagctggacgggcaggaattcatggtgctcaacggcggcccgcagtacaagttcacgccggccatctcgatgctcgtcagatgcgagacgcaggccgaagtcgacagctattgggacaagctgctcgaaggcggcggccagccggtgcagtgcggctggctcaccgaccgctatggcgtgtcgtggcaggtcgcgccgacgcctatccttcgcatgttccaggacaaggacccggccaaggccgcccgcgccatgcaggcgatgatgaagatggtcaagctcgacatcgccgaggtgaagaaagccttcgacggcgagtgatccgccgccgcggccgctacaccatccgccggatcgccttcttgcgccacaccaggcggtagtaggcggtctgcagcagcagcatcgccccgaaggtcacggggtaggcataccagatgccgttgagcccgatgcggtggctcatgaaccaggccacgggcacctcgatgccgatcaggcagaggatcgagatggccgtgggcaccagcaccgacccgctggcccgcatgatccccgagatggccgaggccatgccaaagatgacgaggctccacagcatgatgtgcagcagcgtctgcgcaatctcgatcaccggcgcgctggtgatgaaaaaccccatcaggtgccgcgagaacaggtagcccagcagcaccagtccgccggtcagcaccaggttcatcagcagcgcggtcttggcgatggcgcccagccggtccgcacggcccgcgccgatggcctgcgccccgaggatcgacgccgtgatggcaatcgagatggccggaaactgcacgtaggccaccacctggttcaccgcgccatatgccgcggtggcgctggagccgtagctgttgaccagcgagagcaacgccacctcggccagcgcgacgacgatcatctgcacccccgtgggcacgcccaccttgagcaccgccttcagcaacgtgggatcgatgcgcaggtggcggatgaattccgcatcgggcgcaagcggactgccgcggcggcgcaggcgccatcccagccacagcgtcgaggccacgaaacccaccaccgtggcccaggcggcgctcgcaacgccgagctgcggcaggccgccccatccgcgaatgagtgccggcgtgacgatgaggccggccgccgtggaaaagagcagcgtgagcagcggcgtgaccgtgtcgccaacgccgcgcaacatggcggtcgacagcaggaacacgaatagcccgggcatcgcgatcagcatgatgcgggcatagcgcgtggagtcggccaacacgtcgggcggcgtgcccaggaaggcgagcagcggcgtggtgaaggcgccgccgaacacggccaccgccagccccagcagcatgccgaccgacagcgtggtgccggcgatggccttggccttggcgacatcgcgcgcgccccaggcctggccaatcagcaccgacgcaccagcgcccagtccgatgacgaaggcaatgaaaaagaacatcaccggaaagaagctcgacaccgccgccagcgcgccgacgccgatcatctgcccgatgtagatgttgttgatggtgccggagagcgactgcaggatgttgctgagcagcatcggcgcaagaaagaacaggaaggtcttccacagcgcgcgcggcgcaccgacaggtgcgaccggggtcccgcgcaggccgctctggccggtggctgcgctctcggagcttgctctcatgcggtggtgctccagccggcggcggacaatttttgaaggtggatgcgcaggtccgggggccaagagtcgatcagcgcctcgaagcgctcgcgttcgcccgcgaacagcgcgcgggtggcttcctcgaagccgggcagggcgccagcgatcgcggtcatgaagcggtaggtggcttcgcgtgatgcgcgcacggcgtcgcggtcggcgttgacgcggctcgcctcctggaccagccgtcgcagtgcgaccgaggcgccgccgggctgacgattgagccagtcccagtggcgcggcagcagggtgacttcgcgcgcgaccacgccgagcctcgggcggcctacgccgcgcggggtttcttcaggggcttcggcgctggccgcatgcgccacgacgccggcccggttgtgtacgtcgaagtcgaggagttcaccggtctgttcgttgaacacgagatagggcgtgtcgtccttgcggtcacgcaattgtgcgagcacgtcggcggtgcttccctgggcgatgcgcttgaaggaggcgaagacaatcaggttgccgggtggcgtgtcggatggcatgttggatttctttattcttcggggccggtcgaaagggtgcgtaatctacccgttgaacggctcagtcgacggcgtgccgtcgtggcaaagcgcaaggagcgcaacgttgattttcgacaggctttcagcagccagcgatttcaccgtatcggcgcagattgcttgggcggtcgtgacggcagcttgcatcagttttctgccgccggtgcaaatggttgcgtggcggccgcctccattcgcaccggccgtgcgttcggccagccccgatttttcgagcaggaccattttgcgaaccaacgccgagatcggcaaccccagggatcgcgcaaggtcggccgccggcatgcagccgccttcggcgcacaggagccgatgaagcagcgtgaaatcttcgtagttcaggccatggaaggcgcccagatgctcctggagcttcaggttcaagctggcgtgggcgcggccgatgttgaggcacaagtccagcggatcgatgctcatggcgcgtcgtagccccggtcgccgtggcactgaagctcctcgcgccagagcacaagaagtttttcaagttccgcggcgcggtcgaaggcggggtcgtcgcgctccttgacgcggtcgatcacctcgaagctgaagttcgccgcaccgtgcgtggcccagtcgcgcaccagcgccttgttgcggtgcgagcgcaggccgagttcgaagcgggcgcggttcatcgctccctccacatcgagactggcggccacgtagaggcggccgctgagcgtattgcggatgacgaagacgcccgcggggcggaccgtttccttgtatttcctggcgagggcgcgcctcgtctcctggggcatgttcatgttccatatattatccgggtaaaattaaaagcacaatacacccgggtaaaaataggcaattacccctcgcgcaatcgccgccatcccttgcgagccgacggttcggtcgggcggcggcgaggagggtgaaggggatggcggaggaggggtgagcaccgcacccattgcgcgggttgccggcgggggctttccttcggccctatggcaaacttccacgctttattcgccaagcacgccggtccggccgggcgtgcatgacagggacgtcattcagacatgcaaaaaatcattcgccagctcgccgccgagatcaaggtcggcgagcaccaggtgaaggcggccatcgaactgctcgatggcggtgccacggttccgttcattgcccgctaccgcaaggaggtcaccgatggcctcgacgacatccagctgcgtgaactggaagcacgtctttcctacctgcgcgaactcgaggaccgccgtgccgcagtgctcaagaacatcgacgagcagggcaagctcacgccgcaattgcgcgccgcgatcgaattcgcgccgaccaagcaggagctcgaagacctttacctgccgttcaagcagaagcgccgcaccaagggccagattgcgcgcgagttcggcatcgagccgctggccgacaagctgctggccgacccgacgctcgaccccgccgtggaagccaaggccttcctgcagcccgccacgacgctggacgacggcaagccgggccccgatttctccaccgtgccggccgtgctcgacggcgtgcgcgacattctttccgagcgctgggccgaggacgctgccctggtgcagcgcctgcgcgaatggctgtgggccgaaggcctgctcaagtcgacgctgatgaccggcaaggacgaaaacaacgccgacgtcgccaagtttcgcgactacttcgactacgacgagccgatcggccgcgtgccgtcgcaccgcgcactggcggtgttccgcgggcgcacgctcgaaatcctggatgccaagctggtgctgccggtcgagcccgaaccgggcaagcccagcatcgccgaaggcaagatcgcgctgcacctgggctggagccatgcgggccgcccggccgacgacctgatccgcaaatgcgtggcctggacctggcgcgtgaagctggcgctctccaccgagcgcgacctgttcacccgcctgcgcgaagacgcagagaaggtcgcaatcaaggtgtttgccgacaacttgcgcgacctgctgctggccgcgcccgccggcccgcgcgtcgtgatgggcctggaccccggcatccgcaccggcgtgaaggtggccgtggtcgatgccaccggcaagctggtcgaaaccgccaccgtgttcccgcacgaaccgcgcaaggactgggaaggctcgctgcacacgctcggcaagctctgcgccaagcacggcgtgaacctgatcgccatcggcaacggcaccgcgagccgcgagaccgacaagctggcggccgacctcatcaagctgctcgccaagatggccgcacaggccggcgcgcccgagatgaaggtcgacaaggtggtggtcagcgaggcgggtgcttcggtctactccgccagcgaattcgcctcgcaggaaatgcccgacgtggacgtgagcctgcgcggtgccgccagcattgcgcgccgccttcaagacccgctggccgagctggtgaagatcgaccccaagagcatcggcgtgggccagtaccagcacgacgtgaaccagagcgaactcgcccgcacgctgcaggccgtggtcgaagactgcgtgaactcggtgggcgtggacctcaacaccgcgagcgtgcctttgctgtcgcgtgtgtctggcctgtcggccagcgtggccaaggcggtggtgcgctggcgcgaatcgaacggcgcgttcgcaacccgcaagcagctgctcgacgtgaccggcttcggccccaaggctttcgagcagagcgcgggcttcctgcgcatcaggggcggcgccgacccgctggacatcaccggcgtgcaccccgaaacctatccgctggtcgagcagatcatcgtcaagaccggcaagccgatcgccgagctgatgggccgcgccgagatgctcaagacgctgaagcccgagctgtttgccaacgagaagttcggcgtcatcacggtgaaggacatcctcggcgaactcgaaaagcccggccgcgatccgcgccccgacttcaaggtggcgcgcttcaacgacggcgtggacgacatcaaggacctggtcgagggcatgatcctcgagggcaccgtgagcaacgtggcgcagttcggcgccttcatcgacctgggcgtgcaccaggacggtctggtgcacgtgagccagctgagccacaagttcgtgaacgacgcgcgcgaggtcgtcaagaccggcgacatcgtcaaggtcaaggtgatggaagtggacgtggcgcgcaagcgcatcggcctgtcgatgaagctggatgccgcgcccgcgcgacgcgacggcccgcgcgacaaccgcttcgaaggtgcgggacgcggccagcagcagcagggtgcgcgccgcgacaacgcgccgcagcctgcggggcagatggcgagcgcgtttgccaagctgcaggggttgcgaaagtagggcgaggcaagtttgcagccgcctgttaaactagtcagaacactagtctgacaaggtggctctaaatgaaatcctggcccgtgcaagacgccaaggcgcgtttcagcgagtttctcgaggcctgtctcgccgacgggccgcaaatggtcaccaaacggggggccgaggccgccgtgctggtaccggcggcagagtggcggcgattgcatgccacggccaagccgtccctcaaggagttgctgctctcggccgaggcacgcaccgagtttctcgttccgcagcgcggcgcggcacgccggcggcgcatcacgccaatccgctgaggggcgggcggtatgtacctgctggacacgaacgtcatctcggaactgcgtcggcctcgaccgcacggcgcggtcgtcgcatggctcgcgcccatcgccgacagcaacctgcatctttccgcggtgacgatcggcgaaatccaggctggcatcgaaatcacgcgcgagcaggatgccgccaaggccgatgagatcgagcaatgggcagccctggtcgccgcctcgtacaacgtactgcccatggacgcagaaacgttcaggctgtgggccagactgatgcaccgcagttccaacacgctatatgaagacgcaatgattgccgccacggcaaagcagcatgcattgaccgtcgtgacccgcaacgtcagcgacttcgccggtttcggtatcgacgtcttcaacccgttcgagtcaagcgcggcatgaataaatgaaagccctgcgcatctacgccggccccgctgcccgcaagcacatcgaagcgcacggcttgcgcccgcaggacgtgcgcaccattcccggcgcggcgggcgggccgaagggcctcgtcctcgggccgctcgaccgtttcatcttcgggcgctggctcacgcagtcgagccagccggtgcacctggtgggcgcatcgatcggtgcgtggcggctttcgaccgcctgcctgtccgatccgcagaaggcctttgagcgctttgaatatgactacgtgcgccagcgcttcgacgtgcctccgggacagaagcggctcagcccgaaccagctgagcgcgcgctttgccgagagccttatcgacttctacggtgggcgcatcggcgaggtgctgaaccattcgcgctaccggctgcatgtggtgacttcgcgcgggcgccacatcctcggtcgcgagggcagggcgcgcacgcccttcggctacctgggcgcctttgccaccaacagcctgtaccgcaagggcctgggcgcatggctcgaacgctgcgtgttttccacacccggcgcggcgctgccgttcggcaccaaggatttccgcacgcgccagcatgcgctgagccaagagaacttcaacctggtgctgcaggcatcgtgctcgataccgttcctgcttgccgcggtgcacgacattccgggcgcgccgcgcggtgcgtattgggatggcggcattaccgactaccacctgcacctcgactaccagccgaccgacgagggcatcgtgctgtacccgcattttcagcgggccgtggtgccgggttggctcgacaagggcctgcgctggcgccacaagtccaccggctttctcgaccgcatggtggtgctcgcgcccgatgccgactgggtgcgctcgctgcccaacggcaagctgcccgaccgcaaggacttcatccatttcgcgaacgatccgcaggcccgcatcggcgcgtggagcaaggccgtgcgcgaggcagagcggctttcggaggagttcgagggctggctcgcaaccggtcgcacgcgggacatcctgccactctgaacaggccccgccggggcaaaccccaagggtgcgcacgcgcagcgccttcgagaatggccagctcactcttgtccagagaaagccgccactcatgcagcaggcccgaatttcacgccgccgattcacccttgccgccgcagcggcggccgcgaccttgccgatgcccacgctggcgcaaagcgcctggcccaacaagccgatccgcatcatcgtgccctacacgccgggcgggttcaccgaccagatggcgcggctggtgcaggtcgggctgcaggcgcggctcggccaaccggtgctcatcgacaacaagcccggtgccaacagcctgatcggcgtcgacgccattgccaaggccgcgcccgacggcacgaccttcggcgtcgtcattgcggcctacgcggccaacaccacgctgtatcccaagctgccctacgacccacgcaaggacttgacgggcgtgtcgctgatgggcgtgtcgccgctgctggccgcggtgaatgtcgatgcgccgttcaagaccgcgcgcgaactcatcgactacgcacgcgccaaccccggcaaggtgagcttcggctcatcgggcaacggttcggccgcacacctgacgaccgagctgtggaagtcgctcacgcagacctacatgatccacattccgtaccgtggcgcggtgcccgcgctgaccgacttgatgggcgggcagatccagctgttcttcgacgcgcccaccggcctcatcaaccaggccaaggccggcaaggtgcggctcatcggcgtggcgggcgacaagcgcctgtccgccgttccggatgtgcctaccttcatcgaacagggcttcgcgggcttcaccggcagcacctgggccggcatgctggcgccggccggcacgccgcgcgacatcgtcaagcgcatgtccgaagaggtggcgcgcatcatcaagagcgacgagacgcgcgccaagctcgacgccatgggcacgttcccggcgggcagcacgccggaggagttcgatgccttcattgccgccgaaaccgccaagtgggcgaaggtgatccgcacggcgggcgtgaaggcggaataggagaagagctcaggccgcgagcaccagcaccttgaactggctgggcacgatccgcatgccgacgatgttggagcggttctgcaccgagaggctggtcatgcgcgtgcagggtgaacctttcagcagcaccgtgaatgcgccggtgatgtggcgcgaagggcccatcaccgtctgagacaccacgcccatcagaacgcccgcgttgtcgccgttggtgatgggcgtggtggttgcaaggttgtgggccggcgtgccgccgtagaggatgttccaggcgttgggaatggccgttgggccgagtgcgaagttgggatacggaacgggaatcgcgggcggtgtcttgcagacatctggaaatgcgaggtccattcccatcatctgtgcgttggcaaacatgcgtaaggctccttcaatcaacccatgtggatctgttcggcatcgaccttgaccagctccttgctggtcaccagggtgttcttcgcatgaagccgaagcgtctgcgaggcctggatgtcgatgtgcccggcgcgcacgtgctcggcctcctcggtaatgcggaaactcgagcgcgtgaacaggtgaagccggtcgagcacgacttcgcaggcgcgccccaggaagcgggtgaccagcacgctgaaacgcagctccgcgccctggtaatcgagttccgagacattgcactggccgcgctccgccgtgagcttccattgaggcgcgctcgtggccatggacgtgtccgactggagttcgagcacgcccgcgctgcggatcgcgatgccgcctcgcttcgactgcaaatgcagatcgccgtccaccgcgagcgttgcctggcgcttgtcggcctgggccacgacggcaatcacgtacagcgcctcgtcgttcgggcccgcaaccatgaccgtatcgccgggtgcgggcacaagcaggcagctggcggcgcgctggcagcgcaaggggtggtgcccgtcggcaagcatcaggtcgcagaaatcgccgtcggggtcgcacgcgacgacggtggccatcgatatgccggccaccgccgacgccggttggcgctttgccggcgaggtctttcgcagcagcggttcgagctcgcttgcgggtcgggatactggcggtgctgcaggtgcagcgggggaaggaggccgggccgccatcgtcatgcagtgtcctttgcgtcaggtggtggatagtcgccaagccgcatgaggccccgggcatcccggtcgagccggaccgcgcgcggtgaacgttgccaggccaacctctcggcttcgaacagatcggggtcggaatcgagtacgccggcgcggtcgctccatcgggagccgtcctggtgggcgcggtgcagctgggtgcggtggcatcgggctttctcgaagccggcgttgcgcaggtccgcatacgagaaatctgcataggtcagacggctccccgcgaacgaggcgcgctcgcaccgggcgcgatggaacacgcactgctcgaggctcgcatccgaaaaatcggcatcgcacagcagcgcatcgatccacagcgactggtcgaacactcccgcgcggcagtctgcgttgcgcatgctggcttgcgggaacagagactgcggtgcatgcacgcggtgcatgcgcacgtcgtcgagggcggcgcccttgaagttgcactggacgagccgcgcctcgtcgaacacgcagttcgacatgcgcgcatccacgaactggcagagcgtgaacgactggccggcgaacgactgcccgcgcaggtcggcctccgagaagatggcattgtggaagccggcgccgcgaaagcccgcctcgcgcaggtctgatcgaaagaacacggcagtcgcgagttcggcgcctgcaaagtcggcgttgcccaggcggctctcgttgaagatcgtcttcgtgaccctggcccgctcgaagctcgccccctggaattcgcaatcctggaaggccgcttccttcagctcggcgccttctgcgcgcgtgccgcgcaagtccgattcagccacaacggtgccgatccatcggctggccggcgcctgcatgtcttgcaggctgcagcgcaggagcgacgcaccgtccagctgaatgccggccagcgccgcgccgtcgaaacggcagcgctcgaacaccgaatcgttcaagcgcgcgcgctcgagcccggcctgcgtgaatctgcattcgctgaacaggccgcctgacaggtccaggtcgttcagctgcatgccggtgaagtcttctccctgcaattgcactccgttgcggaccttggacaccagctcctgcgggctcattcgacgggtgtcgcccgcggagccggcacggtcttggtctgctcgaggtaggcaccgtgcgtctcggtgatggtgtcgatctggatctgggacatgtcggcgcgaaagagattggtctcgcgaaggtctgcggacagcaggcgggccttgttgaagttggtggtcatgagattggcggtacgcagagaggcgcgcgtcaggttgctgcggatgaacaggctctcgggggcctgtacggcgctcaggtcggcgcctgtcaggtcgcaggaagaaaagtcgcaggtgtcgagcgtggcgcgtgcgaggcgtgcgccctccatgggtatttcgcgaaagctgcattgcaccagcgtggcttcttcgaagttcacgttgcgcaggctgctgctgcccacgaagcaggaggtgcgcagcagggcacgctggaatccgatgcggtcgtcgccgttggtgtgggtccacatgcaggcttcgagttcggcgcccgagaagtccaggccggcgacccggcacgccatgaatccggccttttccaggctcgcgttccgaaagctgcagtcttcgatgaccgtgtccgaaaggaagccgatgtaggctgcgtccattccgtcgaagctgcagcgcaacagctgcgatccgatgatgtgcagatgatgcatgcgggccgaggagaaattgcattgctcgaacttgagcttctccagcgtcgtcctttcgaagatcgcatgcgagaaatcggcttggctgcagtcgactgctgccaggttggcattgcggaagacagcgcggccaaagcctgcgccggagagccgggcccgtaccagcaccgcgtcgctgaagtcggcgtcgtcgcacctggcgcgggccaagtcggctccttcgagcagcgcacgccgaaagcacgcgccacgcaggtcgaggccggacaggtcggcgccggtcaggtccatgtcggtgaagtcgcggctgccggcaagaaccgcggcgacctgcgcgccaagcgccgccatgcgatcggcgggcagggcgtccacgggtgcctggtgctgcgcggaactgcggtacagagccagcaatccgcgttcgccgttttccgccagcttgcgcatggcgtcgatctggctcgcgggcaatggcgcggtgccggttgccgcggggatgccttcgaacccacgcaccatggccgcgccgtcgacgcggggcggacctttcaattgcgtgcggtcgtgctcgcgcaccagcttgccggtgtcgaagccgactttcctcgactcgctggcgttggcatcagcttcgcgctggagccgctcgcgttcgacggctccctgctcgcgctgcgtgctggcatagcgctcggcctgttccacgaactcgggtagttcgcgcagggtgggcattcgggtaaaggggtctggaagccggcggtcgttgaagtggcgtgccttgtgccccgccgcgatcgccttctgcttcaactcttcgcgaccctgtgcgccgcgctcgcgcatgttgcgcaccagcgccgattccgggttgccgacttcatcaggccacggaccgatcgcttcttcgggcacgagctcgttgtcgcggaacatgtagagcgcgcctttttccggatcgcatcgctgccgcagcacggcggcgtagtgcgccaggccgcgcggggcatcgcgcatctcgatcgccggcatcacatgggaaatgtctgaggcatcgtcttcctcgatgcgcgtctcgccgtggaagacgagcgcgacgcggtcgagatgcggaaagaaccaggccgtggtcaagcgctgggcgacttcctcgacatgcccgggcaggcggtgccgcgcgatcacggcgagggcgcgccagccgggcaggcggccttgctggagcggcacttgggggtgcatgttccagatcgcgtagggcgctcctggcggaatctccatctgaggaaaccgctgaccggccggcgcggcgttgaagagctgccagtccatgtcgctggcaaagcccggaaagagatgggcgcgccagtgcgcgtcatactgcctgcccatgaggcgcatgcgccgcggcgaagcgatgtcgatggggccaaagccggcgggctccggctggtcgtgcggatgatgcaggcgatgcgccggatcttcgatgttgggcaggcgctgcacttcgaggtcatcgaccatctccagcgcgtggccgcggcccagcgggttgtccgcaaagtccggaccgccataggcacgcgtccaatcgattcgcattgcgtcgaacggctgcggcggggtggggcggccgcccacccagaagcggtcgccgaagacggtcaggtccttcgacaacccggcgacctgcagccttgcggcgcagagcgtcttttcgtcctggtgcgcggtgtaggcgaaacccgtggcgagtatctcggcgcgcaccttgggaatacccaggtcgatggcagtcgtcggacccagctcttcggacagcgtcttccagaactcgggctccggcgtcagcacgggctttccgctcatcgacaccatgcacagcgtcgtcaccgcaaggcgctgatcgccctggcgcaggaacggacgggttgttacgctcagccgaagcggtttgacggttttcatgggtgcggcatccgcggacccctgcgctcagcgcgcacgaggaagctccagcggcgtgcgttcgcggtcaatggccaccagtgccggattgtccgcgtcgtagcgcaggtggatggccttctgcggttcgaggaattgcggcaccagcgcgtcttcgacaaaggtgggaatcgatgcggcacgagccacgccggcactgtcggtgtagtcgacctcgagcaccacggcccggacggtttgcccgctggagccgccgcgcgtcatgttgttgggatgcattcgcacattgcggactacgccgtcggcgggctgcccgtcctgcgccagcgcaggccagagttttgcctctgcggaatagtggcggttttccttgcgcatgtagccgatggcgccgacgcccccaacgacgaccgcagtcatcactatgccgaagaaaatccagagaagcgtctcccattcaagcatggcgcaagtgtcacatgacaagatgcatggcctgcgcataggccgccatgccgtccacgaaaaagcgcacggctgccttgccgacctgcaccgcttcgttggtgatgtcgatgcccttgttggcaatcttgaaagtcagcaggtcgaccttgagcacggagtactgcgagttgatgccgtagaactgctggcgagcaccccagaagtcgagcgacatgcccacggcaccgaagcggaaccccgcaccacccgagcgcgacaggcgccagtcgctgctcttggcgtagttgttggtgtaggtctgcgagttgttcgtgtagctgatcgccaagttgttgtagacgttcgatgtggtggcgtagacgttcgtgttgatgacgtgctgcgtggtgttgtggatgtggttcgtcgtgttgaaggtcacgtccggcgaggtgtggaccgtcgggcccgtcacggtggtgctcgacggtccgtcgaccagcacggtgttcgaggtgttgatggtgtcgttgcgcccgccgctcacgaagcggatctcctggccgtcgatggtgccgtggaagccgccggtgatcgcgagcttcacgccacccgtgatcgtgtcgttcagcccgccgctgagcgtgcgcttcttgccgcccgaaatggtctgcgtgacgccgcccgtcacggtttcgctgaagccaccggtcacgtcgcgcgtgtcgccgccggtaatggtttctttcgcgcccgcggtgatgtcgcgcgtttcgccgctcttgtaggtcgacgattcatgcccgccgatgaccgtggtgcgggtgccgtcggtggtgtgcgtttcgtcggcttccacctcgacgtcgaggttgcgctcggcatgcagcaggatctgctcggcgcccgtgcggtcctcgaagcgcagcatgttggcctggttggccgcgccgcccgtgctcgaacgcgtgaggatgccgctggccgtggcattggcgggcagctcccagggcggcatctggtcgttgttgtagacgcggcccgtgatgatcgggcggtcgggctcaccgccgatgaaatcgacgatcacttcctggcccacgcgcggcatgtgcatggtgccgtagttggcgccggcccagttgctggacacgcgcacccagcacgagctgttctcgtccgactggccatagcggtcccagcggaactgcagcttgacgcggccgaagcggtcggtccagatttcttccgggccgaccacggtggcggtttgcgggccattggtgcgcggcttgggcgtcttgcgggcgggccggtagggcacgttcgaaggcagcaccgtgaagtcgaactggcagaccgattccgtgctgccgccggtggagtattcgggctcctgcaggtcgtagcgggtttcggtgaccaggtactcgcggttgtccgactcgcgcgggcaatgcgtcatctcgaacagatagcccggcgccatgcccaccacgttggtgtggcccgcggcaagttcgtgcgcgcactgcagctcctgcagccggatcttcgcgtaggtgtcgccttgctggtgctcgctgtagccgcccagccattcgtagacttcgtagctcgaatgatcgtggcccttggggtcttgccgcacgctttgcagcgaggcgcgggacttcttgaagtcgaagtcgtcgagcatcacgcggcccgaggtgatctgctccgagatgcgccattggtcgatgcagggctccatggcatggagcacccggtcgcgcgggcgataggcaatggtggcaaagcccggcagcttgccgtagccgccggtgtcgtcggccagcaccagcaggtgcgaattgttcgtgtgctcgaagtggtaggcgatgccttcgtgctccatgaggcggctcacgaaagcgaagtcgctctcctggtattgcacgcagtattcccaggggcggtagctgcccgtcaggcgcttttcaaattcgaagccgtatttgcccagcacttcgtcgagcacctcgggcacgctcttgttctggaagatgcggcagtcggtggtgcgcgtgagaaaccagagccagggctgaaccagggcacggtacacgtagtggcggccggtttcgttggcgcggcccacgagttcgaagcgcaccaccgtgccgttgagaaagcgcggcgcgccgccgtccgtgagttcgagcgtgagcgaagtgcccagcagcttcttcaggtcgagattgaagctggtgctgaccatgtcgacctcgaactcgaacaactgcgacagtccttcgtgcccccgcatggcgcgaaacttgagctgctcggcgctgagtacggtgtgaacctggacggtacgcatcattcggaatttccctgacccttggggcttctgcggatgcgaagccttcgaatgccagtctagaaattccttatgtcatatacatgacgcgcggaggctctgccctctgtagacgcagcgcaaacaaagcccttacagggcctccatcgagccgctacatcgaggcttcgagcatggccttgtagtcgccccgcgaagccagccgaggattggtcttgtggcagtggtcggccatggcaccgtcgatgatctgctcgaacatgccgggcgtcacgcccacttcggccaggcccttgggcaggcccaggcgcgcgttcatgtcgcggatcgcatcgccgagatcgccagccgaatcgaggtgcatggcctgcgccatgcgctgcagccgctgctccttctgcaccgactcggcaccggcattgaagtggatcaccgcgggcaggaagagggcgttgagcgtgccgtgatgcagccgcgggtcgacgccgcccaggctgtggctcagcgagtgcacgcagcccaggcccttctggaaggccatggcgccctgcatggaggcgctcatgaggttgaggcgcgcttcccggtcactgccgtccttggtggcgcgttcgatgtgcagccaggcgcgctccaggccgtcgagcccgatgccgtcggccggtggattgaaggcggccgacatgaaggtttccatgcagtgcgcaatcgcgtccatgccggtggcggccgtgagcttgggcggcaggccgagcgtgagctcggggtcgcagatggcagccttgggcatcaaaaaccagctgtggaaaccgagcttgcggtggtcgtcgacgatgacgatggcgccgcgcgccacttcgctgccggtgccgctggtggtgggcaccgcaatgagcggcaccacgcgatcggtgatcttcggcgagccgccttcgatggtggcgtaggtcttgagcgggccttcgtgcgtggcggcaatcgccacgcccttggcgcagtcgatggcggagccgccgcccacggcgatgagcccgtcgcagcgtgcgctgcggtacagctcgacggccgcgcgcacggcggcctcggtggggttggagggcgtctggtcgaacaccgccacttccagatcggcaatggcatcgagcgccttctgcagcaccccggccgcacggacgcccgcgtctgtgacgatcagcgggcggttgatgccgatgcgcgcgcactcgctggacagcagcttgatggcgccgaactcgaactggatctgggtgaggtattggatgagggccatgggcgtgaatgcgtggggcagtacgattgccgaccattcgaatctaacaagagcaaacagtcttgcacatgaataaaacccttggcgctgtcgcgtcgggcacattgctgaccgccaggatggccagcgtggtcgaacgcatggcccgggcgggccatccgagcctggaccaactcaccccggaggaggccaaggcctcgtacgaaaaaggcgccggcgtgctcgaggtgcccaagcccgagctcgcgcgcgtcgaagacatcggcgttcgcgtgcgcgacggcttcgagctgccgatgcggctctatgcgccatcgcgcgagaagctgcccgcgctggtgtactttcatggcggcggcttcacggtgggcaacatccgcacccacgacacgctgtgccgcgtgctgagcatgaagagcggctgcgcggtggtgtcggtcgactaccggctggcgcccgcgcacaagtttccgaccgcttcgaacgacgcctgggatgcgttcgccttcattgcgaacgaaggcgcgcgcctgggcctcgacacgagccggcttgccgtgggcggcgacagcgccggcggcaccctggccgcggtgtgcgccattcttgcgcgcgatgcgggcctgccgctcgcgctgcagatgctgatctatcccggcaccacggcgcaccaggacactgcctcgcaccaacgctacgccgatggccccttgctcaccaaggcgctgatcgactatttcttcggccagtacgtgcgcacgccggccgaccgcgacgactggcgctttgcgccgctgctggccgacgacgtcgacggcttggcgccggcctggatcggcctggccgaatgcgaccccgtggtggacgaaggcattgcctatgccgacaagctgcgcgccgcgggcgtggcggtcgatatcgagatctaccgcggcgtgatccacgaattcctgaaaatgggccgcgcgattcccgaggcgctgcaagcgcaggacgatgcggcgcgcgcactcaaagaggcactgaaaccatgaccgaagaaaccgtaccccagagaaaagacttccgcttctttcaccgcctgcgcgtgcgctgggccgaagtcgacatgcagaagatcgtgttcaacgcgcactacctgatgtatttcgacacggccatttccgactattggcgcgcgctcgcgctgccgtacgaggaggccatgcattccctgggcggcgatctctacgtgcgcaaggcgaccgtggattttcgggcttccgcacgcgtggacgacgtgatcgacgtggccatgaagtgcgcgcgcatcggcaactcgtccatcgtcttcgacggcgcgcttttccggcaggaccagtacctggtgggatgcgaactcgtctatgtgtttgccgaccccaccacgcagacctccaagccggtgccgcctgccttgcgcgaaattctcacgggcttcgaagccggcgagccgatgcgcacggtggagacgggcgactggaaaaccatgggcgaaggtgcgagcgcattgcgccgcgcggtcttcatagaggagcagaacattcccaaggaactggaatgggacgagcacgatgaagtggtgctgcatgcggtggcccgcaaccggctcggacaggtgattgcgaccggccggctgctgaacgccgtggacggcacggcgatgctcggccgcatggccgtgcaccgtgtgctgcgcagcggcgggcacggcgccgcggtgatgcaggcgctcgaggccgccgccaaggcgcgcggcgaccgcgagatcgggctgcatgcgcagcgcagcgcggagcgcttctatgcgcggctgggctacacggtgcacggcgagcctttcgaggaagccggcatcccgcacatcgagatgcggcgcgcgctgggtcagtagcgcgccggcgggtcgggcacgtagcccatctccgaacccgggaaggccgatgggccctcggggcgcggccagcgcggcgggggcggcggcaccgggatcacgcccgcggcaatgaggttctcgcggctgtcgtagcggatgcggaccacttcgtcgggcgtggactgcgcgcgctcgaaggtggtgtgcccgacgtgcgaggtctcgcgccggccgtgcgctgtgccgaggctcggggccggcggtgatggccgggccaatcctcctttcgccgacgcggaggattcggcgcccaaggcgctgtcggcggaacgggcctgtgccgcgggtgcggccggcgcggcctccgccacggccgagggcgcctcgctgcggcgctccatctcgcggctggaactgctgctgccgtcgcggcgcggcagcgcgatgggcggcggaggcggcacaggcacccgctcgcggaacatggcgacgccgatcacgcccacgtcgtccggacggccggtgcggctcgcgtacgaattggcaatcgacgtgaactcgaaggccgcgatctgcgagtcgctcttgcgccaacccgtgatgtcgctgcgctcgccacccgaaaaaacatagccgttctgcagcacgcccgcggtttccccggtgacgacgttgacgccgtccaccgacatcacggccatgatgcgttcgcccatcgcattgcgcgcgcggatggcgtagcgcgcgccgggccggccggcgacccagtattcgccgcggtggcggtagatggacagttcgcggccggtcgtgcgatcgaccacgctgacctgcatcagcgagccgatgcggtcgtatgcagaaggcggcgggggcggccgcaccgggctttcggcgcaggccgagagggcggcccaggcgagggcggtcgagatgaggagtctgcgcttcatgatggttcttccttgccaggagtggatcggtacggcttctacggggcagcaccagcggcagggttaaacgcgcgcaaaaaaatggcgcagcctctttcggggcggcgccaggcgtccgtgtcttcggacgctgggggattcgaaaaaaagactagatgtcttcgagcaacgggtagggcagcggctcgacggtgagcgccggcccgtcggcgccgccggcatgcaggccaccggtttccagggccgagatctggatcgagatcagcgcggcccagccgccaccgggtgccggcgcggcctgcgccaccgtgcccacgggctgctcggcgtcggcggcggcaaacacttcctgccccgcgctcaccggcgcattggcctgcacgaggtaggtgcggcgcttcaacgtgccgcggaactggctgcgcgccacgatctcctggccggggtagcagcccttcttgaagttcacgccgcccacggattcgtagttgatcatctgcggcacgaaggcctcgaccaccggcgtggtcaaggtcacgatgccgctgcgaacctcgctccactgccagagttcggcgtcgagcggcgagccggcgggcaccggactgccggcaggcgcgatccacatggcgcgcggcacgccgtcggctggatagagcgacaccgcgctgatgtcttcgccgatggccgtgcgctggccgggcagcgccgcggcatcgaggccgttggcggccagcgcggtaccggcaaggccgtacagcgcgaattgctccgtggcgtcggtgagcttggccttggcgcgcagcacgtacatcgacaggcgtttgagcgtggccgccaggatgtcgcggctgcagaccagcagcaccaggtcgggctgcggccggatgccgacaaaactcgcgatcacgcggcccttggccgtgcaaagcgcggccaagcgggcttcggcggcgccgagcagcgcgaaatcctgggtgagctggccgtgcaggaagctcgcggcatcgggtccctcggcgcggatcacgccaaggtgggaaagagcggtaacaccattgagaacgacagtagtcatcgctgaattatcatggtcgcagccgttccgtccggtccgcagggaatccgccccggttcccgcaaggccaccgacttttcgcccgattcgtttttcttttctccgctcattcatcggacccgtgcgccgcttcttcctcacgctttttctgctggccgccctggctgcgctcggcctcggcgccgccggactctggtgggtgcaccagccgctcaagctgcccgcacccagtctcgatctttccgtggagcccggcaccacgccgcgcggcgttgcgcaggccgtggccgatgccggcgccgacgtgccgccgcagttgctgtatttctggttccgtatctcggggcaagaccgccagattcgcgccggcagctacgagctggagcgcggcatcacgcccaagatgctgctcaacgtgctggtgcgcggcgaagaagccacccgcagcctggtgctggtcgagggctggaacttccggcaggtgcgtgcggccctggccaaggccgagcaactcaagcccgaaaccatcggcatgcccgacgacgcgctgatggccaagctgggccggcccggcgtgcacccggagggccgctttttcccggacacgtacacctattcgaagggctccaccgacatcgcgctgctgcagcgggccatgcgggccatggacaagaagctggaggccgcctgggcggcccgcgccgccgatttgccgatcaaatcggcggatgaggcgcttattttggccagcattgtcgaaaaggagacaggaaaagccaaggaccgcgccgagattgccgccgtgttcgccaaccggctgcgcaccggcatgccgctgcagaccgacccgaccgtgatctacggcctgggcactgccttcgacggcaacctgcgcaagaaagacctgctggccgacacgccctggaacacctacacgcgcggcggcctgccgcccacgcccattgccatgccgggcaaggcggcgctgctggcggcggtgcagccggcgcaaagcaagtcgctgtacttcgtttcgcgcggcgacggcaccagccagttcagcagttcgctcgacgaccacaaccgcgccgtcaaccgctaccagcgcggtggcggaagcagcagtggcgaacccaaaccgaaggttccgcaatgaatgaaggcctgtttctgacgctcgagggcatcgacggtgcgggcaagtcgagccatctcgatgcgatggaggcgcttttcaggggacagggccgcacggtggtgcgcacgcgcgagcccggcggcacgccgctggccgaaaccttgcgcggcctcatcctcgagcagccgatggatccgctgaccgaatcgctcctggtgttcgccgcgcgtcgcgaccacgtcacgcgggtgatcgagccggcgctggcacgcggcgacgtggtgctgtgcgaccgcttcaccgacgccaccttcgcctaccagggcgcgggccgcgacttcgacacagaggtgctgtcgacgctggagcaatgggtgcagggcagggcagggcccgccgatgcggcgcggctgctgcagcctcacatcacgctgtggttcgacctggcgccagagatcgctgcccagcggctggccggcgctcgcttgcccgacaagttcgagtcgcagccggttgaattcttccggcgcgttgcggcgggctacgcggcccgcgcggccgccgatgcggagcgcttcgtacgcatcgacgccagccagacgcgcgaccaggtctggcagcaggtcgagaccgcgcttgtcgcgcgcggcgccttggcacccgcaagcggggcggcaccatgagcacgcaagcgctttcgccctggctgcatcggccgctcgcggagctgttgcgccagcgcggccatgcctggctgctgcagggcccttcgggcctgggccaatacgaactcgcgctggcgcttgccgccgcctggctgtgcgaacagccgaaggcggaagagggcggtgccgcctgcggccattgcccgagctgccattccatcgaggttcgaacccacgccgacctttgcgtgctgatgcccgaggtggccatgcaggagttgggctggccgctggacgaaaaggcgcaggccgacatcgacgacaagaagcgcaagccgagccgcgagatccgggttgaagccatgcgcgacgcggtcggctttgcccagcgcaccagcgcgcgcggccgcggcaaggtggtgctggtgtatccggccgagcgcatgaacaccatcaccgccaatgcgctgctcaagacgctcgaggagccggtcggcgatgtgcgctttgtgctggcgagcgaggccgcatggcagctgctgccgaccatccgcagccgctgcctgggcttcacgctgccatggcccgccacggccgacgccgaagcctggctggtggcgcacgacgtacctgctgcggacgcggcggccttgctgcggactgccggcggccggccgagcgacgcgctgcggctggcgcgctccggccagtcgcccaaggcctggtcgctgctgcccaaggccatttcgcgtggcgacgtcgcggcgctggcggaccaggcgccctcgcaggccatcagtgcgctgcaaaagctctgccacgacctgatggccgtcggcagcggcgccgagccgcgctttttcgagccggccgacctgccggccgccgtgccttcgcacctggcgctggcgcgctggtcgaagtcgctcgccaacgcggccagaaccgccgaacaccccttcaatgcgggcctcatgctggaagcgcttgtgagcgaggcgcgaaccaccctaaactcagctcctcgccgcccatgaaccaaccagtcgcccccgccgccgccgcaacgcctcaacggccgagcgtgatccagctcgccatcaaggaaaagggcgcgctctatgccgcctacattccgctttttgcggagggcggcatcttcattccgacctcgcgcgaataccgcctgggcgacgacgtctacgtgctgctgacgctgcccgaagacccacagcgctacccggtggctggcaaggttgcgtggatcaccccgcagcgcgccgccggcaatcgggcgccgggcgtaggcatccggttcccgtcggacgaaaaatcgcgccagctcaaggcccgcatcgaagcggccctcggcggctcgatggcctccgaccgacccacccaaaccatctagctcgatagctaggctcgcccccaggctgcgcgcacttcgtgtcgctacgcccaccccctaccgggggcaataccagcggcccggcagagccggttccgcggtatttctggaatggggccagccgccgctccctgacacgccatgttcaccgattcccactgccaccttacttttcccgagtttgcggaccagatgccgcaaatccgcgccgccatggccgaggcgcaggtcgatcgcgccctgtgcatctgcaccaagctcgaggagttcgaggaagtgcaggcgctggccgcccgctacgataacttctgggccagcgtgggcgtgcatcccgacaacgaggacatcgccgagcccaccatcgacgacctggtgcgccgcgcggccatgccccgcgtggtcgccattggcgaaaccggcctcgactactaccagatggaagaacgcaagggcggacgcagcatttccgacatggaatggcagcgcgaccgctttcgcgtgcacatccgcgcggcgcagcaaacccggctgccgctcgtcattcacacccgcgaagcctcggccgacacgctggccatcctcaaggaggagggcgaagacggttccggcaatgccgcgggcggcgtgttccattgcttcaccgaaaccgccgaagtcgcccgcgcggcgctcgacctgggcttctacatttcgttttcgggcatcctgaccttcaagaaggcgcaagacctgcgcgacgtggccgccttcgtgccgctcgaccggatgctgatcgagaccgacagcccctatctggccccggtgccgtaccgcggcaagaccaacaatccgtcctacgtgccttttgtggccaagcagatcgccgaactgcgcaagctgccgctcgaagccgtggcaaaggccaccagcgacaacttcgaaacgctgttcaagggagtaaaaacaacatgaagaaatacatcaagaagttcatttatcttgctgtcatagcagcaacttttgccgcacacgcgggttctttcgaagactttttccgggccgtgcgcggagacaacgccagcggcgtgcgtacgctgctgaaccgcggcttcgaccccaacacgcgcgacgaaagcggccagaccgggctgatcatcgccttgcgtgaaccgtcgcccaaggtggcgcaggtgctgctcgagtcgccgcagaccgacgtcgacattgccaatgccaaggacgaaaccccgctcatgctggctgccatcaagggccagcaagacctcgttacccaactgctgaagcgcgatgccgccgtcaacaagaccggctgggcgccgctgcactatgcggccagcagcggccagctgaccatcatgaaggtgctgctcgacaactacgccttcatcgacgcgcaatcgcccaacggcaccacgccgctcatgatggccgcgatgtacggctcgaccgaagccgtgaagctgctcctggccgaaggcgccgacaccgccatgaagaaccagctcggcatgaccgcggtggactttgccaccaaggcaaaccgccccgaagctgcgcagctgattgccgcgtcggccgaggcaaagaccggccccaagcccgcgcccaaagacggcaaatggtgaaaccggcggcgcccgtcaaagcctgaattcgccgggtttgcgcaggcccggaaaagcactcaaaagggcgcctgcacagtcgtgcgagactctccgtagaaggagaagcagagatgagtacgttcctattcatagtctttttggtggccgtgggattgcttgcgttcgtgatggtcgccaggaagaagtcagcgcaaaacagcagcggcttcgtcgacaagcccaaagcccggccaccgctcactgcacgcgagcaggccatgtacaaccggctcgtgcaaacgctgccggatctcgtggtgctgccgcaggtcagcttcggcgccttgctcacggcccgcacgcgcgcggcgcgaagctcgttcagccgcaaggtcgccgacttcgtcgtgtgcgaccgctcgttcaaggtcgtcgccgtggtcgcattcggcggcgacaaggtcaacaggggcaagtcgcaacgcgacctggaccgggatgcgctgctggtggaggctggctaccgcgtgcttcgttatccgagggttccggacgtggggcgtgtcgaggcggacttcgatccgacgatggcatctgtgagtcctatggggtcctgagggcgtctgagggcgttcttggaccgctcgactgccgccacggccagacacttcactccacaaacaatacaatgtgcattatgttaaatgacatatgcggcaagtccatcctgaagaaccgcccgtgatgctcagccaggccaccaccgctctcgacttcgatacccctggccgcggtcttctggaaatcaccgcggccgtggcgcaatgggtggaacgcactggctatcaaaccgggctgctgacgctcttcatccgccacacttcggccagcctgctggtacaggagaacgccgatccggatgtgcaggcagacctcgaccgttttcttgcgcggctggtgcccgacggcgatccgttgttcaggcatcgcgacgaaggaccggacgacatgccggcccatgtgcgttcggcgctcacggccgtccagctttcgataccggtggccaacggtcgaatggcgctgggcacgtggcagggcatctatctttgggagcaccggaagcggccgcaccaaaggcaagtggtcttgcacctgatggggtcgtaaagggggcgtagcggctcccctgccccggccgctttttttgtcagcggctgcgcgactgtttcttcaggatttcgaggaaagtatccgccagctggttcggcgaatctttcttccgcaccgcaaagacgcgtgcgctggtcgtcaggcccttgatcggtcttgcgcgccgcggaagcgcgacccgcaaaaataggcacgttctttgcgtgactgcaagctcacggtgtaacgaagcactgttttggtgaggtttccgcggtcttgcggattccaggcgcgcagagcgccagcaccctccgcccgcatcctcgcgggtacctctccccctgaacccccgtccgaattgcagccccgcaagggctgcactttggcatttgcattgttgtttcgaatccgctgattc

SEQ ID NO: 5 - DNA, 791413 bp, Variovorax sp.
  source 1..791413: mol_type = genomic DNA
  misc_feature 1..791413: note = Part of the genome (contig); note (original language) = Parte del genoma (cóntigo)
gcggcaaaccagcagcgcggatcacggacagcgtgtccggaagcaagatcgtcagcggctcgcgcacggtgctgatcggcagccagggcggcgttgcatgctcggaatgcccgggcggagtcacggtgggcaatccggtcagtccgtcgcagggcgccaaggtgttgatgggggagccggagctcgatttcgccttgcccggggcaatgccgctggtctggcagcgccagtacagcagctacgtgaacctggagcacggtgcgccgtgcagcctgctgggctatggctggagcctgcctgccgagatgcgcatcgaactgagggacgaggcctgcatcctgttcacagccatggggcgggccatcaccttcgacccgctgcccgaaggcggctcgatctacagcccgagcgaggacatctggctgctgcgcggcgggccggatgcaacttggggccaattggaacgctttcgccacatcccacgcaatctggccggcgacccgcaatgcatcatggccaccgatggagcggccggaacgttctgggtgctggggccgggagcaacgccttccgaacagacgcgggacccagcagccccccccggcatgccttacgcgctgcagtgcatgttcgatcggttcggccggcgccagcgctatgagcgcgacgcttggggccgggtcgtgggcatcgtcgacggcgtgggccgccgctaccggctgaacctgcggcagctgcacgccgcccgggccgcgcagggcctctggcaggccgacagcggctggcggctgacgggcgtcgacctcgtcagcgatccctgggcgccgggcgccagcgagccgatcgcgctcgtgcgctacggttactcggacacgggagaccttgtcaccgtgcacgaccgcgccggccggctcgtgcgcgaattcgcctggcaggcccacctgatgacggcgcaccgccacctgggcgggccgcgccacagctatcgctacgagagcctggcgcccggtgcgcgggtggtcgagcacgccaacgaggaagggctgacctaccggttcgagtacggcgtgtcgcccaaagacaagacgacccaggtgaccgacagtctgcagcgtgtcgacatctaccgcttcgaaggcgaggcggggctgtcgcgcctggtcgaacacgtgcgcgcggacggcaccagggtgcgctacgcctacgacacggcaggtcgcatggcggaggccgtcgaccccctcggacgcaccactcggctgcgctacgacggcgagggccgcctgctgggcaaacaacagccggacggcacgctgtggagctacagccacgacctcgccacagggcggttgatctcggtgagcgatgctgccggcggagtcacgcgttttgcctacgatgccttcggccgcatgacgggcattgtcctggccgatggcagcaccgagcgcaacgagtacccggcgcccgaagatgcgccgatgagctgcgacctccccgtgcgcgtcgtcgatgccaggggaggtgtccagcaactggcatggaaccatgccggccagttggtgcgccacaccgattgctcgggtcacgccagcgaagcgcaatacgaccgctggggacagcggatcaggcacacggatgcgctggggcaaagcgtgcgctacgactacgacatggccggcaagctcagcgccctgcatcagcctgacggcagcgtgacacgctatcgccgcgacacggccgggcgcgtggtgcaagtgctggcgccgggcgatgcgggccccactcccggcatcggcttcgcctacgacctctggggccgtatcacccagcgctggaaccgggggcttgcgctgcactttgtctacgacctggccggacgcatggttcgcttgaccaacgagaacggcgcccatgcgcacttcgcctgggatgcgatggacaggcaggtcagcgaagaaggcttcgacggccggctgcagacctaccgctacgacgccgccggccagctcatcgaggccacggacggcacggcctcgggcagcctgagtacccgctatgcctgggatgccatgagccggctggccgaaatccacgtgccggccacggagcacagtccggcgcgcgtcgagcggctgcaatggaacccggccggccaactgatcgctgcacgaagctacctgctcggtccggggcaactgcagcaactgcacactgaagccctgaccgagcgcgacgcgctgggacgcccgaccgccgaaacccaacgcctctacaagctcggcgagcctggcggcgctgcctctccaaccccgcccgatatcgagttcgagcacaccatctcccaccgactcgatgccctgggcaatcgccaggccagcgagctgcaggacctggggcaggtggactacctgatgtacggctccggccacctgcacgggctgctctacaacggccagggcttgctggacatcgaacgcgatgcactgcaccgcgaggtccggcggcaacagatcctccccgcgagcgcagaggtgctcgtcacccggcgccgatgggacgcgctgggacgcctggaggacgtggacgttgcggggctggaccggtggaatgctttggagggcggcgcaccgtcacacttggtcgaacagcttgcccagtcccactaccgctacgacgccggaggacagctcgccgccgtcgagacccatggaggcggcaggcactatcgctatgacactccggggcgcctgatcggcgctcgaacggccgacggtgagcagcgctggcatttcgacccagcgggcaaccgcctgccatcctctcccggacgcatctcgcagttctcgtcgtcggtccccgaacaggacggtgaccactgggccgcacaggttcgcagccaatggcacggaagagattttgatgtgctgggtccacgcgaagcgccgcaaccgctgtcgccatcgttgaaaggagtgacatgctggcacgacaaccgtatcggtagcagcgacgacacgctgtatcgttacgacagccgaggcaaccgaacagaggccagccgcagggacgggcacaggttgctcatgcattacgacggcgccaatcaactcgtcgaagtgcaggtgttcgaccaaaccgcaagcctcgtgtgcaactatgcctacgacgcccatggccggcgagtgagcaagatcgtgaaagaacaggcccaccctctggcggagatccgggaaagccgtacctgccatggatgggatggagatcggctggtgcgcaccgagcactggcgctcgggccggcagaagcaggttacgcacacggtgtacgagccaggcagcttcacgcctctggtgcaactgagtatcgagggcaccgcgcagaagaacgcactgtccgcgctcgcggcacaggccgcgaatccgcaggtgcagcaagcgttggaagacgcattcagaggcctgcaaccgaacatccgccaggacatggcaaaccgcttgcaggcactgtctgggggcgccctctcctcgtcgatcaccgtgcgccactaccactgcgatccgctgggtacgccacaggcactgaccaacgagcgcgcagagcctgtgtggatggcgcgatgcgacccctggggcaacctgcaagaggaatacaaccctcacggcatcgaccagtcgatcagattgcccggacagcatcacgacgtggaaacggggctgcactacaaccgccatcgctactacgacccgggcttggggacctatgtcacccaggacccgatcgggctgcagggtggcctcaatctgcaccagtacgcggccaacccgctggaatggatcgatcccctcggattgaatcccgcgggctgcgccatcggggctggcgcaggcgtctggttcggcggggtgggggccgcaccgggatgcgccattggcgcaggtgtcggaacggtgcttgtgctcggggcggtcgcgctgggcctctcgggggacacgccaccgcaaagcaacacggcggcgaaaacagacccctggggcgtgccgatcgaccccaaggcagataccctgagtcaggcacacaagaacgccatcagccggacaagccccggctatggtggaaactgctcacccgacaactatgacaagttgcatgatgactacaagcagaaatgcgggcaggccgatgcgctgggcgcctgcaagtcgggcatgagtccgtcccagctttcagcacgaaggcaggctttcgggcagtgcgcccgtgcgcgcgaggaaatgatgaaccagtgcttctcgggcggcgattacaaccacagagagcaagccggcaatgtctggaatgcatacaagaactgcgcaggcactccatgacctacaaagacttggatgagccgtacctgcgcggcaggatattggaagcctttcccgaggatagacttcctcccgattgttttgccgaaagcgcctcgatcggcttcgacggcgaggggatcgcgcatatcaacgaccacctgggcggcaagctctggacagagatcgattggccggccctgctcaaagtgcatattgacgcttggcagagcatttcccagctgaagagcgaagcgtaccagtgcgtgttcccttcgttgctgttgtacatcgcggggggcaacgaggatttcctctctgagcatttcattgagatgcacctgaacctcggcaatgtgttcaaggaggaagagtccaggctcctagagtctctggatgacaggcaggcagaatgcgttgcgcttgttctcgtcggtcgcatcaggaaaaaaaggcagcggcgtctgtgccaagacgcgttggactcctattggggactattcgtgcccgaaggctattaatttggactaatgggatggacgccccctttttctacgagggcgtcgtgaccatcgacgttcaaagctcagaaattatgctgccgttcagtgactagctaaatcgtttgccggtgttcgctttgggccatttgcccggccgtcaaccggctacagtcggccaagaacagaccttcgcaacaacctcagggtgctccagcatccgaaccaaggtcgagcacccgttccgtgtgatcaagcagcagttcggcttcaccaaactgcgctatcggggctggcgaagaacacggcgcaaatggtcccgctgttcgcgcagtcgaacctgtggatggcgcggcggcgattgatcgggaatgaacacttaggagatcagaaaatctgaatcgtcattcaccatggagacgatataaccccagcagacggcggcaagaatctctacgagaccgagaggctgccaaacaatacctcgtctgccgcgcaggtcttgaagacccagttctcgcaatgcaaaggcgtgaccgtgcatcgcagcctctgtcaagaccgcgtaggagcgacgcaggtcgactgaaacacctttgccatgggctaatgaatagccaacacgaaacatcgatggcagatgtcgcctttctgcacccatcgcgtagaagcgataggccttcgcatggtcgcctgctctcgtcaaccagcgaccgaaataaaagcagcccaatggatgcccattagctgccgctcgttcgtagtaaacagcggctcgactttcatctttctgacagccgatcccttgcgtcagcatccaagcaacatacacttggctttcaacatgcccttcatcagccagcgcttgatagagatcaaaggccagataaagcagaccgtccgtgtatgcctttcgggcgagtaccagtttctccgcgcgatctgcgtgcatgcgttcagggctttggatagattccgggaggcggcgccggggggttgaatccgccaggccggattattccaggaggatttctgatcggcagcggaggggccgtaggaggagccactccatcatccaacgccctcaacaggctgatggccctcttgcctgcccaactggcttcccgccgaatgtgacttggcgtcaaggtgggacttcgccgcacgcttacattgatcgggatcaagggatgagtgcgtctgcagggttgggcctccacacccacttgcggcagcctcttgcgatatacggaggcctcaatccaatctcaccgaaattcgggagcccttcgtgggtagaatgctgtgccggggcggtaaggtcgccctactcgcgaaagcgcaagcacctgaatcgcaagctcttcgcttgcatacccctccgtggccaaaagcgagaatggccacttgctaccggagctggtatgtatttatccgtgcccactaagggcgctcgcgtcgcgcaaacacgctcagttgatcttgttttacgggaggctcggcgtctgcatcgcgccgcgcagtccaattccctttctacatctttgccggttcttcgtcgcgtaattgccgcagccgtcgttccaatcaacaatctgcctgagctgttccgcaaccgcaccacactgcgtcgaaagcaccttctcagaacgcttgctcttgaagctggctattccagttgggagatctacaggcccgctcttgatctcgtgcattcgtcagaattggaacactttgcagtcatagagaagggctgggcgaaccttaatctatggttctccaccgagtccgatgcacaggcgtacgcatccgagcacggagggcgtgcgatgtgcgtcggaagccaaggtgtggttgtctcggacttggtgtgcaggagcgtcgctaatgtctgaagtggctttttcattggccgggattgccagtatcagcgcatggcttggattgggtgtagcggctgcagtagcacctgggttggccaggacgcggcttttgctcatttcaggtcgcgttgtgcccgtgggtctatgcatcctctacgtttatctgcttgttgcgcactgggggcctgtgccggacggcggattctcgtccctcgctgcagtgctgaagttgttctctgtgcccggaaagatgctcaccggttggatccatttcttggcctttgatctgatggtgggaagatggctcgtggaccacgccctctcgcatcagcacgctcgctggcccctattgttgggccttcccgtcacgttcatgtacgggcctctcggcgtgctgtcgtactgcgctggtcagtttgtcgcctcgcgcttcgccgagcgcagcggcgttgaggcctaacccttcaatctaggcggggcccaacggcagcacaccaggcccgggctggtggtacgtgttagctctcaacgacgtcacacatatgtacgcgctcaaacaaaagatgctcgctgctttggcggccgcacttggtcttgctatcgcaacgatcctatatgtcgcctataccttccctagcgaggtaacgtgtctgttcattaaatcgatggcgcttgaacctcttgctgatggaacactcgtcgaaccgggcagttctgagttggaacgtgccatctttctcgatctccaatcgcaagccagagtacgaatagaaaagacctttggcactccgcgctcgaggcctgtcgtcgcgttctttcgagattcgcaaaccttttggcctttgaaagtaaacaattacggcagcgcaggctcaatcggaaacgcctgcgtcatcattggcccgaaaggtcaaactgtcgatgttgtggcacacgaactcatgcatcaagaactacgcgaacgggtcggctcttggggtctgttcgctgagattccaatctggttcaacgaaggcgtcgccatgcaagttgattttcggccacagtacacgcttccgaaggaagcgcggatacggcaagaaatagctgcagttcgaggcctcaagtcggttagtcagttcaatcatggcagcgacgaacaactaacgcagcactacgcgttcgccaaggctgaggttgagcaatggctgggcaatgtagggcaccatgatctatacccccgtttagagcgcgttcgtgctggagatagtttcgatgcggttctggtcaagtgagctgagagctaaccctgcattcgagagagacgccgtaaaagtgcggcgtaagcgcgcggtgatcccgtcttgacgacggtcgatcagcgcactgcggttggctgggcagcgctgcggcagcaactctccgactcgaccggccgggtgagtaggcagccgctcaagaatgtcgctgaggtacgcgtgcggctcgtgccccgttgagcttggccgactcgacttaattgctctgaaaaccgcaggccagactacgccagtcggcgaacagtcgtacggctagtgggagtgtttttcaatgaggcgctgggttgaggcggaggtagtcgaccatcgccagaaaccactcattgaagccaggacaggttcaatgagcccccctgcgaaccacagcacttagccgggtgtctcggtgtgggaacgggcaacaagcatcgcgatgtcgttggtggacacgatgtagttcttgaaggcgcgccatcctcagcgtgaagcaaaaactctcggagctgcgggtcgagaccatagcccattggtcctcggacgctgccacttcgggcagtgtgtgctcccagacgccatcaacgtcctcctcggaaatcttctgcttggcgaggtgggctgtcgccagttcgcgcttctagtccaattgaggctccttctacagacgacatgtcggcaagcacccgatgccattttgcgcgactatgcgggggttgaacggttgaacggcggctatcgagcgctgccaacttctgcttcgggcccattgccgtcctcgagtcagcaaggcactgatgccaaacttgtgctcgacggagcgtcgtagaccacagcgatgcgcacactacgtgtcgcaattcgctctttaggcggcccccacgaacttgcaaatctcgctcgaatactctcgcagaaacgcttgcttgttgggaagtggctccgtggtgtgcggcggtggaacgtccatgaacgagaaatggccagccccttcggtgatgcggacatccacaacattccaatcgtgcatggcacgtgcaagccattctgtttgggccggcggggtgatgctgtcggccgaccccacccacgccaaaaccggaattcgcacggcatcgagtgcggccggagcttgaaaaaaaccggttggtggtgccaaaagggcgagacgagccaagcgacggtccggtgcgatgctgacgcgccgacctggccccaaccacatttgtcccccggccatagcgacaagggtagccgcaccaatcgaatgccccacgcctattgctcttgcggagggctcaacgaatgcgtccagtgcaagggtgagtcgtcttgcccggagggtcagttcctcctctgtgggggtagtcgaagcaaggcgctcgaaatgtggtgcaacaaccgtgcaaccagattcagtcaaggcgtccagaagcgtagagagtcgctccggctgaccgcccgatccaactgaaaaaagaacgaccgaagaacctgtggcggttttgcgcactgagacctcaaatgaatcattcccgtctttcagtgtctgcgtcagcattggaaattgctcctcgtggcaagtgatttggatatgggtttgtgcatgtattttgcccagccagtctgctgtcgctacatggcgcggaacagatgcccgaacgcacggctgacgttgagcgatcgctggaggccccgcacggacaggctgtagcgcccgttctcttcgcgggtggcgctcacgatgcagtgggtgttgacgagcacgccgcgatgcacctgcgtgaagtcggcggcgtcgatccgcgacaccagatcacgcaggctcatgcgtaccagcgcctcgccatgggccgtgacgacattgacgtacttctcggcggcttccagacagatcacctccgagaccgggatcatccgcacggtattgccaacgccggcgcggatgaccttgatcttctcaggcgcgtcggccgcatccgtgatcgactgaacgcgctgcatcagggccgccatgccaccggcagccggtgtccgggcgcgctcgtgcagcctttgcttcaggcgttgcacgcagacctgcaagcgttcgagcgtcgccggcttgagcatgtagtccatcgccgcatgctcgaatgccgagatcgcgaaattgtcgtacgcggtgatgaagacgaagagcggctcggcctgatcgtcgggccactcgtcagcgacggcctcggcgacctccaggcctgttttgcccggcatcttgatgtccaggaacatcacatcgggcgccagggtctgggccagttcgatcgccctcagaccgtcgtcggcgacgcccgcgatcttcagctcgggccaggcttcgagcaacaaccgctgcagtgttctcgacagcaccggttcatcttcggcaatcacggcgcgcaacgcgttcacgatggaatcctcacgaccgcgcgaacgccgcacggggatcgagcttgcagagtcagggacgcacgcaggccatagagggtctggaggcgatcacgcacattctccagtccggagccgcaaacctcgccggcatcgtcgccactcgaagcgggctggtgcggcgacaatcccagaccggaatcgtctaccgcgacttcaatgcccccttcgatcgaccgtgccagcacttcgatgcttcctgcgcccaacttcggttccaggccgtgcttgatggcattctcgaccagcggctgcagcagcatcggcgggacggcgattcgctccagttcggcgggcaattcgagccggtaggccagcctgggacccatgcgcaaggacatgatgtcgaggtacgccctcagctgggagaactccgactgcagcgtcgtcacttcgtcgcgtgacgctgcatgcgtgctgcgcaggtagacgatcagctggtcgatcatgcgctcggcctgtcgcgggtcttcgtcgacgagcgagcgcagattcgccagcgtgttgaacaacatgtggggctcgagttgcgcgcgcagcagccgcaattccgattcggtggcgaggcgctgggcttcggatcgagccatcgcctctttggcaagctggtcacgcgtcgcagcggcgtaaaggacgaacgcggccagcaccagaccgaatgcgaacgccaccatgtagtcgcttccatgacccacaacgcggctgatcggttcgtccaggatcaggagcgcgaccaggtgaccgccgaagtaccccgtcgggatggcgatcgcgccggtgagaagccaacggggcagcggccgcattcgcagcagcggtcttgagcggccaagcaccgcgatacacgcgatgaacaccatgccgacacattcgatgaagacgaacaggcgagccagcgtcccgagcccaggagcggcccagaagagcagcccggccgcgagtgcgcacagcaggaacgagccggctgtcagccgcgctgcgccaagccagcgggccggaatggatgaatcaacgctgatcactggcggaagttggctgcatcgcggaactgtagaggttggcacgccatgccgctactgatcaagggcccttgggggcgaatttgtcctcaagccgtcggtttggttgaccgaacggcaaccgctcgatgccgcctcacgaccgttggcaccctcggccgggcgtttgggcgccaaaccagatgcgctcctggcagcggccgccgaaagtgcggacctcaccacccaggagtccccgtgcaacgatcttctctttcaaacacgctgctttgcgccgcggccgccgtctgtgcagccatggtcacgacgaacgcacaggccttcgacggcatcgtggaaaagcaggtgttcaccctgcccgcctacacgaccgtgaacggccaggtcgtcaagggagtgcgcatcggctatgaaacctatggccgtctgaatgctgcgcgagacaacgtgatcctcatcaatcacttcatcaccggcacctcgcacgccgccggccggtatgcggcgagcgacgccgcgccgggttactgggacacgatcatcggcgccggcctgccgatcgacaccgagcggttcttcgtcatcgcgaccgacgcgttggccaaccccaatcgcgcatcggccaccgtcgtcagcaccggcccagccagcatcgacgccgccaccggcaaaccgtatggcatgcgcttcccggtgctggctgcgcgggacacggtggaggtgcagaaggccctgctcgattcgttgggcattcgaaccatctacgccgtggctggcgcttcggctggcgcctggatgtcggtggaatgggcctcggcctacccggaccgcgtgcagcgcctgttgtccgtcgtgggacctggcgtcgacagcccggcctacgccatcgccaagatgagctcgtggggcgcggccgtgaggctggacccgaactgggccaacggcgactaccacggcaaggccgagccgctggcaggcatgacgcaggccatgcggcaggtcacactcgacgcgctcagcttcgcttgggccgacaaggctttcggtcagaagtgggccgacccgggcaaaaaccccggcgaagcgactgcgaatcaatttgcagtcgatgccaccctcgagaagatcggcgaagcgcgtgccaagggcatggacgccaacagttggctgtacacgctgaaggccttgcagttgcccagcgccaaaccagaccgcatcaaggccaagtcgctgttcgtgggtatcagctcggatcagatctttccgccgctcttgtcaaaacgcgcagtagaggtcctcaaggcgcaaggcaccccggcagagtatgtcgagttgaacagtcccaatggtcatgccgatgcactgggtgccacagtcggtcaagccgggccggcgattgcgtcactcctggcaaagtaggcacgcgcgaacatcattgcgtctgcgcggcggccgataccgcggcacgcagaccgagcaggtagctgtcgacgccaaatccgcaaatctgtcctttcacaatctccgcgaacaccgagtggtggcggaatttctcgcgcgcatggatgttcgacatgtgcagttcgacgaccggtaccgtaaggatcgccagcgcgtcgcggatgccgtagctgtagtgcgtccatgcgccggcgttgatgagcaccgcgtccaccccctcggcgaagccgcggtggatgcgctcgcacatctcgccttcgttgttggtctggaagctctggatctccgtgcccagttccttgccgagtgcttgcaatcgggcatcgatctcggccagcgtcaccgtgccgtattgcttcgggtcgcgcttgccgaacatgttgtggttgatgccgtgcagcatgaggatcttcatgggggtgcctgcgttgcgtcagaccaaggggatggtcattcggtcgatgacgccgcacgtatcgggccgcacgccgcgccaccacaagaaagcttccgcggcctgttccacgagcatgccgacgccgtcggccagcttcggcacgccggcgtgctgcgccaggcgcaggaagggcgtaagacccttgccataggcgagctcgtaggccagcttcgcaccctgaagcgtctcggcgggcaggggtggcagttcgcccttgaggctggccgaggtgccgttgatgacgatgtcgaatcgctctcctgccagatcgccgtagccgcagccttgcacgtggccgtgcccggcgaactgctttgcaaggtcgatggcctttgcctctgtgcggttcgccaatacgactacgttcggttgttgcgcgagaaagggcagcagcgcaccacgcaccgcaccgccagcgccgatcaccagcatgcgcgcacccttgagcgggaagcccaggttgcgctggatgtcattggtcaggcccacgccgtcgaagttgtcggcaatgatgcggtcgccctcgaacttgagcgcattggtggcgccggcgagttcggcgcgttcgagccgttcggtggccagcgcgtaggcctgcagcttgaagggagcggtgacgttcattcctcgcccgcctgccttgcgaaatgcgtgcacgtcgtcggcgaagcggtcgagcgagccctcgatcgcccggtagtcgatgtcctggccggtcgcttcggcgaagctgccgtggatcatcggcgacttggtgtggcctatcggattgccgatcacggcgtacttgtcggtcatcactgtctccttacttgctgtagagcacgccatcggcctgcatgtcggcaatctgtgccgcgtcgaaaccgaggctggctgcaatttccgcgttgtgctcgcccagttcgggcgctacctgcgtgatcgaggtgtcgcaccccgacatgcggaaggggaggttcggcaggcggatcttgccgagcaccgggtggtcctgctcgaccaccatgccgcgcgcacggatctgcggatcggccagcacttcgtcaatgcgttgaaccttggccgcaggcacatcaatgccgtccagcagcttcagcacctgggcgaccggctgcgccgcaacccacggcttcaccacttcgaggatctccgcgcgatgggcattgcgcccggcggaagcgtgcagccgcgtgtcgttgccgaaccccgcagggccgccattcttttcgaccagcgcagcaaagcgcttccatgcgtcgtccacctgcgcggcgatcacgaggtcaccatcctgcgcgcggaacacgccgtagagcgtggaattgggcatgtcgtgcccggtctgcaccggcacttcctgtccgttggaaagcgtgtagcactgcaccgcgtactcgtgcatcgacaccagcgtgtcgtacagcgccatgtcgatgtgctgcccgcggccggatttcacgcgtcccagcagcgcggcattgatcgcggcgaccgcatggatgccggtgtacatgtcgccaagcgagatgcgcagcagcggcggcgcctcgccagggttgccgaccatctgcatgatgccgctcttggcttcggcgatgaggccgaagccggcgcggtgcgagtcggggccggtgtggccgtaggccgagatcgagcagtagaccaggccgggattggtttcggcgagttcggcatagcccaggccgagcttgtcgagcgcgccggggcggtagttctcgacgaacacgtcggcactgtcgaccagcttcttcatcaacgcccgcccgcgcggatctttcgtgttcacgctgagccctttcttgcccatgttctgctgcaggaagtagccgctgtggtcgccgacgaaccacgcatgctgacgcccggcatcgcccgtgccggggcgctcgaccttgatgacctccgcaccgagcgcggcgaggcagcgcccgacatagggcccggccagaaagtggctgtagtcgatgacgcgaaagccggccagcggcagcgcttgttgtggcgcggcgctcatcccggcttcctcggcaccatcacgcggtgctcgcccttttgcacgacctcgtcgcgctggttgatgagttcggacggcaacacgaggatgccccagcccggcttgctcttcgattcgcgcttgctgccgacgtggaatttcacgcgcaccgtatcgccgagcttgatggggccgacgaagctccattcccagccgagggacatgcccggcatgaagcgcatgtcgctcttcgtcttgagcccgtcggccaccgagaggccgaacagtccgtgcgccacgcgggtgccgaacggcgtggtgcgcgcataggcttcgtcggtgtgaacgggggtgtggtcgccggtgaggtcggcatacgccatcacgcgggcctctgtcacctcgtagggcgggctgatgcattcctggccgacgacggcgtcgtcccagtacttgtcttcgatggtcaaggtggtcatggtgcgtgtctctctctatgtatgtcgggtgacggttcttcaggcgcgtggatcgatggcgagagcgcgcgccacggcgccagcgctggcctggatgaattcgacggccaggccgtccggcaggcgcagccagttgcggccctgcggcatttcggtcacgccgaaggcctgtgcggcggcgagtgcggcctcgaggtcttcgcacatcacgccaagatggccgaggcggccttcaggccctgcgtagtccggcttggccatgaactgcatgccgccgagggtccagtactggaccggctcttcgagcgtgccctgtacttcgcgcatcgtcatgccgcagacgtcgtggaagaacttgatgtgccaatggatgtctttcacccagatggcgacgtgttccacataggcgcgcggcgtgctcatttcgcctccagccggcgttcgatgcccttgatggcggcaaccagcgtctggttcaccggcgtcggcacgttgtgcttgagcccggcgcgcaccaccgagccgttgatgaaatcgatctcggtgatggagcctttttccaggctctgcagcatggaggtcttgaattcgtagggcaggccttcggcggccatcacccatgcatcgcgcggggccttgatcgacagcttcacgccgatggcctgcgcgacggtcatcgcctcggtcacggccgcgatggccgtcgcctcgatctcgggcaccgcgtagaggctgccgtacacctggcccgtgatgccgctcagagcgccggtcgagacgttgatgagcagcttgtcccacatcacgcccatgatgttgtcgctgacctcgcaaggcagcccggcgcgctcgaactcggccgcgatggccttggcgcgttcgctcacgttgccggcgagctcgccgatcaccgtgcgcttgccacgcgtgccggcaatgatgtggcccgggccgagcagaacgccgccgacgtaggtcttgccggccagcacatgcgcgcggccggcaacgtcggccaggatctcttcatggcccatgccgttctgcagcgacatcagcgcggtgtcgggcccgatgatcgacagcgcaccttcgatggcggagcgcgtgtggaaggacttgaccagcacgatcaccaggtcggctggcgccaagccctcgacgcttgtcgatgcgcgcaccttgacgcggcgttccgagtcgccctccttcatgaggagaccgtcgcgatggatggcgtcgacgtgcgcctggaacggatcgatgagcgtgacgtccgacccgccggccgcaagcgtgccgccgatggcacagccgagggcgcctgcgccgaggaagtagattttcatacgtgtctctcgaaggaatgtctcgaagggtgtctcgaaggaatgccttgaagataggtttgtatgaacatttcgtccatgacatgggatgaatggtctacattccgttttgaaatgaacgcggacgacgacaacctcgatgcgagcacgggcttgctcagcctcaagctgctgcgcctgttcgacctgatctacaccacgcagagcgtgacgcgcgcggccgaccagctcggccaaagccagccgacggtgagcaactggctgggccggctgcgcaggcatctgggcgatgaactgttcgtgcgcaccgcggcaggcatgcagccgacgccacgcgcagaagagctgatcgttccggcgcgcgaagcactggcggcgctgcgccgtgtggccgcgccaccggaagcgttcgatccgtcgagctcaaggcggcgcttccgtatctgcatgacggatgccagccacatcacgctgctgccgcaactgctggcgcacgtccgcgccgtgggccccggcatccgcctggaggctgcgcgcatcgatgaagaaaccggacaggcgctgcagtccggccaggccgaccttgcgatcggactggtgccatggctcgaatcaggcttctatcaacaggtgctgtatccgcaagactgggtgtgcctggtcaatgcccgacacccgcggatcaccgcaaaaggcatgggcttgcgcgacttcaaggccgaagcacacatcggcatcgtcggcggtacaggcgttcaactgctggaggcagcgctattgcggcatcgggtcgaacgacgcatcttgctggagctacccggcttcctgggactggccgccatggtgtcgaccaccgacctcgtggccaccgtgccccgccagatcggcgagacactggcccgcaccaacgggctcgctgtctttgattgcccggtgcccgtgccacccttcaccgtcaagcagcactggcatgcgcgctacaaccaggacccggcgaatcgctggttgcgcggcttgtgcgagcggctttttgccaggaaatcgaacgcgcgcaaatagaggatcgagcctttcgacgacgaccaggtggatgggtgcggcaattcacgacatgtcaacatgctttcttgacacgataacgtgacatgattattctgccgtcatgagcacgaccacgtccacgtacgagagcccgctccgcgcagaacagatggagcagacgcgccttcggatactggaggcgacggcagatgtgttggcggacgaggaggtcaacgaggtcaccgttccgcttgtcgccgtgcgcgcccgcgtgtcggtccgtaccgtctaccggcacttcccgaccaaggaggcgctcttcgatgcgttcggtgagtgggcggaggagcacctccgggtcgtcctcctttcctacccggacacgctcgagggcgtccgcgagatggcgcctgcgctctatcgcatgtacgacgagcgagcgccgctgatccgcgccctcctgtccaagcgcggacaggagattcgggcgcgcacgcggcgccggcgactggcgacgttcgagaaggcgatgcgggaggtcaccggcggtctcggcccggccgagcgccaacgcgcccttgcggtgatctacctgctcgtgagcgcgcccgcctggcaggcgatgcgcgaccagtgggacctcaagggcgaggaggccggcaaggccgccgcctgggccgtgcgcgtgctgacggacgagcttcgccgcaatccggcaagcatgaaggagattgatcatgatgacactcgtcgctgagcagaccttcgccccacccggtccgggatcgtggttcctcgacccgactcactggacgcggccagtgacccgcttccacgcggagatctttcccgacgcgttccagcgcggcttcggcgagagcctccgccgctacggatcgttgctcgagtacctggaggcgggcttcgtcaacggttttccgtactactgcgcacgcgtcgtcggcgcgccgagggaggcggtcggtcacccgccgaaagaggcgtgggacgagctcgcgcgcagtcacccaatgattcagcgccggctcgagacgagcgcgaccgtgttcgagcgcaagctctggcgtgaggacctcgagcgctgggaccgggaggtgaagcccgcggcaatccgggcccacctcgcgctgctcgcggttgacccggcaatgctcgacacgcctgcgctcctcgtatacatcgatcgctgccgagagaaccagatccatggcgggtacatccatcacctcttcaacgtgccggcgctcctgccggtgggcgacttcctcgtgcacgcgcaagagtggacaggccgctcgccggcccagttactcggtctcctccagggcgcgaacccggacccgctcggtgcagacgaggagctcgagcgactgatcggcgcgctccgactggatacgacggccacggccttgctcacgtcggccggagagccgggcgaggtgatcgccgcgcttcgctcgctgtccggcgacacgggccggcacgcttgcgcatacgtcgatcgtgtcgcctggcggccggtcaacggcgaggacgtgggcgacccgtcggtgcacgagcttcccgagctgatcgtcggagcgatccgcacagcattcgaccgcctcgagactccaccggcgaacgacctggaccggaagacctctgacttgcgcgacgcagtgcccgctcggcatcgcgatgccttcgacgcgctgctcgaggaggctcgggcgacctaccggctacgcgacgagcggggcatttacgccgacctctgggcgatcgggatcatgcggcgcgcgatcctcgcggccggccgccggcttacgacggccgggcggctcgccgatcccggccatctcgtcgaggctggctacgcggagctgcgaagcctcgtcgagtccggcgacggcccatcgggcgatgaactggccgagcgcgcccgctaccggatcaaggcgcgctacgcggatgcgccggcgtttctcggcggcgaaccgggcgatccgctgccgcccgagtggctgccgcccgcggcggcaaggctggagcgcgcgatcggtgcagccgtgcaggcgatcttcgccgcgccgaagccacgcaccgaggacagaaaggttcacggtctcggcgtcagcccgggcctgtacgagggcaccgcacgggtgattcgcggcaccgaggagtttggtcgcatcgagcggggcgacatcctcgtcacgaactccacgacgacggcattcaacatcgtgctgccgctcctcggcgcgatcgtgaccgaccggggcgggctgctctcgcacgccgcgatcgtcgcgcgcgagtacgggctgccagccgtcgtcgggtgcaccgatgcaacctcggtgcttctggacggcgcgagagtcatcgtcgatggcaccgcgggcgaggtcgagctcgtcgcatgacggaagcaggcgaccatgaaaccggcagcgcttaccgaggagctcgaggagagcctgttcggcggcaaggccgcgcagctggccgccgccacgcgtgcgggcctgcccgttcccgcgggtgtcgcgcttccgtacgggttcgtggatgcagtcgctgctgacgaaggcgacgcgaagcagcggctggctgcagtctttcgcacgctcggcgccccgctcgtggcgcgctcgtccgcagtgggtgaggactccgagcaagcgagcttcgcaggacagcacctgacgcagctgaacctgcgctccgagtccgagcttgttgacgccgtgtccgccatctggcgctcggcgcactcgccttcagcgttcgcgtaccgcgagcgcctccggctgccccgcgagccgagaatgggcgtcgtcgtacaggagctcgtcgatgcggactgcgccggtgtgctcttcagccgcaaccccgtcaacgggtcggacgagatcgtgatcgaggcggcctgggggctcggggagtcggtcgtggccggtctcgtcatcccggatcggttccgcttgaggcgtgacggtgccgtcgtcgagcgaatcgcgggactgaaggacgtcgccatacgcaccgacccggaaggcggcacaagcagcacacaggtttccgaggggctcgcccgcgtgctctgcctgggcgatgcacagctcgccgcgcttcatgcgctcgcgctccgctgcgacgaggtgttcggcgggagccacgacatcgagtgggcgttcgccggcggccggctctacctcctgcagcggcgagcgctcacggcgatcccaagtccagctgcaggcgaccacacggacgagcgggtgcgcttgccgaactagcgggcgcgatcgactacgcgggcgccctgcccttgacggcccaggccagcgccgcatacgaacgcgcgccatcagcttcgccgtcgagataggccgcctgcacagcctcgcgcagccgcccgcgcccatccgaatccagcgtggcgacgtattccgcgccagggccgtccttgccttcgtagggcccccaatagtccgcgaacgacgagaactccatccggatcgtgagcgtcgtttcttccacgcccttgaatccggcctcgcgccacgccttgcccagttcgccgggccgcgtcatgggccgcgtgtagttgcgggcgcgtcgcgcgccggcctcggggtcgagcatggcggcggtgtcgaagaacatgcggttggacacccagccgcccctcacgtcccacaccgccgcagcgaccacggcgcctggcttcgcgacgcggcgcatctcggcaatggccttgcccggctccggaacgaagtgcagcaccagcagcgagagcacgcggtcgaagctctgcgcggggtacggcagcgcgcaggcgtcggccacctcgaaggcgatgcgcgcatcctcgttgtggcgcctggcatgttcgatatagggctgcgcgaggtccacgccccgcacttcgccggcgcccgtgcgtcgcgccacggcaaaggccaggtgtccggtgccgcatccgacgtcgaggatgcggtccccgtccgcagtgccggtgaagtcgagaaaaggcagcgcgaggaggcggctccagcggcccatcaaccgttcatagccctcgccgtcggtggcgacgaaggtcgaagaagtggtgctcatggcaatccctccgcacggccgggcgcatggaaattgccgtgcaggcagatgctatgcctcggccgatggcggcgtcaacgccggtgcgccgcaacaggtcgggtgcgtccaatgcgaaggcttctgacgaaggtgcgacggcaggatctgcttgtagcgactcgcacaaccgcagcctgcttcgtgcaagaccctcattgcagcatcggcgcgagtggcacgcagcctaaacttttggacatccaaaggcccgacctcagtcccctcatgagcaccccaccgcactaccaagcattccgtggccacgcttctatggatggcaatgaacaaccctgacttcgtttccgaaaaggccgacgccatgaactcctccatcgtcgaacgcctccagagcgctggccgtctggaccgcgtgttcatcgacggcgaatgggtgctgccccaagggcaagctcgcgcctctgtcatcgacccgtcgaccgaggagcctgtcgcggaaatcgcgctgggaactgcgcaagacgtggctacggcggtggtcgccgcacggcgcgccttcaccacttggtccgtgagcgccgcccagagccgggccttgctgctggatcgcgtccacgccctgatcctggaacgcgccgaactgttcgcccaggcgatctcgctggagatgggcgccgccatcggcttcgcgcgcctcacgcaggtgccctccgcggcggagcacatccgcgtggcccgcgacaacgcccgcagctaccccttcgtcacccatcggggtgacatggccatcatgcgcgaggccatcggcgtgtgcggcctgatcacaccctggaactggccgctctaccagatcaccgccaaggtcggcgccgccctggcagcgggatgcaccgtcattttgaagcccagcgagctgtcgcccctgagcgccctgctctttgccgaagtgatgcacgacgccggcattccaccgggggtgttcaacctggtgaatggcagcgggccggaggtcggcgccgccttggcggagcatccggacgtggacatgatctcgttcaccggctcgacccgggccggcgtcctggtggcccaggcggcagccccgacggtgaagcgcgtggcccaggaactcggcggcaaatcgcccaacctcatcctgccggatgcggacctgtctcttgccgtgcccaagggcgtggcgtccgccttccgcaacgtcggccaatcctgcagcgcaccgacacgcatgatcgtgccccgcgcgcacctgcaggaggtggaacggctcgcgctcgaagcggcatcggctttcgtcgtgggcgatccgcgttcgcagcagaccacgcacgggccggtggccaatcgcgcgcagttcaaccgggtgcaggaaatgatcggcgtcggcatcgccgaaggtgcgcagctgctttgtggcggcctgggacggccggagggcttgagccgcggcttctactgccgcccgaccatcttcagcgcggtgcactctcagatgcagatcgcgcaggaggagatcttcgggccggtgctcgcgatcattccctacgacagcgtggacgaggcggtggatattgccaacgacaccatctatggcctgggcgcccatgtgcaaggccaagaccttggcgcggcgcgcgccgttgcggcacgcatccgctccgggcaggtgcacatcaactatccggcgtggaacccccatgccccctttggtggctacaagcgctcgggcaatggccgcgaatacggcatcgaaggcctcgaggaatatctggaaaccaaaaccatcctcggctttctggatgcctcggcgcccagcaacaactgacagactttcagtgaagacatcgcgcatcgcgcaggagtaatcatgaccgtggccctggtactgcatcgcgccgatggcgcgcccgtttcaaccgctttccgcagggcgccgttcggcaaggacgatccttttgcgcggcatcgcgagatcgcgtgggaaggaccgggcgcgatgagcgcgggccgcaccagcttcatcggtgagctcgacgtcgcaagctatccccacatcgaaaccatcgtcgttgtcgagggcgagctgaccctgacggcggccggcgaggccccgctggtggtcggtccccaggcgggtgccgtcatcggatgcgacacctcgcttcgcatcgaggccgcatcccgcgtgcgctttgtgttttgcgcagccgcctgcgacaagccgacgaagcgcggccttttccccttgcacgccgacgccaacttcacgcccaccggcacgctgcccgccgaagtgctgctgggccccgtgcccgagtgccgcagcgacaaggtcttcaccgatgacgccgcgcagtaccttgcgggcgcttgggactcgacgccctatcaccggatcgttcgcgcgcatcgcatgaacgagttcatgcatctcgtggcgggcagcgtgcgcttcgcagcccctgatggcagcgtgctgtctgcgggcacgggtgattcgcttttcgtgccccagggcgcgccgatcggatgggaaagcagcgatcgcgtggcgaagttctacgtgtgccagaccgtcccggcttgaacgagcgagcgagattcatcatgtcgcctccgctgcgccacatccaaacttcgcccacgctgccggcctcggcggacgtcgtcgtgatcggcggcggcatcatcggcgtcttcaccgcctactacctggccaagcgcggcctttcggtggcgctggtggaaaagggcagcatcggcgccgagcagtcgagccgcaactggggctggtgccggcagcagaatcgcgacgcccgcgaactgccgttggcgagcaagagcctcgacctgtgggaacaatttgctgccgagagcggtgaagacacgggcttccatcgctgcggcctgctgtatctcagcaatgacgaggccgagatttcccgctgggccagctggcgcgattttgcgaagaccgccggcgtgacgacccacatgctgagcagccgcgaggccgccgagcgcggtcaggcgaccggccgcggctggaagggcggcgtcttctcgcccagcgacggcaccgccgaccccgccaaagccgcaccggccgtggccgctgcgctcatcaagctcgggggcagcgtccaccagaactgcgctgcccgcggcatcgagaccgaaggcggtcgggtcagcgcagtcgtgaccgaagccggcgtcatcaagacccggacggtcgtgatggctggtggcgcctgggcctcctcgttctgccggcagctcggcatccgctttccgcaggcctcgatccggcaatccatcctcagtgtgtcccctgtggaacatcgcttgccggatgccgtggtgagcgcgggcgtgtccgccacgcgccgcaacgacggccgctacgcactggccatcagcggccgcgcgcgcgtggatccgacagggcagtttctgcgcttcgcgccgcagttcgtgcccatgttcgccaagcgctggcgcaaccttcgtccgggcggcctggaagccattcggagtggccatgaaacgctggcgcggtggcgcctcgacgcgccgacgccgatggagcgcgtgcgcatcctcgatccgaagcccgatcccgtgagcatcaaggacacccatcgtcgcgcgatcgaactgctgccccaacttcgcgatgcaaagatcacgcacgcctgggctggctatatcgacagcacgccagacggtgttcccggcatcggcgaggtgccgggcctgcccggattcattttggccgcgggcttttccggacacggctttggcatcgggcccggcgccggccacctcattgcggacattgccagcggcggcgaaccgatcgtggatcccgcaccgtatcggccggcgcggttcagcggctcggcatggggcaaggtcgctgatttctagcatcgatgttctcgagcgatgtgattgtggtcgacggggggttcggcctgatactcgcccgccacggccgaagctcccgccgccctctgatggcggcctgagaccaggtgtcatcgcgcggttcttcgcctccagggtggcggcgcaagagattggcgcagcatcgtcagaaaggctgttgcccgcgcacttcgcccgaagcgggtgcccagcatggcgacgacgtcggcggcgggaacctcccagctcgcaagcacccgcttgagccgaccggctgccagatcggcagcgacgttccattccgaccgcatcgcgacaccttgccctgccaccgcccagtcgcacaccacggcgccgtcattgctgcacatggtgggacggatacggacggtctgcggctcgcgcgaagcgtgcacgaagcgccacagcgtgacgtcctcgtcgttctctctcaccaccaggcaccgatgccgcagcaagtctgaaggcgcctgaatcggcggagcaccagcgagatagtccgggctcgcgcagaggatgcgtcggttcggtgccagcgtcgtgacgatctggttctgggcgccaggcggtccgatgtggacgatgacgtcgctgctctcgaccaggtgcgcaccgggatggtcggcaaggtccagggtgaccgtcacgccaggatgcgtttttgcaaacgcatcgaccacgggtgcgacatgcagccggccgaagccatgcggagcggctatgcgcagatgcccgctgacggccttcttgcgattggccaaggcctcggacagcgcctccatcgcgtcggccacgatcgtcccgtgcgatgcgaccagatcgccttcatcggtgaggaccatcctgcggcccgaacggtcgatcagccggatgccgattcttgcttccagcgcttgcaggcgctgggtgacggccggcggcgtgacatccatcttccgggccgcttcagcgagcgacgcagaccgggccagcacgttgaagaagcgcagatcctcagagctgatcatttagttgggccttaactcgctatgcaggttcgataaattgtaggttcaatcgatcgggcgcaacatccggccatctgacttggtcggtgccggtccgcatcccgcaggccgcatgggacaagcacaactcggagcacgaccttgggccaggccacagccatgaagcagacgcaagccgaacagatcgcaacgacgccgggagaactggcaacgccttgcctcgtcctcgaccctgcgctgcccgccgggggcgccgacgcggtgctggtcccgtttgccacggaacacctggaaggcgccctccagctttcgcaggagatgtcctggccctatcggctcgaggactgggccttcgcgctcgagctcggccagggcttcgtgctgcgcaacggcgccggtacagtgatcgcgaccgcggcctggtgggcctacggcgacgaccaagcttcatgcgggatgatcatcgtctccagggctacccaaggccgtggccatggtgcccggctgatggatgcgctgctggcggcggcgcactcgcggaccatcacgctgaactcgacggccgaaggtctggcgctttatgaacggcgcggctttgtccgcatcggcgtcatccagcagcatcaaggcgttcccgaccagcgccaccaggcgccaccggccagcctggtcagggcgatggcgccatcggatgtcgaggcggttgcgcgtctggaccagcaggccacgggctgggccaggcggcagatgctggatcggctcatccaggctggcgacggccacgtgcttatgcgtggcggcgagccgcgcggctatgccgtttcacgcctgttcggccgcgggcacgtcatcggtcccgtggtcgccgaaagcgcggccgatgcgcgcgccttgatcgaagccgcgctcgcacgtctcggccaggttttcgtccgcgtcgacaccgcggccacctcgcagctcggggactggctcgaaagcatcggcctgcgccaggtcagtgacgccaccaccatggtcaaggggccgcacatcccgccggcggggcccgcacgcatgttcgcgctggccaaccagtcgttcaactaggagacatcacgatgctgagctcgaagacgccggaaaggcagccatgaagctgacctcgtattggctggacacctcggagcccttccgcagtgccgctgcaggaccggtgcagggtagctgcgacgtggcggtgatcggcggcggcctgaccggctgttcggctgcgctggcgcttgccaagaagggtgcgcgcgtcgtgctcctggaagccgagaccatcgggcacgccgcctcgggtcgcaacggcggcatgtgcaacaacggctttgcgcaggactacgggatgatgtcagccaagctcggcaaggaggttgccgacaggctctatcgggccttcgacgccggagtcgatacggtcgagcgcctggtggcggaagagaagatcgactgcagcttcgcgcgcgtcggcaagatcaagctggcggccaagcccgagcactacgacaagctggcgcgcagccaggaactgctggcggccaacgtcgaccccgacacggagatggtgagccgcgccgacctggccagcgaggtcgggtcggaccgcttccatggcgggctgatctaccgcaaaggcgccggcatgcatgtcgggcgcttcgtgcgcggcttggcggaagcggcggcgcggcgtggcgtggagatccacgagcatgcgccgatgatgggtctgcgaccggcacccggcggagggcaccagatcgaaacgccgaagggtcggctccacgccaggcaggttctgctggcgagcggaacttcgcagacgggaccactgggttggattcgacgccgcatcgtgccggtcggcgcgttcctgatcgtcaccgagccgctgccgacagagacgctcgaccggctgttgccgcggcgccggatggcggtcgatacgaagaacctggtcaactacttccgaacgacgcccgacaaccggctgctctttggtggacgcgcccgcttcgccgtctccaacccgaactccgacgagaagagcggcgcaatcctcaaggccgcgctgcacgaggtcttcccagagcttcgcgccgcacgcatcgactattgctggggcggtatggtcgacatgacgcgtgaccgcctgccacgcgccggcgagcgcaatggcatttactactcgatgggctacagcggccacggcacccagatgtcgaccctgatggggacgatcatggcggaagtcatggacgggcgcgccgaactcaatccctggaaagacttcgactggcccgcgatcccgggccacgtcggacccccatggttcctgccgctggtaggggcctattaccggctcaaggacaagctcgcctgaagcccgtctcgccactcatcaatcgaggaatcaaccatgaacgagcacaagaacctcaacggcctgatcggcgccgaggaaagcacgcgcctgatgggtcagctgcagcgcggcgccagccgccgcgacgtgctggcgatgctgatggccggcggcatgcaggccgcgctggcaggcagcgtcgcggcgctggccaccacggcaaatgcgcagacgccgcgcaagggcggccgcatccgggtcgcgggtacctcttcgggcgtgaacgacacgctcgaccccgccaggcaggccaacggcaccgactacgcccgcggcttcatgttctacaacggcctgacttacctggacggcagcctcgccgcgcagccgcagctggcctaggagttcacgaccaaggacgccaggacatgggtcttcaagctgcgccgcggcgtgagctttcacgacggcaagccgctgacgccggccgacgtggtgttctcgatgatgcggcacaaggaccctgcgaccgcatcgaaggccaaggtcctggccgaccagttcgagcaagtgaccgccaccggccccaacgaggtgactttccgcctgacctcgcccaatgccgacctgcccgtgatcctgggcacctaccacttccacatcgtcaaggaaggcacgaccgacttcagtgccggcatcggcaccggcccctacaaggtcaaggagttcaagcccggcgtgcgctccatcgccgtgcgcaacgagaactactggaagccgaaccgcccgtatctggacgagatcgagttcttggccatcaccgatgagtcggcgcgcgtcaacgcgctgctgggcggccagctggacttgatcagcgcggtcgacccgcgctcggtcgaacgcgtgaaggccaccggccagcacgcgatcttcgagtccaaggcggtctcgtacacggacttgatcatgcgcatcgatcgcagcccgggctccaacccggatttcgtgctggccatgaagcacctgttcaatcgcgagcagatgctcaagaccatcgcgcagggctatggcgtggtggccaacgaccaacccatcggcccggccaaccgcttccacttcaagggcctgccgcagcgcgcgcacgatcccgagaaggccaagtggcaccttcaaaaggccaacctgggcagcgcacccgtgccggtggtggtctcgcccgccgcggccaactcggtggaaatgacgctgctgctgcagcaggcggcccagcagatcggactgaatctggaagtcaagcgcatgcctgccgacggctactggtcgacgcactggatgaagcacccggtaggcttcggcaacgtcaacacgcgccccagcgccgacctggcgttgaccttgttcttcaagtccgatgcgccctggaacgaagcggcctggaagaacgagaagttcgaccagctgctggtggccgcgcgcggcgaaaccgacgcggccaagcgcacccagatgtatgcggacatgcaggtgatgatccacaacgagggcggcatcgggatcccgatgttcctctccagcatcgatgggcacgccagcaagctcaagggcctgtcgcagattccactcggcgggatgatgggctccagcttcgccgaacacgtctggctggaagcatgactttctcgcgcagcgaggtccccgcactggtcggcccttgacgggtgaatcgcaaggtggcctgcagcctttggaaatcagccaccttgccgaaaactaaggcaaccttagtgtgagcaggtacgggttctgggccactgccacccccgaacagcaccactcaaaaatgccagaccccctgcggattgacaaagaaactgcttgggttccgctgcgatatggcatcacctgcaaagggggcagtcctagacttgtttcacctcaacgcagcaggtctaccatgatcttcaaccccaaattcatcagcttcgactgctatggcacgctcatcaacttcgagatgggccccacggcaaaagtcctgttcaaggaccgcgtaccggccgaacggatgccggcgttcctggacagtttccgagcctatcgcctcgatgaggtgctgggcgactggaagcctttttacgacgtggtggagaactccatccaacgtgcctgcaaggcgcacggcatcgaatgcctggcatcggatgctgcctccctgtatggcgccgtgccgacctggcagccgcacccgaacgtggtcgaggtgttggaggcgatcgcgccacacgtgccgctggtgatcctgtcgaactcgatggtcgacctcatccctcacagcgtcgcgcacctcaaggctccttttcacgcggtctacaccgccgaggaagcgcgcgcgtacaagccgcgcatgcaagccttcgagcacatgttcgaccggctcggctgcgggcccgatcagatgatgcatgtctcgtcgagcttccgatacgacctgatgacggcgtccgacctgggcttcatggccaaggccttcatcgaccggggtcacgagcccacgtcgaccgaatatggcgtgagccgcctgaccgacgttcgtcagcttcccgcattgctcggactctgatgttcagccctgacccccacccggaacctcagagggcgatgcctgacgaacgcccgagcgaggttgccgcgctgagcaccgcggcgcccaacctggcgccagccgaggtgcaggcactggtggcgcgcctctacggcatcgacggcagcgtgaaggcgctggccagcgagcgtgatcagaactgcgccgtcgagtccgctgacggcacgcgctacgtgttcaagatcagcaactcgtcagagccggtgtcgctggtcgatttccagatcgccgcacttgagcacatcgcccgcgcatcgcccaaccagcccgtcccccgcgtcgtgcgtacgcgggacggccgcgcgcatgacaccgtggcgctcgccgatggggccaggaccaccgtgcgcatgctcacctacctggagggcgtccagatccgggagacaccgcgcacggccgcacagcgcgcggcgatgggcaagggactggccgaactcaacctcgccctgcaaggcttcgcgcaccctgcggccacgcacgacctgctgtggaacgtgtcggccgcgcaccgcctgaccgcccagctcgacagcctggtcgaaggaccacgacgcgcactggcccagtcgttcatgacgcgcttcaccgagcatgtgctgccccgccttgcatcgctccgggcgcaggtgatccacaacgactatcacctctacaacgtgctggtggcgccggacgacccggcgcgcatcaccggcatcatcgacttcggcgacatgctccatgcgccactggtcggcgaggtggcgacggctgccgccttccacatgaccggcagcgccgacccgttcgagggagcggcgcaattcgtcggcgcctaccaggccgttctgccgctgaccgaaccggagcaggacatcgtcgccgacctcatggcgacgcgccacctcatcacggcgttgatctcggagtggcgcgccctgcgctatcccgaaaaccgcgcctacatcatgcgtcacaaccccgcggcatgggaggcgctgtcgcaaatggcagacctctcccgccacgaagcgcgcgaccgcttgctgaccctcacacgaaatggaagctcctcatgaaaaccaccgctgacttcaacatggtcaacgcctacatccccggccgcgccaacgtcggccccgccactgaggcaatgatcgcgcggcgcaatgcgctgctcggcccggcctaccggctgatgtacgaacaccccctgcacatcgtgcgcggcgacggcgtgtggctgctggacccggaaggccgccgctacctggacgtctacaacaacgtcacgtcgctcgggcactgccatcccgcagtgaccgaggcgatctgccgccaggtgcagactctggcgaccaacacgcgatacctgcacgacaccattctcgagttggccgagcgtctgatcgccagcgtgcccgggacggaccttgcccacctgatgctgacctgcaccggcagcgaggccaacgacctggcctatcgcatcgccaaggtgcgcaccggcggtacgggcgtgatcgtcaccgacacggcgtaccacggcatcaccgacaccgtgtcgcagttttcgccatcgctgggcgtgaccgtcgacctcggtccgcacgttcgcctggtgccggcgccgcggcagtaccacgccgaaggcgccgaccttggcgagcgcttcacgcgcgacgtcgagacggccatcgccgacctgcagcgccacggcatcaagccggcggccttgatcgtcgattcgctgttcacgagcgacggcatcctgcccgagcctgcgggcttcctgaagggagcggtcgaagcgatcaagcgcgctggcggcctgttcatcgccgacgaggtgcagcccggcttcggccgcaccggtgagcacatgtggggcttccagcgccacggcctcgttcccgacatcgtcactctgggcaagccgatgggcaacggccagccgatcgcgggcctcctcgccacagccgacgcattggcagagttcggcaagcactcgcgctacttcaacaccttcgccggcaacacggtttcatgcgcggcggccctggcggtgctggagaccatcgagcgggaacggttggtgccgcacgcagccaagatcggcaaattgctgctcgacggcatcaccgggctcgccgcaaagcacgaggccatcggcgacgtgcggggggcggggctcttcgtgggcgtcgagctcgtatcgaaccggtcgacgcgggcgccggaccgcggcctcaccagcaaggtcgtcaacctgatgcgcgacaagggcgtgctgctcagtgcctgcgcccaggggcacaacgtgctcaagatccgtccgccgctggtgctgtcggcggagcaggcgggcatggtgatcgaagcgctcgacgaatcgcttgccgaggcgcagcagcacatgccgccgacttgaccgtagcatggcgccatgagttcggcagttccgttcgacaggtttgacctcaagatcctcgtgcatctgcagcgcgagggacgctgctcgaacgtcgatctggcggcgtcgctcggcctcagccccagcccgtgtcttctgcgcaccaagcggctgcaggagtgtgggctgatccgcggctacggcgccgacatcgcgctggaaaagctgggggagcacgtcaccgtgttctcggaggtcaccatcagcagccaccgaccgcatgatttccgcaagttcgagcaagccgcctcgaagtacgaggagatcgtcgagtggtacaacgtcagcggcggctacgactacctgttgaaaatcgtggcgcccggcgtcggctattttcaggcgctgatggaaaagatgctggaagacgacatcggcatcgaacgcttcgccagccgcatcgtcctgcgccagtcgctggaacgccgcgggtatccgctgggcatcatcgcgactcaaaaacgttgggagtgatggaaggcccgcggcacgaccagcgccgatcgatcgttcagggctggaagcccgagcgccgcaccaccggctcccactgctggcgaaagctcttgagcatctgcgcggtctctgcctgcgtgctgacgatgggcgtgatgtaggccgtattggccgccttctgcagcgccgggtcctgcatcacgtcgcggatcgcggtggccagctgctgcaccttggccggcggcatcgcggccggggcgaagaaggtgttccagccgtcggcgtcgatcttcatgccggcctcgcggaaggtgggaatggcgggcgcgaagctcacgcgcttcttgcccgagacggccaggatgcggatcttgccggccacgtgctgcgcgtagagcgaatcgagcgtgtcgatggcgatcggcaggttgccgccggtcaggtcggccgacagcggcgccgatccgccgtagcccttgatctgcggctgcacgctgagcgcgtcgcccaccatcaggccgaagaagtgaggcaggctgccggtggcgggcacgccgaagacggcctcttccggatgcgcccagagccggcccacgaggaacatcgcgcggtcgagctgcagcttgttgcccacggccagcgcgaaatcgtagctgctgacctgcgacaccggcacgaagtccttgtcggggtcgtagcccagatccttgaacacgagcggcgccaccaccatgaccgcggggttgccgagcatcagcacgttctgtccggcaggcgcgcgcttgatctccttggcggccagccggccgccttcgcccggacggttttcgaccgtcaccgccacgccgagcctcgggccgaggcgctcggccacgaggcgcgcgatgcggtcggtgctgccgcccgcggtgtagccgaccaccagcgtgagcgggccatcgaagatcggcgtctgggcgtgggccaacggcgcggcgcacgcggcgagtgcgaggcaccatgcggtgagcttgcgccgggaaaagaatgcggtcatcggatctcctgcttgcggtggtggcatcgacacgggcgcgcgcaggccttcgcggcgacaatcgccggcctgcgtttgtttcagtccgtgtaatttgttaccgtttatacgcacgccataaacagttgatctaatccatcacttgcctgccgaggcgcgccggccacacccttttcaccgcttccgatttcctgacttcctatttccgatcgccatgcacggtccgcaagaaatgcccgcttttcccgacgccagcgcggtgcttgcgccgcgctcgctcgacgatctgctcctgtaccggttctcgcgcgcggtgcgcgcaagcaacggcatggccacgcgcctggtcgaaggcggcttcggcatcacgcggcgcgaatggggaatgatcgccacgctcgcgcagcagggcgagatccgctcctcggcgctggccgcgcacctgcacctggaccgcgtgcgcacttcgcgtggcttgcgcggcctggtcgacaagaagctggtggtgcgccgccaggacgccgaggaccggcgcgaagtgcacgtgcggctgagcccctcgggccggcagctcttcgaccgcgtgtttccgcgcatcgcggaactcaacgtcgacctgctcgagggcatcgcgcccgcgcacctcgacatctttttgcagtgcctgcaacacctcgaacagcgcggcaatgccttgagcgcgcagggcgcggtggccgagaaagccgaccggcgcgcgggcggcacgcggcaccggtggccggagtcgcgccaggtttagcgacgcgcgctcagcgcagatcgaacagcgcagccgcgttgccccacgcaatgcgccgcgccacatcgggcggcaggtcgccaagccaaacgcggtagccgcgcatgatctcgtcgtaggcgctccagcgctggttcacccaggtgtcggagccgatcatgaagcgctccggatacttgaggatcagcgcgcgccaatcggggcacagcctgccgccttcgcaggtgagccccggccggtacgagagttcgcccatcagcagcggatagcgttccagcaacgcctgcacccgctcgatgggtgcgccgccgatgccggtgtgcgcccagatgagccggaggttccggcccttcgacggtgcgttggccatgagcaggtcgatcgccacgtcgtccacatgcgcgagcaccgcgagcttctgccgctccgccagcgcgatcagcttcctggccaccggcccgttggcattggcactctcgtacaggtggaactcgccgatcccgcggtagggcccgctcgcggtgccgcgcgccagctcggccagcaccatctcgtgaatgctctcgtcgcggaaccagttgctgtagtcgtcgcggttgcggtacaggcgcacgaagggcaccacggtcacgcccgcggcgcgggtttcgcgcgccgcagccagcgtttgcgtgccggcattgggccgcgagttggccacgatcgccgtcacgttgttgcgctgcatgcgcgcgagcgcctcggcgggcggataaggcccggtgttgccgtcccaggcttcctggttgtagtgcaggtgcgtgtcgaacagcgggccgtcgtaggcctgcgggccttgtgcggcctggccatgggcaaggggcaccacggccaggcaggtggctgccaatacaaaggccgcgaggggcgcgatggctctcatgtgattgctgaagatgaaacgcatgtcgatcggtcgtctcattctggcccagtcctcgattcaacgcgagcgcgtctccgagcctcggtaggtcaaaacgcccagttcccttttcagcggcccggccgtgtaatagaaccgcgcaaccggctcccgcctccgcgccatggaacacgatatggaacccctcatcctcgcccgcgttcagttcggcttcacgatctcgttccacatcatctttccggcgctcaccatcgggctcgcgagctacctggccgtgctcgaaggcctgtggctgcgcaccggccgcaaggtgtacatcgacctgtaccagttctggatcaagatctttgccgtggcctttggcatgggcgtggtgtcgggcctggtgatggcctatcagttcggcaccaactggagcaacttctcgcgctttgccggtggcgtaaccgggcctctgctggcgtacgaggtgctgaccgcgttctttctcgaagcgggttttctcggcgtgatgctgttcggccgcgagcgcgtggggccgggcctgcacttcgtctcgacgctggccgtggccgttggcacgctggtctccgccacctggatcctcgcctcgaacagctggatgcaaacgccgcagggccacgagatcatcgatgggcgcgtggtgccggtcgactggttcaaggtgatcttcaatccgtccttcccctaccgcctggcgcacaccgtcacggcggcctaccttgcaacggcgctgatggtgggcggcgcggcggcctggcacctgctgcgcggcaacgacaacacgcgcgtgcgcaccatgctctcgatggccttgtggatgctgcttgcggcggcgccactgcaggcgctcatcggcgaccagcacggcctcaacacgctcgagcaccagcccgccaagctggccgcgatcgaaggccactgggagcgcacgccggagggcgaaggcgtgccgctgatccttttcggatggccggacatgaaggccgaggtcacgcgcttcgcgatcgagattccgcgcgcgggcagcctgctgcttgcgcacagctgggacgggcagattccggcgctcaaggacttcgcaccggaagaccggccgaactcggccatcgtgttctggaccttccgcgccatggtgggcctgggcgtgctgatgatcgcgctggccttctgggggctgtggctgcgccgggggcagcggttgttttcccagcgcgcgttcctgcgcctggccgtggcgctctcgcccgcgggcctcgtggccatcctggccggctggttcaccaccgagatcggccgccagccgtgggtcgtctacggcctgatgcgcacggccgatgcggtctcgccgcagcattcgacctcgcaggtcgggttcacgctcgcactgttcgtcatcgtgtacttcgtggtgttcggcgcaggcacggcctacgggctgcgcctgatcgccaagggccccacgggcgaccatggcgatccgcccgtgcatggagggcccggagaaccgcggcagcccatgcgcccgctttcagcggcaccggagtccgacgatgggcattgatcttcccctgatctgggccgtgatcatcctgttcggcatcatgatgtacgtggtgatggacggcttcgatctcggcatcggcatcctctttccgttcttgccggccaaggaagaccgcgacgtcatgatgaacaccgtggcgccggtgtgggatggcaacgagacctggctcgtgctcggcggggccggcctgctggcggcgtttccgctggcctatgcggtgatcctcagcgcgttctacctgccgctgatcctcatgctcgtggggctggtgtttcgcggcgttgcgttcgaattccgcttcaaggcgcgggaaggcaagcggcgctggtgggacgcggccttcatcggcggctcgttcaccgccacctttttccagggcgtgacgctgggcgcgtttctcaacggcctgaaggtggtggacggcaattttgccggcggctcgttcgactgggtctcgccgttctcgctcttcacgggcctcgcgctggttgcggcttacgcgctgctcggcgccacctggctcgtgatgaagaccgaaggccgtctgcagatgcgcatgcgcagcctggcacggcccctggcgtggctcatgctggccgtcatcattgcaatcagcatctggacgccgctcgcgcatgccgccattgcgcagcgctggttcagcctgcccaacctgctgtacttcgcgccggtgccgctgctcgtggcgcttgtggtgtacaagctcttgcaggcgctgcgcggcgacgggcacgcgtcacctttcgttctcacgctggccctgctctttctcggctacacgggcctgggcatcagcctgtggccgaacgtcattccgcccgacatttcgatctggcaggcggcagggcccgcgcagagcctgggctttgcgctggtgggcgcgctcctgatcattccgatcatcctgatgtacacggcctggagctactgggtttttcgcggcaaggtgcggcatggcgatggctaccactgacgacccacgcccaggcaggcgcaagtggttgcgccgcctcggctggctcgcggccatctggctcgcgagcgtgctttcgctttacctgctttccctggtgcttcgctttctcatgaacgcggtcggcctcggccgctgagccgcggcgatcccctgccacctacccaaggcgtcggcgccgtccgacaggaggtgcctcttgcaggcgcacgctgggaatatgcagaagtgcgccaccatgatttccagccgggtagaacgctgcggttccaaacaagccaaggaccatgaaaaaccggacggctcatgacgcgaccgtcaccctgaagttgccctcgagcgtgagcggccgcgtgctggtccaggcgcttcgaaacgccggcattcctgtcgatgcgattggcagcgtgacctcgggctatctcttcgtgcggaccacgggccgcttcggcaggcgggcaaatacctttcgatggtttgccgccggcagcaacgaggagtcggtcgccgcattcgccttgccgctcgccgaagaggacgccgagaaccattcggccgcgaacggcgggcaagcccccgctcttccggccacgcagcggcgcgtgcccacggccgtgacctacctgcgcgtatggaaggaactggagcaacacgcacgccgcgcggagtacgacctgcatgcgaaacgaatcgcctactttcgcgatctcgggccgccgcccgatgccgtcgaccgggagttggtgaatcgcgcgtgggccactgcgaaccagtgtctcgcggccgcgaccgacgagatgagctaccgggcttccgaaaccgaatcgccggtaggtcccctcgggttttcggcacggggtgtcgctgcaaccgatagcgattcgcactgactctccgcctatagaacttttcatgtaaacactcgcgcgtcccgcgcgagatcaacggttttgctgcagggatatcccgcatggaatgagtcggctgcgacaatccatcgagggtctaatgagttccactgctcagtccgaacaaaccgtatggcatgaaaaaatctctcctgaggcttgtcacggcatggggctttgcagcgctcgcaccggcggcgcacgccgagcccgtcgtgttgtcgctggtgcacgccgccaccacctcgcacccggcgcatgtggcggcacttcagttcgcaaagcgcgtcgaagagcgcacgcgcggacaggtcagcgtcgagatctttcccgcgtctcaactcggcagcgagaacgaactgctgcagaaagtcaggctcggcgcggtcgacatggacgtgacctcgatgaactatctcatcaagtacgagaaaacgttctccgttgtcattcttccgtatctcttcgacagctatgcgcacgcacaccgcgtgctcgatggcccggcgatgaagtggctcgcaccgcttgccgagaagcagggcttcatcattctgtccaactgggaatggggattccgcaatctcaccaacaacaagcgcccggttaacgtgcctgaagacgtgcgaggcctcaaggtgcgcgttccgcccgtcgccgaactcgaggccaccatggaagcgctgggtgcccaggtcagcaaggtcggcttcaaggaacttcccctggcgctgtcccagggcgtggtcgacggccaggagaacccgatcaacgtcatctactacaacaagctgtacgagacccagaagcacctcgccttgacgcgccacgtgtactacaacacgctccacctcatgagcaccgcgagttgggccaagctcacgccggcgcagcaagcgatcgtgcgcgaagaaagcaaggcggcaggcgacggcatgcgcaagaagatcatcgccgaggaagagcagctcatcgccaggatggcctccgccggagtgaaggtcacgcggcccgaccccgcgccgtttcgcgccgccacgcaaagcgcccgcgcggagattgcgcgctttgccggcgaagagaacgtgcgcacgtttttgaagatggtcgatgcagagcgaaagcagtgatgcacctcgccagcgaagatccgcgggtcggcggccgcaattgagcgcattcctggccggcttctcgtggtggaaaagacctctcagcctgcgggcggagatcgccctcggcttcggcgtcgtcattgcgctgatgctcgcactgggcgttgccttctatctgagcgaacagcggtcctcggccgccatcgacaagttgctgaacagcgacaaccgaatggcggacctgagcttgcgcagttcgctcgcgatgcacaaggcacgcgaagccgaaagcgagctcctgctgtcggcggatcggctcggcgtggcggaggccagcacgcgttcgctgccggccatgcaaaaccatttgctggatatgcgcgagtacctggccagcctgcgaatcgtctcgaccgatccgcggttcagggaccaggtcgatcggatcgaggctcagacccggcaatacgagaacgggttcctcgcgttcatcaagcagcatggcaaggagggcaatctcggcgcggcacgcgcgtcccgccaaggctacgtcgatgcggcggttgccatcgagtcctccgtggaggcgctgcacaccgcggcgagcaagcgagcgcttcaaacgcgaagcgacgtcgcacgcgcagccagtttctcgcgctgggccgccatcgccatgattgcgttggcggctgtcatgggcgtcgtgatcgcacggatcgtctcgctgcgcatcacaggctccatcacgcagctcatcgccttctcccggcgcgttgcctcgggagacttcagcgcaagggcgcagcaggggcgcgacgatgaattcggcatcctcgcaagagccatgaaccagatggccgagtcgatcgagaattccaacgtgctgctggagagcagcgccgacaccctgaagcaccaggccacgcacgatgcattgacggggctcccgaaccgcgcgctgctggaagatcggctcaagcaggccatttcgtacgccgatcgatacgggcggctgatgacggtggtgttcatcaatctcgatgggttcaagctggtcaacgacagcctgggccgcaaggccggcgacgatttgctgaaggtcatggccggacgcatgagccagtgccttcgcagcgtggacacggtggtgcgaacgggcggcgacgagttcgtgatcgtgctgtacgaccagccgggagacggggcagagatcgctccggcactgcgaaggctgctcgaggccattgcgtggccgatccagatcggcggccaggcggtccaggtcacggccagcatgggcgtggccacctatcccgcggatggcgccgacgccgacgccttggtcatgaatgccgatgccgcgatgtcccgtgccaaggcctcggggcgcaacaccttccggttctatgcgtccgagatgaacggcacggtccgcgacaaactcgcaatgcgcgaagggttgcgcaacgccatcgcccggggcgagtttcacctcgtataccagccgcagctggagatgagttcgggccaggtgatcggcgcggaggcattgatccgttggaaccaccccgagcgtggcttgatatcgccggcagacttcatccccctggccgaagagacggggctcatcgttcccatcggcgaatgggtgctgcgcgccgcctgcttccagaacaaggcctggcagcatgcgggcctgcccgccttcgccgtctcggtcaatgtgtccgcgcggcagttcagggagaggaccttgatcgagcaggtcgcccgggcgctcgcggaaagcgggctcgaagcccggtttctcgaactcgagttgaccgaaagcctggtgatggaagatctcgaaagcgccctgctgtcgatgaaggcgctgcagggaatgggcgtgcagctctccatggacgattttggaaccggctattcgagcctgagcgccatcaagcgctttccgatcgcgcggctgaagatcgatcgggccttcgtgcgtgacattccggaagacgaagaagacaaggcgatcgccaaggccatcatttcgctggggcacgaactcaatctgaaggtcattgcggaaggcgtcgagaccgaagagcagctgcagttcctgctcgccaacggctgtgacgagatgcagggctacctcttcagcccccctgtgtcacccaccgaactcgcagccttggtcaaaacatgctccggcactgcacacaggctgagcgcgctgcctgcgtcgatgcgcggctagccgccgaagcgcggcggcgctacaacccggaccgccagctcccgtgaaaaccgaacggcacgcggtggggcaagcgggcgaccgcaacgggtcccccgggcaggttcctggcatcgaacaccagcaggtcgctgcgcttttcgcgttcgcgccaagccacggcgagcagccatccatcgccctcggccgcatccgcggcgcgcggaacgaacaccggttcggacacgacgtcgccgtgcgcaagcgtgtgcatgctgcgctcgccggtatcgaagtcgaaacgggccagactgtcgtagagcacgctctccgaatcgtccctcgcgcgcgaggtcgcatggcaggtgtagaagccgtagcgattgcgccggccggtgtaccgctcatcgatgcgagggaactcggctgccaggtcgtccaaatattcgcgctggaaccccgtgcccttgccggccaggtcgaaggtccagcggcacaggcgcgcggccatggcctgggggtcgccggggcggccttcggaatcgggcagcccgggcgccgtgtccgactgcatcacataggccacgatggtgtcgccctcgtcccaggcattcatcacgtggaacacatggcaggcgtcggtatcgaaccagcgcagggtgtcggcggcgctgccgcggcgcatcacgcccacgtgcgtgcgcttggcggcatcccatgcgagcagcggcttgccacgcatggcgcgctccacgctgagcgtcagcggcgtgactggaaagagcgcatgtccgcaggtcaccatgaagtcgtgcgccatgctggcatgcggcgccttgaacgactggagttgcgtgacctcgcagtgcttgtccatcacgccatagagcatggtcggcgaacaggggccgtcgggtgagtacgcgaagaaatgcagttcgccgctctcggggtcgagcttcgggtgcgcggtgcagcgcgaggtcacgcggtcgccaaagctctggtgtcccttggaagccagcgtgagggcatcgagctcgaagggctgatgcgactcttcgagagcgaacagacggccgccgtgccacagcatgctggtgttggccgtgccgccgttccggccctgcgccagcgggtcgctggtggcggggttgccgaaggtgccaaacagcgcgcgtccggcttcatgctcgagctgccacttcggcgtgcgcacccagcggttgctgtacgacaccttgcccaggccgatgtggaaggcatgcaccatgccgtcgccggagaaccagtggtagttgtcgtcgcgcggtgcgtattgcgggctcgggccgacgcggtacaggctgcccgatagcccctgcggcagtgtgccttcgatgtcgagcgccgcgatgtcgtgctcctcggtcagaggcgcgtagttgccggtgaagaaatgcgcgttcgtcggtgtttctgcgttcacgtggagccttggttgattcaggaggacgatgcggcgtccaggtgcgcgacggcctgcccgacataggtggccaacgcctcgtcgatgcccgagccgagccgcagagcggcgtcctgacggaacgcttgctgcagcttcgcgtgcaacgcggcatcgccgccagccttggccagcgacagcgcctgccaacgcagcgccagcgcgcgcatggccgcgccgtgcgtgggtgcggcctccagcatctgctgccgaacgtcggcgatgagcgggggccacgcgtcggtttgggcaacgtagtgctggcgcagcgtggccatgtcgccggcgctgcagtacggcgcatagagttgcaggcgcgcgaacgccaacgcgtgcgagatgaaccggatgccgccgcggtccacgcctgtcagtgcgtgcagcgatggctcgttccagtgcatggtgtagagcttgatcagcaggccttcatcgccaccggcttcttcgagcagcatcgcaatccagcgctgtgccagggactgcgcctgcgggctctcgggcgatgcgccggccgcgaccaggctgtgcagccacgccgacaattcggcgcgctcaggcgccatcgcgtcggtgaatccgtcacgccgagtgttgagcgtgcgctgttcgtcgtcgctgaagtacttggcgcccgcgaccatgctttcgagcgccagcagccagtcgtcgatctccggctcttcgctggcctgcaactggccctgcactgaaagcagatgggttctcagtgccgatgcctgctggatttcgcggtcgagttgtgcgacctgtcgggccacgacttcggacatatcgccggccgggttgtccaagaggccttgtatgtccgccagcggcagatcgagccggcgcagcgcctggatgcggtagagccgcgccacgtctttgcggccgtacagccggtagccgccgctggatctttcggagggcaccagcagcgcgatgtcgtcgtagtggcgcaatgcgcgcactgtcagcccggtgcgccgggcgagttcaccaatcttcagaaacatgccttccctctcaagttgaaggcatcctagactctgccgcaacgagagggtcaagccctgcagcagggaatttgcaagcagggtatgaaaatggatttcgtcaggccggcgcgcgcttggccagctcgagcttggcgatggcgttgcggtgcacttcgtcgggcccgtcgacgatgcgcacggtgcgctggtgcgcataggcttcggcgagccagaagtcctggctcacgccggccgcgccatgcgcctggatcgcccagtcgagcaccttgcacgacatgttgggcgccaccaccttgatcatcgcgatctcggcgcgcgcttccttgttgcccacggtgtccatcttgtaggccgcattgagcgtgagcaggcgagcctggtccatcatgcagcgcgactcggcgatgcgctcgtgccagatcgattgctccgcgagcggacggccgaaggccacgcggctgcggagacgctcgcacatcagctccagcgcgcgctcggccgcgccgatggagcgcatgcaatggtgaatgcgccccgggccgagccgaccctgcgcgatctcgaaaccgcgcccttcgcccagcagaatgttggacgcgggcacgcgcacgtcttccagcagcacttccatatggccgtgcggggcgtcgtcgtagccgaacaccgagagatggcgcagcaccgtgatgcccttggtgtcgcgtggcaccagcaccatcgactgctgcgcatggcgcggcgcatcggggtcggtcttgcccatcacgatgaagatcttgcagcgcgggctgcccgcgcccgaagagaaccacttgcggccgttgatcacgtactcgtcgccttcgcggcggatggtgcactggatgttggtggcgtccgacgacgcgacggcgggctcggtcatcagaaagcccgagcggatttcgccggccagcagcggcgccagccattcgtccttgtgcgcctcggtgccgtagcgctcgatggtttccatgttgccggtgtcgggcgccgagcagttgaacacctcgcccgaccacgagacgcggcccatcacctcgcacagcggcgcatagtcgagattggagatggccggcacgtcgcggtgcgggtggggcaggaacatgttccagaggccggccgcacgcgcagcgggcttcagttcctcgatcagcggcgagacctgccaggcattgccctggcggcggaaggcatccatctcgtggtggtagcgcgcttcgttcggatagatgtgctggtcgaagaacttgttcaggcgttcgagcagatcgcgggtcttggcggagggttcggcaaacatgaggcgtcctttttgcggggttgggcaattcaaacaccgcggactgttgcgagccgtctcgaaagtgacgcgcgccgcaccccctttttcaatgcccgggcgcgtccggcggcagcagcacgatcttgccgagggtgcttccgctgtcgagcagttcgtgcacgcggcgcgcatccgcgagcgcaaagcaggtggccgggggtgcatgcacgcggccttcggccatgagggcgatggcggcctgcatgagcccgcgccgctgcggcacgtcgtcgtccaccgaatggatcgagaaggtgcgcacggccaggctccggctcaagagcttgcgcagctcgccgaacacatcgccggccggcgggccgttcacgatgttgtaggagaccaccatgccgaacggcgccagcgcgcgcaggcaggcgatgaagagctcgccgccgagatgatcgaaggccaggtcgacgccgcgtccgttggtgagctgcatgaccttctccgccaagccgggcacgtcgctttcgacgatctcgtgcacgccgttggccagcgcgaagtcgcgcttctgcggcgtggaggcggtcccgatcacgcgcaggccgcggtcgcgcgcgacctgtgccagggccgtggccacgccgcccgctgcgccgggaaccaggatcgactgcgcgggcaggttgccgttgctcgacagcatggccagcgccagctggaaattgccgaggctcaccgcatcctcgaaacggatcgcgtcgggaagaacgaaaggcgcggcctcgggcacgcagatggcttcggcatagcagccgccgcgctgcgtcagttcacgcgcgctcacgagcacgcgctgcccgatctgcagcgccgtgacgccggggccgacggcatcgacgacgccggccatctcgttgccgggaatcgccggcatcggcggcatccacttgtaggtgccgttgcggatcagcacgtcggggccgccggcgccgatggccatggccttgacgcgcacctcgcctgtctgcggctgcggcagcggaagttccacctgttgcagaacatcagggccgccgggtgcctggagctggatcgccttcatcgtggtgtgcgtcatcagcgctgcccgtcgtgcacggacaccttgtccttggtgagcccgcccaggcgcgcatgcacccgtccgcccgtgcccatgaccagcgcgaacaggatctcgttcggccgcggcgcatcctgaatgccgatctccatcgagttgtagtggctgcgcacgtacgcggcgtggatgtagtgcagcggcaccatgagccggtagcccgtggcggccaccgccttggccgagggcacgatcgccttaggctcgccgagcacctcgcgcatggcccagcctccagcttcgtgccagaccgcgccgtgctccatctctccgttcacgccgacgatcgcggccttgctgtagacctcgaccttgtcgcgtccgagcacctcgaccagctccgtggccagcagcgtgccgagcgagcgcagctcggccatgaagggcatcaggtccggctcgtagcgccccgcataggggttgtggatgaccgcgcacgcggcggccagcctgagcggcgtggcggccggcggaccgccctcgtggtagatggtttcgatggaaaggctgcgcttgcggatgtcgatcagggacatggaggggtcctcactgtttgggtatgcgtgcatcgttcaccacggtggtccaccgcttgagctcggtggccaccatggcggtcatttcttcgggtgtgctgctgcgcgcttcgccgcccatttcttcgagccgcgcgcgcacggccggcacctgcagggccttgagcgtctcggcatgcaggcggtcgacgatggaccgcggcgtgcccgcgggcgccatgaagccggcccaggagcgcacgtcgtagccgggcacgccctgctcggccacggtcggcagctcgggcatctggctccagcgctgcgcgccggtggtcgccagcgcgcggagcttgccggccttgatgttggccagcacggccgtcggtggcgcaatgatcatcggcacttcgccgccgagcagcgccgcgaccgaggccgcatcgccgcggtacggaacgtgcagcagttcaacgttggcgctcttcaccagcagctcgccggcgaggtggtgcgtggagccgatgccggccgatccgtacgacacgccgcgcgcatcggcacgcgcagccgccaacatctcggccagcccgcggtagggcgagtcggcccgcaccaccagcaaaaacggaaagtaggtgatcgtcgagaccatctggaagtccgacacggtctggtagttgagcttgttgtagagcgcgccggccactgcatggccgcccgtggccagcagcagcgtatagccatcgggcttggcacgcgccaccgtgcccgaggcgatggtgccaccggcgccggtctgcgcctcgaccacgaagggctggcccagccccttggccatctccgtgctgaccacgcgcgcgatggtgtcggcattgccgccggccgcaaagccctggtagatcttgatcggcttgtccggaaagccttgggccaggccgtgaaggggtgctgcgcaggccagggccaggcctgcggcgacgagcaatcgtctgtgccacatggtttgtctccaatgattgtggaatgaaggccgcggcttgtgccgtcgcggtccggttccgcgctgcttcagtcctgctggacgatcgggttgcgcagcacgccgatgccttcgatctcgacctcgcacacgtcgcccggcttcatgaagcgcggcggcttcttgctccagcccacgccggccggcgtgccggtggcaatgacgtcgccgggcgcgagcgtgaagatggtcgacgagtagctgatgagcttcggaatgctgaagatcatgtggcccgtgtggctgctctgcaccacttcgccgttgagccgggtctcgagcttgagttcgcggccgggcgcgatctcgtcggccgtcaccatccagggaccgaagccgccggtcgattcgaagttcttgcccgatgcgatctgcttggcatggaactgccattcgcgcacgctgccgtcgttgtagcaggagtagcccgccacgtggtcgaaggcatccgcttccgcgatgttgcgtccgcccttgccgatgatgacggcgagctcgccttcccagtccaatgattccgacacgtgcggccgcacgatgggctggttgtgcgcgcactgcgagcgccacacgcgcaaaaatatcggcggctgctccgacagttcgcggtgcatgccggcggccagcacctcctggtggtggtccatgtagttgcgcaccgcgcacacgatcttctcggacttcggaataggcggaagaaaggtgatgtccgcaagcttggccgctatcggcagtccttcgacatgctgcgccgcctgcaggtattcgcccgaggcgatgtagtcgaccaggcccgcatgctgcggacgcgccttgccgagatcgaccacgccgtcgccgacgacggcgccccaggattcgcggccttgatggacatatgacaaaagcttcatgggaactccggttgggatgtgaggggtggaaaaaatggtggccgcgtcaggcggcaggtgtcactggtgtcactggcgcgcgcgattcgaactgcgcctgccactgcgcgagcggcatgaaagtgggatccttgcggcaggcctcctcggtctcgcgcatcagcgtctcgtcgtccttcgagagatcgagcggatcgccatgcggctgcgcgatgtagaacggcgtgtcgacgtagatctccaccgtgttgccttccggatcgagcatgtagaccgagagcgcgttgccgtggttgaggccgcggatgctggtggcgccgcgcgcctcggcccgcgccgaaatgtcgcgcaggtgctggatgctcggcaccacgaaggagatctgcatcacggtgctgaacttcgcctccggcggccggcccgacgccagcaccagttggtggtgctggtctgggctggcgctggtgaacaccagctggttcttgaaggtgcggccttcgccgcgatcggtgatcgtgaggtcgaaggtctcggtgtagaaggccaccatccggtccaggtcggtgacgaagatgccgaaatgcgaaggcgtgggtcgggcgaccttgagcatgctgtctccagggtgaggggcggggctgcgcgtccctaggttggtgcggcttcggcggccctgagcgcggccagcacgttgcgctgcgtgctcaggatgtgttcctcgagcagcgcgcaggccgtgtccgtgtcgcggcgcaaagtggcgtccatgatcttgcggtgctcgttcgatttgcggcgtgcggtcttcctgtggcgggcggaaaaccgccggtagcgctcggcctggtcgaacaggctcgcgccccacacgcgctggcgcagcgaggggcaggcggccagcagcgaaagatgaaaggcgcgatgcagctgtgaccagtcgttgtccagaatgacggggccgtcgctcaggcgcgactccaccttctcgagccggtggaacgcggccaggatcgcggcctcccaggcgtcgtcgccgtgggcaatggcctcgcgcagcgcaggcacgtcgagcatcacgcgcatgcgtgtgatgtccgccaggtcgtcctcggagatcggcgccacgcgaaagccgcggcgctcgtcggcacgcacaaggccttcttgcgccagccggctgagcgcctcgcgcagcgggctgctcgagtagccgtaggcggtctggagctcatcgagcttgagcttggcgccggcctcgaaggtgccggccagcacgtcctgccgcaagcgggtgaaggcctgctcgaccagcggcggttcgtaggcgggggagatttcttgtttatgcatggaaatcattttatgcaccgcctctcataccgggccgcccgctcgcctggccccgacgagcacgaacagcatcgtcgcgggcttgtcgccgaggttgcgccatgcatgccggttgccgtgctgcacggcgacgtcgtgccgccgcagcagcacctgcacaccgtcgtcgagttcgagcgtgatctcgccttcgagcacgatgtcgtagtcgatgctgtcggtggtgtgcatgccggggtggtcgggctcgaaggtttcggccaggccgggaacgagacggccgcactcggcgccgaaggcggccgcgtcgaagtcggcgcgcatcatgaccgcgtcgggagggaagctgaccatcatgacgcgggtgccgcccgcggccggtgcgaaccctgcctcgcccgtgcggtcgcttgcagtgcccgcgcccacggtgtcggcggcctccgtcgcccacaacagcgccgcagcatggccgggcaaggtcgtgaactccgcgctgcgcggcgccgcgccgtccgaaagaacctgcgccttgccgttggcgcccgtacccgccaccacgcgtctgatcttcatggcgtgcctcaggggttgatgacgaagttgctgaagccgccgttgcggctcgcgatgcccgagatcgcctcgttgatgcggtcgagcggatagcacacgtgctcgaacaccgagaggtcgagcgtgccggcctcggccatgtcggccatgtcttgcccctcgccggcggtgaaccaggccgagccctcgatgctctgctgctcgtccatcatggtgtgcaggtccatgcccaccatgcccgcaatggcaccgatgttgaaggcgcggccgccgcgcttcaatgcgcgcacgccctgttggaaggtttcgtgcggcgcgccggggcccagcgcatcgatgaaggtgtccacgcccaggccgtccgtgcgggccttggcccatgcgtcgatcgcctcgccgtcggcattggaaaaaacctcgatgcgatcgggggccagcgccttgacgcgctccagcaactcgcggttgcgcccggtgcccaggatgcgcgtggcgcccatggccagcccgaagagcgcaccgccgaggcccagcgtgccgctgatgccgttgatgagcacgctgcggccggggccgaccttcgccttgcgcatcgccgagtacatggtgcccaggtagccgaagcgcgccgcctggttgaagctcacgttgtcgggcagcttcaccagcgcgtactgcggagcgatcatgtattcgcacaggccgccgtacggatagttcttgtacagcttgagcgagttctgcgagaagccgaagtagccgctgaacgcgtagtgcgtgcagttgatgagatcgccgttgcggcaggcgcggcagccgccgcaataaaggctggggttcacgtagacgcggtcgcccggcttccaggtgtgcacgtgcgagccgaccgccgtcacctcgccggccgggtccagcccgaagaccgcgggcagcggcggcagcggcagctccggaaaccaggtcgtccagttggccaggatgttgcccaggttgggcacgatgccgcaggcgcgcacccgcacctgcacgtcattggcggcgggctggggaatcgggagttgctcgacctccatcggggcgccgaccttgtgcagtcgggcggctttcatcgtcgtcatggttgtctccttgctgatgggtttagatgcacaaaagcgtgttttatgcattcttttcgaccaagcggcacggcgccatcggggacaacccttggtgcacggaaccttgttttatgcacaattctagcttcatgcattcaaaagacaccatgctccaacacgacctggaacccgtcgacgtggcggtcatcggcttcggccccgtcggcgcgacgctcgccgcgttgctcggccggcgcggcctgcgcgttgcggtcttcgacaagtcgcagcagatctacccgctgccgcgcgccttcgcgctcgaccacgaggcgctgcgcgtgttccaggagatcggcatcgccggcacgctggcaccgcacatgacgccctaccgcccgacgatctaccaggggagcgacggagaacccatccagcacttcgacatggggccgtcgccctacccgctcgcgtgggcgccgtcgtacaccttcaaccagccggcgctcgaagcctcgctgcgcgaagccgtcggccaactgcccggcgtgtcgatccatctcgggcacgaggtgctgcagctcgaccagtcgccggaccatgcgctgctcggcgtccgccggcccgacggcaccgaggcgcagttgcgcgcgcgctatgtcgtcggctgcgacggcggcaccagccccacgcgcaagcagatgggcctgaagctcaagagcctcgacttcgacgagccctggatcgtggtcgacatgcacgtgaatgaagacaagctcgaccgcctgcctgccaccaatgtccagtactgccatccgtcgcggccctgcacctacgtggtgggccccggcacgcatcggcgctgggagttcctgctgctgcccgacgaggccgagcagcgcgagatgccgcacgagtccatatggaagctgcttgccccgtggctcaagcccgaggacgcccgcatctggcgtgcggcaacctaccgtttccacgtggtggttctcacgcaatggcgcaacgggcgcgtgctgctggcaggggacagcgcgcaccagatgccgcccttcctggcgcagggcatgtgccagggcctgcgcgatgcggtcaacctggcgtggaaacttcaatgggtgctcgaggaacgcgcgcccgatagcctgctggacagctatggcgacgagcgcgggccgcaggtcgaggaggtgacggcaaccgtcaagcgcctgggccagatcatctgcgagcgcgatccggtgcgcgccgcggagcgtgaccgccgactgcgcgagcagcaaggcggccaggtgcgcatgcagctgcgccagagcctgctgcccggcgtgcaccacggattgatcgaccgcgacgagttgcccgcgggcacccccttcccccaggccatcggatcgatcgaggccggcgcggcgccgcagatgatgggcgacctgctgccgcacggctttctgctggtgctgcgccatgcgcccgatgcggccgcgctgcgtgccttgcgcgaaccggcggccgcccttgacgcgcagctgctgtgcatcgatgccgcggccgcggtgtccggcatcgcgacactggccgaagccgacggcattcttgcggcgtggttcgagcgccaccagtgcgaggccgcgctcgtgcggccggaccacctggtctacggcgtggcgcgcggcgctggggaagtcgaggctctgatgcggcgggcctgcagcactctcggcgccacgctgattcgctccgccaccgctctccgggaaccgacatgaccgagactgctttcaccaccccttcgctttccggcaccgaggcgctgctgctcgatctcgaggcagagcgatgcgacgccatgaagcgcgccgactttgcgcggctgcgcgagatcctccatccggcactcacgcatgtccatgccaagggccagatcgacgactacgaaagctacttccgctcgggcggcacgcacgtcgactatcggcagatcgaccgttcggaactgacagtgcgggtgctcggcagcaccgcgctcatgaccggccggcagctgctggtggccgtgcgcaaggacggcagcggcaccgtgcgcatcgactcgcgcgtgatgcaggtctggaccgaacacgagggccgctggcggcaactggcgttccagaccacgccgctggccatgagcgtgacgtgaacgcatggcggcgcgctgtttcgcgcgcctcggcatgcccggtttccttcttcacacgcccgcgggttgtcgttgcatctcgaccagcgcgcgcagcgcggccaggtaggacaatggacccagcccctggaccgtgcccctgacggccggcgagatgatcgaatgcgcgcgccaggcctcgcgcgcggcgatgttcgacatgtggacctcgatggtgggaaacggcatcgccttgatcgcgtcgtgcagcggaacgccatgctgcgtgaggccggccgggttgacgagcgcaccctgcgcgtcgtcgatgtgcgcatgcagaaagtcgatcaagtcgccttcgtggttcgactggatcgtgtccagcctcacgccgagttcgtccgcgagcttttgcagccgcgcgtcgatctcggccagcgtggtcgtgccgtagatgtggggttcgcggcggccgaacaggttgaggttggggccgtgcaggacgaggatcttcatgggcgggcttccgtggctgctgctcatttgcgaatgcgcgcaagctcgtcgccgtagagcttgacgatggcggggtcgtagctggcggcaaagcggtcgaccaccggcttggcgatctgccgcatgcgcgcctgctcggccggcgcgagctcgttgaattgcgcgcccttggcctggagctcgcccacggccctttgcgcggcggcgcggctcacctgccgctgatagccgcgcgattcgtccgcggcctcgcgcatcatcttctgctcggtgggactcagcgagtcccagaacttcttgctgaccagcacgatgttcgccgcatacacgtggttggtggcgctcacgaacttctgcacttcgaagaacttgttcgaaaggatcaccgagtacgggttctcctggccgtccaccgccttcgactcgagcgcgccatagagctcggcaaacggcatcggcaccgggttggccttgaaggacttgaaggtctccaggaacaccgggttcggaatcacgcggatcttcagtccttcgaggtcctcgggcttcgtgatcgggcgcttgctgttcgtcacgttgcgaaagcccaggtcccagtagccgagcgcgaccaggcccttctccggcagcctggcaatcagcgcctgcccgagcgggccgtcgagcagcgcatcggcctgtgcaaagttgcccaccgcgaacggaaagtcgaccaggccgaactccttcacgatgcccgcgagcgaggtggtggccggcgccgacatctgctgcacgccgccctgcagcgccgattgctgctgcatctcgttgcccagctgcgaggccgggaactcctgcaccttcatcttgccgccgctcttggccgcgagcagttcggcgaagcgcttcacgccaaagctcaccggatggtccgcattgttgaggtggccgaagcggatgacgcgctcctgcacgtcttgcgctagggcgggaacggccagtgcaaaggccaggccggcggcggccagggagcgatgaagctttctcaagatgatctccggcagaagtgatgcggcgcgatcttatgagcaaagtggaaactctttccactagtgaaaacacttggcaaaaacgctagagtggcgcctgcccaccccttcgaacgacatgaccgccatactcgaacgcagcttcaaggtgcttgagcacctcgccggccacccggagggccgcgccctctccgcgctctcggccgagctcgacatgcccctgagcgccacccatcgcctgctgagcgagctgatccgctgcggctacgttcgccaggaccagagccacggcgactacatgctgacgatcaagctcgtgtccctcggcctgagcttcctgagcaacagcggcatcgtggacgtggcgcagccgctgctcgaccgtctcgcggccgaagcgggcgaactggtgcggctcgcggtggtcgacggcgacgagctcaccttcgtcgccaaggcgcagggcgcgatgcgtggcctgcgctacgacccggacatgggcctctcggtgaacctgtcgtgcagctccgcgggccatgcgtggctgtcgaccatgaccgacgagcaggcgctgcagctcgtcgccaggcagggtttcggcaagcccgaagacttcggcccgaaggcacccaccagcgtcaaggcgctgctcgcctacctgcgcgcggcgcgcaagcgcggcttcgcgatgatcaacgaggtcttcgcgcccggcatgaccgccatggccgcccccgtgcgcggcggccacggcgcggtgatcggcgtcatcaccatcgccgggccgttggtgcgcctgacggaagagcgcatgctcgaactcgggcccgcccttctcgccacggcggaagatgtcgcgcacgccagcggcgcgtcggctctgttcaggcgcagggcctgaggctttgccttttgaaagctctccgaaagccggcgggggagtctaaagtgttcttgttaatggacatttttccctcttgacgtcaaaatgtggcgcatgaaggacaaaatccgactcccgatcgagctgggtcaagccatccaacgtgcgcgaaaggaaggccgtctgaaggcgaccgacatcgcctcgcgggcaggccgcgcgcgcaacgttctctatcgtctggaacgaggggaagacatcaccctcgcctcgcttttcgacatcttgcgcgccatggacctgacgatccgcctggagcgcctgggcatgccgacgcttgaggaggtcgcagaacgctttggacaggaagacgacgatgcttcctgaaaagatcaagcagctcgacgtcgagatcgccggcgagccggccggccaactgctcaagcactcggtctacgagttccgctatctcgacagccgcgcggagcagccctcggtcgcgctgctcatgccgccgacgcaaccgacgtatcaggacggcgatctcttcgccgtcatggatcagaacctgcccgagggtgacctgtaccttcgtctgcgggcgatgttccccaagcagcagctcacccagatgcacctgctcgcggtggtggggtcgaacggcatcggtcggctgggcttccggctgccgggaacagagcggcttgcggcgcctcggaccatcgaccgcaagaccttgctcgcaacccgctatacgcccgaggtgttcgacgacctcgtgcaggcgtacctcagcacaggtgccggcattgcaggtatgcagccgaagatcatggtgccggatcgggtcagcgttccagtgcccacgatcatcgtgaaggccgccgcagcgtcctatccgggcttgtcggccaacgagttcatgtgcctgacagcggccggccacgccggcatcgagacgcccacgttcgacctctcggacgacgggcaactgctccttgtcgaccggttcgacatttcggcggccgggtctcggatcggtttcgaggacatcgcggcgctgatgaaccttcgggtgcgcgacatccaatccgatcggaagtaccacggcagctaccagcgcatcgccgagctgatgcggtatctccaactgcccagtgagaatctcgagcgcttcttcgagcaggtggcgttcagcatcatggtgcgcaacggcgatggccacctcaagaactacggcttgctctacacctcgacggctgactgccgcctggcgccgatgttcgacgtggtgaccaccgcgatctaccggtacaggcgctatgaaggcggacccgagctcgaggaccgcacactggcgctgaagctcttcgccggcaagggccatacgaaagcgtacccgacgaccgaagagttgctcctgttcggcagcaaggtctgcggggtcgcaaagcccggactcgtactctcgcgaatcgccgagggaatgcacaagacgctggggcgggcggccagtgaccagcgcatcccgaaggatctgctgaacaagatgacggacatctggaccgacgggatgacttacgccaaggcgcagtagatcccccgatgtcgatgccgccgccccgcctagagcttcaggttcacctccacccgcgagtcgcccggcacggatcgcgcgaccaccacgatgcgctcttccagccgctggaaatgcaggtccacccgggcgtcgccgacccgcagctgccgcacgtgcagctggtcgatgtcggccggcagcctcgggtgcacgatggtcacctggcgccggatgccgtcgacctgcaggccgaggcaggcttgcagcagcatgaatgccgagcccgccgcccaggcctgcggcaggcaggccacgggatacgcgatcggcgattggccgggctggcggtcgaagccgcaaaacagttcgggcaggcgcatgccgaagtgcgcggcggactcgaacaggttgtccagaatgcgcaccacgccttcgcgttcgccatagcgcgccatgccggccgcgcacaacgcggcgtcgtgcggccataccgatccgttgtggtacgacatcgggttgaagcgcaccgcctcgacgggcaaggtgcggatgccccaccccgacgcgaaggccggcgatagcaactggcggcccacggccatggcccgttcgacgatcggcaggccggtgaacagcagatgtcccgcgttggaggcgcgcacgcggcagggctggttgcggccgtcgatggccagcgcatagaactgcaggtcgtcgagccagaagcgattctcgaccgcggcgcgcatgccggccgcacgctggcgccagtgcccggcaccggggtcgacgcgccactcggcaatcgccgccatcgcaagaaaggccgcatacacatagccttgcacctcgacgagtgcgatcggcccttcgggcgtgcggccgtcgatgtgaaagatggagtcgtggctgtccttccagccctggttgacgagcccgctggctgcgccgcgctggtaggcgagcaggccgtcggggtggcgcgccatgttccgctccatccactcgcaggctgcgagcagcgcgggccagatccggtcgatggtggcgtggtctgcggtgcgctgcgcataggcgcccgccagtgccacgaagagcggcgtggtgtcgaccccgccgtagtactgcccgaagggcagctcgtcgaccgcggccatctcgcccttgcgggtctcatgcatgatttttccgggctccgcgtctcggaagctcgaggtctggcgcgactgccgcgcagcaagaaactcgagcacgccctgcgccagcctggggtcgatccacagggtctggaaagccgtcacgatggcatcgcggccgaagggcgtcgagaaccacggaatgcccgcgtacggatagggaccggtgggcaggtcggtggtgagcaacgcgaggtcggcgcgcgagcggtcgagccacgcctgaaacaggcggcccgaactctccagccgcgaaccgcgccgctgccgcgcgcgcatgcgccatcgcgcgagcacgccggcctccctgaaccgttcggggccgggccgcgcgggctcggtgcccacttcgacgtagagcgtccactcgccgtgcgccgcgagcggcactctgaagttggcggtgccggcgtcgagatgctgcggcacctgcgagaagccgatgcaggcccgccgcagcaccgtgtcgagcccctcgtagcgcagctccacggcctgcgcgccgactaccggcgcatcgaactcgccgcgccgcgcgcgctgctggccgcgcacctcgaacatgtcgcggaagtcggcgccgaactgcagcgcgagcggcgcctctgcgggctggtcgctgtagttcacgagccgcagccgctcgaacagccgcgcgccccagagaaagcgcttgcgctcgagatggatcacgccctgcggcatcgatgtggagccgagcaccggcagcggacggttggtgaggtttgcggtgaagaacacgttgtcctggctgacgccgctggacagcagcgacggccgcgcgccgttcaagcgcagcacgaaggtcgagagcatgcgcgtgtcatggtgaaagagtccatccacgcccccgtccacgtcgccatgcgcatccatcacgaagtaggtgtccccctccttgagcacgaaggcatgctgcaccgcgcgttcggtcgccggctcggcctgttcggttgcaggcacttcctggctcatgctcacgccgcctcggggtagagttcgctctgcggcggaagcacgctgccgccgatgaggcgtgcgtacagctcgacataggcactggccatcgtatgcgccgagaaccgccgttcgaacacctgccgcacgcggccgcggtcgagcccacctgcggcatgcaccgcttcgacggcctgggctacgtcttcgacgatgaggccgctcacgccgtgctcgatcacttcgggcaccgagccgcagcgccatccgatcaccggcgttccgcaggccatggcctcgatcatcacgaggccgaagggttcgggccagtcgatcggaaagagcagcgcccgcgcaccgccgagaaacgcggccttgtcttcatcgccgatttcgccgatgaactcgaccagcgggttgtcgagcagcggccggatctcctgcgcgaaatagcgcgcatcgaccgcatcgaccttggccgcgatcctgagcggcatgccggccctcgtcgcgatctcgatggcgcggtcgggccgcttttcgggggagatgcgcccgaggaaggccaggtagctgccagggttcggctggaaggcatagggcgtctcgtcgagcccgtgcgaaatgttggcgaaccagttggcaaagggcagcggcttgcgctggtgccgcgagatcgaaaccagcgggtattgcttccagcgcatgtaggcaccgggcaggtcggcgatgtcgaggcggccatggagcgtggtgagggtacgggcggccatgtcctcgaagaaggggaagtgcagcagatcgacatggaaatgcagcacgtcgaattcgtccgctcgtcgccgcacctcgtgcagcatgttcaggtggctggccaggtcggacttcaggggcgcggggtccaggcgcagggcctgcgcccgcgtgggcgccagctgggcccgggtctgcgtgtccgcggaggcgaacagcgtgacctcgtggccctggtcgaccagcgcgttggccaggtgggcgacaacccgttcggtgccgccataaaaccgtggcggcacggcttcgtacaagggggcaatctgcgcgatcttcatcgtcaagacagtctcctcggaaggaaatgaatgaacagcgaagaagaatggaagcgtgcagcttccatgcgcccattttgggccgagcgttcccgaatgcaagggggacgatgtcagccgccgccgctacttgcacgcagccccggcttgttccggattttctcttgcgtgacagaaggttttgcggggcggcacggatcgcacggtgagtccgtgccgccgggcgcaggcggctgcccgctggctaccccaccgtatcgaaccccggcgcctgcgccatctcggaggccttgtagatcttgtgctgcgccgtggggccaagtgcgtcggagaccaccagcaggcgccagagcggttcgcgtgcggagcaggcgcgttcttcgctcgagagctggaacgcgggcaggcccgtggcggtgcccttcaccaccacccggagaagcgttgcccccttggcgttcgacacctcggtgtcgtagccgaggccttggctgctcaagtcctcggcgttgtagccgtagcccttgaagtggcgcatcacgtaggccagcgcggcgacttgcacgtcttcgcgcgagacctggccggatgctgcctggccctcggccgcggtgtcgggaacgctgcctcgggccctggaggccttgatttcggcttcgtcgggtatccatccccgcgggccgcgaatcagcaccgcgagcttttgggccggctcccagatcgcgacatgccattcgctctcgtcgcgcacccgtgtcgacaccttggcgcccttgttgctctcgagttcggcgatgggcacacggttcgtctgcacaacggcgcgaaagccctggcctgcatcgaaggtccgcttgagcagcgccaggcggtccttggcgcgctggatctgaaagggcgtgcgttcggcgccgtccggccgatgatgcgtgtccagcgactcgaggcagaaccagcgtcccccggcacccacgctcacgtattccgcccagatggtggcaatgacgttgtcgccggttgccagccaggcttggtcgaacggcttttcgcgcgcgtcgaacacgcccatcttggcgacgatttcgaccggcgtgagcctcggtcctgacaggcgcatctcgtcgatgacggcgagtacggggggatcgacttccttgtccatgcagcggggggttttggcgaattggggggtgggagtatgccgtatcggtggccgccttttggagatggctggccattcgcacacctgttacggcggccctacattgtttcgcctgccggagggtactcctcggcccaggcagaatccggcgaaggcttaccgcacatgaattccccgacccggctccccatcctccaactcgacgacgtaggctttgcctatccggagcagcccgcgctggcgtccggctggtgcgcctcggtgggcgaaggcgtcacgctgctctacggcgacacaggcaccggaaaatcgaccctgttgcgcgtgatcgcgggcacgctgcccgcttccggaaggctgacgctggcgggcgcgcgcctcgacgcggagcccgaagcctacaagcgcaacgtgttcttctgcgatccggccacggatgcgttcgacccgatcaccgcgcgtgcctgcacggctctgttgagcgagggcgacggcggcttcgacgcggcactctggcaaacgctggtcgagggcttttcacttcagccgcacatcgagaagccgatgtacatgctctcgaccggatcgaagcgcaaggtgtggctggccgccgcgctggcctcgggccggccgctggtgctgctggacgagcccgagggcgcgctcgacgcacgctccatcggctgcctctggaaaaccatcgggtcgctcgccgcacgccccggccatgccatcgtcattgcgagcagcgcgcgcctcgaacatgtgccgcagatcgcgctcgccggctgcatcgaactgccgcttgcctgagctcaccggcgccagatcttcctatgggcatcccgatagccgttgcctgaatcggagctgttcgccggtgcgccgtcaaaagctcaggccgcaagcacctgcaggttgccgacacccggcagcacgcgcagcgtggcggccagccgcaccgaatagtcgcggctgaagaccgtgctgacctcgatgtattcgcagcgcgcttcggccgtggtcagggtcagcacggcatagccgcgcttgctggtctcggcgtagcgcaggtcgtcgaccatgcgcttgaaggcatcggacagcaggtcgttggcgatcagcggcacggcccgctcgaagccgggggaggacaccgaggaggtaccgaattccacccccacccgctggcccgagggatcggtgaggttcccggcccaggcgttgtgcgtgtcgcccgccagcgagatcaggttcttgccctggctgcgcgccatggcaagcacggcgtcgcgcgcggccgggtagccgtcccacgcatcgaggttgtagggcaccttctgctgcgcgaccagggcgcgctgggtttcattgcgcgcggactccggcagcgccagcgccgcgaggtactcggtcagcttctcgaggctgaagtcggtcgcaatgctcaggggaatgtgcatgcgcatcatgagcacctgctggccgagcacctgccaggtgcagggcgatgcggcgatgcgtccggacagccagtccacctgcggctggcccagcagctgccgcgtgggcgcggaggcctcgccggccaggtattggctgagcgtgacctgcttgtcgcggccgatgaggcgggtgtcgagcatgtgcaccgatgccagcgtgccgatgtcgaacgagcggtagttccgcagcgggttggcggggtcgggcagccgcgtcggcagccactcatggtaggcctgcacggcagccgcgcgcctaacggcaaagctgccttcggtcgactcgtcgtggttctcggcgccgcccaaccacgcgttgtcggctacgtcgtggtcgtcccacacggcaatcatgggcagccgcgcatgcagggcacgaaggttgttgtcggtgcggtactgcgcgtggcgcaggcggtagtccgtgagcgtcaggatctcgtggtcggggaccgactcgcggtcgatggcaatggcgagctgcgaggcatagcctacccgcccgaattcgtagatgtagtcgcccaggtgcagcaccacgtcgatgtcggtgcgcttggcgatctcggcatagacgttgaagtagccgctcgggaagttggagcacgacaccaccgccagcttggcctgcgacacgccgcccaccggcagcgtcttggtgcggccgacgggcgagttctcgttgcccatggcaaagcgatagaaataggtgctggcagcctgcaggccgacgacgtccaccttgaccgtgtagtcgcgctcggggcccgtgctcgtggtgccgcgcgcaacgatgatgccgaagccttcgtcgctcgccacttcccagtcgacgttgatggtgcccggtgcgggcgccgtcacgcgcgtccagatgatcacgcggtcggacaacggatcgccgctggcgatgccatgcttgaacaccgagctcgaaccgtctggcggcctgccgcccccgaagcctccaccgaagccccctcctccgtgaccgcccccacccccgccgcaggcggtcagcccgatgccgccgcccgagaacatcgcgaacagcaccgcgctccgcaagagcgatcgtcgggtggtgcctgtcaggccttgctggggatcgatgccgccgtcgtgagcgatggggcttgcctggtcattcttcttgtcgtcgtcagtgcgcatggctgtctcctggtccgccgacggtgagacgcacggcacgcctcaatcccctttcgacgtcggcgccattgaatgtgaagactttggttttcgacgtaggcttgcgccgatgcccgcgtcagccggaagcgcacggcgcgcttcagatgcttctgcgccgcgccgtccgatcagcgcatcagtcgcattcctgaaagcgcttgcactcgggggcgacgtggatggacgtcaacgtgttctcaccatcgatgtgcttcgcggtgaacctcacccacgcgccttcggcgatgcccgcgagcagcgtgcggtccctcaccctgaatgcctgaaccgtgaacgggatcttggcccttggaatcaacttcagccggacgtaaagcttgccgtcggactcttccttgaaggaggtcaggcgcgcgtacgtggtcaccggcctcgccgcctcggcggcggtttcgacaggcttcgtttctgccgcgtgagcaggcgcccccatcaccgtggcaaggctcgacgcgaacacgagaatgaagcgcagcataggtgtggatgaagtgtgaggctgcccgattctgccaactgcaaccttcggcacagccaaagcctccgaagattaccggtggctggcgtcgtcaggcggccttgccgcgcaggcgagtatgaatgcgtgggcaccttccgggaggctgcggtctggaagaccaatcgctgcgtagcggctcaggagaaggtacttgtagtcccccgcctgccagacatgcttgattcgttcccaaggaatggccgccctggcatcgccgaaggtgatttcaactcctgcaggagtcagtgcaacttgccgaaccggatatttgcgcgccaagcgcctggcacttgccgggcgcgcgaagtaaaagatgaccgggctgactaccgaaaggaccaagaacacggaaaaaaagatggtgaaccatctttgggcgccaaggaggactgcaaatgcgactacagctgcaagaaacgccggaggcccaaaggtcgacaaccgaccaagctcaatcaaggagcgggcataaaacaatcgctccgcccgagcagcgccttcttcatcgtagtgggcttcgaaaacgaacacgacacctgtggacttgggttcgctgtccaggcttgaagggcttgaagggcttgaagggcttgaagtttgcatgagtccacacttcggcaatggcgctatccgccgatgcgaacaacaaaaacctcgccgtgtctcaaatggcctttgaaccaatccttgccaccctgcctcgcaatggcctgttggcaggagcagctcaagagagcaaggcgcaagcgttcgggatgccagttggtccaggtcgcacccagtaaaaggagctcaccgtcgaccccgaagttggcggcaatgggcgatcctttgccgacagtcagttgaagtgacgcatctgggcgtttgcgctccagcttcgtcggctgagggggattcgacgtcagttgcatctcgtattcagcctgcgcagcaaggtgctcttcggaatcagcagcgatatctgccaatggcgagtccgcttcatgaatgctcacaagcttcacgcacagctcgtcgccttcagccaggctcatttcttcgatccattgcacatgggattggcgttcgctcccaaggtctcgcatgcctccgatgcgtagcattgcaggatgctcgccatcgaccaagatgcttagatgcaacgaaataagaagcgcgtctgctgcccccgcaatcacaacgggcaggccattgcatcgaacttcaagtgcttgcataggattcgtgcactcttgtcccgactgtagccgttcgcataaccgaataccgtgagccgaagtggtgcccgagcattggtgtcccccttggtcagacgtcttcacgtccggccaaggcgcgcccgacaagcgcggacattgccgcagcgttctcggtcccctctgccgcaagtccggcgacggtcccttgcctgtcttgcaggtcttcgtcctggctcgccttgagcttgccaaccaggcggtcgatcggaatttctatgcccaccacggcacgcacgagcttgtcgatgaattctgctggtgcgtccgtcaccttccaaggcgattgctgtttggactcatggacagccgtgaggcgaaccagcaggtcgcgcagccacgcttcatcggtgatggcccgggcgacaccgtgcgcatgggcgactgcgtagttccaggtgggaaccaccttcccatgcgcctgcttgcccggataccagccaggcgtgatgtacgactgagggccttggaacatgaccaccgactgatccgaatcgggaagctgcctccatacgggattggcgcgcgagacatggccaagaagcgttccgaacttgccgcgagacctgtccagcagaaagggaacatggttggcgaccagtccttcgctgctgggcgcaacccacgcgccaaggggatgggcgtccatcagcgcctgggcttcggcgaggtcgggcagcacatggtgctttgatatgtacacaagaactccaagattcagtcaagtcgagggcgctgtcgcgagagggagtgcacctcctcgagcgccccggctattttgtcccctggaactcccgtctccccaacgaggcggcgaatcaactcatcaataagggccgatgctcttgacagtaccgtcgctctatgtcgagtggctagatgcaaacaggaggtacttaagactacattcaaaaaaccagaaagggccggctttcttgaccccgtcaagtgccggcaatgggaggatcgaatgccgctcttgttcttgatgagactgcagcacaccccgctgcccgtacgggtcgtccagccggaagagatccgccatgtctcggtgcttgtggccacgggcctgatagaggccgacatcgcacccctccatccgaccggcccctacgctgcatcgcgcatagcgacggtgaagcgcattacggaggacggtgctgccgaaatcgcgaagatgagcgatgcgcccaagcaggtgaaaacctcgatgcgattcgcacgggggcagcggctgatgtgatgagtctcggctctcggtttcagggcggcggaagagcgccaatctcgaagacgtcgccgtgtccaatgtgtttgcctgcgttccagatggatgcgatcggcctggcaaatctacaccgcgcggggcaactgcatctgcggcattgccaccacatcgcgaagcgaagtgaagcgtactgtgttggcttcgctcgccgatacagaagcatacgtcgagtgcttccaagggattgcattcccctgaagatccggcatcgcggcgaaccggccgcatgaccaggaatcatcatgccctccctcttcagaccccttgccatcgccgccgcgagcgccgtattctgtgccgcagcctgggcacaggccgcagacatcggccgtccgccggctgtcattccggtcgcgtcggaacctccgccaaggctcgtcgtgtatccgccgctggccgaaccgctggcacgcggagtcgtcatcgtgcagtaccggaccgagaacctgcgcatcatcccggtgttcggcaaggccgccgttgatgtatcgccgcgtgtcggccacctgcacgtcacggtcgatgaccggcccggcacctgggcccacaccagcggcgatccgatcatcgtcgtcggattgaagcctggcttgcacaagatgctgatcgagcttgccgatcccggccacaagatcctcggcagcgaaacggtctcggtgaatgttccggagccgaaggcttcggaagcccacgcacactgacagacaagctgccgccgggcggcctcccgcttactcgatcgtgaccttgccctccttcacgagcctggcgaacttcacggtctcttcacggatgcgggccgccatgtcggccgagctgtcgccgatggggtcggcgccaatcgcgcgcatcctctcgccgaattcgggcgacttgatgatcttgaccatctcggcgttcagcttcgccacgatgtccttcggcgtccccgccggtgccagcacgccaaaccaggtgccgatgtcgaagcccttgagcccggcttcttcgagggtcggcacatcgggcagcacggcggagcgcttggccgtggtgacggccagcgcgcgcagcttgccacccttgatgtgctgcagaacgggtgtgatggtgtcgaaggacatcgccacctgaccgccgagcaggtcggtggtgagcggaccgctgcccttgtacggcacgtgcagcaggttgacgccggtgctggcctggaactgggtgccgatgagatgctgcgccgtaccgttgccattggagccgtaggccagctccttgggcgatgacttggcaagcgcaaccagctcggcaaccgacttggccggcgtgagcgaagcgttgaccaccagcacgttcggcaccatcgccaccgtggtgatgggcgccaggtctttctggaagtcgtacggaagttttttatagacgctggtggcgatggtgtggtgcaccgcccccatcagcagcgtgtatccatccggcttggccttggcaacgtaatcggcgccgagcgtggcaccggcgcccggcttgctttccacgatcacaggttggccgaggctcttggacaacgcatcggcgagcgcgcgggccagcacgtcggtcgtgccacccgaagggaacggcaccaccaggctgatcggcttggccggccacggctcttgcgccgcggcccagggcgcgatggaaaatccgagagcggccatggcggctcccgccagggctcggcgcccgatggcgaatcgttggttcaacatgtcttgtctccaggttgacgggctgcgccgttcttctcgtggttcgatgcgtatccgctgctgctgagctctatgcggcctgccgctgccgctcggccgatgcgagctgcgtgcacacggcctgcgtgacctgtgcggtggtggcggtgccgccgaggtcccgcgtatggagcgcagggtcggccgtcacggcctcgacggccttcatgacgcgctgggcggcctcggcctcgcccagatgctccagcagcatcacgaccgaccagaaggtgcccaccgggttggccaggcccttgcccatgatgtcgaaggcagaaccgtgaatcggctcgaacatcgaggggtagcggcgctcgggatcgatgttgccggtcggcgcgatgcccaggctgcccgcaagcgcggcggccaggtcgctgaggatgtccgcatgcaggttggtggcgacgatggtgtcgagcgacgccgggcggttgatcatccgcgcggtcgatgcgtcgaccagttccttgtcccaggtgacgtcgggaaactccttggagatctgcagcgcgatctcgtcccacatcaccatggcatggcgctgcgcgttgctcttggtgatgacggtcaggagcttgcgggggcgtgactgcgccagccggaaggcgaagcgcatgatgcgttccacgccagcgcgcgtcatcatcgatacgtccgtcgcggcttcgatcggatggccctggtgcacgcggccgccgactccggcgtactcgccttcggagttctcgcgcacgatcacccagttgagatcgtccggtccgcagcgtttcagcggaccgtcgatgccgggcaggatgcgtgtcgggcgcacattggcgtactggtcgaagccctggcagatcttcaggcgcaagccccacagcgtgatgtggtcgggaatatgcggatcgcccgccgagccgaacaggatcgcgtccttgccgcgcagcgcgtcgaggccgtcgttgggcatcatcacgccgtgcttgcggaagtagtcgccgccccaatcgaagttctcgaactcgaacttgaagccactgccggccgcggccagggcttccagcacctgctggccggcgggcaccacttccttgccgatgccgtctccggggatggttgcgatcttgtacgtcttcatttgcggctgcgtcctgtgattgggtagggccgattctgtcggttgcacccgatcggatcgcaggggtaaagtgaatccatcattaacctcaggtcaacaatcttttcgatcatgagccacggcatccagccctccgaactgggcttcttcgtgcagattgccaccggcggcagcctgagcgccgcggcgcgcaacctgggtgtgtccacgccggcggtaagcaagcgcctgtcgcagatggagcagcggcttcgcatgccgctggtcaaccgcaccacgcgccgcatgagcctcactcccgagggcgaggtgttcctggaacatgcgcggcgcatcctcggggagctcgacgacctcgaccagctgctggccaaaggccggggatctccgaaaggcctgctgcgcgtgaatgcgaccctgggcttcggccgcatgcacgtggcgccggtgatctcgcgctacagccgcctctgccccgacgtcgaggtgcagctgcagttgtcggccgatccgccgccgctcacagacgatgccttcgacgtgtgcgtgcgctttggcgagccgccggacgccagggtgatcgcgaagcgcctggcgccgaaccggcggctgctgtgcgcctcgcccaagtacctgtcccagcgcggcatgccggtggtgcccagcgacctggcacgccacgactgcatcggcattcgccaaggcaacgatgcctacggcgtctggcggctgtcgagcggaaagggccgcaaggaacacaccgaggccgtcaaggtgcgcggcgcgctcaccaccaacgacggagagatcgcggtgcgctgggcactcgatggacacggcatcgtgatgcgcgccgagtgggacatcgagcgctatctggccagcggccgcctggtgcaggtgctgccgcagtaccgaacgcccagcgccgacatctacgcggtctatgcgcagcggcaccagctctcatcgcgcatcagggtgttcgtcgattgcctgtcggaagccttcgggcggctcggtgccggtactggagctagctgaggtcgaattgattcaggttgaccacggcctgcctcctcgacgagtattgaaggtggcgtcgccagatgatgatgatgatgccgtgccggcgagcctgcgacgccggcaattccggagacacggaaacacggagacaaacaatgagcaaactggtagccccggtgcaagccctgcgctggcgaatcgcgatcatggcggcggcactgcttgccggcctttccggctgtgcgcagatgcccgcttcgggcgccgcgcccgcggtggtcgagcagcttctcgtgcgcgagcgccaaccggcctttggaggcaccgctttcggcaatgccggcccctacgagcgcgtggtggcgcaagcccaggtggcgctcgatccggcgcatccggccaaccgcggcatcgtcgacgcgggagcggcggcatcggccgacggcaaggtccgctacaaggccgacgtcgtcatcctgcggccgcgcgacagcgccaggtcgtcgggaacgtgggtggtcgaagtcgcgaaccgcggccgcaagctgatgctcgagatcgtcaacggcggcggcctccagaccgaccgcgccgaagaagccggcacgggctggctgatgcgccagggccataccctgctgtgggtcggctggcagggcgacatcccggcggacgccaccggcaagaccgtcggcatggtgctgccaacagccatgcaaggcgggcaaccgatcaccggcgccgcgttcgaagagatcgtgttcgatgcgcccggcccgcgcggcaccttgcctttgagctacccggccgcctcgctcgatccggccatgggcgagctgagcgtgcgggcgcggcccgaagctgcgcccaccgcgatcggtgccgcgcattggcgctacaaggatgcgaacgcgatcgaattcgaacgccccgccggcttcgatgccggtgccatctaccagttcaggtacacggcacgcgacccgcgcccgatgggcctgggcatggcgtcgctgcgcgacgtcgtgtcgcacctgaagactggcctgcccgatgcgaacggccagccaagcccgctggccgacctgaagcccagggtcacggtggcgatcggcatctcgcaatcgggacgcttcctgcgcgactgggtgtggcagggattcaacgcggggccgcgcggacagcgcgtgttcgacggcatggtcgcgaccatcgccggttcgcgcaagacctacaccaacgtgcgctgggcgcagcccggccgctactcccgccagcatgaggaccacttcttctacggcgatcagtttccgttcagctacgcgaccacgaccgatccgctgagcggccggcagggcggcctgcttgcgcgctgcgctgtcgaccggacctgccccaaggtctttcagctcgacagcggcctcgagtactggcaaggccgcgccgcactggtcgtcaccgatggcgccggccgcgacatcgcgctgccagacgacgtgcgcgtgtacctcatgtcgtcgacgcagcacgtcaccgcgcgcaaccccacctcccccatctgcgagacgcccatcaacccggcgcagcagcagccggtgtaccgcgcactgctgacccgcatggtcgagtggtcacgcgacggcaaggccccaccggccagccgccatccgaccgtgcgcgacggcacgttggttccggcgactgccgcgtcgatgcggtttcccgatctgtcgccgctcggcgtgacgctgccgacgcccaaccttcttacggtgaacgatgacagcgcgatgcccgcaaggcccgacgccacgcgcgcatacacggtgctcgttcccaagaccgacgctgacggcaacgacgtggccggcatccgcctgcccgacgtcgccgtgccgctggccacctacaccggctggaaccggcgaaagaccggtttcgcgccgggccagttgtgcggcctcgacggcagctacctgcccttctcggcgaccgccaccgaggccgccgccaagcgcgacccgcggctcccgatcgccgaacggtaccccagccgcgaggcctacctggcgaaagtgaaaagcgcggtgcagcgtctgcaggcggacggcctgatgctcgacgaagacgccgcacgctggatggacaacgcagccaaggatgggcggattgcggtgctgccataacctttttttcttggaggtcccatgaattaccaaggtagctgccactgcggcaggatcgccttcgaggtcgagggtgacattcaaagtgcgatggcatgcaattgctcgatgtgccagcgcaggggatcgctgctgtggtttgtgccgcacgatcggctccggctcaagacgccgtccgaggacatgagcacctacatgttcaacaagcatgtgatctcgcaccgcttctgcgccgtctgcggcattcacaccttcggcgagggcaccgctcccaagggcaacaagatggcggccatcaacatccgatgcctcgagggcattgatctggatgcggtgccggtgcagcatttcgacgggcgatcgaagtaagtaagtgctacccggcgcgatgggccttgcctgccgctgcaaccgcgcaatcatgcgcacctgatccaacctaggagaaccaggatgaccagcaagaacacgatttgtctttggtacgacggcaccgcgctggacgccgcaaagttctacgccgatacgtttccggacagcgcggtgggcgctgtccatcgcgcgcccggcgactaccccgccggcaaagagggcgatatcctgaccgtcgagttcacggtcatgggtatcccttgtctcggcctgaatggggggccggcgttcaagcacaacgaggctttttcattccaggttgcgaccgacaaccaggccgagacggaccgcctgtggaacgcgatcatcggaaacggcggccaggaaagcgcgtgcggctggtgcaaggacaagtggggactgtcctggcagatcacgccacgggccctgatagaggcgatcgcagaccctgatccagcggctgccaaacgcgcgttcgaagccatgatggagatgacgaagatcgacatcgccgccatcgaggcggctcggcgcggctgacgctcgggcatgggctgtcgatggtcatcgaagcagccctcggaccctcgcctcttgaggtgcttgccgacaatccggtcgatgacctcagctgctgttccttgccatcaatgcatgagacaaggtcgtctgtgaaggtcagcgcgaacgtcgctggccggcatcatgaagtctgagacaccttcaccggaccgttcagctttccgagagccactgcacggagcgtcggagcgagtaccaaatcgcgcgtcatttgtgaactagttaatgaaatgagggctggagttaacaatggttaaccccaaccgggcccttgttacatatgctcgcgcgctcacgctcggcgctccggcacagagggcttgttcggcagaggccgtacttcctgatcttgttggtacagcgtctctacaccgcggcggcgggacccaccaggaagatcatgaacagagtttttcgcatcgtatggaacgatgctcttgcggcatggacagtcgtctcggagttgagcagaggtcacgcgaaggcaagcagcgctgccagtgcggcaggtgccgcggtggcccttgctttggcgaccttgtccatgcccgccgcggcagattgcgtggccgcgggcacagccatctcgtgcggcccgacaggcggaacacagggcacgacggtcggggccgggccagccacggctgacaacacctcggtggatgtccaacctggtgcattgatcagtacaggcaacacctccgcgatcagccttggcaacaatgccgtcatcacgattcgcggcggcgccacggtccagaacagttccgtcaacggcaacagccagtacccggggggcatcggcgccaataccgtcgagttcaacagcaacagcaccctcaccatcgagcagggcgccaacgtcttcgccgatggaaccgccggcaattcggaggccgtcaatcccgtcggtagcggcaacacgatcatcaatcacggcaccgtgcggtcgaccaatgcggcgatctggttccaggcgaactcgggcaacaacaccatcctgaacaccggcacgatggaagcgggctatgtggcgggcagcagcaaccctggcaccgcgacggtgttcggagccaacggcacctcggccgtcgatttcaccaacaagggcagcgtcatcggatcgctcaacttcgccaacggaaacgatgccttgcatgtcttcacgggctcgtcgatcaccggcaacatcaatggtggtggcggcaccaacctgctcacgctcaaaagcgaaaatggcgccgcatcgacctttgcgcccctctccctcgccggattccagacgctgcagagcaatgccggcatctggaccttcaatgtcgcgctgccgggctcgggcatcaccagcacgaccgtgaatggcggcaccctgatcctgggcgccaacgccagcacctacacgggcagcatgaatgtcgcaggcccgggcgttctgcaaagcaccgcggagttcgcgccccaggcgatcggcaatgcagggctcgtgcgcttcgcccagccgaccgacgcaacgtacaacgggcttgtcaccggttccggcggcatcgaaaagaccggcgcgggcgtcctcacgctgaccgcggaccaggctttcaccggtctcaccaccattaccgcgggaacgctgcagcttggcaacggcggcaccgccggctcggtgcaaggcaacatcgtcgacaacgcgacgctgaccgtgaaccgctcggacgcgctgacgctgtcgggcaccatcagtggaagcggcgcactcgtgcaggccggcgtgggcaccacgatcctcaccgccgacaacagctacaccggcggcaccaccatcaacgcgggtacgttgcagctcggcagtggcggcaccaccggcagcatcgtgggcgacgtggtgaacaacgcgacgctggtcgtcaaccgctcggatgcgctgacgctttcgggcaccatcagcggcacgggctcgctcgtgaagcaaggcgcgggcaccaccacgctgaccgcggccaacagctacagcggcggcacagcgctcaagcagggccgattgaacgtcggcaacagcctggcgctgggcaccggcacactggcaatggacgacggcaccacgctcggcttcgttgccgacggcctgaacctcgccaacgccattgagctgacgggcaacaacgatccgatcatcgacaccggcgccttcagcgaaacgctcagcggcaacatcagcggcggtggcttcatcaccaagctgggcagcggcacgctcacgctctcaggtaccaacacccacaccggcgcgaccaatgtggctgaaggcacgctccgggccggggccaccggctccttcagcgcggcctcggcgcacaccgtggcaagcggcgccacgctcgacctggccgggttcagccagacggtcgcttcgctggccaacagcggcacggtctcgacggtgggcagcgctccgggcaccaccctcactgtcaacggcgcctatgtgggcaacaacggcgtgctgcggctgggtactttcctgggcgacagctccagcgtgagcgaccggctggtgctcgatggtgcgagcgcctcggccagcggcaagaccagtgtgcagatcacccagctcggcggcctgggcgcgctgaccacaggcaacggcatcgaggtggtctcggcgctcaatggcgccacaaccaccgcgcagacgagcaaggacgctttcgccctgagcggcggccatgtcgacgcaggcgcctacgagtaccgcctgcatgcggcggacgcgagcggcgccggcgagaactggtacctgcgctcgacgaccacagtgacgacgcccaccaccacaccaacgacaggcacgggcggttcggcgggcggcaccgcaggcacgatcgccgtgcaggtgccgacctaccgtgccgaagtcccgctgctgtccgcgctgcccagcaagctgcgccagatggacctggccatgatcggcaacctgcaccagcgcatcggcgacgatgatgtcaggacggctggcgtcgcttcgagcggcagtgagcgccgggcctggggccgcgtgatcgccgccgacatcgacatccaccagcaaggcaccgtcaacccgcacagcaagggcaacgtcaagggcttccaggccggtaccgacctgttcgccacatcgaactggcgcgccggtgtgtacgtcggccagctcgacggccgcatccgggtcaacggcttcgcgagcggcatcgccgacttggccgtcggctccaacgacctgcgcagccagtacctgggcgcctacggcacctggaccgccgactcgggcttctacgcggacgccgtgctgcaggccggacggcaccgctacaccgcccaacccctgtcgacgctgcgcagcggaggcaagggcgacagcctgatggcgtccatcgaagtgggccagtcctttgcgttgggggcgagcggctggaagatcgagccgcagctgcaactgattcaccagcatctcgggctggacgacatcgcgatctccggtgcgcgcgtgcggcaggacagcgacgacggctggatcgggcgcatcggcgtgcgcctgaagggcgagatctccacgagcctcggcatgctgcagccttacggacgcttcaacgtctacaagacaagcggtggcgccgacctgacccgcttcatcggacccgctggcatggccgacatcaccggccgcaccggctccacctccagcgaactggccggcggcctcacgctggcgctgagccagacaaccagcgtctacggcgaagtcggcaagctctgggcctccggtggcgacgcaaaggtgaagagcacggtgcaaggctcgctggggctgcgcatgaagtggtgagccggtcgcttcgttgaccgaaccgcttggactccaagcggttcggttctcgcgggtcatcctttccatacggaccgcggaaaaatgcgctgtacatattctgaaaaatacgtatgatacgcatcatgccaaccgcaaagcacaacgccaggacagccgccaaggaggcctcgcacgagcgcatcgtgtccgcggctgcccgggcgatccgtcgcagcggctacgacggcactggtgtcgccgacatcatgaaggaggctggcctgacccacggcgccttctacgcccactttccgtcccgcgaggccatgctggccgaagcagcggcccgggcatgcgccgagacagccgccgcgaccgcgggcgtggttgccagcgtgccgcctgcgcaggccttgaactccatgctccgcacctatctgtcgcccgagcacctggcgcaggtggagctgggctgccccctggccgcgctgggctcggaaaccccgcgccaggcgccggacgtgcgccgcgtgaccactcggcacatcaaggaaatgatcgatttcgtcgcccgccaatcgccggactggggtcagcctgctgcccacgaacgcgcactcgtgaccgtcgccaccatggtgggcacgttgatgttggcgcgcgcggtcgacgaacccgcgctgtcggccagcctgtgcgaggcggcgctgaagcacctgcctccgcgctgaatccaggtcgcgaagcagcgccttttttctcgctcataaatatgatgatcatcatgcgacatgcaaaaaatggcgctttcatgccgaaccactaaccacccctcgccacaccggaacaaggaaagacatgaaatcactcaccttcaaacgctacggcaagtcgcccgggatcggcttcaccgacgttccccgtcccacgctgaagcccgacgaaatgctggttcaggtccacgctgcgagcgtgaacccgatcgacaacatgatcccgaccgggctcttcaaagccgtcttgaagttcgagtttccggctacgctgggcagcgacttggctggtgtggtgaccgaggtcggcagccgcgtaacccgcttcaagccaggcgatgccgtcttcgccaacatcttcgacttgggcaccggctcgatcgccgagttcgcggtggttccggagagcgctgccgcgctgaagccggccaacctggacttcgtgcaggccgcatcgatcccgatggtcgggatcacctcgtggcaagcgctgaaggaacgcgtcaatcttcgggccggccagaaggtgttcattccggcaggctccggcggcgtgggcacctttgcgatccagctggccaagcaccttggcgcccaggtgggaacgaccaccagcacgggcaacgtcgaactggtgcgcagccttggcgcagacgagatcgtcgactacaagaagcaggaattcgagaacgtgctgcgcggctacgacgcggtgcttggcacggtcaggggtgatgcgatggaaaagtccgtcggcatcctcaagtcgcggggcgccatggtctccctggtcgggccgctggacgcggcattcgctcgcgcccgacggctgaacttcgtcctgacgttcgtcttcgcaatgatgagccgaaagatcaagcgcctggcgaagaagcagggcgtcacctactcgtttctctttgcccgccccgatggcaatcaactcgccgagatcggcgaactcctcaaggccgagcgcatccggccggtgatcgacaaggtgtttccgttcgagcaagccaaggaagcacttgaatacctcgcccagggacgctccaggggcaaggtcgtcgtcaaggtgcgatagcggtattggtccccctcttttttatttggagattcccatgaagatcgaaaattccgtcgccctcgtcacgggcgccaatcgcggcatcggcctggcattcgcacgcgatctgctcgctcgcggtgcccgcaaggtctacgtgggtgcacgcgaccccgcgacggtcacgcaagctggtgtccaggccctgcgcctggacgtcaacaagccggaagacgtggcagccgccgcggcgctggcgaccgacgtgacgctggtgatcaacaacgcaggcattgcccagcccggcggctttctcgcggccgacagtgaagagatcgcacggcgcatcttcgagaccaacttcttcgccgtgctgcgcgtgagcaaggccttcgcgccgattctcaaggccaacggcggcggcgcgctgctcaacgtcctgtcggttgcctcatggatgaacggcggcgagctggccgcctactcggcgagcaagtccgccgcgtggtcgctcaccaatgcgctgcgcaccgaactgtcggcgcagaagacccaggtgctggggctgcacatggcctatgtcgacaccgacctcacgcgcgggttcgatgtgcccaagtcgagcgcggaggagatcgtcgcgcgcgcgctcgacgggctcgaagccggtgccgacgaggtgctggccgacgaaatcacccagcaggtcaagcgcgggatgacggcaccgcggcccagctacctgccgcaggcggcctgaaccgttcacgcatcccaggagctcatgcaatgcgtcattcgtccaaagccgccgcgctcgctctcgcgcttgcggcatccgccatttcgcagtcggccggggcagtcgatgctccggccgacggcgcgaagcctcgtgcgccggtgacggcccaggtgccgcgcgtcacctgggccaacgttcccacgcaatccatctccgcgggcggcatcgatttcgcgtaccgcgaattgggaacgcagaacggcggaacgcccgtggtgtttctggtccacctggctgccgtgctggacaactgggacccgcgcatcatggacggcattgcggccaggcaccacgtgattgccttcgacaaccgcggcgtcggggcgaccagcggatcgccgtccagttcgatggagcagatggcggatgacgccatcaccttcatcaaggcgaaggggttcgagcaggtcgacctcttcggcttctcgatgggaggaatgatcgcccaggagatcgtgctcaaggagccgcaactcgtgcgcaagatgattctcgcgggcacgggccccgcgggcggcgagggcatcagcacggtggcccgcattgcgaattacgacctgctgcgcggcttgttcaccggccaggatccgaagcaattcctgttcttcacccgcacgcccggcggcatcgaggcgggcaaggcctttctgcagcgattgaaggaacgtccggaaaatcgcgacaaggaaatcacgctcactgcctacatggcgcagttgcgggcgcttggggcctggggccggaaagaacccgccgacctttcggtggtgaagcaacccgtgctcgtcgccaacggtgacgacgaccggatggttcccacgtcgaactcgcacgacctggcgcggcggttgcccaacagcaccctggtcatctatcccgatgccggccacggcggcgtgtttcagtttcacgccgacttcgtgcccacggcgctcgaattcctcgcccgttaggactccgggacgcgttcccgccaaaggcaaggaaccaggcggatcgcttcagccggtcaagcgcgaggcgttccgggcacccccgccagtgccttgtccaacgcggcaactgcctccgcccgctgcgccgtggccgacgccgaccggtcgtgctggatgagcagcaccgcgaccatgccgatgaccgccggaatcgcgatggcgatgaagttctggtgcagcgggaggttcatgcccaccagcatgccgatcaggatgggggccaggatcgcgccactgcggccgacgcccaatgcccacccgaggccggtggcgcgcacggccatcggatagaactgcccggcataggcgttggccacgatctgcgtgccgatggtcgaggccccggccagcccgatgagaacgaagagcgccggcgtcggcatcttgtagcccagcagcgtgagcgaaacggctgccagcgcatacatccccgcgagcacgtacttgatgtggaagcggtcggcgagccacccgccgccgatggcgccaaccatggcgccgacattcagcaccaggacgaaggtcagtgccgagccgaggctgtagcccgcgctcgccatgagcttggtgagccacgaactcagcgcgaagaccatgaacaggcacatgaagaacgcgatccagaacatcaccgtgctgaagccgcggccgtcgtagaagaggtgcttgatcggcgcgctgtcggcccggtccttggccggcaccacgaagctgtcggtggccgacggttgatagctcgggtcgaggcgcgaggcgatcttcttgagttcttctgtgcggcccttggccagcaggaacggcatcgattcgggcaccgacttgagaatgagcggaatcaacagcactggcagcccggccgcgaagaagaccgattgccagccgtagctctcgatgagccctttgccgaggatcgccgcgatgatgcctccgacggcatagccgctgaacatcagcgtcacgagggtggaccggatcttcttcggtgaatattcagtcatctgcgccaccacgttcggcatcacgcccccgatgccgagcccggccaggaagcgcatcgcgctgaatgcgatgggactctcggccagccctgccgcagcggtgaagacgctgaacaagcccacgcagatgacgattgcccagcgccggccgatgcggtcggcaatggtgcccatgaagatggcgccgaacatcatgccgaagagcgcggagctgaccatgaacccggcattggtcgcgtcgacgcccatcttcttcatgatcgaaggcagtgcgatgccgaccaccgcgaggtcgtagccgtcgaacacgatgatgagcgcgcaccagagcagcaccagcccgtggaagcggttgaagcgggcatcgtcagccagcttgtgaaggtcgatttgacgcatgactcttgtctccgattcgaatggcaaagatgcctgtgcaccgccccgtctctcaacgggagttgcagagctgtgcggcgatgcttgcgatcatggtcttgccggctcggtgggtccaacgcattttccggatgccctttatgcggcctgtgaatgttggggcgggtctacccacaggtcgcgcccacccggcgcccgatgctgcccccatgtgatctccgaatgcgcgctatcaccgatctttgttggaccgtatccctccgctctcatagattgaccggcaggttgagcgccgttgtggcgctgccccgcaccaaggagacaggtatgcaaggaaagatcggcctcgaggaacatttcgcgattcctgaaacgctgcaggactcggccggcttcgtgcctggcgcgtattggaaggagctcagcatgcgcctgctcgaccttcatgacgtgcgcctgcgccagatggacgcgaacggcatggagatgatgatcctctcgctgaacgcgcccgcggtgcaggcggtgccggaccccaagaaagcgtatgagcttgcggtgcgcgccaacgactttcttgccgagcaggtggcgaagcggcccgaccgcttccaggccttcgccgccctgccgatgcaggaccccgacaaggccacgcaggaactcgagcgctgcatgaccgagctcggctttcgcggtgcgctggtcaatggcttctcgcaggtcggcacgcccgacaacgtcgtctactacgacgcgccgcagtacgcatcgttctgggccgcggccgagcggctcgacgcgcccttctatctgcatccgcgcaatccgctcgcgagctgggcgcagatctacgaaggtcacccatggctgctcggccccacatgggcctttgcacaggaaaccgccgttcacgcgctgcgcctgatggcaagcggcctcttcgatcggcatccgggtctcaagatcatcctcggccacctcggcgaagggctgccctacaacatgtggcgcgtcgatcatcgcaacgcctgggtcgaggcgcccaagacctatccggccaagcgcaagctgtgcgactacttcaatgaaaacttctacctcacgacatcgggcaacttccgcacccagacgctgatcgatgcgatgctggagatcggatcggaccggatcctgttctcgaccgattggccgttcgagaatgtcgaccatgcgtcgaactggttcaacgacgccagcatcagcgaggccgaccgcaagaagatcggacgcaccaacgcgttgtcgctgttcaagctgccgcaatcctgagccgccccggaaaggcaaggttgctaccaatgatcgacatcgacgagtggaccatcaccagcgccgcgctgaaggcgcaaggcgcaacgcccaacccgcgcctgaagaccgtgatggacagcctggtgcggcatctgcacgactttgcgcgcgaggtgcagctcaccgaagccgagtggtcccgcggcatcgactttctcacggccgtcggaaagatcaccgacgaaaagcgccaggagttcatcctgttgtccgacgtgctgggcctgtcgacgctcgtcaccgcccagtgcaaccggcgcccgacgggctgcaccgaggcgacggtgttcgggcccttctacgtgcccgacgcgccggagtacaagcacggcgacgacatctccaacggcgcgagcggcgaaccctgcttcgtcggcggaaccatccgcgggatcgatggcgagcgcatcgcccatgcaagcatcgacgtgtggcagtccgacgatgagggctggtacgacgtgcagcgccccgagctggaccatgcgcagggtcggggccatctggagagcctcgaagacgggcgctaccacttcaagtccatcgtggccgtgccctaccccattccccacgacggcccggtcggccagatgctggagcaactcgggcgccatccgtggcgtcccgcgcacctgcatttcatgatcaaggcgacgggctacgagacgctcatcacccatgtgttccgcgcgggcggcagctatctggaatcggacgccgtgttcggcgtgcgctcctcgctcatcgccgactggaagcgccacgagcccggcttcgctcccgacggcacgcgaatggaggtaccgttctacacactcgactacgacttcgtcttgaacagcgtgccgagggactagacgcatggaccgattcgtctacaccgcgagcgcttcgcgcatcgtcttcggcgccgacagcatcgaccagcttccggcggagatcgagcgcctgggtgcccggcgtgcgctcgttttgtgcacgcccaaccaacgcgggcaggccgaggccattgccgaccggcttcccggccgcgtcgcattcatcttcgacgaagcggccatgcacgtgccgatcgagatcgcgcgcaaggcgcgcgcactcgcctccgagttgaaggcggactgcgccctggccgtcggaggcggctccaccatcggtctcggcaaggccattgcgctggagtcggggctgcccatcattgcggtgccgacgacctatgcggggagcgaagtaacgcccatctacggcatcacggaaggcggcctcaagaagaccgggcgcgatccgcgcgtgcttccgagcgtggtggtctacgaccccaagctcacgctgtcgctgcccctggatctgacggtcacgagcgcgatcaatgccatggcgcacgcggcggagggcctctacgcccacgatggaaatcccgtagtcgcgttgatggccgaagagggaatccgcgcctgcgctgcgtcgctgcaaccgcttcgagacaacccgcacgatctgccggcacgcagcctggcgctctacggtgcctggctgtgcggcacggtgctgggggccgtgtcgatgggcctgcaccacaagctgtgccacaccctgggcggcaccttcgacttgccgcatgcgcaagtgcatacggtggttcttccgcatgcgctcaggtacaacgccggctcggcgccggaagccatggcccgcatcgcgagagcgctcggcgttgcggatgcgcccatggggttctttgaactggcaagaatgcatggcgcgccggtgtcgctgaagtcgatcggcatgcccgccaacgggcttgaaaaagcggccgagctggcggcgtcgaaccagtacccgaatccacggccgctggaaatagcggcgctgcgcgccttgctcgaccaagcatgggacggcgcgccaccaacgccctgatcacttgctccgcgtctgcgacacgggctcgcggctcgatcgctcgtgaaagagtccgaagatcagctcgcgcagccagcggttgccgctgtcctggtgaaaccgctcgtgccactgctggcgaatctcgaagggcctgacctcgaagggcgcttcgacgctgcgcaggtccgcgcgcgttgccaccatcgccttggcaaggcgtgccggcgcggtcagcagcaggcccgacgtggcgacgatcgacgtcaagcccagcgagtgggcggcggtgagaaccacccgccgccgatcgagcgcgcctgccctgtccagggtttgctgaagctgcgaatcggtcgttccctggggccggtacgcgatgtgttcggccgcgaggtagtcgtcgagctcgatgcgctcgcgcgcgcccagcggtgacgccttcgacatcagcaccacgaaggtctcgtcgaacagccgctgctggtagaacgaaggccccatcgattcccaactgccgagcgcgatgtcgatctgcccgtgcagcattcgctgccgggcatcggccatggaaacgtccacggtttcgaagcggacgccgggcgcgatgccgcgtgcgacggacagcagctcgggcatcatgaccagttgcccgatgtcgttgaccgcaatccggaacgtgcggctcgatgtctccggctcgaaggtccggccctggtcgacagcctgcgccaggcaggcgatgccttcctcgatgggcgcgatgagccgctcggcgacgggggtggggaccatcccgtccgccgtgcgcacgaacagcgcatcgttgaagcgttcgcgcatgcgcttgagcgcgttgctcaccgccgattgcgtcatgccgaggcggtcgcccgcgagcgtgacgctgcgcgtggcgtagatcgcctggaacaccaggaaaagattcaggtcaatggagttgatgttcaccgcgtcgcctccttcgccgagccgtcattcgttgtccaggactgccaggttgtcatagaccatccgaagcatgtcccggagggactcggcctgcgcggcagtcagcccggacaacgatacgcgctcgtacacctgggccaggggaatgatgcgcagcgtgagatcgcgtcccgcctcggtcaggctcagcgcgagcgcgcgggcatcctcgtccgaccggtcgcgcaccagcacgccgcgctgcagaagtccgtcgaccacgcgggagagcgtggaagggtccgtcgatgtgtgcagcgccaggtcggagagccgctgatgcgccttgtggtgcagcgcgacgcagacccgccattcggtcagcgagagcctgaactgcttgagttccttgctgaacgattgccccattcgcatacctgcgcgtgcaagcaggtacggaatggctcgctccagatcgtggtccggcaatttgtctgcaactacattcaatttagggggcacctcggtgcggattttccgtacctcccgaggctccgccgacggtgattttcttgtggccatgctgaatgctacaggcagattccgcagcggatatagcgtaaaccccaagcaattattagttgcgtttgcaagttttatggacttcaatcgaggccttcgctatcgcgttcccctcaaattatctggagaccaccatgactgaagccgcgaacccgtttgctcaactcaaccgcgtcgacctccccgctccggctcgaaagtcacccgtgaaggacgctccttcaatcgaaacaatagctgcatctgcaagcaatttggtgcccatgctgcgagagcgggcccaacgcaccgagcaggaccgccgcgtttccgaagaaaccacgcaggcattccacgatgcaggcttcttcaggctgatgcagcctgcacgctacggcggctacgagtacgggttcaccgcgttcatcgacgtggtcagcgaactggcgcggggctgcacgtcgtcgtcatggggctgctcgctgggcgccattcaccagtggctggtcgccatctttccggaagaggcgcaggacgacgtctggcgcaaggacccgagcgcgatcgtctgcggctcgtatgcgccggcaaccatggccgagaaagtcgatggcggctacctcgtgcaaggcaagtggctcttcgcgtccaacgtggacaactcgcagtgggcactgctgggcgttcagtttccgcccgaagaaaaaggcgccccgccgacggccggctttctgcttgcgccgcggtcggattgggccatcgaggacaactggcacgtggccggccaggcgggtacggggtccaaggcgatcgtcatcgacaagccgaccttcattccggggcaccgcaagctgaccttcgcggaggcttcgtccaacgccccgcccggcgccaaggtcaacgcaaatccgatctaccgcattccctttctttcggcggtgccggtttgccttgtgtcgcccatcatcggcaccgcgcaaggcgcggtcgacgagctgatcgagctggccggcacgcgggtcacccggggcgccgttgccggaggcggcagcaggctgagcgaattctttcccgtgcagtcgcgcctggccgaagcctcggccagcgtcgatgcggcgcggctcctgctctaccgggacaccgcacaggtggagcagatggccgtcgacggccacgtcatcagcgtcgagcagcgcatccgcaatcggcgcgaccatgcctttgccgcgcgactctcgcgcgatgccgtcgaggcggtgttcgccagcgtgggcggtgcgggcctgtcgctgaaccagccgatccagcgcatgtggcgcgacaccaatgcgatctctcgccacatcagcctcaactgggatgcggtgtcttcgatggtcgggcaatacctgctcggcctggagcccaagggccagtactgatcgggggcgccggccatgtactcctgggctctcatcacgggcgacgcggccgagtcggtcgatgcccgccaactgcgtcaggcgcttggcgcctttcccacgggggtgtgcctcgtgaccaccaccacgccggacggcaagcgcgagggcatgacgatcaactcgttcgcctcggtgtcgctggatccgccattgatcctgtggagcatccgcgacgacacgcgcagtgccgatgcgtttctcgcaacccggccgttcaacctcagcgtgctgaccgccgagcagcgcgacctggcctggcatttcgccaaaccggcggcggacaagttcgaacgttttgcaggagcgttcgagaccggttccaacggatgcgcgcggctcgtcgagagcgtcgcaaccttcgaatgctcgacctactcgcgccaccaggagggtgatcacaccatcatcctcggccgcgtggagcgcttctcccggacggacacgccgcctctgctctttcattcagggcagatggggtcgctgtgggagcttgccgaaaccctggcgcggccgcgctgaagccgtcgctcgctcaatgcctgtgccggccgacgtactcgatcaacgccttcagcttcgaaggctggtcgtgccggctcgggtagtagagatggaagcccggaaaggtcggtgagaaagccgtcagcacgcgcttcaaccgcttggcccggaggtggggacgggccagctgctcgaaggtgtaggccagcccgacgccttcgagcgcagcgtccaggccgaacatcgtgtcgctgagggtgaggttgcccgcgatgtcgtagtccaccagctggccgtccacctcgaactcccacttgtagatcgcccccgtggcggcaaagcgaaagcggatgcagttgtggcgcacgagatcatccgggtgccgaggcgccggcactcgctgcaggtactcgggcgaagccaccaccgcaacggcgacgggcccgccgatgggcacggccaccatgtcgcgatgaatgctctcgccaaagcggatgcccgcgtcgaatcccttctcgacgatatcgacgaaaccttcgtcattcgtcagctcgaggtgcacatgcgggttggcgcggagaaagccatccagcagagggcgcagtaccagcgcggttgaaacccgcgcggcattcagccgcaaggtgccggaaggccggccctggagagcgttcagctcgtcgcccgcatcgatgacctgcccgagtgccggaccgacacgcgccaggtaagcctcgcccgcttccgtgaggctcacgcttcgcgtggtccggttcaacaggcgcacgcccagtcgcgcctcgagttgccggatggcctggctcaatgcggagggcgacaccgccaggtccgcggcggccgcggtgaacccgccatgttccgcaaccttccagaacgccatcaatccgtcgagttggttcagcttcatactttgaagcttaacttcacacggtttgcagcattgccccatttttctttcagatgcatgttcgtacagtctgcgcacccacagcccacgaaagaccaaagacatggcaagagcacgcacaacgcgagccgcggccgagcgcaccacagccgttcggcattcccttgcggcgactctcgccgcagtggttgcgacctgcgcgggcatcgcatcgccgaccaacgccgcggccagccaggcgttagcgcagaagtacacatgcgtcgcgtgccatcaacccgcgacgaaaggggttggtccatcgtggcaggacatcggggcgaaatacggcgacggcaaaggaacggccgcgcaacttgcggccagcatcaaggccggcagctcgggcaagtggggttccatgccgatgcccccgcaagcgcaagttcccgatgcggatctgcaggcgctcgcgcagtggctcgctgatggcgccaggtagccgccgcatcgcttctgattttttctctctttctttcattcctcccaccttcggagatccgcccatgagcgcgctcaacgtcaacggccgaaaccacacagtcgacgccgaccccggcacccccatcctctgggccctgcgcgacacgctgggcatgaccggcaccaagttcggctgcggtgccgcgctgtgcggcgcctgcaccgtgcacctggacggccaggccatccgctcgtgcatcacgcccatctccgcggccgagggcaagaagatcgtcaccatcgaagccgcgaccgatggcagcgaccccatcggtgccgccgtgcacacggcatgggtcaagcatgacgtggcgcagtgcggctactgccagagcggccagatcatgagcgccacggcatttctcaagtcgcagcccaagggcaagcaacccaccgccgccgagatcgatggcgccatggccggcaacatctgccgctgcggtacctacgcacgcattcgcgccgcggtggccgatgccgcccgagccctcgcctgaaagagcacccaccatgttgcccacccacatcgaccccagcgaactgccgcgcgcgctgcagcgcctcatgaccgcgggccaatccgacgaagccgccacgctgccgcgccgcagcttcctgaagctagccggcgtcggcggcctggcgatcggcgcgtttccgcacctggccatggcacaggctgatggcgcggcaaagccggccggcgcgctcaagcccacgcagcaaccgctggccttcgtgcagatcgcggccaacggcgaagtcaccgtgacccacaaccggcttgaattcggccaaggggtgcaaacgggcctgccgatgatcctggccgaggagctcgatgccgactggagcctggtgcgcagcaaaagcggcaccaacgacccggcctaccacgatccgatcttcggcatgcacctaacgggcggctccaactcgatcaagaacagcttcacgcagtaccgcgagctcggcgcgcgcgcgcgggccatgctgctgtccgcggctgcggcgcgatggaaggtcgacgtggccacgctgcgcacgcaggccggcacggtgctgggcccgggcggccgcacgctgggctacggcgaactggccgaagcggcgatggcactgcccgtgcccgagaaggtcgcgctgaaggacccgaaggatttcaagatcatcggccgcccgaccacgcgcctcgatgcgcgcgccaagagcagcgggcgccaggacttcggcatcgacgtcaagcatccgggccagctcacggccgtggtcgcgcacccaccggtgttcggtgcgcgcctgaaatcggtcgatgacagcgcggcgcgtgccgtgaagggcgtgaaggccgtgctgcgcgtgccgctggaccgcggcgccgaaggcgtggccgtggtggccgacggctactggcccgccaagctcgggcgcgatgcgctgaagctgcaatgggacacggccgccgtcgagaaggtcgacagcgacaagcagctggcgcaatatcgcgaactggcctcgaagccgggtccgcgcaagttcgacgccgacatggcgccgctggccaaggcaccccatcagctcgaagccgagttcgtgttcccgtacctcgcccatgcgccgatggagccgctcaactgcacggtcaagctgtcgggcgaccgcgccgaactgtgggttggcacacagtccgcagggctggatgcggcggcggccgcacgcgtgctgggcctcaagcccgaacaagtgagagtgaatgtacagatggcgggcggtggcttcggccggcgcttcgtgggctcgagcgattacgtggtcgaggcctgcgagatcgccaaggccgcgcgcactgccggcctgaacgcaccggtgcgcctgctctggagccgcgaggacgacatcaagggcggctactaccgccccatgcacctgcaccgcgcgcgcatcggcttcgacgagcgcggcaaggtgctggcctgggaccacgtcatcgtgggccagtccatcaccacgggcacggtgttcggcgagttccaggtgaagaacggcatcgacgccacggccaccgagggcatgcgcgatccgtacccgctgccgatgcgcctgaccgtgcaccaccccaagctcaacgtgccggtgctgtggtggcgcagcgtgggctccacgcacaccgcgttcgtgatggagaccttgctcgacgagatcgcgcgcagcaccaaacaggacccggtggcctaccgcatgcagctcttcggcgacaagcacccgcgccaccgcgctgccttgcaactggcggtggaccagagcggttacggcaagaagcagctgcccgccggccgcgcctggggcgtggccgtgcacgagtccttcgagtccgtggtcgcctatgtggtcgaagcctccgtcaaggacggccagccggtgctgcaccgggccacggcaggcgtgcattgcaacctggccgtcaaccctcgcagcgtcgaagcccaggtgcagggcgccgcggtcatgggcctgtcgatgtgcctgcccggtggcgccatcacgctgaaggacggtgtcgtgcagcagggcaacttcggcgacttcaccgtggcgcgcatcaccgacatgcccgagttcgccgtgcacgtcgtgcccagcgcggagccgccgaagggcatcggcgagccgggcctgccgccgctggcgcctgccttcgcgaacgccattgcgcagctcaccggcaagccgatgcggcagctgcctttcaacttggcctgacgacggcggtgggcctgtgaaattgcgcgctctgaagcgctatatccgtgagcttgaccatgaaccctttggacggcatcacgtcggacggttctgggtcaagcgcggtcatatcggcccctcactcgctgccggcggttgttttggtgcgggtcctagaagcaccctgcgctcacgccaagcgccctgcacgaaagggtctgtgaccgcgtagacgccgtgccccttgcgcatgatgatgttcgcgtcgcgcagttcttcggagatccgttgcacctggtcggccgtcacgtcgcgtccgaccacggcggcgtactcgctcaaggcgtcggcggcaaacaggcccgtcacatcgccatccgcgcgagcaatacgggcaaagatggccccggcgaggactcccagatcctcgaccttgcgcaactcgacgtccgccgccgcgctcttcagcgttgctgcaatcactggaagaaggtgatccgcctcctgtgggttctgatgctgcagctgccgcaaggccttggtcaactcctcaggccgtcggcccaaggtgttgaacgcttcgactgcgacaggcaggctgggcaggaccatcgctccctcgctcgcaatgcccgtgaggacatagtcgacaaagtcctccccgagggtggggtactcgaccgtcgatgcgccggcgaaagcgtgtttgccctgcagggtcatgccaaccacttgagcgcgatgcgacccggttccgatgaagatgaagtggccgggtgtgttgggcctcgggttgatcgcatcgcgggcagccttgatggccagcagcatctgggcgccatcgtcacccgcgagcgcctgctgcacctcgtcgacgatcagcaccacgtcggtcttggccaagtcgacgacctcggtcaaggcctgagcgagagtgggcccgcctcgagcgcccaggtcggcgagctgaaagccgaatttcagtcccgcggcgccgatgtccaggcctttgagccgcttcagtcgccccagcgcacccgaagcgggagtctgcaggtctgccagggccttgcggatggccgcgtggatcagcgtggcgggatctgccttggtgtcggcccacaggtcgacatagatgaccaatgcgcccatggcctccaggacagggatcaggtcctgttgcagaaaagtggtcttgccggtgcgcctgagccctgacaggaaaagcccggatcgcaggccttggtcaagaaagcctggccggagtagttgcctggccatctgctcggccaaggctgttcggcgaaagaagtccattttgagtgatttagtcaaaaaacctaattagcagtattgactaaaacaggaaaaaaggaaagccgcgtgggagaagccccatcgatccgacccagaaaacccggcagtatggagctgggagccagaaatcacgaatgaaatcaataagttagcgaaaccgaatcgcgaagatcgaaagaacaaatccggattggctcgcgaaaccggcgacagctacaacgacaaaaagtgatgcacctcgggcttgcccggccccatgtgaaaacgcatggcctcgccttgcaggtcggcgtcggcatgcgacacgcggtggtgctggcgcaggtgctcggcccacgactcgacgagaaaccactccacgatgcgctcggcatcgaccgtgtgctcggtgatgccccaggcgtaggcgccgtcgcgccggcgctccagcgagagccgcttcatcacggcgaggaacgccgcgcggtcgtccttgcggatgcggtactcgacctggatcatcacgggcccgcggtcgtgcgcgacgggttcggtcaccagcggttcgggccagtggttggagggctgcaggtcggcctcgccggccggcagtcgcacgcggtggaacacgagcgccaccaccacgagccccaccgcccccaccatcagcgtggccggcacgcccacctgctgcgcgaccaggccccagcccaggctgccggcggccatggcgccgttgaacacggtgaggtacaccgccagcccgcgcccgcgcacccagttcggcaggatggattgggccacgccgttgagcgtggtgagcgcaatgatccagcccaagcccagtaccagcagcaacagcaccgcgagccacttcggcggcgcgaacacgaggctgcccatcacggccgcagtaagcagcgacgcgagcaggatgagcccgtcggcgtcgagccttgcgcgcagccgcggcatgaccagcgcaccggcgatcgcgcccgcgcccaccgcccccagcagcacgccgtagaagccggccgtgccgccgagcatctggcgcgcgaccagcggcagcagcgcccagaccgaactggcgaacaggaagaacacggccgcgcgcagcagcaccacgtgcagctccttgctggcacgcgtgtagcgcaggccggcgcggaaggcgccgaaaaaattctcggacaggccgctgtcgacggcggccgggcgcttccaccacaaaagcgccgcgatcacgaacgcatagctcagcacgtcgatcccgtaggtgaccgccgcaccgaagctcgcgaggatcaacccgcccgcggccgggccgatggagcgcgcgatgttgatgccgagcgagttcagcgccaccgcgcccttcagctcgccacgcggcaccagttccggcacgatcgactgccaggtcggccccatcagcgccgcgccgatgccgcccacgaaggtcagcgcgatgaggtactcgacggtgagcgcgccggtgtgcgagagcaccagcagcgcgccgctgacggccgcgagcaccagctgcacgaagatcaggaaacgccgccggtcgaggatgtcggagagcacgccggccgggatcgccagcaagaagatcggcagcgtggccgcggtctggatcagcgccaccgcggtcgggttggccgagagatcggtcaccagccacgagctcgccacgtcgcgcatgaagctgccgatgttgccgagcacggtggcggcccatagcaccgcgaacaccggctggcgcagcggcgcgaaggcgccgggctgcgggggcgatgcggctacgccggcttggggttcagtcatgcgcacgctcccgcaggtcatgccaggccaccagcaggaagccgccgaccaggcccagatgctcgaagaaggaattggccgccatgaagcgctcgggctgcggcatgtcccagaaccgcagcgcaacgaaggtcgcgagcagcgtgaagccgcccagcgccagcgcgccgagccagcgcaagaagcccgtgaggatgagcgccgaggcacccagttccagcacaatgacggccacggccagcggtgccgcgggcgacaggccgaagtggttcatctccgcgatggcggcgttgaaatccaccgccttgttgaagccgccctgcagataggccgcgcacagcagcagcaaggcgatccagcgcagcgccggggtgggtggccagcgtttcgtcatcagaccgcccagcaggcgcagccgagcgcgccccagaagctcttgaggtcggcgatcggcagcttgctgctccacgccgtcgcgtgctggtggccatgcacgctgcagttgttggcgcaggcgcaggacatggccgcgtggcgcatcgccttttgcagcggtgcgccctcggcatcgccccagccggcatagccgccgaagctgcgcaccggcgaccagtcgggcatggccggcggcggcgcgccctcgtcgtgcgactggagcggccccgcggcgtacaccaccttgccgccgaccatggtcaagagcgccgtggtgtcggcgatctccgactccgcgcaggcgaagaagtcgcggtcgggcaccaccaggtcggcgagcatgccggcctcgatgcggcccttcttgccgacctcgttggagaaccaggtcacgttctcggtccacatgcgaagcgccgcttcgcggtccaggcagttgcgctgcggatagagctgcatgccgcccacagtcttgcccgtgaccagccacgacagcgacacccacgggttgtacgaggcgacgcgcgtggcgtcggtgcccgcggacaccttcacgcccttctcgagcatgcgcttgaccgggggcgtggcctcggccgcaccggcgccgtagcgctcgacaaagtattcgccctggtaggccatgcggtgctgcaccgcgatgccgccacccagcgcggcgatgcggtcgatcgatttttccgaaatggtttcgcagtggtcgaaaaaccagttcaggcccgccagcggcgtgtctcggttgaccttctcgaacacgccgagcgcgcggtcgatggtctcgtcgtaggtcgcgtgcatgcgccacggccacttgttctgcaccagcacgcgcaccacttcttccagatcgccttccatctcgggcgccatgtcgggccgcggctggcggaagtcctcgaagtcggcggccgagaacaccagcatctcgcccgcgccgttgtggcggaagtagtcgtcgccctgcttgtatttcgaggtggcggtccagttgaggaagtcctgcttctcctgcttgggcttctgcgtgaagaggttgtaggccaggcggatggtgagctggccggcgtcggccagctgctgaatgacttggtagtcctcgggaaagttctggaagccgccgcccgcgtcgatcgcaccggtcacgcccaggcggttgagctcgcgcatgaagtggcgcgtcgaattgagctggtattcgaaaggcagcttcggtcccttggccagggtggcgtagaggatgctcgcattgggcttggccagcagcaggccggtcgggttgccggccgcgtcgcgcacgatctcgccgccgggcggcgcgggcgtgtccttggtgtagcccaccgcacgcaacgcggcgccgttgagcagcgcgcggtcgtacaggtgcagcaggaacaccggcgtgtcgggcgccaccgcgttgagctcttcgatggtcggcaggcgcttttcaacgaactggtgttcggtgaagccgcccaccacgcgcacccattgcggcgccggcgtgatcgcgacctggcgcctcagcatcgccatcgcgtcggccaggctgcgcacgccgtcccagcgcagttcgaggttgaagttgaggccgccgcgaatgatgtgcaggtggttgtcgatcaggcccggcagcacgcgccggccctgcaagtcgatcacgcgggtgccgctgcctgccagcggcaggatgtcttgcgcgcggcccacacgggtgaagcggccgtccttgatggccacggcatcggccaccgggttggcacggtccagcgtggtgaagcggccgttgtgcaggatcaggtcgggggcggtggtgcctgccatgtcggttgtccttgaagggttggattgtgccgatgcggtgccggccagcaccgcgccgagcgtgccgaggcagagccgccggcgctgttcgtcgaatgatggatcgctcatgcgtctttgcccggtgcggcggcctggccggccttggcgcattgtggcaactcgccgaacacatgcggcttgacctggtggtgcagccaggaggtggccgcggcctcgggctggagccagcccttgaccaggggcggaatctgctcgccgagcaggattccgagaagccccaccaaggcgatcaccggcggggccggggaacgcacctggaagagcgcgtagatcacgccgaccagaaggcccagcgcaagcgacaggacatagggcttcatcgggatgcgcccgctcagccttcgtgcgcgccgaacatggtcttggcgtaggtcacgcccaggccgtaggcgccgccgaacttcttcgcgatgccggtggtgagctcgtaggtgtcggtgcgggcccagtcgcgctgcagctcgagcaggtattgcagcgaggtcatcggctgcgcgccggcctgcaccatgcggtccatcgcgcggttgtgcgcctcggtggacacgtcgccgcaggcgtcggcgatcacgaacacctcgaagccctggtcgagcgccgacagcgcggggccgacgatgcacacgccggtccacaggcccgacagcacgatgcgcttcttgccgatctcgttcacgcggtcgatcaccgccgcgtcttcccaggtgttcatcgaggtgcggtcgagcatcttctggcccgggaacgcgtcggtgatctcgctgaacatcgggcccgagaagctcttctcggccacggtggtgaggatggtcgacacgccgaacccggccgccgcgttggcgacgagggcggcgttgttgcgcaggttcaccgcgtcgatcgaatgcgtggcaaaagccatctgcgactggaagtcgatcatgacgagcgtgtggtcggcgggggtgagcagcttggcgccggcggtgggggtggctttgatggacatggggtactccgtttgaaagattgaagaaaaagaagaaaggaacaggggaatggctgcgtcgattagttcgatttgattcacaattgcttcgaagaagaatccccgaggcatggatgaatcatctttctttccgaggggccggttgacgaaatttttcgccttcaatcatcgaatttttcgatgattaatttccaaggacctgcccgtgcgcaagctcagcctcgaagccatcgaactcgtcgacgccatcgcgcgccacggctccttcgccgctgccggcgcgcgcctgaacaaggtgccctcgaccatctcgtacgccgtgggcaagctcgaggagcagctgggcatgctgctcttcgtgcgcaacgggccgcgcgtgacgctcaccgcggccggcgaagaaatgctcaaggaaggccgctggctgctcggcgccgcaagcgatctcgaatcgcgcatgcggcagatcgccaccggcttcgagtcggagctgcggctggtgcacgactcgctgattcccacgcaggcgctcatcgacgacatccgcgccttcgaggcgttgcgctgcggcacgcggctgcgcatcggctgcgaggcgctcaccggcacctgggaggctttgcgcgaagggcgcgccgacatcgtcattgccgcgggcgaagggccggccggcgggggctaccaggccgtgatggtgggcagcctcgagttcgcgttctgcgtcgcgccgacgcatccgctgacccggctcggccggccgctgcatcgcggcgacctgctcgaacacaacgccatcgtggtgagcgacagcgcgcgcaccctgtccgaccgtaccgtggggctgctcgcgggccagcatcgcgtggccgtgccgagcatggccgcgaagatcgcctgccaggccgcgggcctcgggcatggctttctgccgcgggcctgcatcgatggcgacctggcgcgcggcacgctggtcgaactcgccaccgacgaaccgcgcccgcccgaggccttctggctcgcctggaagaccaacgcccgcggccaggcgctgcgctggtggcgcgagcggctcaaccgcacgctggtgccggcgctgctgccgcgctcgctctgaacaccgctcttcagaacaccaggcgaggagcatcctttcgcaagagcgcgcacgctgccggcggtgcccaggcctcagccagcgcctcggacagcgcagccagcagccgcggcacatcgtcggcggcattggcatgcaaggcttcggccacgatgagcacacgggaggtttcgtcgcgcacggcggagcgggcgctttggcggtgcgtccaccgccgggcgtgcgcacgaccgtcgacatccgcgaagatgacttcgccgcgttcgggcgtctccgtttcgcccgagaacgccaggtagctttccgtgccgtccgcgcaccgcacctccagcccttcggacacctgcgacaggtcgaacaccgcgatcgggatcgcgaaggccaccgacaccgcattgcaaagatcgacgagcgggtgaatcggcggcagcgagccttccttcctgaaccgccgcagcaaggattcggacgcgcaccggtactgcgtgggcttgaggcccatgcgcccgaaggtgcggcgccaggcctggatctccggaagatcggcttccgtgccgacggcggcgagcctcgcgcgcgcgatgccgtggtagtgcgccacctgcgcctccacggagacgttcgtgtggatgccctgggccagcaggacgccgggcaccagttcggcatgccgctcccagatttccggcgaatgagagaagaagaaatgcatggcgcagtgtgtcgctcgcgcggcggcgcgtcttgaacgctattgcagtggcaccggccgcccccaggcgcgctgccatgcgccgggcgtgtagccgaaatgctggacgaacgtgcgtgtcatgtggctctgatccgcaaagccggccgccatggccgcctccgtcaacgcggcgccctggcggatgagtccgcgtgcgacttcggtgcgctgttgcagcagccacgcaaacggcgtgacgccatggacctctttgaagcgccgcagcagctggtatttgctcagccctgaagcagccgcgagctcgctcaggctcggcggctgtgcgaggctgtccgcgagcatttcgcgggcgcgcgaaacatcagccgatgccagagggacggacagccggcgtgcgccatggcgcccgacgagcatggtgcaggcctgtacgagcagctcctcgcagcgcagtacgtcgggccaggcctgtgtctccagcatgcgcaggagttcgcagagcgcgccccgcaaccggtcgtccaggatgaccgggcgaatcaatgccatgtcctgcgccgcgccggcggatgccgcatcgatcgcccaccgaagcgcatcgggttcgaggtacagcattcgccagcgccgaaagtgcccgccgagcggccggccgtcatgcacctcgcccgggttcgtcgcgatgaggttgccggcataggcatcgacgttgccgcatccgctggccgagctttgggcgccctcgtcgatgaccccgactccgaacgtggcatgccagtgccggccgtagtggcgatcgctcgaaatgctcgtgccgtgcacgccctcccagggagagccgaagacgcggcagacgtggtgcgggttcctcatcgcgcggagtatgcatgcgctgggtccgctccctcggcgtgggccgttcgatatatgctggtgttccggtgcggcatcacggaacatcgcggaccgtgccaacaaccaagaaagacgcatgcaccgtatcctcgtcatcctgctggggctgctgctcggccttgccggctgcgacggcggcagctacacgaaaaatggtttgcagtgggcttacgacggcacccccttcaagcccgatgacccaaagacgtttcgcgccctggacaaacacttcgcgcgcgacgcgaagcgcggctactaccggggcagcaccatcgacggcagcgacggcgccagcttcgaggcgctgtccgaccatgaggcacgcgatctccagacggtctactactgcgacacctaccgcaagggccaggagtactgggcgattcaatacgttcgcgtcacgcccatccgggacgcgcatgcgccgacctatcgcgtcctgggcttcggctatgcgcgagatcgctcgcgcgcatacgaagacggcgtgggcttcgcggtgcgcgacgcggcgagcttcgagccattgggcccgcaatttgcgcgcgattcagagcgcggctatttcgctcgtgccgagattcccggcagccacggaccgacgttctcgctgatcgacgcggggtacgcgcgcgatcgcaccagcgcctaccacgcccacatcgaaaccgacacgcccaatcgaggaccgtaccccgtggtgcgcaccctgcgcggcgcggacaccgcggccttgcgtgttctgggccgcggctacgcttcggacgccacgcgtgtctggtatcggggcacgcccgtgcttcacgccgatgccgcgagcttcgcggtggtcgacgatgtcgcaagcgacatcgatgcaaatgaccgcacgggctcctggcaacaaggacgaaaagctgccgccgccacacgctgagcccggccggccggccaaggcagatgcagaaagtttcccctgccgccgcatgcactggctacgatgtgtccacgcctacaaggagcaccgacatgtcgaatcacgtttacaagtcgctcgaactcaccggctcgtcgcccgtcagcatcgaggatgccgcgcagacggccatcgccaaggctcacgagacggttcgaaacatccagtggttcaccgtcaccgagacgcgcggccacgtggtggacggcaaggtcgcgcactggcaggtgacgctgaagatcggcttcacgctcgagtagcaactggctgcggccggccggctagtcggcgatcacatggaggctgtgcttgctgcggcgcgcgcgggcgcacatccgcgccagatccagcaggaagccgaccacggccggcttgtccgtgcagcccggcaccaccgccaggatgtccttgcggagcgccgtcaggccgtcgcctgaaaccaccatctccgcggaggcgccgtagtagtgcttccagaatttctgcagcgctccctgtttcagttcatcgatgacaagcgaatagccatcctcccagatggattcgtccatcgggaggctgggaaggcccggcgtctcgggccgcattccttgtggcacctggatgattcgccgcattttttcagccgctagctgcagttgcccggcgcaccgttgagttcgggaaactcggtgacaaccgtgccgttggttgcgctttcgacgatgagacgtccgcacttttcgccggccgtgccgacgatctggttgaggttggcgtcatagcgaacccgattgtcgggctgcacgacgcgggtcttgttcggtgcattctggaccatgcggcagaaggtctgcgccgcggtggcattggtgcagtactgcggcagcagttggctcgcgccggacgttgccgtgcaatggcgcgcaaagatgtgctggtagccggtcgcggtgacgacgcactgggcatccacgcccacctggctctccgccggcttcgatccgatgccctggcaaccggttagcaccgccatcgagacggcgcaaaggatggcgagttggcttgtgttcttcatgatcttcttcctcagcgaaatttgatgatgtagttgatggacagattcttcggccgcgtttcagaagtgagccgcgcgggcttgatgggcgcgctggtctccaggtcgcccgacgattggccggccgcattgccgctttgcgacaccgccgccagcgtcaccgccttgtaggtgtgggtgtgcgtctgcaaggcgtcgcattggtaggtacccacgccgttggcggtcccgctgcccgtcggcgccatgcgcaatgcggcatccgggtccatgcccgagcccgcatcgttgccgcgcagaaagaggcctcggtagtcgggaatgcagaagtcgtcgctgacccctccgtacaggtagcccagcgccgcgaagagttccgggtacgcgctgaccttgagcttgcgcccgtcgcacagcatccagccctgtgcctcgaggtaggtggtcgggatgtcgtcgcgcttgggcgccgtcaccgagttctggctcgcgcaggcggtgttcttccagatgttgttggcgtcgcccgaaacggggttcacctgtccggcaaaaccgcagacactgcctatgacgcatacatcgaacatgtcgcatttcctttgcggtgaagcccgttgcgaacggcggcgtcggaagatcgacgccgccgtggcgcaatgggccgcgggctgtctggaaggccggcgatcagcgggagagcaggcgcagacgctgctcgttggacttggccgtcgattgcggcgcatcccagctgccatcggcgttcagcgtcgtggtgagcgcgtagatgccggtgggatacggcagttcgagcgggttgttgatcgagttgacgtcgatcacgtcgccttccacgtagtcaccgtaggcgatgaagtacttggggtgcggcgagaaggtcaggctctggttcggacgcgcctgcactgcgtacacggtgctgcccgacatggtcacgccgaccgaggcgctcgacttgatcgggatgttcggcgattcgctcaggtagaaccgtgccggatcgggacccttggtggggttcacgaactggtaggccttgttgtagtccagcgtgatcatgttgttgccgccggtggggtcataggtttcggcggtcgagtactcgatgccgggctgcagatcgcccgtatcggcccatgagaaaccggtgttgacggtccactggaacttgatgcgcgtggtcggacccggattggaaaacttggagaaccaggcgagcgacatggcgttgggtgcccagttggtcggatcgctttggaacaccatgaaatacgccgaatggctcgcatggttgttgacggtaacggaatagatattgcccatgtcgctctccagatgaagtggttggtggaacagtccggaccgctgtgggaccgaactggaaccaactctagggagccaccctcttcaacggaattacaggcgattacacgaagcgccgtctccggtcgaacggccgttcagctgcgtgcgccgccctcgatgaggaacgggtagttgccgaaacgcacatcgccgcggcgacgctcgaccagcggcgcgtcggccgaatgcgtgggcagcgcattcaagatctggtgcttcgcgcggaagatctggatgttcacgtaggaaggctccacgccgagcatgcgcgacagctcgtccagcgcgatccagccctggctctgcggcgcaagcccgcgttgcgcgtcttgcgaacgcaccctcgcgagggtcacgagggtgtagtgatgaatgcgctcgccaagggaaaccgacttgccgtccgtcaccaggctcaggctcgtgtgctcctcgttctggctgacattgaagtgaagggcaacctccaccggcggcggcgacaccgacgcaatctggttttctgccgtcgattccaggtcgtcgcacagcacgaactcccacgtgctgccggaggtccgcaccatggcgccatcgcccagctggtcgatgccgtcgatgtgctcgagcacccattggccttcgcggaaatagacgttcacctcaggctgctgcgcgtccggcaacaggttctcacgcaagctcagtgccaccggcgagccctgcccgtcactcggaaagagacaggtcgccggaggcgccaggtcttcggcgatccaggccgattcctcgcccaggcccaactggatttctgcgcccggcggcagcacggtccagcggccgctcggcaggcgttcgccattcagcgtggtgccgttgcggctctgatcgacgatctcccaggccaggcgattccaccggaccagcgcatggatctgcgacacgtcgggcgcctgcagcaccgtctggcaggccgatgggcgccggccgaaggcatgcatggggcgcagcacgatgccgcgttgatcgcgcttgttccggaagatggccatcggcagtttttccttcgtcgtgttcagacatacagcgcctcgggattcaagtcgctttcctgcaagggggtgtcgcgccatcccatggcaagcggcacttgatagagccgtgggttgcccagctcgggccagatgtggcacaggccgggcacgaccactttcacggtgcgaagcggaatatccggccgcgtgtagtcgagaaccaccgtctccatgccgagcgacgcagcgatgcgcacgcagcgttcgatctcttcggcaatgtccgcgccggccgccacggccgccacggccgccacggccgccatggtgggtgggcgcatcggtgccgcatcgccctcgccatcaccctcttccgccggcatgagaaaacgtggcgcgtcttccggaccgcccgaatgcggtacggaaaatttctttccggcggcgatgagctgggtcatttccgtgagcgcccgctcgcaggcgagcacggcactcgggctgcaaccgaagccgatggcccagtcacccgttgtgcgatgccggccgatggcggccacgaccggaatgccgaagtcgtgggtgaggtccagcgcccagtgctgccattgcggccccaggctgcgcgcaatgcgagcgcggctttgcacggcgaggcacccgaggtcgatggcgggcctgcggatttcgccgtaccaccagatggcggcagcgtcgcgctccaccagttcgagaaagccttgaaggatggcttcctccagcgtgttcccggcagcgcagccgttcgacgtccacaccgaatgccgctggctctccaccggggcattggcatggcagaaggccagcggcagatagcagcgggacctggatgtcagcgaccaggccggtgtccaccatgccggctcgtgtgccgacggcgccggcgaagccaccgcatgcggcgggccgttcgttttcagttgcatgcgctgcctgtcgctgaaaagcgcgagcgcctgcggcaggatgcagcgcgcgtccaacgccgacgccgccgcgaaaacggaggcttcatcgccctggtgaaaggcggcgtaccgctccacggcttcgcacattgcactggcacgggactggtccgtggacatgcccttgccaaggcacacctggaccagcacgctggcggaaggatcaccgtgcgcggctggcgtcctgaagatttcgctgcggtagaccgtgagtgcatcttccgcttcggtgcccaatggcacgacgcgcgcaatgacgccgcacagcggatcgaggtgcggcgccaggcgctcgagcgtggcggccgcgggcatcgtgcgccagccgccatcgggccgggcgcttgcaaggcaaggcgcgggcaccaccggacgacgctgaagttgcgccatgagccccgcatcgccgcactgcggacactggggcctcggcgcgacggcatgcggctgcgcgggctcgatggtccacagcgcctggccggcgtttgcaacgatctccagcgccagcggaagcaggtgctccagccggtcgcgagcgagcttcgcgtcggcgcgtaccggcaagccgacgcttcggccgccgtgcctgtcctgccaccaggccctggcaggctggttccgcagcaggcgatacgcgaggcaatgccagcatgccgtggcggcggccgcatgcggcgtgaacagcggtccgaccatggcccgctcgcccgtcggcttgaccagcagccatggccgcctttcggcccgctgctgcgtatcgatcaggccgagcctgggatccaggtagtcgtcgcagaggacgacggtgtgcgcttcatccccacccaccgcgcgcgcccagcgccgggccgcttcggggtccacgacttgcgacagcacgatggcgtcgacgtgcgcctccacatcgacgcgttcgaacggcaacgaaaaatccggaacgacgtggcgctctgtgtcattcaccggcaccggccttgccaggccctgccgcatcaaggcttcgagcgcatgcagcatctctgccagcagcgcgggcacgccctcttttctgcaatgcgaggccaggctcacacgctcgcgcagcatgcgctcgacggccagcacgccgggcgcgccgagcaggaacaggtcggtctcgctcaacagcagcaggccgtccggccgcagcagcggcggcaggaacttgccgtgccactcgaaaacaccggtgaagaaatccatcgagggcaggctatgcgtcatgcggcgatcccagcgcgaagcgggcgaccgtgtagggccagcggccggtcgccgcgcggaatgcggcctcgaagagccgatgcgaatcggagaactgcgaatagagatggtcctcggaaagcgcgcgaatcgacggatggatggccgcgatgcgggccgaatcctcgaagcccgagaccaccggcagatgcatgccgcccacctgcaccggcatgcccgccaggaccggatggacgtagtccagcacgacgacgcttgcggactcgcgccgctcgaaacgttgggccagatgaagcagcatggcctccaggggtgcctgcggcagataggggcacacgccttccagcatcaccagtgcgggccggccggccggcagatcggccgcatccagccacgccgggtcgaggatcgagcacgccaggttgcgctctccttcgttgggcgtcacgtgctgctcgcgcaggcgaatcgcgtccggcagatcgacgttgagccaatcgacgccagcgcctcgcgccacgcgcggccccagccgcttgcggcgcgtgcacagccccgcccccagcgtgatgccgatgccgcgcggatgcgccgcgaagaactcggccgccaggcgatcgatcagtgcagcgcgcaggaccacgccgcggacgaacgccgcatcccgcgtgccggccgacaggtcgaacggcagcgccgcggcaatgcggcgcgcctccggatcggagaagaccgacgcggcgatgacgctctccgacccggcccgggccgcgagcgtcagcagcagcgtcgcggtggcgccttgcaacgcagttgccgccgtcccttcgggcggggactcagcaagtgaagggataggcactgcccgtgttgttgtacgcggtgagcgcaatcggccgcatcccctcctccgccggtgcctgcgggtagttgagctggatcgtgttcttgatcagcgatccgtccgggccgcctttcaggttccactcgccgcgtgccgcatcccaggtgagcttcgggtgggtgacgaaccggatctggaaattgaacgggttgttgtagcccagccattggctcagcaccggggccttgtcggtggtgggatcgccggtcaggtcacccaggaactgcggagattgccacgcgagggcaatggcgcgcagcaccacgccgccaaacgccagcaacgaatccggaccgccacctggaatgccgagtccggtcggcagcgcgccttgcggcggtccgacgggcttgtcggttttctcgaaggccgcggccgcgcccatgaaattcgggaacagctggtagtaggcggccagggcttcggtcgcgtgagacgacgtcggcgcctgcggcaacacgatgacgaaggcatcgtcggggctgatccagccggccgtcagcaccggcttccattcggctctctgggccggatcgctgttgaggtacaggctgatgttcaccagcggccacagcgtcagcaggccgaagtcgcggtgcagcagcggctggatgtcttcctggtcgagcagttcgcgtcggtacgcatcgtcctgccacgatcgtgcaagggcccggaggtaggcgagacggaattcgagcaagggctcggctgcactttggcgctgggtcatgatggctcttccttggttaagaaaaatgcgcaggcgtcggcttgcgcggacacaactccggccgcatggcggccagatccttcaagcgtctggacacatcccggtcggccggcgcgagggcctgcaacgcggcgagcgcgtcgaactcggtccggtgttttccaccttcccgcgcgacctttgcggcgcgggagaaagacagcatcgctgccccgcgttcggcgcccgcgcccagaaggtagcgggccttcttcaggtgcagttcggcgctgtagagcctttcgttgagttgctccaccaggcgcaggcagtcgtcgatgcggtcgatcgcctcgtcccatcgctcgcggccggccagcgtttcggcggcgaaggcgcggtagtacgtctggcaatagcggcaccccatgttccacagggcctgcaccgtgccgtcggcctgcgcgatgtcttgcggatcgcccgtcgaccagcagcggatgatgtccgcatagccctggaacgccggcaggccgtagcgcgccgtgatgtcgagcagctcggtggtgctcgcccgcgccgccgccctgtcgccacgggcctggtggcccaggctctgatacagcagggccatgctcagcgaaggaatgtgggacatctcccgggcccactgcacggcctgggcggcatcggtggccgccgccttgtcgtggccggcgaaccatcgcaccagcgaacgccccgtggtcgcccacacgcgcgtgtcgaaaccgaaatccgccgcatggtgcgcgtgcgcctcggggtcgtagcgctcgacggcatctgtcaacgcgcgttccgccatcgcgaaccggccgtcggaatagtgcgcgaggcccaggtaggtctggccggcgaccagcacgccctcgtcctgctgatgcctggcatggccgagcagcctgtggctcagccgccgcacctcgtcgcggttgctcgcgacatggtggaaggtgatcatggcccacaggtgctgcacctgcttttcggcggccaccgtgtcgtccagcagttcctgcgacagggcgatgcggtccaccacctgggcatgggcccagccgtacttgttcatcatcgcctgcgtgacgtagctgttcacgtccagccgggcttcgcgctgcagggcgccggccagatgtccgatccagccgtcgatgtgctgcgcataggcgatggtttcgtcgttgagcgaacggtgctgcgtgaggcgaagctgccgcaccgcgtgcacggccgcctgcgcatggtctccggcatcggcccaatgctgcgcgacgatgcccggctcgttggcgacgcgctgcgggtcgctctgcagcagggcctgcgccaccttcttgtgctgctgccggcgctgcgcgacgagcatgcattcgtacgcggtgtcgcggatcagcgcatgccggaagacgaaggcgtccgcccccgcgccggatggatcggccggcatgacgagccccgcatcgcgcagcgcctccaactccctgtccaccatttcgcgcgtcttgcccgagcaggcgcacagcaaccttgcgtcgaactgccgcccgatggtggccgccagttgcagcaggctcttggccggcccgaggcgatcgaagcggctcaccagggagtcgcgcagcgtgacggggatggcggccggctgcgccgtgtgcttgaagacccaggcaccgccctgttcgaccagataggcgtccagcagcatacgcgccatctcctgcacgaagagcggcacgccgtcggtgcgggcgacgatgttgcggatcaccgcggcatcgatctttctcggtgcgagcacctggcgggccagctggctggcctctgcatcgtcgagccttcgcacctcgatgcattcggccttcaggccttcgggcttttcccattcaggccgagccgtcagcaccagcagcacacgccggtcggccagctgcacgatcaactgctcgataaattcgatgctcgtggggtcggcccaatgcacgtcctcgaccaccagcagaagcggcgccgaggcggccatgtgcaacagccactgagcggtcgatttcagcagcagtgccttctgcatcgcgggcgacacttggcttggctgctggcccgcgcccagaggaagcgacagccacgaacagaagatcggcgtcacggcagggccgtcgcagccagcggtctgcagggcctcgttcagttggccgcgttgatcgtccggcgatgcgcccggcactgcttcgagctgctggcgcagcagcgccaggaacggcatcagcgcgctgttgcggtgttccggctggcattgggcgttgacggacttcgggccgccttcctctgccacgtgctctcgcagcacgtcgacaaggcaggacttgccgatgcccggctcgccgcggagccacaccgcgcgcccatggcccacggcggcctgcgcccattcggcccgcaacagcgccagctcccgatcacgcccgatgcacatgcggctcagcgcacccggcgtggacgcgggcggcgatgaagattgcttctgcgcatccagccggtaggtctgaacaccggcggacagtcccggcatgctcacgctgccggcctcttcgaaatgcgcgtggcgcgccaacaggcgataactgctttcgctggcaagcagcgtccccatctcggccgtgccctccagccgcatcgccacgctcacggcatgccccgagggaatctcgccgcccgccaccaccgccatgccggtgtgcatgcccatgcgaatgcccaggtgcgcgccgtgggcctgccggatggcggccgacctgctgcggccgagggccgtcagctcgagcgccgtcatgcacgcttgccgcgcgtcggtgtcgctcgcatgcgggtagccgaacaggacgatcatacgatcgcccagcgtgcccgccagcaggccgccgcgccgtgtggccgcttctgaaaagcggccgagctcttcgcgctgcagcagctccaggttctcgatgtccgaaggcagcagagacgcaccctcgccctccccttcgctctcgccggcgtcgggccagaccgcgacgctgcagcacagcaccgtcagttgccgcttctcggaaaaagcccttgccgtggccacggtgcgcgccagcggatcgtcccctgggccctgcgccggcctgaaggcacccacgaggtcgtcgagcctgagccggccgagttcttcgagcaacgcggatgccgatccgcagcgttcggcaggcttcttcttcaacacacgccgcagcagctccgcgaccgggtgcgcggcaatctcggccggcagcggaacttcctgcgggctcagttgccgatgcacgatctcggcggccgaatcgccctggatcgcgggcgcgcccgtcaggcattcgaggaacatcaacccccaggcatagagatcggagccggcgctgggcggctcgccgcgaagctgctccggcgcgctgtatgccggcgtgccgaggcattcctcgtccatcgtgagcgttgcgaactgaacctctctttgcagcggcatcacggtgccgatgccgaagtccagcaccttcgcatgcggcagcgcgccggtgaaactcaccatcacgttgtcgggcttcaggtcgcggtgaacgatgccggcgcgatgcgcgcagtccagtgcatcgagcacttccgccatcagatggccggtctccgccgcggtcagcgagcctttgcgccggatcaggctcttgagcgtttctccgggcacgtattcgaagacgccatacacgcaggcgccctgctcgcccttgttgagcaactgcacgatgtgcggatgatgcagcgcggcgcagagtttggtctcgcgatgaaagcgggccacgcgctgccggccctcctgcagcttcacgaccttgatcgcgaccgtgtttcccgtgtggtgttgcgttgcgcgatagacagtgccgtaaccgccaacgcccagcacatcgagcacgtcgtagccgggaatgcgcaacggttcatccggcgcaacatgctccgttgcgtcaatgcttgcaatgacggcatcctgcatttcagcccccacctggttgattggccaacgcaaattcgaagtgcgtcgcggctacggttggccgcgcagtcaaatcgatcgaaacacgatttgttactgtagctgaggggcgatttttttcgtaagagattcttcaaaaagaaagcgcattgcaggggcaatggaggtctttctaacgcgttgttcttcggttgtaggttgaaagaactcgcgctttttggcgatcgacttcagccgagatcgatgcatggtttttttggcccgggccaacgagggcgtgcaccgtcggctgctcgactatcctccgctcgccgcgcttgctgcatctctcgtccttgtgagccgtcgacgaagccaggcaccaccgatccgccttttcgcaaaagagaaagagtccgttccatgttccgcaccctgctcaagtccaagatccaccgcgttgccgtgaccgactgcgaactgcactacgagggctcctgcgccatcgacgaagacctgctcgatgccgccaacctggccgagaacgaacaggtgcacatctggaacatcaacaacggcgagcgcttcgtcacctatgcgatccgcggcgagcgcggcaccggcatcatctcggtcaacggctcggccgcgcgccgggcatcggtgggcgacctcatcatcatcgcggccttcggcctggtgccggaagaccaggtggcaggctacaagcccaagctcgtgttcgtggatggcgccaaccgcatcaaggaagagcgggcgcacattccggtgcaggcggcgtctgaagctgcgatggcgtagcgcgaagcgcgacggcacgccaggcatcaacgcggaccgcgcgatgtggggcaaggtgatccgcgaagccaaggtcaggctggactgaaggaagacggccgcggccatgccgatcgcgctggcgggtattcttcgccatcgaatctgcgacggaggcagtggccatgtacacggaacaaggcggcgaaggtcccgacctgcttctcatgctgcacggcatgggcgcgacgggggcggtgtggtcgcccatgtgcgccgaggccggtgcccgctggcagggccgctggctcgtgctcgacctgcccggccacggccaatcgggccggcaagacgcctatgccatcggccaatatgccgccagtgtggcgcgcgccgtgctgccgcacatccatcccacgggccggctcgtggttctcggacattcgctgggtggggtgatcggcctcgcgctggccacgggctggttcggcgtcacaccgcaccgcgtgtttgcagccggcatcaagatcgcctggagcgatgaggagctgcgccgcatggaggcgctcgcatcgcaacccgcgaaacggttctccaccgaagaagaagcgtgggaccgatacctcaaggtgtcgggtcttgcgggcatcgccggtgcggcggcacccgtcgcggcgcggggcattgcacacgacgcggatggctggcatctcgcgatggatcctcgcgccaacggcgtgggcaagccaccgctgcctgaactggtcgctctggcgcgctgtcccgtgcacctcggtcgcggaggccacgacgcgctggtgaccctggaacaaactcgcgcgctcgatcccgatgcgcgggacctgggggcgcatggccacaacgtgatggtcgaggcgcccgcgcaggtctgggactgggtggcctcgttctcatgagatgagccggtgccggggccggtctcaggcccttcgaagcggcaccacccgaacttcggcggcgcgcgccctcagctggccgcatccgccgtcgacgtcctggccggccgaatggcgcagcttcgtcaggatgccgcgctcgtgcagcatgcgggcgatctgttcgcaacgctcccacgacgggcggctgaacgccacgccgtccaccgcgttgaaaggaatcatgttcagcacgccgtatttgccggagagcagcctgacgatgccctcgatctcctccggcccgtcgttgacgccttcgagcagcgtccactggtactgaatgggatagccggtggcccgcgcatagcgctcgcctgcggcgaccagttcctcgggcgtcatgttcggcgcgcgcggaaggagcttcctgcgcaggtcggccttcgtggtgtgcagcgagagcgccagcgcgggcctcacacgggcttggctcagccgctcgaatgcgcgcggatcgcccacggtggagaacaccaggttcttgtggccgatgttgcccaccgtgccgagcagctcgatggcttcgatcacgttgtccaggttgtgggccggttcgcccatgcccatgaacaccactttgcgcaccggccggcgcatgcgcgcgagagcgacctgggcaatgatctcggcgctctccacctggcggagcaagccgtcacggcccgtcatgcagaactgacagccgacggcgcatcccacctgcgacgagacgcacaggccgtctcgaggcagcagcacgctctccacggtctggccgtccgccagggcgacgagcagccgctccgaaccatccgcaccgggatgcaccgcgtgaatgcgcgccagtcccgcaagctcggcctcgatggacggcagggcctccagcagcgatgacggaaagaaggtccccggcagtcgcctgccgctgttgcggggcagcgcatgggaccacagccgcaagatccgctgctcgtggctggggcccgcgccggcttcgcggaggcgccgtttcaattcgtggattcgcatgcgctgcttggggctaaggtgctgttgggcgtgtcggagatggcgtgagttgccttgcgcgtgactgggtaccatcggccatgcttctgtagccgaagtttccgtgtctgcggtcgccggttccaggcccggacccggacccggaccccggttttccgattatcccgccactcggagtgcgcaggccgcgctcattcatgccaaacgaacccctcactcagatcgaattggccgacgccaccggagcggacacacgctcggagacgcccaaacgacgctggccgtccgttgcggccgcgttcatgcttcacgcgtgcatcttgttctgcgtcgtcttgctgcctcccatcgtttacgacgccgttcgaacttcgacctaccagggcatcgaatggctgcatttttcaggcggtgtcacttatcccctgtacgccatctactggatagcgaagctcaagaattttcgcgccaagttcatactgattcatctcactgtcgttctgacggtcgcagtggccacggccttcgcgagcaaccgacacacacccctgttcgtggcgtttgtgccgaccgcggcttccgcccttccgcttctgggtgcattggcttcatggcttcacggcagccgcaagctggctgtgacctaccttgtcgggagcttgctcgcactcctgatagccatacccgcttccttgctgatcatctacggcatggcgatgtcgtccgttggccccatgcgttattaggtcatcgactgcttcgcctgatgtcgaccaggctcagtcctcgagctcgctggccgtggcgcgtttgcgcgcgggtgcctgacggcgcactgcgcgtgcggtggtccagggcgcgagcagccctccctccaagggctccggcaccggcagctccaatgtggcgatgcgaacggcgtcctttccttcgacgcccaacgcccgcagagcgctcgcgaccgcctgttccgtgaaatccttcggtgagcgcgtgggcagcatcgcgtgcacgctccccaggaccgtcatggaaacgatgttcgtcgccaggcgcatgggcatgtcggcgaagcggtggtgccgcatgcccagttcgagatcgcgcttgacgaagtcgagcagcacgcggccgccgcgcatctccggccagcccagccggaccaggaatccagccacctcgcggttcgccatcgcaaggcggatggccagcctcatgccggtcgagacccggtgcgccggatcctcgaagtgcaccacgacaggttccgccatgcggatgatgtcgttcatcacttccagagcgagcgcgtcgaagagcgtgtcgggcgcgtcgaaatacttgtagaaggttccgcgggaaacctcggccgcctggatgacatcgtcgatggaagttgccgccggccccttcttggcgacgagctggatggcgctttcgaacaggcgtcggcgcatcctgtcgcgccgttccgcggcgacccgggtccggtggtcttctttctgcatgggcgaattctgccttgaggcggacgcggcgcggccaggccgcgtcaacccggttcgtgccggaatgtgtagtgcgcgagccgccggccaagggcctctgcgtcgccgtccgccgaccaccgcaccacgatgccgcgtgtcgcgtcgcggacgacctcgcacgtgcgcagagtcacgcccaccgcacgcgcttcctcattcaccacggcggagatctcgcgatcgaccagtgccggcttgaagatcttgccgaccggcgtggtcggaagcgccggcagcacgtgcacctgcttcggccatgcggcgcgttccgcgatcctgcgttcggcccaggccaggagttcctccggcaaggcggatgcgccgggacgcagctgcacatagaccacggggacttcgcccgcatgggcgtcgggacgcccgatcgccgccgccagggcgacggccgggtgttcgtgcatcggttcctcgatcagcttgggatcgatgttgtggccgccccggatgatcagttccttgctgcggccggtgagccagaagtacccctcggggtcctgccgccccatgtcgccggtgttcaaccagcggcgcgccgcatggcccggctcggccgggacgtcgatccacaggcccacgttgtgggcggcgttcaggtagccgagaaacaggttggggccggagatggcaagcgtacccacttcgtcgaccgccgcctcgcggacgtaatgccctgccgcgtcgagcaccagcaccttgatttcctgccatggcacgcggatcccgatcgcaccggccttggcgaccccccccggcgggttgagcgtggagacgcagcccccttcggtgagaccgtatccctccaggatcttcacacccgtctcgtcctggaagcgcttgatcagttcgaagggcatgggcgctgcgccgcagagaccgaactgcagcgagctcagatcgtgcccgtgcggcgagacctgcatcagggccgaatagacggtgggcacacccgagaaggagcacaagcggaagtactccgcaatgcgccagaacagcgggatcaatcctggggcacggtagcccgaaggcgtgccgagcaccacgtggcggcccagggcccatggcatcaatcccgtgccgatctgcgcgttcacgtgggagagcggcaggccgcagaacagcgggcccgaaagcccgctgtcgccgaacatggcggcgagctgcatggcgttcgcagcttcggtgcgatgcgtccggacggcgatcttgggcagcccggtcgtgccgcccgtgcagaagcaggaagccacgtcgtccaggcacggcggctcgaattccaggctttggccctcgaccttgcgcagctcgtcatggagatcgaggaccggcagtcgctcgagctgcccctgcagcgcgccgcccgcggcggagtgcggcggtgctgccgcacgcgcatagcggcgcgcggaaaccgtcaggaccgcatgcagtcccggcacctgctgcgcgaccgcggacaccttctcccacaggtcgcttccaggcgtgggctccagcgtcacgagcagcttggggcgcaccacgagcatcagctcgcgcagcatgtccggctcgagcagcgggttcatcgcgaagaccacgccggcagcctcgccgccccagatgacccagtgcgtctccggaagattgggaaggacgaaggccacgacgtcgccgcggccgaggccaagccggcgcagcagattggccgtctgggtgatgcgggcaagccattcgccgtgcgtccacgtgaacgggcgcgcgtagtcggccgcctcgagaaaaaacgagaccgccggcgcgtccggcgcacgccgtgcgccgcgcgccaacagctcgtacgtgctgcgcacttccgccagcggatcgggaacggcttcttccagccggcgcacgtcgtccggcgatccgattccggacgatgagacgagccgctccggcagctcgaaggacgcgggcggggcggcatgtggatcgtggttcatcggtgggctcgggaggaatggcttagggaaaacgacaagtctgtcataatgacatttacgtcattatcacatcacttcgtcatctggcccacctgtggaaaacccatgcaatcccttcgcaatgtcgctgccgccacggaagctggtagccgttcacaagcaccctcgatgcgaagttccgcggcgctgcggcagccggaagccattccggacagccgcctgccttccggcatccagcgcctgaaccggccgcccgcagccggccgcgccgtctcgctggctttcctgcgctggcagaagaagtcgctggcaaagaccgagcggttctggcgcgactttggattgacgatcgtgcattccggtcccgagcgcatcgtggcgcgcggaacagcgggtacgccatgcgtcgcggtggccgagcgcggaccggccaaccgcttcatcggcgccgcgttccagatgtcggccgagacggacttgcgcgtgtacgagcgcgagttcgccggcagctggctgcgccccgaccaactgccggtggaagcccgcgggatcgagatcctcgatccctcgggccgcccggtgtggctgctccaggacctgccatccgcaccggcgctgccaagccgcgcccccgtggtcgcgatgaccaacaccgcggcccatgcaccccgcatcaacgccacggtgcgcacgccgatcgaacccgcccgcgtggtgcggctcgggcatctggtgctgcaaacggtggacttcgccggcatggcgcagtggtacatgcacgtgctggggctgatcccgagcgacgtgcagtacctcgccgacggcagcccggcgctggccttcatgcgcctcgacctgggttcgcaacccgcggaccaccacacgctcgtcctggtcggcgccatcgaggagcgctacgaacacagcgcgtacgaagtgatcgacctcgatgcgctggggcagggacagcaggtgctgcgcgccggaggctggcggcacctgtggggcatcggccggcatctcctgggcagccagctcttcgactactggcgcgacccggacggattcgagtacgagcactacaccgacagcgacctcttcaccgcggactcgcagacctgctactcgccgctcgacttcggcggcatctgggcctgggggccggacgccccggcctcgatgaagcccggcaagaaccttcgcaccgcgctgcgcgtgctgcgcctcgtgctcggaaagcgcatcagcgtgcagcgcctgaagctgcttgcccaagccatggacgcgcccgcgcgtccgtggtcctgacccccaaccccaactggaaacctgacatgccacgcatcctgcttcgctgtgacgacggcacgcgcaccttctgggccgtgcagttcggcccccgcctcgcccccctggacattgctgccgcgaccaccggcgaactcctgtcccgccattgggcggccctctgggaggtccgggaggaccaagccaccgtgccgctcgccaaggtgcgcgtgctggcgcccgtgacgaccgaccagcagtttctctgccagggcgtgaactaccgcagccacgtgaaggagtccggactgaagctgagcgactttccgttcaacacgctcttcacgaaggccagctcgtgcatcacgccggccgatgccccggtcgtccgtccggcgaacgtgcaattgctcgactacgagatcgagctgggcctggtgctgcggcacgacatcccggcaggcaccgtcgtcgcgccggatcggctgcacgaatggctggccggcgtcacgatcgtcaacgacctgtcggcgcgcgacgtgcaactgccgcaaggacagttctacaagggcaagagcttccgcggcttcgggccggtcggccctggcatcgtgctgctgagcgccgacgagtggaagcgctggccgcagctgcgcatgcgccttgcggtgaacggacggccgcgccaggatgggtattgcggcgacatgatccaccagccggccgcgaccctgaccgaactcgcttcgatcgtcgacctgcatgccggcgacctgatcgccaccggcacgcccgccggctgtgcggcccgggccccgggaaagctggtcctcttcgtgatgcggcatttcctcggcgaggccggcaagtggcgcgccttcatcgcgaaggggcgcagcaacccgatgtacctgcgcccgggtgaccgcttgagcgcgaccatccgcaccgacgacggcagcatcgacctcggcgaacagaccacggcgatcgtggcgccctgaaacggaacgggccatcgccctcgacagcgaggcgctgcgcatcctgcagtcggtcggcgtgcaggagggcgacttcgccggcgtgccggatcaacgccccgcagcaccggcgagcgccgaccgtgcagccgcgatgacgggactcgcatcgttctcgtagaacgagagcaactcccgcaggcgttccggatccgcgctgccggatcccatgcgttgtgccgttgcaagcgcggtgagctcgtggaacgcggcaccctgcgagcgcgcgaccgcgatggagcgcgccaacgccgcggccgccgcagcgccgtcgcccgcttcagcctccatcacggcctgctgcagcagcaacggggagagcagcatccgctcggccccttcggccagcgccaggccggcttcgacgctcgcgcgggcgtccgcgtgacgtccggcttcgcggcaggcctcggcatggtggaaatggaagctggcgagccccgtgcgcattccgagctgttcaccggtcctggccgctgcacgcatctccgccagcccctcgtccacgcgcccgagggacaccagcgctcgcccgtgcagccaggcgaagttgctgcgtgactcgggcaccgtctcctcctgaatgacttcgtagaggcgctcggtcaaggcaagcaccgtgtcgtgttcgccggccagcgaatgcacgatggctgcgcagtacaaggcggcgacttcggtcagcgggtggccgccgcctgcagcaagcgccgtggcgcgctgcgcgaggctccgcgccgtggcgggctggccgatgacccagctgaccagcgccagcgccgcggtggcttccgattccgggtcctgcacgaagcgggtggaaggcagcccttcggcgccggcgcaggcctccagcgccccctgcagatactgctcggcgccgacaagatcgcccgtcatcatggacaccaggcccatggcattcagggccgtgatccggagcgcatggtcgccgttgtgttccgccagggaaagcatctcggtggccagcgtgcgggccggctcgaattcggcgcgcgcgaagtgcacccaccagcacccgtgcagggcgcgcggccacgaggggcagtccacggcgccgacggcccgcgcgcgctcgaaggccgcggcaacttccggttcggagagcacgtgcaggcggctgatcgcaacggcttcgagcacccgcaggtcttgttcgagcggcggctcgatgccgcccttgccgatctggagtgcacgccggcaagcgtgcagcgcctcgtgcgcggcgcctcgcgccatggcgcgcgcagccaccacggcaagctgcgccgccgcggcggccggcgcgccgccgcgctcgagatggagggccagttcgcctgcaatctcgtcgggtgcggaccggtggagcgcttgcagtgccgcggcgcagctgcggtgcaactgcagcttctgccccgcggacaggcgctcgtacagcacccggcggtagatggcgtggccgaacgcataccgtgccgcgatgcggccgtccgccagcgcggatgcgccggtgcttcgcacccagggcacgcgcgcggcggtgtcgtcgagcagccggagcagctcgggctccggcaactcgaccacctggttcagcaggacgtggaggaactcgatgccgcacacgctcgccgcgcccaggacgcgctgctgctcgtccgacaggcgcgagacctgccgctcgatcagcccggcgatgctgcgcggcaccgccagctggtcggcggcggggaagccctttccgggggcgatgctttccgaggccttcagttcatcgatcacgttcacgacgaacaacggcagcccggaggtgtgcgcatgcagggcccgcgcaaattcctcgggaacggattcgccgatgcgcgcttccaggtaggcgccgagctctgcctccgacagcgcttccagctcgatctcctcgcacaggcgaagcatgcgcagttcctggcgcaggtcggcgagcgggtgatcctccaggatcagttccgtgggacggaaggtgcccagcaccatcaaggccgcgggattgcgccggcgcgcgaggtatcgcagcagatgcacggtggcgtggtcactccagtgcaggtcttccagcaccagcaggagcggccgctcggcggccatgcggtcgatgaactcgccgaactcccgcagcatgcggtcctggttggcgccgccggcttgctgctggaggccttcctgctctcggtcttcgatcaaccagggaaactgcaagagccatgtgggtgccacgcgccgcatcgtctgcaccacgctggcaccgccctctccgcggcacagtgcgttcagcgcttccagcacgggcatgtacggctcggcgcgtccgtagtgttcgatgcattgcccgaagccctgcctgccctctgcggaggcggcgaagcgctcgacgacggtgctcttgccgatgccggcgtccccgagcacgaagacgaacctgcgctcgccgcggcgcgatgcggcgagcgccgattgcaggcgggcgaacgccgcgtcgcggccgaccagcaggcggtccggcaccaacgccggcacaagcgcaacgggcggggtcgccgccaccacggcagcgtccacgacaggcgcgatgaagcggtagccgcgccgtgccgcggtctggatgaagcgtgcgtccttcgcatcgtcgcccagcgcctgccgcagctggctcacgatgttcttcagggctgcttcgttgatgtggcggtggccccagaccgcatccagcagcgcgtctttcgtgaccagttgtccgggctggcgcaccagggcgcacagcacctggaaagcccgcggcgcgagttcgagggccgcaccgtcccgctccagcagtgcctgggcctcgtccagccggtaggggccgaagcgggcctgcaggggtgatgtctggttcatggatggatttgcaagctcgatcgataccgaatcgggaccgcggcgagacgacttcaggacgccgcgatttcaaactctcgccatgaccctgaacccgcacccgacctatcccgccgccggcgcgtacgtcatccggatgcaccacgacgcgaggcccgaatccggccagctgctcggccgcgccgagcacgtcgcaagtggcgacagcaccgattttgccaccgcgcaggaattgaccgcctggctgatgaggcacgcagccggaattcgcaaggcactgacatgacaacaaggagagttttgatgaacgttcaatgggccatcgcaccgctggcagccgccaccctgctggccgcctgcacgggcgaagccgccaagccctacgaggaggtgcggcccgtccgcgtcgccgtcgcgggccgcaacaccggttcggtgggctccgcctactccggcgctatcgtggcgcgctacgaaagccagttgggattccgcaccggcggcaaggtggtcgcgcgcctcgtcgacgtcggcgccatcgtcaagcgcgggcagcccttgatgcgcctcgaccccgagcaggaggcgctgcaggtcgtttccgccagcgccgacgtcgacgcggccaagagccgtgttgcgcaggcgcgcatcgatctgcagcgcagcgagcagctgctcgcgcgccagttcgcctcgcgcgccgagctcgaccagcagaagctcgcgctcgaccaggccgaggcccagttgcgctcggcccaggcgcagcgcgagatccacgccaaccagcgcggcttcacggtgctcaccgcggaccgcgatggcgtcgtcaccgcgattggcgcggagacggggcaggtggtcggggccggacagtcggtggtgaccgtggccgccgagggagagcgcgaagtggcgatcagcattccggaaggccgcgtcgacgaactgcgcaaggcgcgatcgctgcaggtctcgatctgggcacaccctggccggcactggaaaggcgtgctgcgcgaactggcacccgccaccgacagcgtgacgcgcacctacgccgcccgcatcacgatccaggatccggaccgcgagctgctgcgcctgggcatgacggcttccgtcagtgcgcccgacgtggatggcacgagcgcgatacgcctgccgctcacggccatcgtcgatgcagaggggcgccgccacgtatgggtggtggatcccaagacgacgcgcgtggcgccgcgcgaggtggtgctgggcagcgcgcaggacgacagcgtgctcgtcacctccggccttgcgggcggtgaaaccgtggtgacggccggcgtgcacatgctgcaggccggacagcaggtgaagctgcccgcgctgccgaaggccgaagaggcccggggagacgcgcgatgaagggcgtcaacctctccgagtgggcgctgaagcacccgcagatgatcgcgttcctgcttctgctgctgacggtcacgggcgtcatggcctaccgcagcctgggccagaaggaagaccccgagttcaccatcaagacgatggtggtgcaggcgtactggccgggaagctcggccgagcaaatggcggaccaggtcaccgacaagatcgagaagaagctgcaggaggtggccgacatcgactacacggcgacctacgtgcgaccgggggagacccagatcaaggtcaacctgcgggacgcgaccgcgccttcggcggtacccgacgtctggtaccaggtgcgcaagaaggtcggcgacatccgcgccaccttgccggccggcgtgcagggcccgttcttcaacgacgagttcggcgacaccttcggcaacatgtacgccctcacgggcgacgggttcggcaaccgcgaactgcgccagttcgcggacgcggcccgcaacgagttcctgcgcgtgccggacgtgaacaaggtggatctcgtgggcaagcaggacgagaagatctacgtcgaagcctcgaccgccaagctggcctccctggggatcgacccggcgctcatcgcctcgaccctggcccagacgaacgccgtcgcggccgccggcacggtgcaggccagcgccgagcaggtgcggctcacggtgagcggcgagttcgactccatcgaaggcatccgcggcatcggcatccaagcgggcaaccgcaccttccgcctgggcgacatcgcggaggtacggcgcggcttcgccgatccggcggtggccaagatgcgtttcaacggcgccgaagccatgggcctggcggtcagcatgcgcaagggcggcgacgtcatccgcctgggcgcggagctggacgagacggtgaagcgcgtgcaggcgaacctgcccgtcggcgtgcagatccatgccgtgagcgaccagccgcgggtggtggaggaatcggtgcacgagttcaagaagagcctcgccgaagcggtgatcatcgtgctggcggtcagcttcctctcgctgggctttcgcaccggcctggtggtggcgctgtgcatcccgctcgtgctcgcgctgacttttctcgcgatgtacctgttcggcatcgacctgcagcggatctcgctcggcgcgctgatcatcgcgctcggtcttctggtcgacgacgcgatcatcgcggtggagatgatggcgctgaagctggagcaggggtgggacaagttccgtgccgccacctacgcctacaccgcgaccgcgtttcccatgctgaccggcacgctgatcaccgccgcgggcttcctgccggtcggctttgcgcgctcgggcacgggcgaatacgtcgtgtcgctgttccaggtggtgggcatctcgctggtgctgtcgtggatcgtcgcggtgctgttcaccccctacatcgggttcaagctgctgaaggagaacccgcacgccgcgcacgacgaggaggcggtgtaccagcgcggcttctacaagcgcttccgccgcttcgtggatgcctgcctggtccaccggcgctgggtcatgggcatcaccctggtgctgttcgcgggatccctcgcgctgttcaagctggttccgcagcagttctttccggcctccgaccggcccgagctgatggtggacctgtggatgccgcaggcgtccacgttcgaggccagcgcgcgcgaggtgcgcgaggtcgaggccatgctgcgcaaggacccggacgtggtcgcggtcaccagctacgtgggcaccggcagcccgcgcttctacctgccgctggacgtgcagacgcccaacctgaacctgggcgagctgatggtgatgacgcatggcggcgaggcgcgggaacgcgtgctcgtgcgcctgcagcgcatcttcgaccacgagctgcccagcgtgcgcggccgggtgaaccgtttggagaacgggccgcccgtgggctatccggtgcagttccgcgtcttcggcggcgacgaccagcgcgtgcgggagatcgccggccaggtcgccgacctcatgcgcaccaatccgcacgtgcgccacgtcaaccaggactggggcgagcggaccaagcgggtgcgggtggacgtcgaccaagacaaggcgcgcgcgctcggcatcagctcgtggcagatcaaggcggcgctagagggctcgctgaccggcacccccatcacgcagttccgcgaaggcgaccaggacatcgacgtcgtctcccgcctggtggcggctgagcgcaccgacctgaacaacctgaaggacgcgaagatctatctgcgcgaagggaaattcgtgcccgtgtcgcaggtggcgcacctgaccctcggcagcgaggaaagccagctctggcgccgcaaccgggtgccgacgctgacggtgcgcgctgacctctcgggagccgaagcgcccgacgtgacgcgcgccctgcttcccggcatcgacgcgctcaccaagcagcttcccctcggctacggcatcgaggtgggcggcgcctacgaatcgagcgccaaggccgaggcgtccatccttgccgtcatgccggtgaccatcgtcgtggtcctcctgctcctgatggtgcagctgcaggacatgaagaagatggggctggtgctgctcacggcgccgctaggcctgatcggcgtcagcgccatcctggctgccttccgcatccccttcggcttcgtggcgatgctgggcgtgatcgcgctggccggaatgatcatccgcaactcggtgatcctggtggtgcagattgaccagggcctggcgaacggtgcgccgctgtggaccgccattgtggagtccgccgtgcagcggctgcgccccatcctgctgactgcgctggcggcgatccttgccatggtgccgctgacgcgctcggtcttctggggcccgatggcctgggccatcatgggcgggctcgcagtcgccacgctgctgacgctcgtcttccttccggcgctttacgccgcctgctaccgggccgaacggccgcaatccccctccgccgaagcggcgacaggaacctgatcatgaacgtattccccccaagcgcccgctgggcgctgctggccgcactcggccttttttctgccgcggcgaatgccgtggacctggtcaccgcctacgaggccgcgctgcagcacgaccccgcgaagctggccgcggaccaggcacgggtcgcgggccgcgaactggccgtgcagggcgatgccttgctgcgcccgcagatcagcctgcaggccggcgtgagccgcatccacgatcgctcgtcgggcaacatccctcccgcgctggcgtcctacctgtcttcgtccgccacaggcacggtaagacaggccggcgtggtgctcacgcagcccctgtacgacgcgaaggcgagcgcgcagaagcagcagcttcacctgcagtcggatctcgcggagacgcagttcgagcagtctcgccaggacctcgtccagcgtgtgtcggaagcctacttcggcgtgctgctggccgaagaggccctgcgagtcgcgcaggcggagaaggccgcgctcgggctgcagcgggaccgcgcccaggcgcgattcgacgtggggcgcggcaagatcacggacttgcgcgaagcgcaggcgcgctacgaccaggtcgtgacgaaggagatctccgcgcgcagcacgctggatctgcgccgggccgggttccgcgaaacgaccggcttgcccgccgaagggctggccggacttgcggagggcttcgtccccagcgcgccggttccgggcggcctcgaagcctggcaggaacgcggcgaggagcacagcacgctcgtgctcgcgaagcgctcccagctcgagatcgccacggccgaaatcgggaagtaccggcttgccgcgcggccgacactgaacctggtggccagctatacgggcacggggcaaagcggcaacctgtcgccgctgcagggcatggatggccgcagcacgggcagcgtgggcctccagctcaacgtgccgctgtacgccggcggaggcatcgactcgcgcgagcgtgagtcgatcgcgaaacaaggccaggccgagcaggaactggccacggcgcggcgcgatgtgcggctgcgcgtgcaggatgcgttcctcgcggtgacgacgggcgtgtcccgcgtggcatccctcacggagtcgctgcaatccgcccgcacggccctcgaggccaccatgctcgggcgcgacgtgggcacgcggacggcgcccgacgtgctcgatgcgcagcagcgcatgttcgaagccgagctcgcgttggcgcaggcgcgcttcgactatctgctcggccgcgtccgtctctccgcggcggccggtgaactcggcctctccgacgtgcgcaccctgaatggcttgcttgcctcgcgctgagaggaccggtgccatgcggtcccccttcgccctcgccagcaccgccgtgcgcctggcctgcgcctgcatggcgagcgcgctgctgctgggctgctcggcggcccgcccctggatcaacgcgccggtccgcaactccgcacccgctcccctgcccctcttgatgcaagcgcagccgcagcatgccgaagccgttcaggagcgtccgatcgtcgccgccgtggccttgtcgggcggcggtgcgcgggcagcggcgttcggcctgggcgtgctgcaggaactcaaggccacgcagctggagatcggcgggagaaaaaccaccttgctcgacgaggtcggcctggtcagcggggtttcgggcggcagcatcctggccggctactacgcggccttcggcgacgaggttttcacgcggttcgaaaaggactttctgctggtgaacttccagaacggcctgctgcgccaggcgctgcatccctccacgttctaccgcctcacttcgccctggtggggccgcggcaacgtgctgcaggaacggctggatgccgtcttccgcagcgcgacctacgggcagctgcgcacgcggcggccatggccgcgcctgctggtcaccgccaccgacctgaccacgggcgtgcccttcgagttcacgcccgaacagttcgcgctgatctgctcggacctggattccgtgcccttgtctttcgcggtggcggcgtcgtcctcggtgccgctcctcctgagtcccatgaccttgcgcaaccatgccggcagctgcgaccgcccggcgcaggagcaacagccgccggtcaacgcggaccggaacctgtcggcccgcatgctgcatctcatcgcgcagagctacagcaacgccgcggaccgcccctacctgcacctcgtcgatggcgggctcgtcgacaacctcggcgtgcgtggcctggtcgaccacgccgccgcgggtggttcgctgcgggagagcttccgccacctgccgccgggctccgtccgcaagatcgtgctcgtgagcgtgaactccgaacgcgacatcggcgagcggctggacgacacggatcgcgtgccgagcacgggccaggttttgtcggcgctggtgttcggggccggaagccgctacacgaaggagacgatcgagatcgtgcaggacacggcccgccgcgcggcggccgagctggccacggagcgcggccgcgacggcagcccctttgccgccgatgcggaattgcacctgatcaacgtcagcctgcatgacgtgcccgacgccgggctgcgccgcgcagcgctgcgcgttcccacctccttcgagatcctgccggtccactcccaccaactggtcgcgggcgggcgcagtgccttgcgcgaatccccgcagttccagcaactgctgcgcagccttggcggccccggaaaggcggcgggccttgtcgcgagcgacgccgcgggccagcagtgagcatccccgccatgccctctcttcccgacatgcagctctattggagcagcagcttcctggctgccaacgcattcatcggcttgaacctgctcggcgcgctcgtgctgggcatggtggtgggttacgagcgctcctacaacggccgcgccgcggggatgcgcacctacggcctcgtgtgcatggcctcgacggcgctcaccatcttcgtcggctttgcgccgttctggtacggcggcgcggcctcgcaggtcgcgcccgacgcgacgcgcgtggtccagggcgttgtcacgggcgtcggcttcctgtgtgccggcgtcatcgtcaaggatggcctgaacgtcagcggactcacgacggcagcctccatctgggccgcctccgcgatcggtgtgctgctgggcgtgggcctctatgcggcggccttgctgctgtcggtgctctgcatgctgtcgatgtcggtcgtccaccagatcgagctgaagctgccgggccgttccatcttcgacgtctccctcagcttttgcccggacgccgccccggagctcgaagagctcacccaggtcgcgctggcgcacgggtaccgcgtgatgcgcgggagtttcagcgtcatgtacagcgacaacgttcccgtctggcggttctgcgtcgtttcgctggaccgctcgcgctccacgtcgcccgcgcagatggcccagggcctggcgcgttccggcgatgtcttgcggttcagcattgttccgttgaagaactgagtgccgctggagcaagccttctagccagtccgcgagcggcgccagcgcgccggcccctccaccgtccagccgatgccggccgccgggtcgaggtcgcgatggcagcgcgtgagtccgtcgtccaggtcgagcgtgacgccgatccgccaatggccggcagcgccgcgctccacctgcagcacggcgaagccgttgcccgtacccacggcggccgtgaccatcgtggcgacgaaggcaccgggcacggggccgagttcgacctggccgtcgagccagaacgcgtcgggccgcgcattgacgaaggtccagggtgcatacaggcccgaggacacgaccgagatcacctcgaccggcccgtccgccgcctgcagccagaggctcgacacgctcgacatgtgccggtcgcccgacagcagcaccacgtggcgcgcgcgggtgtcgcgcagcagttcgagcagcgcgcgctgagaggccgggtacccgctccagtcgtccagccctaggcgctctgccaggtcgccgaaggcggcggcgcgcggcatcgggaacagcgccaccggcgagacgatgaacttgggcaacgcggcgggcgcggcctccagccactttttcagatcgcccatgccggcctcggcgcggatcgctgcgtggtccaacggggaggcttgcgcgtccgtgcgcagcgcccgccgctcgcgcgtgctgcgcgtgtcgagcatgtagaacggaaagccggccggcgccacgcggtagtcgaagggacgctggtcgaggtgcgggccgatgccgcgcaccagcttgtgctgctgcgcgaagtagccgtcgagcgcggcgcgcacggccggcgttccatagggatcggggtccggctcccaatcgtccatcacctcgtgatcgtcgagcaccggataggtcggcagcgaggccatcacctggcgcagcgcctccagcctgaagctgagcgcataggcttggccgacatcgtcgccgccggccggcacgaagagccccgcggtctggtccacgtacacctggtcgccggccagcaccagcaactgcggcttgtgcggtggcgcgagcagctcgagtcgctgcgcgaggcgccgatacgacgcctgtgcgggcacccggtcgaccaggcccggcacgtactggcaactggcgagcgcgaagcacagcgaggcctgcgcgagctcgccctcgcgctgcacggcgccggtccaagcggggtcgagacgcaccatggcgcgctcgcgctgcgcgtcggtggccgcgtccagcgtccgcatcacctgcttgcggatgggctcgttgggttcgtcctgcggctctgcgaacagcccgggcgcgagccgccggcccagcacctcgacggggccgcgcgccatgggcaggtcgtcgtgcgccgtcagcaccgcgaagccctggtactcggcgagccggtcgtcgaagaggtcgatctccaccgcctcctgcaagagcttttcgcgcgtggtctcgagcgccaccatccattcgaagtcgaagcaccatcgcccgtcgcggcgccacgcgggtacgaagaccacggcgcgcgccgacacgtgcgcggggggcgggcgcagcgccagccggcaatgcagccggcccgcgttgccggccgcgcggctcgcatggccgagccacgggccggtccacggcaggctggcgcgccagtcgggcggcaccggctcgccggggccgggcttcttgtcgaaggcctcgaggaaccgcacgatgtgcgggaacacgtcggtgcaggccttctcaccgatcaacgtgtcctggtggccgtaggcgccgagcaccagcagctggtgcggcgtgccttcgccgaggaacaggtcgcccgcggaaggcttcgacgggtccgacgggtccggcagctccggtggttcgcgcggcaggccgccgtccttgccgaacacgcgcttgagcagccagaagctctcgtacgaaccgcgccagtcgaacaccgcgttgcgctgcccgtgcagcatgaacaccggaaagccgaagcgctggccgacctgctcgaagccgaccgcgtggccctgcccaccggcgtcggtcagcacctcttcgcgggcgtagttgccgacctgggcaaggccccgcaccttcacgaagccgtagatcgaatcgagcgcatcgagcgtgtccttgccgatgttgtgcagccgcatggtctggccgaagatggcgtcggcccggtgccgcacggccgcgaagcccggtgccttgcgcaggcgctcggcctcgccgtcgtcgtcggcgtagggaaaggtcgccagcaggccgtcgacgagcaggcgcttcatgggcgtgagctcgggccgcgtgtcgaactcgtcggtgccgacgaactgctgcaggtagcccgccacatagccccggaagcggttgaaggccgtggcgcgcagcagcggccccacctgcgacagcaccaccgcgccgatggacgcatgcagccccggcaggcgcagcaccgccacgctgaacatggcggagccgatgcagtgcgccaccacgtcaacctggaccggcgccgcgtcgtcgggcgtcgcgtatgccgcctgcacggtgcgcagggcatccggaatatcggcctcggccacctcgtcgaacgaccagtaggcgcgcggccggttcgcgaagccgatgctggtgcgcaggtcgagcacccagacctcgcgcccggccgcgagcaggctgtgcaccaggttgcggggaatgctcttgtgcgcaaaggtggaaccgctcgcgccatagccgtggatcagcatcacgggccgcgtgcccgcgcggcgcaccggcggtcggtagcgcgacagcagccgcggcggcgcgctgcccgggccggccgcggtggcgagctcgacccgttcgggccgcacgccatgcacctcgcccggcaggcgctcccagtcgcgctgcggcgagtcgggcggcggcacgaagtgcagcaggtgaacgtgcagcacgatgcgcagcacccacagcgccagctcggccaggtcgcccagctggttgggcatgtcctgctggtgctcgacgcgcagcaggggttgcagctgctcgacgaagtaggaagggtccagcaccatgcggcccagcggcttggcttcatcaaggccgacgtgttgcagctcgccctcgctcaactgccgccacgggttgccgccttcgacgaacgcgatgcgcttggtgagccgcagccggtcgcccaccttcagcggcgcgccgcgctcggcccgctccaccgcccagtcgtattcgatgaggcgcacctgcccgaagtgcgagcacagcgccatcaggtccgccatggccgggccttcgaatgtcacgctctcctggccttcgttgccgctcgggctcgccacggacgagcgcgcagccagcagcacctctgccagcgccagcagcttcttgcgcgccagcgcgtggctgcgcaggatgcgctcgatgctgtcgctcttctcgcgcaccagcatcgatgcggtgccggtgcaatgcgcgacgggcgcgtcggcgcccttgccgaagcgcaggaccaccactggctgggccagcgcgcgcggcgccccgcgcaaggcaggcacgtcgatgggctcgaactccacctcggcgctcagcgcgaaggcctggccgtcgatatgcactcggcccgtcatgcgctcacgcaacgagacgcgcgtgggcgcgggcgcgcggggatgggtcaggtcgcggcgcaacgggcgctccgacgcgggcggcggtggcgaaccggccagggccagggcccagtcggcggccagcactggcactgcgcgctcggccagcgcggcgatggtgagcgaagggttgatgccgagcgacaccggcacgatggagccgtcgagcaccgccaggcccggcaacagcgacggcgctcccgctgcaccgtcgtagacgcggccccagctgtcgaccacgccgcgctcgggtccatcggccatgcggcagccgcccagcggatgcaccgtcagcaccgagcccaccggatccagcaggccctccaggctgcgcaacggcggcagcgggttccacaacggattgggcagcacgcgcccgccgaggccgcccttgccgtcgtgggccgcgtgcagcgcacgcatctgcgccgcgaacaccggcagggccgcgaccttgtcccacatgacgcgcacctgcgcatcggccagcaccttgtcgctaccgccgcagccgaccagttcgatgctgccggcggcgccgtcgtcgcccatcattccgtagaccggcgtgcggcgcagcatgtcgtcgtccacggccagcggatcgcgcacttcgtcgggcgcgtggaggtcgaggtccatgtgcgcgagcgcctgcagcgcgtcggtggtggtcaccacttcggccagcaggcggcgcagcggcgcgggaatggcgaactcctcgatcaccagtgggcgctcgcccttttccccgcaggtgcgcagcaggccggtgatggtcgggccgatgccgcgctttgcgggcgcgtcgccttcgggtgcgctggacagcgcttcgtcgtgctgcgcggccgccaccgcgatcatgtcgccgttggccgagaagccctcgcccagcgcctgcgagatgggcaggcccgcggccttggagcgcttgagcagctctgtggaacccagcgtgccggctgccaccaccacccgccgcgcgcgcaccacgtagggccgggcgttgtcggtgcgcgccttgcgccggtcggtgaagaagaactcgaccgcatagccggccccgcccggcaaggccgcgatgcggtacgcggtgccgccggtgaagaggcgcgcgccgcgtgcatgggccagcgccaggtagttggtgtccagcgatttcttggcgcggtggttgcagccgctcacgcagtcgccgcagcgcaagcaccgatgcatcgccacctgggccggcgtgcgcgtgccgtcctcaaaggcgatggcgacgcgggccttgccgcgcgacgccgcatgcaggcgcgcaccggccttcagcagggagtcgagcttcgacacgctctcgggaatctgctccaacgccagcatggcctcggccttgtcgtagccctccgccagcgccgcgaggtcgaggcccgtgggccaggcgccaccctcgaaggcatcgggcgtggcacgctccatcaccgccgcgttgatgagcgacccgccgcccagcccgttgcccagaagcgcgttcacgtccccgcccaggcgcaggtcgaacagccccgaggcgttgccgcgcgcgggcttgccgtcctgcatgctgaagcgcacatgccccggcagctcggcgaaggtggccggaaattcgcccggcaggtattcgctgccacgctccagcaggtagaccttgatcggcaccgcgccgggtgcgatgccgggcgatgcgtcgaccgacagcgcgcccgccagccgcgccgccgccaccgcgccgccgtagccgctgccgatgatcagcacgtcgcagtgcagcgcgccgggcggcgccgcgaggatctcgcgcaccagcacctcggcaccctgcgagagcaggcggtcgcccggggcatcgtcagtgtggcggccgccgtcgttcatgttcggctcctcgcgggatgggtggcgaattcaggaaccttcgatggccgcggccagcgcgcggccgagcccccggtcgtcgacgggcttgcgcagcagcggcagcgcctgccgccgcgccgcctcgaccaccgccgggtcggtgtcggccgtgaccatgacgatgggaagcgcagggtttgcggagcgccgcgcgcgcaggcgctcggcggcatcgaagcccgagacgccgccgccgagccggcagtcgaccaccaccgcatccggctcgccgacctggcccagtgcctcgtcgagcgtggcggcggacagcacgcggcagcccatcgcgcccagcgcattgaggtaggcgccgcgcaccatcgggtcgtcctccagcaccagcacgcagcgcccggccaggctccacggtgtgtctgcgccgccaccctcagggccgtcagcacccacgggtgcggcgcgcggcaggcgcagccggaagcaggcgcccgcgccgaggctggactcgagctcgaccggcacgcccagcaactcggccatgcgccgaacgatgcccaggcccaggccatgccccgcggtgggcgcggcgccggagcccggcgcctggagctgcaccagatcctcgaacacgagccggtggttctcgggcgcgatgccggggccgctgtcctgcacggtcaactcgacttcttccttcgacgcgtcgggtgcttcccgcgtgcggacccgcacctcgacctgcccgcccgcgggcgagaacttgatcgcgttgtccatgaggttggccagcatgcgccgcagcagatcgggatcggtgcgcacctccaggcccggcgggcagtccgtgcgcaggccgacgccgcgcgccgacgccgcggcgccgaagctggcgatcacggcggtcagcagccggtcgatccgcacacgctgaggctgggccaccaccacgccggcatcgagcttcgacacgtcgagcagggcgtcgagcatggcgcgcagctgctccaggctgctgtcgaccacctcgacgatcgcgcgcgcatcgggtgccatcgccacgtggcgcagcgcgcccacgttgagggccatggcctgcagcggctggcgcaggtcgtggctggcgccggccaggaagcggctcttgtcgttgttggcgcgcaccgcctggtcgcgggcgatggccagctgcgcgcgctcgaactccagcgaagtggccagcgcctggttctcggcgcgaatgccgaacgactcctcgaaggtctgcaggttgcgccgggcaaagcgcgtctgcacgccgaagaacatcagcaccagcgcggccacgccccagccgagccagccgccggccaccagccacatggcggccgtgggcacgaagagcaggcccgcataggccaggaaggcgggcatcacggttgcgctggtggacacggcgcccgcgccccacgacaccaggatcatcgtgaggaccgcgtcgagtgtcgggtcgagtcgggccatgaagagagccgcggagccgttgcaggcaccgatcagcacgttccagtacacggtggcgcgcagccgctcggcgatcgggcgggcgcggtcggcggccatgcgcgcgagcgcggcggcgcgccactcgcggctcgcgatcaccgccgcgaaccagccgagcacccagggcgccggaacgtcgcgccagacgatggccgcgacgacgacggcggtgagcagtatctgccagcgcagccccccggcctgctcggcgaccacctgcaggcgccgttcgtccagctcgtccagcgcggccggcatgctcacgtggcctcgagcgcccatgccgcctgcgcgtcgaagacgcggcacatggcatcggtgcggttgcgcgcgccgagcgcccggtagaccatcgacaggtgcactttcacggtgccctcggcaatctgcaattggcgcgcgatcagcttgaccggcatgccccgcatcgccagcgccagcacctggcgctggcgcggcgacagctccacgcgcaggaagccggcaaggtcttcgcgcggcagctcgtcgggctcgcgcgcgcgggtcacgtcgtcggccagcacgaactcggccggcaggtagatgcggtggcgcagcaccacgcgcagggcggcctccatgtcctcgagccggtacgacttgggaatgaagccggccgcgccggcttcgatgacctcgcgcacgcgctggggcgagctttcggccgactgcatgcacacgggcgtggcctcgaaatgcgccttcacggccttgagcgcggcaactccggagagctggggcaggtggtagtcgagcagcagcaggtcgacgccggcggggtccagctggcaggcttgctcggcgtcccgcacggcctcgaagtggaaggggcggccgggttcgatctcggcggccatgcgctccagcaggaggcgcgtgccgttccagacgatctcgtggtcatcgaccagcagaaccttcatacaggcctctcgtctacggtgaccctccccgtccgcacgcaggttagcgcaaagccccccaataagcgagcgcccgcacctacaccaaaggcctagtccgatggccacgccgccactgcgcggcgggactaggccgccgaccggaaaacgccccgccagcgcctaggcgctgcgttcaattgttgcggcggggcccgcgcggaagactgtccgcatcgatcgccacttcgcatccgatgcaccgaggaccgccatgaacacccccaagtctcttgccgcgatacgtgccgcatgggaaccccttgcgtgccggttctgcctcctggcgctccaccacgtggagctcgcgcgctggctgtgcgccgcggccatgatcgcggtctcgctgctggcgggctgcgccgcattgcccggcgacgtgcaccgggtcgcgtcgcacgcgcgcaccgacgtcggggacagcgccctggcgcgcatcgccgccgcgtcgctgccggctccggacggcgcgatgtccgagacagccgacatctccggcgtgcgactgctgccgggcggcgaccaggccttcgacgcgcgcatcgcactcgcacaggccgcacggcacaccgtcgacgcgcagtactacgtggtggccgacgacacttcggggcggcaattcctgcgcgagttgcgcgacgcggcgttacgcggcgtgcgcgtgcgcctgttggtcgacgacctgtacacgggcggagaggacgagatgctggccgggctggccgcgcacgccaacgtggaggtgcgtgtcttcaacccgctgccggtgcgcagcggcggcctgcgcacgcgcgtgctgctgtcgctgcacgagatcggccgcgtgaaccggcgcatgcacaacaagctcttcattgccgacaacagcttcgcaatcacgggcggacgcaacgttgccgacgaatacttcgggcgcagcaagcctgccaacttcatcgacatggacgcgctcctggccgggccggcggtgcgcgcgctgtcggcgagcttcgatgcgttctggaacggcccgctgtcataccccttcgaggccatcgcggccggtggccgcgcgacgccgggccctgcgcgcgaacgcttcgccgcgctggtgcgcgatctcggacgcttcatgcctcctgccgacgagcccgatgcgctgggccgccgcccggtcggcgcgcagctggcgcaggggcgtatcgagctggtgcccgcgaaggtgcgcgtgattgcggacgcggtggtgcaaggcccctccgcaagggacgcgggggacgccggcgggaacgtcgaggaagccgcggggccgcaaggccgcgagggcgcggtcatggccgcgaacctcgatctctttcggaccgcgcgctcggaggtgctcgtcgtctcgccctacttcgtgcccatgccccgcatgatcgacgcgctgacccatgcgagccgtgagggcgcgcgcgtgtcggtgatgaccaattcactcgccaccaccgacgagccgctggtgcactacggctacgcgcgctaccgcagcgcgctcctgcaggcgggcgccatgttgtacgagctgatgccggcgagcgaaccgcatcccgccgggagcgacaccgaaagcggccgcggctcgctcggccgcctccacgccaagctcgcggtggtggaccggcgctggttctacgtggggtcgatgaacatggaccggcgctcggcgcactgcaacaccgagctgggcctgatcgtcgacagccctgcgctggccggcgagctggcggacctgatccagcacgtgcgcatgcccgcgagcttcaccgtgagcgcggcaccgcggcggggcggcctgcaatggagcttcctgcgcgatggccgccgctgggtgctgcaccgggagccggaatcgaactgggcccagcggctgcgctggtcggtgctgtcgctggtggtgagcgaggatttcctgtgatgcggcccgtgcctttgccccctgccctgccctttcgccggtgcgccttcatccatgcgccagcagcatcttcatgaacgtgatgccgttgcgctgccctttgtcctcgtcgcagttgttgaagatgatgtgcgtgttgcgcaccttgtaggccaggcgcaccacctccgccatgatctcgcgcagctcccggtcgggatagtcgtagtcgaagcgctcggccgccgaggccgcgcccttgatgttgtaggtgtcgacattgcgcccgtgcaggcgcaccaatgcgaagtcggcgttggtggtctccgccagcagcggcacgctgttggcaaagccctgcgggccgtcgacgacggtgtgcacggccccaagcttgcgcaggaactcgacggtgccggcgcgatgcgcttcgtcccaccatgaccggtgccggaactcgatgctcaccgtgtggccggccatctgctcgacgcaatgcgccacatgcgcatgtccctcgcggttgcacaccagccagggcgggtactggaagtgcaccagcccgagcttgctcgcctgcctgagcggtgcgatggcctcgcgaaagcggcgccacaactcgacgctgatctcgggcggcatgccgcggtagtagaaggccttggtggtggtcgtggccagggcttgctggatgtccttgtgcagcaccttgggatcggtctggtggccggtgaacagccggaaggctttcacgttgaaggtgaaggcgtcgggcgtgcgctcggtccagagccttgcattggcgggcgctggaatgccgtagaagctggagtcgatctcgaccagcgggaagatcgacgcgtagtggcgcaggcgcgcctcggaggtcttcgcctccttcgggtagaagcgaccgcacgcgagcagcgtcttgtcagtccatgaagccgtgccgaccaggatacccatcggcgcaggctaccggttgcagccactcgaccgcagcctccgtgggcgacattgtgcgtaggcggggatcgcgccaaagctcgcgcgcgacctcctccagttccagcggatcgacggtatgccaccgctgctgcagccggtgcgcgcaagcggcgatccagaggggtgcaggaatggggtccatgcctcgatgatactgtatttttaaacagtactaataaggttttcaaaatatgtcgccgaagtgggtcgccggtactaacattcaaccgttcgacgcgtggctcggcacgaggctgccgccgacgatctgctcgctcgtgccaggagagtcgcgatggcaagtcccatgaacgtcaacaagctccagacgaaatcccatgacgaaccggacgaggttcgggagcccgaaaagacccgggtcgaagtggtccgcctcgagggctacacgctcggacgcttcaaactcgagcccgggtggcgctggtcgaagtgcatcaagccggtcgtgggcacggacagctgccaggtggctcacgtcgggtatgcggtttccgggcgcatcaccgtgcagatgaatgacggtacgaagaccgtcatcgaggaaggcatgtcgtacaccattccaccgggccacgacgcatgggtcgaaggcgacgaccggttcgtcgccttggagatgatgagcgcagaggaatacgccaagcccaagagctgatccggggtgggggccacaggggcagatttctgcgggatggtcgaacgggggatgcggtccggcggactgatcacaatcgcctgcggcggcagcggttctgttgcgccgcgaaaccgttcgattcttcctccctcagcgatacatgtttgccctgacccgcctgacgatcgaccgcgcccggaaagagcgcctgccccaagttgccggaagcctggcgttcacgaccttgctgtccatcgtgccggtgctggccgtgagctttgcgctgctcacgcgattcccggttttcgcgcggttcaaggatgcgcttcaggagttcttgctgagcaggctgcttccggcggacattgcgcgcacggtgctgaagtatctgaaccagttcgccgccaacgccaacggcctgacctggatgggttcactcttcttgctgggcgcagccatcgcgatgctgctcaccgtggagaacgcgctgaaccagatgtggaaggtccggaagaatcggccgttcctcaagagggtcggcctgtatctgctgatgctggccgtcgggccgcccgtgctggggctgagcctgtgggccacgtcgtatctgctgggcatttccatgggcctgatcggcgcgctgccgcactcgctcgcattcgtgctcgacctcgggccgctcatgctcggcctggctgtattgacgagcatgttctacctcgttccgaacaccaaggtgcggctgcgtgacgcctttgcgggtggcttgatcgccagcgtggcttttgaactcggcaagcgcggcttcaccaactatctcgtgaaggtgcccacgtacaaggcgctgtacggggcgttcgcggcgcttcccatgttcttgctgtgggtctacttctcgtggctggtcacgctggtcgcggccatgatgaccgccaacctggcgctcacgcgcagacggccggccggcaagcccgccagggggtaatctccgtctcgatgagcccaccgcaaccccgccccgccgcatccatctggaatcgcttctggtccccgaagagcttcctcgaacagattccgccagaggcgtccgcggccgaggccaaagccatcgagcacaggaacaacgtctggctcagaacctacatggacatgtacatcctgaggtggggcgggctttgggcggcttcgtcggcagcagctgttctgatgacggatgcatcggctttgctgttcgcactcgccctggtgtcgaacctggcggctcttgccggcttggtgctcatgatcctggcctatcgccgcgcgtccaaggctgttcaagaggacgctcagaaaggccggcactgatagcttgacgcctgcgcgcggtcaccgccgatgtagtgcgggtagccgggatgccggcacatgggacgcgagccctgcactgcaaacggcggaaggggcgccttgacaacctgcaccagggcattcgcgggtgcgtcgccagcgttcacccatcggtccagcggatccagcaggtccaccatcgtcggcactgccggcccacccgcgaccgcgcgagagttgccggcatgcgtcgagccgggtgagacgtaaagccgcactgagctttcggccgcggcggcgcccaggcgcgccacgagtgcatcgtgatattgaatgcccatgagtgcgctctgtgcgcgatccgcggcgttctcgcgcaggatcagcttgccaccgcgcccgaagaacgccgacaggtccgggttcgtggagtccatcaacgccgaggttttctgcacctggtcgcggaaatcctcggggcgatagccgcgcacgtcatggttcttgtcgcgcgcaatcgcatagcggatccagttgcttccatagatccactgggtggaattgcgcgcggcgtccggtggcgcggcgggtgccgctgtgccggaaacccaacgcaccatgctgagggcggaggggccgtcgaggctgtcctcgtgcccatagagccattgcggatacgctgtgaggccgttggcgatgggaaagggaaacacatagggcgagtgaatgccgcgcatgagacgcaactcggcatcggacaggcagtgcacgccggcgtcgctgccaccagggcagcgcaagcgctgcagatccacgcgggcctggcaccccatgtagttgctcacgacaccatcggccagcccgtcgagcgcgtcgcatgcgtcggcagtggccttggcaatgagcgctgttttttcggcctgcagccagtcttcgtgttgcggtacctggttgcgcacgaaggcatggaacaggccggtccagttgatcacggggacgacgctcacgatgccgtcgtagtcggcaggaaaccgctgcgccatggtcagcccttcgcggccgccttcggaaccgccgaagtaatacatgcgctgcggttggcgtgcgtagtacgcgcgcatgatgtccacggccacgtccttcaccttcttgtaggaagcgaaggcgaagttctcgagcatctcgtcgttcagcgcgaaggcgccgggctctccggctggaaacgcggaggcctgatggccggagtcctgaccgaaggtcgcatagccccgcgcaatggggaggggatcgtccggcgccgcatcgcgcagaggcgtcaacccggtgatcagcaccccgttgaagcccccgccaccgtactgcagggccttgccgttccaggtggtcggcaggttcaactgaaagttgatggcctgggccgcggggtcacgcgatgcaatggtgccgctgaccttgcagaactgcggcagggccggtgcgaacgccccgccattgaccgccgcagcggaggccggcgtgagaacagccgaagcgaccgaggccttgccgctgggcaatcccattgcgccgggtgcgacgacatggcgcgcgaggccggcgcaggcgcttgcgagccggtcggcgttcgggaccgtgccgcacgccgacaaagacaaggcaagcagcgcaaaagcggtgcgaggcaatgtccggaaagcgaaatgattcatggtgtctccaggcgcttttagtacatcagctggtcagggctgtgatagtgcattgaaatctcgccagagccccatattcgccgcacacctgacttcagaacgcgtggcgcagcccgaagtcgtagcccgtcgcgctgcgcggcgccaaacccgccacacctgcacctgtcgacgcgaaggcggggcccccaagcccggcggccatgatggcaggattgttctgtccgttcttgatccgggcacgagccaccgtggcgtagagcgcggtccgcttcgacaggttgtggacgtagccgagcgcgagcttgttcaccgaggcgtcgcgatccagtgcctgcaaagccggtgcggcggaactctggtcgttcttgaacttgacgcgagcgtatgaagccttcaatacgccggcaccgaccggaacggtcatgccgatcatggcgccgttgtactcgtcgttgtcggtgaaggttcgtctgccggcgctcaagggagcggtggtggtctcagccttgtctttgacctgcgacaactcgcccatcagcttgaggacaccgaaatcgtaggacgcgcccaagttgatcgtgcgcagttgctcggaaagccgggtgccggccacgaccccggcctcgctgatcaccaaggtgtcagctgccgtgctctttccgtaggcaaccgccacatcgaccgggccgcttgtatagccaaaccgcccgccgtagtagcggccacgcttggatggagtgtcggacaggtagctgtacttcacggtctcaggcagggcgtacatgacctgaccgtagaaaccgcccagattgcgcggcaggaagtagccgatgctgttcgatgcccgaatcgcgttgtcattcgcggcaatggcggagcccgggccgcgcgccgtggcaatgttgccgctgatgctcttgatgagattttcgccgacgccgactgcgcccatcggatcgaacacgctctcgttccagtagctcggaacatagtcacggccaagcctgagttcaccgaatccgcccgacaggctcaccgtcgagcgacggctgaaggaggccagagcggttgcgccgctgtcctgggtgatgcctgactcgagccagaaccctgccgccagtccgccgcccaggtcttcggtgccgcggaagccgatccggctcgaagaattggcgccgctcgacaaggcagtctgcgagcgcgtcacctccgcaaaggcgagcgccgacgccgacgggagtgccaacgtgttgttgtagaaggcgcttttgacgctgtagtgactgactgctgaatcagcgacgccgaatagcgtcagggacgactgcgccgaagcagcggccgaaacggccagtgccgcaaaggtgatcaaggacttgcgcatagcaggtgtctccaagggacgaacaagggttgccggcgccctgcgacgctggcggtggttgcggcagcctgccgcaagaaggttcggcagcgatggccggtctgggtagttcggcggatcaatccgccgcgagcaggcgaatgtcctgcggcgccagggcgccttcggccaccacgtcctgccagcgatcgaactcgcggcgaacgcgttcccgcagtgcagaggggggaccggcctcgacccgcgcaccttggcgttcgaatcgagcaaccacttgcggattggcaagaacctcgttcagggcgcggttgatctgtgcgatcaccgcgggcgaggtccgtgcaggggcaaagagcccataccactgcgagacatcgaccccctcgatgcccgactccgacaacgtaggtacggcaggcaatgcttcgagacgcgccggggccgcgacggcgagggcgcggagtcggccgtcgaggatgaagggatgcgcggtgaacaggctcgggaacatgacctccgagcgaccatcgagtgtgtccacgatggccggcgctgcaccctcatgggttctgccctccatcctcgtacccgtgttgagttgaaacaactccgccgcgaagtgtggcggcgtaccgtcaccggctgacgcatatcggacgttgcctggcgcgctgcgcagatgctcgaggaggctgcgaacatcatcgaagtcggcctgccgattggccaccatcagcgtcggcgacgatccgatcaagccgaccggctcgaagtctttgacagggtggtaacccagcttctggagtgccgggttcatcgcgtgggtgcccacgtagccgaacatgagggtgtggccgtcgggttctgccctggccacatactcgctcgcgatggcaccatttgcgccggcccggttgtccacgagaacttcctggccgagcaacggcttcagttcggccgcgatgatcctggccatcgtgtcgttgccgccgcccgcgcgggttggcacgatgatcgtgatgggtttgcgcgggaacgtggccgactcacgtgcaacggcctcgggccgcgtaaagacgtagtcgggcaactgcatctcgccctgcatgatctttctggcggtacgcaccagcgccgccgctttcactgttgcgtcgttcgctcgaccctcaagctcgacttccacgtcgatctgccctgccgggtgcaggagaaccaggttgtggcgccccggctcgcgagcggcggcgcttgcgaccgtgcccgggagtgcgaaggcgctgagaacgccaatggcacccgtgaccgcatgcgaggcgtggcagcggcgcggggtgaagtagcgcgaggtgatgctgtccggagagtctcccgcgctgaccagcaccggcttgggaatgacgctgcctgagacatccccgagtcccatcaacaggccggcctggagacgcaacgtttcgagccgctccagcagcaccgcattcgagtcaagcgccgcaggcttttcgctgccggtgacgccaaggtcatgcgcgcggacgatcatgagcggcatggccgcatcgatgcacgtcacctcgacgccatcgatcgtgtcgatccgccgaccggtcggaaagaccttgcccgtcaccgcgccccacgcatccaaaaagttcagaagaatcggtgcagccgtaccggccacgccatcgatgcgcgcgtctccctcataggtgacgcgcttgccgggcgtcctgaccgtgacgtcgatgcgcgatcgcgtgttgacgttgaagacgcgtacccgcgtgattccgtcctgcgcctcgatcagcccctgctcgatcgcgaagggcgcgacgcccgacagcatgttgccgcagttcggccgggtgtctacggaacggtgtccgactcctacctgcgcgaacaggtagtccagatcgcagcccggttcttttgaacgggaaacgatggcgaccttgctgttgagggtgctgccgccacccaagccatcgagctgcagcggatcggaggcaccgatcgcgccgatcagtgcctgatcgcgctcctcgtcgctttcaggcagccactcccgcaggaagaaggggccgcgcgaggtacccgcacgcatcagcacgcagggaatggtcctgctcatctcagtcggccgaaagctttgcagcctggaccaccttcttccacttgacctgctcctgctgcacaaaggtgcgcatctgctcggacgtcatgacttccacctcggcgccgtggtcctccagcttcttgacgacgctcttgtcggccagagccgcattgagcaccttgttgagttgctcgatcaccggcttcggggtcttggccggcgcgaagaagccgtaccactgcgagacgtccacgttgtcgacgccttgctccttgagcgtcggcacgtccggcatctgcggagaacgcttggtaccggccacgccgatcgccttgagcttgccggccttcacgtagggcatcgcagtgaaaaggcttgggaacatcacctgtgcctgacctccgatggtgtcggtgatcgcaggcgccgatcccttgtatggcacgtgaagcatgctggtgccggtcgagagcttgaacatctcggcagcgaaatgcggtgcggtcccgttgccagcagacgcgtaacttgtcttgtcgggcgcggccttgagcgcggcgacgagttccttcgcattgttcgccttgacggaaggggtcacgaccatcagcgttgcggacgtgcccaccatggccacgggctcgaagtccttcaccgggtcgtagcgcagcttctgcagtgcgggattcatcgcatgcgtggcgacatagccgagcatcagcgtgtagccatctggcgcagcgcgcatgacgaactcgctggcaatcgcgccgttggcgcccgccttgttgtcaacgacgaccggctgcttgagtgcagccgacatcgcctggccgatgactcgcgccatcgcgtcgttggcgcccccggcggcggtcggcacgacgatggtgatcgatttttcggggtaggcggcaagcgcgctgctgcacaagagcacggccgcagaagccagggcacacaggacgggtgcgttacgggtttgcatcgatgtctccgatagttgaaatgtgggggtccaggtcgcttcctcgaccgtggacgtatggtgttcgcatcgacgcttgctgtgaattgcatgtttaggatcgattgatgcacactgtcgatcagtcaaacattgctggcggtacgagacgatggccatcaacttcaacctcaacgacctgcaggcgttccgcgccgttgccgaactgagcagctttcgcaaggcggctgaagcgctgcacgtctcgcagcccgcgttcagcaggcgcatcgagaagctggaagaagcgctgggcgtacggctcctggagcggaccacgcggcgagtgagcctgacggcggtcggacgcgatttcgaccggaaggtgcagcaactgcttgacgatctggacctcacgctgctgggcatccgcggcgtggcgacaacgcgcatgggcgaggtgaccattgcttgcgtgccatcgacggtctactacttcgtgtcgcaggtgatctcgcgctatcacgagcgctatccgaaggtccgggtcaaggtcttcgatgcgagcgccaacgaggtgctggccgcggtgtcgcgcggcgaggcggattttgggctgaacttcattgggggccaggaacccgacatcgagttcaagccgctgatggaggagcgcttcgtcgccgcttgccgacgcgaccatccgctcgcgggcaagcggaaggtgagctggaccgaactggcgaagtacgactacatctcggtgagcaaggcgtccggaaatcgcctgctgctggaccaggcgttgtcgggtttgccagggcgcccgcaagcgatctacgaggcgcagcacgtcacgacgatgctggggttggtcgaagccgggctcggagtcgcggcagttccctcgatcgccatgccgggggccgatcacccgcttttggtcagcgtgccgttggtcgagccggtcgtcagccgcaaggtgggcctgatccggcgcaagggccgcaccctctctccggccgccatgcagttcttcgagtttttctccgagatgaagggcaagcgcgtccaggccgggagaaagcgcgcttcggcttgaaggctcagcggcgcgccgtcagtacccgatcgaccatcacgccggcctgaccaaggttgttgacagggtcgcacatcgcgtcgagttgggcgcgcgtgacgtgcttgctgatctccgggtgctcggacaggatctcgatcagcgggcgattcttgctgatcgcctcgcggcagaggtcatacacaaggtcgtgagcgtactcgcggccgatgtacggccccagacccatcatcaccgcttcagacatcaccaggccgttggtgaggccgatgttggcgcgcatgcgggtagcgtccacctccaggcccttgagaatgaacttggtctgcttcagcgcaccggacatcaggcagaagatctcgggcaaggacacccattcgatctcccatgggccggtcgagcgctcgtggtcggccaccatcgcatccatcagcgcagcggcatgctggcgcgccacggagatattggcatggatgtacaggcaggagatcgggttgcgcttttgcggcatggtcgacgacgagccgcggccgggtgcaaaaggctcgaacacctcggccacttcggtctgcatcatcagcttgacgtccatcgcgatcttgccgagcgagccgcccaccagtccaaggaaggcgcccacttccgcgatggtgtcgcgcaccgtgtgccaggaaatcagcggctgggcaaggccgagttccttcatcaagccggcctgcgtttccatcgcgcccttctccagcgaagacagcgtgccggacgcgccgccgaactcccccatcagcacccgtggcttgagctgctgcaggcgctcgcggtgacggtcgatcccggccaggatgcttgccatcttgtagccaaaggtgattggtgtggcctgctgcaggttggagcggccgatcacgggcgtgtcgcggtacttctttgccagcgtggccagcgcgtcgccgatctcgtccaggtcttgctcgaccaaagcgaggccctcgcgcatctgaagcaccgcggccgtatcggtgatgtcctgggtggtggcgccccaatggcaatactcccccagcttgtcgcgacagttggcgttgatctgattgacgaccgcaatgatcgggtagccgatctgctcggtcttggccttgagctttgcccagtcgatctgggagagctcgcagttgcggacgatctcgtccgccgcttccttggggatgatgccgagctcgccctgcaccttggccagcgcacgttcgatgtcgaggtacttggcggtgcggttctcgtcagaccacacgtcgcgcatgcgcgcgtcgctgaacatgtcgccaaagatgcgcgagtcgatgatggtggaagccatgaggttggatctttctgggctggatgttgaggggagggtcagttgcgggccagggccagcgtgcgttgtgcctgcaggaccacaggtcgatcgaccatgcggccatcgagccgcgcagcgcccggggaggcggcatcggctgccagaactcgctgcgcccactccagtgcttctgcggagggtctcagcgcggtgtgaatgggctccacctggctcggatgaatgcacagtttggcgccaaagccaagagcacgtgccgaagccaggtcggccaaaaggcgcttgcggtcgtccagctgcggtgtgaccccggcgaccggcgccggcagacctgccacgcgcgaggcaatcgcgatgcggctggccgcgtaggtgagacccgaagcgtcgtcttcaatttcgatacccaggtccaatgcgaaatccagcgttccgaacaccaggcgcgacacgcccgcggccgcaacgatgtcgactctggccacgccgcgcgcactctcgatcagcgcgaggacgctggccccgggcagcgcggcaagcgtggccgcgacctgctgtgcagactcggccttgggcagcagaacgctgcgggccccgactttgcgcagcgccgccaggtcgtcgtcgaaccacggggacgcagcgtcgttgatgcgaaccacggtgcgcgactgatcgtccgcggatgcggtgcggagccaatctgcgattgcttggcgggcgagcgccttgtcatcggttgcaactgcgtcttcaaggtcgaggatgacggcatccgcgccgcttgccagcgccttgccgaagcgttccggccgcgtgccaggaacgaagaggtaggtgcgagggatgctggaagcaacggacatgatgcccacctcagacagccttggatgcacgcagcgcatcgatctcggccgcgccgtagcccagctcggccaggatcgcgtcggtgtgctggccgagcgcgggcacggggtccatgcgcgggcccacgtcccaggtgccgggcggcagcatggcgggcagcgggccattcggcgagccgacttcggtccagcgcccgcgtgccttcagttgcgggtgggcccagacgtcgttcatggtgttgacttgggcattggcgatttgcgcgagttcgagccgctccaccacctgcgccctggtcagggacgagaaggcctcgacgatgatcccgcgcagcgcgtcgcgctcggccaccctcttgaaattggcggtgaagcgaggatcggcagtcagcgccggtcgctgcagcaccttctcgcagaaactggcccactcgcgctcgttctgcaggcccagcatcaccatgttgccgtctcctgtgggaaacgggccataggggtagatcgttgcatggctggcgcctgttcgcggagggggtgccgcaccttcgaaggcgtagtagagcggatagctggtccattcggccagcgactccagcatggagatgtcgatgcgctggcccttgccggtctggccgcgctgcaacagcgccgcgagaatgctgctgtacgcatacatgccagcggcgatgtcggcgatggatggaccggccttgcaaggctcatcgggcgtaccggtgaccgagacgaaccccgcttcgctctgaatgagaagatcgtaggccttcttgtcacggtacggcccggggttgatcgggtcgtcgccatagcctgagatgtcgcacacgatcaaccccggctttgcggcagacagcttgtcataccccaagccaaggcgcgcggcggcaccgggcgcgaggttctgtacgacgacatctgccttctccacgaccaggcgttgcaggatcgtggccgcctcgggatgcttgacgtcgagcgtcaggctttccttggagcggttggtccagacaaagtgcgacgccaggccgtgcacgcgctcgtcatagcctctggcgaaatcgcctgaacccggtcgttcgatcttgatgacgcgtgcgccgaggtcagcgagttggcgcgtggcgaaaggcgccgcgatcgcgtgctccagcgtgacgaccgtgaggcctttgagtggctgcatgtgttgctctgtctgagtgggtgggagttgatggagatcagcgcaggaccgcagtcgcgtccatcgtgagccagccttcgtgatcggaggcccagagccggatggtctttccgtcggcttcaggttgtccctggaggtggaaaggatgaaggtcgaaagttggccgcaccgccttgaatcgaaagctggccacatcggcttgcggcatctggcgccgaaggagatccatcagcagcgttgcaatcaacggtccatgcacgatcaggccaggatagccctcgaccttggtgacgtactgcctgtcatagtggatgcggtggccattgaaggtaagcgccgaatagcgaaacagcagcacgtcatccggcacgatggcgcgcctccattgggcgtcggcaggcgcagcttgtggcggtggggcgacgtcgttcggaccctgcgcctcgcggtagacgatgtcgtggaactcgacgagcgccggatcgctgctgtcgttgcaacgcacctcgtgccggaccttgacgaagacaagcgtgccggtgcggccctctttgacggtcacgtcctcgatggtcgaggttcgcgcgacccggtcaccgactcgtatgggcgagcgaaactcgaactggctgccggcccacatgcggcgaggcagcggcaccggaggaaggaagccgccgcgcttggcgtgcccatcggcgccgatgtccgactgttgatgcatcggcagaaaatacaaccagtgccaaaggtacggcaaggtggtacccgtctcgacgggcgttgaagggtggtccagcgtggcggtcaacgcgatgacaggcgtcgggttgatggcgtcctggacggtctcgctgcgtccgatccaggcgcgaagttcttcagcttgaagagtcactcacttgtctccggttgcggctcctatatctgaggaaccttgcgaacgagtctcgcgccttggcagggcaaagtgaattgcaagattcagaacgattgatgcaggtggtgcataaaacgccgagcagatgttggcttggggagagttcaagctgaaagggatcgttttttacgcaacttggctcaggtgcccgcttgcagcaggtggccggtgctccgagttattccagcggccggacggaagccacttgttcgaggacgaaggccacgcgcgcctgcacagacaactttggaatgacgcgagtcgcggagcgggcaactcgctcctatgcgccgacagtgtcggcgtatgtcgaggctggaatgctcggggcgaaggtccgcgtgtggccagactgtagccgtcactctgccggcgcaaaggggcctatggcggctgtgcgctttcgctccgaagtgcgcatccggcgacggggacatgggacaaattggtcgtcaggcaggccgaacagtggactccttgtctggcaggctgtgtttttggggcaggagtcctacgaaacaagactgtcagtatcgtttcacagaactcccgcacggacttcactccgacttcacctgggtcacgcacactgcctgtcgacagcggttcggcgctggtagaggccagggagaaaaaaagccgctcagggaaccgcctcgatgccgacccgctgtcacttctcatgttcagggcttgcaagtccggcggcagagcgatctgccctcatccgaccttgggtcgaggactgacttcaaggctgacgtgcccgagtgaatcggtggtgcctagcgctctggctgctgcctcgccttgtacacatctaaaagccgttgaagcacggcgcgttcgtcatccggcatgccgtttccaagatcgacgacgatgccgttgagcaagtagtactccgtgtcatcacgaacggagccgcgcgtgacgatgcgcttatacgacgaggcatatcgacgacggacttctgacgccggcgattggttagctggactggtcgatttgaatcacatgctccggaccaaactgaacgagcgtccctagttcaagctcatcggtgcaatatggctggttgtcgagcgcgccaacgtagcctgacgggccggtggaccgcacgatgacccacattcgctcaacgtcaacttcgccgtcatgctcgattcggaagacgagtttcacgatgtcgccaggtaccaagcacgtcctggcttcgagtggaggaagataaaacgtcgcgggtgcagccgcatgcatcgcttccccgttgtctagttcgaaactgaccatgtgccgcggccggtgtacgtatgtatgtccggccgcggccgcgccctaccctcagcccgccacggcggccagcgccgcgttgaacgttgcgctcggccgcatcactgcatcggtcttgcgcacgtccggcaggtagtagccgccgatgtcggccggcttgccttgcacggcggcgagttcgtccacgatcttctgctcgttggcggccagggcatcgacgagcggcttgaagtgggcggccagttccttgtcttcggtctgctcggtcagggcctgggcccagtacagcgccaggtagaagtggctgccgcgattgtcgagctggccggtcttgggcgacgggcccttgttgttgtccagcagcgtgccggtggcggtgtcgagtgccttggccagcaccttggccttggcgttgttggtcttgatgcccaggtcttccaggctcacggccagcgcgaggaactcgcccagcgaatcccagcgcaggtggttctcttccaccagctgctgcacgtgcttgggtgccgagccgccggcgcccgtttcgtacatgccgccgccagccatcagaggaacgatggacagcatcttggccgaggtgcccagctccatgatggggaacaggtcggtcaggtagtcgcgcaggatgttgccggtggcgctgatggtgtccagcccgcggaccacgcgctccagcgtgtagcgcatggcgcgcacctggctcatgatctggatgtccagtccggcggtgtcgtgctcgtgcaggtacatcttgaccttggtgatgagctgcgcctcatgggggcggtaggcgtcgagccagaacaccaccggcatgcccgagttgcgcgcgcgcgtgacggcgagcttgacccagtcgcggatggcggcgtccttgacctggcacatgcgccagatgtcgcccgcttccacgttctggctgagcagcacctcgccggtatcgagatcggtgatgttggccacgccgtcctcggggatctcgaaggtcttgtcgtgcgagccgtactcctcggcctgctgcgccatcaggccgacgttgggcacggtgcccatggtcttggggtcgaaggcgccgtgccacttgcagaagttgatgatctcctggtagatgcgggcaaaggtgctctcgggcatcacggccttcacgtccttcaggcggccgtcggcaccgtacatcttgccgccgttgcggatcatcgcgggcatggaggcgtccacgatcacgtcgttgggcgagtggaagttggtgatgcccttggcagaatccaccattgccagctcggggcgatgctcgtggcaggcgtgcaggtcgcgccggatctcgtcctgcgtgctctgaggcaaggcggcaatcttgttgtacaggtcgaccatgccgttgttgacattcacgcccagctcctcgaacagcttggcgtgcttctcgaaggcctcgcggtagaagatcttgacgcagtggccgaacacgatggggtgcgacaccttcatcatggtggccttgacgtgcagcgagaacatcacgcccgtgttgtgcgcgtcctggatctgctgctcgtagaaatcgagcagggccttcttgctcatgaacatggagtcgatcacctcacggtcgagcagcgaaaccttcgacttgagcacgatggccttgccgctcttggtgagcagttccatcttcacgtcgcgcgccttgtgcagcgtcatcgacttctcgccgtgatagaagtcgccgtggtgcatgtgcgagacgtgcgagcgcgacgcctggctccaatcggccatgctgtgcgggttcttgcgcgcgaattccttcactgccttgggcgcgcggcgatcggagttgccctcccgcaggaccgggttcaccgcgctgccgatgcacttgttgtagcgcgcgcggatattcttgtcttcgtccgtcttcgggctctcggggtagtcgggaatcttgtagcccttgtcctgcagttcactgatggcggccttcagctgggacaccgaggcactgatattgggcagcttgatgatgttggcttcgggccgaagcgtcagcttgcccagccctgccaggttgtcgggcatccgctgcgtttcgaccaacgcctcagggaactgacccaggatgcgggcggccaccgagatgtcgctggtggcgacgtcaatgcccgccggcgcggcgaaagcctggatgatgggcagcagcgaggccgtggccaagcgcggcgcctcgtcggtgagggtgtagatgatctgggagttttgggcggtcatggtagctttcggggcaggctgaacaataacaacaacgcaatgtcacgagacggacgcgtggcgaacgggcgcaaactttaacaagttgaggcggggcgcgcatggcattgtcggggcttgggcccgtggctcgcggccagatgcgcctggcgctcaggaacttgtggtatcgattctcccctttcgacgcaggctcgcttctggccggaagcggcgctttccctcatgaatggttgtccgggaagcggtgatacatgaagaactgatcgtcttgcttccagcctctttcctcgtagagactctgggccgaaatgttgccacgcgcgacattcagtgtcacgcgagcagatccaagcgaccaggcgtaggactcgacggccgagagcagcttggaagccaggcctttgcgacgccccgactcctggacgaagaggtcattcacgacaaagacccgagagagcgagacggaagaaaaactcgggtagagctgggcaaatcccacggccgttgcaccgtcatggcagatgaaaagcaccgactctccgtgatcgaatctttcacgcagaaacgaacgtgcggcgaccacatcgcttgcctgtccctgaaaccgccggtactggtcaaagagcgtcgcgagttcctcgagatcggccagaacggcttggcggacggaagctgagttcatgtcgtattggagcgtgtgttgggaactgggcggcgatagggcaacatcattgcggtcgcccgcgttgcgtccagtgcagcgatacgcgggtgccttcgccgcggcggctgtcaatgcgcaggcgggcgccaatcgcgtcggcctgctcccgcagccccacgagtccgtagtgccccgctgtgtctgcactcggctcgaagccgatgccgtcgtcgccgatctccaattccacgtcgtcgttcgcaatgcgttgcaggcggatcacgagtcgccgcgcgcccgcgtgatgttcgacgttgcgcagcacttcctcgcacatgtggaacacggtctccgccggctcggccgccagggcagccaaagcgggttcgatctggcagtcgagctcgatgccggagcgctcgctcaggttcttggccaactcggccagtgccgcacccagtccgatgtcgcgcaccgggttgctgcgcagttggtcgatcgcgcggcgtgcctcgtccagcccgtcgcgcgccgcgcgctcggcccggaccagctcgtccggcagcgcatcgggccggctggatgccagacgtttgagcacacggatctcggtgagcatcgccatcatggaatgcgccagcgtgtcgtgcagcccgcgcgccaggcgcaggcgctcgcgcaccaccgccgcatcgcgtgactcctgcgccagccggttgatctcctcggtgcgctgccgcacgcgttcgtccagctcggcattgagccggcgcaactcgtcgcgttcgcgctgcagcgtgtccagcaatcggtcgagcgcgctgcccagccgcgcggcttcgtcggcgccttgcggcacttcgatgcgcgtcgcgctcccggccagcaccgcgtccgccgaatgggcgatcacgctcacgcgccgcgtgaggcggtgcgccacgatgatgccggcgacggcggtggcgaagcccagaaggctcagcacgatcgagatgcgccattcgatggccgtcgcgaaggccgcgaccgattcgaccggctggatcaccacggcctgccagccgagccggcgcagcgtgccgtcgcgggcattgggtggggacgcaatcaggtagggccggttgtccatgagccgccttgtccggatgcgcgtaggcaggtcggatccatcgttgcccaagccggcgacgacggggtcgaatggcgtgatgggatcgccgacatcctgccagcgcttctccagaagggcactcggcccgtggcgcacgatgccgtcgcggtcgatcagcagccattcgcccggcgaggcgcggatctcggtcaccatcttctgtacccagctccagctcaggttggcggccaccacaccgatgatcgccccgtcggcattgcgcaccggcgcggtgagcttcaggaagcgttcgcgcggcgagcggccttcctcgatccatgcggcgtccaggccttgcgagatccacgcgtgttggttgacgttctggccgaccacctgctcgtcggtcgctgcgacgatgaagccatcggcatcggtcaccgccagccagatcaggtctggaacgccgcggcgcaccgcttcgagcgatcgcttcaggcgttcgccttcgctgtgctgcacgtcctccgacagcatggccgccaccacgctgaccgcctgcaggcgcagcagcagtgcggtgtcgagttcggcattgacgtgctcggccgcggcttccaggcgctggccgtgctgctcgagcagcgtcgcacgtacgaagctgcgcagccacaggtttgccacgagcgccaggcacaaggtgagcgcaatcagcagccagccaatcgcggcggccatggagcgccgtggatcgatgcgacgtgcgaggttcattggcagcgcattctcgcaaacggcagccatgactttcggcatgggtacttcccctgagccctcggggtttgtctcgatccgccgcgtgacttccggcaggcgcgccggcggcggtttgcggcaacagttgcacccatcgcgatccgtgcctgcagcgcgactgattcccacccctcaacgtgccgcgacgcgatcggcgcgacaacgaatggagacgaaacgaatgaacaaaaccacttccctgacaccgactgcatccggcgcgccgccgcgcttgttcgacaaccgttggctgcaactggctgtcggcatcgtctgcatgatcgccaccgccaatatccagtacgcatggaccttgttcgtgccggaaatccagggcaagttcggctgggagcgcgcgtcgatccagatcgccttcaccatcttcgtgctggtgcagacctggctcgcgcctatcgagggctatttcatcgacaagttcggaccgcgcctgatcgtggcctttggtgcgctgttcatcggcgcggcctgggtcatcaactcgcaggccacgacgctgatgggcttctacctcggcgcggccgtcggcggcattggcgtgggctcgatctacgccacctgcatcaacaacgcgctcaagtggttccccgaccgccgcggcttggcggtgggcctgacggcgggcggctacggcgccggctcggccgccaccatcctgccgatcgccgcgatgatcgaatcgtccggcttccaggaggctttcctgttcttcggtttgctgcagggctcgctggcctttgccgctgcctggttcctgcgccagcccaagggcaacgaggtgcgcggctcggccaaggtcgcgcagagccggcgcgactacacgctgggcgaagcgcttcgcacgcccctgttctggctgatgatcctgatgttctcctgcgtggttaccggcggcatgatggccgtggcccaactgggcgtgatcgcacaggacctgggcgtgaagaacttcaaggtcgacctgtacttcgtcaccatggccgcactgccgctcgcgctgatgctcgaccgcgtcatgaacggcatctcgcgtccgctgttcggctggatctccgaccacatcggccgcgagaagacgatggtgatcgccttcacgctggaaggcatcggcatcatcgcgctgggctacttcggccacaacccgtgggccttcctcatcctgtcgggcgtggtcttcctggcctggggcgaggtgtattcgctgttctcggcactcgcgggcgatgccttcggcaccaagcacatcggcaagatctacggcgtgctgtactgcgccaagggcattggcgcgctgttcgtgccgctcggcaacctgatgatggaggccaccggcacctggtcgaccgtgctctacacggtggcggccctcgacctgttcgcagccttcctggccatcgtcgcgctgcggcccatgctggcaaggcacacggccagcaatgcgtcgtatgcgtcttcgccggcgcctgacctcgcgatgccgggcggcctgtcgcccgcgggccgcacggcctgacctgagtccactgccattcccacgcgcacccgtggagccggctttgccggtctctcgggtgcgtttcgcattcaggagggggcgccgcagcccttgggggtggttacttcttcaataccagcacagccagttcggtgcgggtgttcgcgtgaagcttttgcatgatccgactgacgtggttctttgccgttccctcggccaggttgagcgccgtggcgatctggcgattgccgtagcccttggcgatcagctcgagcacggcggcctcgcgttcggtcagcggtttggtcgcatcgggctgcaatggctcgcctggcgcggcggcctgcggcgcggcgcggacctccggcaccggcgcaggtagcggctcctgcgcgacgcgatcggccagcagccggaactggtccatcaccttgcgtgcgatctgcggcgtcagccgtgactcgccgcgatgcaccgcccggacggtgtccagcacctcttcttccgaagcgtccttgagcaggtaggcctgcgcgccggcacgcaccgcgtcgaagaccagatcgtcgcgattgaaggtggtcagcaccatcacgcgcgtgtgcggcaaggcggccgatatctcgcgcgtcgcgagcacaccgcccttgcgcggcatgtgcagatccatcagcaccacgtcgggcagcaggcggcgggccaactccacggcttccacgccatcggccgcctggccgacgacctcgatgtccggcgcggcgtccagcagcatggccatgccgcggcggatcagcgcctggtcgtcggcgatcagcacgcggatccgcggtgcggcatgcgggacggggaacgacggttcggcgatggtgctcatggcaaggtcgattgtgccccgaggcggctcgaacgcagcgacttcggcttggtcaagatcggacatccgcgcaccaggctgcgagttcctcaagcagcccgttccacccgcgccggcccgaccaagtagttgcccggcgtcacgccaaagcagcggcgaaaccatcgggagaaatgggcctggtccacgaagccgcaatgcgtcgccacctcggcgggcgagttgccctcacgcagcatcgccttggcgcggccgatgcgcgcgagccgcgcatagtgggccggtgtcatgccgacggccgagcggaacaggcggtggaagtgttcgcgcgacacgcccaatcgctgggcgagcgaagcgggggccatgcggcacgcgtcctccgtcgtcagggcctggcagacggcttcgacgcggacgtcgcccggcaggcgctcgagcggcacgcgctctttcccggtctgcgagcggaggatctgttcgagaagactggcgacttccgccccgtctttcgattgcgccgccgcagccaatgcgcgggctgcgcgttcgttcttccagacccgctcacgcagcacgccgcgctcggcaggtggccacgcgaggcgcgcaccgacccagtcatgcggcacatacagcatcaccatccggaacccctgcgcgctgacgcccgccgtgtgcagcatgaacggcgccatcagcacgaggtcgccggcttcggccatgtgccgttcaccggcgcacgtgaattcgcatcgcccttcgagaacggcgccgacgctccactcggcatgccagtgcaattcgaaacgggccttgggatcggacgcgaacatcgcctcgatctgcgcgccatcttccattggcagaccgatcacgtgcgaggtggtggagaagttcattctgcgaagggtagcgccgtcggcgccctcacgcgaccagcgcaccgcggaccgtgatgcccatccagcccgcgctggcctgcgtcgcttccacccgtccgagcagcgagagttcttccaccgggtgctcgtgaaaccgcagcgtcgccctgccctgcgtccagcccgattcgacgcggtccacgatgtcggcgcgcagatagcgcgcagccgcgggaatgccgggctgcgtgaggtcgggccaacccaccgcaccgatcgtcggcgcggagagaaagcccaggcgcccggtttccttgtcggtcagggtgaccgtggcatcgaccagccggcgctccttcacgctgaggctcgcgccgagccggctgcccttggacaatggcgcggccgccgggtgcgccagcggcaggctgcgggtcagccaggtctgcccgatcttcttgggccagccctgcagccagccgcgcagcaatgaaatgtcctggtcgacgtagatcaggggacagtagaagcgcgcatcagcgccctgccctgacgcgatctcgagcaccacgatggtctcgcggtactgcgcatagacggggtcgagcagttcctgcccgtcgttgccgcaggattgccaatccgcgaaatgaacgcagcccttgccggtggccacgccgagttccggcggcaccatcgccgcgcccagcccggcgtcgaaggcgaattccacgttgacgagccagccggcgtaatgccagggcggcgcctgaacaagggcgctgcggccagaagaagtgaaaggcggtgtgaaagaagacggcggcatcggttttctgcgagttggagaagacaacgccgcacgatagggctgcgaactccgaccgtcttgtacgccagtgatctgcatccgcaacgagcggcagatgacctgcgccagccatcattttagaaagtgatcgcaaacttacgagaaagatgcctaaatgccgacgacgccacgctgcagtgcgaaatccagcagcacccggtcggtcggctcctccggccaggtgtcctgcgcgagccagcggtagaaggtggtggcggccacgcggcttgccggaccgtcccgccgccaggcgcgcgcgatgggggcggccatctgttcgagccgctcggcctcgaagcgagtgcatacctcgccctgcatcggctggggcatctcggcgaacacggcgcgcgcctgccccatgcggtcgttctcccagagctctcggatgcgccgcagccgatcggcctccgacagcgcagccacaggcggcgcaagcacgggctgctgcccgttgccgccggacgcaggctccatggcggtgacgccggcatagcccttcttcagcgcgtccttgaaataggccgccggcgacttgagctccggcatggccgtgttgcgcagccgctggtccacgtggtccagcgtggcgcggatctgcccttcatcggtcgtggcgtagaggtcttgggcctcgtcctgcttgaggcccagcgcgatcaggcgcccgaccagctctaggtcgaagacgttccggttcgatgcactgatgtcccccaggcgctgctggatcttgggaacgaccctgaactggatctcctcgatcttgcggccgcgcttgtgctcgatcagctcgagtccgaagtcttcgcacagcgcgtcgatctcggccagcgccttgctgatgacgtcgcgcttgagaaagcggtagtcgacttccttgatgtcgctgcggcccgtcagcaccgcggcccaccagacgacgtcctcgcgcatcgacaggcgcccgggcgaggtgagatagcgcgcgccgatctcgtacagcacggcggcggaatagctgcgcatctggctgctcatctcgagcagcacgcgcgtgtactggtgcggcttgaccagccgctccttgatctcgtccggatagcgccaggtcaccatgcagggccgtcccctgccctgttcctcgatggtgacggtgccgagcagctgcgacgacacccaccgcttgagggagctgctgctggtcgaccactcgatggtcgtggcctgcatgtcgcgcaggtgcgatttcagcagctcggtgttgttcgaattgaagcgggcgtcgccgatcagttcgctgagcgtcagcttgtagaccggctcgtccacgccctggcgctgcgagtggtagagcagcgcgttgtagatgcgccgcgaaagcaaggtgagccgcccgcgcttggggcggatggcgatggcctcgttggccttggccacgctctgctcttcggccgtgggcgattgccggggcggagaccgtgactgtgaattttcttcctcgaccatggtctgctgcggcaataaagtggtttcacatcatgcctttgcattgtgattcagtcaattcacattaggcgcgtaacggtgccttggtatgtttgcagataaacacttgggatattgaagagttgaggatgcgttttcctgtggtgtgacaggtacttacgtccgcggctgtgagatcggttgggattgaatgtgagattggttggggtttgaagtgagcctcgttgggagactggcgcgacttttgtgagttcggatgggttccaatgtgagtggatatgggttgccgccctgtccacagcccgcaatgatgcgcaaagcgcgcgatgaacccggcttatcgggttctgcaggcaccccagcccggtttgtggcggcatccgaaccgcgctcgctgcctttaggggccttgatccccaaccgtcctcacaatacttggcggtgcggagacgggcttgtcgatagaacttgtccattcgacagattctcatagaattgccagattctgtcgaataaggccatacaaaatgtcagttcccgtgccgccggtcagtggaaacctggtttccaccgagcatcaggttcccccccgccaaaccatcaacatgcagaagatcgcggcgcttgccacgcgcgccggatcgatggtggagcagatccgcggcatgctgctggcgcccgaggcccgcaagatcccgccgacctactccaccgcccagctggccgcgctctgcggtgtcgacaaggcccatgtcgcctaccgcatcaccaaggaggatctcccggccggccggctgacgccttcgggcggcaagcgaaccttcgagctcgatgaactgcgccgctggaccaagacctaccgcgcagaaaagatgcggccggcgggccgcaaggccatcaccatcgctgtcggcaacttcaagggcggcgtggccaagaccaccaccgccatggtgttggcgcaggggctcagcctccgcggtcaccgcgtgctggccatcgacaccgatccgcagggttcgctgaccacgctgcacggcctgttgcccgaggccgaggtgaccgaggacatgaccatcgggccgctgtgcgacggcagcgagaacgacattcgctacgcgatccgttctacctactgggatggcatcgacctggtcgcggccgcgccctttctcttctccgccgagttcgccctccccgcccgccagatgcaacaacctggcgccaagttctgggacgtgctgaatgagggcctggagtcggtgcgggacctgtacgacgtgatcgtgatcgacacgcccccttccctgtcgtacgtcaccatcaacgcgctgtgggccgcgaacggaatcgtcgtgccggtgccgccatcgggtctcgactttgcgtcgtccgcccagttctggtcgctgctcgccgatctgggcggcaacctcgacggccagagcaaggaccgcgagggcaaggccttcgactttctccatgtgctgctgagccgcgtggacgcagccgatccagccatgccggccgtgcggcagtggatccaggcgacctacggcgagtacacgctgccggtcgagatcccgaagacgagcgtgaccagcaacaaggccgccgagttcgccacggtctacgacgtgcagaaatacgagggtgccgccaagacctacaagcgggcggtcgacgcctacgattcgttcgtcgaactggtcgaacagtcggtgatcggcgcgtggacagcgcaagggagggctctgcaatgaccgtggtgccaatgcacgccactccgtattccggtggaaacctggtttccacgtccccgttccttctgtatgttccggcaaggctggagatcgtccaaactgtggaaacctggtttccacagcagttcgcgccgcactccgaattcggggtggcaatgccgcaaggtccgcggaagggcgcttgccgcggccgctggaaatcccgtttcccgacgttgagcgctgcgcatgccgcgccaaggagtgtccatcatggctagcacccgcaagcggctggaggcattgaccgccggcctgatgcttccccaagccgccacggagccggtcgccgcactcgccgcggaggcgtcgcccgtggtgccgccgtcggcatccaacgccgtggaaaccaggtttccaccagccgtcggcggaagcctcgcaccccggacgggtccgggccagatgatggctttccgcggccagatccagcaggtcgagggcgagatggcggcgctgcgcgaaaagctcagccagtacgaaggctcgctgccgacacggaagatggaccccaagacgatccgtccgagccgctgggccaaccggcacgacgcctcgttttcgagcagcgcgttcgccggcctcaaggcggacatcgaacacgcgggcggcaatgtccagccgatcctggtgcggccgatcaaggaagagcccggccagttcgaaatcgtcttcggccatcgccggcaccgcgccgcgctggaactcggcatcccggtgctggcgtccatctgggtcgacgaactgggcgacgcggcgctctttgccgcgatggatcgggagaaccgcgaacgcgcggatctgtccaactatgagcagggcctgatgtaccagcgcgcgctcgaggagcaactgttcccgacccagcgccagctcgccgaggcactgggcgtgagccacacctgggtgcgcaaggcattgatggtcgcgcagctgccgcaggcggtcgtcgagtgcttccgcagcccgctcgagatcagcttccgccatgccgagcagatcaatgccgccatggaaaaggatcggcgcggtgtcctgaagcgtgtggagaggctgcggggccacagccttgcgcccgcgatggtggtcgcgcggctgctcgatgcgaaaccgggattcgaacgttcggaaaagctcgacgtcgtttcgggcggccagaagctcgggacgctggttcgcgccaagagcggcgagatcaccatcaccctcagccctgaagccgcgaccgacgccagcccggaggcgctcgaggccggtattgcagaggccctgcgcaaggcacgcaccttgtgagcggagccgcccaggggagggcggcgcggtgaatgtgagaacggttgggattctttgcgcctggccgactcggcagatttcgccgcgccgtttgccgtgcacgcaagccctgggggcaatccgcactgaaaaagaagaagggcagggaagggcagggcgccgtcctcaagctgcacgagaccccacgccgttctccagtcctgcttcaagcgcttgcgatgccttggtcgctgccaggcccatcgtttccgagcaactggcatgcagcatattggccccttcacgatcaggccgtgaacctgcccccagggccacacggattgccgctcttcttctcgtcgccgatgacggcattccggcgccgccgaggcatgcgctcggcatcgtcctgccgcgcctcgcggatcccgaagacgatgcgtaaacttggcgctccccgccgccacggccccttcgggaccaacggaccggcgcgaatcaacgcgctggacatccgctgctgaccagataaaatcgttattaatcaatgacttaggcgcgacaccttaaggaagtgcgttcttgcaacacaaaatgtgtattgatgattacttcagttatcatcaagcaattcatgacacagaccatcgctccagtgccaggcaagcagcagcccaaagccatattccgccgcgcatcgacgagccggccgatcctcgcctaggatcggaagacatggcttccgtccccacaccttcccagctgtcccatattgacgacgacgaactcgctcggcttgcagtgagctggcgcgcgcttgcgggacgcggcgaccgcgaagcgttcgggatcgcgcatgcgctcgaggtcgagcagcgccggcgcacgcgcgagagccagctgcagcagctgccgccggaggagcccccagagccgcggccgtggtggaagttctggcaatcgaccggcgaccggaacccgacatcggcttcatgaagaccggcaccgcgcgcaagctgcaccgggggcactttgcattcatgcgggcgctggcccagggcctggacgaaagggccagctgggatcgctacctgcggctcgaaggcgaacacaccgacctgcgcacggtgcgccgcaccatcgcctggatccgtgacgagttcgcggcggcggcgcggcgcgaaagcaggcccggcaccgcccgcctgatcctgctcgatccggatcgcttcccggcggcgccggcactgccgagccttgccgagtttgccgcggcgcagggcctcgaagacttctccgaaaccgaacagatcgaggcctacgaagcagcgtatcccgccaccggcggcgggggagggcagggcgctcgcccctcgcgtcgcgcccaggtgatcgagcgccagctcgaagcactgcgctggctcgagaacctggtcgcgcaggatccgcggccgggcgacagcgtattggcctggctcaatccttcggtggccgcgcgcctcgagcgtgccggtgtgccaacgctttccgcgctggtcgaccgcgtcaacggcatcggcgcgcgctggtgggcccacgtgcccggcgtgggtgaactcaaggcggcgcggatcctcgactggctgtgcgccaaccagcaggcgctcgggttgcgcatcggttcccacgccttgaagcccagggcgcagctcgcgccgctggcgctggccgcggtggtaccgaccggaaccgcgctcgttccttacgaaaagttcgtcctgcccgccgaactcgacggccgcgcaggcagcaaccgcgcgccgcgcgaacgctgtctgctgatggccgcgaatgatcacgaggcgatcggcgcgtggctcagtgccaagcgcccgggcgatgcgaccggcgagctgtcggccacccagcgctcctaccgcaaggaggccgaacgcctgctgctctgggccgtgctggagcggcgcaaggcgctgtcgtcgctcaccgtggaggacgccatcgactaccgcgacttcctgctcgatccgcccgaccgctggtgcggtgcgcgccaccaccagcgctggtcgccgctgtggcggccgatggaaggaccgctcgcgcagtcggcgctgcgccaggccattgcgatcctgcgaagcctctacgccttcctcgtgaaccagaactacctggtcggcaatccgttcgcaaccctcgcgccgccatcgagcctgcagcagccgctcgattcgcgccgcgcgctgagctttgcgcaatgggaccacgtcgacgcgctgctccaggcgcacgccgacaccgaagcccggcgccggctgcgccgcggtatgcgctggctctatgcgaccgggctgcgtctggccgaaatcacaggcgcgaaatgcgaggacctcgaacaggtcgaggaccgcatcgcccacggcgtggccgagaccggctggcaactggccgtggccggcaagggcgggcgcgggcggcaggtgcccgtgccggccgcgctcgtggccgagctcgaggacgaactcgcgcggcatggcttcgagcggcaggtcggcgccgtgagcaaccgcggcattcatgtgctcgctcgcttcgacaccgaatcgcggcgtccggtggcctggtcggcctcgggcctgtaccaggcgatcaaggcctttgtcgcgcaggcctccgcgggcctgcagggcgccgaagcgcagcaattgaagaaagcgagcactcactggctgcggcactcgcatggcgcccatgccctgcggggccgaaacggccaggtgcccgtgccgatccaggtggtgcagaacaacctcgggcatgcctccgtgggaacgacggccatctacctcaccaccgatcgcgcgccctccctggcaccagtgcgcgccgctggctaaaggcaggcccgcggctgagtgcacgtcgcatcgcacgcaccggtggtccgccgagccataccgaaactcgctacctgctagcgcgtttgcatgctcgctagccgcccccgatccgcgcaagatcacggcatgcacacagtggtcttctgcactccgatgcgcggcacccggccgcgcggcccgctcttcttcaaccaactggcggagcgccatgccggctagcaccatggacaaggactggctctgtttccatcccgctccgtcgaagccgcgcttcacgccgccggcgggtgctgtggacgcgcactgccacgtattcggccccgccgcgcagttcccgtttgcgcccgagcgcaagtacacgccctgcgacgcttcgaaggaccagctctttgcgctgcgcgatctgctgggtttcgaacggaacgtgatcgtgcaggcgacctgccatggcaacgacaaccgcgcgctgctcgacgcactggcgcactccaacgggcgcgcacgtggcgtggcctcggtggctgcagacgtcagcgacgccgaactcgggcggctgcatgaagccggcgtgcgcggtgtgcgcttcaactttctcaagcgactggccgacttcacgccgcgcgaagtgctgatgagcattgcgcagcgcattgcgccgctgggctggcacgtggtcgtgtacttcgaggcccaggacctgcccgaactgtgggacttcttcacgcgtctgccgaccatcgtggtggtcgatcacatgggccgccccgatgtgagccagccggtcgatgggtcgcagttcgagcgcctcgtgcagctgctgcgcgagcatccgaacatctggtcgaaggtgagctgtcccgagcgcttgtcgctgtccggtccgccgacgtacgacgacgtggttcccttcgcgcggcgcctggtcgagaccttcccggaccgcgtgctgtggggcaccgactggccgcatcccaatctcaagacccacatgcccgacgacggcacgctggtcgacatgattccgcgcatcgcaccgactgcgcagctgcagcgccagttgctggtggacaacccgatgcgcctctactgggcctgagacgggcgcggcggtcgcgtcgaacgaccggccacaggctgcgcctgcgcggggggcgcgcagccctagactacgcttcatggacctcaagcagctggagtactttgtccgcgtggcggagctcggcagcttcacgcgtgcgtcgatcgtgatcgatgtcgcgcagcccgcgctcagccggcaggtgcgccagctcgaggtggagctgcggcagaaccttctcacgcgcaacggccgaggcgtcaccgtcaccgatgccggcaagctgctgctcgatcacgccagaggcatcctgcaccagatcgagcgtgcgaaggaagacctcggccgcatgcggggcgcactcgccgggcgtgtcgcggtgggcctgccgcccagcatcgcgaagcgcatcgccgtgcccctgacccgcgccttccgccagcagctgcccgatgcgcgcctttccatcaccgaggcgctctcgagcgccatgcaagagtcggtgaccgcgggccgcatcgacctcgcgctgctctacaaccccgcaccgtcggccgacatcgacagcgtggtcatcctcgaagaagacctgtacctggtgggcccggcgcagcccggcggcacggccgatggcgaagtctcgctgcgcgaggtggcgtcgcaaccgctggtgattccgaccaagcccaattcgatccgcatgctggtcgaggcagagatggcgaatatcggttgccgaccgacgatcgcgatggagatcgatggcgtggccgcgatcctcgatctcgtcatcgatggggtggggctggccgtgctgtccttgaatgcggtgctcaccgcgccccgcccggaggcctttgcgacccgccggatcgcgaatccgccgctgcgcagccggctggccctggccgtcagttcccagcggcccgccacgctgacgcaacaggccgttctgaagctggtgcgcgaggtggtgagccagacgatgaacgggtcggcgccgcccgcgtgagcatggggcgcggacccctggaggctcactgcttcggaataccggccagtcggatgacttccgaccagcgctgaatctcgttcttcaggagttctgactgctgctgcggcgtgctgccctgcgcctccacgccgatctggcgcagccgctccttgacctcgggtgcggccagcgccgcgttcacctctttgctgagccgctcgacgacggccggcggcgtcttggcgggcaccgcaaaggcgttccatgaagccacgttgaacttgggcgcgccgctctcggcgacggtgggcgtgtccggcaatgcgaacgagcgcttcgtgcccatgaccgcgatcggatgcagcgacttgccgctgatctgcccgaggaggggcgcgaggatctcgacgccggcgtcgatctgtccgccgcgcagggccgtgatcatggccggggagccgttgaacggaatcacctgcgcgtcgatgccggtgctgcgtttgagcagctcggccgccagatgctgcgtgctgcccacgttgatcgttccgatgttgacggtgcccggatgcgccttcgcatagaccagcaactcctgcatggtcttgaacttcgagtccgcggaggtcacgacggccaggtcgaaatagccgatcgtcgaaaccggcgcgaagtccttcacggtgtcgaacggcaggcgcttgaagaggcccacgctcacggcattgccattggacatcagcagcacggtgagcccgtcgggcgccgccttggccacggtgtcggcggcaaccacgccgcccgcgccgggcttgttgtccacgatgatgctttgccccatcgattccgacatcttctgcgcgacgacgcgcgccgtgaggtcggccacgccgccgggcccgaagggcaccacgaggcggatcggcttcgtgctggagagctgcgcattcgcgcccatggcgatggagaccgcggccagcacgagcgccgaccgccgcgagatcttgaggagggtgttcatggggttgttcgattcactgtgggacaagcttgcacaaggtgtcagaagcggtgccgcatgccgagcacgaggcttccccgccgctcgtatccggtgagccggtccgagaggtagaccgcgtagaggtcggtgcgtttggaaagatagtggtcatagccgagcgctgccgtcgtgcggctcgtatccgtgatgggcatgtccctgcgtgtctgcgcgacagacgccatgatgcggccgacgcccacgggcaccgccacgccgagctgcgtggtccgggtcgtggtgcggatgtcgggcgtgtcggtatgaaagtactggccgtagagcttcaccgcctcgaagtcgtacgagagtccggccatctgcgccttctggctcgagaccggcgccaccaggcccggacccgccttgacctgctgtgccgagaccaccgcggcgaacgggcccttcgcatagttgacggtcaggttgacgttgcgcacgccgccccggttggccacctcgccaagcccataggccgcggacacgcggaaccccgccatgtcgggcgacgcgtactgcagggtgttgtcccagacgctgtcgcccagcaccgcgcggttgtagcccgtgctccagacctgcagcatcaccgggctcaggttggccgatgcgagaaagggattgaagttgccggtggccgcatagagtgcattggtctgccggcccgcactcacctggccgtaggcgccgccgaggccgacataggcgttgcgcgagaagtaggggtcggccgtcgtcctgccgaaggtgccgctgtcggcctggaagaaactctccagcgcgaagaacgaccgcaggccgccgcccaggtcttcgttgccctggacgccccaataggaggtcgtcatgccgccgctgttcaataccttggtgcggccgggctggtcgctgcggcgcagcgaacccacgtactcgtcgacgacgccgtagatgttcacgctgttcgccgccgatgcgctttgcgcgagggcgggaaacgatccgagcgaagcggtagtgaggcccgccgcaaggcaggcgcgggtgcgcatatccatcttcttgtctccgtgtttttttgaaacgccgtaggtgtcttgggtcttggccggcgtgatggactatcgccactccaccggccgttcgctatccgacccgggcacttttagatatgtcgcggcggcatacctggcggtggctcggggtgcaggcctgcgaggtcaggccggtccgcgcaaaccgccccgctcgcagtctcgctccaccaccggcacctcgcgccagttgagcagccgcaggctcaggctggacgagagcgacaccttcaggttctcgaccgtgccggtgctggaacccaccgacaaggtggtgccgtcgttgctgctgctggtgaagcgcaggtccgtcaccgcgtacgacacggagatataggccgcgctgttctccagcgccgactgcccggtgccgaagttgaccacgtagactcggctggtgcacgaggggctgcatgcatcggccgtggtgagcgtcgaggcgaacgccaccacgccgctggtggtcgtggggctggtgatcatccgccaggcgatgccgctgctgctgtcggtgccaaggtccttgcgcctggatgcgtccaaaaacaacgagaggcagttgccgcagccggactgggcgcagccaacccagtcggctgcacctacgagtaggtggacacatgcagccgccaccggccagaatcagtttttcaactgccgtccaggcgaaggagctcttgatgagtttggatttcccttttggtcgcatggcactcgccttctgcttgggttcgctgctcaccgtgacttccgcgatcgccgatgaggccaccagccaggcgacaaatgagcatctcgtcgtcgaaaaattggctgctcgcacggggccggagagcgttgtcgtagagagtgcgggcccctacgctgattccactcgcgccctcttggtgcggggaggaggcactggccgtcaggcggagtttttgctgcgctgagcgatgacgtgagggcgcaggagtgcgccgctccgcggccattgcaggaacggcagaatgccgccaagccgtcggagacggccaccagcggacaccgaggaccgctccctgaatcgcatacaacatccgcatgaatcccgtcgcattgccagaccaccggtcttccgagcaccatgggctcgtcatcatcgagggcatcatgggctccggaaagtcgacaaccatgaggtttgtcgcgaaggcgcttgaagatgcaggccggccggcacttggtgttcacgagcgcgccgacccgcaccccgtccgagcgaccgatgagctccagcactggtttgaaccctggcgcgaatccacgggtgaacaattggcgcgtcgagctgtttcaaggtggcgctcgtttgttgaagaggttcgacttggctctgcggtgcccgtgttagacggccagctctttcacggcgaccttaccaatctcttcctgatggaggtgagcttcgatgaaatcgcagcgtattgcgagagccttgcccagctcatcgggccattgcgcccgctcgtcatctacctgcggcaggagagcgtggagcgcgccgtgcacaccgtttgcgcagagcggggggaggcctgggtgaagtatcaggtcgactggaagttgaagggaccttacgcggtgcgccggaacttgattggtctcgaaggtctcatcgccctgtaccaggactatcgaatcatgacggacgcgctgttcgaccgattgaagctggacaagatgcccattgagaactcgaagcgagactggacgcggtacaaccagcagatcctcgaacgactcggcctggacagcgtaccaagcgccaattgagttgcgctttcacaggcagaatccggccgaggctgtgtggaaacgcactcggcacatgagtatgccgaactcggccgctcgacagcgcacagtagagacagaacgcggccgtcgggccaccgccgcaacagtcagaccgatctacgcggcgagagcgcgattgcaagggctcatgccccagccaattgcatcgccttcatcgttctgacgaaccccaacaccttcattacacgcttgaagttgtaggccagtacatgcaagctcatctcggtgctcacatgcgccagagtcctggtcaggaagtgggttgatcccatccagtgtttcagcgtgccgaacacgtgctccacggtgcgtcgtcgcaaggtcatggcgtcgggcttgcgatcaaggcgttgctgcacccgatcaagcaccgcttcgtgttcccagcgtcggatgcggcggtagctgctggtcgtgcactggtctctcatggcgcaaccagggcaagcgctgggccaatagacgtgcagcttgttgtcgttcttctccagcgtgctgaacctgtagatcgctcgttcacccgcggggcattggtattcgtcgtccttcgcgatgtagacgaagtcggtcttgtcgaagcgacccgcggccttggcgttcgatgtcatcggtttgggcacgaaggccgtgatgccgtcgtcctcacaggccttgagctccgtgccattgaagtagccccggtcggcgaaggcttgaagtctgggcttgtccatagcctcgcgcgcagcacgcgccatcctgttgagctgcgcgcggtcgttgccgacgttcgtgacctcgtgcgccacgatcaagtggttcttcgcatcgaccgccgtctggacgttgtagcccaccaagcccgaaccctttgcctgcgagatcatcgagcgcgcgtcgggatcggtggttgaacgctgcccatcaggctcgtgcctcaactgctccttggcttcgtcgagctggcgcatctgatcgcgcagcttcctgatcttgtcttgcagtcgctcggtcttggcttcgacctctgagggttgtgtacggtccgccgtctccagtgcgtcgaggtagcgctggacgctttgctcgatttgttgctggcgcttgtcgatcttggctggcgtgacgttgcggtcccggctgttcaccgccttgaacttgctgccgtcgatggccacgatggcctgcgtgaacagcttgagttcacggcacatggcgatgaagcgcttgcagacattgcggatgccagcaccgttgttgtggcggaagtcggcgatggtcttgaagtccggagcgagccggccggtgagccacatcagctcgacgttgcgttgggcctcgcgttccaggcgccggctggactggatgcggttcaggtacccgtagatgtagagcttaagcagcaccgcggagtggtacgacggccggccggtggcggcggggtccacgcctttgaaaccgagtgcttgaagatccagttcttcgacaaagacatcgacgactcgcaccgggttgtcttcgccgatatagtcatcaagacactccggcaacaacgcgacctgctgtcggtcttcgccttcgatgaatcgcttcatgggcacctcgcagagaacgggtgccatgattttatttagatgagtcccgacggcgaagcgttttcacacagcctcggccaggaccggacatcgcgcctcgtccgctgatgaacaccatccgaagtgcccatgttggagatgagtccgaatcgctcgctactgcattccgtctttcttcatttcatctattgcccagcccttgtgcgaagtgaaaaagaatagtcgccacttgccgccttcgaagcgccagcggctgaagcttgggtcgctcacgtcctcacgcttgtacttaccatcggtcttgggcggtatcaagccgacctgacgcaacacgacgctagcagtcccatcgggcatcatgcggacggccttcacctcccaccggagatcggtgttcttcacgtcgtactcgaaggcggttttcaccgccgccttgcccttcatgcggccgtagtggtcgagcgattgggtaaaccagacgtcctcggtcatcgagcccaggcaggcattcacatcgtgccggttccaggctttctcgaactggacgatggtgtcgcgcagggtggcttcggtgccgctgccctgggctttcttcggttgcgcgctggcatagcgcccgaacggcgtcgctacggcggccaacccgatcaggagagcttgtcgcttgttcatggtccggcacctcctgaccgcagcttggtcgcccactcgagcgttgtcaatacaggtcgcccgtcagcgaactcacgtcaggattggtcgacgcattggtccacctcaggagtccacgactttcgagccccttggaagtcggtggggaccagagctcttcgcgagaatgcgccaagggcgaccctacggagacgccggcttgaaggtccgctgtggtttcgaggaatgtctcttctgagcccgcctgcgccgttgcgaggatgcggccagaaccagtcattcattgagcaggctcaattcgcctcattggtgtgaggtgggacaagcctgctgcccagaccccatccagatgcggttgaccgccaagccccaccggcagcgcagatcctgtttcatggccgccttccgaatttttgcctgcagatgatgcggcgctaaacactgggcgacagctcaatccaatggcacgtcaaggctcaccttcacgtggtccatcgtcaccagcgtgcgaaagcgcttgacgttgttgctctcgaagaagagcgcgcggctcagcgccgtgtactgcgccatgtcgcgcacgacgaagatcaggatgaagtcccactcaccagtgacgtaatagcactgctgcacctgggggcaggcgcggaaactgcgcttcatcgcgtcgagaagctcgatctgttcgctttgcgtttcaacctgggtgacgatggtgagcggatggcccaaggcggccggttcgagcacagctgcgactttgcgcaccacgccgttgtctacaaggcgcttgagacgccgattgacagccgctgtggaaaggtggatgcggttgccgagctcgctttgcggcagtgagctgtccacctggatgagttcgaggagacgaatgtccagggcgtcgagttcggtcatggtgttcggagcgagcgcaaagggatggaaacgcaaaaacgttgcgtaaacaaagccgattctgcacacctatcccgcggcttcgtcaataccatttcgtctcgaaccgcatctcccgcaaattctcttggacaggaacacatccatgacccaggtcaacctgaacgccgacatgggcgaaagcttcggcaagtactcgatcggcaacgacgaggagttgatgaagatcatccagtcggccaacatcgcctgcggctttcacgcaggcgacccgactgtgatgacgcgcacggtccggctcgctaccgagaacggagtgtcgataggcgcacatccgggcttcaacgatctctggggcttcggccgccggcagatccggatgaatgcgcgcgacctcgaatacatgatcacctaccagatcggcgcgctgcaagcgatcgcccatggtgcttcggccaaggtcacgcacgtcaagccgcatggtgcgctgaacaacatggcgcatgtcgacctcgaagtggcgacggcgatcgcacgcggcatacgcgctgcggacccggagctgatcttcgtggccaatgcctgctcggagatggtgaccgcgggccacgcggccggactgcgcgtcgccgaagaagcctacgtcgaccgaacctattccgacaccggtctcatgacctcgcgcactgaggaagacgccatcatcaaggacgcggaggtcgcggtacgccaggtgctctccttcgtggaggagcaggccgtcatcacccggtccggcaagcggcttgcggcgcgcatccagaccttctgcacgcacggcgacgagccgacggccgtcgtgctggcgagcaaggtgcacgaacaactcaagcagcgcggaatccagctggtaccgctgaccgacctgaagttctgaacacgaggatccacacaccatgcaccttcatcatctccattgcggtgcggctcgaagggctgcgctactcaccatcgccctggctggcattgcgctcgcccacactggacccacgcgtgcggacacctaccccgagcggccgatacgcatcgttgtgccatttccagcgggcgggtattccgatgcgctggcccgcatcatcgcgctcggcatgggcaagaccttcggccaggccgctctggtcgacaaccggcccggggccggcggcaacatcggcgccgacttcgtggcgaagagccctgccgacggctacacactggtgatgggcacgatcgggacccacgcgatcaacgctacgctttatcaaaaggtgcccttcgacggcgttaaggacttcgcgccggtggccttcgtggcggacgcggaaaccgtgctcgtggtcaacccctccgtgcccgcacgcacgccgaaggagctggtcgcgctggcgaaagccaagcccaatgaaatgacgttcgcatccggaggagcgggtaccaccgggcacctggcgggggagctgttcaaggcggcgaccggaacctcgatgacgcacattccgtacaagggaaacgcgcccgcactgacggaccttgtcgccgggcaggtctcgctgtcgttcgcgacgctgcagccggcgctgcccttcatcaaggccggcaagctcgttcctctggctacgctgggcaagacgcgctcgcccgcgctgccgaacgtgccgacgctggaggagtcggggatgggcgggttcgaagtgcgtaactggacgggcatcctcgccccggcaggcacgccgtccgtggtgctgaagaagctgtcggatgaaatcgacaaagtcatgcgctcggaggaagtgcaggccaagctgcagaacgaggggctcaagtacacgccgatggggcccgaggtcttcagccggttcgtgaagtccgaaactgacaagtgggccaaggtcgtgaaggcggccggcgtccaagccgactgagccgacgcatgctcttcagcaatcctcacgcgtgccggcgcgcctatccggacgaactgcgagatatcctgagcatcgcgcaggccagacgcacgcgaagctggttatcgacgtggccgatgctttcgcccgagccgacaccgctgtggcgccttcccggcctggcgcgcgaactcggcgtagcggcggtctttgtaaaggacgaatcgaagcgctcgccgctgggcagcttcaaggcactgggcgcgccggctgcgctggtgcacctggtcctgcgcgagcatcccgggtgggatccggaagacctgctacgcggcgcccacaaggccgagctgcgagagctggtcgtgatcaccgccaccgatggcaaccacggccgggcactggccggtgcggctcgcagtgtcggcgtgcgttgcgtcgtcgtgctccacaagcacgtgagcgccgagcgcgaggcggaaatcgcggaactcggcgccgagatcatccgcgtggaggggaattacgacgcatcggtcgcgcatgcggcggagctcgctcggcagagcggatggcaagtggtctcggatacctcgtacgaaggatatgagaccgtgccccgtgacgtgatgcagggctatggaacgatcgtcgacgagctgctcgagcaggaaggtggctctgcacaattcactcacgtgatcctgcagggcggtgtcggcggactggccgcaggcatcgccagctatctgtgggaggccttcggcgcggcacggcccgcactcgtcgtggtcgagccgcgccaggcggactgcttgctgcaaagcgcgatgcgaggacggccgtcgcgggccacgggctccgttgattcggtcatggcgggattggcgtgcggcgagacctctccgctggcctggcgtttcctcgaaggcaccatcgacgggttcctgaccatcgaggaccatcaggccgtcgaggcgatgcggcgaatggccagaggctcgcgcgaggacattcccatcgtcagcggtgaatccggtgccgccggcgtggcagccctctgcgaactcgcccagtcggcgatgctgcgcgcgcgcacttctatcaacgcgaaatcgaggattttgctgatcaacaccgagggcgccacggcgccttcggtgtaccgagagcttgcgggcatcgatgcggccgaggtcctgcaaaggcagcgcgactgggccgtcacagcgacttgagttcccgcggttggcgccgagcattctgaagaacgaccgcgtcacctgaccacactttcgacaagatcggagttccggacgaccctctcgagcaactaagaggaaatttttgtgccgcgcgtccactccttcacgatacaagatgaccgcagggaggcaaactgagcccatgctcagggcactgctctttattcttgctgctctcgtaccgattggccttgtttatgcattcggcgcgtggaccctgcttgcattgttcggaatgacggccgcgacactgctgttttcaacaaggaaagcacggggagctgaggcgacgcagggtggcaggcttaccggataccacaccaccacggcggcgaatttttagcctccgtgaacggggcgaagaggaggctgcgaagtaagcttgacgggcagaatgcggccaagaccggacctttgcatcaacggcacaatcgcgtgaatttcaggaggagcaggtatgcagattcgtagcattgctgcttccgatttcgacgcggtccatcgcctgctcatgaccagcgggtgggctcatcgagtcggtgacgcaaaggacctcggccaactgatttcggcgtcacagcgagcggtggttgcggtggcagacgacgaaatcgtcggcttcgcgcgcgcgattaccgacggaatttccaacgggtacgtgtccatggtcgtcgtcgctgagcggcatcgacgactgggcatcgggcaggcactcgttgaacgcctcatcgggtctgaaccgaatatcacttgggtgcttcgggcgggaagaacgggcgctgcagaattcttcgcgaagctgggcttcagcgcctcatcgaccgccatggagcgctcgcgacgatgatcgccttacggagggaagtccgatgcaggaaggcaaaatgccgccaagaccagacattcgagcttgaatgcggaaggttgcttgagtatggaattgagcggcaagagcatcatccagggcttcttcttgctcgcctgcgcgacacttctcgctctgttgttcttgggtgcctggatgctgaagaaggtgttgcctgaagaacatccgatgaagagcaggctgtcacctgaagggcttctgcatatcgcaaagattcttgcagcaacgctgattgcggcgtactttgtgggtgcagtaatcttgttaggaaggatgcggccaatggcggaccttcgtcatacactttcaataaacaagatcgccgccgcatgaacatcttggctgacatgattgccctcgttgctgtgactggactcatcgtctggatgttcttcaatgctggccaagcggtcccactcgccgggtatgttctgggttcagtatgctttctactcgtgctcggcatttggggtctgattgcggttgacgacttggacggtcccggtgctagcctgggtttagcgatcacatctacggtatcgctcctttgtctcggcgcgggaataggacttgtcgcgggcgcaatgaaaagtgttgcacctgtcgtgggcttcgggctcggattggcaagtttctgcgcgattcatctttggatctttcggtctaccagtccatgggtgggcgcttcgctcctgctggtttgctgcatcgggggcatggccgtaggagcatttcagaagagaggtgctctcggcccctggggcacagcggcgccgacaaacccataggcaagaaggccaccacctaagccggtgaccagcccacggccggcaagagtcggccacaaccagaccttcgtcgctcccctccaattcacgcccattatgagcagcatcggcttaatttttcgcgaagaccaagatctgacgacgctgccaccggattggactccggcgccacttggagccagacacttggtgaacgctgctgtggtgcgcgctcttggtagcgaggcggccacactgtcgctgcgtctcaccatcgaaagcccggatgaaagtcctgaccccagaacaatttcggccgtcggcgtttggggccccctggaaagtgcagtcatccgtgggatttgccgcgagctttctgctcgcttttatgatgctgaggccggtgaattcatcgaactttaaacatcgccagtcggccaagaccggaccttcgaccctaccctctgacttattgcgatgagccaactctgcaccttcgcgggcgtccgcatcgctctccccaacggctgggtcgacatcagcgacgacatgcccgaaggaacaccgcccaccctagcaaagtcggatggggtcggggcactgcagttttctgtaggacggtatctttccggcgctaacccacaagtcagcccggatgaccttgacgcgatgctcaaggagttcgccgacacacgttcgcttggcgtggctggggacgttgaacgaggcaagtccgcaagccactatgtcggcgggagcttcctgcatgcaggcgacgtgatccgcgcctggtacttgaccaacggcttcgacgtggcacttgtcacctacgtggcagcggctgaaagcggcgatgccgcggccgagctcgccgacgcgggcaccatcgtcaggtccgtcgaattcgactgaacgtcaaagggcaagatgcggccagaagcggaagtccatatttggagggaaacggatgaagtacctcgatgacctcattgatcgatggcacgctgaaggcctgcatcttttgcccgccgcctcagaggtcgaggtccgcaaagtctttcgagccgtgggagcggaagcaaccgctgatgtgatagttctgttcacatccattggcggcatgggggaaatggacaaagaattctggcgtctgtggacgctcgatgaaattaagtccgagaatgcagagcactcgccaaacggcgtgctgttctcggactacctgatcgcgtcatggtgctttaggctgaaggccaactcggacggcaccagcgcggtcctagtggattacttcgacggttctgatccggtcgtggttgccaacacactcggtgagttcttccgcttgtattcgacggacgcgactcgcttggtcgatccagcatcgctcgactaagacgtagtcgctcagcgaacggcagcattcgggatttggcaaggaccgcttcgggcccaaaccagccggtgagcaccacatccgcaagggataataggcgcctttgagtactgcgcaggttcaacggcgcagcgggcgaaagtcctagggcgcgggacgccagggccaccacgccgcaccccctacctcctgaagttcaaaggcgttccgcagccgagtgtccgggtcggccgcacggctcgccgcgcacgcagctcagtcagtgcgcgccggacgcctgcagcgacagccgttgcgcttccagcgccaacggaacgcggacctgggcaagaagcccgtgcgagccggacttgagcacgacgtcgccgccgtgggcgcgcgcgatcgagcggcacacggccagcccgagtccgctgcccatggtgtgcgaggcgcgggcctgcgaggtgcgatagaacggcttgaacaccagctcgagttcgctggccggcagccccggtccgcgatcgccgatttccaccacggcatcgggcccgtcggtgaacaggcgcacgcgcgcctggtggccgtacttgacggcgttctcgatcaggttgtcgagcacgcggcgcatgccgatcacgtcgacctccaccggcgctttttccatgcgctgcagctgcacgtccttgccgacgaacaccgcctgctcgaccacgtcctccaccaggctcgcgaagtccatgcgctcgcgcgcgctgaccaccgaggcatcgcggatgaagctgagtacggagccgatcatctgctccatctcttgtacgtcgtcgagcatgccggcgcgaatgtcgtcgggtgcgtcctcgatgcgaaagcgcagccgcgtgaggggcgtgcgcaggtcgtggctgatggcgccgatcatcacggtgcggtcgtcgacgaagctgcgcagccgcgcctgcatgcggttgaaggcctgcgccgcgcgtccgatctccgccgggccatcgagtgccagcaccggtgccaccggatcgcggcccaattgatcggccgcgcgcgcgaagccggcaatgggacgcaccagccggcgcgagaacagccagcccacgggcaccacgatggctgccgcaatcaggaaccacagcagcacgcggcgctgccacgcgttcgggaaggactcgggcaccggctgcaccaccatccagctgccttcgcgcgtatggaccgccgcgatgaagtcgccctccacgaatggtgccggcgccaggccgaacaggccgcgcgcggcggggcgcactgtttctgcggcagtcccggtggttgcatcggccggcggcggggtcaggggtttggcggcgcttctgggctcgcgcggcgcctcgacggccgtgcgcggcggcgctgcgttcgccggcgcggtgctgggcggctccgggcgcgtgggctcggtgcgcggtggcggcgctgcgggggctcgcacggccggcgcttcagccgttgcaggtgccctgcgttgcagcgggcgttcggtatccagcagaaggcttggcggtgtgacgggtgccgacaagatgccggggcccatcggctggccgggcatgccgggaggcggcggcccaggcaacggcgcctggggcgcggcggcgcccggggcggcaaggctcggcgcaccggtggccccgggtggcccagatggccggggcggcaacgtcgcggcaccggtgccgtccggaccgccaatgcctgccggcggcggagccaccggactgcccagggagcccgcacccacgaaccccgggcccggcgcagtggcgggcgcgcccgtcgcggcacctggcgggtcgcttggcggaggaccggctgccggctgctgctgctgcgcagatccacccacgctgccccccgagccgcgccccacgccgaaaccgccgccgaacccacccgggcttccccggaatccggatccgccggggcctccgggccccccaggcatcgagggccctccaggcccgccaccggcctggacccgctgaaagcccgcggggccgaaagtggtggcgatctggcgtgcggccgcctgcggcgcggcttgcgtcggcgcggtggcgacggcgcccgtggtgcctgcgaacggcagcggggtgaagaagtacagccgcacctcggcctcgtcccgttctatcaggcgagccaggtcgcgccgcgagcgctcggaggtcaaccagccctgcccctggggctcaggcgcgcgcgcctgcagcgagcgctgcagcaggtgcgcattgcggccttcggcgtcttttcctgaaagtacgcgcgcgatgtcgcccagctcccattggcgctgcggctcgggcggtagcagcatggtcagtgccagggtcacgccctgcgccacgaccagcccgcccagcagcagcgccatgatctgcagcgcgagcggcgggcccgaccaacgtcgtgcggttccttgggggttcatgggctgatgctggcacgggccggaggcgatgtcacgccgggcggggtgccatccgtgctttcggtgtgcgagtctgcggaccggttgttgcagcccgatttcacgacattgcagttcatttcattgcggtcggggcggcgggcagcaccggcaccgggcctatgatccgctacccgattcgccgcaccgtgaacctgaccacccgcatcctcatcgtcgacgacgacgccggcatccgcagcctggtggcgtccttcctggagaagcacggcctccaggtcgacggcgccagcgatcccgcgcagatgcgcgagcggctcgcgcaggcggactacgcgctcgtcgtgctcgatgtgatgatgcccggcgaagacggtctgagcgcactgcgcgagctgcagaagatcggcgggccgccagtcatcatgctgtcggccgtgggcaccgacatcgaccgcatcgtgggcctggaaatcggcgccgaagactatctcgccaagccctgcaacccgcgtgaactgctggcgcgcatacgcaccgtgctgcgccgcaccgccaatgcggcggcgtccgcgcctgcccaggcgtccaatgccgcgcgcgaggcgccggccacgctgctgtacttcgcgggctggcgcatcgacctggaaacccggctgctgcacgaccccaccggccggctggtagacctctccgacggcgagttccgcctgctgcgcgcgctggtccagcacccgcggcgcgtgctgaccagggaccagctggtgcagtacgcgctcggcgcggacaacgactcgtacgaccgcgccatcgacgtgcagatcagccgcctgcgccgcaagctggcatcgggcgaggtgaaggccgagctgattcgcaccgtgcgcaacgagggctacatgttcatgccggccgtcacgcacacgcctgcggcctgaggactgcggccgagtcgcggcaaagagccgcaacacggtgaaatcggtgcgcaatgaggcggcctcaagctcggggcttcgcattcatcatctctatcgattcatgactctcttcgacttgctgtgggactggcgcaccttgatggcgctgagcgtggtcgatgcgttcctggtcgtgatgttcttcgcctgggacgcgaagcacctcgcgctgctcacccgccggtgcaacctggcgcatgagctgccgcaggcgacgcagcttcgcaccggcccacgagaccgtgacgccttcaaccggaaagtgtgagcttcgaaagaggagaaaaatggccagccgccgcgcacgcccgcgctgagggcgcgaggcgttgcaggccaggcggccaggctagcgcgcgatgccgatcgtcgcggtggcggtgtagcccgccgttgcgctgccgctcatcgcgagcgtcatggcggcgatctgtgccgcggtgttgtcgctgaacacgttgtcgctcgcgagcgtgacggcagcgaagttggccacgctctgggtgtagcccgaggcgtagggatacaccgcactgcaagcagcgctcggcattgccagttgcgaggtcaggacggaattcctgccggtggtggcgctggcgaggctcgcgaagacctcgaaatgcatgtggggccagcggcccgaataacagccgggaaagatcgtcgtgaaagtgacctggccgttgctgtcggtcacctgcacccctcgcaggtagctttcggtcggcgccgaatacagcgagtagctgccgccctggtcgcagtgccaaaggtagattgcgtagcccgacagtggggcgcagctcgagttggtgttgaccagcgtgagcgtgagcgtcgtcagcacgccgggtgcctgtgtcgtcgagctgatgaagctgctgcggatgtcgctgcggacaatgccgctggcagtcagcacgtccgacgtggcgccggacgaagtgttggtgccgtcggccgggtagggccctgcggtctcgccaggcagggcggtgcaactgctgctggtgctcgtgctcgtgctcgtggagctgctcgaactcgacgtggaagaactcgttccgctcgccgatgctgtggtgctcgtcgaactcgtcgtggccgtggtcgccaggcccgcgaggctgctcccgtcggagccgccgccaccaccgcagccggccagcaggagcgccgagccggcggcactggaacccagccaggccagcgccttgcggcgctcgagaagctgcgcagagatcagcggaaggtcatcggccaggcgatggccatgggccgtcgtcgcgaaagcactgtcgttgctctttgtatggcggggatcgtggattgacactgtggctccgtgggtgggttgagcccggagcttcgagccgcgatgttgccggcggatttcggcgctttgcgcttttgttgcgagaagacctgtgcgttgcatcgatcgatgaggcatgcgtcgacctgccggaactcgaagcgcgcgtgcgtgcgctgctgcgccgcagtaccaactccacaccgcgggtgcagcccgtggtctccggccacgtcgcgatgttcttcgatgcgcaagagctgcgcgagctgcagcaacgcgcgggcgccgaggaactgcaattggcgcagaagctgctcgcgatggcgggcgtgtcctgcaacagcacggtggtgatcgggcgcagcgccgagaccatcgttgccagcgcgcgacttcggctgcgaccacatcgtcttcggccgcgaagagcccggcctggccggacgcatcgtcggctcgctggcgcagcaggtgcgccagctgctgggcgcgagcggcgatctgcaggtcatcggctcctgatatcggaaccggcttcggctggcctcgcattccacccgaatgcatgcagtactgaaaaaggcgtcatcccatcgatgacgccttttcttttgtccgcaagcttgtggagggacgctgcgaggccgttgctatcatcgaaaaatgcagtcccgaaccactgccgcggcggcgaaggagacaccgtgcggctcaagctgagaacgaagacagcgctgctgatcactttgctcgtgcttgccctcgtgggtgcaacgggcgggtggcagtaccggagcctgtccagcgagtacgtcgacctgatgcgcgagcagcagcaggcactgaccgagagcgccgcggccgatctcgactacaagctgggcgttcatctggccgccctgtcgcgtgcagcccgcgaacttggcgagcgcggctttgacgatcccgcggcgcagcagcgtttccttgccgacaaggacctgcgagcgatgttcgacaacgccgcgctggcgacgctggacggcgccatcgtcgccatcaacccacccgcgagccggcctccgaacgtggccgaccgcgactacttcaagcgcgtgcgcgacctgcgccagccggccatctcggcgcccttgctcaccaagggcagccagcagcccgccgtggtcatggccgtgcccgtggaagggccggacggccgcctcatcggcgtgctgggcgcggcgctgaacctgcagcgcgccaacgtgctcggcgatctgagccgcgccaccgtcgggcgcgggggctactacgagatcgtcacgcgcggcgactcgccgcggatcgtcatgcaccccgacgcgaagctgctgctcaagcctgccgatgccgccgccgacgccttcgcgggcaaccccgagcgcgacctggcaacgcgcgccaccgtacgcagcgccgactgggatctgcgcttgatcgtgccggcgcgcgccgcctacgcgcccctggaacaggcgaggcgaaacctgctgctgcagttgctctggctgggcctgggctgcgcgttgctggtctggctgggcacggcttggttcatgcgtcccctggaggcgctgagcaatgcgatccgtaccctgcgccattcgccggacagccaggtcaagctggatgtggtcgccaacgacgagcgcggcgacctggcccgcgagttcgacgcgttgatggccgagctgcgcgagcagcgcctcgaggtggccgcggtcaccgacgcttcgcccgtgggattgttccgctgcgacagcagcggccgcatgacctatgtgaatgacgagtacctggcgattcacgggctcgagcgcgaggacgcggaagagggctggctcacgctcgtgcgcgagcagatccgggagaaggttcgccaggattggattcgcatcgtcaacgccgccgaaccgctgaacgccacgcgccggctccaccgcaaggacggcacgcaggtgctggtggcattgcgaagccggcccgtggtcgcgggaggccgcgtgctcggacacgtgggaacggtgaccgacatcaccgaacgcacgcgggccgaacgggcccttcgcacgctcacggccatcttcgacatgacgaccgactacatcatccagaacgatgcgacggggcgactcatctacatgaatccggccgcgcgccgccgcacgggagtggacctggatgccccgatcgagacgctgaaagtgtccgacttcaatccaccgcaaacgctggagagattcaggtccgaggtggtgccgaccgcggtcgccaccggcgtgtgggtgggcgagtcgatggtgtgggacacgcagcggcgcgagttcccggtcagccacatggtgattgcgcaccgcgacaagcacggcaaggtggaatacttctccggattgatgcgcgacatctcggcggccaaggccgcggagcaggcactgcgcgagagcgagcaccgcttgcgcatggtgacggaccacctgccggcactgatctcctatctcgaccgcgacctgcgattccggttcgtcaacaaggcctaccaggactggttcggcgtcgagcctcggcagctgattggccgcagcctgcacgagttctacggcgacgaggcgtgggcgcagatggaaccgtacatccgggcggccctgggcgggcgccaggtcacctacgagcggcgggtggtgggacccggcgggcgccgcgacatccaggccacgctggttccggagcgcaacgaacagggcgaggtgatgggcctctatacgctggacagcgacatcaccgcgcatcacgaggcggaggaagccctgcaggaaagcgaagcccgcctgcgcacggtggccgacgcgctgccgatgcgcgtggcctacatcgatgcggacgagcgctaccggttcaacaacctggcctacgaacgcgaattcgggctctcccgcgaccagatccaggggcacaccgtgcaagagctcctgggcgagcccgcctaccagagcgtgaagccgcacatacgcgccgcgttggccggcgagatcgtcaccttccagagcgaagtcagccagagcgacagctacaactgctacgaggcccagtacatcccccagcccgcggccaatactgaagccatcgtcggcttccacgccgtgatcaccgacatcacgcggcaaaagctcgaggagaagcgcctggtgaacctggcgcagatcgatccgctcaccggtcttgccaatcgcgcgggtttcgaagcgcgactgggcgaggccatggaccgcagccgcagcgcaggtgccctgatggcgctgatgtacctggacatcgatggtttcaagcagatcaacgaccagttcgggcatcagacgggtgatgagctgctgaaggctttctcgaacaggttgtcgcaaggcctgcgctccagcgacgtccgtgcgcgcctgggcggcgacgagttcaccgtgatcatggaggggctgccccatgccgacattgcggtctccgccgcgacgaagctggtcatggccatgcaggcgccattcgccatcgagcagcagcggacgatcaacgtcaccgccagcatcggcctggcgttctaccagggcggcgccgcgacggccgctgcgttggtcaagcaggcggacgagatgctctatcgcgccaagcgagcgggtcgcaacaacgtgcaggcggcggccctgccgagcggtggcggctcgtcctagtctttacaagctcagctggcggccggtagaaatttcatcgtaattcgcgacagccttactggccgttcacatggcgccggcaggatagaactcctgaaaacaacgactcgaaggagttgcgatgaagaagttgtcccttgcattggttgcagccgctctggcctcattggccgcgctgagcgcgcctgctcaagcgcagccgcatcatggagacggtggctaccgtcctcacgtggtcgttgttccgccgccaccaccgcgccacgttgtgcggcatggttacgaccaccgctatgaccgctatgaccgctatgaccgccgtgccgactatcgtcatggccaccgctacgcacgccgggacagcgaccgcgacggcgtgcccgatcgctacgaccgccgtccccacaatccgtatcggcgctgagtgagagtccccgaagaggggagttcggtccgcttgcagcagtcaagttcgtcaagatctgaggcacagctctacgccgccaccgcggctgtcgatacggcgcggtgtgcgcggtcaaagacttgctggaccgtcgcccggggccgtagtagcggcgctacggttcaaaccaaaacgacaactgcttgtgatgcttgatcgccaacaaatgaacgatcggagattggtccgtccggctgtcgtgcacggaatacagcaccaagtaatcgtccatcacgtactcacgaacgtttgcagtcggcttatgcgatgccagtagacgctgcagtcgttcgaacaccatttgcgcctccaccgattcaggctgacgactcatgaacggccggcccatccgcggatgccgctccagatgcgttagcactacgtcggtgagttcgtccagcaatcggtcatagccctgcggaaattcgctcacgtcccagagagccgcaatgccttccagattggctgtgaattcgctgcgtaaaggatctcagccagcggctcgctttcctcgctcgccagcgtcagcgagtgatccggcgggcctttaacgcagtcagcctttcgcgtgcattggtcgaccggcccgccgccacatccgccagccccttctcgatttcactgagcagcagaagatgaatgctcgcgcgctccaggcggtgatagtgatcaagtcgcttgacgtcgatcattgctaccgcaggctcgccgttcttcgcgatgatcttctctgcgccgttctgcacctgctcgaccaattcggaaaggtgcgcgcatgcgctcgaaaatggcacgatgtcgcggacagtgatggacattcaggttctcctgaatacggaatttcgctctcgaatgtaaacatcattctgtttcgcgcggccagccgaagacgaccgggatctcgtaaaaaaagtcttccggaggcgctggtccgagatgcgacaggagacaacggcgcagaacggctggctgcgctgcccgcgtccagccacaagctatagggcaaaaacggcgtacgcgcggagtagggcgccgcggccccgcggctcacgccggcgtcatggccctgcgcacgagcagtgtgtcggtgaactgctcgaaagcgagcaccttcccgccctgcagttgccagacatgcgccacgcgcgcctgcatcggcttgccggtggcgtggaacgtgccgtggtaggtgccgataccgacgatgctgtccccggcatccaccagtcgttccagctcgaagcggtagccttcccagtcgcggccgagcacggcaaagacattgtcgatgacggcctgcggaccgacccaggtgccggcgcacggaaagccggccatctcggtccagcgcacctgcggcgacacctcggccatcaaggccgcgagatcgccgcgagccgaagccgcgtagtggtctcgcacgacgtccaggtggctgcgcgcactcaccacttcatttctcccttgttcaccttggcgccaatgtccagcgccacaccaaggcccgcgtccgggtaagcctgcttcatggcgctgatgagcgcggcactgttggcggccttcggcagctcctgctcgtagcgcaccaggtaggcttggctccaggcgatctgcgatgcgtcctgcttggcgcccacggcgctgtggcccggaatgacccgggtcggctgcagggcggccatcgcggcgagcttggtggcccagtcggcgcgctcctgcggcgtttgcgcatcggcggtccagaggtgcaggccggcgtatacgttcacgccgccggcgatggtcctgagcgacggaatccacacgtagctgcgatgtggcaggctgtcgtcgaggccgcgcacctcgatcgactggccttccagcgcaatggcgttgcccgccagcacctcgggcagcggcacgctcttgggcgcattggcgcccatgcgcgggccccacacctgcagcttggtggccagcgtggcctggatcttcttcagcgtgggcgccgtggtcacgaccttggcgtcggggaagtactgcttgagcacctcgatgccgaagtagtaatcaggatcggcctgggtgatgaagatggtcttgagcgtcttcttgctgtcgagcaccatggccgcgatgcgcagcgcgtcggcgcgcgtgaagccggtgtccagcagcacggcgtcggtctgcccggccaccagcaccgagttgacgtggaagctgttggcatcggcgttgtagacctggagggtcagcggcggagccgactgcgccgatgcatcgttggcgacgatgccgagcgtcatggcggccggcagcaaggcaagggaaaagaacttgatcgttttcatgagggactccatcgaagctgagggttacggatgggctcatcgtattggttcgcttctcgaagataaacttcggttcgatcaaatgattgtcaaccgattcgattcaatcccatggaccatctcagcgccatccgcaccttcatcgagatcgccgatcagggcagcctgacccgtgcggcggaggtgctcgacctctcgcgcgccatggtcagccgccatctcgaagggctggagcagtggctcggcgcgcggcttttgcatcgcacgacccggcgcgtgagcctgagcgatgcgggacaggaggcgctgccccggttgcgccagatgctcgagctggcctcggatgtgcaggccgtcaccggcgcgcgccggacggagcccgcgggcaagctgcggctcaccaccagcctgtcgttcgccctctcgagcctcacgcgcgccatcgtggagtttcagggccgctatccgcgcatcgaggtcgaactgctcacggtggaccgcacgatcgatctggtcgatgaacgcatcgacctggccatccgcatcaccaaccggctggacgaaggcgtggtggcgcgccagatcgccacctgccactcggtgctgtgcgcatcgcccgcctacctggagcggcgcggcgtgcccaagcggcccgaggaccttgccgcgcacgagtgcatcacccacgcgttcggcacgcgggccgagtaccggctgcgcaagtcgggccggtcggtcagcatcgcggtgaggggtgcgctgtcgagcaacgaaacatcggtgctgcgcgaggccgcgctggcgggcgccggcatcgtgatgctgcccacctactttgtcggagacgaactcgcgcgcggcgcgctggtgcggctgctgcccgaccacgagcccgaagcgctgggcatccacgccgtgatcctgtcgcgccagcatcagccgcggccgctcaagctgctgatcgatttcctggccgagcgctttggtggagcccttgccccctgggaccagacgccgccgccggtgctgccatcaaggcggaaggctcgcatcgatataaagccaaagcgccggccctgaagggcgcactgcccgcgtggtcagcgggatgcgcaggcagccgctctcaactgcctttggacttgcgcccgcgtgagctcggctttgcgggcacgctttttccgtattcgttccaccacgtcgtgagcgcctccatcgtcggaccgagggcgcgcgcctttgtcgtgatctcgtattcgacgcgcggcgggacttccgcgaacaccgtgcgcgacaccaggccgtccttctcgagttcgcgaagttgcgccgtcagcatgtgctgcgtgatggcgggaatcgcctttctcagctcgccgaagcggtagatgcgctgattcagcagccacatgatttcaagcttccatttgcccgacagcaatgcgaatgcgcggcgcatttcctcgtgcatgttgatctggtcatcgccattagtctgctttttcatactaagcgtcgctttttcatcctacttgcgggatttcatcttagacgacatccttgctgcaacccgacgcaattctcgtcgctcagcaagaacccatgactccaaactacccgtactggatcagcacgacgctgctgtccctgctctacctggcctccgcaatcatgtacatcgccaagaggggctgggtccgccgggcccttgccgacctgggctatcccgcctacctggtgccgatcctcaccgccgtgaagttcctggccgtggccgccatcctgtcgcgcgcgagcgtggctttgagcgacctggcctatgcgggcatgttctttcatctgctgctttccgcgtcggcgcacctcggcgttcgcaagcccggcggcgcgctgccggcggcggtgggcctcgtgctgctcgctgcctcgttcgcgacgcagaacaccgcccgcgacattccgtcgccctacgcccgggccgcagcggagcaccgggtaactctcaacccatggaaatcatcatgactcgactcaatggaaaagttgccgttgtcaccggtgccggccgcggcatcgggcgccctacaacatggcgaaggaggcggtgcgcgcactgacccggtccgccgcgcgcgaatggggcgccgacaggatcaccatcaacaatgcgctgccggtcgcggacacctggggcgcggccgacgctcctgcgccagccaacgcgctcgcccgtcatggatcgccggaggaggacgtcgcgccggtcgtgctgttcctcgccagcaaggatgcgcagttcctgacgggctacagcctgacgcccgatggcgggatgatcatcgacagcgcgcgctgagccgcaagaaagcgcgagcgagggagcgagcacgcacgcgaacaccggggaattggatgcccacgcagatcgattgcgcacttctctggatttcttgcctgatcctatggcgccggtgctgttttgtagatggagatctgctcgcgagttagagtcttcggcggaggctccgagcaacatggcacccacaccccccgacgccgcagcgcagtgcagattgctgcaggaagcgatggcgcacgtgatcggcgcgcggaccccggagccgggcgacttcgcaactcccatccccggcctcggcttcttccggcgcgaatcccccgcgccgcctgccgtgtgcatggtcgagccgagcatcgtgctcgtcgcccaaggcgccaagcagatgtggatcggcggcgaggcctatccctacgacacctcgcaattcctcatcacctcgttgaacctgcccgccaattcggaggtgagggtggcaagtgcggagcagccttgcctcggtctggtcttgaagttggacatccgcgtgctggccgagctgatcgcgcagggcaattttccgtcgcgtggcgatcgctcggtcggggcgggtgtgggaatcggtacggcaacgcctgccctgctggcaccgatcgggcgcctgctggcgctgttggacgagcccgaagccattccggttctcgcaccgatgatccatcgggaaatccactaccggcttcttggcagcgatcaggcggccaagctgcggcagatcgcctccgtggacgggcagggccaccgcattgcaagagcgatcgactggctgacgctgaactatgccctgccgcttcgcgtcgatgaactcgcggaccgcgtgcagatgagcacgcccaccttccatcaccactttcgacaactcaccgccatgagcccgctgcagtaccagaagtggctgcgattgaacgaagcgaagcgattgatgctgaacgaacacctggatgcggcaagcgcggctttcagggtcggctacgaaagcccctcccagttcagccgcgaatacagccgattgttcggggctccgcccaagcgggacatcgaggtgttgcgcgggggagccaagggtttcgatgcacgcgggcaggagctggcgaacccggcatgagaacttaggtccgaaggtcgttgcgacctcataggatcaggcaagaaaagcagcgaattgctctatcaatcgccgcgcagcttgagaagaatggtggtcagggcacccgcctcccggcgcggcttgcccgcacgacttgcccgaacttcgaacaacaggagctgacatggaaagtcccacgacgacgacccccttgatctcgcgacgcgacgcgctcattgccggcgctgccaccgccgcggcggtttcctcttccgcgcccaccgcggcggcggcacaggctgcaccttcggcatcggcatcggcggtgccccgttcaaagctttcgctgaacgtcaacggccgggttcattcgctcgagctcgacacgcgaacgaccttgctcgatgcgctgcgcgaacacctgcatctgaccggcaccaagaaaggctgcgaccacggccagtgcggcgcctgcacggtcattgcggacggaaggcggatcaacgcctgcctgacgctcgccgtcatgcacgagggcgggcagatcaccaccgtcgaagggctcggcacgccgcagaacatgcacccgatgcaggccgcattcgtcaagcatgacggctaccagtgcggctactgcacgcccgggcagatctgctcggcggtggccgtgctcgacgaaatcaagcgcggggtcccgagccacgtgagcacggatctcaccgcgcgtcctcttttctcggccgaagaactgcgcgagcgcatgagcggcaacatctgccgctgcggcgcctactccaacatcgtcgacgccatcaccgaagtggccgggagcagagcatgaagccgtttacctatgagcgcgcgcgttccccggcgcaggccgcggcggccgtcgcacggagcccgggtgccaggttcatcgcgggcggcaccaacctgctggacctgatgaagctgcagatcgaagcgccgacgcatctggtcgacgtgaacggtcttgccctcgacaagatcgaaccgacgcccgaaggcggcctgcgcatcggcgccctggtgcgcaacaccgacctggccgccgacgagcgcgtgcgccgcgactacggcgtgctgtcccgcgcgctgctgtccggcgcctccggccagttgcgcaacaaggccacgacggcgggcaacctgctgcagcgcacgcgctgtccctacttctacgacaccgaccagccctgcaacaagcgccagcccgggagcggctgcagcgctatcggcggcgtcactcgccagcatgcggtggtcggtgcgagcaaggcctgcatcgcaacgcatccgagcgacatggctgtggcgatgcgcgtgctcgacgcggcggtcgagacggtgcgtcccgatggccgcacgcgcgtgatcccgattgccgatttccatcgcctgccgggcgaaaccccgcacatcgaaacggcgctggagcgggacgagctgatcaccggcgtcacgctgccaaggcccatcggcggcacgcagatctaccgcaaggtgcgcgaccgcgcctcctatgccttcgcgctcgtttccgtcgcggcgatcgtgcagcgcgatggctcgggccgcgtggcactgggcggcgtggcgcacaagccatggcgcctcgaggctgcggaggccgccatgccgcagggcgccaaggccgtgaccgcgcagctgctggccggcgcgcagccgacgcacgagaacgcattcaagttgccactggccgagcgcgcgctggccgcggccctggtgcaagcgaggagctgaccatcatgaaattcgacacgcccgcaaccaccaatcccatcgaccagctcaagatcatcggcaagccgacggaccggatcgacggacccgcgaaaaccacgggctccgcacgctacgcctatgaacgaaacaccgaggtgcccaacgccgcctacggctacgtggtgggcgccggcatcgcgaagggccgcatcgcctcgatggacctgagtgccgcacgcgcggcaccgggcgtcctggccatcgtcaccgcgcgcaacgccggcaagctgggcaagggcgacttcaacacggccaagctgcttggcgggcccgagatcgaccactaccaccaggcggttgcactcgtcgtggccaacagcttcgagcaggcgcgtgccgcggcgcagctggtgcgcatcgagtacacccgcgcaccggggcgcttcgatctgagcgcggaaatggctgcggcgaagatgcctgcgcccagcccgttctcgggcgagccggaaacgaagaccggcgacttcacgggtgcgttcgccgcggccgccgtgcagctcgatgcgagctacaccacgcccgacgagtcgcacgcgatgatggaaccgcacgcttccatcgccgcctggaagggcggcaagcttaccctctggacatccaaccagatgatcgcctggggcgtcggcgacgtggccaagacgctcggcatccccaaggcgaacgtccgcctggtctcgcccttcatcggcggcggcttcggcggcaagctgttcgtgcgggcggatgcggtgcttgccgcgctgggcgcgcgggcggccaaacggcccgtgaaggtggcattgcagcggcccttgatgatgaacaacaccacgcaccggccggcgaccatccagcgcatccgcatcggtgccgcgagggacggcaagatcaccgccatcgcgcacgaaggctggtctggcgacctgccgggcggacaagccgagacggcggtcaaccagacccggctgctgtacgccggcgccaaccgcctgacgaccacgcggctcgccgtgctcgacctgcccgaaggcaatgcgatgcgcgcgcccggcgaggcgccgggcttgatggcgctggagatcgccatggacgagatggcggagaagctggggctcgacccgatcgagtttcgcgtgctcaacgacacgcaggtcgatccggagaagccggagcgcccctattcccagcgcaagctgatcgaatgcctgcgcaccggcgccgaacgcttcggctggagcaagcgcaacgcggcaccggcaaagcagcgcgacggacgctggctcgtggggatgggcgttgccgccgcgttccgcaacaacctgttgaccaagtcggccgcgcgcgtgcgcctggacaaccggggcatggtcacggtggaaaccgacatgaccgatatcggcaccgggtcgtacaccatcattgcgcagaccgctgccgaaaccatgggggtgccgctcgacagggtgctcgtgcgactgggcgattcggcgtatccggtttctgccggctcgggcgggcagtggggtgccaacaactcgacctcgggtgtctttgcggcgtgcatgaagctgcgcgaagccgtggccagcaagctcggattcgctgcggccgatgcggagttctcggacggcttggtgcgcgccggcgagcgtgtggtgccgctcgcggaagcggcgggcgcgaacggcctggtggccgaggacggcatcgagtacggcgatctcgacaagaagtaccagcagtccaccttcggcgcgcacttcgtggaggtcggcgtcgatgccgccaccggcgagatacgcgttcggcgcatgcttgcggtgtgcgccgcgggccgcatcctgaaccccaagtccgcccgcagccaggtgatcggcgccatgacgatgggcgtcggtggcgcgctgatggaagagctggcgctcgacaagcggcatggcttcttcgtcaaccacgacctggcgggctacgaggtgccggtgcatgccgacattccgcaccaggatgtgatcttcctggacgagacggacccgatctcttcgccgatgaaggccaagggcgtgggagagctcggcatgtgcggcgtcgcggcagccgtagccaacgcggtttacaacgcgacaggcgttcgggtgcgcaactatccgatcacgctcgacaagctgctggatcgcttgccgccggtggcgtgagctgctgaggtcatgccgctgcggccgccggggctctgctgcgggtgttcgcgatcagggccgcgccggcaaggcaaaggatcgcaagcacggccagcgccgaactggcgcctcggccgaaggcggccacatccacgcttgaaagtgccgggccaccgccatttccaagaatcatgcgttgcgcgccggaaggaagccccgccatcgccacgctcagcgtcagcgcggttcccaccatgatgccggtgttctgcagcgtcgaccggacgccgttggcaatgccccggcgctggggcaccacgctctggaggatcgatgcgttgttcggcgtcacgaaactcccgatgcccaggcccagcacccagaggcacagcgacagttgcaggtcaccgatcgtgggctgcagcagcgcagccagcagtgccaatgcgcatgccgcgagcagcatgccgcccacgcagatggattcgggcctgaagcgctgaagcaggatgcccgccacgggtgcggccatcagcatgccgaatgcgaccggtgcgatgcgcaggcccgcctccgacggttgcaggcccgcgcaagcctgaaggtacaaggccaccagcaagagcggcgcagcttgcgtcatcgacaggagcaggatgccggcgtaggcggttcggcgccccgggtcgccgaacagagacgggtcgaccagcggactggccaagcgcatctgaatgcgggagaaaagcccgatggcgcagagccccgtaagcatgaatgcccacacgggcgtgctcgtccatccgcgggtgcctgccatcgagagcgcataggtcacgcatccgatgccgatgagggaaagcgccgcgccggccaggtcgaagcgctctggcgcggcggccgcactttggggcaggaccttccaggaccacgccagcacgccaagcccgatgggcacgttgagcatgaagagcgcgcgccagccccaccacgagacgacgaagccgcccgccagcggccccacgacctgggcgagggccgcgaccatggcgagcacgcccagcgccagccccatcttgcggcggccgaacgcatcgctcaccaatgcgctggcgttggccatgacgcccgccgcgccgatggcctggcccacgcggctcgccagcatcagctcggcggtgggtgccagggcgcatgccgcgcaggcgaccacgaaaaggcacagtccggcgaggaagagccggcgccgtccccagagatcggccagccgtccaaagctcaggatgcaaacggtgctgaccagcatgtaggacagcaagatccagcttgcctgcgtgggcgaggcgtgcaggctgcgcgccacggcaggcagcgcgacattgagtgcgctgagattgaggaaacacagcagcgcgcccaagctggcagcgaggagcaccgcccagcccaccctgtctgcgtcatcggtcatcgatttcagtcttcgctcttgaaccccgatgcctggacgatggggcgccagtacacccgatcctcggccatgatgcgcttcaggtccgcgcccgggagcccggtcggctcgaggcccatgcgatcgacttgtccgcgcacttgcggattgcgcattgcggcaagaagggccgtctccagcttcgcgaccacctccttcggagtccccgccggcacgaatgcggcataggcggcattggcgcggtcgaaggcgtcatagcccgactccttgatcgtcggaacgtcgggcagccaactcaagcgcttggtgcctgcaacgcccaatatccgcaacttgcccgcgcggtggagttcgagctggctggccagcgcgtcggtgcccatcggcacatggtttccgatgatgtctgtcgcgagcggcgcaccccctttgtaagtgaccggcgtgagcggtacaccgacggccttggacaactgcagcacgctgaagtgcagcccgcctccgaggttggtcagtcccacgcttgcgctggcaggattcttcttgatccaggccacgtactcgggaatcgtcttgaacggctggtctgcgccggcggaaacgacgcagggcacattcgccaggtgcgcgacaggtatgaaatccttgtcgacgtcatagttcagccgcgcataggtcatcggaaaaaggacgaaaggcggtgtggcgccgatcaggatcgtgcggccatcgggacgtgcggtcttgaccgcctcgatggaaatccgggtcgaggcgccgggccggctctccaccagcacgggttccttgagcgtggtgcgcaaatcctcggccagcgagcgcgccagattgtcgagggcgccacccggcggaacgccgatgatcagccggatgggcgcgttgttgtcggcatgcgcggcagcgccgatcagggcaatcgacgcaccgagaaaaagtgtcttgaggaacgaggccatggtggaagtaccttcaaagttgagaacgaaacgggagaggaacggactcagaaggcgagggccggcagcgcgttggctggccggtgcgcggcttcgaaagacgacgcggcctgcagcagctgcaagtcctcgcgaaagcggccgaccagctgcatgccgatgggcaggccatcgcggcctgcaccgcagggcaggctgatggcgggatggcccgtgaggttgaagggcatcgtccacggaaaccagttcggccgcacctcggcatacgcttcgccatcgatctcgatgctgccgaacaggtcctggtcgattggcagggccgtgcgcgacagagtgggtgtgaagatgaagtcgtgggtctccaactgggcctggaccttgcgaaagagcgcggtcctggcaaacatggcctgctggaaggcgacaccgtcgacgtgctccgcgagcgcgagctgctgcagcagcgacggactcaacgcgctggcatgcgtttcggccagtggcgcgaaacggccgcgccagctggtgtggttgatcacccgccacaccggctcgacgtcatagccctcgctcgacatctcctcgagttgcgcgcccatcgaacgcaacgtggcaagagcggcttcgaaggccgcggcaacgtcggcggagatcggtcgcccctcgagcctcgcggaatacagaatccgtttgccacgaagatcgccggcgggctgcagcgcgtcgaagtagcgctgcgccggcacgcccagcgaccacgggtcggacccgtgggcgcccgtcatggcctgcagcatgagcgccgtgtcggccacgttgcgcgtggtgggcgtcacgtaggtgtagttgccgaaggcatcctgtacctggctgtggggcaccacgcccaggctctgcttcaagccgacgacgccgttgcatgcagcgggaatgcgcgtcgagccgccgccgtcggtggcgatggccaggggcgcgacaccggctgcgatggacgaggccgcaccgccgctcgagccgccactggtgcgcgttgcatcccatgcgttgcgcgtgcttccgaagagtggcgcatcggtcaggcacttggcgccaaattcggacgtggtcgtcttgccgatcaggatgccgcccgcctcgcgcatgcgcgccacggccaccgcgtcttgcgtgggaacgtggtcgcgatgcagcaccgagccgtaggtcgtccggacgttcgccgtgtcgacgatgtccttcaccgtgaacggcagtccgtgcagcaggcccaacgtctcgcccttcatcagcgcggcttcggcggccctggcctctgccatcgcctgttcgtggcagagcgtgatgaagcagttcaggtgcggctggaccgcgtcggcgcggcgcaatacgtcttcgacgatctccactggcgagagcttccgctgggcgacgagggtgcgcatctccgcggcggacatctcgaagatctccgatggcggaagacgagggaagtttttcatggtgtaaatgattgacgcgctacaacatggagtccaatactgttttcttgaaaaggcatatgcctagcgtatggcagcaccagacttcagaacgctccgctacttcgtggctgtcgccgaggaacgcagcgtcggaaaggcggcgcgccggctcaacatggcccagccgccgctgtcggttcacatcaagaatctggagtcggctgtgggcacgccgctgtttcgcagggcggcgcgtggcatggaaattaccgacgccggccatgcgctcttccagcgcgcgaaggaagcactgctgcttgccaatgaaggattcgacgccgcgcgggccatcgggtcgggcagcaggggccggctcacggtcggcaccatggtcgtgctttcgtacctggtgctgccgcgcctggagaacgcgcttcgcgcgaagctgccggacgtggagattcagtacgtggagctcaatgccgccaacaacgtctcggccatcaccgattcgcaagtgtccgtggccatctgcattccgcccatcgcccacgcaggcattgcggtcgagcgcatcggcacccagcctttgatgctggccgtgcgtgcggattcgcccttggcccgaatggccagcattccactggcgcgactgtcaggcatgcccctcatcgggctccccgtgcccgatggcgacgtcgacaaatccatcatcgcttcgatgctcaggcggcacgatgtgagcatgccgatcgcgcagcgcgtggcgaccatggtgtcggcgttggcgctcgtgctggcgggcaggggcgtggccatcttgcccgcctgcgcgcgtatcggccggccgccgggcgtggtgttcaggcctttgcgcaacgtcgacgcaaagatggacatcgccgtgtgctggcgcagcgattggcagagccccttgatcgagccgtttctggcgtgcgcgcgcgcgtccctgcgccaggcggcttagccgatcgggggttctctcatcgctgcagcaagccgttcgatggcagcgtctcgtccagcagcttgcgcgccgtctcgacgccggccaccggcagcagtttcggatcgagcaggcccacctgcaccagcacgctggcctggtcccagtagatatgctcgtggtagagcttgtcgccgcggaacttgaccaccgccagcagcggaatttccacccgctttccggtcggaggaacgcccggcagcatccacgggatttccgtggtgtgcgtgaagcagaacagcatctcgtcgaccacttgtgtggcgcccacggtgcgcgagaccggcaccagggaggtatcgggtggattgctgttgacgaagtggttcgtgtagaagtggtgcagcgccttgtagcccacgccgccggtcatggtcggaatgtggttgacgtagggttcaggcaccatcgtttgcatggtgtcgtcgacattgcgcgtgccgaactcgtattcgcagtgcttgtcccatagcgcggccaggtcgtggtgcgggccgatggccgacttgagcgcggcaatgctgcgctcgtgggccatgagcgccgaagggcggtggtagtgctcgccgcccgtgcgtgcaaaggcgtggtcgacacccgggtacacctgcacctcgacgttcggccggccgcgcagcgtctgcacgatgcggtcgcgcgcttcgggcgggcagaagccgtcgagctcggccgcatgcagggcgagccggcagcggatgttgtcggcctcgtccagcgccgcatcgatgcccacgccgtagtagccgacggcgacgtccgcatcggtgcggcacgccgccaggtaggccagcttgccgcccaggcagaaaccgagcacgccgaccttggcgtcctgaacttcgggtcgcaggcgcagcgtgtggatggaggcctggatgtcttccatgccacgggcctcgtcgaagccctgatacagcgcgaatgcgcgctgccagtcgtccggcgaatagccaagctcgacgtcgggctgctggcgccagaacaggtcgggcaccagcacgacgtagccttcctcggcgtagtagtcggccacctcgcgcatcgttgcgttcacgccgaagatctcctgcgcgagcaccaggcccgggccgctgcccgagcgcggcacggcaaggtagccgctgaaactgccgctgccgtcggtggcctggatgcggattcgggtcgtggcgccgggtgctttttcctgcatgtgagtgctccgttcaagggttggatggtgcgggccatgcgttcattgcacgcattccgggtgtcgcgtcgtcacctggtagtagcccgaatgaaaaaccagcggctcgccgtcgaagcggtcgtagcgctcgacttcaccgatgaagatgaggtggtcgccgccatcgtactgcttcacgttgcggcagatgaaccgggcgatgacgccatccagcagcggcacgccggccgcgccatcgcagcaatccaccccgccgaacttgtccgcctgcggggtcgagaactgccgcgacagatgatgctggtgcgccgccagcacgttgatcgcgaaatggctggcgccggtgaagtccgccacgctcggcgcctgccgggccaggctccacagcaccagcggcgggtccagcgagaccgacgaaaacgaattggcggtcatgcccacgcggcggccgtcgatcgcccgggtggtgatgacggtcacgccggtggtgaactgcccgagcgccttgcggaagtcgcgccggtcgaagcggtcgcaggccgcttcgcgcgcccgggtttccaggaagcggtctgcttcggcggcatcgaaccaccagggcgcgaagacgcgcgggtcgtcgaagccgttggcgatggtgctcgccaccgccggcacgtgggtggcgctctgcagcagcttctgcatgtgcggcttcgggggcgcgagcaggctgtgggtccaacaggtggcccagcgggcatagccttcccagtagcggtcgaaggtctcctgcatccacgccgcatcgaacggtgcatcgccgtgttcgaggatccgtttcaggtagatgtcggcgcacttggccgcgttgttggcgccctggccggtgatcggatcgttgagcaccacggcatccgccaggcccagcaccttgcgtcccgagggcagtgtggccacgggcttgcgcaccgtcggagcgaagcggccgacgaggatgccgttgtcgtcggtcagctcgatgtccgtgcagcgctctgcttcccagggcaggaaggtgtcgagaatccgcttgctgcgcgcgagatgctcctgcggcgtcttcacgtccgcccagcaatccatcgggccgcccggcacaccctcgaacaccatgatctcgcaggggcccgtggtggtcagcgccgggaacacgaagtattcgcccacgccggggatcaggttgaagcacacgcgcgcatggggcagtgcgggcttcattcccttcacataggtgagtgccaatgcacgctggggctgatcgaatggcgagcgctcggcgtcgcgctcgaacagttgcgaaatctcgcccttgccactggcgacgaccacgaggtcatgcgccgccgcgcaggcttccagcgcgtcgagcccgacgtcctgcagcaccagccggccgccgcgcttctcgaactcggccatccaggcgggtatcttgagccgctggtcgaccgactgcgcgggcccgtcgagccttgcgctccactcgatggacttgccgccttccaggttgcgcaccgcgatgccgatgccttccacggcggggcattcgtccgcccaccagtccagttccagttcgcgctcggtctgcagtgccgtctcgaacatgcactggctggacatcaccggtccttcgaagatctctttcgccgtgcggttcgaaaaaatcgtcacctcgtaccccgcgcgctgcaggccgagcgcgagctgcatgccggactgtccggcgccgacgatggccacgcgttgcgtcatgggttcactcccggctacgcgacggccgcgcaggtttcgatgtagcggtccgcttccgcgggatccgcaaaccacggaaagaaggtgcgcggatcgtcgaagccgttggcgaaggcgctggccagcggcggcatggcgccggcgctgccgagcagcttgagcacatggggcggtggcggcgccagcagcatgttggtccattgcatgacccattgcgcatagccgaaccagtagcggtcgaaggtctgctgcatccacgccgcatcagccgtgccattgccgcgcgcgaggatgctcttcagataggtatcggcgcatttggccgcgttgttggagccctggccggtgatcggatcgttgagcaccaccacgtcggccaggcccagcacgcggcgccccgagggcagcgtggccaccggcttgcgcaccgtcggcgcgaagcggcccgcgagaatgccgttgtcgtcggtcagctcgatgttcccgcaacgcgcggcttcccatggcgtgaaagtgtcgagaatccgcttgctgcttgcgagatgctcctgcggcgtcttcacgtccgcccagcaatccatcgggccgcccggcacaccctcgaacaccatgatctcgcaggggcccgtggtggtcagcgccgggaacacgaagtattcgcccacgcccggaatgaggttgaaagacaccgcggagaaaggctcgcgcggcgtcattcccttcacataggtcagcgccaatgcgcgctgcggcttgtcgaagctcgacttgtgggcgtcgcgctcgaagagcttggagatctcgcccttgccgctggcaaccagcgtgagatcgtggctttgggtgcaggcttcgagttcgtcgatgcccgcgtccttgaagacgagctcgccgcccttcttctggaacaggtccatccaggccgggatcttcacgcgctggtcgaccgactgcgcgctcgaattcaaccgcgcgacccagtcaatggccttggcgcccttttgctcgggatggggaacggccagcccgatgccatccacggtgggacagtcctgcgcccagaggtccaggcccaggtcacgctcgatctgcagcgaggtgtggaacatgcactggctcgacatgaccttgccgtggcggatgtcctcgcccgtgcggttgctgaacatcgtgacctcgtagcctgctgcgagcagaccgagacccagttgcaggcccgactggcccgcgccgacgatggcgattcgcttcattgcttgctccttgatgctccgttcggagctagtccatcaacttgggaatggcgggcacggcctgctcggggcccatggcggcatagccgccgtccaccgcgtaatcggaaccggtcacgaagctggcatggtccgaacacaggaacagcaccacctgcgccacttcgtccggatcgccgacgcgcccgagcagatgaaagggcgcggccacgcggtcggtcttggcgcggtcgccgccgctgagccggtccatcacggccgaccatgtccagcctggcgacacgctgttcacgcggatgcggtccggcgccaggtccatcgccatgttgcgggtgagctgcgccatggcggccttgctcaccggatagagccagcgcccggtctgcgccacgcgcgacgagatgctcgtgaagttgaccaccgccccgccgcctgtcgccaccatgtgcgggtgcacagcctgcagcatggccaccgcgcttgccacgttcacgttgaacgaagcgagccagtcggcgcgcggcgacttgaagccgtcgtccaagtaggagcacgccaggttgatgagaaagtgcacaccgccgtgccgcgcggccgctgccgccacgcaagcccgcacctgcgcgtcgtcggtaatgtcggtgcgcgcgaagtgcacgccggtgccgagcgaatccgccagcgcctggccgttgtcggcatcgatgtcggcaatgacgaccttcacgccggccgcatgcatcgcgcgcaccacaccggcgcctatcagcgtggagccaccggtgacgatggcgctcttgccttcgagtcccttgaacatgacgcttgctctcctcggttgatcgggcaggccgggttggcctgtggagcgaacgttatgagcgagcaggcccttggcgaatcccgcaaacgcaagccgtgtccctggcgcgcaggttttatcgagggcgggtccgaattgtgggcggggatggtttttgctagggtgccttggtcccatggaaaccgccacgaccccaccgctgccgctgcagcgctaccggcttttcgagagccacgacatggacgaggcccgcgaaagcgtggcgcgcgtgttttgtccgcacgggctggtcatgctgcggcctcgcaccgagctcgatgcctgccatcacagcgcgcgccttcatcgggacgtgagcctcaactatgtgcagtacggccccggcgtgcagatcgaccccggctacctgcaggatttcttcctgttgcagattccgttgcgcggcggcgccgagatccgctgcggcgcgcagcatgtggaagccacgcctcgccttgcctcgctgccatcaccgaccgagccgctgtcgatgcgctgggccgacgacagcccgcacctgatcgtgcagctgtcgcgctccgcgctgctctcccggctcgaagccttgctccaggcgcccgtcaggcagccgctggtgttcgaccttggcgtgccgcttgacaaccccgccctcgcgcccatggtgcacttcatcgactatctgcggctcacgctcgacgccggcaccgcactgcaggccggcagctgcctggccgagcatgccgaggagtacctgatggccagcctcttgatgtcggcggggcacaaccattcgcgtgccctggccggcgacgcgcagcgcagcctgctgccgcgcgtggtccgcagggcacaggaatacatggcggcgcatgtcgagcaacccttgtcgctggccgacgtgtgccgcgaagtcggctgcagcgcgcgtgcgctgcaactggcgtttcgccagcatgcgggcctcggcccgatggaattcctgcgcgaactgcgcctcgacaaggtgcgcgccgagctgcgggtgccgggccatggcggcgtgcgcgacgttgcgcaaaaatatggttttctacacatgggccactttgcggcgcagtaccgaacccgcttcggcgagcgaccctcggaaactcgagcgctgcgagccttcttctgacgcatggccgttgcaggtctgattgaaaacacgtgctcgcgcgtgcccgcatgagcgcaagccccaccacccaagaccccgacctgctgcgccgcttgctgcgtgccaaggaccggatggacgccgcatcgcacgaggagtggcccgtcggacgactggcgcaggtgagcggcgtgtctgaagcccacttcgcacggtcgttcaagcaggccttcggcattcccccgcaccgctacctgctcacgcggcgcatcgagcgcgcaatggcgctgctgcgcgacaccgacctgcccatcaccgacattgccttcgacaccggctgggcgagcctgggcaccttcgggcgcacctttcgcgacatcaccggcgacagcccgagcgcggtccgctcgcgcgggatgcaggcggcgcaagagatcggccgcgtgcccgtctgcatcgccaacgccgcgcgcaggcccgacctcacgaccgcagtttcggagaagcggcgcctggcggcagacggtacaaacgagccccaacaacaggagagtccatgaaagagggtattgaagtcgtcggtttgtacgtgcgcgatcaagacgaggcgctggcgttttatgtggagaagcttggttttcgcgtccacacggacgtgaagaacggcgactatcgctggctcacggtgcagcacccggagcagccgtcgttccagctcggcctggtcacgcccgggccgccggtgctcgatgcggcgacggcgcaggcgttgcgtgccctcgtggccaaaggcgcgatgccgccgctcgtgctgacggtggccgactgccgtgccgcctatggccgcatgcttgccgcgggggtggagttcacgcaggagccggtggaccgcttcggtaccgtggacgcgggctttcgcgacccgtcggggaatggctggaagatgattcagggacggggctgaaagatcaccgcaccggaacgtgcacgtcccatttttgcgcggggctcacggtccgggtgcattccaccgcgatgacgcggcggctgcgtttcagtggtttgctttcggcactggtgtcgaaccaccagatctcatgccaccgtgccttcagggcgacggcacatcgaggaacgagaactttcagattcggttccagcgcctgccattcgctctgggggtttcttgcgttctcctgtgcaacgaatttgcgggcttcctcccgtatctcgtacaggccatgcaccgcgtcgttggaacgcatgtcctcgatgcccgtcgatgaaaagcagtgtgtcgcccaaatgagcagccacaagggcaggaggttgtgatggatgtgcatgcaggcggtcgcgcagaggtgtcggataacggatcgctgctgcgatcacaagtgtcgactgtcagaaggattgagtcccgcgtcccttggagtcaaatacttacgcgccgatcaatcactgtgaatcgccccggattttgtggaggccggttggtctaagtcatgccgccgccatggcggcctgactggcgagttgccggtagcacgtccagcgctattcggtcaccagcacgcccgacaacaatctcgtcgggcgtgatccgaaggactggcagttccagtgaacccgatgcgcgattaccggcgcatcgatccgggcgacgcatcttgtcgttttttcacggccgcgcggcgacgatttgcgtggttcggttcttgcggcatttatacaattacacacaatatgccaaaaatgtcacagatttcaagaaaaatgagtgaggtgtccattgaccgatcgtcgccggttccgtcgatcctccgccactggagtcgcgcgcggctcatcgcgatcggcctgctgagcacatgggtcgcggcttgtggcggtgggtcgtcgggcccttcgacagcagcgctcgttgcaggcacaaccgcacccgcacccgcacccgcacccgcacccgcacctgcacctgcacctgcacctgcacctgcacctgcacctgcacctgcgcccgcacctgcgcccgcaccttcgatcactacagccctcggcaagcccggccggctcctcgtgggcctcggcgcggccaatacttttgcggacatgaaggcccagcagatcgctccggacatcatcgatacctatctcgtggcggtcacgggtttcaactctggcggcggtaacgcatggcctcaatggcaatacaactatccggacggtggcgtcgtgacgaaattctccgccgacgtcgcggccatgggcgccgtgccgatgttcaccctgttccagatgccttccctgcggggtggcgacgtcaccgtcatcaacgacgcgccgttcatggccgcctactgggcgcaagtcaagttgatgtaccagaagatcggcgagaccggcctccccaccctggtcaacctcgagcctgacttctggggcttcgcagagggcagtgcccccggcggcgacccggcgaagttgccggcgcgcgtgagcacggtgccggaatgcgccagccaaccgaatacggccgtcggcgtcgtcggttgcctgttgacgctcggacggacgtacgcgcccaaggcgaggatgggcttccccccgtcgttgtgggcgggggatgcaaacgccaccggcagcttcatggcaaaactcggtgcagacaaggccgacttcatcgtggcgcagacgagcgatcgcgatgcaggttgctttgaagacccgaaccccgtgccaaattgtgcgaatcgtggtcccggcccgttctacctggacgagaacaacgtcaccacaccgaatttcaaccagggcatcaacgattggagcatcgtgcggagccacctgggcggcctgccgatcctgtactggcagacccccatgggcgtgccgtcgacgacccccggcggaactccgaagcactatagggacaaccacgtccagtacatgctgacgcatccaacgcagtacacgggcaacggcacattcgcgatcgtcttcagtcccggggacgccacgtcggcggacatcacgaccgatggcgggcagttcgcgcgcctgtcccgcgcctacctggcgaacccggctccgtttccccgctgagctcaacgggagaacaaggaaccgccgagcgcggttgttggtcgcattctgccgcgcccgaggccagcgctgcgcggcttggcggcgcagttccaagctcagtgaaagaaattccattcccaatgaaacacgatcacaaggagacggccccatccacctgcgtctggatgacactaaacgcctcggacgggttcggcgagcgagagatggaacgtccgatgacgatgtgactcgctccccaacgtatcgcgtcgaacggcgtagccactcttgcctggtcattcttcgcatcggtttgcagctgcgtgcctggggtaacgatgagcatttcaggcggaaggaggtcgcgaagcagccgggcctcctgggctgatgcgaccacgccatggcagtcggccgcagcggccagcttggccagtcgtacgacttgctccgggaccgtcgtgtccaagcccagttccctgaggtcttcatctcgcaagctcgtgatcaccgtcagcgccagcacgttcaacttggggtatgcgcgagcagcttccaccgcggcacgcagcacggcagagcctccggatgcgtgaacggtgaccatcgacgctcccaaagcaccggccacctgtactgcagcggcgaccgacgtgggtatctcatggagcttcaggtcgagaaagacttccttgccacccgagatcagcttttgcaccacggccgggcccgccgcagtcaacagttgaagaccgaccttgtagaaccgcgccgatggtccgagccgctccaccagttcgaatgccccactggccgagtcgaagtcgagagacacgatgatgttgttcttctgtgtcattgcagtgcaaagtgaaagggtcgttcggatgatcggtgctggctgcatccggccgttcgacagcgcgtcgctcttgcttctctaacgaagatgttgaccgaccttctgctgaagtagcgccacaagctcgggctgcatgaactcatagcgatcaggaacgtccaggcacacgatcttttttccttgcagcgatgccgtaaaccgctgcttgagctttgcccggtgctgcttttccatcacgaagatcaggtcggcccattcgacctgttcggcgctcagtacgcagtccgcgtcgggtgcgaggccagcggaatccgtctcgatgccgggccctgcgaacacgctctcggcggtggggctgcgaagcctgttcctgctgcagataaagagcacgcggcgcatcggtggtgtccggatgggatggtagggccggattctggcagacgcccgacggaggctgctcgtcagcgtccgctcgctggccagctcagtccacccgggtctcgggaagcttcgcaatcaccttgatctcgaagtcgaagccgtagagccacgtcacgccgacgccggtcagcgtcgggtgcggcgcgttgccccaatactcgggcaccagcttccagattctctcgaacttcgattcgggatcgacgatgaagatggtcacgtcgatcacgtcgtcgaaggtgcagcctgcggccgcaagcactgcgttcagattgccgaatgcgagccggacctgtgcttccaggtcgggctcgggcgagccgtcttcgcggctgccgacctggcccgaaacgaacaggaagccgttggaacgaatagcgggcgaatagcggttcttttcatagagcgcctggcgcccgggcggaaaagcgacgtcacgtgtggtcatggatgtgccttcttcattgaacgggccgaagccgaccctgtggttgcgatgaagggactctagacatccgcgcctcgccgataaaccggcaaagccaataatcactgtttgggaatgccgaacaatccggaagcatcaggagcagagagatggaccgtttcgatgcgatgcaggcgtttgcccgcgtggtggaagcaggcagcttcaccaaggcggccgagacgcttcacgtgagcaagaccaccgtgacgcagctggtgcagcagctcgaagcgcggctgcgggtcaagctgctcaaccgcaccacgcgcaaggtcaacgtcacggccgacggcgcggcctactacgagcgcgtggtgcgcctgctgggcgacatggacgatgccgagaccagcctgtccgatgcgtcggcgttgcccagagggcggctgcgggtggatgtgcccagtccgctcgcgcgcctgatcctggtgccggccttgccggcgttccacgcgcgctaccccgacatccagttcgacatgggcgtgagcgatcgcatggtggacctgatcggcgagaacgtggattgcgtggtgcgcggcggcgagctcgccgaccagtcgctgatggcgcgccgcgtgggcgacctgcagctgggggtctacgcggcgccgagctatctgcagcgcgccggcttgccctcgcacccgcgggaactcgagaactcgcatcaccgcgtcgtgggcttccactggccgcgcaccggcaaggtccttccgtacaccctgcaccaccagggcggcgagagcatccaggtgcaaggccgctacgtgctggcggtggacgacggcaatgcctacctcgcggccggcctggcgggcctgggcgtcctctggctgccggactacatgtcggatgcgcacgtggcgcgcggcgagctggtgccgctgttcgaaggctggcgcctcgatccgatgcccatctacgtggcgtttccgccgaaccggcatgtcagcgccaagctgcgcgtgttcatcgattgggtcgccgcactgatggcgcaacatgcgcctgtccagcgcccggccacgcagcggtgaagaggatccggccttctacggtccggagcgccgaccacggtcagtacacgtcgcggcgatagcgtccttgcgcaatcagcgcgtcgagccccgcggcgcccagcacctcgctcagtgccgcatccacgccgggcgccaggccttcgcggctgccgcagacatagactacggcgccatcggcaatccagcggcggagctcgtcagccgcttcgcgcaagccgtgctgcacgtacctgcgctcgggctgatcgcgcgagtagacgaggtcggcgcgcgccagcatgccgatggcccgccactgcgcggcatccgcggcgcagaaggcatcgtgcgcggcttggcgctcgccgaataccagccagttgcgcgcatggccccgccgcacccgttctcgcaggtgcgagcgcagtcccgcgtaaccagagccgttgccgatgaagatgcagggcagatcctcgtccaccagcgcgaaggccggattcgcgaccagccgcatctggaccgcatcgccgatctgcgcgccggcggtcagccagccggaggcgagacccaagccgccttcgtgccgcacctggcgcaccagcagctgcacgcggtcgtccgctgagatcgaggccaccgaatagctgcgcggcgctggccgcgggtgctggtgcgcatcggcatcggcggcggcgtgcgcgccctgcaacagcacctcgaccagcgcacccggctgccacgccggcgcgcccgcgcgatgcagttcgatctcgaacagcggatggccctggctgcccggattgagcagctggcggcgcaccagccgccaggattcgaagggccgctcggcagacgaggccgcatgcgacggccatgcggcgcgcacatcgaaggcctcggcgatcgagcgctgccagcggccgatggcttcgggattgccgttgtcgacctcgaccatcgggaacagcgcctgcgcgccctggttgcgcaggtcgcgatcgagcgtgcggccgaaaccgcagaaggtggcgtagtgccagtcgccgagcgcgagaacgccgtagtgaacgtgctgcaactgcgaacccgcctgctgcgcgaacttgcgcgcgaaggcacgcgcgctgtcgggcgggtcgccatcgccggacgtgctgacgacccacagcaccttgcggaaatgaagcagggcatcgacgctgagttcggccagggtcttgaccacgatgccgaggcccgccgactgcagcgcggccgcggtctgcagggcgacgcgttcggcatggccggtctgcgtggcgaaggcgatcagcacctgctccgggccctgcccggtgccgccgcgggcaaggcccagctgcgcgcgctcggcgcgcagcgccttccgggttcggcggcggccgaggtacagcatccagccggtgatcgtgaacagcgccaggcccaggctggcgagcatcatcaggatgcggccgggaagaccccagtaggtgcccatgtgcagcggatagatgctgttcacgaggcggccggccatgggcttgtcggcatagcgctcgtgctgcgtcgcttcgcccgtcgccgcttgcagatagagccggttgcgcgcgcgctcgtgctcgggcgctgcgcgcaggtaggtggcttcgacctgcgaggcattgcgcgtgggcaggcgcagcgtgacctggctccagtcctccagggtcgtctgctggaaggagcgccacacgcgctgcaggtcgagccgcaccggcgcgccaccggcggccgcgtcggcgggtccggcgccctgcatgcgctgcatgcgaacggcgcgcccttcaccggccgcatcgtcgatcacggtgcgcaccgcgtcgaagccccagtagagccccgtgaagccggagaccaggtaggcgagcagcgcgacggtccccgcgactgcgtgcaggttccacaggaaggcgcggccgctgagcgcaaagtcgagccgcagccagctgcgccacgcgagcggcctccgtggccagcgcaggtacaggcccgacagcgcgagcaccagcaggcccgcggccagcgtgcccgtcaccggcttgccggtatcgcgcggcagcagcagccagcggtgcaggctttcgacgaactcgaagaaggcttcggcgcgcggctccggcagcagggcgccggtgtacgggtcgagcaagcgcgtctcgccgcgccgctcgccgggcggcggcgtgaagttcacgcgcgccggccggcctggctcggcgaacagcgagatcgttgccacgcgccgccccggctccgcggcctgcagccggtccagcagctcagctggtgtcagcggccgggcgtcagccgcatgcggcaggcgatgcagggccggatcgatcaggtcggtgatctcggcgcgaaaggacaacaccgcgccgctcagtccaatgaccagcaacaccgatccggccgtgatgccgatgaaccagtggatctggaaccaggcgcgtcgcaacaaagccatgacttgcccgtcctcagagatcgatcttgacggtggccttgatcgtgcgcggaacgcccaccgccagccgtgtgcccgccgccgaccagtagcgcttgtcgccgaggttgtcgacattgatctgccacagcgtccgcttgccgaagagctgcgtcacatagcgcgcgccggccgcgaagatcgtgtagccgccgatgaagccctgattcaggtcgtcgatcggccgcttgccggtgtagtaggcgccgccattgaccgacaggcccggcaccgcggcgatgtcgtaggagaagaaggcgctggccgtgtatttggcggtgttctccggcatcttgccgttgtactgggcgttgatgccgcggaactcggcgtccagcgtctgcgccgagagctgccaggcgagctgccgcgtcaacttgccctgcgccgagagttccagcccgcggtagcgctggcggccgtcggccacgaaggtgttggcgctgttggtgtaggcgcccgggcgttcgatgtcgaacagcgcggtcgacagcagcgtgcccgagccggtgagccagcgcagcccggcttccttctgcttgctcacgccaggcggcatgcggttgttctggttcgcggtgccggcaggcgcgacttcgccttcctcgacgccttcggcataggagacataggccatgaggtcgggcgtgaacttgtagctcaacgcggccagcggcgtggtcttcttcacgtcgtagtcgatcttcggcagcgtcgagctcgcgaactgcgtgctctcgaagcgcgtatgccgcacgcccgccaccagctgccattccggcgaaaagctgatgcggtcgagcgcgtacaggcccagctcccggctgtcctgcgcgccggtggtgggctgcgtgagcagcgcggtcagcggtagatagccgatggcgcgcggaaaatacaggttctgcgccgtggtggcgccgccgtagttgcgctggaagatcggatcctggctcttgtcgctctgcgcggcacccagcgtgagctcgtgctgcacgccaccggtcgcgaaggtgccgaacagttcggtgcgcagcaggtcggagcgctgctccaggtgctgcacgttccccgtgatgcggcctgcgccggtgcgcacgttgtagttgctgaaggtggccaggcgacggtcgcgctgggcctccgaatggccggcttccaccatcagtgcccagttgtcgctgagggagtagtcggcccgcagctgcgcggttttcacctcggcctcgaacaccgccgacggcgggccgatgagcttgtgcggatcgggcagggccggcagcgcgatcagtccgttgacggccgccaggcgcgcaatgccggcctgctcggtgatgctcttgcggtagtactccagatcggccttgagcgtgagcctgctgttgacgcgccagtcgaaggcggccgacaggaacttgcggttgccgtccacgccgtcgatggtcgagccgagctgcccgcccgccgcgttgatgcgaaggccgtactggttccgatcgccaaactggcggccgaagtccacaaagccctgcatcgtgccctggtcgtcgaagctggtgcccaccgaagtgaccggcgtgctgcccgcgcgcttggtcaccaggttgatcacgccggcgggcgaagtaaagccgtagtagagcgccgaggcacccttgagcacctcgacgcgctccttgttctccatcgggatctcggacacgttgggaatcgcgagcgagccattgaggcggtagttggtgcggttctccacggcaatcccgcggatcacgagctggtcgaaggtatcgccgccgttctgctggcgcgtgacgcccgccgtgttgcgcagcacgtcgtagatgccggtcgcgccctgcagctcgatgacctcgcgcgtcaccgtgttgacagtggctggcacctccatgatgctggccccgcggaaggtgccggcctcgacggtgttggcgacgaagccgctgtcgcggtcggaccggacggtgaccgcgtcgagctcgccgcccacggcaacggtggaggaggcggcctgcgcgcaggccagctgggccgccaacgcgagcggcagaaagacaaagaaattgcgcatggaatcgcctgtcgacggggcttgatcccggcgacgacatctgaaagagagctggagagcgggcgattgtaagtcaaacgaatgagaattattcgcatgacggagcgttgcaggccgttgtcggcacggtcgacgcctgccgcatccgcgaagctcggccagaacccgtagcgcccgcgcgagagcgtgccgaacgctccccgcgcctcctcagcgccgccgctcgatcgcgctctcgcggtagtggcgggctttctcttcgtacatcgcgcggtccgcgcgctgcagcgccgcgtcgagctggtcgccgacatcgcaggttgccacgccgatcgcaaggttcagcacgtgtccgctctggcccgcatagaactggttgttcaggtcgagcatggaggcgatgcggtcgcgtatcgcctcggcgccgcgctcgtccgtcttgggcagcacgaccgcaaactcgtcgccgccgatgcgcgcgggccagccgggctcttcgaccgccttgctcagcacctcgcccacgcgccgcagcagcgcgtcgccggcggcgtgtccttcctcgtcgttcacgggcttcaggccgttcatgtcgatcaccagcaccgacacgggccagggacccttgcgggacagccggttgatttcttccgagaagaagacgcgattgcgaagttgcgtcagcacgtcgtgcttgcccaggtactcgaggtaggcctcggcctttttcctggccgtgatgtcgatcagcgacaccagcacgaggtcccaggtggcgagccggtcttcgagcacggcaaactgcatgtggatgttcagcaggtcgcccgtgagcgcgtagttgacgacctcacgctgctgcagcatcttgccgttccagaggtcctgcagctgctcggcaaaggagtcgtgcatctcgtcgcggaagatgccggagaggttgtcgagcagctcgctcttgtcggccgcgccgaacatccgcagggtctcccgattgacgtcgatcacgcggatctcccgcatgcagcgcgtgatgaactccgggtgcaccttgatgaaggtcgcaaaatcgctgatgccccgcttgcggatgtcgtcgagcaggagcttgaccccgctgaagtcttccacccacagcgacaccggcgaacgctcgaacagctcgcgcgcgtagcgctcgctctccaggcgcagccgctcggcccgcacgcgctcggtgatgtcgtcgagcgacaccagcacgcgatcccacgaggcctcatggccgggcagcacctgcacgcgcacgtgcacgtccagcctgcggccgtccagcgcatagttgaccgtctggttgtcgaagcagagttttccgcgccagagctggtccagctcgtagatcacgggcgcggtcatgtcgtcgcgaaagacgctgtcgagccgcgacagcaggtcggcctggctttgcgcgccgaagagggtgagcgtgctctggttgacgctcagcacccgcagctgcgccatgcattcgcgcacatgccgcggctcggcattcaggtgggccaccagatccaccacaccggcgctgcgccacgactcgaacagctggcgcagcccgctgtagtcttcgagccagagcgacatcggcgcaaactcgaacatcgattcgtagtcggtggtggacggcatggattttttcctttgcgcgaggggctcgtgtccgcaatgatgcaccctcggcggaacgcggcaatgcgcggcccatgcatttcagcgcctgctggcgcggtgccgtggcggcggcgtaacgccgcgcggattcagcttgtgaagtacaggccgctatacaccggcacacaatgatcgggaaacccgggcaggtcgatcgaacgctcgggcacctgccactgctcgcgcagcgtgtagcccagcgcctggacctccttgacgaagcggcggcggttgtagacgtgcatcggcgcgaagcagccggcgccgatgttctgcgtcgtcacatagtcctcgccgccataaagcggaaccttgttcaggagaatgtgccgcggacgctgcccgcactgctggagcagcagggcggggcgcgcattctcgagatagtgcagggcgccggcagagatccagatgtcgttgccgggcagcgcctgcgcgaggtcgtcggtaaagctcaatgcgccggcctcggcatccggcttgctggccatctcgcggccgatggtagcgatcgcgggcacttcgaccacgcgccaggacaggtccttcggcatctcgaaatagcggcggtaggcatagaaatggacgcccaccgagccaccgatgtcgagcaccttggtggcgccatcgcggaacgcgcgttcgagccaccacatcaccggatagtcgtaggcaaagatcttcttcgtgcggacgtccacgtactcggccgccagggcggcgtggtcgaattcaggactggggggcagcgaactccgcgcctcggcaaagctcttgaacaggccgaagtaaccggcgaaaccggcctcggaaaaaaaccgccggcgccgccagcgctgcagcgccggccgggcgaccggcccttccaggatcttccggacgatttgcggagcaccggagtaagccatgttgcgtcccatcctctcgacgatcatcgcctgccgcggttctgacgcgcggtgggctgattcgaaaaatggccggcacggtcttcccgaatgccagccgggaatgccgtcagcatacgatgaaagtagtaacaaaagatagtctttatggctgggtgcgcggagccatgccggtcagtttccgggcgcgatgaagtccggatggcgcgcgcagctctgctccagcgccaggtcaagcatcgaagcgcacgatgagctgcgtccccgtgtaggtcggcgtgaccttgaagcccggcgcattgatggccgagaagcggccggtcagggcgccgctgctgatgaccgtgagcgtgtcgcccgcgctgggcacaaaaccgggcttgaagctcaggttcagcgttccgtccagggcagccacaccagccacgctcaggcggcccgcaccattgccgcccagattcaattgcagcgtggtgcctgccagctgcgtgtaggcgcccgccatcatgagcgtcgaaggcgcgttgcagaccagcgtgccaccaccgacgtagacattgcccttgccgaaggccgcggtggcgtccgcctgcagcgtgcctcccgcgagctgcgtgccgcctgcgtagctgttgctgccgccgagcgcgagcgtgccgctgcccttcttggtgagcttgccggcgccggagatgttgttgcgccagctgtccagcgcatggaagccaccgaggctggcgtccatggtcacgaccacgtcgccgttgaagacgccgtagccgtcggctgcgtcgaacaggttgagccggccccagccttcggggtcgtccatcaccgggtagcccgaaggcaccgccgtggtcttgagcaccacgcggcgctgcgtggcgtcgagatacggcaggcgcgtttcgagcagcacttcggcgcccttgggcaccacggccggcctggtcgcatcggccacctgcttgaagccgaaggtcaggcggcgcaggtagtcggccttgctcgcggcatggtcggcaaagcggtcggccgcaacgccctgcgaatgggcaaagctgttgaaggcggcggcatcgctcgcacccacggcggccatcagcacggactgcgcctgcgcataggccgcgctcttgcgcgcgacgttggccccggtggccaggctcgcggccgccgcggcctggccctgcacgcgcccgccgaccacatccagcggcgaatgcatgcccgacaggatgcggttctcaccgagctcgagaccgcgtgccaccatctcctgaaaccgctgcggcaccacgtagccgaacgcgatggccttgcgcacggcctcggccgtgtggccgctcacgaagccgccgtcggtagggggcgtgctgctcttggcgggctccagcgcaggcaccaccttcacgctgctgctccagcgccatgggcgcgcgtacttgtaatagcgcttggcgggttcggtggaggcgttctcgccgatgttgttgagcaggtccaccacggtgccgaagctggggttggcagcgccgggcacgccgatgtcgctgccggtgtcgttgtagagcttggtggtggcgtcggcggcgatgccggtgatggtggtgctctgctgcgtggcggcgcgccaggcgctggtgagcgggcccatgccgtcgctgatgctgtagcccttgccccggcggtcgtccagataggcggccagttcttgcgcactggtgcgcgcgttggtggcgtcgacgacgtactggatgttgctgttcagtaccccggcgttgaggatcttgccgtcggtggcgtcgcccggaatgccgctccacgtggatgggacgatggccggaaagctgccctgtgccggcgccgatacgcccgcgtcgaccagcagcgtgctgggctgccagaggtcgaggaagccgaccagcacgcgcacgccggcattggtttccttggtcgcgtagcgcgcatcgccgcgctggttggtcgcgatgttgtcgacgaaaggcggcgtggcgaccgggtcgggcacgggggcggtgtcggtgaagcccaggtcttgcggcggaccggccacgacaacggcgggcgggttcgtggtggccggtggcgtaccgacgatggggaacgaggcgccgccgtcaccgccaccaccgcatgccgaaaggcagagggccgcgacgagggtgatggcgaaggtgcggttgaaggacgggagggacgacatggtgaagtggagggagagattgtgaaaacgcaagcggaacgatcgtccgacacggccccgcgcaatctatccacgcaacaagtcgtttttattaataatcgtttgctgcgctgcaatcactccccttggcgcgcctccatccgttgccccgtaccatgagcttcatcgtccagatcttcgatcgcattaccgccaccgacgtgcgcagtgccctggctgcatgcaaccgcgatcaaccggtcagcccccgggtggctgccatgttcgagcaattcctgcgtgaggtgcagtgccatttcccgctggcggcccgtgccaacggcgtggaccaacccctgatctggaccgaaggcctgccgctggggcccgtggaaagttctccgctcaatctgggcgtggaggtggatgcactggacgacaccgtgctctccaccctgggccatgtggcggccgatgccgggctgcagatgctggagccgcagggcggggcactgtaccggctggaccggcaggtgatcttcgacgatggcagcgccgagccctttgccgaacggacgccccgggccgagccgcgcgcggtggccgctgcgagcttcgatacgacgaagacgccccattcgctggatgtgctgtgcggcgcgctgatggaaaagctggggcctttgggcttcgaggcccagccccatccccactgggagcacgtgcggctggtgcaacgcacctacgggcccacggtgcaggcgttctgcatccaggttcagcccgagcatgaccgccagtacgtgcatttcatggtgcgctggtggttgcccgccgtccgcgaggcctggctggagcggctcgacgagatcggcggccccgagctgcgcgaccgcatccggcccctgttcatgccggagcatgagcgcatgctcggccacttccatggacggcgcgatccgcggctggccgacgacacgctgcgcagcgagggcgacttgcaggcgtatgcccaggccctggccgtctggtgcgccgagcagggcatgtactttcagaatgcacccaggaacatggcggaactgggaaagatcatgctgtcggtcgaccatttgagcaacgtgctcaaggctggcgagagcggagtgcatggctcgttctacctgccccagcagatgggcctgctggtgctggcgttgacctgcaagacgccgctgcgcgaagtgtggctggagaccttgcgccaccgccagcgcgtgacccagcatgtgcagtggaagcacgtcacgggcggtgacggcaacgcgctgttcgagggcatcctggccagcctgaccgaacggccgcctgcccttggaggctgacgcggcgccgtcggtcagtttccgggcgcgatgaagtccggatggcgcgcgcagatttccggcagcgaactcagcgtgcccgagaggtgttcgcgcagcgccttctgcgccgcggcgccgtcgcgctttgcaatggcgcgcacgatggcgcggtggtcacgcaggatcgcctcggtcttgcccgccgtgggcaggtgcaggcgccgcaggcggtccacatggcccgagacgcggctcaccaggtcccagaggctcggcacattcgcggcttcgtacatgaggtgatgaaacttgcggtcggcaccgacgaactcgccgtactgccgcgccgctgccagcgtggcctgcagagcgacctgtgcttcgagctgcgcgaccaacccgggcggggcctcctcggccagctggtgcacgatctccagctcgatggagcggcgcaggaagtgcgcctgccgtgccgcatcgatgtcgatgcggctgaccagggtggcgtgctggggaaacacgtccaccaggccttcttcgctgaggcgcagcaaggcctcgcgcaccggcgtctggctcacgccgaagcggtcggccagctcttgccgcaccagcaccgtgccgggcacaaggtcgagggagaggatggcatcgcgcagtttttcgagcacttgcggtgcggccaggcgggtgcggtcgagtcggatccgggggagggcagtcattcgctggaattctcgctttgacgcagtgatatattagtgttttaatgtagtggatctcacacgaagactcgtttttttcagccctcgatgccacgctcctacgacaccctgcgcagtgcccgctggttcgcgcccgacgactttcgctccttcggccaccgctcgcgggtgatgcagatgggctacgcgccaaccgactgggtgggcaagcccatcatcgccatcgtgaacacgtggagcgacgccaaccagtgccattcgcacttcaagcagcgcgtcgacgacgtcaagcgcggcatctttcaggcgggcggttttccgctcgagctgccggccatctcgctgtccgaaagcatggtcaagccgacgaccatgctctaccgcaacttcctggccatggaaaccgaggagctgctgcgcagccacccggttgacggcgcggtgctgatgggcggctgcgacaagaccacgccgggcctcacgatgggcgcgctgagcatgggcctgccgttcatctacctgccggccgggccgatgctgcgcggcaactggcgggggaaggtgctgggctcgggctccgacgccttcaagtactgggaccaacgccgcgccggccagctcagcgaccaggcctggcaggagatggaggctggcattgcgcgcagccatggcacctgcatgaccatgggcaccgcggccaccatgatgggcattgccgaggccgtgggcttcacgctgccgggcgcctcgagcattcccgcggccgatgccaaccacgtgcgcatgagcgccgaatgcggccgccgcatcgtcgagatggtgtgggaagacctgacgcccgccaagatgctcacgcgcgacaacttcgagaacggcatcgcctgcgcgatggcgatgggatgcagcaccaacgccatcgtgcacctgatcgccatgtcgcgccgcgccggccatccggtcacgctggacgacttcgatgccgcgagccgctgcgtgccggtggtcgccaacatccggccgagcggcgacacctacctaatggaagacttcttctatgcgggcggcctgcccgcgatgctggagcgcatccgcggccacctgaagaccgaggcgcgcacggtcaacggccgcaccatcgggcagaacatcgagggcgccgaagtcttcaacgacgacgtcatccgcccgcttgccaaccccatctatgccgaaggcgcgctggccgtgctgcgcggcaacctcgcacccgacggcgtggtgatcaagcccagcgcctgcgcgccgcacctcttgcagcacaccgggcgcgcgctggtgttcgacgactaccccagcctgaaaagggcggtggacgatcccgaactcgacgtgaccggcgacgacatcctggtgctgcgcaacgccggcccgcgcggtgccggcatgcccgagtggggcatgctgccgatcccgaccaagctcttgaagcagggcgtgaaggacatgctgcgcctgtcggatgcgcgcatgagcggcaccagctacggcggctgcctgctgcactgctcgcccgagtcggccgtgggtggcccgctggcactggtccaaacgggtgaccgcatccgcgtcgacgtgccagagcggctcattcacctggaggtgagcgacgaggaggtggcgcgccgcaaggccgcatggacgccgcccgcaccgcgctacgagcgcggctacggctggatgttcggccgccacatcctgcaggccaacgagggctgcgacttcgactttcttgaaaccaccttcggccggcccgtgccggagccggacatcttttgaagacctgaacggagacccatgtgaatccccagacccgcgagaagctgatgaaagtcagcaccgccaccctgtgcacggcgctgttcaagcgcggcctgcgcaaccagttcatccagaacgtgcatccgctcaatccggcgctgcccaacatggtcggcgaggccttcacgctgcgctacatgcccgcgcgcgaagacctgaacccgatcaccgtgttcaacgactgcaaccatccgcagcgccaggcggtggagcaatgccccgtgggcgcggtgctgctgatggacagccgcaaggacgcgcgcgccgcatcggccggcggcattctggtgagccggctcatgaaacgcggcgtggccggcgtggtcaccgacggcggctttcgcgacagccccgacatcgcgaagctcggcttccccgcataccaccagcgcccgagcgcgccgaccaacctgaccttgcaccaggccatcgacatcaacgtgcccatcggctgcggcgacgtggccgtgtggcccggcgacgcggtggtgggcgatgccgagggcgtcatcgtgattccggcggacatcgccgacgagatcgcggccgaggccaccgagatgaccgtgttcgaagacttcgtgcaggagaaggtgctcgaaggccgctccatcctcggcctctatccgccgaccgaagagcaaagccgcaccgagttcgcggcctggcggcaggcccacggccgctgacggcctgccttttcaacaaacatcgacaaagagagacaagaccatgcccttcatccagcgcgccgcgcgactgctgttcgccgcatccgcttccgtcttcgcacttgcacctgccgcagcgctggcgcaggccgaatggcccgccgccaagaccatcacctacgtcgtgcccttcacggctggcggctcgaccgacatcgtcggccgcatcctggccaacaagctgcaggagagccttcaccagtcggtggtggtggacaacaagccagggcaggccggcggcatcggcgcggcctacgtggccaaggccgcgcccgacggctacacactctttggcggcaccatcagcacgcacgccatcaacgccagcctctacaagaagctgccctacgacccgatgaaggacttcgagcccgtgtcgctggtcgggcggctgcccaatgtgctgatcgtcaacagccagctcggcgtgaactcggtggccgagctgatcacgctcctgaagaaggacgaatccaaacgcaccttcgcgtcgtcaggcgccggcacctcgacgcatctggcgggcgaaatgttcgccgacatgatcggcgtgaagctcacgcatgtgccgtacaagggcacaccgcccgccatgaccgatgtcgcgtcgggcctcgtgcccttcatgttcgaccaggtgaccgccgcgctgcctctcgtcaagagcggcaagctcaagctcctggccgtgaccaccggcaagcgcattgcgctggtgcccgagttgccgaccatgatcgaatccggcgtgcccggtttcgagatgtcgtcatggcaggccgtctatgcgcccaagggcacgcccaagcccatcatccagcgcctgaatgccgagatcgtgaaagcgctcaagcagcccgacgtgcaggccaagctctccggccaactggcgatggacatcgccgccagcacgcccgaagaactgcgcgaccacatggcccgcgaaattccgcgctgggccgagctggtgaagaagtcgggcgcgaccgcggattgacgaggcgttgccggtcttctagccgttcaatacgagagacccgtgcggatactgcgcgcacatgaattcgacgaacgcccgaaccttcggcgcgggaagccgcctcgatgtatgcaggacccagagcgcgggctccccgcccgacaccatgccccactgaaccagctctccgcgcgtcaactggttccacgcgatggactgcggtatcagcgcggcgccggcgcccgcgaccgcggcgtcgcgaatcatcaggaacgatgacagtctgagcctggggatcggctccacgacaaggcgtccgtcatcgagcgtccaattgccggcttgaaagttggttgaaacgatgccgggaaccgggctgaccttgcccttgcctggctttggcacgggcacggagggcgccgccacgaccaccagccggtccttggcgaagcaccggcccaccaggctgctgtcggggcttggattgatccggatcgcggcgtcgaactgctcctcgacgaggtcgaccaggcgatcgtccgccaccacctcgcacgtgacctcggggtaagccgcgcagaacccggcgcagatgcgtcccatcgccagctgggagaacagcaccggcgaggcgacacgcaaacgcccgcgcggaaccgacaagccctcgcgcgcggaagtcatggcttcggccacctcgtgcatgggcccttcggtgcgatccatcagcatctggccggcttccgtgagcttgagtccgcgggcgctgcgctcgatgagtcgcacgccgagttgctcttccaggtccgcgatgcgccgggacagggtcgccttcgatctcccgctcgcgcggcttgcctttccgaggccgccattcgctgcgaccagtgcgaagtcgttcaatgcgttcaggtccatgtgttccgtatttgaaacgaggtgtcttcatttttgcatcttcgttttatcgatgcaacgaactatcttctcctcatcgcaacttcgatgagaggaaattgaaatgaccaccacgcaacgcgccgtgctgatccgcgcctatggcggtgtggccgccgccgagttcgccgagatcgcgaagcccgcagccggaccgggccaggtcctggtccgcgttcgggccgcgggtgtgaacggcatcgactggaaagtccgtgaaggcttcgtccgggaggctttcccgcttcaactgcccgccgtgctggggatcgagcttgcgggtgtcgtcgaggcggtcggccccgacgcctcgcgctttcgcgtgggcgatcgcgtcatgggtccgcttggcggcctgggtgcctatgccgatttcgtggcagtcgacgaagcgaacctggtgcgcacgccgcaaggcctcaacgacgttcatgcggccggcatccccgtggcagccgtggccgcctggcaaagcttgcaccacgcgggtccgatcgtcgcgggtcagcgaatcttgatccacggtgcagcgggagggctgggcggctatgccgtgcagtacgccaagcgggcgggcgccgaagtcttcgccacggcgtcgaccgcgcacgtcgagtacgtgcgcagcctgggcgcgaaccacgtcatcgactaccagaccgaacgcttcgaatcggtcgcgcgggacatcgacctggtgctcgactacgtgggcggcgaagtgctcgatcgctcgtggcaggtgctgacggaagacggtgcgatcgtcggcacatcctcgcccgacatccttgcccgcacgccccccggccgccgcggactgtggttcatgaacaagccggacgcagccctcctggaacggctggcggcggagatcgcccaaggcacgctgatctccaagctcggcgaagtcgtgggcttcgacgacatccccgcggccatcgaacgcaatcgcaccgaccctcgcatcggcaaggtcgtcgcggacttctcgcgctgatcgacccctgccccttttttacccatctaaccctggagattttccatgagcattctcgtcacaggtgccaccggcaccattggttccctcgtcgtccaaggcctggccactgccggcgccgaagtcagcgccttcgttcgcacacctggaaagcaacgcttcccggcgggtgtcaaggaggtcgtcggcgacctgaccgacgtgccctcattgcgcgcggcactctcatcggtgcgcacgctgttcctgctgaacgccgtcacgcccgacgaagtgacccaagccctcgtcgcgctgaacctggcccgcgaggctggcatcgagcgcatcgtctatctgtcggtcatccatgcggacaagttcaccgacgtgccgcacttcaccggcaagcacacggtcgagcgaatgatcgagagccagggcattcccgcgaccattcttcggccggcctacttcatgcagaacgagcgcatggtccagcaggtgatccagggctatggcgtctatccgatgccaatcggctccacgggcgtcgcgatgatcgatgcgcgagacatcgcggatgtcgccgtcgccgaactgctgcgccgcgaccgcgcgcccgcgccgtcgccgcgcgtgacgctggagctggtcgggcccgagcggttgaccggagcgtcggtggccaggatctggagcgccgcgctcggtcgcgaagtggcttacggcggggacgacgtggcggccttcgaaacacagatggccgcgcaggggccatcctggctggcctacgacatgcgcctgatgatggccgggatccagaagttcggcatgcacggtgcggagggagcagcggaccgcctgcaggccatgctcgggcgtccgcttcgcaagtacggcgacttcgtcaaggaggccgttgccgcgtcgtaaggctgcgcggggctccatcgccgtcgccatccgcgtcgacagggcgggcgtccgaggagccctgtttgcgctcgctgggtgcggcggaggtcatcgagccttgtatgcggccagaaacgcatcagaagccacctgatcggccagggccctcaacttcgcagccgagtcgggacccagcacggcctccacccggtcgttggctgcagcccagtgcgcaacagcttttgacagcctggctttgccaagcggagtgagaacgccgtgcttggtccgccggtccttggcgtcctggcgcagctcgaccatgccgtcgcgcaccagcggccgcagcgcatgggtcagggccgagagctggatcgcgagccggctcgccaggtcctgcagtgcgggtccttgctgatcaggcccggtgagcttgtgtatttctgccatgagcccgagctgcgtggccttgaggtccagcggcgccagcgcttcgtcgtacagctggccgagccgccgggccgcgaggcgcagtgcggtgttcgtgcagacccgtccgccaaggatgtcctgctcatgttcggcgggcttgttgcgggtgcgctttgcatcgacaggcgtggtggtgattcccatgatcagaaaatggttgagtgccgaaccatcggcaagcggccgcggatcaaacctacatttgagccctcaacttatttggttgagcactcaattttattcgaaggccatcaatgacaactcccaactccaacaaagtcgctcttgtcaccggggcttcctccggcatcggcgccgtctatgcggatcgcctcgcggcacgtggatacgacctgattctggtcgcccggcgcgccgaccgcctggaagcgctttgcgcgcaggtttcgaaggcgcacggtatcaaagccgaagcgatcgtggccgatctgacccaggacgaggacctggcgcggatcgagacgatcctgtccaccaacgccgacgtgcgcgtgctggtgaacaacgccggcattgcgcggctcggaccggtggcccagcgatccgcgggcgatgcgctgtcccagatcgccctcaacatcacggcgttgacgcgcctgagccaagcggtcgtgccggccttcatcgcgcgaaaagagggggtgatcatcaacatcgcttccgtgctggccatccattcgctccccatcagcgcggtctacagcggcaccaaggccttcgtgctgcagtacagccggggtctgcaggaagagctggcgggaaccggcgtgaaggtccaactggtcctgccggcatcgacagccaccgagatctgggatctgtcgggcgtgccgttggcggccctcaaccaagacgccttgatgacgaccgagcacatggtcgatgcggcgcttgcgggatgggaccagggcgaaacggtcacgtggccgtccgtcgccgatgcagcgctgtgggggaagtacgaggccgcccgctccgaactgtttgccgcgacccaggttggaaagccggctccgcgctacctcgtgggctgagcccaccaggccaccccacgccgtcctttatttctcttttcccgctccatttttttcaggacagcccatgcttttcgacgccttctccctgcgcgccattccgctcaagaaccgtgccgtgatgtcgccgctcacccgcagccgcgcggtcgacaacaacacgcccaacagcctgatggccacctactacgcccagcgcgcgagcgccggcctcatcatcacggaaggcacctcgccgtcgcccaacggcctcggctacgcccgcatccccgggctgttcaatgacgcgcaggtacaaggctggaagctggtgaccgacgcagtgcatgccaagggcggcaagatcgtggtgcagctcatgcacaccggccgcgtgagccaccaggccaacctgccggctggcgccgaagtagtgagctcttcagcggaaacttgcccgggccagatgtggacggacacccaaggcagccagccgcacacgccgccgcgcgccatgaccgaggccgacatccagaccgcggtcggtgagtacgcaacggccgcgcgccttgccatcgaagccggcttcgacggcatcgaactgcacgcggccaacggctacctgctcgagcaattcctgaacgccaacgtcaaccgccgcaccgatggctacggcggcacggccgaagggcgcaaccggctggtgctcgaagtcgcccgtgcggccgtgaaggagatcggcgccgagcgcgtaggcatccgcctgtcgccgcatggcgtgttcaacggtgccggcgccttcgaaggcgtggacgaacagtacctcgcgctggtgaaggagctctccgcgctcggcctcatgtacgttcacgtgctggaccattcggcaatcggggccccaccggtcccggcaaagctgaaggtcgatctgagggcggcgttcgacggccccttcatcctcgccggcggtctcgacaaagccagtgcacaactggcgctgcgcgaaggccgtgcggacctggcggccatgggcagggctttcctcgccaaccccgacctcgtcgaccgcatgcgccaggacgcgccgttgaacgcgcctgcgccggacacgttctacacgcccggcgccaagggctacacggactacccggcgcttgccgcttaagcgccaaagggcgctgcaacgaggctcagaggccgccttggcagaggtacttggtgtgcatgtagtcgtcgagaccgtgcaccgagccttcgcggccgtagcctgattccttcacgccgccgaagggcgccgcctcggcggccagggcgccttcgttgatgccgacgatgcccgattcgagcgcgtcggccacgcgccagatgcggcgcacgtcggtcgaatagaagtaggcggccaggccgaagggcgtgtcgttggcggcggcgatgacctcggcctcggtgtcgaagcgcgtgaccggaaccaccggtccgaaggtctcttcgcagctgcattccatggtcgcgtcggcgttcaccagcaccgtcggtgcgtagtagttggggccgtcgcagcgtgcggagcgcagccgttcgccgcccaccacgacgcgtgcgcctcgggccacggcatcgcgcacgtggcgttcgatcttgtcgaccgcgcgcgcgttgatcatgggcccgatctgcgaacccgggtcggtggccgggccaacctggagcgcccccacgcgcgcggccagcttgtcgacgaaggcgtcgtgcaccttggcctgcacgaacacgcggttcgggcacacgcaggtctggccgccgttgcggaacttggcggccatcaggccttcgacggcggcatcgatgtccgcatcctcgaacacgatgaagggcgcgttgccgcccagctcgagcgacatcttcttgagcgtgtcggccgaggcgcgcgccaggtgcttgccgaccggcgtggagccggtgaagctgatcttgcgcacccgcgcgtcggccagccacacgtcgaccacctcgggtgtgcgctcgcgcgaggcggtcacgatgttgagcacaccggccggcacgccggcttcctgggccagcttcacgagcgcgagcgaagtcagcggcgtgtcttcggccggcttgcagaccacggtgcagcccgcggccagcgcgggcgcgatcttgcgggcgatcatcgcggccggaaagttccacggcgtgatcgcggcgaccacgccgaccggctccttcaccgccagcatgcggcggcccgtgacgggcgcgggaatcacgtcgccgttggcgcgcgtggcttcttcgccgaaccattcgacgtagctcgccgcataggccacttcgccgcggccctcggccagcggcttgccctgctcgcgcgagatgaggcggcccaggtcttcctggtgcgccagcatgaggtcgttccagcgcttgagaatctgcgcgcgctgcttggccggcaccgcgcgccaggcggggaaggcggcatgagcggcagcgaccgcggcacgcgcatcggcggccgtgccgtcgggcacgctggcaaagacgccatcggtggcggggtcggtcacgtcgaggcgtcggccatcgctggcttcgcgccattcggcgccgatgagttggcggccgggcagcaggtcctggcgttcaagtgtcagagtcatggtcgattcagggttcgttgagttcggtaaggaggtcccttccaggaacaccgcggaaccggctttgccgggccgctggtgttgcccccggagaggggggtggcgtagcgacacgaagtgcgcgaagcctgggggtgagtcaattcgcaacgcgttcggcaatcgcgatgcccacgtcggtggtcgaagccgtgccgcccaggtcgcgcgtgcgcggtccgtcgcgcagcaccgcctcgatggcgccaaggatggcgtcgtgcgcagcgcggccggcgccctgtccctgcgtaagaaagtccagcatcagcgcgcccgaccagatcatggcgatcgggttggcgatgttctggccgtagatgtcgggcgccgagccgtgcacgggctcgaacagcgacggaaacttgcggtcggggttgaggttggccgacggcgcgaggccgatggttccggtggtggctgggcccaggtcggagaggatgtcgccgaacaggttgctcgccaccaccacgtcgaagcgcgtaggctgcagcacgaagcgcgccgacaggatgtcgatgtgctgcttgtcgaccttcacctcggggtagtcgcggccgatggcgtcggcgcggccgtcccaccacggcatgctgattgcgatgccgttgctcttggtggccaccgtgaggtgcttgcgcgcgcggctgtcggcaagttcgtaggcgtagcgcagcacgcggtcggtgccgtggcgcgagaagaccgattcctggatcacgatctcgcgctcggtgccttcgtacatcacgccgccgagcgaggtgtattcgccctcggtgttctcgcgcaccaccagatagtcgatgtcgccgggcttgcggcccgccagcgggcagggcacgccttcgaacaggcgcaccgggcgcaggttgatgtactggtcgaactcgcggcggaacttgagcagcgaaccccagagcgaaacgtggtcgggcacggtctcgggccagccgaccgcgccgaagtagagcgcgtcgacgccgcgcagctgctccttccagtcgtccggcatcatctggccgtgctcggcgtagtagtcgcagctggcccagtcgatggtgcggcagtcgagctcgaagccgaagcgctcggccgcggccagcaccacgcgcagtccctcgggcatcacttccttgccgatgccgtcgccggcaatcagcgcaatccggaatgtgggggtcatatccgagcctctctggttgatggggcaactgcttttgccgatgcggccgccgtgcggtccatgtcgtccagccagccgcggcgcagctcgggcacggagcgcgcgagcagttcgtagtaggggtgatgcgggccgcgtgcgtagtcggcgcgtgccacctgcgagagcttgcgcccatgctgcatcacgacgatctcgtcgcacaccgagcgcacggtgtgcaggtcgtggctgatgaagaggtaggacacgccgagctcgcgccgcagctcggccatgaggtcgagcacggccgcggccacgacggtgtcgagcgcggaggtcacctcgtcgcacaggatcaggtcgggctcggccgccagcgcacgcgccaggttgacgcgctgcttctgcccgcccgagagcccacccggcaagcggtcggccaccgtgcgcggcagcttcaccaggtcgagcagctcgtagatgcgctgcttgagcggctcgccgcgcaagcccttgtagaactgcagcggccgcgccaggatgcgccagatcgtctgcgacggattcaatgccgtgtcggccatctggaacacgatctggatgcggcgcagttcgtcggggctgcgctgctgcagcgtgggcttgagttcgtggccgtcgaacatcacgctgccgtggcagggcttgagcaggcccgcaacggcccgcgccagcgtggtcttgccggagcccgattcgccgatcacgccgatggcctgaccgcgatagagcttcaggttgatgtcctcgaggatcagcttggccggttggcccttggcgtccacggcgccgtagccgcacgaaagctcgttcacgtgaagcagcagcgcggaatcgcccgaggtctggcccgaggcgcgcaccgcgggccgcgccgccgccagcaggcacttggtgtagtcgtccaccggggccgagagaatctgctcggtggcgttcagctcgctcatcttgccgttgcgaagcaccaggatgtggtcggccatctgcgccaccacggccaggtcgtggctcacatacacggcagtggcgcggcgctcgcgcaccacgcggcggaaggcgcgcagcacttcgatctgcgtggtcacgtcgagcgcggtggtcggctcgtcgagaatcacgaggtcggggtcgccgatcagcgccatcgcggccatgagccgctgcagctggccgccggagacctggtgcggatagcgtgcaccgatggtttccggatcgggcagagccagttcgcggaacagctgcaccgccttcgcctcggcctcggcccgcttgcacaggccgtggatgacggtcggctcgaccacctggtccatgatcgtgcgcgagggattgaaggaggcggccgcgctctgcgcgatgtaggagaccgtgcggccgcgcagcgagcgctgccgcgtcgcatcgagtgccagcacgtcggtgtcgccgatctgcacccggccggccgagatgcggcagccgctgcgcgcatagcccatcagcgccagcgcggtggtggtcttgccggaaccggattcgccgatcagcgccagcacttcgccgggctggacggagaagctcaggttgtcgaccagcgtgctgctgccggccacgatgctcaaaccctggacagtgagtggtgcgcccatcaacgtactcctcgttcgcgcgcggcacggccgggcaggttgtcgataacgagattgaccgcaatggtcaggctcgcgatggcgagtgccggtacgatcaccgaggcgccgcccatggccagcgcgccgatgttctcgcgcaccagggagccccagtcggcggccggcggctggatgccgaggcccaggaagctcaggctcgccagcagcagcacgacgtagacgaagcgcagccccaggtcggccagcatcgggcccaggatgttgggcaggatctcgcgcagcatgatgtagagcgtgccctcgccgcgcgtgcgcgccacggtcacgtagtcgagtgcgttgatgttgacggccagcgagcgcgccatgcggtaggcgcccggcacgtagatgatgcccgccgtgaccaccagcatcggcaccgaggagccgaagcccgccaccatgatgagcgcgaacatcttgctcgggattgccgtgagcgtgtccaggccgcggctgagcaccgcgtcgatccagcggccgctggcagcggccagcagcgccagcgtgatgccggttccgctggccagcagcgtggcgaacagcgcgacgccgatcgtgtagcgcgccccctcgatgacgagcgccagcatgtcgcggccgaggtagtcggtgcccagccagtgcttcgcgctgatcggcgcgaagacgttcgaggtgcccatgcccgccgcgctgtgcgagagcagccaggggccgagcagcgcggcgagcagccagaacagcagcaccgcgaggccgagcaggccggttgcgccgaagccgctgagccagcgcagcgagccgccccggcgctgttgcggcactggcgcgagggaagccgcggcgctcgcgaccgttggagaggtggacgtttccatggagcttccttcagcggtgccgcagccgcgggttggcgaggatgccgcagatgtcggccgtcgtcaccaggatcaggtaggcgcagcaaaagatcatggcgcaggtctgcaccagtggcatgtcgcgctgcgagacgccgtcgaccatcagcttggcgatgccggggtagttgaagatggtctcgacgatgatcacgccgccgagcaggtacgacaggctcagcgccacggcgttggcaatcggccccaccgcattgggcagcgcatgcgccagcaccatgcgcatcggcgaggcgcccttgagccgcaccatctcgatgtagggcgcctcgagctggtcgatcaccgcagcacgcgtcatgcgcatcatctgcgccacgatcacgcagcacagcaccagcaccggcatcgcgaaggcgcgcagcagctggcccaacgactcgatgtcgttgacgaaggagagcgccggcagccagcgcagctggaccgcgaacaccagcaccgccagcgtcgcgaccaggaactccggcaccgacaccacgcccaccgccgtcgtcgaggcggcgcggtcgaaccatgagccacgccagaccgccgaggcgatgccgagcgtcagtgcaatcggcaccgagaacagggcagtgacggccgccagcagcagcgagttgggcaggcggctggcgaccagttcggacaccggcatctgcgtggtcgcggagcggccgaggtcgcccctcaccatgccgaacagccacttcgcgtagcgttcgggcgccggcacgtccaggcccatctgggcgcgcaacgcggccaccgcctcgggcgtggcgtcctggccgagctgctcctgcgcggcatcgccgggcagcaccgcggtgatcgagaacacgatcaccgacaccgccagcagcgacagaagcgccagcgcgatgcgctgggcgagaagcttcaggatgacatggttcatttcggtgctcccaggggcgggatgagcggctgcgggcgtgtcatgcctccagccatacgttctcggcaaagttgtagcccatgaggccgcccagcgggatgggcgacaggcccttgagcttggacgtgtggccgtccaggctcgaaaggaacagcggaatgccgatgccggcgtcctgatggatcatggtctgcatgtcggcgtacatctgcttgcgcttggccaggtcggtctcggcgcgcgaggccagcagcagctggtcgaacttgtcgctcttccagcgcgactcgttccacgccgcgcccgactggaagaactgcgtcagcagcacgtcggcgctcgggcgcggattgacgttgccgaagcccacggggctgttgagccagtggttcgaccagtagccgtcggccggcatgcgcttgatgtcgatctccagcccggcgcgctgcgccgtctgctgcaggagcagcgccatctccaccgagtagagcgccgcgggcgaagccaccatcggcaccttgccggtgatgccggacttctgcaggtggaacttcgccttgtccaggtcgaaggggcgctgcggcaggccggagaagtagaagcggttggtcgggtcgatgggctggtcgttggcgaccaccgcgtagtcgagcgcaatggtcttcttcatctgctcgcggtcgaacaggtgcttcatgccgagcacgaagtccgggttggcgccggggcccacgtccttgcgcatgatgaggtcggagtactggccggactgggtgaccaggatgccgaagccgggcgtgcccttcacgcgttccaccgagcgcgggttgaccgagccgaccaggtccatgccgcccgacagcagcgcgttgacgcgcgcgctctcgtcgccgatgcccacgaactcgatctcgtcgaggtagggcttgccgggcttccagtaggcgtcgttgcgcaccatcagcgagcgcacgccgggcttgaactccttgagcttgaaggggccggtgccgatgccggcgttgaagtcggtggtgccttccttgacgatgtggaagtggaaggtgcccaggatcaccggcaggtcggcgttcggcgaggtgagcacgaaggtgacctcgttggcgccggtggccttggcgctctcgatctgctcggcgagcaccttggctttggacgcgacagccgggtccttgtggcgcatgaccgagaacacgacgtcggccggcgcgagcgccttgccgtcgtggaaggtcacgcccttgcgcagcgtgaagacccaggtcttggcatccttcgtggtgaaggattcggccagcgcgggctgcggcgtgaggctggcgtccagcgaggtcaggctgttgtagatcatgttgcagcgcgagtagtcggtctggttcgactgcttggccggatcgagcgtgtcggtggcggcggccgtggcgcctgccacccggatgcgcccgcccttccttggcgtctgggcatgggcggacaccgccatgccggcgaggctgccggccagggtggcctgcatgccaccggccatcagcatcgcgaggatgtcgcgccgcgaggcgccgcgtttcagcgaatccatcacgcgaaggctttcgctgggaccgacgaggttttcgaacctcttgttgctggtgtcgctcatggtggggtactcctgtggggccgatgactgagggttgaagaacaaacaaacacggaacgaaaagcgggtggactcgcgcggcgctcaggccagcttgtccttgagcgagtagtaaagcccgaccgccggcaggaaccagggcggtccgaagtggccggggatggcgggccagtcgcggccctgccaggggttggcgcgggcgtcgccgttcatcacggcggccatgcgctcgcccatgtgaaccgacatctgcgtgccgtggccgctgtagcccatggcgtagtagagaccgttgcgttcgcctgcgtgcggcaggcggtcttgcgtcatgtcgaccagtccgccccagcaatagtccagccgcacggcgccgagttgcggaaaagtctcggccagcccggcgcgcaggatctcgccgctcgcggcatcggcctgcgggctggacaccgagaagcgcgcacggccgccgaacaccagccggtggtcgggcgtgaggcgaaagtagtgatggatgttcgcgaccgtggtgtaggtgcgccgggccgcgagcagcgcctgcgcgcgctccgcgccaagcggctcggtcacgacgatgaaactgccgatgggcacgatgcgccggcgcagccagccgaagctgccgtagccgccgtggcgcgtggcgcccgtggccagcagcacctgctgcgccgtgacggtgccgccagcggtgtgcagccggtgcgcatggctttggcccaggcgttcgatgcggttcaccgcggtgccggtgtggatctgcgcgccgtggcgctgcgcggccgcggccaggccctgggcgaagcggcccatgtgcatctggccgctgcgcttgtagagcagcccgccgtgaaagcgctcgctctgcacctcgccgtgcacctgcgccgcatcgaggatctcgacgtcggtgtccacgccatcggccaccaggcgctgcgcgctgcgttcgagcgcggccatctggttggcgcgcgtggcgagcttgagcttgccgtggcgcatgaagtcgcagtcgatggcctcgtcgcgcaccagccgcgccacggtgtccaccgcgtcgtcgtaagcgcggtaccaggcgcgggccttctcgatgccgaccttggccgccacgtcggcatagtccacggccagcccgttgttgacgtggccgccgttgcggcccgacgcctcggccgccacccgggtgccggcctccagcaccgcgacgctggcgccgcgcttggccagcgccagcgccgccgacaggccggtgaagccgccgcccacgatcgcgacgtcgacctgcgccggcagtgcatgcactgccggcgagaaggccggcgcggaatcggtccagtaggagtcgagcttcatggcgtggggcgtttcaatctggaaggatcagaggccgacgacgccgggcaggccgccgatgtcctggatctcggtgtagcggtaggccgggttgcccgggccatggccgcgattgacgaacaccttgttgacgatgccgatgtcgtccgccgacatcaggtcgtagcgcaggctcgacgacacgtgcagcacgtcttcagggttgcagccgagcgagtcgagcatgtactcgaaagcctgcaggcgcggcttgtaggcttgtgcctgctgcgcggtgtagacgcggtggaacggtgcgccgagcatggccacgttcttctggatctggtcgtccgaggcgttcgacaaaatcaccagcgggatttccttggccaccttggcaaggcctgccgccacgtcgtcgtgcgggctccaggtgggcaccgcgtcatagatcttctgcgcgtccaggtcgaagtactggatcttccatttcttgcagaggcgccgcaccgcgttcttcagcaccacctcgtagggcttccagtcgcccagcacctcgtcgaagcgataggcagtgaagtcggcatggaactcggccatgcgctcggccggaacgcggtcggcgaaaaggtcggcggccatctccttcatgcggaaccgggtgagggtgccgtagcagtcgaaggtcacgtatttgggacgaaaagtcatggtctctgatcctgtgtaaaaggtggcaaatgcgacaaactcactacgaacacattacgaagcgattgcagcacgctcccgctcgaggtatgtagggaaaaacggtgcttgccgaatcgaagctgcggtttgcgggggtggcgacggcatgccgtgcggtgtgcccagcgggtgtgcggccatgcacctcggtgcgtcgccgcaaagtcgatgagcacgcttttgaagcgcagattggcttcgaacgcccagcacccccggcccttgccgaaggaagttgaacggatcgaaggcttgcatggcgatagggtgcaggaagtggccgtcgatcctaggcaggatggctcagcatttgtgtgcgtatgcgcccgccccgccgcagcgaattgcgaaaccggggcgcgcggcaaccgaagcttgcaagttgcgaaagaaggtgaattcggtctggtgcggcaccgcaatgtcgtccaagatggatgcgccattccttcgcaacagagagttttccccatgcccgaacccacttcgaacgcacccgccatggatggcgtggtgctcagaccgatgacggccgccgaccttccacatgcgcatgcgctgtccgccgaactgcgctggccgcaccgccccgcggactgggaacaggtgttcgcgcatgccgacggcattgcggtcgagcgcgacggcgagatcgtcgccaccggcctgcgatggctctggggcaagagccacgccaccatcggcctggtgatcgtctcgcccgcctgccagggccgccgcatcgggcaccggctcatgagtgcgctgcttgaagggctcgagaaccgcacggtgctgctgcatgccacttcggaagggcggggactgtacgaacggctcggctttgtgcgcaccggcgagatgcggcagcaccagggcattgcgctgccggcaccgctgattgcgctgcagcccggttggcgcttgcggcccgcgggcctcaacgagttgcccgcgttgcaggcgctggacgcagcggcgcgaggcatgccgcgcgatgcactggtcgccgagctgctgcaaaacgccgatgcctgcgtggtgctcgaccacgacaacgagccgaagggcttcgccatgctgcggcgcttcggccgcggccatgtcatcggcccggtggtcgcgcccgacgccgagggcgcgaaggcgttgatcgcgcatcttgcgggcctgaatgccggcaacttcacgcgcatcgacatcgacttcgacagcggtctggccgaatggctcgagagcatcggcctcttgcgggtggatgcgccgacgacgatggtgcgcggcgcaccgcttgccgttcctgcgcaagggccttcgctgttcgcgatcgtcacgcaggcgctgggctgaggcgcacgatggaaacctccacctttctctacaagtccgaccccgtgcgcggccgccagtgggccgaggtgttcggccgccaccggcccgacatcgactttcgcatctggcccgacatcggcgatccggcacgggtgcgctttctggcggcctgggtgccgccggacgacctggccgcgcgctttccgaatctcgacgtgctgttttcctcgggcgccggtgtcgaccagttcgactttgcggcgctgccgcccgaattgcccgtggtgcgcatggtcgagcccggcatcgtgcgcggcatggtcgagtatgtgacgcacgcggtgctcggcctgcatcgcgacatgccgcagtaccggcgccagcagcaggaagggcagtggaagccgctgcccgtgcggcccgctggcgagcggcgcgtgggcgtgctggggctgggctcgctcggccaggcggtgctggcgcagctggtctcgctggggttcgactgcgcgggatggagccgctcacggcatgaagtcgatggcgtgcagtgccatgccggggccgacgagctgcccgcctttcttgcgcgcaccgacatcctcgtgtgcctgctgccgctcaccgattcgacgcgcggctttctcgatgcgaagctgttctcgatgctgccccagggcgcggggctggtgcacgtgggccgcgggccgcacctggtggagcgcgactttctggacgcgctcgccagcgggcagatcggcgatgcggtgctcgacgtgaccgaccccgaaccgctgccgcccacgcatgccttctggcgccatccgcgcatcgaactcacgccgcacatcgcgagcatgacgcagccgctgagcgccgccgaagccttgctcgacaacctgcgccgctttgaagctggcgagccgatggtcgggcttgtggatcgcacgcggggctattgaattgccctggcttcgacggggcagggcggccccgagggtatgatcccggccctccgacccccgccatgtttctgcgccgcgtactgacccgactcctgctgctggccgtgttcttcaacacggtcatcggcatgcctgcgcacgaagccgtgcatctcaaggcagaggccgcggtggccgcactgtcggtcccgcaggcgaacgacgaggccgatgccgcggagcatggccaggaagccgatggcgcgtgcgcgtggtgcctggcctacgcgcatctgggcacggcgctgagctcgccaccggccgcgcatgcgcccccggtgcatgcgggtcttccacggccgcaagccctgctggccttcgtccccagcccgggccattggcctttcgcctcgcgcgacccgcctcgccccgtcgcctgaacgccgccgttgcggcggcaacttcgctcgccctgcagtcccgtcgcccggcgtgaagtcacgcgccacgggcggcgcgcgtccggcccttgccgggctcgccgctgcgcccctcgtcttgccttgcccagtctccctccatgatttccatccaacgctcggggcccagcgcgccccttcctctggccttcgcggtcgcggccctcttcgccggccctgcggccgcccagtcttccggtgccggccctgaggccgcccagttgtccacgatcgaagtggtcggccgcaccgagtcgggcgcctatcacgccgacgaggccgccggcgccaagaccgatttgccgctgcgcgagctgccccagtcggtacgcgtcgtcttgcgccaggccatcgacgacctgggcgcgaccaggctcgacgacgtgctcgactacgtgggcggcgtctcgcgccagaacaatttcggcggcctctgggacaacttcgccatccggggcctgcccggcaacgagaacaccggcatggccacgctgctgaacggcttttcctcgaaccgcggcttcaatgccccgcgtgatctggcgggcgtcgaacgcatcgaattcctcaagggaacggcggccgctctctacggcagcagcgagcccggcggaacgctcaacatcgtgtccaagcggccgctctggaaagcggcccattccgtcgaaggctatctgggcagccacggcctcaagcgcggtgcgttcgacagcaccgggccgatcggcgagaacttcgcttaccggctcaacgtcgccgcggaagaccgcgacagcttccgcgaccatgtgagcgcccggcgagaagtgatcgcgccggctttcacgtggaagctcggccgcgacaccgtgctggagtattcgggggaattcttgcggcacgccaccccgctggaccgcggcgtggtcgcggtcggcaaccgcctgggcgccatcccgcgcagccgcttcctcggcgagcccgcggatggcgacgtgacggtggagaaccagacccaccaattcatcctgtcgcacgaatggaactccgcgtggcgcagtcggctgggcctgtcctaccgcaagacttcgctgaacgggttctcgaccgaagcgagcgcgctgggcgccaacaacgcgaccctcgcgcgccagcggcgcttccgcgacttcgactcgaacgacattgcattgcaggccgagctgcagggcaccatccggactggtgccatcgagcacgaactgctgttcggcctggagagcttccgcttcagcatggactcgatcatgctgcgcgccaacccgacggccgcacggccctatgcgatcgacatctacaaccccgtctacggccagttccaaccggttccgggccgcaacaccgacaccctcgaacaccagcgcaacaccgcgttctacatgcaggacgcaatcaagctcgcgcccgcatggcgcctggttgccggcgtgcgcgtggacagctaccgccagtcgctcgagaaccgcatcgccggcaccacggcgcgccaggatccgtcatcgacctcgccgcgcattggcctgagctggctgccgacgccgcaatggaccttctatgcgaacgccggccgatcctttcgccccaacgtcggttcagacgttgccgcccagggcttcgaaccggaaaccggacgcgcgctcgaacttggcaccaagtgggaaagcgcggaccggcgcatgggcgcgaccgccgcggtgttcgacatccgcaagcgcaacgtgctcacgtccgacccggtcaacaccggctactcggccgccgccggcgagatccgcagccgcggcttcgaattcgattttgccggccagctcaccacgaactggcgcctcaacgccagcctggtgctcaacgacgtggagatcacgaaggacaacacgctggcaatcggcggccgcctgctgaacgttccgagggtcaatggcagcgtgctcgcggtctacgagaacgcattcgccaacgggcagcgctacggcatcggcgggggcgtcacgcatgtgggcaagcgcctgggccaggcccgtacgcaggccgacgccaacgccgcaacgccgtctttcgagctgccgagctacaccaccgccaagctggtcgcctactggcgcatcaaccccgcgctgcgcgtgacgctggacatcgacaacctgttcgattccacctactacgccagctcctacagccgcctctgggtcacgccgggtacggcgcgcaccatcaccgtcggcttgcaagccaagttctgagcgcgggcgaatgcaatcatgaacttgaccaaccttccatcggcgcgcgccacggccgcgcctcatccggccctcgaagccgccggcgtggtcgccggctacggcgggcacaccatcctgaacgggctggacctcagggtcgaagccggtgaaatctacgcgctgctgggcgccaacggcgccggcaagaccaccacgctgagcctgttcctgggcttcgtgcagcccgcgcgtggccgcgtgcgcgtgaacggcgccgaccctgtggccgacccgacgtccgcacggcgccagctcgcatacatccccgagaacgtggcgctctacgagcacctgagcgcgcgcgagaacgtggcctacctgctcgatctcgcgggccagcccgccaatgcgcaggcgatcgacgaggccctcgcatccgccggcctggacgctgcggcgcacgggcggcgcgtttcggggttttccaaaggcatgcgccagaaagtgtcgatcgcgctggcgctggcacgcaaggtgccggcgctgctgctcgacgagcccacctccggcctcgacccgctggccacggccgagttcaacagcctgctgggactgctgcgtgcgcaaggggtggccatcctcatggtcacgcacgacctgctcagcgccgccgacgtcgccgatcgcatcggcttcatcgacggcggacggctggtcgaggaagtcgcagcgtcgggcccggagcgcttcgacgtgcgggcattgcaccggcgctacgctggccaggaggcgcaccgatgagcgcggtactgcgcatcgcgcgcgaggaatggcgcctgctgcggcgcgaccgcgtcgccgtgctcgggttgacgctgctgctgctgttgtcggccgtggctgcattcacggcctgggaacagcgccgcaccacggacgccgagcgcgcgcgccaccaggcgcgggtggatcacgagttcgagggccagcccgaccggcacccgcaccgcatggtgcactacggtcacttcgtgttccggccgctgaatccgctggcggctttcgattccggagtggatgcctatacgggccacacgctcttcctcgaaggccatcggcagaacagcgccaatttcggcgacgtacggcagtcgtcgctgctgctgcgcttcggccagctcacgccggcattcgtgctgcaggtgctggcaccattgctgctcgtcttcgtgggccatgcggtcctggcacgcgagcgcgagtcgggcacgctgcgcatcctgctggcccagggtgttcgagcgcgagaaatcgtggcgggcaagctgctggccctgagcggcgtggccgcgttggtgctgctgccggcgctgctggcgctgacctggatcggcgtcgcaacgccggcacccgccagcctggcagtggcgctggcggcgggctacgggttgtggttgctgatctgggccgtcggcatcgtcggcctgtcggcatggttcgagcgcgggcgcgatgcgctggtggcattgctggcggtctgggcggtcagtgtcgtgctcgtgccgcgcctggcgcccgaactcgtggcctcgacgctggcgctgcccatgcgcttggagaccgacattgcggtggcgcgcgacctgggggcactcggcgacagccacgaccccgacgacccttacttcgccggcttcaggaagcaggtgctcgcgcagtacggcgtctcgaaagtggaagaccttcccgtcaactacaagggcctgctcggcatggagggcgagcggctgaccagtgcgctcttcgagcgctatgccaacgccagcttcgagcgacaggacgcacagttgcgccgggtcgaccgctttgcactgctgagcccggtgatcgcgctgcgccgcctctcgatggcggccgcaggcaccgatctgcagaactaccgccgcttcgtcgagcaggccgagcaccatcgctatcgactggtgcaggaactcaaccggctgcaggccgaaaagctcagctacgctggcgaccgttccagccgcgacagccgcatcagccaggcgcactggcacgattttgccgactttcactatgaagccgcgcggcccagcgaggccctgcgccacgcggcaccggccgcgggtgtgctgctgctttggctggccgcgctcaccggcctgttggcgccggccacgcgccgcctggggaggatcgcgcgatgagctggctcgcccacgaatggcgcctgctggtgcggtcacgactggtcctggttgcgctggcattgctgttgatattgacgaccctggctgtgctgtcgggcacgcgcgagcttgcgcgccagcagcagacgattgcgcgcctggccgagctgcagcagcacgatctggcggcgcaagcgcgcaagtacacccacggcggtgaagccggctccgccgcctactacaccttccacggcacctgggatgcaccgtctcccacagccttcctcgcgctcgggctgcgcgatgccgcaccctacgtgttgcgcgtgcgcgcactggcgctgcaggctcaactgcacgaaggcgagagtttcaatcccgagctggcagtggccggacgcttcgacttcgctttcgtgctggtgtacctggcgccgctgtttctgatcgccttgttgtacgacctggtgtcgggcgagcggcgctcgggccggctgggtacgctcctggccatgccgggtgccggccgccgcctgtggcttcgccgtgccggcctgcgcgcggcgctggttttcgcttgcctcgtgctgccggtgctggccggtggcctctgcagcggcaccccgatgacggccctgaccaccgcgctgctggtcacggcggcctacctcgcggtctggagcgggctggtgctgatcgtggcaacgcgaagcggaagttctgccgccaacgcaacggcactcatgggctgctgggcggtgctgaccctcgtcctgcccaccatcgccaacgccgtgcttgcgcgcgcggtgcctgtccaccagggcgtggagctgatgctggcgcagcgccaggccgtgcacggcgcgtgggacctgccgccagaggccacgatggagaagttcttccgcacgcaccccgaatggaagcacaccgcaccactgccttcgggctttcactggaagtggtactacgcctttcagcagctcggcgatgagagcgtggcgccgcaggtggcggcttaccgcgaaggcttgctcgcgcgccagcgctggaccgcacgcctgggttggctgctgccgggcgtcggcgcgcaagccgcgctgcatcgccaagccgataccgatctgcaggcgcaactcgcttaccaggatcgcatcgcagatttccacgcgcggttgcgggcctactactacccgtacttgttcaacgaagtgcgcttcggtttcggcgacttcgccgcccagccgcgtttcagcgcgcaggccaggtccgcggagacacctgtgggtcagttgctggggctcgggctgatgggcatattggccctggttctgggtgtggccgccaccggtcgggtgcggccggtgtgaaggcgcccatgaccaatgcatgacggcacgatctgctgtagcgactcgcacaaccgcagtctgctttgtgcaaggccctcaatgcagcacccgtgcgaggggcatgcggcctaagcttttggacatccaaaggcccgacttcagccccccatgacgcaccccaccgcattgccgcacctcgccacgctcgacgccatcgaccgtgctcacctcattcatcccgtctcgccctggcgcacgcacgaggagcgcggccccaccgtgctggcctcggcccgcggtgcatggctgaccgacgcgaacgggcatgaactgctcgacgccttcgcgggcctctggtgcgtgaacgtgggctacggccaggagagcgtggtgcaagccgcggccgagcagatgcggcggctgccgtacgccaccggctactttcatttcagcagcgagccggccatccgcctcgcggaaaagctggtgcagatcacgcccgcatcgctgacccgcgtctacatgacgcttggcggctcggaggcgatcgacgccgccgtgcgcttcatcgtgcagtactacaacgcgatcggcaaaccgtcgaagaagcagttcatcgcgctggagcgcggctaccacggctcctcgtcgaccggcgcgggcctcacggcgctgcccgtgttccatcgaggcttcgacctgccgctgcccacgcagcactacattccgtcgcccaacccgtaccgccacgcgcaaggcgccgatccgcaggcgctgatcgccgcatcggtggcctcgctgcgcgccaaggtggccgagctcggcgccgacaacgtggccgctttcttctgcgagccgatccagggttcgggcggcgtcatcgtaccgcccaagggctggctcaaggccatgcgcgatgcggcgcgcgagctcgacatcctcttcgtggtggacgaagtcatcaccggcttcggccgcaccggccccatgttcgcctgcgacgccgaaggcgtggagcccgacctgatgaccatggccaagggcctgacttcgggctacgtgccgatgggtgcgacgatgatctcggagaaggtctatgccggcattgccgacggcgcgcccgcgggcgtctcggtcggccacggcgcgacctattcggcgcacccggtgagcgccgcggtcgcgctcgaggtgctgcgcctgtacgaagaaagcggcgtgctcgccaacggccagcgcgtcgcagcccatttcggggccgggctcgatgccctgcgcgcgcacccgctggtgggcgattcgcgccaccgcggcctgctgggcgcgctggagctggtgagcgacaagcagagcaagcgcggcttcgatgcggcgctcggcctgtcggaccggatctttgccgcgggctaccgcaacgggctggtgttccgcgccttcggcgacaacatcctcggctttgcgccggcgctcactttcaccgaggacgagttcgcccagatgttcgcgcgcctgaagaaaaccctcgacgaagtgctcgacgccgccgacgtgcgcgcggcgctggccgcctgagcgggaaagcattgccccgggaccccgccggcgaagcagaatcgggctctctccgttactcaggaccgccatgtctgaagccttcaagatcgaccgactcgacctgcgtatcctggcgcagctgcagcagaacgggcgcatgaccaacgtcgacctcgcggatgcggtcggcctctcgcccagcccctgcctcatccgcgtgaagcggctcgagcaggccggctacatcgccggctacggcgcgcacctgcggctcgagaagctcggcgacacgctcaccgtgttcaccgaggtcacgctgcaagaccatcaccgcgaagacttcgtgcgcttcgaggccgcgatccgggatgtggacgaggtgctcgaatgccacctggtgagcggcggttacgactacctgctgcgcttcttgacgcgcggcgtgaaccactaccaggaagtgatcgaggaactgctcgaacgcaacatcggcatcgcgaagtacttcagctacatcgtcatcaagtcgccgttcatcaagacgcattgcccgatcgaacggctgtttccccacccgcgctgacccggctcttgcgatcctctgcacttcaggagaaacgccatggccaccaccaacaccgtccgcctgcaccgcgtgctgcgcgccccgccggagcgggtctatcgtgccttcgtcgaacccggcgcgttcgagcgctggctgccgcccttcggattcaccggcaaagtccacagcatggagcccgtggtcggcggtgcctggcgcatgtccttcaccgcctttggcagcggccacagccactcgttcggcgggaagtacctggaactcgtccccggccagcgcattgcctacgatgcggcgttcgacgaccccaacctgccgggcaccatgaagaccaccgtgacgctgaccgcggtgtcctgcggcaccgacatgtccgtcgtgcaggaaggcattcccgacgtgattcctgcggagatgtgctatctgggctggcaggagtcgcttgtggcgctggcgcagttggtcgagccgaatattccaggctgagttagccgcaggggtcactcctgcccctagccggccggcggcaatctcctggcggcccgcacaagcagtcgtgcgcccacgcacaagtgcggcggcggtgcagctcctacgctcacatggtgcggtgcagcaggctggcgtggtgccagccggctcgcgccgtctccacaggagcctcggacatgcaaaaccttcccttcccggccggactctgcgtccggcttcgcgcattcgtattggcccgcatgcgcggtgcgtccgtcgcggcgatcggcctgtcggccctcgctttggcagccgcgccggcccacgccgaggccgtgaaggccccggccgagtgctcgacgctgcaagccaaatacccgcagttcaagggcaagaccctggtcaacgcgatcaacccgcacacgcccggctacgaaaccatcgatcccaaggacccgagcaagtacatcggcttcgacatcgacctgggcgaaaccatcggcggctgcctgggcttcacgctgacctacaagcccgtgacctttgcggcgctgctgaccacgctgcaggccggccaggccgacatcgtgatctccgacatctacgccaccgaagagcgcgccaaggcggccgacttcatcacctattcgaaggtgttcgacggcgtgctggtggccaagggcaacccgaagaagatcaccggcatcaacgcctcgctatgcggcaccgtcgccgccgagaacacgggctatgtcgaggtgccgctgatccaggcgctcggcccgcagtgcaaggccgtgggcaaggccgagcccgagatccagctctacgacaacaaccagaattgcatccaggccatcctcgccggccgcgccgacacctacatcaacgacgtcaacacggtcgacagtgccgtcaaggcctacccggacaagctggagaaggcggccgcggtgacgatcccctattcggtcggcattgcggtgcccaagggcaagaccgacttccgcgatgcggtgatggccgcgctggtgatcttgcagaaggccgggatccacaccgcgctgctcaagaaaaacggcctgccggtcgagaacctcgaggcgccgcggctgctcgtggcgaagtgacatgaggtcttcacgcgcactccgttcgctgccccccaaggaggctgccagtaccttcggaacggccgggcggtactgacatggagctcttcctccattacctctccatgccctacctgatccagggcatcgtcttcacgcttgcagccaccggcatcggattggcgggcggggtggtggtggggctgttgctggcggcaatgcagctcagccgcttcaagccgctggccgcgtttgcccggggctatgcggtgattttccgcggcacgccgctggcgctgcagatgatcttcttctacaacgcgctgccgcacgtgggcattgtgctgcccggactcctggccgccggcttggcgctggcattcaacgaggccacgttcatcgccgagatgttccgctcgggcgtcgtcggcgtcgaacgcggccaggtggtggccggccaggccctgggcatgacgccgcgcgtgctgatgcgccgcatcatcgcgccgcaggccttgcgctcgatgatccccgcgatgggcaacgaggcggtgagcacgctcaagaactcctcgctcgcctcggtgatcgcggtgcaggaactcacgctgcgcagctcgcagctggcctcgtcgaccttcgatttcttctcggtcttcttcgcttccggcctgatctacctgctgctgaccggcgcaatcagcctggtgcagctggcgctcgaagcgcgcttcgacctggaccgcccgcaggcggtgcgcggactggcgcggtggctgccgcagcgtgccgcggcgcccgccgcgagcccttcgccttcggaagaagcagccgccgcggaggtgccgccggccgatcgcgaagatgcggcgccagccgcacggtcggtcccgacggcgcccgcgatcgaacgcgcagcccgggctacgcggctggccgacgcgcccgtggccttgcgcatcaacggcgtgtccaaggcctatggttcgcaggccgtgctcagggatctgagcctcacggtacaggccggcgaagtggttgcgctgctgggtccgagcggctcgggcaagagcacgctcctgcgctgcatcaaccatctcgaaagctgggacgccggacaggttcatgtcggcggccaccgtctcggctttcgccccgatggccagctcatgaacccgagcgacctggcgcgcgagcgcgggcgactgggcgtgggcatgctgttccagcagttcaacctgttcgcccacctgacggcgcgcgagaacgtggccggcccgctgcgctgggtgcacggttggacggcggaggacgccgatcggcgagcacatgaactgctggcgcgggtggggctggcccaccgcgtcgaagcgctgccgcgccacctgtccggcggccagcagcagcgcgtggccatcgcccgcgcgctggcgccggggcccagcgtgctgctgctggacgagcccacgtcggcgctcgatcccgaactggtcaacgaggtgctggaggtgattcgccgccttgccgtcgaggaaggattgacgatggtcatctccacccaccagctgcggtttgcggccgaggtggccgaccgcgtggtgtttctttccggtggccgcatcgtcgagagcggtccggcgctcgaggtgctgcagcgcccccggcaccgcgaaaccgcccgattcctcagtgtgatgtcggccgacgtgctgccggccgcttcgacacccatgcccgcctgagcctgcccccaagaaccccatgaagcatcacatcctccccgtctctccccaaaccatccactggggctatttcagcaaggcggtcgcgccgtcgctcgtcgtgaagtccggcgatcgcgtgacgatcgagaccctgacccatcatgccaacgacgaccacgagcgcatgatcgccggcgacccgggcgccgagtcggtgttcgcgtggacgcgcgagcacaaggccgtgccgcgccgcggcgccggtcccgtggaggggcctttcaagctcggcgagggcgagggcgtgggcgtgcacctgctgaccggcccggtcgtcatcgaaggcgcggagccgggcgacgtgctggaggtgcgcatcctcgacgtgcgcccccggcccagctgcaaccattgctatgcgggccgctgcttcggctcgaacgtggccgcgtcctggggcttccattttcgcgacctgatcgaagagcccaaaccgcgcgaagtggtgacgatcttcgagctcgacacctcgggcgagcccttcgcgcgtgccgtctacaactacgtgtggacgccgcagaccgaccccgacggcgtggtgcacaacatgatcgactatcccggcgtgcgcgtcgaccatgcgctggtgcacaagcgcgaagacatcctgcgcaacgtcaaggtgccggcccgcctgcacttcggcaccatgggccttgcgccgtcggaatccgacttcgtgagttccattccgcccagctacaccggcgggaacattgatgactggcgggttggcaagggcgcgcgcatgtactacccggtggccgtgcccggcgccttcttctcggtgggcgacccgcacgccgcgcagggcgacagcgagcttggcggcaccgcgatcgagacctcgctgacgggcgacttcgagttcatcctgcacaagcagtccgggttgggcggcaccttgctcgagggcctcgaccacccgctgctggaaaccgaagagctgtggtcggtctacggcttcacctaccccaactacctggctgccctcgggccggacgcgcagacggtgattgccggcaagtcgtcgctcgacccggccatgcgagatgcctttcgcaagctgcgccgattcctgatgaccgtgcaccgcctcagtgaagacgaggcgatcgcgttgctgtcggtggcggccgacttcggcgtgacgcaggtggttgatgccaactggggcgtccatggttcgatccgcaagagcatcttcacgaaccgctgactgcggggttcggcttaccgcgaacgcgaccgacatgaatacttaggtcggccacaggcgatcgcgcttttcgcaaggatttcagagcgctcgccgccaagtatcgcgaggatccgaagtaggagcccaccggcggaatgcggccaacagtagaccttcgacaccgcctccagttcaacgcaaccgcatgtccgcaggaacgcagttgtccaggcccaaacctcgcccatgctgagcgtcaagccggtgcgtaggcacctgtgcctcctggccaggccgtgagcacttcatatcccccgggcgtcacagcgaccatgtgttcccactgcgcggacagagacctgtccttggttacgacggtccacccgtcgggcagttgcctggtttcgcgcttgccggcgttgagcatcggttcgatggtgaagaccatccccggctccaactcgaggccttccccgcgccgcccgtagtgcagcacttgcggttcatcgtgatagacctgcccgatgccgtgaccgcagtattcgtgcaccacgctgaaatgctcccgctgggcgaccgtctggatggcatggccaacatcgcccagcgtcgcaccaggcttgacctgccggatgccggccagcatggcttcgtatgtcgtctccaccaagcgccgcgccagcacgctgggggctccgacgaagtacatgcgactggtgtcaccgaaccagccatccttgatgaccgcgacatcgatgttgatgatgtcgcccttcttcagaatcttggtcagagaggggatgccgtggcaaaccacctgattgacggaggtgaggatggtcttcggatacccctgataccctacgttggcaggaatggcgccctggacattcacgatgtggtcgtggcagatgcggtcgagtgcctccgtgctcacccccggcacgacgtagggctcgaccatacctagaacctctgcggcaaggacggcggcccgccgcgccatctcgagttcctcggtggacctgatgggaacaccgtgagccatcagtgcttccccgtcgaggatgcgcgaggcttgccaggatcgggcgtgacagccacggtgatgtccaggccccccgcgagttcggctcgtatcaacagttggcagatttcccggtggtctaactccgggtgcatttcggtcagcatgccgacgcgcatccagtgctctgcctgcgcattgatggacctgctgagcgcgttcccagccacgcgcaggttctcgtgcatcaggtccgaaatttttacgatacccatcagtgatctctatatgaaatgtatatgaagtatatacgtttcgtatggcgcagcgctaacagtcggtcccaggtaggcatcagtacagcaaattgcatctacccatcaaagcgtccattccaggccgtacacgatgcctcgccggcgggccctcgtagcaatcattgttggtcgagggccgacgtctgcatggccggagacggggcggcaagcacaaggtgctcaaccgttcatgacccgcgcaaagatggcctgatgcagccatcgcggtgtcgccgataccatcgccaccgcggccttgttgttgaagcctggaacgacgctcatgcggccggtgtgcagcgcatgaatccccgcccgcaccaccggctccggcttcatcatcagcagcttgagtccccaagtaatcttctgcttggcggcctgcgcaaagccagtgtcggacatgccggggcacagcgaggtaacagtcacgccgtcgcgcttgaactcacggtgcaacgcatcgccgaggcgcagcacgtaggccttggctgcgccatagacggccatgttttccaccccaaagtgagccagcatgctggcgacgagcaatatctttccgtggccccgctcgcgcatgtcctcgccgaagagtcgcgtcatgaccgtcaggctcgcaatgtccagctgcaacatgtctaaggcgctttgcatgggcgtgtcgaggaaggggccttgcaagccgtggcctgcgttgttgatcaggatctcaaccgcgatcgcgcgctcgcgaagactggcttgcaactcgtggacggcggccatgtccgagagattgacctgctgcacgatgacttggaccttgtactcctgttgcagcgctgcagccaaggcttgcagccggtcgagccgacgtgcgatcagaatgagcgggtggcccctggccgcgtattgcctggcgaattcttcgccaaaaccactggacgctccagtgatgagaacccaggagtcgacggtggtcgccatgatgttttgcctttgttgaagtcgaggtgaagcagaaggtggccggcacccttgctttcaggcaagattggagaccgatggtctgtaatttagcagaccaacggtcttttagcaaatggaacgtgatcaccgcatgaattcccccagctcatacgtacgcgctcgatccgccgagcagaaggaagagcggcgccgccacctgctggccacagctcgagaaatgctgcgccaggacccggccgccctcgatttggggatcaacgagctagcgcgccaggcgcagatgaccaagtcgaacgtctaccggtatttcgagagcagcgaggccgtcttgatggacttgctcgtcgaagaatatgcaagctggcatgccgagctgagcacggcgctggcgcgcggcggcaaggccggcgctagcgtcgaacacattgctcgcgtcttcgcctcgacgattgctacccggccgttgctttgccggctgaccagcatcctgccgtccatccttgagcgcaaggtgtcgttcgaacgcatggtcgacttcaaaggcaacctgctggcggttcggcaacgggcagcgcaagacttccatgcccgcgtgcccggcatgccggtgcaagccttcgaactggtggtgaagcatgcggtgccgctgatcatcgggctctggccgctcagcaaccccgcagagatggccgcgcaagtggtcgagctgcccgagttggagagtctgcgatacgactttgagcaggacctcgaacatgccctgctgatattgatgcgggggttggccacagcgtagaaggcgttctcgagcctggaatgtcactgttcgttacttcgctggactgctacgccggtgactggtcttcgaaaacaccatgcataccggactgccgcaactcgtgacttcgccggtcgccgaaaggattccatcgaactgtgagacttccaaggcgacgatgctgtcgctatcttcattgagcacgaacagcgtttgcccgttcggagcgagcgcgagatacctcggagttcgcccctgtgacggaaacgcaccgatgaatgcaaggtggcccgattcaccgtcgatactgaagaccgcaatgctgtcgaagccacggttcgacgcgtacaggagcctgtcgttcgcatccacagcaatctccgacgccctgctgtttcccgtgaacgtgtcgggcaacgttgagagaacttgtcgcgggaccaggccacccctcttgggatcgaacagatacgttgtgaccgtggagtcaagttcgttgacgacgtatgcaaatggcttggtgccgtggaacgcgacatgccgcggcccagaacccgcgcgcgcgtcgacatatggcgtttcggtcggctctagccgaccattccggaatcgaaaaatgaagacgcgatcgaggcctttgtctggtattacaacgaagtgcccgctcggatcgaaagggttgaagtgtggctttgagaacggctgctctacgcggtgtggtcccggctcacccggcagtgctatcaactggttgaaatgcccaatcgagccgtcctcgagaattgggagcactgcggccgtcccgctcaggtgattggatacgaccatgaagcggccttttgggtcgagcgcgagatgcaccgggttcttgccgccacacgtccgccggttgaggagttccagttccccgtccgcaatgttcacccgaaacgatgagacctcatgctcatcgccgtggacggcgtagagcacatcgcccgcccggttcagcgccaggaaagatggattgaccaagtcgccgagaacttggatcaactccagcctccgctggtgactgtccaggcgataaacgctgatcccctcgccgcgcgcgttgcgcatccgggtagtgcgcgatccaacgtatgcgtacatgcttgaacgagcgacttactgcgaagatgaaagctggattgccgcagcccagcgcgcggccatggccggcgagttgaagcaggtcgtgtcttgggtcgccgtgcttacggcgcgctcaagcaactggatgtctgcctcgtgctggcgagccacatgtggatcctcgaagaagatgaccttgctacaggtgcgattgagtacgagttctgcgatctgcgcatcgccacccatcggaccgctccggtagcgtgtgacccaagggcgatccgttggccaaccgcgggccaaggccatgtcgttgagtagcccgcccgtcgttccggtgcccacgcgggacgaaaaccgtgagagcagatcaaaatgggcggcggcgaactccaccatctgatccttgaacgcatcgtgcgcgatcagcgcgacggtttgacttgcgacagaactcccgaagccggcgtcaccggttcctgcatgggccaactcgaccgcgatccactccgcggcgccggcagccgtcgatacgaacggcttgccgtgaatcacgcactgacgcttcagcgcctgggtctccgggtagagggacgatggatccacagggtccaccaggtagatcacgccatcgagttcgctctccgtggtcagtcctccggcgatgcacgacgccaggcgcatcacgccgccttcgacaccggagggaaggcgaaccagcgacccgctattgctgagcacgccctcgcgggcgagcgcgtcgtaggtgccgcctactgcgtgcagcttgagattcagcgaacgaatactgtcttcgtaggccttcgcccagcgaagcagtgcgccatcgacactttgtcgatgcagccgattggcgacgagaccgaatcgcatgcgttttacctatgcgcgccgaacgtggtgcgcagcgagtcaatatgtgcgtcaggcaacgccgacgctttctgaccgctcagcatccacagacgcgcggtctcttcgagttcctcaagcgttgccatggcccccgcaggtgtctcgtgccagacgtttgggccgagtcgctctagcatcactgcccgaataggggtcgaatcagaaagccgccgccgctttcatccgaaagccgcacgctgatgttgcccaccatcacatgggcatagccgcgttcgaaaaggctgcggccgacacggcagatttcttcacgtgccgcgctgtcgttcatcggccgttccaatcttggtgatgcgcgccgtgttcaggtgctggcgcaggtactgggaggcttccatccgttcgcccttgacgagcagatcgatcagcacgagatgctcttcgcattggcgatgcagcctgttgcggtccaagcgggtgccgtactcgactacgcgccgcatctggttcaaggtgcgaagcgaatcgagcaagaagcgattgtttgcgccggcgatcacggtctcgtgaaagtgcacgcccgcacggaacagctcggccggcgtgcagcgctcgataccgccggccagcaattcgatctgctcgcgacggcatttttccagctctgccaggtcgacctcgtagcccggctcgagaatggccgccggttcgatgatcatgcggtagcggtaactttcgcggtgcgactccacgctgctgagcagcggccggaagatccagccgcggcccggtttgcggtcgatcatgctttcccgagccatgcggttcaggatgcgctggacctgcaggcgcgggaggccatagcgctccatcaggtcgttctcggcaacttcatccggcagctcgccatggatgcggtcgctggcgatgcgcatgtacagcacctcttcggacgccgggttgggcgcgaactccagctcgcccaactcggacggcatcttcgcgacctgaaagccacggttcggctcggatgtcaccgccccgacgccctgcaggtactgcagcgccttgcgcaccggggagcgcgacacatccagttcctcgcacagcgcctgctcggtcagccggtggccgaccgggtagccctcgcggcggatcatttcgatgattctgcgggcgagcgtgggcgtgagcgcgctgacgttggctggcgaggcaggcttggacatgggcggagcaaggtgtgggagatgctgcactttacgactcaatcgagcagacgaaacgcgctggtgaagaagtcggtcgccccgaagttgcccgatttcaaggcgatgtgcatcgtgcccccctttgcatgcctggatgccgcttggcaccacggcacgccgggagcgatctgtgggccgatgcgcatgctgcggatgtccagcgcctgcacgcaagcgccggagctctcgccgcctgccacgaccagctggccgacgccgcgctcggccaggccgcgggcaatcgtcgccagggcgtgctccacaatctcgcccgcgcgcgcgctccccagctgcgcctgtaccgccttgacggtttcgggcctggctgtggcgtacaccagcaccgggcctgccgcgatccgcgagctcgcccaatcgagcgcacgcgccgccacatccacgccttcggcaagctggagcggatcgatggcgaagccttcgcccccgttggcgaggaaatgcgcgacctgggcgttcgtcgccgtcgagcagctgcccgagacaatggctcgcaggccgagcggcggcggcaggcgcgcggcatcggctgccggcgtgatgccgaagttttgcggcagcccgatcgcaacgccggagcctgccgtcagcagcggcaggttcgcagatgcgcggcccatggcgatcagatcggcgttgctgatcgcatcgacgatggccatcgccacgccttcgctgcgcaacgctgcgatgcgctggacgatggcggcttcgccctgcgccaccgtcccttgctcgatcaggccgacccggcgttgcgtttgcgactgcagaacgcgcacgaggttggcgtcgtgcatgggcgtcagcggatgattgcgcatgccggattcgtgcagcagctcgtcgcccacgaagagatagcccttgaacaccgtgcgcccggtctccgggaacgccggacaggcgatcgtgaagtccgccccgagcgcatccatcagtgcatccgtcaccggaccgatgttgccttcggccgtggagtcgaatgtcgagcagtacttgaagtagaactgccggcaaccttcaccctggagccaccgaagggcttgcagggactgctgcacggcctcggcggcggcgatcgtgcgcgacttcagcgcgaccacgaccgcatccgcctcgtcatccagcggcccggagggcacgccgatggtctgcaccacgcgcatgccggcgcgcaccaggttgttggccaggtcggtggcgcccgtgaagtcgtcggcaatgcagcccaggacagcttggctcatggtggatcaggcagcggccacggtcttgaccacggcctcggtgaaggccttgcaaccgatggtgccgccgatgtccttggtgcgcgtgtcggggttctccagcaccttgtcgacggcgcggaccatggcgtcgcccgcgtcctgcaaggccttgttcttctgcttgtcaccaacccagcggaccatcatcgccaccgacaggatcatcgacgtggggttggccaggtccttgccggcgatgctcggcgccgagccatgctgggcctgggcgcagcacaggtcgtcgctggccatgaccgatcccgccagacccaggctgccggacagttcgctggccaggtccgagatgatgtcgccgtagaagttggtcgccaccagcacgtcgaaacgctccggctccttgaccaagtgcgcggtcgaggcatcgaccagcagatcgtccagcgcaacctctggaaagtccttggccacgtggcgcacggcttcgaggaacagaccgtcggtcatgtggaagctgttggccttgtggatcgcggtgaccttcttgcgccgcgtcatcgccagctcgaaggcgcggcgcgcgatgcgctcgctgcaatgccgcgtgatcttgcggaccgacaaggccatgtccgggctgggcatcatttcgccccagcccctggacatgttgcgatcggggtagaagccttcggtcgcctctcgcatgatgacaaggtccatgctgcggccttcccgcatgttggactgcaggtagggccgcgtgcgggccggacgcacgttcgcgtacaggtccaggccgacgcgaaagcccgcggacacattgcgcccgcctttttccggcgcggggtaatcggcatgcgactgtgtgcccaggatgatgccgtcataggtcctggccttgtccagcacctcctggcgcaaggttgtgccgtgtttctccaggctcgtgaacccggcgtcttcgtagtcgtagctgatgttgaggtcgaagcgcttgtcagcggctttcagcacttctaccgatgcggcaacgatttccgggccaatgccgtcacacggcagaacgatgaacttcatggggtactccagtggtgggtagggtggtgtgaatcaacgatgcgaatcggccggggccgtcgcgcagagacttttcagaaggcgaacagcgctgtcggggctggtaagaactggcttgccaagcgcggcgtggaccaatcgctgggcccgcgccatcgagaactggccgagcatgacgacgtcgcaagctcgaaggtcggccgcgcgcgaagcaatcaggcggtcgtgcgcagcgccgtctccttgtgcaaggaggctcatcgcgtccggaacgaaggccgtcttcagttcgatggcgacgtctttcgcacgcgcgagttcgagcagttcatcggacatcgaggcaacggacggttcgaaggttgacaggagaccgatgcgcaagacaccggcagccggtgtcgtcgagatcgcttccagaaacatcgcgtagttgggcttgtgcgtgggaactgccactgacgcggccgccgcgtcgatcgcgggcccgaacgccgagcaggtgaaaaggatggcgcgtgcccccgctcgctcgctgtattgcgcgagttgtacgaaacgcgtgaccagcgcctcgcccaattcgcccgcagccgacaggtcggcagacagcgcgtcatccagcaagttggcacgttgcgcctgcggccaaagccgttcaaaggcctcgtggactggtgccatcgccaagggcgtggcgtgtattagggagatccttggtgcaagtatctttgtcatggctcatcttgtaggggttgatcctgattgtactatgtatatgatggatacaatcatggaaaacccgccgcgacatgttcgccgcatctttttgccaaccctggagactccatgaatcgcttgccgaaccgccgccaacccctcattgcggccctgtcccttgccacgctcgccaccctcccgacctttgccgctgcacagggcgcagccgactacccgacgaagacgatcaccttcgtcgtcccgtatgcagcgggcggaagctcggacatccgctcacgccagatcgcgcaaaaactctcggtgtacttcggcaagccggtcatcgtggagaaccgcccgggcgcgggcggaaacatcggtacggactacattgccaaggccgcgccggatggccacgtgatcggcctgggcaactttgcgccactggccgtcaacaaggtactgttcgcaaaactcccgtttgatccggcgacagatctggtgccggtggcaatgatcgagcgtgggccgctggttatgtccgtcagcctcaactcgcccatgaatacggcccaggatgtggtcgcacgcgccaaggccaagcccggcaccatgaccttcgcctccggcggcatcggcggcgcccatcacctagcgggagaagcctttcagcaaagcgcgaaggtcgacatggtgcatgtggcctacaagggcggcgcgcccgcgaccaacgacctgattgccggcaatgtcgacatcatgttcgagtggatctatgcggtgatgccgtacctcaagggcgactcggccaagctgcgcccgctcgccatcacgagcgacaagcgctcgccgctgctgccggacgtgccgaccttcaacgagattggcatccagggcatggagatgtccaactggtttggcgtcgtggcgcccaagggcacgccaccggcggtcatcgcgaagctgaaccaggccatcaacaaggccatccgcgagcctgacgtcgccgagaagatcacctcgcaaggcaatgaagtcgccggtggcacgccggaggcttttgcgaccttcatccgctccgagtcggaccgctggtcgaagctggtgaagtcgcacaacatcaagcccgagtaagcgtcctccgtttcacgagacgcctcgaacatgaagggctcattcctccagcggccgcttgccggtcttgctatcgcctgcgcgttggcagcccccgcgttgtcacctgctcagacgccagcggcatatccttccagacccgtacgcctcgtggtgccctttgccgcgggcggacccaacgacgtcatggcgcgtgtgctcgcgcaacgcctgacggcggacacgggccagccttttgtcgtggacaacaaggcaggggcgggcggtgtgatcggcacggatgccgtggccaaggcggcacctgacggatacacgctcggcttcgtcagtgcgccgttcacgatgtcaccggcgttgcaggccaagatgccttacgacacccagaaggacttggcggcagtgaccaaggtcgccgaatcgccgatgctgatgatggtcccgtccgactcgcgcttcaagagcgcggccgagctcatcgagttcgccagcaagagtcctggcaagctcaactacggctccggcggcaacggcagcacaccccacttgaccaccgagctgctcgcatcagtgacgggcgcaaagttcacccacgtgccctacaagggtggcggcgaatcgatcaaggccctgatgggcggcgaggtggatctgctgatcgatagcattaccagcaccacggcgcccctggcgtccggccgcgtcaaggccctggccatcagcggagccaatcgatcgccgcgaatgccgagcatcccgacctttgaggaggctggcatcaagaacttctcgatgacgcattgggtcggcgttgtagcacccgccaagacaccacctgccgtgctgtcgtcgctgcatgcgcagattgcaaaggctctgcgcgcgccgcaagtgattcagaagtacgccgaactgggcgccacgccagcgccgacgtcggcgcaggatttccagaagttcgtgaatgacgaaacaaagaagtggcagcaggtcgtcaagagcgccaacatccacacgcaatagagatgccgcccttcgagttgccgccgcttgcgacggacacgcatgtgcacctgttcgaccccgccagcttcccctacgccgaggggcgtcgatacacaccaccgcctgcgaccgtcgccgaccttcagcaagtgcatcgcgcgttgggggtggagcgcgtcgtccttgtccagccgagcgtgtacggcttcgacaatgcctgcctgctggatggacttgcgcaacttggcgatcgcgcacgcggcgtggctgtgatcaaggaaggcaccacgcgagatgaacttctgcgcctctaccaagtcggtgtcagaggcgttcgcttgaatgtcgaggttgcagggagaacagacgcgcccgcttgcgccgaagcgctgcgcacaatggacgacgcccttgaggacattcccatgctggtgcagctctatgcccctgtcgaggtcacgctggcatgcagtgacgtcattcgggccatgtcgcgtcccgtgctgatcgatcacttcgggcttgtccgagcctccgtcgccgggcaggtgaactcattgccacagctcatcgagttgatgggcggcgccaatgtctggatcaagctctccggtccccatcagatttccagcgacacgccgaactacagggacgttgcccctattgcccgagcgttctgggacgcagcacctgatcgctctgtctggggatcagactggccccatacgggcgggacatctcgccccaaagatgcactagcggagcaagtcgagtccttcagacttgtcgacgaccaacagcaactcggcttggttgcgcagtgggtgcctgatgaatgggctcgccgcgagctcatggtgagcaacccggaacgcctgtttggattctagaaagcctcgcatgctcagctttgcgaggaccgcttcggattttgatcagcgcgtagtggttgactccaaagtgacgcagggctcattccttctgatagtcaacacccggcggccgttgccggccggcaaacagcgacttgcggatgaccgcgtgcacgccccagttgccgtcgacgacttgcgtcacgccaaagtcgacagcgactgacatcagggaaatcgcctcgtcctcggtcagccccatcgcggtcatcaggaagcgccgggtcttgcggaaggcgtcgcgcatggccgggtcgagcgaagacttttcgtagatcgcgctgcgtgccttgtcgccgaattcctttaaatagtccgcgtggctgaagccgtggatcacccactcgtcggcagtttcgaccaaggggtagtcgatgtcggcatagggttcgccctgcagctggtccgccttgtgcaggacgatttggaaaacgcccgtcagcgagcattcgatggccgtgccgcacagttcgctgtcgccctgcgaagcgtgcggatcgcccaccgacagcagcccgccatcgaccccgacacgcaggtagagggtggcgcccttggcaatgcgccagttgtcgaggttgccgccaaagcatgagggcggcaccgagtcgacgaggcccgtctcggcgggcgcgactgcgatcacgccaaagtgcggtcgcaccggaatggtcacgccctggagcacgccatggttctcgacgatcgatgcgcggtcgaccggaattccgggatagtcgatggtcgggtgcagcacgccattcggatcgagctgcggggtccagcgaaagttgtagacggcatgagcgcaggcatcgccctggctgcagtcgacctcgtagatcgtcaccacctcgcgctgcctgggctcctcgatcaggtcgtcgtaatggaagccccaccacgcggcggcattgctgccgaaggcgcgtccctcgtacttggcatctgccgccaggcgcggcgcgagatcgaggatgcgcacctccagcacgtcgccgggctgcgcgtccttcacgtagatggggccggtgcagatgtgcaccccaaagccttcgccgctgccgcggccgtagatcgatgcatcggtggggcccgcgccgcggcggtccacggccttgtgctcgcgcgtccactggaagacgctctcggcgccggagtcgcccttgatcatgcgctcgtggtcgtcgtaggcgtgctgcgtcagcgtctcgatcgtcacgatgtcgccagaggcaatggtcagcacgggcgggatcgagcggccaaagtagccccagtggatggtctgcgcggtggccggcaagtggtgatggtggccggcgagggcgctgctgacgtgctgcgcggccgatgccgcatgcgcggtggccgcggcgccgtcatcggccacggcccgagcgtttacacgggcggtggaagccaccgggtcctcggccggcgtctcgaagtagcccgacggccagccccgccggatgcgcttgcgcagcgactgctggctggcctcgttggcctgctgccggtattgccgcggcgacatgctgtagcggtcgcgaaagcaatggctgaaatgcgccggatcgttgaagccccagcgaaagcagatgtccgagatcgacaggtgcccgtactggcggttggcgaggtcggcgcggcagcgttcgaggcggcactggcgcacgtaggcggtgaaggtctggccgaggccctcgaagagcttttgcaccagccgctccgacaggcgctcgtgcgccgccacggccgccagtgagagcgatgcatcgctcagattggcatcgacgtattggcacagccggtgcaccgtggcggcgcgcgtgctgctgatggcgggcgaggccgggtcctggtgagcggccaggcttgtggcaatgaactccgacagggccgactcgactggcgccacgtcgtcatcgctcagggtgtcgaaggcgtcggacagggcggtcagcgtgcccgcaaacatgcggcccaagcccgcacggcccgacaggtggccgagcgcgaatccttgcccgccgggcagccgcgccttcaggctggcgcgcggcatggacaccatgaactgccggaagttggagcggaaatccaggcccgcgcgcgcctgggccggtccgaagacgatgtcgccgggcgccagttcgatggtccgccgtccgtcgtgcagcgccgcatcaccgctcaggtgcagcgcgagccagacggcatcggctgcgtcgcccagccgctggagggtctgcggcgacgaggtgatgcgcgccatgccaaccccgcgcgcagtgcgccccgcggtcagcgtgccataaagaggtgcggccgccagcgccatctcgggcctgagacggtgcagatgcagggcatcgcgccaggcgtggggccgctggtgcaccgggtaggagtcggtcgagaactgttcgaactgcacggcggcgctttctggttgcttgcgcagggcgcgcaagacacgtgccacttgccgcgccccagaagagttggcatgcaactggcttggcgtgatgcatgtcgaactccgtggccgggcggcagccgcgccgacgccggctcccgcctcggcctcaacttgccgcgatgtctcccatctttcacatgatcaccggtgcaccagaaccggtcgccccgttcagccacgcggtcgaagctgacgggtgggtgttcgtcaccggacagatgccgttcgtcggcacctcgctggacacgccctatcccgaaggcatcgaggcgcagacgcggcaggtgttgaagaacctccagacggtgctggccggttgcggcctgggcctggagcatgtgctgtcggtgcgcgtgtacctcacgcacttcgacgaagactacgcggcgatgaacgcgatctacgcccaacatttttcggacggaaggcggcccgctcgaacctgcattggcgtgaccggcctggcgaagggcgcccgcatcgagatcgatctggtcgcacggcgcggcgacgcgccgtgcgcgaccgacctgcccggctgaagccaagcctcagcctttgctccgatcagcactcaggcggctgacctgcgcgagcagccactccgcgagttcaaactccacaccttgcagctcgctcgaccccaaccatatcaatccatattggctgccgtcagggtcaaagccggcaggtgctgccaagcttcctcgttccacatcgtcaacggcgagtacgagcggactcagcgctacacccaggcctgcggacgcagcctcgacaatcagggagtgatggtcgtagtaccgaatctctgtgggtcggcgcgccgaaggatgggtcttcagccattgcgcccacgcgtcaggtcgagtcttcgacccgagcgcgagatagtcaccgtgttcgaacctcggcaccagttccggcctcatgacgggcccgaccttttcggggaatagggcccggacgttccatgtctcgggcacagcgaagtcgagccgccgaattgcgagatcgacgtggttcttccgaaagtccacgagccctccacccacggagaggtggagggcaatgtccggatgcgccgcttgaaaaccgcccagccgcggaatgagccagcgcatggccactgaaggctcgcaggagagcaccagggtagtcttgccagcactggtggcacgcaggctctgcactgtggcggccagctcaccaaagaacctgctgagggtgagattgagcgtctctccggccggtgtgagcttgaggcctctcccattcttttcaaacagcctgaccccgatgtcattggcaagtttggtgatccggcggctgacggcgccgtgtgtgagcgcaagggagtctgctgcgaggcggactgaccccagcctcgctgttgcttcgaacgcccgcagatcgtcgagcgaaggtatgtctgatcggtccattggtgacaatgtatcaccggtcatcttcagaaactatcgcttttcatagcttgatggggttctgataattgatgcatgcgcaccgatcatcaacccaacatagcggtcctcgccgatgacctgacgagtgcggcggatggcgcggcacctttcgtcgctcgcggcctgactgcgtcgatcggaaggggccagcttccgcgccaagcggtagcggtcgtcgcagtcgatagcggttcgcggtctgccacttcgtcgcaggcattcgagcgggtcgctcgattgaccgaccggcttgccggctgttctgtgctctacaaaacggtggactccacgctgcgcggccacatagcgcaagagctcgaggcatgctttgccgcgagcggccgcacatcactggtgtttgcgccggcattcccccaggccgggcgcacgacggtagggggaattcagttcgttgacggcattccggtttcgcagagcgcgtatgcccatgaccccgtgcatcccgcgcggcattccgcgctggtcgacctggtcccgagctccatcaagaatgtcaccttcctcgatgcggtaacgcaggaagaactcgactcgcggattgcttcaatagaggatccagagtcgatcctgtgggtcggctctcccgggatggctgcagccctgtcgcggcgttttgtgccggagaagacaccaccgttatcggtcgatggcatcagcagcgatgtgctggtcgccgttggaagcgcgaatctgcgcagtcacatacaggccgatcaactccagcaggccagcggcgtcatgctgctgcgcggaccaaaggcgcgagagcaggattcggcggcggtgctgcgccgcatcgcagagggggcggcgctagagcttcgcgacccacgcttcggcgcattgatcgccaccggcggcgacacgatggaagcgatcctggatcttctcaacatccgtgagttcgagattctgcaagagctcgatcccggattcccgctgggtcgcgccaggcttggcgatggacgcttgctcctgctcgccatgaaggccggtggctttggcagtgacgacgctctggagcgcgctgtcgcgcgcatacgcggaacaactcaaaccttgcgaacggattcacagtgaagaacatttctcccccgcttgccctgaccatgggtgatgcatccggcattgggccggagatcgtggcgaaggtacttgcgaagggcggcgaacgcgtcgtcgtgttcggcagccatgtcgtcatgcagaatatcgtgagccggctggggttgaacatcgaggtgcgacgtatcgatgcacccgacgcggcccagttccagccgcagaccatcgaagtcatcgagaccacccggattgccgagcttccacccatcgggcagatcagcgcgatctccgggcaggcggctttcgatgccatcgttgcagcgatcgcggcagcgaagtccggagaagtgagcggtatcgtcacggcgccgatcaacaaagaggcgatggccagtgcgggaatccgctaccccggccatacggaaatcctggcggacttcggcggcgccaagcgcgtggcgatgatgctggcgaatgacgatatccgcacggtgctcgtcacgatccacacgtcgctgcgcaaagcaatcgaacaaggcgatttcgacgcccagatgtctgccatacgccttgcccacgagggtgggaaggccctgggcttcgcggccccgcgcgttgccgtagcgggtctcaacccgcacgcaggtgaaggcggccttttcggcgatgaggagatcaggatcatccggcccgccatcgaagcggcccgagccgaaggcatcgatgccagcggcccttacccgggcgatacggtcttcatgcaagcacgtatgggccggttcgatgttgtggtggcgcagtaccacgatcaagggctgattcctgtgaagtatctcgggctggaaaagggcgtgaacatcacgctgggcctgccgttcgtgcgcaccagcccggatcacggcacggcattcgacatcgcaggccgggggatcgcagaccacgcaagcctggaaacggcgcttgcctatgcaaagcgccttgtcgctgcgcaaaccacgacgaactaacttcgaaaggaaccagcatcatgggtctacgtttcatcttcatgcttacgcgcaacgaccgcacggttccggatgcggcgcagcaactccagactgcactcggccttggcgtgcggcacattgggttcaaggacatcggcttgccgctcgagcagctgaagggtctcaatgcggcgatcaaggccggcggtgcaacctcctatctggaagtggtgtcgctcgaccgtgaaagcgaaattgtttcagcaggggcagccgccgaaattggcgttgacattcttttgggtggcacgcgggtcgatgacgtgctgcccatcatcaaggacacaggcattcaatacttcccgttccctgggcggattaccggccacccgagcgtgctcgagggcaccatcgaagaaattgtcgaaagtgcccggacgattgcagggcgcgatggcgtgcatggcctggacctgctggcatatcgttcggcccagaacgtacccgagttgatgaaggccgtctgcgctgcggtctcgaagcctgtctacgttgcaggctcgatcgccacccctgaacgaattgcagtcgtccagagtgctggggcagcgggtttcacgatcgggactgcggcactggacggcaaatacccggcccctggcaatgacgtgccgagccagctcgccgcaatccttcgcgacgtcgctgccctgaacaagcatctttcgaccattcccaagaagaatttgtcgactgcgtttgccggccaggtcgaggggcagggcgacaacgtgcaaatcaaggtcgccaagttcgagggagcctctcgctggtcattcagacagcacggcgatgaactgttctttgttcatcgggggcgcctgctcatgaaatttcgtgaccgcgaggagatcgtcgagaccggagagttcatcgtcgtgccgcatggcgttgaacattgcgcagtggctttggacggggaaccttccgaggtgttgctggcaactgcgactgcgtagttcccgccggcggtggttgcacaccgcataccctggcaaacgctcacggtatcggaacgcggatttatgcggtcaaatacaggttttgccgctcttgatgcagaaccgatatgaactaccgccagatcgagtgcttccgtgccgtcatgcacacaggctcgatgacgcttgccgcgacgcagttgcacacgtcgcagccgaacgtgagccgtgccatcgcgctgctgcagggcgaaacgcagctgaagctgttcgaacgcgtcggacagcgcgtggtccccacgcctgaagcgcacgcactgctgaaggaagtggaccgcgtctacgtcggcctgcagtccatcggcgacgcggcggaccgcatccgcacgctgggggtcgaaggcttgcgcatcgccgtatcaccgggcatcggcgtcagcccggtgccgcgcatattgcaggtctttcgcggaatgcgcccgcgcgttccggtcgtggtccacacggccgattccgcgaccatctgcaagtgggtgtcgtccgggtattacgaactcggcctggtcggctatgttgcgctgccgcaggaggtcgacaccacgctcgtgcattcggatcgcgcggtatgcatcgtgccgcgggggcaccgcctggcgcgcaagcgcaaggtcgttccggcggacctggccggcgagtcattcatttcgcatgcgtctccggacgtggtgcgtgcggccaccgaccgcgtcttcgatcccgaggtgcgcaggcttgagatcgagacgacgctgggcaccacgatctgcgcgatggtggcgcgtgggctgggcgtgagcatcgtgaatccggcgatgctcagcgagcttgcgctcacgggcgtgcattcgctggcgttcgagcctgcgatccagatcgaatgccacttggtgcttgcccgccagcagccggcgcaggcgctcgtcgcagacttcctcgaggccatacgcgtcgtgacgcgcagccccgacaacacagagcgcaagaaggtcagccgattgcctgcgtgaccagtgcccagccgccgtgggcaggcccgcgctccggtacgcgaccgcggaccatgacggaccctccgccggcgcgtggcagccccaggctctccagccattgggccaagccgcccgtagcgtgaacgtcaacgcgcatgaagccttcggcgtgacggcagcattcggcgatcagcaggcgtgcggcatcgagctcgggcgctgccaccggtcctacggcatggccgcggccatagcggcgaagcaccgcgaagccggcgacatggccgcctcgctcgatgacgactgttttctcctgagagaacaaccggcaaagcagttcgccgcgggccatacccgcgccacgggtgtccatcgcgatcagagattcgacgtccgcagctgctagcggccgcagccggtcgccctcgcgcttggccagcgccggaaaggccgcaagcacgccctggtgctggtcgatctcccctgtggcgacgaatcccaggcgctcatacaggccacggcctgctgccgtcgcgtgcagcagcacatctcgcgtggccaggcgatcgagcagcgcctccatcatgcggttgccgatgcgctgaccctgcagttcaggcgcgacgatcacgaggccgatggtggcgtgtttcgcgccaaattgccacgacaacgcggttcccagcactttcccgtcgcgttcggcgaccacgccttgcccgagcgacagcgcgaactgccagtcttcgatccgatgcggccaattcaaggtgctggacaacgcgtgcgccgccggcaaatcgcttggttcaaacgggcgcagtacggcatcggccgtgaccgccgtgggctcgactgcgattgtggtggaggggaacttcatgcagtcgagtatgggtatggggatgcatgcggtcgaataaaaattcagaggtcgttcattcgggtttgatatgcaggtccgatgtaccgcagacccgcgacatgcgcggtcacgcctatcggtgtgcaagagtggttcatatcaatgctgtatggataccgcaaaaacttgtatttgaccgcatgtatcggccttccgatactgcacgcactaactcgactccccgccatgacttcagcattgcccacgtctgccgccctagtggaagggggcacgatcattgaacgcttcaggcgcgctggccacctggaccgcatcttcatcgacggcgaatgggtgctgccccaagggcaagctcgcgcctctgtcgtcgacccgtcgagcgaggagcctgtcgcggaaatcgcgctgggaactgcccaagacgtggctacggcggtggctgcggcacggcgcgctttcaccacctggtccgtgagccccgcccagaaccgtgccttgctgctggaccgcgtccacaccctgatcctggaacgcgccgaactgttcgcccaggccatctcgctggagatgggcgccgccatcggcttcgcgcgcctcacgcaggtgccctccgcggcggagcacatccgcgtggccagtgacaatgcgcgcagttatgcgttcgtcacccatcggggagacatggccctcgtgcgcgaggccatcggcgtgtgcggcctgatcaccccctggaactggccgctctaccagatcaccgccaaggtcggcgccgccctggcagcgggatgcaccgtcgttttgaagcccagcgagctgtcgcccctgagcgccctgctctttgccgaagtgacgcacgacgccggccttccgccgggtgtgttcaacctggtgaacggcagcgggccggaggtcggcgccgccttggcggagcatccggacgtggacatggtctcgttcaccggttcgacgagggccggcgtcctggtggcccaggcggcggccccgacggtgaagcgcgtggcccaggagctcggcggcaaatcgcccaacctcatcctgccggatgcggacctgtctgtggccatccccaaaggcgtggcgtccgccttccgcaacgtcggccaatcctgcagcgcaccgacacgcatgatcgtgccgcgcgcgcgcctggcggaggtggaacggctcgcgcgcgaagcggccgccggcttcgtcgtgggcgatccgcgctcgcagcagaccacgcacggcccggtggcgaaccgcgcacagttcaaccgggtgcaggaaatgatcgatgtcggcatcgccgaaggcgcgcagcttctttgcggcggcctgggacggccggagggcctgagccgcggcttctactgccgcccgaccatcttcagcgcagtgcactcccagatgcagatcgcgcaggaggagatcttcgggccggtgctcgtgttgatcccctacgacagcgtggacgaggcagtggacattgccaacgacaccgtctatggcctgggcgcccatgtgcaaggcaaagaccttggcgcggcgcgcgccgtcgcggcgcgcatccgctccgggcaggtgcacatcaactatccggcctggaatcccaacgcccccttcggtggctacaagcgctccgggaatggccgcgaatacggcatcgaaggcttcgaggaatatctggaaaccaaagccattcttggcttcaatgcttaggagaaaaaatgaccgtggccatcgtgctgcaccgtgccaacggcgcacccgcttcaaccgctttccgcagggcgccgttcggcaaagacgatccgtttgcgcggcatcgcgagatcgcgtgggaaggagcccaatcgatgatcgcgggccgcaccagcttcatcggcgagctcgacgtcgcaagctatccccatatcgaaaccatcgtcgtgtcggaaggcgagctgaccctgatcgcgaccggggaggctccgctggtgctcggtccgcaaacaggtgccgtgatcggatgcgggacgtcgcttcgcatcgcggctgcatcccgcgtgcagttttctttttgcgcggccgcttgcgacaagccggcgaagcgcggccttgtcccacttcgcgccgacgccgacttcaagccgtcccgttcactaccggcagagatgctgctagggccggcgccggagtgtcgcagcgacaacgtcttcacggacgacgccgcgcagtacagcgctggcacgtgggactcgaccccttaccaccggatcgttcgcccgcatcgccagaacgagttcatgcatctcgtggccggcagcgtgcggttcgcagcgccggatggcagcgtgctgtcgatggacaccggcgacgcgcttttcgtgccccagggcgcgccgatcggatgggaaagcagcgatcgcgtggcgaagttctacgtggtccaggccgtccaagcttgaacgggcgagcgagattcatcatgtcccctccgctgaaccagattcaaacttcccccacgccgccggcttcggcggacgtcgtcgtcatcggcggcggcatcatcggcgtcttcaccgcctactacctggccaagcgcggcctttcggttgccttggtggaaaaaggcaggatcggcgccgagcaatcgagccgcaactggggctggtgccggcagcagaaccgcgacgcccgcgaacttccgttggcgaccaagagcctcgacctgtgggaacagtttgccgcggagaccggtgaagacacgggcttccaacgctgcgggctgctgtatctcagcaacgacgaggctgaattgtctcagtgggccggctggcgcgattttgcgaagaccgccggcgtgacgacccacatgctgagcagccgcgaggccgccgagcgggggcaggcgaccggccgcgcctggaagggcggcgtcttctcgcccagcgacggcaccgccgatcctgccaaggccgcgcccgccgtggctgctgcgctcatcaagctcgggggcagcgtccaccagaactgcgctgcccgcggcatcgagaccgaagccggacgcgtcagcggcgtcatcacggaagcgggcgtcatcaagacccggacggtcgtgatggcgggtggcgcctgggcgtcctcgttctgccggcagttgggcatccgttttccgcaggcctcgatccgccaatccatcctcagtgtgtcccctgtggaacatcgcttgccggatgctttggttatcgcaggcctgtccgccacgcgccgcaacgacggacgctatgcgctggccatcagcggccgtgcgcgcgtggacctgacgccgcagttcatgcgcttcgcgacgcagttcgtgcccatgttcgccaagcgctggcgcagccttctcccgggcggcctggaaggcattcgtggaggccatgaaacgctggggcggtggcggctcgacgcgccgacgcccatggagcgcgtgcgcatcctcgatccgaagccctgtttgaccacgatcagggagacccaccgccgcgcggtcgaactgctgccccaacttcgcgatgcaaagatcacgcacgcctgggctggcttcgtcgacagcacaccggacggtgttcccggcatcggcgaggtgccgggtctgccgggattcattttggccgcgggcttttccgggcatggttttggcatcagccccggcgcgggccacctgatcgcagaccttgccagtggcgccgaaccgatcattgatcccgtcccattccggcctggccgattcagtggcactgcatggggcaaggtcgctgatttttagatcctgaacaggagataaccatgaatgatcacagcagcaacttgaaaggtggcgacatgaagcggacgaacaagattggcgatgcccccatgggcagactgacacggcgagacgccgtatttgccggcgcagccacctttgccctgggttccctgggctccttgggtttggcgacgagtgctcgcgctgccgcgccggccgcgaagccaacgggccaggccatcctcggcttctcgcaggaagtgaccgtcctgcatccgctgatgaccgccaacgaggtggaccagggcgtctggtggaacctcttcagtccgctgtggatgcttgatgcggaagggaagttcgtgcccctgctggcgaagtcggttcccaccatcgagaacggcggcatctcggccgacggcctgacctggcgcgtcgaattgcgcaacgacgtgaagtggcacgacggcaagccgatgacggcggaggacgtcaagtattcgatcaatctgatgaagaacccggccttccgcgcccgcaaccgcacggccttcgagtacatcgcgtccgtgggcgtcgagggcgaccacgtgatcacgtggaagctgaaggaaccgtacgcaccgctgacatccgtgctgagttggaccttcatcgtgcccgcgcacattctttcgcagaacccggacccgaactctccgctgtttgccgctgcgcccgtcggcaccgggccgtttaagttcgtcagccgcaagaccggcgaccacgtgatcctcgaagccaatccgaattactttggaaagggtccgtcgctgaaccggctcatcttcaagtacgtgccggacctgaatgcgatgtacacgcagttcaagaccggggagatcgactacgtcggcctgcagggcattccggccaacttctacaaggaagcaaccgcgctgcgtggccgccgcgtccatgcagcgccccgcggcgcggtggagaacctgacgctcaacctcgctcacccggcactcgcggacaaggcggttcgcaaggcgctgaacattgcgatcgaccggcagtcgatttgcgacctcgtctattacggcgtgcccaagccggcgaacaactacctcgtcccgacgcactgggcttccaatcccaacctgccgaagcccgagtacgacccgaaaaaagcttccgcgatgctggaccaagccggctgggtgcgcggcccggacggtattcgcatcaagaacggcgtgcggctgtccttcacgaattcgacgacgacgggcaaccagctgcgcgcgcagacgcaacagctcattgccgacgacttcaagaagatcggcgtcgagatgcttatcaagaacctggtagcggcggtgctctgggcagacttctggcgaaactccgagttcgacagcctgatgaccgcgccgacctacacgatcgcatcggatccggacatcacgcaccgcttcggctccgcaagcatccccaaggagaccaaatcgggttcgaacgtgagccagtacaagaacgtcggggtggatacgctgctcgcccggggccgccaggaatacaacctcgccaagcgcaaggagatctacgccaaggtccaggagctgatcatggatgacctgccattcctgccgctgttctacgaggtgcagatcgaaggtacgaagaccggtctggacggctatgcgaacaacgtgaatgcgctggccaacagctggaacgcggccagctggcgctggacggcctgacgcatcatggctcgctaccttctgcgccgcctgctgcagtcgctgctgctgctcgcgctcgtctcgatgatcgcctttgccatcctgcatcttgcgccgggggggccgctggcgcagtttgtcgccacaggcgatctcggccaggaagacgtcgaccggctgatgaagcagtacgggttggataggcccgtgccgatccaatatctggactgggccggaagcattgccacaggcgattggggcaactcttaccgggaccagttgccggtgctgaagaagatcggcatgcacgtcggacccacgctcgaactcatggtgagttcgaccctgcttgcgatgttcatcggcggcatgatcggcatcctgggtgcggtgcggcgctattcgttcttcgaccacctggccaccatcggcgcgatggtcgcgctgtcgatccccacgttctggttcggcctggccgtcatctatgtgttctcggtgaacctgggctggctgccggccggcaaccgcgaaacgatcggtgacggctccttcatcgaccgtctgcagcacctggtggcgccatgcatcgtgctggcgctggtgtccaccgccgtgtggagccgctacatgcgctcctccatgcttgacgtggtgaatcaggattacatccgtaccgccaagtccaagggcgtacccgccatgcagatcctgctgcgccacgcgctgcgcaacgcgctgctgcccatgatcacgatcacgggcttgcacgtgtccacgctgctcagcggcgcgctcgtgacggagaccgtgttcacctggccgggcatgggccggctctttctcgacagcgtcagcaaccgggactaccccgtggtgatgggaatgctcatgttcacggcctgcatggttctcttgggcagcttggtcgcggaccttctctattccgtcgcggacccgcgcatcaaaggagcgtcgaaatgagcaccgtcccgaccgtaccgctggttccgccacgccgcacgctcgccgaacgctatccggccctgaggcgcttcctgcaccatcgggcggcgctcctgggcgtaggcatcgtgctgttcatgacgctcttgagcttcatcggcccgttgctgatgccgttcaatgccaccgataccgacatccgcgcgcggttggcggagccgttcgggggcccgcacgtgctcggaaccgatcccttgggccgcgacgttttggcgcgcctgatgtatgccgggcgcatctctctggctgtcggcttcgcggccacggcactgtcggtggtggtgggcgtcctggtgggtctcgtggccgggttctaccgcggcgcgatcggtgctgcgctgatgcgtttcgtggacgcgatgctgtgctttccgaccatcttcctgctgctggccgtcgcggccctgatcgagccgtcggtcacgtccatcgtgctgctgattgccttggcgagctggatggaggtggcgcgtgtggtggaagggcagatccgatcgctgcgcgaacgcgatttcgcgctcgccgccgaatcgctcggcgccagcgacagccgcatcatgttccgcgagctcctgcccaacgcggtcgcgcccattgtggtcgcagcgacgctgaacattgcgcacgccatcctggccgagtcgtacatcagctttctcggcttcggcatccagccaccgacgccgagctggggaaacatgctggagaacgcgcagagctacctgaccaacgcgccctggctcgcgatcgtaccggggctggccatcacgctgaccgtcacgagcttcaacttcattggtgacggcctgcgcgacgcgctggacgcgaaactggatcgatgaaatgcttgatatgaaccgttttgagccgatcaccgccgagcatgccgaagccgccattggtgcggagaacatcctggacgtgcgcgatctgaacgtcgcgtttcgcacagcagccggaaccgtgcatgccgtgcgcgacgtcagcttctcggtgcgccgcggcgagacactggcgctggtgggagaaaccagttcgggcaagagcgtgacctgcctagggttgctcggcctcaccccgcccgctccgtactgcacgatcagcgggtccgcgcggcttgcggcgcgcgatggccagacgtacgagctggtcggctcgcctgagcgtgtgatgcgacgggtgcgaggtggcgtcgcttcggtgatcttccaggaaccgatgacgtcgctgaatccggtgcacaccgtcggcgctcagatctgcgagagcttgcgcatccaccttgggatgcgcgggcgtgctgccacggaccgcgctgccgaactcttgaaccaggtcggcatctcagatccgaagcgccgtttgacgaactacccgcacgagctgtccggtggcatgcggcagcgcgtgatgatcgccatggcgattgcgtgcgaaccttcgctgctaatcgcggacgagcccaccaccgcgctggacgtgaccatccaggcgcagattctcgaactgctgcagaagctgcagtctgagacccggatggccatgatcttcatcacgcacaacctcggcacagtggccgagatcgccgatcgcgtgatggtgatgtatgcaggccggatcgtcgagcaggccgatgtcgttacgctgttcacggagccccggcatccctatagccgcggcctgatcaactcggttcctcggcttcattcgaatcgtgcccgcaagacgccgctgttcgcgattccgggcaacgtgcccgatccggcctcgcacccgccgggctgcaccttcgggccgcgctgccggcacttcgagccaggtcgctgcgatgccgcggtgcccagcctggatagcgcaaagccgggccatctggtgcgatgcgtccgttggccggaaattgaaggagccgcgtgatgctgcaaaaacaacttactccccctttgttgcaagtcgagggattgcgcaagtggtatccgctcggcggcggctggtttggcaagccggcacagaacgtcaaggcagtcgacggcgtcagtttcgagattcgccgaggcgaggtgctgagcctagtgggcgaaagcggctcgggcaaaagcacgatcggccgcgccatcctgaacctggacccgccgacggcagggcaggtgcacttcgacggagaacccctggtgggtctctcgcggcgccagatgcggccgctgcggcgcgcgatgcagatggtgttccaggacccgtactcgtccctgaacccgaaacacactgtcgaggaactgctctcggcgccgctcgaaatccacatgcccgagctgacggtgcaggaacggcgggatcgcatcgatgccgtgctgaagacggtggggctcaaccccgcgcatcgttcgcgctatccgcacgagttctccggtggtcagcgccagcggatcggcattgcccgtgcgctcatgaccgagccgcagctgctggtggccgacgagccggtgtcttccctggacgtctcagtgcaggcccaggtgatcaacctgctgctggagctgaagcagcggctcggcctcacgatgctgttcatcagccacgacctcgcggtggtgggccatatctcagaccggatcgccgtgatgtacctcggccgtctggtggagatcggcgacgccgaatcgctgttgaacaacccgcggcatccgtatacgcgtgccctgatggccgccgttccgaacatcgatccgcggcagcggcgcccgcgcgaactgctcaagggcgacattcccagcccgctgtctcccccgtcgggctgcgcgttccgcacgcgctgcccccacgcccagtcggcgtgcgcgagcggggtgcccgaactccggctcatcgagcgcaatcacgcgaccgcgtgcatccgcgacgacatctgacgcaggcgcagctcgatcggcccttccgcttttcgccttttggcgcgttccgaccatgggcgccatctgaatcttctccattcaacaaaggatcatttctcatgagcaatctcaccttcttcaaatatgacgacctgggtaccgcgcgtgagggcggcccgctgcccgagcgcgtcatcgaaggcgacgccaagttcaagaattgggacgtcgaacgttctgccgacgaaaaggtgcgcgccggcgtctgggagacgacgccgggcaccttccggtccatcaaggggggcaccatggagttctgctacatcctctcgggcgtgtcggaaatcacggaagacggaaagccgccggtgcgggtccaggcaggcgacgcgttcgtgatgaagcctgacttcaccggcgtgtggtgctgcatcgagactacccgcaagatctgggtcgtctaccagtaggccgcatgtctttcttgtacaaggccgaccccgtgcgcggggcggaatgggcacgcctgttcgccacgcaggcgcccgacattccgtttcatatctggcccgacaccggaaaggcggaccacgtgcgctatcttgccgcgtgggtgccaccgcaggacatagaacggcagttccccaacctggagctcttcttctccaccggcgcggggatcgaccagttcgacctcgccgcgctgcccccggagttgccggtggtgcgcatggcggagcccggcgtcgtcgcgggcatggtggagtacgccacgatggccgtgctcgcgcttcaccgggatctgccaacctacatccggcagcagcgcgagggctgttgggctgcgcaccgcgtctatcccgcgtcgaagcggcgcgtgagcgtcctcggcctgggcgtgctcggatgcgctgtgctggaccagctgcgcacactcggcttccagcttgccggatggagccgaacgcgccgccagattgacggcgtggcgtgctacgcgggtcgggaagaactggcggcgatgctggccggcaccgacatcctcgtgtgcctgcttccccttacccaggagacgcgcggcattctcgactccaaactgtttcagcatctgccgcgcggtgcatcgcttgtgcatgtcggccgaggggcgcatcttgaccatcaggcgctgctcgatgcgctggagagcggcgggctgtcgggcgcggtcgtcgatgtcaccgatccagagccgctgccgcagggccaccccttctgggcgcacccgaagatcctgctcacgccgcacatcgcgagcatgacgcagccggagacggccgtggaacaggtgctcgacaacatccgccgacacgaggcaggcgcgccgctgatggggctggttgatcgtttgcggggatattgagaccccctcgtcaagaaaatgaaaccctcgatgctgtacttgtccacccgcggccatcccgaccgcaagcacttctgccaaatcctgctggagggcttggcgcccgacggtggcttgtacctgccggagcaatacccgcaggtcactcccgagcagttgtccaggtggcgcgatctgccgtatgctgaactcgcctttgaagtgctctcgctctacatcgacgacatcccggcggaggacctgcgcgcaatctgccgcaagacctataccgaagaggtgttcggcacggaggcgatcgtgccgctcaagccgctggaagacggtctctaccttgaagccttgtccaacggcccgacgctggccttcaaggacatggcgatgcagctgctgggcaacctgtttgaatatgagttggcgcgccgcggcgaagagctcaacattctgggcgccacttcaggtgacaccggcagcgctgccgaatacgcgatgaagggcaagaagggcgttcgagttttcatgacctcgcccaatggccgcatgagccctttccagcaggcgcaaatgttcagtctgcaggacgcgaacatccacaacctcgccatcgaaggcgtgttcgacgattgccaagacctcgtcaaggccgtgtccaacgatctcgagttcaagcacaagtacaagatcggcacggtcaactcgatcaactgggcgcggctcgtggcccaggctgtgtactacttcgccggctacttccaggccacgcagtccaacaccgaacaggcgagcttcaccgtgccgtcgggcaacttcggcaacatctgtgctggccatgtagcgcgcatgatgggcctgcccatcgacaagctcgtgctcgccacgaacgagaatgacgtgctggacgagttcttccgcaccggggtctatcgggtccgcggcagcgccgacacctacgaaacctccagtccatcgatggacatttccaaagccagcaacttcgagcgtttcgtgttcgacctgctgggccgcgatgcgggcatggtcaagcgcctgtttggcgaggaactcgcgaagaacggtcgtttcgatctgagcgccgacccggtgttcacgctggcccgtgcgcgctacgggttcctcagcggcaagagcacgcacgccgaccggctgacgatgatccgcgacacgcaccagcgctttggcgtgacgatagacacccacacggccgacggcctcaaggtggcgcgcaacttcgtgcagcctggggtgccgatgatcgtgctggagacggcgctgccgatcaagttcgccgcgaccatcgcccaggccttgggccacgagccagaccggccagcgcagttccagggtatcgaagacctgcccaagcgcgtgacggtgcttgcggccgacgcggcgcaggtgaaggcgttcatcgccgcccacctgtcctgatcgcagcatggctgtcttcaccgaagttccgtacgaggaggctgccgccttcctgcggcggctgggccttggcaacttgcaggctatggccgcctgcagtggcggcatcgagaacaccaactacttcgtcgacacggatcgcggcgagtacgtgctgacgctgttcgagcgcctggcatgggagcaattgccgttctacctgcacttgatgcagcatctggccagtcgcggcgttccggtgccaaggccggcgccagatgccgacggtcgcatcctgcaccgtctcagggataagcccgccgcagtggtgggaaggttgcgcggaaagaatgaactggcgccggatgtgcagcaatgcggcgcagtgggcgaaatgctggcgcgaatgcacttagccggcagagactatgcccgccaccagcccaacctgcgtggcctgccgtggtggaaggaaaccgtgccggttctgctgccacacgtcggcaacgaccaacgcacgctgatgctggatgaactggccttccagacacgtatcgccgcatcgcccggctacgcagccctcccgcgagggccggttcatgccgacctgtttcgcgacaacgtgatgttcgagggcaggtgcctgagcggcttcctcgatttctactttgcgggttgcgacacctttctgttcgacatcggggtctgtctcaacgactggtgcgtggatctggacagcggacgcgccgacggcgtccgggaggcagtatttctgacagcctacgagtcggtgcgcccgctcgtgcttgaagaacgtcgtctgttgcctgcccttcagcgagccgcggcattgcgcttctgggtatcgcggctccgggattgctacatgccccgcgaagccgccgctctgaaggctcatgaccccagccacttcgaacgcgttctgctccatcgcgtgagcgacgccgccggcgcaggcattttctagaaaggactttgggccgccctgggccctgatgatcaatcatgagaaccaccgcagatttctacgcctcgctccgaaccgaactcgagcaaatacaggccgctggcctgttcaagcttgaacgcacgatccaatcgccacaaggaagccagatcgccaccgccgatggacgggaagtgatcaatctctgcgcgaacaactatctgggcctgtcatctcaccccagcgtcatcgaggccgcccatgacgcgctggctgcgcgcgggttcggtttaagttccgtccgcttcatctgcggaacgcaggatgtccacaaaacgcttgaagtgcgcctctcgcaatttctcggcacggaggacaccatcctgtacgggtcggcattcgacgccaatggcggcttgttcgagacgctgctcggacccgacgatgccgtgatcagcgacgagctgaatcacgcgtccatcatcgatggcatccgcttgtgcaaggccaagcgataccgctatcggcacaacgatgtgatggacctgcgcgagcaactgaaagcggcggatgaagcaggagcccggtacaagctggtgttcaccgacggggtcttttcgatggacgggaccattgcccgcctggacgaaatccgtgatgtctgcgacgagttcggagccttgctgggcgttgacgactcacacgctaccggttttctgggcaagcgagggcgcggaacccatgaatatcgcggtgtcttcggcaagatcgacatcatcaccggcaccctcggcaaggcgctcggcggtgcatccggcggattcacgagcgccagagcggacgtcgttcaattgctgcgccagcgctcgcggccctatctgttctcgaacagcctggccccggtgatcgttggcgcgaccttgaaggtgctcgatctcctggaagccgacacaaagctgcgcgacagcctggaggacaacacacggtacttccgcgccgggctcgcggcacgcggtttcgaactgaagccaggcgaacacccgatcattccggtaatgctctatgacgcggagctctctcagatgttggctcgtcggttgctcgaactgggggtttacgtgactggattcttctaccccgtcgtgcccaagggccaggcgcgcatccgcgttcagatcagcgcgcagcacaccgtttcccaactggatgttgcattgagcgccttcgcgcaagccggcaaagaactgggggtagtcgcatgaccgggctccctcgcattctggtcatcggcgctaacggccagttgggcaccgagctttcccttgctctggcggaccgctacggcggggacaacgtggtgggcagcgaccgtctggaggtgggccggcacgccaatctccgctatgagatgctggacgccacggactttggccaactcacgaaggtggtcgagaagcatcgaatcacccagatctaccatctcgcggcggccttgtcggcaacgggcgagactgcacccgactgggcgtggaaactcaatatgggcagcctgttgaacgtcctggaggtcgcacggcaacgcaagctggacaaggtgttctggccgagctccatcgccgcctttggtccgacgacacctgccgatgccacacctcagcgaacggtcatggagcccagcaccgtctacggcatctccaagctggccggcgagggctggtgccgctggtacttcgagaaccatggcgtcgatgtccgtggcctgcgctatccgggactcatctcctacaaggcgagccccggcggtgggaccaccgattacgcgatagacatcttccacgcggcccttaaaggagaacgctacacctgctttcttgccgaagatgaaccgctgcccatgctctacatggacgacgcggtgcgcgggaccctggagttgatggaagcccccagtgcggccatctccgaacgcggcagctacaacctcgctggcgtgagcttcacgccccgcgagatcgcgcaggagatacgcaagcatctgcccgacttcgaaatcgtgtatcagcctgatttccgacaggcgatcgccagcgggtggcccgattcgatcgatgacagctgtgcacgtcgcgactggggctgggctccgaagtacgaccttgcggccgctgtccgcgacatgctgaagaacctgtctcccatgtcgatgccaagcgcagagctcggtgtggcaaatggtgagcaagtggccgcaaattgacaacccctgaatgacaagcaccatgacactgactctcgaacgcacggacctgatgcccggacgccaattgatcggcaccgaatggcgcgaggcgagcgacggacgccgcctcgacgtcaccgaccccgccaccgacgacgtcttcgccagcgtgcccgacggcagcgccgccgatgcgcgcgccgccgtcgatgccgcccatgccgccttcccgacctggcgggcggtgcccgccaagcagcgcgcccagatcatcaagcgctggaacgacttggtgatggcgcaccaggaggacctcggccgactgatctcgcgcgagcagggcaagccgctggccgaggggcgaggggaggtggcctatgccgccagctacatcgagtggtttgccgaggaagccacccgcgccaacggcgacgtcattcccgcgccggtgcctggccggcgcatgttcgcgctgaaggagccggtgggcgtggttgccaccatcacgccctggaatttcccggccgccatgatcgcccgcaagatcgcgccggccctcgcggccggttgcaccgtggtgtgcaagccggccgaagacacgccgctgacctcactcgccttggtcaagctggcccaggaggcgggggtgccggcgggcgtgatcaacatcgtcaccgcgtcgcgcgaacgcacgcccgaggtggtggacgtgtggctggacgacgcgcgcgtgcgcaagatcagcttcaccggctctacgccagtgggccagcacttggcgcgccgttcggccgacacgctgaagaagctgtcgctcgagctgggtggcaacgcgcccttcatcgtgttcgaggacgctgacatcgatgccgctgtcgaaggcctggtggcggccaagttccgcaacggcggccagacgtgcgtctccccgaaccgtgtgttcgtgcaccagcgcctgcacgacgatttcgccgacaagctggccaggcgagtcggagcactccaggttggcccggcgagcgacccgcgctcgcagatcggtccgatgatcaacgcgcgcgcggtcgagaagatcgagcgccatgtgcaggatgctgtcgccaggggcgccaaggtgctcaccggcgggaagcgacttgtcgatctgggcccgaactattactcgcccacggtgatggtgaacgccgatgccaccatggcctgcagctgcgaggagaccttcgggccggtggtgccgatcacgcgcttcgacagcgaggccgaggtgatcgccgccgccaacgacacgcccttcggattggccgcgtacttctattcgcaggacgtgcgccgcatctggcgcgtggccgaggcgctggagacaggcatcgtcggcatcaacgaaggcgcgctcgccgcggaggccgcccccttcggcggcgtcaaggcctcaggctacggacgcgagggctcggtgcacggactcgacgactacctgcacatcaagtacgtgtgccaggggcagctgtagcagcttacggtcccaacctggaatgcgggtgtgcgcgtccaacgaagtggccgtgcccggcgaactgatcggtcgtcgcggtccgaccgcgctaaagcgccctcgcgcctgtctggccgcgctgcatcttaatcagtggccgccgagttcttcgccaagctgggcttccgcgcctcgccggcggcgatggagcgcccgcggtcgaaatcgtccgcggattgatgggggatgcaaaaggcagaatgcggcagatcgccccgtgtcgatttgctgcgggctcgttcgtcgtgtcagttgagggtcatcctctgcacttcaggagaacgccaccatggcaaccaacaccgtccgcctgcatcgcgtgctgcgcgccccgccggagcggctttatcgtgccttcgtcgaacccggcgcgttcgagcgctggctgccgcccttcggattcaccggcaaagtccacagcatggagccggtggtcggaggtgcctggcgcatgtccttcaccgcctttggtaccggccacagccactcgttcggcgggaagtacctggaactcgttcccggccagcgcattgcctacgatgcggcgttcgacgacccgaacctgccgggcaccatgaagaccaccgtgacgctgaccgcggtgtcctgcggcaccgacatgtccgtcgtgcaggaaggcattcccgacgtgattcctgcggagatgtgctatctgggctggcaggagtcgcttgtggcactggcccagttggtcgagccgaatattccgggttgagcggcagcgcacggccaacgccgtgtcttccggtatcggcgaagtacccgccgagttcggccgacacatcgacgttcagaacgtcgccgacccggatgaaggcatgagcgatcgcggtggccccggcgcgccgtccgtgcgaacatccgcgcccatgagcgacattcatttcggtatcgaccgcttttcgcactttcaaggcgtgctgcgccttgcaggccatgccttctcgcgcagcgccgaggtgcaggccatcgaattgctgctgggcgacgggcaggtggcggtcctcgcgcgcatccggctgccgagcgtggacctggcagggcgctacggccgggtcgcggtggcctgccgcttcgacgagacgctggtggtgggcgaggacatcgcgccgctgctgtccgcgcgcttgcgcatccgtctgagcgacgggcgcgagcacctggtcgacgcccccggctcgctcggccgtgagaaccgggtcgagaccctgttcgatcgcttcaagtcgatggtgtgcacgcggccgcccgggcacctgctggaggtgggctcgcgtgcgcgaatgggcgtgacgcggcgagattggctgccggagggctggcactacacgggaatggacgtggtaccgggaccgaacgtggacgtggtgggcgacatccacctggccagcagcttcctgccggccgaaggcttcgacgcggtgatgtcgcacgtggtgttcgagcacctgatgatgccctggaaggcggcggtcgagatcaaccgcgtgatgcgcacggggggcgtcggcgccatccttgcgccgcagacctggagcctgcacgaggagccgtgcgactacttccggttttcgcgccatgcgtggcaggcgctcttcaatgccgccacgggcttcgagatcatcgaagcgcagcacgacatgccggcctacatcgtcgcgcagcacctgatggcggagacggcctttcgcgaactgccgggcatgctgagctcgggcgtgctctttcgcaagaccgggcccagcacggtcgactggccggtggatccgtgccagatcagcgacgaccgctacccggtggtctgagccgcgacgctgcgccgcgcgaggatcgacagcgcgggcccggccgggtggtcgggctcgtcattggcgatgcgcacgtcgtcgaagccgagcgtggccagcacctgcagcagcgcgtcgcgttccatccaggccggtgcgtgcacgagcccgccgcagaagatcgggtcctgctgctggcccgggccgtagggcacgcgccggtggtagcgcacggtgcggccgcgccaggcgatgttctccacgccggcgaccaggtcgcggcgggcgtcgccctgcggcattgcggcgtcgtcgatcacgtgtgtccagagaaacaaggtgtccgtgcgctcggccagcgcctccagcagctggagcggattggccatgtgatagagcacgccgctcgcgacgatgagaggccagcggcgcgcatcggcagcgaagaagcccatgaagtcgcccagcacgaacgaggcgtcccgcaagccgcacagttccttgacgatcaggcacttgagaaaggcctgcctgttggcctcgatcgcaagtaccgagcgcgcgcctgcctgcagcagcgcggcggtgtgcgcggcctccagcgggcccagctccagcacgtcgcgaccctgcagcccgccgagcgtttcggccagccagcgcatgcgcacgtcgtcccagaggtcgctgcgcgtgccggcgctcaggccgagcgcgggtggcaggctgccgacccagctgcctcgcatcaggtccagcgcgttctgcggatgaggcgagcgcagttcgtaggcggcctgttcgggcgcgccgccgtcatgctcgatgttttcgcgcatcgcctgttgtgccagggccaaccggtccaggccgctgccgcgcgccccgcgctgcagcaccatcaaaaactcgcaacccaggcagtcatggaagaaggtctcgcccagcgagatcaggccgagctcgcgcagctcctgcatgatcaaccggaagctggaggccgtgaacacccaggcatggcaatcgcggtaggtggcagggtcggcgcccagcgcgttgtcgtagcccgcatgcgccacgccgggcatgccgaaggggcccggcgagcccggtccccacacggctgcgccgccgcgcgtggcgctgtaggccgcctggtcgtagagcgcgcccacgttgtgccggcggcgtccgtcgacgaaggcctgcagcacctggccggtggtcgagaccgggcggaagtagtcgaaggtgtagcggcgatcggggatcagcaggtacaggcggcccgtgtccgacagcgcgcgctcgcagcgctgcaagaaatggatcgggtcggtcaggtgctcgaacacgtggctggcaacgatgtgcgcgaagcgctcgccgggcggcagcagcacatcgagttcggcaccgtcgtcgatggcgtccacctcctcgatcatcgcgacgtccacgttcggatcgtccgcgtacttgcgccgcagatcgtccgcgcttgcatggtcgaccaccgacacgttgaagccggcggacttgcgcaggatgggcgagtaggaggccccgaactcgagggcccgttcaccgggcgcgatgtgggaacggatgtggtcgcggaagttcatgggtgaagcacggctgtgcgcggggcgtttcaagatgtataagacccgcagtgtggcccagaagggccggctttgaccaaccggtgtgcggagacctcatgcgattgatccattccctcctgtccttcgcgcgtcgccgcaccgtccagacggttcttggctgttacaccgcgggttcgaagctgctgcagcagccggccgtgcgccgcgagcgccggccgcgcttcgaatccgacaaggtcgtggtgccgccgcatggcgaggtgtatgcgatcgtggtcaagtacgccggccatggcgaatcggccaatctgcatgtgctgctggacgcattgcggcgcgccaaggtgaacacggtgctcgtgtgcaacggcgaggtgcccgcggaggagctgggtgcgctctcgcagcgggttcaccgggtgatggtccggcgcaacgtcgggcgcgacttcggcgcctaccgcgccgccacgctgagcctgctgtcgcagggcgtgaagccggaacggatgatgtacttcaacgacagcctgctctacatcgagggcaccgagctggaccgcctggtggccgagttcattttcagcgagttcgacgtggtcggcctgggcgagaaccagtaccagcatcacatcggctcctttgcgctgtccgtgtgtggcgccgcattcgtacatccagaattccgccgattctggcaggactacacgccttacgacctgcgcaagcacacgatccacgccggcgaattgggcctgacggccatgctcaagaggctggcctgctcgatcgacgtgatctacgacgcgacgcggctcgcccgcaagctgcgcgacatgcccctgcacgaagtggtggacgccacgcgatggctgccttacggctttcgccggcatgtgctgatgaccgtgctgggccagtccttcagtgcgcgcgaactgatcctcaacgccgacgtgcctagcggcggcgttgccgcaagcgacgcggcgatggccgatccggggcccgccggcacgccgacgctcggtgcattgcgcagcctgcgcgaagcggacggacgcgtcgccttgctgggccgggatgcgcccgcgtacgcggcgccgaagacgagcgaagcgcacgccatggcacaaagcgcgcagcggttgtcgcgccagctgctgatcgatcacatcctggagcacgtgaccaacggcagccagctgcatttcggcttcggccttttctatcgcctgctgggctgcccggtggtcaagcgcgacctgttctcgcgcggcctgtatcgcgagcacgactgcgcggacatcctggacaacgtgcccgcaccgacccgccagcgcctgctgcgagacctcatcaaccggggtcgcctcgacatgcagctgggcttctggcgcgggctgctctttcgcaacggcatgctctgagcccgcgcagcggttctcgaagccgcaaccggtcgccgcaagaaaactacatcgccatcacgacgaagaccttgcgcagggtctcgtgcacgtgccactcgccggtggtattggccggaaagaacagcgtgtcgcccgcgcggatgttcaaaggttcgccggcggtcggcgtgaaggtgcaggcaccagtgaggatgtgcatgacctcggcgttgggcaactggcgttcgaagcggccgggctcgcattcccagatgccgctgtcattgccccctgcacccgccagctcgacgtcgatgccgcgtaggcggcagggcggctggctcagcgggcgcgcgggcgtgccctggtcttgcaggccgccgatggtggcggactgctgcagaacggtgatgctcatggtcagcgccccgcctcgacggcatcggccagctcggccagcgtgtggaagtggtagtcgggttcggtgcgcttcgactcgatggtgccgcccgatcctttctgcgcgtggcgacgctcgatccagcaggtggtgatgcccagttgcttggagatgccgatgtcgtggtactggctttgcgccacgtgcaggttgtcggcctgcttgtagccccatgcgccttcgaagcggccgcgcgcataggcgaagtagcgcgcgtcgggcttctcgcacagcgcatcgtcgcagctcaacagcatgtcgaagggcgagcccagggtcttgtcgaaatgggccagggcccaatgctgcgcgttggtcatcgtgaccagcttgaagcgcttgtgcagccgctgaagtgcttccaccgaatccggaaacgcgggccactgcgccaccgaatcgcgcaggccttttgccagcgcatcgctgtcgggcaagcccagtgcgggtgcgatggcgtgccagcagcgctccaggtcatcggggtaccagcccgcgttgccgtcggcgcgggcggcccggtaggcggccagaaagtcgtcgtcgctcacggcggcatcgggcaccgccgagcgcaggtaggcgagcatgccgccttcgaaatcgatcagcgtgccgaccacgtcgaaggtgaggaccttgaaatcttgcagggacatacgagagaagctccggtggaaaggggaggaaggcgccgccgcggcgacaggcgagggggtcgtgcgctacaagcataggagccatcgcgttcccgttcacatcgaattgggcttgcgatccagcacaggatttcgcagtcgtgccgatgtcagcatcttcttcggcgcgacgccttcgcgacgcggaactgcctgaagttcggatggagcgttgcactgtcccttttcgtgacaggtgctcgccgcagcacgcatctctgttgcagtctggcgcagaaaaccgatccgtttgctgcgccagatcgggcccattgcgttcaagcccaggtggcacggcgcgtgcaatgcagcacaccagcggctgcgcggcatctggtttgcgcggtcgccttccacccctacccaacggagacgaaaagaccatgcaatacgccagccccaacgcccccggcgcgaagatcgagttcaagccggcctacgacaacttcatcaacggcaagttcgtgccgccgctgaagggccagtacttcgacgtcatcacgccgatcaccggccagccctacacccgcgcggcccgctcgggcgcggaagacatcgagctggccctggacgcggcccacgcggccaagggccaatggggccgcacctcggcgggcgagcgcgccggcgtgctgctgaagattgccgaccgcctggagcagaacctcgagttgcttgcctacgcggaaaccgtggacaacggcaagccgatccgcgagacactcaatgccgacattccgctgaccatcgaccacttccgctactttgccggctgcctgcgcgcgcaggaaggcgcactgagcgagatcgacgagaacaccatcgcctatcacttccatgaaccgctgggcgtggtggggctgatcattccgtggaacttcccgatcctgatggccgcatggaagctcgcgcccgccattgccgcgggcaactgcgtggtgctcaagccggccgaatcgacgcccgtgagcatcatggtgatggccgagctgctggccgacctgctgccgcccggcgtgctcaacatcgtcaacggctacggccgcgaagccggcatggcgctggcgggcaacaagcgcatcgcgaagatcgcattcacgggctccacagccacgggccgggtcatcgcgcaggccgcggccggcaacctcattcccgccacgctggaactgggcggcaagagccccaacatcttcttcgaggacatcgccgatgcggacgacgacttcttcgacaaggccgtcgaaggcctggtgctgtttgccttcaaccagggcgaggtctgcacctgcccgtcgcgcgcgctgatccaggagtcgatctacgacaagttcatggcgcgcgcgctggagcgcatcaaggccatcaagcagggccatccgctggacaccgacaccatgatgggcgcccaggcgtcggccatgcagatggacaagatcatgagctaccttgcgctcggcaaggaagagggtgcgcagtgcctcaccggcggcggccgcgcgcagctcggcggcgagctggcgggcggctactacatccagcccacgctgttcaagggccacaacaagatgcgcatcttccaggaagagatcttcggcccggtgctcgccattgccaccttcaagaccgaagccgaggcgctggagattgccaacgacacaccctacggcctgggcgccggcgtgtggacgcgcgacggcagcacggcctaccgcatgggccgcgcgatccaggccggccgcgtgtggaccaactgctaccacgcctatccggcgcatgccacgttcggtggctacaaggagtcgggcatcggccgcgaaacgcacaagatgatgctcgaccactaccagcagaccaagaacctgctcgtgagctattcgccgaagaagctcgggttcttctgagcgcgcagcggccgcgcgcgcatccggcgcgcggcttgctgcacgaggagcgctgccgctacttgccggcggccgcgtgcggcttgctcaaggaactggatgcgttcacgccggcatcctcgtcgacgccgaccgcgagccggtccaccagttcaccgccgagccaggccgtgaccagcgcgatggcggcacccgcgaaggcccagaccatctggcttggcaccggggcatagtccctgtcccgcagcaagaagctcacggcgaagagaagcagcaccaccacgttgccggctccgtgcatggcgccgatgcgcttggcgcgcgttcccgctggaatgcccagccagtcgatggtgccgaagggcgcggcgagaacaccgcccaccaggccagccgcgatcatccaataagacacggccgccatgacctggctcctgccccccaggtagatgaggtcgaagaccaccgccgtggccagcagccccagcggaaagaccaccagcatctggtgcaccgagtggccgaggaaacgaactcttgcatgcatgggattacctccattgcctgactgagccctcatctgagccacaaccaccgacatcccgcgcgggccggggccgccagtcggggtcggtactttcctactagcgaaggcgccaggcgccgactggatagacctacagcgtagacggatgcaccgctctatctacaatggagcccatgcaccgggttcgccttttcgtcctttggatcatgatgtttgccgtgcctttccaggcctacgcggcggcagccatggtcttttgcggaccgggccatgagggtgcggtggccgcggcgccggccggaccggcggtgcacggcgatgggcatgcggaccatcgtcacccccacgaagccgccgcgcaagatgccacgcagcccgcgcacgacagtgccgacaccaccgcccatgcagcgcccgatgccatgcacaagtgcggcacctgcggcgcctgccatggcaccgccctgatcagcacgctggaactcgcggtgttccagggccttccccgcgccgacctgaccgagcccgccagcacggtggccacggtcccgccgcgccttctcgacaaacctcctcgcgcctgaagcgttcgtgcgcctgcgtgcggcccggtcacgggctgccgcgagcgcgcatgcatcgcctgcgtcatgcctgccccatgggcagcttcgacgcactcgttcatgaactcgcgaggacgccatgttccattcattgccggccgcttggctggccgcactttccgctttcgcggcgctttccgccgcggcgcaacccgcgcccaccgtcctggactacaagtctgcgctggagggctaccggccctttgccgacgtaaagccgatcccgtggaaggaggccaacgagacggtctaccgccgcggcggctggcaggcctacgccaaggaggccgccgaaagcaccccacccgctgcggccgaaccgcccaagggcgcagccgctgaacctcaggcgcagccaggccatgcgatgccgatgcctgcggccaaggagaagccatgacgcgcgccttgcgcctgacggccgtcgccgttgcggccgccttcctggccggctgtgcttcggtgggcatcgacgatgccctgcaggacacgaacatccaggcgcagcagttcaccggcggcaagctcgaactcagccgcacgcaggaacagcgtgaccgccgctcggcgctggcgcaggagctgctgtccaggccgctctcgcagagcgacgcggtgcagctcgccctcgccaacagcccggccgtgcaggcgctggtcgcccagagctggggcgacatggccgcggccgaccaggcgggcaggctgcccaacccggtcttcaacttcgagcgcatgcgcatgaacagcgagctcgagatcgggcggctgctgtccttcggcctcgtcgatctcatcctgctgccgcagcgcctgtccatctcgcgcagccaatcgacccaggccaaggtgcagctcaccggcgccgtggtcgaccaggtgacgcaggtgcgccaggcgtgggtccgcgccgtcgccacgcagcagatgctgcagtacgccgagcaggtcaatcgctcggccgaggccagcgcggaactcgcgcggcgcatgcagcagatcggcaacttcagcaagctccagcgcgcgcgccagcaggtcttctatgccgacgcgaccacgcagctggcgtcggcgcggcatgccgccaccgccgcacgggaggagttggtccgcgcacttggcctggacgacgcgcaggccgtccggctggccttgcccgatcggctgcccgatctgccgaaggcaccgcgcgaggccagggaagtggccgccaccgcgaccgagcagcgcctcgacgtgcagcttgcgcgcgcgcagctggacgtggcgggcaagtcgcaaggcatcaatctgctgtcgaccttcatcgacgtggaggtgggcggccggcgcgacacggtgttcgacaacgccgaaggcaccaagagcacgcggcgtggcttcgagctcgacattcggctgccgctgttcgactggggatcggcgcggcgcgatgcgctgaatgcgcaatcgctggccgcggccaatcgctacgacgccacggtgcgcggcgcctcgtcgcagctgcgcgaaggctattcggcctaccgcacggcctacgacatcgcgcggcactaccgcgacgagatcgtgccgctgcgccaggccatggccgacgagaacgtgcttcgctacaacggcatgctgatcggcgtcttcgagctgctggccgaagcgcgcgaccagatcgcgagcgtgagcaacgccatcaatgcccagcagcagttctggctggccgatgccgcgctggcggcctcggtgatcggcaaacccacggccatgggtgcttcgaccgccagcgcgggtggcgaagccgcctccggcggtgcggcccactgagcgcagaacgtgcgctcatcaacgattcgaacgacatgacaaacagacgcaatttcctgagcggcgcaggtgccatcacgggtgccatcgcggccgcgagcgtgagcaaggtggccatggccgccttgcccgagcccgtgctccagaccaagcccgacaccatgccgccgctcgtgccatcgggcggacgcccctacaaccccgtggtcacgctcaacggctggacgctgccttggcgcatgaacaacggcgtgaaggagttccacctcgtggccgagccggtggtgcgcgaaatggcccctggcttcaaggccaacctgtggggctacaacggccagtcgcccggccccaccatcgaggtggtggaaggcgacagggtgcggatcttcgtgaccaacaagctgcccgagcacaccagcgtgcactggcacgggcagcgcctgcccaacgggatggacggggtctccggccttacgcagccgccgatcaagcccggcaagaccttcgtctacgagttcgtcgcacgccggcccggcaccttcatgtaccacccgcatgccgacgagatgacgcagatggccatgggaatgatgggcttctgggtgacgcatccgaaggccgagcatccgctgatcgagaaggtggaccgcgacttcgtgttcttgctcaacgcctacgacgtggagcccggaagcgccacgcccaagatcatgacgatgctggacttcaacctctggtcctggaacagccggatcttcccgggcatcgattcgctcaacgtgaggttgaacgacaaggtgcgcatccgcatcggcaacctgacgatgacgaaccatccgatgcatctgcacgggcacgaattcctcgtcaccggcaccgacggcgggccgacgcccaagagcacgcgccactacgaggtgaccaccgacgtggcggtcggccagatgcgccagatcgagttcctggccgacgaggagggcgactgggcctttcactgccacaagagccatcacacgatgaatgcgatgggccacgacgtgcccacgctgatcggcctcgaccacaaggacgtggtcaagcagatcacgaacctggtgcccgactacatggtgatgggcgagcgcggcatggccgacatgggcgagatggagatgccgattcccgacaacaccgcgcgaatgatgaccggcgaaggaccgttcggctcggtcgagatgggcggcatgttcagcgtggtgaaggtgcgcaagaaccagaaggccggggactattcgaaccccggctggttcaggcatcccaagggcaccgtggcctacgagttcgacggctcgccgcccgaaaccgcgcgtcggcgcgatggcggcgcggccgcgatgccggcgcagaacatgccggcaaagaacatcgaagtgaaggttcgcaagcccggcagcgggcatgcggggcactgactccttttatccgtttctctctctctctctttttcaccaacccccaactctcagaaggaaatcatgaagcacatcctccgcaacaccgccttcaccgcgctcttcgctcttgcggccgcagccgcctctgccaccggcaatcacgccggcggccatggcgacggcgacgaagccatcggcaagcccggcacggccgccaaggccacgcgaaccatccacgtcgacatgaccgacggcatgcgcttcacgcccgctgacatccgcgtgaaacagggcgagaccgttcgcttcgcagtcaagaactcggggcagctgaagcacgagctcgtgctcggcaccgagaaggagctcaaggagcactacgaagccatgaagaagaacccggagatggaacatgccgatcccagcatggtgaccctggccgccggcaagagcggcgagatcgtgtggcagttcaccaaggccggcaaggtcgactttgcatgcctccagccgggccactacgacgccggcatgaagggcgccgtgacggtcgccaagactgcggccaagtaaacccgacaaactttcaggagatacacatcatgtcgaagattcgcatttcactcatggcggccatggccgcattggcattcgggggcacggcccatgcgcagtcgcccaagtccgacacgcccggcacagcccaggccgcggccccggaactcaccgacggcgagatccgcaaagtcgacaaggacagcaagaagctcaccatcaagcacggcccgctgaagagcctggacatgcccagcatgaccatggtctttgcagtgagcgacgaatccgtgctggacaagttccaggccggcgacaaggtgcgcttcgatgccggaaagatggacggcaagatcgtcgtcacgcgcatcgaacctgcgcgctgagctccaaaacaaacgcgccttcggggaaggccgcttcgcatacgaaatcgtcccaccgtgaagaattgcggacccctgcattatttggcgtcctgattggcttgtcgccgacgtggcgcaaagagtaggcttctttccggatctcgagatccggaacagacgctgactttgagccaacgtcgtgtcctccaaaaaggcacccaaccgatcgaagactttctgtcatcgatcttgggttgcgataagaaatcagggtgaaccaacaatgaagaaatgcaatgttcggcgtgcagccgccgtgctggccgcgagcgcgtgtgtgagtctgggcgcttgcgccgcgacccctccggagccggccgccgggaactcatgggagctggtggtggcccccttcacgcaccattggcacaaggacgcagaacaccgcaacgtcgttcttctcgggctggagcggatttcacctgacgggtcggcggtgggcggtgcgctcttcaaaaattccttcggccaggtctcggcctatacgtactacggccatgagtggcatggactgctgggctccgactcgctgtacttcaagttgtccggcggcatcatctacggctaccgtgggcgcttcaaggacaaggtgccattcaacgtcggaggcttctccccggccatcattccggccatcggctggcgcctgacgcccagggacgcgatccaggccgcggttcttggcaaggcgggggtgaccttctcctacaaccgccgcttctgacggaccggtgcccgaccgggcaccgcacgctaccccgccaacgcgcacatctcggcaatgagatcggccttgccctcgaagccgatgccccggcagcggcggcagcatgacgtagccgttctgcaccttcacgccgtcggcgttcagcccccaggctctggaaccgtggagatggcgcttcggcggtctatcttccggctcagcacgatggacgtctgcgtctggttgatgccgtcgagctggccgagctggtccagcaggacgtccagcttttcgggcgtgtcgcagcgcaggaagagcatgtagtcgaactggccgctcaccgccgaaagttcttccacttccggcacgcgttcgagcgcccggatcacggccggagcactcttcgcattgacgctgatgccgcagatcgcgcgcaccgcggcatgctccagcttctgtccgaggcgcacgccataacccgcgaccacgccctcgcgttcgagccgggcgatgcgcgcgacgacggtggtgcgtgcgatgttgagctttcgcgccaggttggccgcaggctcgcgggcgttggcctgcagcaggctcaacaggtggcggtcgagatcatccagtcttccatccatcgaacggtctcctcaaatcggaagtgatttgaccggcatgctacggcagtgcgtgcatggacagacatgcggcggcccgccgcggcggtccgccacccgcgcggagcgcgctcaggcttcggcggcttctttgtgcgcggggctcgacgcgctcacgccaaggccctggtagtagtggcccacgcgcgtcgcgagaaactcctcgagcggtgcctgctcctgcccgacgaatccgcgctgcggcagcttgccctgcaacagcaactcgagcacgccgaccacgccggcggccgtggtgagctcgatggcggtgcgttccttgccgcgaagcgtggcgccgaagacgcggcccacgcgggtttcctgctcgaagcgcccctcgcgcagccccgaggccgaagcgaacacgatgacgatgtcctcgcggctgtgcggcaccgcgtgctcgagcacctggcgcagcaggtcgcggcgctcgatcaggcgcaggtcgtgcagcaggaagttcatcgcatcgcgatggcccggatagcggatggtcttgtagtcgagattgcgcaccttgccccgcaaggtctcgcacaaggtgccgagcccgcccgaggtgttgaaggcctcgaaggcttccgcgtcgagcgtgaaggtctcgtggccttcgagcggctgcaccgaaacgagctggccgttcacgatcgcgtcgcaggcgttgcagtattcgttgatgacgccgtcgatgctccaggtgaagttgtagcgaaggctgttggtggcattgcgcgtcagcgcgccgacgcgaaggcgcaggtcgtacagctcgtcgaagtgtcccgccagatggccgccgagcatcccgatcacgccgggcgccaggccgctttgcggcatcagcaccgagatggcttcgctggacagctggcggatggcgtgggtcgcggccacatcctcggtgaggtcgaagtagtgcacgcccaacttggccgcctgcgtggcgacgcgcgcggcgaggaagaagggcaatgcgttgatgaccacggtgtgcgatgccagctcgctggcgagcgcggtgtcgtcttccacgttcaacgtgatccgccggaccagcgggtcgctggagggcttgcccgccagttggtcggccagcgtcacgggcacgcggtggtattcggccaccatgtcggccaccgtgctgcccaccttgcctgcgcccagaaccagaacgttcctgagttgtagctgcttcgacattttgtttctccaaggagcaaagagagagggctccgtgaagaaaaatatagaagcaatggctggcagctgccagagcgcagaacgtcgaaagcgctggccgtttcgccgcttcgaccaactcgggtgacgattcgaggtgccgcctcgttcgatccatcttcgaatcaggaacccggaggcaggttgttcattcgcgttgagcccggaacgcggcttctccggcgtccgacacctcgacccatttcttgtcgggcacggcttccgcggtgtagttgtcgtgccagttccaccacttgtaggtcggcgtctgggggtagccctcgggcgagtcttcccagacctcctgccggcccagcggcgtgatgtcgaggtagttccaggtgttccccatctgctcgtcgccgcggttgttggtgaagtacgtgcgaaacacgcgatcgccattgcggaagaacacgttggtgccgtgccactcgtcgacgccgaagtcggcgtcgaaactgtcggtgagggtgaaccacggaatctcccagcccatgcgtgacttgaggcgcgcgatttccgtctgcggcgcacgcgagacgaagacgagggtggtgttgcgcgcgttcaggtgggcgacgtgggcaacctggtcggccaccatggagcagccccggcaggcgtggtcgggccagccgaacacgccgggctcgaagaaggcgcggtagacgatcaactggcgccggccgtcgaacaggtcgagcaggctggccttgcctgcgggtccgtcgaatgcatacgctttttccaccgccacccaaggcattcgccggcgctcggcggccagcgcatcgcctgcgcgggtgtgggccttttccttcacgagcagtcgttcgcgcgcggcctcccacgcctggggcgacacgacaggtggtgtcttcatgatgggctgttcgcctttgcgtccgttctcggttgaggtagtcatcgctcaaatctcctggttgggcgaactcccgcgcctcatggccgaagcgcgattcatccgctgcttgttgctcatcgctcgttgtcgagccgggagagagacagtttggcgccgcaagtcgaaggctgggagtaacaagtgtggcgggattgaggaagcgccgctgcacagcatgctctgctacgatctggtcacgggaaaacagcctcccgttctgcaaggtcagacggtgtcccgtccaagcgctggtgacccatgacggagctatccgtggacaccaccttgcccgacgcacttcctgcgctttccgcacccctccaacctgtttacacgcaggacgcgcgatgagcgccaccccctcgtcccggccccgcaaccttcttgcgcccctgctgcctcccggggccgatgccggcgccttgcccttgcttgccgcgcgcgggctgcgcgcgtttggcgacgggtacatggccgtgctgctgccggcctacctgctgtcgatcgggctcggcacgctggaggtgggcatcgtcagcaccgcgacgatgctgggttcggcgctcgccacgctcgcggtcggcgcgtggggctatcgcttcccggccggacggttgctgcgcggcgctgccttgctgatggcggccacgggcctcggctttgcgggcctgtcgtcgttctggccgttgctggtcgtcgcactggtcggcacgctcaatcccagttcaggcgacgtcagtgtgtttcttcccctcgagcatgcacgcctggctgctgcagcacagggccatgcccgcacggcattgttcgcgcgctacagcctctcgggcgcgctgtgcgccgcgttgggtgcgctggccgccgcggtgccggactggctggttcggcacagcgagtttgcgcggctcgacgcgctgcgcggaatgttcgtgatctacgcggccatcggactggccgtcttctggctctaccggaatctgcccgcgcatgcgggtgccgacaacgcgcagagcgtgccgcctgtcgcaccggcaccgcttgggccatcgcgccgcgtcgtggtgcgattggcggcactcttcagcgtcgattcgtttgccggcgggctgacggtcaactcgctgatgtcgctgtggctgctggatcggttcggcttctcgctgacgcaggccggcgtgttctttttctggaccggcttgctcggtgccgcgtcgcagcttgccgcacccgtggttgcccgacgcatcggcttgctcaacaccatggtcttcacccatttgccggccaatgtctgcctggtgctggcggcgctggcacccagcttgccgatggtgctcggcctgttgatggtgcgcagtgcgctgtcgtcgatggatgtgcccacgcgcaccgcctatgtgatggcggtcgtgaccccggcggaacgcagcgctgcggcaagtttcaccgccgtgccacgcagcctggccgcagccatcagcccgacgatcagtggcgcgctgttcgcggccgggtggatctcgctgccgctcattgcctgcgggctgctcaagatttcctacgaccttgcactctggcgggccatgcgacgggatcgagtcgacggcgagtgaggagaggagggcttgcagtgccgcgcgcaacgatgtagaacgatggcgttaaaagtcaggttcgcaagcacttcgaacagatagcacgctggtccgaaaggagatgaagcatgttggcagccgaatgcgcgtgggccatcctgcgcgccgagcacgctcgcacccgtgagttgttggctcggctcaatacggcgatgaagacggaggaagacgaggcgtgcgtccggcgacgggcgaccaccgcgctcagagtcatcgaacggctcgaagccttcgaagaagcaacgcatcgccccaagggcgtcgtcatgctggacatactgcgcggaaggtcgagcgaagccgacgagcttctcgatcaactcggctccgaaagcgaacactgcagcggccttctctcgcaagccaagctcgtcttgaagcttgccgaggctggcgacatgaacgcagcagccaaagccgaagccttgttgcaacagcaccggcagatcatgtacgcgcatctggacaaggaagacacgcttttgcattcgcaaacggcgctgctgctcacggctgaagaatgggccgccgtggtctcgtccatttcgaaggaggtacgcgccgcgaaagaacgtgaacgtcggcggccgcagcagcaaccgcacaggcaagtctcgaagcttgcgtcgtgaggaaggcagccaacagggttcagctcggctttgacgactgccttgcgccggtcctgccgtcgtgctcaagacctcaggttgccggagggcgtgtgttctccagcaggagggtgcgcaacgcgcgtttgccgcgcgcgttctgagttcggtaggcttgtcgcgccagctcgacgaagcgctcctcccccgcatcgggcagaggttctgctgcactttgagccgcatcgagccaaagtgaaggcttgccgcaatgggtctcgatctgccgggccaacttgtccgagatcacgcggcccttcttgatctggctccacatgctggcagagatctggagtttctccgcaaacttggccgccaagccaagtggctccgccccattggacgcatgctccgccacaaagtcgccgaagagaaggaggacgttgcttcggcgaagggctgggagtgacatgcttcggaatgcgtgccgcagggcactgtgatcaacggccgcgaacaacgcgatcgtggtgagaaaaaaacacagcgccgcaaaaagatgttgcgcggtggagtaaacccagtttacattacatccatcgacgaaattgcttcgtccccgtttcatccgcaacaacttcgattcatcgagaactcgccaaacactggaaccatcgtgaaagcaaacttgacctcactgaacattcgacccgcatcgggccgggcgttcgtgcgcgtctcgttctgcggtggtcgcagcctgacgacatccaagatgcattcgcagctgaactcccttcccgcgatcccggccagcttgtggcttggacagcagtacgaggatcagccgcacccgggtggaggtagcgcgtaagcgcgcaccttccaagctctctcaccagaggcccggattccgaaatggatccgggcctttttgtttttctcacctcacgttgcggatctcgatccgcaccaaaccgcgaatggcgctcactggtgccggccgccacggcagtgatcgcgctgccgtgaactcacccgccaaatggcgccagtgggtgatccttaaaaatttgccgcgagtcgcgcccctcactggtggggcgaacgatttgcaaaaaacttgcagccgtagctcagtcaggcagagcgcaacgtcgccaacgttgaggccgagggatcgaagccctcctgctgctccatttcgggtgtgcctttgcagcacctccagaggccaaccgcgtcggcggcctggagggatgtgcacggtctggacccaaccatgtgcagcgatgtcgacgtgagcgcgcaagcgctcgaatcgcgtgaagacacaaccgaaatggaatgccccgatggcggaattggtagacgcaccggcctcagaagccggggacgaaagtcatgagagttcgaggctctcttggggtaccaccagcttgttgagtgcctagttcaattggcagaacaccggtctccaaaaccggcggttgaaggttcgactccttcggtgctcgccagtattcgccttgccagtagcttggcacaaacaatttgccctcgtagctcagcctggcagagcaactcccctgtaaggagacagtcgtccgttcaaatcgagaccttgggcaccagatatcgaacaacgtcgtgttcgatcgacagttcagatctgtcctgcgcacccatccataggccgttcgccaagctggaaccaaggcacctgactttgactcaggcaatcgcacgttcgaatcgtgcacggtctgccaggagcatgccaaatatcggggcgtagcgcagttggcagcgcggttgctttgggagcatcaggtcgcagattcgatttctgccgccccgaccacacaagagcgagaccgggcgaattacatcgtcctctcgtggaaaccggcctcaaagattgggaggcgccggaactcgtaaccggacacctttggagcattggccgagaggtccaacgcagcggcttgctaagccgtggtcgcgcaagcggctcgttcgttcgaatcgaacatgctccgccaggatcgatggggatgtagctcaactgggagagcgagtggtccaagggcgctgtttcgaaaacagatggtcggctccgccggtacgagcgttcgactcgctccgcatccgccaacttcatcaaccatttccctcccgcgttagctcaattggatcagagcactggcctacgaagccgggggttgcacgttcgaatcgtgtgcgcggggccatacacctggagtgcgagcagcatgggtgactgcactggactgtaaatccggcgtccttgacgtacggggttcgaagccctggcactccaccatgacatgcgggcctggccgagcggctaggcggcgcccttccaaggcgttcaggcgggctcaactcccgcggcctgctccaccccctgcgtcgtgccgaatggcctggtacgcatcgttccagtttcaggcatggtatgcatcgttctgcaattgcgtgaactcgccttccttcgatctgccggccagcacttcggcccaatcggccgagttgatgcaagtaccttcgcggttggtctgggcctcagagtcgcaagatcggctaagcaggccgcccgccgtagcgacatacttggcagtaatgagaactgatcgagccgaacagaattacagggaccgtgtcgcgcgcatcgttgcagtgatcgttgccgacccgatggcagagcatcgcctcgaagatctggcgcgcatggcgcatttctctccgtatcacttccaccgcgtttacagcagcatcgctggcgaaaccgttgctgcgactgtgcgtcgcgtgcgcctggcgcttgcgacacgtttgttggagaacggtgccgagagcattacccaggttgctctggccgtaggctatgacagcccgcaggcgttcacgcgtgccttcggccagttcacgggccagtccccgagcgagttcaaggggcagatgcaccggctggagttgaacgccggccaggcacggcgcgaatctgacactcagacagcaccaaccgtgcggatagtcgatcgccctgcgcagcgtgtgtatgccctgcgacatcgcggaccacttgcgaccattcctcacacgcaaaggcgcctgcaacttcattccgccaccaacgccgtatcggaatcgcttggggtgtcttacggcgatcccgaggacgctgagggcttcagatactacgctgcggccatatcgcccaagccttggccggtcgtcgacgcaggggtcgaaatgctcgacatcccggccggccgttacgcgctgcactgcctcgccggcccttacgcccgcatcagcgcggcgatcaatgcgctctacagccggtggctgccgagcagtggtcatgaaccggacgatcggccgacgttggagcactatctgaactctccgcgcaccgccgtccaggcggacttgcgcaccgatctactgatccccattcgtttcgcgagcgcccaatgagcctgacccgtctcttttctctcgccaccacactgtgcctggcgacaaccttgacgcatgcggccggcttcagcttcatcgaggtgcccacggccaatgatggtcctgcgttgcgtggcgcggtttggacgccctgcaaggctccagctggccgcatcgcgctcgaccccttggtgattgatggagtgaaggattgcccgatcgaaggaacaaggctccccctcatcatcgtgtcgcatggtcaaggtggctcactcctcgggcatcacgacaccgcgagcgctctcgcggacgctggcttcgtcgtcgcgtcgatcagccacgcaggcgacaacttccaggatcagagccgccgggacgatctgttggttttcacctcacgccctgcggacatgaagcggttggccgactacatgctcgggggctgggctggaggtccgaagctgaatccggatcgagttggaattttcggtttctcgcgaggaggctatacgggcctggttgcggctggcgctgcgccgaacttcaagctgcgcaaggatctttgcccgccactctcgttcggaccgctttgccggaaaatccgtggcgatgagcaaccccctctgcctgtgccagacccgcgcatcaaggcggccgtgatcgtcgatccgctgagtttcttcaatgccgaagggctgaaaggtgtggcggtgcccattcaactgtgggcttctcaacatgggggcgacggggtcacgccggagagcgtggaagcagttcgccgcgatttgcccaagcctcccgactggcatgtggccgccaacgccgcacacttcgcctttcttgcgccctgcgcgcctgcgctcagccgggctgcgcccgagatctgcatcgacaaagacggattcgaccgcgtggccttccacggcgcgttcaacagcgacgtggtgggcttctttcgccgcactcttcaatagctcgcaggtcggcgaacgcctgcttcggagcccccagatgtctgcatcagcacctgggtaacatcgagctgcacacgaaggccacggggttcttggtgacatggcgtatctggaggccaagcagttgcagagtcaaggcaagtatgtcgagatgcggaagatgatggacgacgccacaaacgcctgcgcgcgaggtggccagtgaaacgcctggcggctgggctgttgtcgctcgtgatggcagcctgcgcagccgcgccattgaagcgctgccccgagcccccggaaggcaccgacttcggcgactactcagatgaggcggtcaaacgtgccacccgggatgctccggcgatcgcctttgttcttggaaaagggcggcgtgccgagcttgccgggctgctggcgcgcggagacgaccccaacgcctgcctctcgggcatcagcatgctggccttcagcgcgtcattcggcgacctggaggaagtgcgcatgctgctcgatgccggtgctcgaacggaccggccactcgacagcggcggtgacacgcccttgtttgccgcgctgagcagggggcactacgaggcagcggagctgttgctggcccgcggcgcaaacccgttgcacgtcggcgacctcggcgcgacggcgttgcacaggatgtccatggcgccggtgcccacgaacgatgcaggccgcgcacagcagcaccgttgggcggctcgcctgctggcgcttgggttggaggtcgatgtccgcctccatcggggcgccacaccactgatgcttgccacggccatgcgcaaccgagaactggcgggcttcctgcttgccggcggcgcggacccgaatgctcaggacaaccgtggcagctctcccgtctcgctcgcacgaaagcgtggcgatgccgattggatcgaactgttcgagcgggcaacgtctgcgggaaaagtttgcccatgagtctgtcggaaaccgaaaaccagacccgcgtgttcttcgacgaatttgttgaggccttccgttctttcaacggaagcggaggcttgggcacacgacgcaatcctgccggagctcgttgggcggtgccttgcaggcagcataggtcgcagcgttacgcttgctcttctctagactcatcaccctttgcgtttttctccaggaggcttcgtgaccctaccgcccgccagtccagcaccggacgtctttcagatcggcagcacgtcgttcgctttcgcggcggatgcgaatgtcgagtttgtcgacggaggcatgcggttcgacctgaaggcggttccggtgcctttcgacgccgcccgccatgaaggtgtcttcgaggtggttgcagggaaggtcgctccccgattcttctccgccacctttcatttcgatgaccgctcggaagagccgcaccgtgtgtttgcctatccggtcgagaagccgcgcgtcgatttcggcctgttcgatgaaggcctgaagtacggcctgaggtttttcgggcaagtcgacctcgcgcccgatcgcatcgcgctgagcggcgtgctgcgccaagactacgaggacgatgcgcaaggcgtcgtgctgcgtgtcgtgtggaacttcccccgcggtgaagtgcggttgcggccacgcaacttcgagagcatcgaagccgccctggcggcgccaccgaagcaggtgcgtcaccttcactggcaccaggaatggcgcgcaccgaaagccgaagcatttccatcggaagtattccgctggacagagctggaatggctttcgatgcagtacgcctccaaggagcacgcccgcttcatcgcgcttccggacgagataggcacgctgcagaaactgacccgcctgcgcctcagcaacaccagcgtgctgcacctgcccgacgtcatcgggcagttgcggagtttgcgtgaactgagcttcacgggcggcgcgctcaagagcatctccgagcaggtcgcgcagctcgagcaactggaagaactcaacctgtcctacaaccagctcacctcgttgcccgagggcatcggccacatgccggcgctgaagacactggacctgcgcggcaacgcgttcgagtcgttgcccgcctcgatcggccgcatcgagaatctccggatcgacccacgccaccgggcgctgtacctcgacacgcgctaccgtcccgaaatcgacgtggcgatggacggtgaagtgtttcttgcgcgcagcagcccggcgcacctggcactgctgcaagccgccttgacgcggcacggcttccttcagcatgagccggcgctgcgccgccatgcccgccaggcactgcgctggcgaaccacaacgcccgacgagcccccggtgctcgggggcacccgcttcggcggcgccccggatctgccccccggcgtggactatcccatgacgaacggccggcactggcatttctatgcccagctcgacctcgagggcgtggccggcttgcagtcctggttgccgcgcaccggacggctgtactttttcgccgagggccaggacggatccgaccggaccctggtgatgcacgacacatcgccccgcgcctctttgcagccctacgagtggggccgcgatgcacgttttgtggacggggacaatgtgcccgaggcctacgcggcctaccgcgccacggtggatgccacggtgtccgtaccttgcctctatggggcatcacaccgctacacgggtgaggacgccagcctgatggagatctggggcgacgatgagcagtacgaggcctacacggccctggaggccgagctcgccggcagtgacgactcgcagcacggcgtgcacctccagaacgcctttgtgttcacccagcaggagagtccggaggagcaggcgatgggcacccagggcgggcagctcgacgagtgggtgaacctgctgacgctgtactccgaccggcatcccggcttcagcttctgggatgccggtacgctcaccttcaccatccaccgcaaggacctggccctgtgcgacttctcccgggtctgtgtttcgctggaaagctcttgacgttgcaccacctgacagccatacggtccatgtacaagacctcttccaaatcgttgtgtcgcagaacattgtttgccatggtgcccatgcttgcttccacactcctccttgcagcgccagtcgatcgccccgcatcgggcagcgacgtggacgagacccgcacggtcacccagcgtcctcagccacctctggactgtctttcgatcacgttgagcggcgtcacggtgcttctcgatcggcaggaactggccaggaaagccgccgtcccgtcctccccatggacgacggaggcagaacggctggcactcatcgaaggcaagcgggcatccgcactgctgtcggcggccgccaccggcaagggtgagaacggttgtacgcaaatcaacggggccttggatggcgaggcgcaggccgtggttttggccgcgctggagagcggcgcctccacggtccttgcggacgactcgaagcatcccatcgccgcagtggccatccgctacctgggcacccgctgcggcccgctgtgcgggcgggggcacatcatggtgtacgtgccagggcaaagcaggccattcctggtgcaggactggtgggtttcttaggcgcttcgctctccttgcacggaggggcgtcgcggcaaacagcatgagcgcctgcagctaggctgcggcggtacccggatcaatcgcgcgatacaaagaacaaagaacatgccttcttggaaacgactcgaaaagctcaacggtggcgatcagatcacctacaccgacccgctgctggacaccccgaaggaagtctggttctacagcgcagactacgaacttcgcatctggcatgacggcgctctggagcggcatgtgcctgcatcactcccactggccggagcggtgcagcagcgcgtcaccttgtaccaccagctgagggaactgttcgtcgatgtggagcagcgagccgactgtttgctggtgcggcgcggcgtcttgaacggcaagtggatcgccatgcagcaacccaccggcgaactcgatgcactgcgggcccggtaccgtgcgctggggtttcaggaggtcacgccgtggaatgcgtcgaagaaccacgtgaccaggcgcgaataccgcaaggacgccggaaccctggccgtcaaggcctggaccgtggaggtggatggaatggctgtcatcgagaagagggtggaaacccctgcgaaggaccgccaggcggccgtgtcgctagccgaggagcgcatcgccgctcaagaagagtcggggttcacgctgcacttgatcgagttgatgaaagcgaagcatcccaacccgatgccgaagcgaaatggggctgcaccagcctcgtcgaaggccctgtctacgctggccaagcccagcaatcccttcgaagcggtagatgcggccgtggcgctgctcaaggacctgcatgtgcggctgccccagatcatgttcatcggcgagtgcctgcgcgatgaggaaaaggaggcgcgggtcaatgacctgggcgaggacgcctcgttttttctggagatgcaccaacagcgcgtcgggcgctggatcgacctaccatcccaggagccgcgcgaggcggagtcgagctgggactatttcgccagggtctacgactcgatcacctggatcgtgagaggtcaggccgatgacggcatggcgatgttctattgcgggaacgtctcgggcggtggctggagttgcctggagatcgacagcgacggcgcctacgacatgtatgagctgatggatgccaccgggaacgacgaactggagcacctgttcgtgttccatggtggatggcacagcaaccgttcctgggccttcgatcagcgcacggtttcccccactggtgaacatgccatcgtcccattcgacgaaggcatggccgaactccctcggcgcacacccgccggcaagatcgttcctttcggcacctggctctacaagcgcgtggtgacgatggccaagatcatggcgcgcaatgcgcatgacctgaacctttgatcggagaccgcctgaccgccgagacgcccgtggaggggcagcctatttcgcgcacctgggtaggatcgaactgcacacgaaggtgatggtgtccgcgccgaagtaaaactgagctacccgtaaaactggctcaacttccggtcggcgccaacacgcttcgaggctcgatgccgtccgtcgacgcgtactgccgacatgcgccccttcagcaccgagcagcacgcgatccaagcgcaccgcaacctcagaacacaccaccatggcaggctactggaccgacctctattcttttgtcgccgcggcgatccgctcccgcgatgccgtatacatcgtgctctcggacgatgccgtggccgcatcgaaactcgcgatgtcgagcgtcacgcagtggaagccggacacgtggggaaacggggggcataccgactggcgcaccgcgggcgtcgccttgacccagcatccgcgcgtgcaactcatcgcagtcagcgagttcggatccgcgttgctcgtgggcggaggcgaccgtcatgaggaagccatcgcctcccccgactcttccccagatgaccgtggcccgctgcgtggcgtgcgttgcgtcggcggcgagatcgtcgtcgtcggcatggaccgccaggtgtacctacgcaagggcgacaatgcctgggtcagcttcgagcgcggcattccccgcaacaccgacccgaaggccatctccggcttcgaggcgatcgatgggcgctcgatggacgagttgtacgcggtgggctgggacggcgagatctggtactgcgatcacggcacctggaccacccaatcgagccccgtcaacacagttctcgtggacgtttgctgcgccggcgacggattcgtctacgcctgcgggcgcaacggcatgttgctcaagggccgtgccggacagtgggaggttctggctcagaccggcttcccggaagacctttggaacctcgcctggttcgacggccgcttgtacgcctcgtcgatggatgccgtctacgtgctcgaagacggcgaactcggccccgtgtacatgggcgaggaccaggccaagacctgctaccggctgaccaccggtgacggcgtgatgtggtccatcggcgcgaaggacctcatgtgcttcgatggcaccgcgtggactcgcatcgactgagctggcacgccaagcccatgtcgatcttgtcgcgctccgccttccccgtcatcatcgagcaacacgtcgaggcggccatgcacctgcacggcacctggcagttgttgctcgacgcgccccatgcccgactgcaccaactggcccgcctcgacgagcgcctgatcgcgctcgctgaagcggtgcccgggatcgtcggtgcattcggttgggtgtcctcgcgtcacttgcgcggcgtcacgaagacgctgctcgactctcccgtcccgctgcgccgggccgtcggcctgcaggcatgcgccgcgcaccgggtcgatccgggcggggtgatcgccgctgcgtgcagcgacgccgacaccgcattgttcatcgccttccgggatcttggcctgcgtcacatctccagccccgccaacacgggcccgtggccttaccaaaacgccatggcgatggatgtcgaggacatccctgcaagcccatggtggatgagattcgggcgaactgtacggatgggcgcgactacggctcagactgctgttccgcacgcaaatgcctggtaatgccaaaggatccaaatcgatgctgcaatggaccggatggcaaacagatgactggccaccatttgcttccatcgaaggagttcgtagcgcatgcggatcgaggttctgcagatgccacaacccaattcgcagtgccatttcatgaaagcttcggattccatgcaacaggtcctcgcgtagagacgaagggcatcgcattcataccgatgaagctcgcgcaagtttgacgtgctggcgcccgatgggtgacagcgaacggacatggctgcgcggcagcggccccaatgtggggcatgcatccccaaatcgggggcaactggcatcttgcgcaccacacttgtttttcagttgaggtgcatgagtcttgtatgccattgggcacgattcctgcgattcaatgccagcagggctcttggcatgcttgccgtgcgcttgagaacaaatcacaactattcctcaccattcaagcatcatgaatttcagcaaattgcacatcgtcttcggactgaccctcatcagtttcatggcaaccagtgcagttcacgcgcaaagcgcgttggacaccatcctgaagaacaagaagatcgtgatcgcggttcctcccgacttcccgccctatggatcaatgggccgagacttcaaaatgcagggactggacatagacatggccacctacatcggtaccaagctcggcgtggaggtcgacctgatacccgtgaccagcgccaatcgcattccgtacttgcagaagaaaaaagctgcattggtcatcgccaccttgggcaagaatccggaccgcgagaagcagatcgactttaccgccgcgtattcgcctttctatcaagccatctttggtgcaaaaactctgaacatcaagagcttcaccgacttgtcggggaagtcgatcgccgtcacgcgcggctcagtcgaggatcaggaactcaacaaggttgcgccagcgggtactgacatcaggcgcttcgaagacaacaccagaaccgtcgctgccttcgtttccggccaggcgcaattgatcgccacaggagcgtctgtcgcgaacaacatcatgaccagcaatccgacgctcgggaccgcctacaagttgctgcttaaagagagtccgaactacatcggcgtggctaagggagaagactcattgcggttgatggtcaacggcatcattgatgaagcgaagaaaagcggcgagctgaacaagatgtcgatgaagtggctggagcgcccagcaggggagttgccgcagtagatattgttgattgccgtcgaaaattgaccctctaaagcagtaagttccgtctaagactgacccacgtaaaaccctaccctgctctttttaaagcaggggatcctaggagtgatagacgtggcgacattgagtgtcatcagacgttgggccctgcgcgagcagatgtccatccgcgagatagccaggcgtacaggccacagagatcggcggaatccaacaccacggcctatcgaagggggtagccacctgggttctctgcctcctcgtcgcgcctggtcggatagaacggcttcttctcgtcgagttcgtagaacagcaggccatggattcccatcgcctgggctttgaccactcgacgtgcccacagcgcttcgaacgcactgttgagagttgcttcgtcgcccccgcgcccgtagacctcgtcgatgaatgcgatgtcctggccatcgggaaagatgagcgcgaactcctcgtcggtggcggcaaagatgtcatacacgcagttcactgcgccgtcgatgacctgaatgttcttcataaaaagctcggaatggagccgacatcgtaggtcggctgctggccgcattctgtccgaatgagcgtgactagaggcttagcagaatcaagaccacaaacaaggctaacccaccgacaacgatgagcgtccggagccatatagcgccgcgaatagccaggctcggaacctgcgcagcaaatgctctcaaccgatccgccaacggatgtcccctcggaagagccgctgcgatcagcagcgacccaacgatggtcaacacggcaagtaagacgagcgcggcaaccgcatagccaaacaccatccaaaaagcctgcttcaaggaacagcgcatgcgccagccgagactgggcacgcgcaagctgcactacctgttgcgcgagccgttgcagcgccagggcatcgagttggggcgcgatgcgaatcgccgccatggcctgaagtgcgcgatgaccgacggctacgactgctaccagaacgcgctggccgagcgcatcaacggcatcctcaagaccgaattcctgctgagccagccaactgacctggctcaagtcaggcgactggtggctgagtccgtgcagatctacaaccacgagcggccccatttgtcgctcaaaatgcaaacgcccgatgtcgtgcatcgggcgtccgtggtcggctgaggccggctatttgggtgtcaacgcaattcaggacgggtcactggccgcgaagcgcgaaggcgccacctacggcggcccgatctggacgaagtcgctgaccgactcgaagttgtcggcggcccacgcgcgcagcgattcaagcgcctcggcttccgatggcccgaaggtctggtggtgttccagaggcgtggaattgacctcgtccggtgctttgggcgctcggcggtggggcatccagtacagggtcgcggtgtagcagacgaggtcctgggcgacctggaccaggcccgtctgatggccaatcttcagttcatagtagggcacggctggacctgcggtggtggttgaaatgttaactttcgactgtacgcgagtaaccccgtcaggggtcgttcagtggcggaaatcaggcattcgggacttcccgaactgccagccatgggctccgagttgcagaatgcctctggtggttgcaaaatggaaccccagaggagcctcgtatgagccaggccgtaaagatctcagacattgaaatgaaggcgctgcgtgatgcggcgcggttgaacagccggtcgatctccggccaggccgagcattggcttcgcatcggccgtgccatggaacgtgatccggaagtcggttattcccgggtcgaactggccctgcgcggcctcgagccgctgtcgctcgattcgctcgccgaagccgagcaggacgacttcatccaggccctggccgacgcacccgctactgcggcggaagaagacttctggcgcgaccgccggcgccgcggcgtgggtgtcgggctcgatgagaaggatcgattggtgtacggcacacccgcagtgaaacgttgagcaccgcgtgagccgcccgacgatgatcatgcttgccgggccgaatggcgccggcaagtcgaccttctatgaaatcgtcattcgtccgcgaatcaaggcgctgttcatcaatgccgacctgatccagcgcgaggaactcggcgatccgtcgatggccgcggcctaccgggcggccgccatcgcggagagccgccgcaggcaggcgctggagaagggcatcagcttcgtctccgaatccacgttctctcacgagtcgaagctggcgctgatccgcgatgcccaggccgcggggttccgggtcgtggtctatcacatcaacgtgcgccgcgtggagctctcggtcagccgggttgggcaacgggtggaagagggcggacacgacgtgcccgaagacaagatcagggagcggttcgagcgcaaccagccgttgatccgcgaagccgtgctgctggccgatcatgctttcgtttacgacaactccgggctgaacatgccggcagagcgcctcatcgccttcagcaagggccaggtgatcgccgcctctgcagacctgccggattgggccagggcgctctatggccgggagctcgggctggcttgaggcgaccttcgcgtgcgccctcggcctacgcggatcttcgttgccggctgtgcaggtttggcaagaaggtagccgaagctcgcaacactccaaccgcccgacgaaaggtctttccatgagcgccaacgagccatctctctccggacccattgccgatgaactgacgccgctggaaatttccaaggcgatgctcgagagcgaagaagatccgaacaccgcgcggccgctcacgccgctggggcaggccgcttcgggcctggggccaagacgcgcccgctcgtcatgggcgcttgcattgcgcagccctgcgacggtgtggtgcgccatcgcgggggtcggcctgatcgcggcgctggtctatgtggcgcgggagcctcgtcggtcccggcgggcgggttgaccggcctggggtagctctcgttcttgctcgctggtctcttcaggcgcatattcccgattcggttgcggggccggcggccgaaagactcccattgcaccggccacgcgggagaaagccatgagcaagacgattgtcgaaaccgcggaggctccttccgccgtcgggccgtactcgcagggcgtgcttctcgacgggtggctctggacgtcgggccaggtggcgctcgatccggcaaccggcgcgctcgcggggacggatgcggccgcacaggccgaccgcgcgctcaagaacatcgaagcgatactgcgggccgcaggctcgagcctcgaccgggtcgttcgcgcaacggtctacctgaccaacatggacgacttcgcgtccgtgaactcggtgtatgcgcgctactttcccagcgcatttcccgcacgggcgtgcgtcgaggtgtcacgcctgccgctgggggcattggtggagatcgacgtgattgccagggcggccgcttcgcctgaatgaaaagccgcagcgggcccctcaccctcttttgcgagcggtagagaggcccggacgatcagtaccgatcgtcgccatagcggcgatagtgctcgcggcgctcccactcgcggcggcgccattcgcggcgctccgcacgacgttcttcccagctcggccccggctcgtagtagaccggcgcgggcgcaacgtaggcaggcgccggctggtagcgcactggcggggctggctggtagtagacggggggcggcggcgaatatgcgggcgcgggttcgtaatagaccggcgccggttcgctgctcaccaccacgcccggcacggacacgccaacggaccagctcgtgccggcggtggccgaggccatcccgaaaagagcgccggcggccaacgcgccagagagagccagcttgaggccagttcgagtcaaaatcatctcatctcctgaagatctgggaacaatcccgatgtacttccaacgcctggccgcgccgggtcgcgcacatcgcgactgtgaagaaggttccaagatgtcacgggaggaagaagggcatccggcctccgggtgaccgatcattcgcgatcattcgtctaccagggaggcaaaaaaatggcagcccagcgtccggtcacgatcgacgaatacatccgcgcggcgccgcgcgagggccagccgcatctgcgccggctgtacgcgctcctcaagcgcgttgcgccagaagccgaagaggcaatcaagtggggcacgccgttcttcgtggagccccgcttcctgttcgccttttccgcgcacaaggcgcacctcaacttcacgccgacggcggaagggctggagccgtttcgcaaggaactggaagcgcacaagacgaccaagggcatgctgcagatcccctacggcgagcccctgccggaagcgctcattcgccagattgccgaacaccgtgtgcgcacggtgcgtgaacgcgaagacgacgccttctggtgacgccaccgcggcgggagggcgagctcaggacttcggcttcttcgcagatctggacttggccgcactgttgagtgcgatggcctcgcgcacgagcgccttgaaggcggactcgtcgactttttcgccttcatggatgtcgatggcgcggcgcatgtttccgtcgaggctcgcgttgaagagacgggccggatcctccaggaaagcgcccttggcgaaggtaagcttcaccttgtccttgtaggattcgccggtgcagacgatgccgtcgtgcgaccagaccggcgtgcccatccacttccattcctcgacgacttcggggtctgcgtcctggatgagcttgcgcattctgcccagggtttcgccgcgccagccgccgaggtcggcaattctttgggagatgagttccgatgccggctggcttgggctcgcatccgattttttcatgttctgatcctggaagttctgcggcccgacgtcgacgtcgaagatccgctggccgtctgaatctgcggaatttaaccgaccccacatgacacgctttcttcattccgccgactggcagatcggccgccagttcgcaaccttcgattccgagcacgcgccgatcctggccgaggcgcgcatcacggtggtcgagcggctcgcggcgctggccatagagcaccgggtggacgccgtgctcgtcgccggcgacgtcttcgacgtgcagaccgtttcggagcgcacgctgcgccgtctgttcaatgcgctgtcgggctatgcggggccctggctcatgattcccggcaaccacgacgccgcccttgccgaaagcgtgtggacgcgcgcgcagcggctgggcttggtgccgccgaacgtccatccgctgctggtgcccgaagtgcgcgtgttacaggcgcagggctttgccgtgctgcccgcgccgctcgcgcagcgccacacctacaacgacctcacggcctggttcgacgcggccgaaacgcccgcgggcatgctgcgcatcggcctggcgcatggcagcgtgcagggcttgctcgcagaagacatcgactcggccaaccccatcgcgcccgaccgcgcatcgagcgcgcggctcgactacctcgcgctcggcgactggcacggctgcaagcgcatcgacgcgcgcacctggtacgccggcacgccggagccggaccgcttcaaggacaacggatcgggtcaggcgctgctggtggacatcgccgcgccgggcgccgagccgcaggtgactccacttgcagtcggccaattccgatggcaatcgatcaccgcggcgttgcaggttgcgagcgatggctacgcgttgatcgcacggctggagccgctggattcgcacgacgtggccgagctgcgcgtgcagggccagatcgacgtcgcgggcctgcagcgcctgcgggcagccatcggccgcgcggaggcgcgggcccgccatctgcaggtcgatctgtcggcgctgcggctcgtgcccaccgacgaagacatcgccggtctgcaggccgacggctacctgggcgaggtggtgcaggaactgcgtgatgcgcaggccagccccgattcgccggaggcgcgcgtggcgcaggatgcgctggcgctgctggcggccgagctcgcgcagcgatcgccaatggcatcggccacggcctccagggagggcgcttaagccatgaagctgcagatcacccgcctgcgcgtcgagcagctgcgtcgctttcgctcaccgctcgaaatcggcggcttcgagcccgggctcaacatcctggcggcgcccaacgaggccggcaagagcacgctggtgcgcgccatccgcgcggccttcttcgagcgccaccgctccacggccgtggaagacctgcggccctggggcgagggcagcggcgcggcgccgctggtcgaactcgactttctgatcgacggccagggccaccggctggtgaagagctttctcggcaagaagcgctgcaccttggcggccggtgcgcgttcgttcgacggcaccgacgccgaggaccacctggcccagctgttcggcttctcgtttgccggcaaaggcgcgagcaagccggagaactggggcatcccgggcttgctgtgggtggagcaggggcgcgggcaagagctggacgtcagccatgcgcgcgaccatctgcacgacgcccttcgcgacccggccggcgattcggcagcggcgctggctgcgagcggtggcgacgcgatcctcgacagcctgcgcgcgcaacgcgacgaactcctgacctcgaccggcaagccgcgcgctgcccatgccgaagccattgcgcaagtggccatgctggaggcagaactcggcgccatcgacgtgcaggtcgccgcctaccgccagcaggtcgaccagctcgcacagatgcgccagcagcaccaggccgacgagatggcgcggccctgggaagcgctgcgcgagcagttgctggccgcacagcaccgcaacgacgcactgcaggcgagccaggagcagctgcgcaacgaccgcacgcgcctgcgccagctgcacgaaacccgggagctgctcgcaaaggaactggccgggctcgttcagcagcagaccgaagcgcaaacgcgcgagcgtgcctgcgaagagaccgccaagcagctgcacgacagcgacgccgccgtggcccatgcgcgccaaagcgcagcggaaacccaacgccgcgtcgacagcgcccgcgacgcctggcgtgcggcgagccaggaggcccagcgccgcaatctgcagcagttgctgcagcaggcgcagaccgatgcggcgcgcagtgccgacagcctcgcgcgcgcggaggaggcccacgcgcggctcgcggccctgcaggccaccgccgcggcagcgccgaagatccgcgccgccgacgtcgagcagttgcaaacgctcgagcgtgccgagcacgatgccgatctgcgccggcaggccgtggccacgcggttgcagttcgtgctgccggaaggccaggccctcgaactgcaggcgcgcgacggaagccacgacctgcgcgggcagggcgaacggctcatcgacgcacccgccacgctgcagctgccgggcggcggccggctggtcatcacgccgggcggcgacgacctcgtggcgcttgcgcgtgcgcacgccgatgcgcgcgatgccatgcgcgcggcgctgcgggcctctggcgtcgacgacatcgcgcaggcccggtcgcggctcggcgcctcggccgatctcgatgcgcagatcaagctcgcgcagcaggccctcggcatcgtcgcgccgcgcgggttggaagcgttgcgcagcgaacttgcacaggcgcaatcacgcatcgccaccgcgcaggccgccttcgaacgcctgcccgcggcaacggccgcacccaccctgtcgatcgaggaagccgaggccgcccagcaagccgccgtagcggccgagcacgcagcgcagaagacgctcgccgaagcgcagcgccggcaatcggcggcgcaggaggcgagtgcatcggcccggcgcgaattcgcggcagcgcaggcggcgctcgcggaccccggccgccagcagcgccatgcccaggccagccagcaatggctggccgcgggcgccgaggccgaggcgctgaccgcccgcatcgaccagacgagcgccgacgtgcaggccgcgcggcccgacatcgtgctgcaggacatcgaccgcctgcagcgcagcatcgaacaggtcacgcgcagccatcagcagcgccgcgagcaactgctgctgctcgaaaacacgctgcagcaggccggcgcgcagggcctggaggaacagcgggaggccgtggccggacagctcgtgcaggcacggcgccggcatgccgagctgcagcgccgcgccgatgcgctcgcgctgctgtgccacaagctcgagcaaaagcgccaggccacgctgacccggctgcaggcgcccctgcaaacgcgtatgcagcactacctgcctctgctgatgcccggggccacggtgcacatggacgcggggcttgcgcccgccacgctgacgcgccttaccgccggcggcgccgccgagagcgggcagttgcacgagctgagcttcggcgcccgcgagcagctgcggctcatcagccgcttcgcctacgccgacctgctgcaggaggccggccggccgacgctgctgatcctcgacgacgcgctggtccacagcgacgctccccggctggcgcagatgaagcgcgcgctgttcgatgccgcgcagcggcaccaggtgctgctgttcacctgccatccggaccactggcgcgacatgggggttgcgctgcggccgctgggctgaggggccttgcacgcacgccgacacacatccggcgaagcgcgcctcttttcgaaagccttgaaaagtggcatgttgtctcctcgttccgaggagcatcagatggccactgcacgttctatcgcttcgctgtcgctcggcttcggcctggtttccatcccggttcggctctactcggctaccgaggggtcggcgacggtgcatttcaacctgctgtccaaggagggcgagcgggtcaagcagcagtacgtttccgccaccgaccctgccaaggtggttgcgcgttccgagatggtgaagggctacgaattcgagaaggaccggttcgtgatcttccagcccgaagaactcaaggccctggaggagggcgcgagccatctcatcgacatcgtcgccttcattccggcggatgcagtggatccgatctactacgacaagccctactaccttgcgcccgacaagcgcggcggcaagccgtacaacctgctgaagaaggcgatgctcgaaagcggccgctgcgcgctcgccaaatgggcctggaaggcgaagcagtacgtggtccaggtccgcgcccaggaagaggggctgattcttcagcagctgctgtacgcggacgaggtgcgttcgctgcaggacctggagatcgagcagctggagccgagcgcgtcggagctcaagctcgcgctgcagctgatcgaccagatctccgaggaaagctacgacccgacccgcttcgaggacgaggagaagaagcgcatcctcgccgccatcgacgcaaagatcgcgggcgaggaaatcgtggctgccgagcatccggaggatgcggccagcgggcaggtgatcgacctggccgaaatgctcaaggccagccttgcgcgccattcgacctcgggcccgaaggtgcgtccggccgcggcaaagagcagcgccagtccgccggcggtcacgcccttgcgcagtgtctcgagcaaggccaagcgcgcgcccaaggcgcccgaaaaggctgctcccgccccttcacgcgcgcgcatgaagaagtgaaagcctcgaccgaattcgcgtcgccctacaccctgcgcggcgtggtccagctgctgggcctctcgcggcacgccgtgagcaagctcatcgaactcggcttcgtcgcaccggtcaagacgccggcgggaacctggcggttctcgttccaggacgtggttcttctgcgctccgcccatgagctgcgcgccgcgcgcattccgacgcggcagattctccggtccctgcggcagctgaaggccacgctgcccgcgcagatgccgttggcgggcatccgcatcaaggcggagggcgaccgggtgaccgtgcgctcggcccatgcgcactgggagccggacaccggccagctgctgctggacctgagcgtcgagcccggcacgggctcggtgagtttcctgttctcccagcagggccgggcgtccaccaccgccgacctcgacgcgctctttgagcaagccgaggcgctggaggccacggcgccccaggcggcggaagccacctaccggcagatcctgaaagaggagcccggctacgcccatgcctacctcaacctgggcttcatgctctgcgaagccggccggtgcggcgaagccgcggacctgtacgacgtgggcgtccggcactgcggcgacgaccccctgatgcactacaaccacgccgtggcgctggagggtgccggccgcatccaggacgcgctggccagctacgagaaggccttgcagctgcagcccgacctcgccgatgcccaccagaacgccgcactgctgtatgcggagctggggcacaagcaactcgcgatccggcatttcagcgcgttccggcgtcttcagagcagcacgtaggcgccagggggcttcttcctacgagcaatgcggccgcttcgcgctagcgtcggccatccgacccaccgcaagtcgcaaggagttgaatcttggccaccgccagcagaaccctctggaaaggcgcgatcactttcgggctggtgcacattcccgtgggcctgcacaccgcgagcaccgagcagggcgtcgatttcgactggctcgacaagcgcagcatggaccccgtgggctacaagcgcatcaacaagagaaccggcaaggagatcgacaaggacgacatcgtgaagggcttcgagtacgaagacggcaagtacgtcgtcatctcgcccgaggagatcgaagccatctacccgcgcacgacgcagaccatcgagatccagcgcttcatcgatgccaacgagattccgttcgtctatctggaacggccctattacgtcgctccgatcaacagggggcagaaggtctatgcgctgctgcgcgaggtgctcctcaagaccggcaaggtgggcctggccaaggtcgtgatttccaccaagcagcacctggccgccctgatgccggccggcgaggtgctcgtgctcaacctgcttcgctggggcgatgaggtgaaatcgctcgcggggctggacctgcccgcggccggggtcaagggggccaaggtgacggcctcggaaatgaagatggccgagcaactcgtgaaagacatgagcgggaagtgggaccccgacgagttcaaggacgagttcaagcacgcggtcatgaagatcgcccagaagaagatcaaggccggcgacaccgaaacggtgatcgagccggaagaagaagggccggcccagggcgcagagatcatcgacctgacagagcttctgacgcgcagcctcaagggcggcaaggccgccaagtcggccggctcatcggcgaagaagaccgcgggttccaggaccagcgccagtgcaaagaagaccggtgccgccgcgaagaaggccccgcgcaagaaggcgcccggccctcgccgcaaggcggcctaagcagccgggcgagccctatttgccgccagcctgcgtggcttccgtcagcgcggccgacacgcactccagcgcgatggccagttgcgtgagcgtcggcaatccgaagcccagccggaacaccagcggatcgtcgccgaaccacggaccgggtgcgacccgggtgctgtatttttgcagcgttgcataaaagcgttcgacggccgcggcgtcgaagacgtcacgcttgagccgcacgcagcacagcgccccggcatcgggacgcacccactcgatgtggtcgggatggcgcgacacccagttctcggtgaactgcaggtgttgcgcgaggagcttgcgcctctcgccgatgatccggtcgcgctgcctgaacacggcgagtgcaagcgcctcgtcgaccggcgagcatgagatcaccgtgctgaacttggccgtgataagagcctggcgcagcgccgcgtcgcgcgtgatggcccagccgatgcgcaagcccgccgagccgtggcatttggacagcgaggacaccgagatgaccttgcgccccaggcacgcggcgctgggtgccgcggcatcgtcgccataggccgcctcacggtaggtctcgtcgaccaccagccaggcctcgggggcatgctcggccagcatcgccacgatttcgcgcaaggtctgcgcgggaatggcgacacctgatggattctgcggcgaggccaggctcacgatcctggtcttcggcgacagcagcttgcgcagcgcgtccgggtcgacccgatagcccgtgtcgaagcccagcggcagtgcgcgggtcacggcgccaacggccgccagcgcgttgcgcgcgagcggaaacaccggctcggccacgatggcttcgtcgcccgcctggcacaacgtgaaggcaatcagaaaaagggcgtgcatgccgccgaccgtgaccaccacgtcatcggcatcgacgccatgctcgttcgcgatctcctgccgaaggttctggttgcccgccgctgtgccgtagtcgagcgaaaagtcggcgtcgctgccgaaagccgagtcgatcagttccgccagccgcacgctcgggcccacgctttccgcgagatcgaagcggggcgccttgctgaccagggagatgatctcgttgtccggaaaccgtgccatgtggtgctgcttgaaccgttgctgtcgatgcactcatcttgcagattcgcggcccacgataacagccacaatttcctgaaattgagtgcagtacagttgcatgcagcgtcgtccatgcaaagaggagtcatccgtgtcgcagcagccactccggttccgttatgaagaagttgccgatttcgtcgccggcctggccggccgcggcacgctccggcccggggcgcgggcaccgtcgctgcgcgagatcagcacgcagcagcgcaccagcctcagtaccgcggtgcaggcctaccgcctgctcgaagaccgcggcattctcgaggtgcggccgcagtcgggctactacgttgccaaggcgccgcccgccttgcccgtgcccacgaccacgcggcattcggtccggcccgccaaggtggagctgtcgggtctcatgctgagcctgctggagcacgcctcggacgaagccctggtgccgctcggctgcgccattcccaaccagcgcctgctgtcttcatccaagctcgacctcgttcttgcgcgcacggcgcgcgtgaagggcgggcagtgcaacacctactcgccgccgcgcggcgagatgtcgctgcgcctggagatcgcgcggcgcgcactgcgtttcgggcaggcgctgtcgccggacgacattgccatcacctgcggctgtaccgaggcgctggcgctcgcgctcgacgccgtcacggagccgggcgacgcggtcgcgatcgagtcgcccacctacttcgggctgctgcaggtcctgcgcgcgaagaatctcaaggtggtcgaactgcccaccgactccatcaccggcgtggatgtcgatgcgctgcgcgatgtggtggcctcgggcaaggtgcgcgcctgcgtgctggcgtcgagcttcagcaatccgctcggctgcaccattcccgaagagaacaagcgcaccatactgcgcctgctcgccaagcaccgcgtgccgctgatcgaggacgacgtgtatggcgacgtccatttcggcgaagagcggcccctgcctttcagcgcgctcgacaggcacgacaacgtcatctattgcggctcgttttccaagacgctcgcgcccggctatcgcatcggctggatcgtgaccggccggcacatggcgcgggtgctggagaccaaattcgccaccagtcttgcgacaccggtgctgacgcaggtggcgctcgccaccttcctgtcgaacggcgactacgaccgccacctgcgccgcatccggcgcgagtttgccgacacgctgggccgcatgacgcgcgtgatcgagcaggcttttcccccgggcacgaaggtttcgaggcccgcgggaaacttcgtgttgtgggtcgagctgcccgagccggcggatacgcggctgctgtttgccgaggcgctgggcaagggcatctgctttgcgcctggcgtcgtgttctcggcaagcggaaagtatgcccactgcctgcggctgagtggcggccatggttgggatgcgcggatcgagaagggcttgcgcaagctcggcgccatggcctccaaggcgttcgcggcccacaatcgccaaccatgatttcagtccatcttcacggccagcgctttcaggttcgtgccgccgccatcgtccttcatgcgggtcacgtgctcgtgcaccgggccccgggcgatgggtactgggccttgcccggcggccgggtcgaagtgggcgaagaggcatcggccacgatcgtgcgtgagatgagggaagaactcggcgaagaggtcgagtgcggaccgcttctccatatcgcagagaattttttcgacctggcggaaaggcggaaccacgagatcgggttctactttctcgtctcgctgcccgagaactcgagccacctcgacaaggcgcgaagctaccgggggatcgaagaccacctggagctggagtttcgctagttccccgtcgcggagcttgcgtccatcaacctgcggcccacgtttctgcacgcatccctggcggcagatccgctggccttctcgcatgccgtgcagcgcgaatacccgtgatcgccagcgctcgcgactgcatgcacagccccacgaggtcaagcctcgccggccgtcaggagaggggccagcgacgaagatgccacctgagcttcgcccaggtccgccatgcaaggtatatggccatgactacacccttttctgccgttgcaccggatgaagctcacctgcgcatctcgaccagataggcgcgaacggcatcggctgaattgccgaccactctcaccgcgtctcgcagctgcgtctcggaacatttcagcgcctcggtccatgaacgcacttcgtgcggctcgtcaatggcgatcagcttgcgatccagtcctgtcttccttgggttgtcgggcatgtttttctcctgttgtcacggcggcacaatgcctccggcacttcaggttgagcgctgcgaaggggcagcgccatgccgttttgacgcgtcttggtgagggtgactctcctacgttgcgcccgcatcggtgcacgggtgccccggccagggcgccacgggccgagaccacgtcccccggcgctgactagggcgagcggggtgacagttgcgcacgcaaccaccgggccaggtcggccatgacctgcgagcccagcggcgatacggcggtgaagtgaatgcaggcgtgaatggcgccggggtagtggcggtgcgctgtcggcacgccggcctctgcgatgcgctgcgccagcgcatggccttcgtcgcgcagcgggtcgtgccccatggtggccagccaggtgggcggcagcgtggccagtgcctgcgcgtgcagcagggcgaaatcggcgtgccgcaccagctcctggcgcccgccgaggtagcaatcgatgaaccactgcatgacgccatgggtgaggaacttgccctcgccgttctcggccattgatgggctcggttcgctgtagtgctgggcgaccggatagatgaggcccagcgcacgcggcgcaatcgtgccggccgaacgcagcgccgccacggcggcgagctgcgcgcccgcgctgtcgccggccagcgcgatgcgcgacggatcggcgccgagcgcttgcgcgtgcgtggccacccatcgcagcacacaggccacgtcgtccaacgccgccggaaagggatgctcgggcgccagccggtagtccaccgccaccaccacggcggccacgtcgtggcacagggtgcggcacaccttgtcgtgggtttcgaggtcgccgatcacgaagccaccgccgtgcacgtacagcagcaagggaagcggcccctgggcgtcgggctggtagatgcgcagcgtcaacgggctcccgggtccgtcgatgacgcggtcggccgccgatgcgatggccggcgccggcaggcccaggccggcggccagctcgcggtagatctggcgcgccaccggcgggggcagcgactccagcggcggattgccttgggcagcggcttgcgccagaaagccggccagcgccgggtccaggggcgccgtgtcgagtgcggagggaatggaggtgtggctcatggcggctcagatgtaggtcgatgccagtccgccatcgaccgggatgttggcgccgctgatccagcgcgcctggtcgctgcacagccacgcgatcaccggcgcgatctcgtcggcgaagccggggcgcagcatgcggtgcgcatcggcctgtacgcgctcctggccgagcatgctcacgaagtcgcccaggatcggcgtgaacaccgggcccggcgccacgcagttcatgcgcacgccgtgttccagaaaccatttctgcgactgcgtggcgctccagacgatcagcgcttccttgaagtactggtagcaggtctcctgcggcacggggtggtcgcgcagccaatgggcgccggcctcgaagccttgcgcggcggccagggccttgtgcggcgccaatcgctgcggccattcggcgccgaggatggaggccacgttgacgatggagccgccgcgcgggatgcgcggcagcgcctgctccgtcaggtggcgcagccccaggtagttgacgtcggccaccagcttgacgggtgccgtgccgggcacgccggcgatgttgcacagcgcgtcgaagcgctcgggcaactgcgccacggccgcatcgatggcggcgacggaactcaggtcggccttgacgaagccgtcgagcgtgagactcgggtcgttgcggtccacgccgatgacgcgggcgccggcaaagcgcgcgatgcgcaccacctcggcgccgatgcccgacgacacgccggtgacgacgatggtttttccttgaagctgcatgagatgtctcctcgtgggttcagtagccaactaacgctcagaacgggtaggcgtgcggcgcctgcttgatggtcagccactgccactgggtgtattcctcccagtcggcggggccgcccacgctgctgccgttgccggcgatgccggggccgccgaaggggttgacgcactcgtcgttgacggtctggtcgttgatgtggaccatgccggagttcaattgcgcggccattgccatggcccgtccgatcgagggcgagatcaccgccgacgccaggctgccctggtggttgttggccagggccacggcctcgtcgtcggtgctgaaggtgatgatgttggcgacgggaccgaacacttcttcgtcgtacacgcgcatgccggccttcacgttggccagcaccgtgggtttgtagaagaggccttcgctggtgccgccggccagcagctgcgcgccggccgcaatgctctcctgcacgatggcgtgcacgcggtcgcgctgcttcgcgtcgatcagcggccccagggccacctggccgctggcaccgtcgcccaccggcaggtgctgggcctttgcgaccagccgttgcgtgaaggcggcggcgatgctttcgtgcacgatgatgcggttggtcgccatgcagatctgtccctggtgcaggtaggcgccccaggcggcattgctggccgcgatgtcgaggtcggcgtcttccaggacgatcagcgagttggcgccgcccagctccagcgtgaccttcttcagatgtcgccccgccagctcgccgatgcgccggcccacggcgggcgagccggtgaaggcgatcatcggcacgtgcgcatcggtcaccagcgcttcaccggcggcggcgtcgccgggcagcacctgcagcaggccggcgggcaggcccgccacttcgaacacgcgggcgatcatgaagccgccgctcaccggcgtgcgcgagtcgggcttgaccaccacgccgttgcccgccgcgagggccggcgccacggtgcgaagcgtgaggatgagcggaaagttgaagggcgagatcacgcccaccacgccacgcggcacgcgccgcgccaggctggtggtgccatgcgcactcggcaacacctggccctgcgattgcaagggcatggccgctgccaggtggcacagggtgatggcctcgcgcacctcgtgctgtcccttgggcaggatcgcgcccgtctcccgggccacgtacagcgccagctcgtcgaagtgctgctcgaacagcgccgcggcccgcaggaacaccgcggccttctcgcgcggccccacctgcgcccagctcttctgcgcctgcgccgcggcggctgtggccagcgccacgtcttgcgcgtcggcaatgccgacggccgccatcacctggcccgtggccggttcgacgacgttgcgcacaccgcctgcggacgcgacccatgcgccgttgaacaccttgccggcccaggccgccgggtccaggaacgccagcttctgcgaaacacccatgactcaccccttgcgaaaaaagttgatcggcttgccatggtggaaatgccgcggcaccgccttcttttcgcaacgggcataccaagggtgcggtggcggggtggcccggggccgctacgcggggctgttttcattcgggggttaggggaattcccggagttgtaatagttattgcagataactggtttaccctgatccgggctttcaccaaatgctcaagaatcggccgcccgtttcaccaaacgatgaacttgaaattgaccaaagccattgcctcaccggtccccgggcggatctccctggccgaggtggcgcgcgccaccggcgccgcgctgggccgtttcgacggcgccgacgtggcgcgtgcgatgagccgcttcgacgcctcgcacgtgggaagcgaagagcacccgaccattgccgacatcagcgaatgcctgttcttttcgcccggcgacggccgcatctggctgcaggaccagcgcatggtgctgctgcataccgaggcgctggggtccctccggcgcgagctgatcgacagcctgggccacgggaaggcccgcggcctcttcacgcgcgcgggctacgtcagcggcgcgcgcgacgcgcagctggtgcgcaagcattggcccgaggccgagccggccgcggccgccatggccggcacccgcctgcatgcgctggaagggctggtgaaggtcgagctggtgcacgcgcgctacgaccccgagacctcggactacgaaggcgaattcatctggcaccactcggtcgaagacgacgagcacatcgcggcctacggcatcggcggctcgccggcctgctggatgcaggtgggctatgccaccggctacgtcagcacgctgttcgggcggctggtggtgtttcgcgaagttgcctgccgctcgatgggcgagagccattgccgcgtgatcggaaaatccgccgagcgctgggacgacgtggaagaagacatgcgctacctgcgcgcacgtgacttcgtcggcgtttccgtcggcgtgtctccctacggtggcgcggcgccgcgggccgccgagttgcccacgccgccgcgcaagagcgacgcgatggtgggtgcgtcatcggcattcaacgcggcctgccacttgctgcatcgcgtggcgccaaccacggccaccgtgctctttaccggcgagtccggcgtcggcaaggaaaagttcgcgagcatgctgcacagcatcagcccgcggcgcgacaagcccttcgtcgccgtgaactgcgcggccattccggagacgttgatcgagtcggagctgttcggcgtggagcgcggcgcctacaccggtgccggtgcggcgcggccgggccgcttcgagcgcgcccacggcggcacgctgttcctggacgagatcggcacgctgagctacgcggcccagggcaagctgctgcgcacattgcaggagggcgaagtcgagcgcgtgggcagcacgcgcagcgttcaggtcgacacgcgcgtcatcgcggccaccaacgtcgatctgcgccaggccgtgcgcgagggcaggtttcgcgacgacctgttctttcggctcaacgtctttcccattcacctgccgccgctgcgcgagcggcgcgacgacgtgccgcttttgatgagccatttcctgcagcactacggccgcaagcacggccggcaggtcgccggcttcacgcaagccgccgtcaaggcgcttctgaactacgactaccccggcaacatccgcgaactgcaaaacctcatcgagcgcgccgtgatcgtggcgcccgaaggcagcctgctcgaagtgcatcacctgttcacgagcggcgagacgctggacaagaacgtgctgtcggtacggccggatggccacctggcaggcgctgggtctgtcggcgccttgcccccgcaggccgcgcccgcaagccaagccgtgccggacagcatcggccccggttccttggggcaggtcgaagagacgctgatccgccgtgcgctggagcaatgcggcggaaatctttcagcggctgcgcgtgtgctgggcatcacgcggccccagctggcctaccgggtgcgcaagcgagggctcgtcgtgaagtcagggccgggttgagggacgaaacatgaacggacgccggtaaaccaacctcgctggattgactctcagggtttgccctaatcgccggtccggcgattcggacaggctcgtcgctccgcatccggatcgtcggcaacgcgctcgcttcatctccgcctcatctttcatgaaatcaacgacttagagagcgttgcgcgcgttgcgccgcgtggcacatcgattgctgtgtaccaaggccggccgcatcgcccgatgcggctttcggccacgacacaggagacaaaccgatgagcaccatgggtgaccttgaccccacggaaactggcgagtggatcgatgcgctcggcgcggttcaacaacaccgcggcagcgagcgtacgaactttctgttgaatcgcctggtcgatcagggccgccgcgatggggtgtacgtgccccgctcgctgaacacggcgtacaagaacaccatcccgcccgagcaggaagaaaaatcccccggcaaccgcgagatcgagcaccgcctgcgctcgatcatccgctggaacgcgatggcgatcatcctgcgcgccaacaaggactcgtcggaactcggcggccacatcgcgagcttccagtcggcggccactctctacgacatcggctttggccacttctggcatgcggccaccgacacgcacggcggcgacctgctgttcatccagggccacagctcgcccggcatctatgcgcgcgcttttctcgaagggcgcctgagcgagcagcagttgctcaactaccgccaggagtccgagggcggcggcatcccgtcgtatccgcacccctggctcatgcccgacttctggcagttccccaccgtgtcgatggggctcggcccgctgatggcgatctaccaggcgcgctttctcaagtacctgcatggccggggtctggccgacacggcgccgcgcaaggtctgggccttcatgggcgatggcgagatggacgagcccgaatcgctcggcgccatctcgctcgcgggccgcgagagtctggacaacctcgtgttcgtcatcaactgcaacctgcagcgcctcgatggcccggtgcgcggcaacggcaagatcgtgcaggaactcgagagcgtgttccgtggggcaggctggaacgtcatcaaggtgctctggggcagcggctgggacgcgctgctcgccaaggacaagagcggcaagctgctgcagcgcatggaagagtgcgtggacggcgagtaccaggacttcaagagcaagagcggcgcctacgtgcgcgagcacttcttcggcaagtacgacgagacgaaggcgctggtcgccgacatgagcgacgacgagatctggggcctcacgcgcggcggccacgaccccgagaaggtgtttgccgcgtatgccgcggccgtcaagcacaagggccagcccacgctgatcctgcccaagacagtgaagggctacggcatgggcgaatcgggcgaaggccagatgatcgcgcaccaggccaagaagatgacgcaggacgcgctgcgcggtttccgcgaccgcttccagattccggtgtccgatgaagagctgcccaacgtgcccttcatccagctggccgaagacagccccgagatgaagtacctgcgcgagcgccgcgccgcgctcggcggctacctgccgcagcgccgccgcaagtcgaccgcgctcgagattccgccgctggccaccttcgagcgcctgctcaaggacaccggcgagcgcgaaatttccaccaccatggccttcgtgcagatgctcggcacgctggtgcgggacaaggccatcggcaagcacgtggtgcctatcgtgcccgacgagtcgcgcaccttcggcatggaaggcatgttccgccaactgggcatctggtcctcgctcggccagctctacaagccgcaggacgccgaccagctcatgtactaccgcgagtcgaaggacgggcaggtgctgcaggaaggcatcaacgagggcggcgcgatgtccagctggatcgtcgcggccacctcgtacagcacgaacaacgtgccgatgatcccgttctacatctactactcaatgttcggcctgcagcgcgtgggcgacctggcctggctggccggcgacatgcgtgcgcgcggcttcctcttgggcggcaccgcggggcgcaccacgctcaacggcgaaggcctgcagcacgaggacggccacagccacatcctggccggcaccattccgaactgcgtctcgtacgacccgaccttcgcctacgaggtggtgaccatcgtgcgcgacggcatgcgccgcatgtatgccgagcaggaggacgtgtactactacatcaccctcatgaacgagaactacacccaccccggcatgcccgagggcagcgaagcagggattctcaaggggctctatcaattgagcgacggcggcaagacgcccaagaagggccaccgcgtgcagctcatgggcagcggcaccatcctgcgcgaggtgatgttcgcggccgagctgctgaagagcgacttcggcattgccgccgacgtgtggagcgccaccagctacaacgagctgcgccgcgacggcatggccgccgagcgctggagccggctgcacccgaccgagccggcgcgcaagagccacgtcgagcaatgcctcgaaggccacgacggcccggtcatcgcggccaccgactacatgcgcaactacgccgaccaggtgcgcgagtacgtgcaggccgcgggccggcgctacaccgtgctgggcaccgacggcttcggccgcagcgactaccgccgcaagctgcgccgcttcttcgaggtcgaccgctggcacgtggccgtggccgcgctcaaggcgctggccgacgacggcgtgatcaagcacgcggtggtggccgaggccatcgcgaagtacgggctcgatgccgagcgcgccgccccctggaccgtctgaggcaaggcagcaaaacatgagcaacgcaatcgacatcaaggttcccgacatcggcgacttcagcgacgtgccggtcatcgaaatcttcgtgaagcccggcgacacggtgaaggccgaagacccgctggtctcgctcgaatccgacaaggcgacgatggaggtgcccgcgccgcgcggcggggtggtcgagtccatctcggtgaagctgggcgacaaggtcagcgaaggcagcgtcatcatgacgttcaaggccgagggcggcgctgccgctgcgcccgcgcccaccgaacccgccaagcccagcgtgagcgccgcgcctgcggccaccagcgcgccggccggcatcgccgaggtgcgcgtgcccgatatcggcgacttcaaggacgtgccggtcatcgagatcttcgtgaaggtcggcgacacggtgaaagccgaagacccgatcgtctcgctcgaatccgacaaggcgacgatggacgtgccggcgccgctgtcgggcgtggtgacggccatcggtatcaagatcggggacaaggtgagcgaggggtcggtgattctttcgctcgctacgggcgatgcgcctgtggtggggggtgcgccctcaccccaaccctctcccgcgagcgggagagggagtgatgcagcagcggcggtgtcgcctgccggcaatgcggaggtcgaagcgggcttcgcactcgcctacgctggccctgccgtgcgcaaactcgcacgcgaactcgccgtggacctcggcaaggtcaagggcaccggcgaccacggccgcatcgtgcgcaccgacgtcgaggccttcgcgaaggacggtggtgtatctgccgctccggccgcgtccaaggctgcatccgctcccgcgggcggtggcgttggtggcatcgacctgttgccctggcccaaggtcgacttcgccaagttcggcccgaccgagcgaaaagaactgtcacgcatcaagaagatcagcgccgccaacctgcaccgcaactgggtcgtcattccgcacgtgacgacgcacgacgaggccgacatcaccgaccttgagccgttccgcgtgcagatgaacaaggagctggaaaagtcgggcgtcaagatcagcatgctgcccttcatgatgaaggcggccgtcgccgcgctgaagaagttcccggagttcaacgccagcctcgacggcgacgccctggtgctcaagaactactggcacatcggctttgcggccgacacgcccaacgggctcatggtgccggtgatccgcgacgtcgacaagaagaccgtgcccgacatcgccaaggagatgggcgagcttgccaagctcgcgcgcgacggcaagctcaagcccgaccagatgtcgggcggcaccttcaccatcagctcgctgggcggcatcggcggcatctacttcacgccgatcatcaatgcgcccgaggtcgccatcatgggcgtgtgcaagagctactggaagcagcactccagcgacggcaagacctacacctcgcgcctcaccctgccgctgtccctctcatgggaccaccgcgtgatcgacggcgccgccgctgcgcgcttcaacgtctatttcgccaacgtgctcgccgacctgcggcgcgtgctgttctgaaggaagctcccaatggcacacatggtggaagtcaaggtcccggacatcggcgaattcaaggatgtcgcggtcatcgaactgctggtcaagcccggcgaggtcatcgcggtcgataccgggttgatcatggtggagtccgacaaggcctcgatggagattccgtcgagccatgcggggacggtgaaggaactgaagatcgggctcggcgacaaggtcagcgaaggctcggtgatcctcgtcatcgaaacggctgctgctgctgcctcccctctcccgcttgcgggagaggggccgggggtgagggcggcggccgcaccctcaccccaaccctctcccgcaagcgggagagggagcgaggcagcgcctgcgcccgtggccggcagctacaccggcaaggccgacatcgaatgcgaagtgctcgtgctcggcgccggccccggcggctactcggccgccttccgcagcgcggacctcggcatgaagaccgtgctggtcgaacgctacgccacgctcggtggcgtgtgcctcaacgtgggctgcatcccctcgaaggcgctgctgcacacggccggcgtgatggacgaggtgaagctgctcgccaagcacggcatcaagtacaccgcgcctgaagtcgacatcgacgcgctgcgcggcttcaaggacggcgtcatcaagaagctcaccggtggcctggccggcatggcgaaggcgcgcaaggtcgaggtggtcaccggtgtcggcagcttcctcgatgcctatcacctcgaagtggtgggcgagggcggcgcgaagaaggtggtgaagttcgccaaggccatcatcgccgctggctcccaggccgtgaagctgcccttcatgccggaggacgaacgcgtcgtcgactccaccggtgcgctgctgctcaagggaattcccaagcgcatgctggtgatcggcggcggcatcatcggcctggaaatggccacggtgtattcgacgctgggcacgcgcatcgacgtggtcgaaatgctcgacggcctgatgcagggcgccgaccgcgacctcgtcaaggtgtgggagaagttcaacgcgccgcgcttcgacaacgtgatgctcaagacgaagaccgtcggtgccaaagccaccaaggccggcatcgaggtcagcttcgaaggcgagaaggcgccttcggccccgcaggtctatgacctggtgctggtggccgtgggccgcagccccaacggcaagaagatcgcggccgacaaggccggcgtggccgtcaccgaccgcggcttcatcgacgtcgacaagcagatgcgcaccaacgtgccccacatcttcgccatcggcgacatcgtgggccagcccatgctcgcccacaaggcggtgcacgaggcgcacgtggcggccgaggcggcgcacggcgaggcgtcgttcttcgatgcgcggcagattccctcggtggcctacaccgaccccgaggtggcctgggccggcaagacggaagagcagtgcaaagccgagggcctgaagatcggcaaggccgtgttcccctgggccgcatcaggccgcgccatcgccaacgggcgcgacgagggcttcaccaagctgctgttcgacgaggccacgcaccgcatcgtcggcggcggcatcgtcggcacgcatgcgggcgacctgatcagcgaagtgtgcctggccatcgagatgggctgcgagccctccgacatcggcaagaccatccatccgcatccgacgctcggcgaatcgatcggcatggcggccgaggtcttcgaagggcattgcaccgacctgcccccggtgaagaagaagtaggccccgccatgccgctcgcactgtctttcgaggccctgggatcgggacccgcggtggtgatcctgcacggcctgttcggcgcggggcgcaactggaagcaggttgccgaggcgctggccgcggaccaccgcgtctacctgcccgacgcccgcaaccatggcgcctcgccgtgggccgaatcgatgtcgtatgtggagatggcgggcgacgtgctggcgctgatcgagcgcgagcaattgcagcggcccttcgtgatcggccacagcatgggcggcaagaccgcgatggcgctggcgctctcgcaccccgaagccatcggcggcatcgccgtgatcgacatcgcccccgagagctacgccgaccagttctcgtcgtacgtgtcggccatgcgcagtctcgaggtggcgagtgccaccagccgccgcgaaatccagcaggcgctggccgacagcctcggcgccgacgcgccggtcgacttcttgatgcagaacctgcgccggcagaacgaccgcttcgactggcggctcaacctgctcgccacgggcctgtgcatgcgtgagctttgcagctttcccgacgcgctgcgcgaagcgcgctacgacggccccgcgctcttcgtccacggcgcggagtccggctacgtgcggccttcgtcgctcgccggcatccgtgcgctgttcccgcacgcggggaccgaacgcatcgccgacgccgggcactgggtccacgccgaccagcccgcggcgctgctgtgcggtctgcgcgactggctggccgatgccggcgcggccaccccttactgactttcccacggagacaccatgtccgacgaaaaactgcgcgaagccgccctcgactaccaccgctttcccacgccgggcaagatctcggtgaacccgaccaagccgatggccacgcagcgcgacctcgcgctcgcgtactcgcccggcgtggccgaggcctgcatggagatcgtgcgcgacccggccgaggcgatgaacctcacctcgcgcgccaacctcgtggccgtcatcaccaatggcaccgccgtgctgggcctgggcaacatcggcgcgctggccggcaagccggtgatggaaggcaaggcctgcctgttcaagaagttcgccggcatcgacgtgttcgacatcgagctcgacgagagcgaccccgacgcgctgatcgacaccatcgcgcgcatggagcccaccttcggcggcatcaacctggaagacatcaaggcgcccgagtgcttctacatcgagaagaagctgcgcgagcgcatgaagatcccggtctttcatgacgaccagcacggcaccgccatcgtcgcggctgcagccatcctcaatgcgctgcggcatgtgaagaaggacatccgcgaagtgaagctggtggcctcgggcgccggtgcggcggcgctggcctgcctcgacctgatcgtgagcctgggcctgccgatgcatagcatcttcgtgtccgacagcgcgggcgtggtctacaccggccgcaaggagcagatggacccgaacaaggcccgctacgcgcaggacacctcggcgcgcaagctggccgacgtgatcgccggcgccgacatcttcctcggcctctcggccggcggtgtgctcaagcccgagatggtgaaggagatggcgcgcgatccgatcatcctcgccatggccaacccgacaccggaaatcctgccggaagacgcgctggccgtgcggcccgacgccatcctcggtaccggccggtcggactatccgaaccaggtcaacaacgtcctgtgcttcccgttcatcttccgcggtgcgctcgacgtgggcgcgaccaccatcaacgaagagatgaagctcgccgcggtgcgcgcgatcgccgagctcgcgcatgccgagatccccgaggtggtggcgcaggcctacggcgcggtcggtctgcgcttcggccgcgactacctgattcccaagcccttcgacccgcgcctgatcgagttcgtcgcacccgcggtggcgcaggccgcggcggacagcggcgtggcgacgcggcccatcgccgacatgaaggcctaccgccagcgcctgtcgcagttcgtctaccagtcgggcagcagcatgcagccgctgttcgccgcggccaagcaggcgcccaagcgcgtggtctacgccgagggcgaggacgagcgcgtgctgcgcgccgcgcaggtggtggtcgacgaaggcctggcgcgcccgctgctgctgggccgccccgaggtgattgccgagcgcatcgcgcagtacggcctgcgcctcacgctcggcaccgactgcgaggccgtcgacctgctcgaccccgccgtgtacggcgatgcggccgaggcctactaccagctcaagcgccgcgacggcgtctcgcgcctggtggcgcagaccgagatgcgcagccgcggcacgctgcttgcggcgatgctggtgcgccagggccgcgccgacgccatgctgtgcggcacgctcggtagctacggcgaccacctgcgccatgtgcgcgacgtgatcggcctgcgccccggcaccaagaccatggccgccatgcagatgctgatgctgcccgggcgccagctcttcatctgcgacacgcacgtcaaccgcgaccccgatgccgcgcagatcgccgagatcgcgctgctcgcggccgaagaggtgcgccgcttcggcgtgacgccgagcgtcgcactgctgtcgcactcgaacttcggcggctcggacgcggcctcggccgtgaagatgcgcgaggcactcgcgctcatcaaggcgagcgacccgcagcttgcggtggaaggcgagatgcgcggcgacgcggctctgtcgaagaccatcctcgaccacgagtttccggactcggcgctggagaccgaggccaacgtgctcatcatgcccaacgtcgatgcggccaacatctcatacaacctgctgcgcgtggcggccggcagcggcatcacggtgggcggcatcctgctgggcgcggcgcgctcggtgcacatcctcacgccgtcgtccacggtgcgccgcatcgtcaacatgacggcgctggcggtggtcgatgccaactcgcaccgcaacgcggcctgacggcggcacggccatgagccggcccaagcccggcaggtgcatgccgccggcgtctgaaattttctaggagatatcgtggaccaccaagtcgtacccaagcccttttacaagtccctgtacttccaggtcatcacggccatcgtgctcggggtgctgctggggcatttctatcccgacaccggcgcatcgatgaagccgctcggcgacggtttcatcaagctcatcaagatgatcatcgcgccgatcatcttctgcaccgtggtggtcggcatcgcgggcatggaagacatgaagaaggtcggcaagaccggcggcctcgcgctcctgtacttcgagatcgtgagcagcgttgcgctggtggtgggcctcgtgatcatcaacatcgtgcggcccggcgccggcatgaacgtcgacgtgagccagctcgacgccaagagcgtcgcggcctacaccggcccgggcaagatgcagagcaccaccgacttcctgctcaacgtgatcccgaacacggtggtcgacgccttcgccaagggcgagatcctgcaggtgctgctgatcgccgtgatgttcggctttgcgctgcacaagttcggcggccgcggcacgctggtgttcgacgtgatcgagaagggctcgcacgtgctcttcgtgatcgtgggctacatcatgaaggtcgcgcccatcggcgccttcggtgccatggccttcaccatcggcaaatacggcgtgagttcgctgctgcagcttggccagctgatggccaccttctacgccacctgcctgttcttcatcttcgtggtgctggggctgattgcgcgcgcgcacggattcagcatctggaagttcatcaagtacatcaaggaagagctgctgatcgtgctgggcacctcgtcgagcgaatcggtgctgccgcgcatgatggccaagctggagaacctgggcgcgaagaagtcggtggtcggcctggtggtgcccacgggctactcgttcaacctcgacggcacttccatctacctgaccatggcggccgtgttcatcgcgcaggcgaccaacaccgaaatgtccctcacccagcagctcacgctgttggcggtgctgctgctcacctcgaagggggcagcgggcgtcacgggcagcggcttcatcgtgctggcggccaccctctcggccgtggggcacgtgccggtggccggcctcgcgctcatcctcggcatcgaccgcttcatgtcggaagcccgcgcgctcaccaacctgatcggcaacggcgtggccacggtcgtggtcgccaagtggaccaatgacctggacaccgtgcgcatgaggcgcatcctggacaacgagacggaggccgaggccgactcgcccgaggcggtgctggacaaggtcgagacccacatgcctgtggcccagccccgctgaagcatctcatgcctgtacggagcagccaaccatgaacagccccgtgcagaagcaccgagtcgtcatcgtgggtggcggagccggcggcctggagctggcgacgcgcctcggcgacacgctgggcaagcgcggccgtgcggacatcacgctgatcgacaagaaccgcacgcacgtctggaagcccaagctgcacgagatcgccgcgggcagcatggacctgagcgcgcacgaagtggactacctcgcgcaggcgcactggcatggcttccgcttccggctcggcgagctcaccggcatcgaccgcgagcggcgcgaggtgcaggtggcgccctacatggacgacgagggccggctggtcacgccggcgcgtgccttcggctacgacacgctggtgatttccatcggcagcctcagcaacgacttcggcacgcccggcgtgcgcgagcatgcgctgcggctcgaatcgaaggcggacgcccagcgctttcaccagcgcatggtcaatgcctgcatccgcgcgcacgcgcagaccgcgccgctgcggccggagcagctgcacgtggccatcatcggcgcgggcgccaccggcgtggagctggcggcggagctgcaccgcaccacgcgcgaagtggtcgcctacgggctggatcgcgtggacgccgagaaggacatccaggtcagcgtgatcgaggccgccgaccgcgtgctgcccgcgctgcccgcgcgcatgtcggccgccaccgaggcgctgctgcgcaagctgggcgtggacgtgcacacctctgccaaggtggccgaggtgctgcccgagggcgttcgcctggccgatggccgcgtgctgccggccgagctggtggtgtgggccgcgggtgtgaaggcggccgatttcatgaaggacatcgcggggctggaaaccaaccgcagcaaccagctcgcggtgctgccgaccttgcagaccacgcgcgatgccgacgtcttcgcgatcggcgactgcgccgcctgcgactggcccgaggccaacggcggcaagggcggcctggtgccgccgcgcgcgcaggcggcgcaccagcaggcctcgcatgttgcggcgcagatccgccggcgcatggcgggcaaggcgctcaagccctatcgctaccgcgacttcggctcgctggtgtcactcggcgagtacagcaccgtcggcaacatgatgggcggcctgatcggcgggaacctgatgatcgaagggctgttcgcgcgcctcatgtacgtgtcgctctacaagatgcacgagctggcgctgcacggcatcgtcaaggtttcgctcgacacgctcgcacgcctcatcacgcggcgcaccgaacctcacgtcaagctgcattgagcagtcacggccatgacccaaccttcttacggattcgacgcggcctcgtggttgcaagcctggcagcaggggctgtcgcagggccaccagcagtttggtgcgctgatgcgcagcgcgctggaggtcgcaccgctggacgcgcgcggcaaggcgcagatggatttcgcgctgcgccaggtgatcgacgccatcaacccggccaacggcctggcgaccaaccccgaggcgatgcaggccgcgctcgactcgggcggtgcaagcctgttcgaaggcgtgcgtctctttttcgcggacgtggcgaaaggccgcatctcgatgtcggacgacgaagccttcgaggtcggccgcaatgtcgcgaccagcctgggcggcgtggtgttcgagaacgagctgatgcagctcgtgcagtacacgccgtccacggccaaggtgcacaggcggccgctggtgatcgtgccgccctgcatcaacaagttctacatcctcgacctgcagcctgcgaattcgctggtcgcgtatgccgttgaacagggccacacggtgttcctggtgtcgtggcgcaacgtgtccgccgagcagggccacctgggctgggacgactatgtccagcaaggcgtgctccaggcactcgacgttgcgcgcggcatcgcccgctccgacaaggtcaacacgctgggtttttgcatcggcggcacgctgctgggcagcgcgctcgcagtggccgctgcacgcggcgagaagccggccgccagcgtcacgctcctgaccgcgatgctcgacttctcggacaccggcgagctgggcctgatggtggacgaggccatggtcgcgacccgcgaggccaccatcggccgcggcggcctcatgaagggccgcgagctcgcgaccgtgtttgccgcgctgcgcgccaacgacctgatctggccctacgtggtcaacggctacctcaagggcaaggcgccgccggccttcgacctgctgttctggaacggcgacgacaccaatctgccggggccgatgtactgctggtacctgcgcaacacctacctggaaaacaagctgcgcgagcctggcggcacggtgcagtgcggcgtgccggtggacctgtcgcgcatcgacgcaccggccttcgtgtatgcctcgcgcgacgaccacatcgtgccgtggaagaccgcctatgccggcacggcgctgctcggcggcaagacgcgcttcgtgctcggcgcgagcggccacatcgcgggcgtgatcaacccgcccgcgaagaagaagcgcaaccactgggtcggcgatcttgcctcggacgcgagtgcctggctcgagggcgcacaaagcatcgacggcagctggtggcccgcgtggagcgactggctcggcacgcacggcggcgcgaaggtcgctacgcgccgcgagctgggcagcgcggatttccccgtcatcgagcccgcgcccgggcgctatgtcaaagccaaggcggcctgaatccggctgccctcattcccttcacatcaacccccaaaggagactctcatgtcagacgatatcgtgatcgtggccgcgcaacgcacggcggtcggcaagttcggcggcgcactcgccggcacggccgcgcccgagctgggcgcgcatgtggtgaagggcctgctcgagaaggccggggtgccgggcgatgcggtgtccgaggtgatcatgggccaggtgctcgcggccggtgcggggcagaatccggcgcgccagacggtcatcaaggcggggctgccgattggcgtgccgggcctcaccatcaacaaggtctgcggctccggcctcaaggccgtgatgctggcggcgcaggccgtgaagtgcggcgacgccgagatcgtggtggccggcggccaggagaacatgagcgccgcgccgcacgtgctgcccaactcgcgcaacggccagcgcatgggcgactggaagctggtcgacaccatgatcgtggatggcctgtgggacgtctacaaccagtaccacatgggcaccacggccgagaacgtggcgaagaagtacggcatcacgcgcgagatgcaggacgcgcttgcgctggcctcgcagcagaaggccgcggccgcgcaggacgccggtcgcttcgacgacgaaattcttccgttcagcatcgcgcagaagaagggcgatccgatcgtcttctcggccgacgagttcgtgaaccgcaagaccaatgccgacgcgctcgcaggattgcgcccggccttcgacaagaccggctcggtgacggccggcaatgcctcgggcctgaacgacggcgcggccgcggtgctggtgatgtcggcctcgcgcgccgccgcgctcggcctgcagccgctggcggtgatccgcgcctatgcgagcgccggcctggatccgtcgctcatgggcatgggcccggtacccgcctcgcagctggcgctcaagaaagccggctggaaggcgcaggacctcgacctgatggagatcaacgaagccttcgcggcacaagcctgcgccgtgaaccgcgagatggaatgggacacgagccgtatcaacgtgaacggcggcgccattgccatcggccatcccatcggcgcctcgggctgccgcgtgctggtgacgctgctgcacgagatgcgccgccgcggcgccaacaagggccttgcgtcgctatgcatcggcggcggcatgggcgtggcgctggctgttgaacgcgcttgaacgcgcctgaacgaatttctttcctgtcacacacaacgcacctaggagcaatcaaatgagcgagaagaagcaacaagtggtcctcgtcaccggcggcatgggcggcctgggcgagacgatctccaccaagatggtcgatgcgggctacaagctcgcggtgacctattcgccgggcaacaagtcgcatgccgagtgggtggcgcagatggccgagcgcggctaccagatcctggccgtgccctgcgacgtggccgactacgactcctgcgcacgggccgtgggccaggtgcaggaagccctcggcccggtcgacgtgctggtcaacaacgccggcatcacgcgcgacatgaccttcaagaagatggaccagatcaactggaacgccgtgctgcgcaccaacctcgacagcctgttcaacatgagcaagcaggtggccgacgggatggtggaccggggctggggccgcatcatcaacgtgtcgtcggtgaacggctcgaagggcgcgttcggccagaccaactattcggccgccaaggccggcgtgcacggcttcaccaaggcgctggcgctcgaggtggcgaagaagggcgtgacggtcaacaccatctcgcccggctacatcggcacgaagatggtcacggccattccgaaggaagtgctcgacagcaagatcctgccgcacatccccgtgggtcgcctgggcaagcccgaggaagtggcgggcctgatcatctacctggcctcggaagaggcggcgttcgtgactggcgccaacatcgccatcaacggcggccagcacatgcaatgaacggacggccatgatcctcaaaaacggcatcgatcaggtcgcactgatcaacaagttcaccgacgcctcggccaagcagggcgaagccatccgcaaggccgtgcacgaggccacgctcaaggcgctgcagggccgcgagctcacgctcgcaaacatccggcaggtgctgggcacggtcaccaaggcggcttcggccggcgccgaggggagcaagctgcccgcgcccgacgtccaggcgctgctggccaaggccttcgccggcatggacggcgcgctggagcaagcggtgctggccaaccagcgtgcgctgcagcagctggtcgaccagggcgtgagcctgcgcgagacgcagctcaagaaggcactggccgacatcgagaagatggaagacacgctgtttgccagcgtgcgcaaggcggcgccggccgacggcccctggagcgccgtgttccaggcggcgcagggcaagggcacgggcaccggcgcacgcgccaccgcggcgctcgaacttctcatggaagacacgcacaagaacctgcgcgacggccgtgcgctgagcctgcgcgcctcgcaggcgatgctcgacagctacgcaacgctggtgagcggcgtgctgatcggcatgtccgaagccctgaagcagggcggggcggcgaagcgatgacccgggccggcggcggccgcgctgccgccggcctgaaaggaacccgatggacgcgctgatcctcgcccgcatgcagttcgcggccaacatcacctttcacatcctgtttcccacgatcagcatcgcgctgggctggctgctgctgttcttccgctggcggtggctccgcacgcgcggtggcaccgatgccgtgttggcgcagggctggctcgatgcctaccgcttctggaccaaggtgtttgcgctgaccttcgcgctgggcgtggtgagcggcatcaccatgagcttccagttcggcaccaactggccgggcttcatggagcgcgtcggcaacgtggcggggccactgctgggctacgaggtgctgaccgcgttcttcctggaggcgggctttctgggcgtgatgctgttcggccatggcaaggtcagcgagcgcgtgcatctcatgtcgaccttcatggtggccttcggcaccacgctgtcggccttctggatcctggcgctcaactcgtggatgcagacgcccgcgggccatgagatcgtggacggcgagttccacgtggcgagctggttggcggtgatcttcaatccctcgttcccgtaccgcttcgcgcacatgctgctggcatcggcgctgacctgcgcgttccttctgaccggcctgtcggcctggcaggtgctgcgcggcgcggggcagcgcagcgcggcccgcgtgatgcgcgtggggctcacgctggcggcggttctgattccggtgcagatcgtggtgggcgacatgcacggcctcaacacgctcaagcaccaaccggccaagatcgcggcgatggaaggcgtgtgggagaccgagcgcggagcgcccctcttgctgttcgccattcccgatgaccggacgcgcagcaaccgcttcgagatcgcggtgccgaacggcgcgagcttgatcctcacgcacaaggccgacggcgagatccgtgggctcaacgactttcccgatgcgcacccgccgccgctgccgatgttctttgcgttccgaatcatggtcggcatgggcatgctgatgctcgcgaccagctggctcggctggtggctgtatcgccgcacacgctggcagccggcgaagctgccgcgcgcgctgctgcggctcttcgcgggcatgaccttctcgggctgggtggccaccgtggcgggctggtacgtcaccgagattggccggcagccctacattgtctacggcctggtgcgcacggccgacgtggtgtcgaaggtgccggccgcgatgatcgggctcacgctggcgctctacgtggcgctgtatctcgcgctcatcgtggcgtacgtggcggtgctcaagtacatggccgaaaagcccgacgaggtgctggcgacggaggcggccgaacaggccctgacaccggcgggcgcgatcacctcgccgattctcgatggaggccgcgcatgagacgccgggccgctcccaagtcgaatggcaccgcagcgcgcagcgcggaggttagccaatgaacgcgatgatgagtttcgacgccgcattgccggtgatcttcatggcgctgatgggcgtgtcgatgctggtctacgtgatcagcgacggctacgaccttggcgtgggcatgctcatgcaccgcgccaccgacgccgagaaggacgtgatggtcgcctccatcggcccgttctgggatgccaacgaaacctggctggtactgggcgtgggcatcctgctggtggccttccccaaggcgcacggcctggtgctgggcgagctctacctgccggtggcgctgatgctgatcggcctcacgttgcgcggcgtggccttcgattttcgcgtgaaggcgcgcgacagccacaagcgcacctgggaccggctcttcttcgcgggctccacgctggcctcggtggcgcaggggtggatgctggggcgctacatcagcggcttcggcaccggctggaactacccggtgttcgctgccgccatcgccgtggcgctgccgatggcctacgtgctgatgggtgcggcctggctcatcatgaagaccgaaggcgcgctgcaggagcgcgccgtgcagtgggcgcgtaccgcctgggcgcccatggtcggcggcatgctgctgatctcgatggccacgccctggatcagtcccgaggtgcgcggacgctggttcgcactgcccgaaatcctggcgctggccgccattccactcatgaccggcgcggcgctgcttgccgtgcgcgccctgctgaatacgcgcatggtgcgcgggccggtgtgctggctgccctttgtgctgctggtcatggtgttcgtgctcggcttcctggggttggcctacagcatctatccctatgtggtgatcggccagctcacgatctggcaggcggccagcagcgcaccggcgctcaaggtgatcctggtcggcgtgtgcatctcggtgccggccatcgtgggctacaccgtgttctcctatcgggtcttccgcggcaagaccggcgaactgcgctatgcctgagcagacactgggcctggccgaaaccgcgcgtgacacccggcaccgggcagccactgatgcggccttcgcggccttgtgcaataacgggctcatgatttcacgggagccgacgcggcacttcgacttgccttctcatacccgcagacggtggcgcagcctgccgcgctggatcggcgcgctggcgctggtggcactggccgccttcgccggccatcacttcgccttgcaaaacggcctggcgcggctacgcgaagcggccgaccaccggctcgacatgctggcgaccgggctcgatgccgacctggcccgctttgagtatttgccggcgctgctggagatgacccccatcgtcccggcgctgctgcgcgcgccgtcggacggggcgctgcgtgacgcggtcaaccgctatctcgatggcgtcaacgccgccgcaggcgcggaaatgctctacgtgctcgacgccgcaggcacttcgctggcagcttccgattgggaccgggccggcaccaccgtcggccaggacctgtcgttccggccctatgtgatcgatgcgctgggccagggcaagggccgcttctacggcgtcggcatcaccagccgcaagcccggctactacctctcgtacgccctgcgccgcgaccagcccgtgcgcggcgtggtggccgtcaaggtcaatctcgaggagtccgagcgcgcctggcgcatgctgccgggcaacgtggcgctgatcgaccagcgcggtgtggtgatccttgccacccgcgaagacttgaagttccggccgatgctgccgctggacccctcgcagcgggccgaggtgctgcgctcgcgcccctatggcgaggccggcctgcagccgctgcaatggacactgaaggaggcactggcgcgcgacgtgcaggtcatttcgctcgacggcgtggaccagcttgcctcgaagcgctcgctgcgcggtgcgccgtggcagctgatggcgctcgacgacctggcgccggtgcgcgtgggcgcgcgcaacgcggccatcaccgcgagcctggcgatggcggtgctgctgctgcttgccgtcacgctgtggcagcgccgccgggccgtgcggcagaagctggccaatcaggcggcgctgcaggcggcgcacgactccctcgaatcgaccgtggccgcgcgcaccgcgcagctgcgcgccgcgcagggggaactggtgcatgccggcaagatggcggcgctgggccagatgtcggccggcgtggtgcacgagctgaaccagccgctcacggcgatgcgcaccctctccgaaagcgccgccatcctgctcgacaagagccgcttcgacgacgtgcgcggcaacctgcagcgcattcgcggcatggtcgaccgcctggcgcgcctgacctcgcagctcaagaccttcgcgcacaagagcgaactgccgctcgcgcccgtgccgatggcgcaggccgtggccgacgcgcaggccatcgtcgccgaatcctcgaagaagaacggcgtcgccatcgaggtcgacgtgcagcccgccacggtgagcgtcatggccgaggaggccgcgctgggcagcgtgctcgtcaacctgatgcgcaacgccatcgacgccatgcaggcctcacccgcctcacggcgcacgctgcgcctggaagcccggccgcaggacggccgcgtgatcctgcgcgtgagcgacaccgggcccggcattccgcccgacatcctgccgcgcctgttcgagcccttcgtcaccagcaagccggcgggcaccggactcggcctgggcctcgtgatctcggcacaattggtgcgggccatggacggcacgctgcgcgccgccaacctggcggagggcggcgcgtgcttcgtcgccgacctgccggccgccgttcaggccattcttattcccacccccacaggagtgatcaacaagtgagcgaagcccctgccatccgggtgctgctggtcgaggacgacgaagacgtccgcctcagcacgatccaggtgctgaccctggccggtttcgaggtcgaagccttcgcgagcgccgaacgcgcccgcccccacatcagcttcggcgtgccggccatcgtggtctgcgacgtgcgcctgccgggcctgagcggcaccgaatggctgctcgaactccaccacaccgacgccgagctgcccgtgatcctggtcaccggccacggccacatcgccatggcggtgcaggccatgcgcgagggcgcctacgacttcatcgagaagcctttcagctctgagcggctggtggccatcgtgcgccacgccatcgagcgccggcagctcacgctgcaggtgcgcgcgctgcgtgacgcgctggaaaactggcacggcatccaggcggtgctgatcggccgatcggcgcagatgcagcaggtgcgccgcaccgtgatgaccttggccgaaacctcggccgacgtgctgatctatggcgagaccgggaccggcaaggagctcgtcgcccgctgcctgcacgagcacagcgagcgccgccgccagcacttcgtgccgctcaactgcggcggcctgcccgaggcgctggccgagagcgagttgttcggccacgaggccggcgccttcaccagcgccaatcgcgtgcgcgtgggcaagttcgaatacgccaacggcggcacgctttttctcgacgagatcgagagcatgccgatggcggtgcagatcaagctgctgcgcgcgctgcaggagcgctccatcgagcgcatcggctccaacaaggccatacccttcgactgccgcgtggtggccgcgagcaaggacgacctgaaagacatgagcgaccggcagaagttcagggctgacctgtactaccggctcggcgtcgccttcatcgagctgccgccgctgcgcgaacggcgcgaggacattcccctgctgttcgagcatttcacgctgctggcggctgcgcgctacgagcgcgccgcgccgatcccgagcagtgcgcaggtcgccgacctgatggcctatgcctggcccggcaacgtgcgcgagctgcgcaacgtggccgaccgcttcgtgctcggcctcctgggcgagcgcctgacgcaggtgcgcggcaacggcgaagacatgcccgccttgccccgcggactgccgcagcaagtcgagtccttcgagcgggcggtgatcgtcgagacgctgcgcaagcaccagggcgaccagccggccaccgccagcgcgctggccatcgcgcggcagacgctgcacgacaagctgcgcaagctcggcattgcggcggacgagttcaagtcctaggggcgcaagatcgtccgatcggttgtgtcggcctaccagcgctgcggcaggcggcgagatgtgtggaacacgcgcaggatttcgacggtgtcgcctcgcacgcgataggggacgatgtagcgggtctttggcacgatcaattcgcgcgttccaggcacgcgtccaggccgaccgaggcctggctgaagtgcaagcatggccaccgactgaaaaattcgaccgacgaccagcctggccgcagccgcatcgtcggtggcgatataggtggcttcctcgtccaggttacgcagagcggcgcgcagccacttaatccgcattcaccttccattttcttgcgagcgctgcaacttccttgtcgcttgcgaagtcttcggcgtccgcttccttcagcgcagcgcgcacttcgccgatctgccactcattggtttcgacataggcgcggatcgcttcggcggccaggaacgacttgctgcgctgagtcgcatcggcgaggtggtcgagccgattcttgacttcgtcgtcgagtcgaatggtcatcgtggttgacatcagtaaaaccaggttcgtattcggatgtacacatcctagcacgacggcctcgcgtgtcgattcacaggggcatgctgagccagtccggacgccgggtcggcaaacgcaaccttgcatcggcacggccaatcccgtacgctggcccaacgtccacgcgcagcacccgagcccttgcgggccgccgggccggccttgcggacgccaaggagacatgccatgccaagccgatcgaacggcctcacggccgaaatggaagcggtgcgaacgctggcgctcgtcggccccgcagccgcgggcaagagctcccttgccgaggccttgctgcacaaggcgggcgccatcggggcgtgcggcagcatcgagcgcggcagcaccgtcagcgactacgacccgctcgagcgccgcatgcagcactcgctcaacgcgtcggtgatgcacctcacgcatgccggcacgcgcatccacttcatcgacacgcccggcggtcccgacttcctcggccagagcctgccggcgctggaggcggtcgaaacagcggcggtggtcatcaatgccgccaccggcatcgagccgatggcggtgcgcatgatggagtacgcggcctcgcgccacctcgcccgcatgatcatcgtcaacaagatcgacgcgcagggcgtctcgctgtcgggcctgctggccgacatccaggccaccttcggccgcgaatgcctgccgctgaacctgcccgacagggtcggcaagcgggtgttggactgcttcttcaaccgcttcgggcagtccgacttcggccccgtcgaagcggcgcaccgcgcgctggtggagcaggtggtcgaggtcgacccggcctttgtcgaccgctaccttgaagagggcgacgtggatccggcggagctgcacgcgccgctcgagcaggcgctgcgcgaaggccacctgatcccggtgtgcttcgtctcgtcgcgcagcggcgccggcgtggccgagctgctggacgtgatcgtcaagctcctgcccgacccgaccgaagccaatccgccggagttcctgctcggcgagggcacggatgcgaagccgatgcaggccacgcccgacccgtcgctgcacgtgctggcgcacgtgttcaaggtcacggtcgacccctacgtcggcaagctcggcatcttccgcgtgcaccagggcacggtcacgcccgacagccttctttacgtcggcgacggccgcaagcccttcaaggtggggcacctgttcatgctccagggcaaagaccatatggaggtctcgcgtgcgataccgggcgacatcgtggcggtggccaaggtcgatgaaatccatttcgacgccgtgctgcacgacgcggcagaagacaaccacatccatcttgcgccgctggcgttcccggtgccggtgcacggcatggccgtggagcccaagcggcatggcgacgagcagcgcgcctgggagattctcggcaagctcgcggccgaggatccgtgcctgcgcatcgagcatgcggccgcgaccaacgagacggtgctctacgggctcggcgagcttcacttgcgcatcgtgctcgagcgcttgcgcgaggtgtaccgcttcgaggtcctgacccggccgccgcgcattgcctaccgggagacagtgagcgcgccggccgcggggcatcaccggcacaagaaacagaccggcggcgccggccagttcgccgaagtcttcctgcgcatcgagccgctggcgcgcggtgccggctttcaatttgccgacgaagtcaggggcggggcgatcccgggccagttcattcccgcagtcgaaaaaggtgtgcgcgaagtgctggcgtgcggcgcgatcgcgggctaccccgtggtcgatgtgcgcgtggtggtgcacgatggcaagcaccacagcgtcgacagcaaggacatcgccttcgcgaccgcaggacgcaaggccttcatggccgcgatccgcgaggcccggccagtcgtgcttgagccgatcgtgcagatcgagatcgccgtgcccgaacattcggtgggcgacgtcacgaacgatttgtcgtcgcggcgcggcctggtcaccggcacgtcgcccatgggcgccggcaccgtggtcgtcggcgggcaggtgcccgaggccgaactggccaactaccagtcgcggctcaatgcgatgaccagcggccagggccgctacacccttgcgttatcccactacgaagccgtgccgccggccgtccagcagacgctgatggggcagtatcgggtgcgggaggaggattaagtcaggccgggcccagccttccgccaagcgcatcgtcgacgttgcgatgaaaacgcagcacctcgtgctcgagccggccgagatggaaatgcgtgttggcgccgctggacaggccgcgctggatcgccaccgcggtggcgatgtcctctttctggaagacggtctgctcgatgagctggaaggtcttctcccaatgggcggtccaatcgtcgccggtgcggtccggcggaatcagcatcgtgtgcacccagcggacctgatccggcgccggcgaaaacatgccgatcaggctcacgtagtcggggtgccagatgagaaaggtgttcgggaacacgagctgcgtcggcgtggcgagcttgcacagtgcgtcgcgaccctgcggcggctcgaaggcctcgaaggccgcgcgccgcgccaccagcgagtcctggtgcggcccggcatgcaggttgaccgtgtacgcgtcggcaaagaagggatagatcgtgtcgcggtgcagcacgcggatgtgatagccctccaggaaggcatcgaccgtcagcttccagttggcctggtacacccggtcgaccttgcggaacacggtcatccggggcaggcccatccagtccatgtgcgcgcccagcccttgcaggaaggccgcggccgaaaacgcggccccggggctccgcttgacgacgaccagcccgctggcttcgtcgcagggcagttcgaccaggttcagcgtggcggggtcgatgccgtcgaaggtctgtgcatgcaggcgatggcgcagctgtccatcgagttcgtaggtccaggcatggtagggacagaccagggccttgcaggccttggccttggccggctcggcgccggggtcggagctggcgatcaatgccatgccgcggtgccggcagacgttgaggaaagcgcgcacgcggccatcggccgcccgggtcaggacgatggggacgccgagagcgtcgaagggcagggctgatccgatcggaatttccgaactgtgggccgcaacgatgggccactggccgaacagcgccgcctgctcctgctgccaatgcagcgggtccgtgtagtggctgaccggcacggtgccggactgctcgccttcctcacgcgtttgggtgagccgagcctggtcgagacggcggaccatgtcggccagcgtcgccggcatcggtgcagcagtgttcggattgatcatcgggatcgcttcgcatcgtggtgagccatggaacagccctcagcttaggttgaatgcgtgccggacatgttcagctttcgtgggaggtcgccggcaggtgcgcagccctggccctccggcgcattgacgcgaggcgtgttcagcttttcccggctcgcgcgggccgtcttgcacccgccgcggtgaaccccgaagatgagccccttcctccatgggagctcgccatcgcccacgcatgaattcgatcgtcagacctcgccgcaagcccgtgcagtcgcgcgcctggatgaccagttgcgcgatccaggatgccttcgtcatgctgctggtcgatcggggctacgagaagatctcgatgcgcgagatcgcaggtgtcgcgggcgtcggcctgggcaccctgtatctgtactttcccggcaaggagtcgattgccgcggtcaccatccgccgctggatgcgcaagcaggccgcgatcctggcggaggcctccaaggtgtccactccacgcacggccgagctggcggcccgagccatggtgcaagcgcacgtgcgaggcctgctcggccaggaaaacgagtggcgcgcgttgcttcatctcgaacgccgcatctcttcgcccgccagctaccgcgagatctaccgcgaattcgtcggcctgttccgcgatgccttcatcgcctcttctgactggcctgtgggggccgacccgctgcgcaccgcgttcaatgcgttctcgatggtcgatggcatcgtcgggcatgcgctgctggtgcacgaggcctgcccggatgcgggagaactggcgagcgacgtggagtgcgcggtgtccggttacatccggtccgtacaggcgcaggcgcgtcaaaccggcgccatggagacatgctggccagcccctgcatgacgccgctgctgcgggatttcaccaaggccctacggccgcaggggcggcgcatacttgctgcagcgccgctcgtcggcccctccggggttccgggcgactgtcaggaggcacgccttgcagcgaaccgacatagccaacccggcctatttccacaaggtcgtcgattgccagtacgcctgcccggcgcacacccccgtccctgaatacatccgcatgatcgcgcagcgccgctacagcgacgcctacatgatcaactgggtttccaacgtctttcccggcatcctggggcgcacctgcgaccggccttgcgagccggcctgccggcgcgggcgggtcgaggaaagcaacgcgaaggatcccgagccggtggcgatctgccggctcaagcgcgtggcggccgacatgaaggacgatgtgcgtgcgcgcatgcccaagctcgcacccaagaacggcaagcgcgttgcctgcgtcggcgcggggcccgcctcgctcaccgtcgcgcgcgacctggcgccgctgggctacgaagtgacggtgttcgacggcgatgccaaggccggcggcttcatccgcacgcagatcccgcgctttcggctgcccgaatcggtgatcgacgaggagacgggctacatcctggacctgggcgtcgaattccgcggcggcgagcgcatcgactcgatgaaggcgctgatggccgaggggtgggatgcaatcttcgtcggctgcggcgcgccgcgcgggcgcgacctggaccttcccggccgccaggaagcggcggccagcatccacatcggcatcgactggctcaactccgtctcgttcggccacgtcaccagcatcggccagcgcgtgatcgtgctgggcggcggcaacaccgcgatggattgctgccgatcggcccgccggctgggtggcaccgacgtgaaggtcatcgtgcgcagcggcttcgaagaaatgaaggcctcgccctgggagaaggaagacgcccagcacgaaggcattccgatcatcaacttccacgtgcccaaggccttcgtccacgaggagggcaggctggtgggcatgcgtttcgagatcgtccaggccgcgtacgacgaccagggccgccgcacgctggtgcccaccggcgcgccggacgcctgcttcgaatgcgacgaggtgctggtggcggtgggccaggaaaacgccttcccgtggatcgagcgcgattgcggcctcggcttcgacacgtggggcctgccggcgctcgacaagaacaccttccagtcgacggtgcccaacgtgttcttcggcggcgatgcggccttcggccccaagaacatcatcacggccgtggcccacggccatgaggccgcggtgtcgatcgacaagctgttgcgcgccgagccggtgtacgttcgcccgccgcccatgactaacctggtgtcgcagaagatgggcatccacgagtggagctatgacaacgacacctccaacgacctgcgctacaaggtgccgtgggccaaggccgaggcggcgctggccagcatccgggtggaggtggagctgggcttcgacgccgccaccgccttcaaggaggccgagcgctgcctgaactgcgatgtgcagaccgtgttcaacgagaccacctgcatcgaatgcgatgcctgcgtggacatctgccccatggactgcatcagcttcaccgccaacggcccagaagccgagctgcggacccggctcaaggcgccggcgctcaacctggcgcaggacctgtacgtgtccggtggcctcaagacgggccgcgtgatggtcaaggacgaggacgtctgcctgcactgcggcctgtgtgccgagcgctgtcccacgggggcatgggacatgcagaagttcttgctgaagatgacgccggcggggcagggggtggcgcaatgagtgccgtacggccgcccgaaagggtgaatgaaggcgcgaatgatggcgcgaaggaaatggagagcctgggcctcatcccgcagatcgaagcggtcaacgatttcgtcatcaagtttgccaacgtcaacggctcgggttcggcctcggccaacgagctgttcgccaaggccatcctgcgcatgggcgtgccggtgagtccgcgcaacatcttccccagcaacatccagggcctgccgacgtggtacgaagtgcgcgtgaccgaagcgggccacctggggcggcgcggcggcaccgacatgatggtggcgatgaacccgcagacctgggatgccgacctggccgaactggagcccggcggctatctcttctacgacagcacgcggccgctgccgccgtcgaaattccgcagcgacatccgcgtcatcggcatgccgctcaccgagatctgcaacgccgtctaccaggacccgcgccagcgccagctgttcaagaacatcgtctacgtgggcgccctggccatcctgctcggcatcgagccccacgtcatcgaagagctgttcggcgaacagtacaagggcaaggaaaaactgctggcctccaacgtgcaggcgttgcacctgggctgcgacttcgcaagggaaaacctgcgcgaacccctggggctgcaggtgcggcgcgccgaccgggtgggcgaccggatcttcgtggacggcaacagcgccgcggcattgggctgcgtgtatggcggcgccacggtcgcggcctggtatccgatcacgccgtcgtcctcggtggccgaggccttccagaagtactgcgccaaattccgtgtcgacccggccaccggccagcaacgattcgccatcgtgcaggcggaagacgagctcgcctcgatcggcatggtggtcggcgccggctggaacggcgcgcgggccttcaccacgacctcggggccgggcgtttcgctgatggccgagttcatcggcctggcctactttgccgagatccccgtcacgctcatcaacgtgcagcgcggcgggccttccaccggcatgccgacgcgcacgcagcaggccgacatcctgtcctgtgcctacgcctcgcatggcgacaccaagcacgtgctgctgtttcccgaggacccgcacgagtgcttcgagcacgcggcggccgcgctggacctggccgaccggctgcagacgccggtgttcctgatgacggacctggacatcggcatgaaccagcgcctgtgcgcgccctttgcctgggacgacagcaaggcctacgaccgcggcaaggtcatgagcgccgaagagctcgaggcgggccgcgacttcggccgctacaaggacgtggacggcgacggcattccctggcgcacgctgccgggcacgcatccgaccaagggcagctacttcacccgcggcacgacacgcgacgcctacgcccgctactcggagcgcgggccggactacatctacaacatggagcggctgctgaagaagttcgcgaccgcggccacgctggtgccgcagcctgtgctgcgcccggccgcccaaaagaccgagctgggcgtgatctatttcggttcgaccagcccggccatgcacgaggcgctgcaagcgctggaagaacgcggcatccacgtcgatgcgctgcggctgcgcgcctttcccttcccggacagcgtggtccgtttcctggcgcagcacgcgcaggtgttcgtggtcgagcagaaccgcgacgcccagatgcgcagcctgctggtcaacgaactggacatcgatcccgcacggctggtcagggtgctgcacttcgacggcacgcccatcacggcgcgcttcatcgtgcggtccatcgacacgcacctgcaggcgcaggcatctggcgccgccgatccgaaggagcctgcatgacctacctcgccaagccccggctgcaccacccgacgctggccaccaacaaggtcggctacacgcggcgcgactacgagggcaagatctccacgctgtgcgccggctgcggccatgactcgatctccgccgccatcatcgaggcctgctgggagctggacatcgaaccgcatcgcgtggccaagctctcgggcattggctgcagctcgaagacgccggattattttctgggtgcgtcgcacggcttcaacaccgtgcacggccgcatgcccagcgtgctgaccggcgccaacctggccaaccgcgacctgctgtacctgggcgtttcgggcgacggggattcggcttccatcggcctgggccagttcgcccatgccatgcggcgcggcgtgcgcatggcctacatcgtggagaacaacggggtctacggcctgaccaagggccagttttccgccaccgccgaccagggctcgaagagcaagaagggcgtcgtcaacaccgacagccccgtggacctcgttgccatggcgctgcagctgggtgccagctacgtgggtcggggcttttcgggtaacaaggcgcaattggtgccactgatcaagggcgcgatcagccacggcggggccgccttcatcgacgtgatcagcccctgcgtcgccttcaacaaccaccccggcagtaccaagagttacgactatgtgcgtgagcacaacgaggcggtgagccgcatcgacttcatcagtgggcgagaagaaatcgccgtcgacatcgagccgggcgaagtgatggatgtgcgccagcacgacggcacgctgctgcgcctgcgcagcctgcatcccgactacgaccccggcgaccgctacgccgccatggcctacatgcaacggcaccaggaaatgggcgaggtggtgaccggcctgctcttcgtcgacccgctggcgaccgacctgcacacggcgctcaacacctgcgaccggccactcaatgcactggggcccgctgaactgtgcccgggcgcccaggccctggaacggctcaacgccaccttgcgctgagcggcggttcgctgcaccattgccatccttctcttctggagggcgcatcatggccgagcgcaccgttttccaatccatctcgcgcaagcatgtggtcagcctgggcccgcaggccagcgcgcgcgacgccgcgtgcgtgatgacgcgcgcgaactgcggcagcgtgctcgtcatggagctgcccgacatcctgctgggcatcctgaccgagcgcgacctgatgacccgcgtgctggcccgggggctcgacgccgatcgcaccgcggtgcgcgaagtcatgacgcccaaccccatctgcgtgccgcccgaaacgctggtgtccgacgccgtggtgctcatgctcgaacggggctttcgccatctgccattgatggcgggaacgaagatcctcggtgtgttctcggtgcgcgacgcgctgccgcgggagctcggcacggcggtgagcctgaccgaattccgagagcaagtgaatgacgcgctggggtaggagctaccgtctccgaaggacgattggatggcaagattcattttggtgccaggtggttggcacggggcgtgggcattcgaagctgtcagccatgcgctatcaagcgaaggccacgaagttcaggcgctcactctgtcggggttggacggcgagcctgcgaatggagccaatctcgaacgtcatatcgacgaggtggttcaaacggttcgcgggcgcgatacgaaagccgttcttgtcggtcattcgtatgggggcatggtcatcactggcgcggcggacaaggaggcatcgcgcgtcaaggcgatcgtctacgccgatgcctatgtgccggacaacggtgcatcggtttggtcgctcaccaccacgaactatcgggagcgtttcatagcgggtgtggctgcggatggtttgacttgcgcgccgccggcccatctagacagccgatgccgccctcatccaatcgccactttcctgcaggcgatcaagctgactggcaactggcgcaacgtccgcagcaaagccttcatcgccgcgtgcggctgggaaggaagtccgttcatcgagttgtacgaacgtctgcgactggaccctgattgggcgacgcatcgcctcgactgcgcacacgacgttccgcggctggcccccgaagctctcacgaggattctcttgaagtacgtgtaggcaagccgagcgccggctgttcattccaagtagtcaatgaactgcgggatcacctcgcgcaggaagcggatttcctctgtgggaatgctgcgcgactccaagtcgaaatggatgaaggtgccatagggcgtgccgcatcctcgcgtcagcagccggccgtagtacgactcgaccatgccggcatacggtcggttcgtcaggcgctgatctccggaggcatggctggtcacgaactcgccgtgctcgagcgcgtactggcagaagctcttgcccagaggcaccaccttcagccaggtgcggtattcagagtcgcggtcgaaggcatgcgccgcgcgcatcacgtcgccgttcaatttgtagatcgccgtgaaccgataggacgtcctgtcgttgagcaaggccagcgccggagcgatgccgcggctggcaagaaggctgcgaacggccgcagcaggcgctggcaagtcgacgtcgagcatgggtactttggttggggcgtgggcgcgaatcttacgtaattcttgctgtgctctggaacagggtttgaccctcatcttgtcaacgaaaacccttaagtaccccgcgagtctcgcggctctgcaccttcgactggccgggcgcttcggaagggcgcgcgccggccgtgggagaggcagaatgcggccaacctgtggagtttcacgcctcttcatcccgctcagatcatcctgcgttgccaggcacaggcgtgttgagcagctgctgctcccacaggaacgcgatgccgctgccgccggcatgctgggtgatcacctccgtcagtgctgcggcttgatcggtccgagcccaatcgcgctgccattcggcggcgagcgccatccaggtcatcatgttcgcgccggccgcgatcatgcgctggatggcgacctcatgcgcctcgactgaaacaccgcccgacgcatcggtgatcaccgtaacgtcccagccttcgccgagggcctggattgtcggcatcgcgacacacacttcggtccacaggcctgcgatgaccaactgcttgcgacccgttgccttcaccgcgtccaccaccttctgatcctcccacgtgttgatgaacgtgcggtcgatcacctcttggccggggaatacgtcggtgatctggggaaagaggagcccgcctcgcgcagcgatcaccgtcgtcaagatggtaggcacgccaaaggccttggcggccttcgccagccccgccgtgttgttgatcaccatttgcggttcgtggctgttcacgttcgcgagttggtaaggctggtggtcgatcagaacgagcactgaatcttctggacgaagaagcgaagtaaggccgttgcgaaaagtcattgatgcatcctttgttgccgctttgagcgggattgaattgcggcgaacgttcgcctgtggcgacgttgcctggatgcattgtgttgttcccagttgcgatgcggtagtaccatttcgcggcgagctgtgtcgcgaaatggggaacgctcagttggacatcgaagagctacagaccttcgtagaagttgcagatgccgggggggtgtcggctgctgcgctgcggctcggcgtggccaagtcgatcgtcagtcgtcggctgttgcggcttgaggcggaacttggtgtccagctgctctcgcgatccactcgcggggcctcgctcacagaagccggggccacattccgggaccatgcggccagggtctgcgccgagatcgacgcagcccgggatgcgatcctgcccgccggcgaccttcgcggccgtttgcgggttgcggcgccgctttctttcggccccactcacttcgctcccatcctcgcggaaatggcacgacgccatcctcagcttcacatccaggcctgctacagcgatcggttcgtcgacctcattgcggagggctacgactgtgcgatacgggttggctatcttcaggactccggcttgatcgcaagacgaatcggtcgtatccatgggaagctggtcgcaagcccggactacgtcaaggcgcatgggtcgcctgagaccccagaggagctcagcgcccaccaagcccttatgcagggagccgaagcctggcaactcatggacggcgacaggatcatcacggttcatccgcaggggcgcttcaagagcgacaacggcacggcgttggtcgccgccgcgatcgcaggactcggaatcgcgtacctgcccgattggctcacccatgagcatctggcctccgggacacttgtgccggtcatgacacgtcatccaccaccgccggcaggtgcctatgtcatccgcccgccaggtcagcatcccgcacggaagattcgggtcctcaccgagctcctgatcgagtattgcgaccggtctccacaccttgcgggagctgcaccggtctgagtgcgcatcgacgttgatgctcggttccagggtgaagccaacggaacgccaagggcagcaacgggcccaaagctccgaggccgcgaccggctacagtcggccagaagccgacctcctaggcgtggctccgctacccttctgccaaatggaaaagatcaccgtcaccgccgcgacgcccgaagaactccgctccggagagctcggcctcaagctgcgccactacaactacagcttcgtcggcgagtatcccgagcagcagtacatccgactcaacgccagggacgggaatggccggttgctcggtgggctgcgaagctttgtgtttctctactggctcaacatcgaagtactgtttgtcgaagccgacgtgcgcggctcgggcctgggcagccgcctgctcgccgaagccgagcggcaggccatcgagttgggtgcgacgaacgccaagctcgacaccttcgagtggcaggcgcccgcgttctaccggaagcacggctacgaggagtacgcgcgcatcgacgactatgcgcccggcttctacctggcctccatgaagaaatcgctggtgcgctgagcagcgatacaagcttggcccgatcagagaagcggaccttcgtggctcaggcctgggtgatcctctgtcacgactagactcctggacaccatgaacctcccccggaacacgatctcgaccaaagcgcacgctgtgcccatgcccagcaacagcgtgctagcgcctctttacgcgaacgcggatctgttggacgcctttgcaattcaactgccggtggaggcgagcgatgatctggaggtgctggcacgcacggcgttcgagagccaggcggggtggattcgtgcgctcacgtgtgtccgcgatgtggtgatggcgacagttggcgtcaaatcgtctggcgccgtcggtcttgccggagcggcgcgtgggcgggttatcggctacctaccgctgctgtcaaagagcgctacggagttgatcgtgggcgcggatgaccggcatcttgacttccgcgtcaccatccaacttcgcgccgatgcagcaaatggtcgcgagctgctcgcaggcacggtggtgcattgccataacagactgggacgtatctatcttgcgacgattgctccgtttcatcgcgtgattgtgcgggcgaatttggaacgggcagtaagagaaatgaggacttgagcatgtgtagggagccacagttgctgcgccctgtgcacagttgctgcgccctgtgcacagttggtgagcctggccgttcgaagatggttagcctttcccacgggggcgtcgctgtggcatcctccggccagccgccttccggccagccgccttccggccagccgccttccggccagctgcggacattcgaggccgcgccaaattccgtctgcttcttggtcctgaatcgtcaagcatgtctcaagttcatttgatcgagggcccagtcggggccggaaaatccaccttcagcgcagctctggccgcaagcagcgatggcgtgcatatcccgctcgacgagtggttcgcagcgcttttcagcccagaccgcccggagggcgattttgtgccttggtatgtccagcgcaaggaacggttgctgggcctgatatggaaccacagccgcagaatactggtgtcaggtcgaaacgttgtcctcgagcttggtctgatccagcagcaaccacgaatccagttctgtcgaatgatcacgaacgaagggtttccgcttcacctccatgtcctcgacgcgcccttggaaattcgtcgtgggcgtgttcgacgcaggaatgaagagcgaggtcctacgttttcgatggtcgtgccggaccatgtctttgagatggcgagcaagatttgggagccaccggacgcactggaatgcgaagagttcgaggttagcttcgtcactgaagggtcgaaggcgtcgtttgacgcttgaggaagccggccagcacgcgtcttgaaagtcggctgtcgagcaaatcaaaagccggctttgggccctttgcgccttcagctcgtgcggctacagtcggccaagaccagacatccgaccagcacctccagtttgcgtccaagaacaagctcatgaccagctacatcagtctcagagaccgaaggttcgacgtcacgtcagcggtggttcgccaattcgacggactgtggagcgtggagattgagacggagccgaaggagttcgatggcgaaatgtggtcacccaggctgtatcaccagggtctgcggctgctgacgcatacagaaggcaatccggaaggcgcgagcacctcatggagaaacaaatcggatgtcgcataccctcatccggagttggggttgatgtacgtgttcggccaccacgatgtgtacgacacgacgttggcgttcggtcgcatggacgccgggcacatcgaactcgcgtgggacgggctttgcgacgtattctggtccggcgacttcacagaggccgtaccctttcagtgccgctgcgtcgcatctgtgcgccacggctgatggcaggacgcggccaacagccgtcactcgtgtcagaggctcaacctgaatgaataagggcgagattgcactcaagatcactaatcacgaaagcgttgaaagcctgattggcttcgcctcatcgtggttggtcgatcttggcttcgtatcgcacgcagggccgacctgtgcactgctgatgccagatgaccctgaagagatcgacctgcatgaccaggagcaattcaactggtttcgagcctcagtggtcgagtctctgcacgtggctgggctgaccggagtctgcgtggcggcagggccaactgaccctgctgcggaagacgtccgccgactctgagggcatttggtttcgagcaaccgtaccgcaggcgaggcagaattcggccacaacccgacgctcacaattccgccccacttcgcccatcagcagtcatccatcaacccacatatgtccggtgcgaaggtagtagttcagttcattgctgcagacgttggtggtcgaacaatgcccgcctacttgacgaagaaataccgccctcactttcgcgtcgggagcggagagtacttgggcgtcgtcttttccggcgatgaatcgagcgcaccaattcagcctgggatttgtatgaatgcggaggtaaggttcatctacgtacccaatgtcgactacggggatctagtcgtcggagcacaatttcaaatccttgaaggtgcgcggattgtcggaatcggcgtgatcagtgacctggtcacatgaaagtcccgtcgcggccaacaaccaccgatatcaccagattggagaagatctaatgcttgctcgcattttcttcattgcgctgacagtcgcgcccaccttttcgagtgcagcatgctctgcgaccctgcgctcccctgaccaaacggtggcgatcagcgacaacggatgcgaattttctgaagagatgatcttcgtgagcgctcggacaagtgatcgaaagttcgtcgagctaccgcccatttcgttcaccagtcagtgcgtatggcatgtctcaagccgagactcgaagcagccagacggattccattgcaactcgaatggcgcaactgtattagcaggtacgacctacaaggagacacccggaaggaagaaggtctgtggcgattcgaggtggcccgtctacaaatgcacgaagggttgcacgcaacacaatgtaccgctctattttgagatcgagccttacgaatgctgaatcaaagtctacgggtcatcgggatcggctgccccaaagtcaacaacggccctatgttcattcgacttggtcacatctgcaggtcacggagggcgtaaccacggactgctgaaggacccgaattccgcgcgagcctgaggttcgtcgaagggagttgaggggccttgatccgtccgcgactccggccctgagcctgcttgcaatctcggacctgcccttgggctgatcggcttggcgcgagcggtctggttcgccgtgggttcgtcggcaccaacgaacaacaattggccgactaaacagcaggcagaatccggccatgacccgtcgttcgccgtctgtcttcgtgggtgcggtacatagctgtgacgaactctgaaattgaaaacctgtggatcgaagcttggtcgaaactgatcgaaatagtcaccgccaagtctggcaaataaacagtgatgatgtatgcccagttgaactggtacttagagaggggaggtatcgtgcatatccgtagcgtccgtgcgccttgcggcttgagatctctttggcgtgccagcgggccgacagcgcttctttgtctcgcaatgaccggatgtgcgcctattccatatgccgatccagataacaagaccgaccaagtgccgctcacgattgactatacgggcactcatgtcaatccccaggtatctctcttcctggacccgaagacttgtagcgcacctcgctacattgcgatggatgacactacaacaagaacgatctacgtccctgtaaatcaaccttcaacattgttcgttggcggtgcgcggcttacgggaggattgggtgttgctttttgtcagcgcttcgccatcactgcaagtttcgaccgcggtgctcgctatagattgacccaccatacgagtgacaagcaatgcacgttgcggctcactcgagttgaagatggcgtcacacgcgatatatcttcctctatgagatcgcggcaagagagaaatcctgctctaccggggccgagagatggtccgtattgcgtagatcaatactaggttcgggcgtaagcatgtggccacatccgccctcacaagcagtcgttcggagcagacttagtcagggattttgatgacctcgtatagcttcctttgggacggaaccgaagcaggatgggtgctccttcatatctcgcgttggatgtcgggccttaccgctactttcgacgatggaggccccagtccaagagaaattcaggcactccggcgagcagttccgtcaatcggcgctatgtctgccagcgaagccgttggacagctcgcaggtaggaaaagcgttgctcttggcgagttcgacgaccgcgagggccgacgaattgccaaggaactgcgcgaccatggggtacaggttcaacagcagacgattgaccgttccggttacttgccgttcaacgagctcaatcagcacgtaatggccatcgaagacgaccttgtggcgcgggatgtcactgatgaagctttgaggcggggcgttcctgtgagacatgtggaagcctgaggcgacggcaggggaagcgtcgaaccaccgaccggctacagtcggccaagagctgacttccaaggaagcctcgcagaatcgaagctgcgaccccagcctcagaaatcaccggaaattgcgatggatcgtgtagccgccctaaatttcttgagatccctcactcggacggaactggctttgctcatcgcggaggcggccgaaaagtggactgtaggggatttagcagagggccgctcggtcttccgacttgccgagtgctttgccttcaggggtgttgacgaacaacgccccgaatcagcctacctggccctggtcgcctatccggcgaaaccagaagactacgccggtcacgacggggttgaacaagatggctcgtgctcaaaatgcggcgtggaagtttgttgtgcagcaaaggtggccatttgcccggtttgcggtggagaagcgctctgcacatagccaggccgcgatctacctcagcaaaacttgaaaggcagctttgattgagggcttccaaggacgacttcaggcctcacgcggccctcaagggcttcgactacattcggccaactgcggcccttccaaccagccctccacttcgaagctcatgttcgacctaatcccccaccctacgggtcgcaacgaaaacatcgctcgctccgggcacctacaagccacttggtgaaaacgagcagggcgtgtggtatatcggcgctgatggcaatgttcgaatcttctataccgaaaagaagagaagcgatggcaagaggcttcttgcgagctataccggtggcatcctcgtaccgtccatgcctcatagccagccctcggtttttatcattccttccacagagagattgatgcttgtttcagattcaatggatgccgaggccgtgaagcttgggcaaatgaccgaaggacagatccatgcggaagccgcggtcaacacgggtgcgaatctcattggagcggccttgggaggcgccatcgcagacggcctcctcagttacgacgcacggggcttgagggtgattccgcagactgcgggggcgccaggacttgtgacttggttggatggacgctaaatcactgaacagctcaccgcttcgaggcgatgcaccgtctacttggggctcgatgcttcagcacaatcaaccgagtggtgaggccggtcccggccagaacctgtcgttcgcccgtcctgcagaatccggcagaagcagacgttccacgcgacggcatagtggtgcttgaagaatatttttctctacagctgagatttgctgagcgctacgcggcggttgcagattggcccttgggcgcgtcgatcgcgcactgcacaaacctgcggcggcgtctgaatctttggggacctgcaggcgcaaaccgctggaacgacttcgtcgctcggatcggcgacccgaccaatggcaggcgcgatgcgctttccttatgcatggagtggtacgaggatcgtccacgcctcgctacagggcggtcgttcggctgcttctcgttcgatccgcccgacgccagcggcgttctccgcattcacttcgtccctccggagaacacaagcacaagccctctggcttccgcgaataccggtgccagagtgcaggagctgtgcgaactgttctcccatgttcgtcgcacggagcgcggcgtcttgtcggttcgcggcatctcctggctctacaacctcgatgcttacaggaggctgttcccgcgctcctatgcaatgtcgattcaacccatcgacgtgccgctgcatctcaacggcagttcaacttggggccaggttttgaactggcgtcaggaggtaaagccggacatgcgtgacgcgctcctggcccgcttggccacgatgagagcagaagcaccttgggaagcctttccgctccaggcgctgaccgccacaagtgacgtcgccgagttttatgagcgctttacctgacttggacctgctaatggcaacgggctgacccctcgcacgtgggtggcagaattcggtcaataccggtcgctcacggactgacctgaaatcgtccggaagcagacgctctcgcaaattacaggttcttcatgaacgatccagcgcgcattcctcaggcgatctttgatgccgtctcgccacttctggagccggagtgggtcgaactgattgttgactacagcgtagacgaaacccaaagcgacatggcggcgagctattcgctccaaaaggacgggcacctcgaagaggttgcaattttgctcccgcatgtcgtagatggattatttcgagccctgagggacagtcttcccgatcgggcgacgcaagcattctcggcctgccgttaccacgttacgcgaagcggctccttcgaagccgagtattcatacgacaaagtcgactgggatgacttgttggcgcgctccggatggaacttcccggacatcgcgaccaagcgagcacagtgaatggcgccgacccgacgtgcggctacagtcggccaagagcggccggtcggcggcgtcgcagaattaaccggttagccgacagtagcggcgcacgcacgacatttgagttcggggatgagagcgctcgcgcaagaaacctatttttcgtttctaccgatacatcgtcggttaccacaagtgaagatatatgacttgggaatatcgaataatgagccgagacggcgcggtcgctatctacgaggtttactactatgaagacggtagggtacgggggtacagcgcggaaccaacgtttcctgcgggcgaaaccgttgaagagctacgagccaactgcgatttgtaccttgctgcactcgggaagccagttctcgaatacagcagttagcggggggcaagttcaggtctgtgcgatcatttgcccagagacctgaaatctcttagcgatgaagtcgaagctgatcgttctgggctggcgtaggtgacatcactgctggatgcagccgggaccgttcatttacttgcgcaactggcctcttttgcaggatcgtctagatgatgcgtgagccccacccctacccagagatttactgcgacttcaacgcgaggatgaccgaccgtgggtattcactggaacgaatgggttcaatccgggatttgagtaagttaggcatcgagctggaaggagccgtcggcaaacgcttcaccttcgtcacggacgatgcggacgaaaacggcgttcctgatgacatcatgtccaacggtgtagtgatcaaggatgagcgatacgggtttcttgcccttcttgatgctccagacgacttctattggcgttcgcaactgattcgctgcgatgaagcgtagttagatctaaatctattgaacggccgctatcgcggatcgcggatgtctccttcgggcccgttgccgactttcgccttcctccaaagccgtcattcccctcgagccgatctgtggcgccggtgcgcctgggtttaaaaaaagcccacggctgacacctatggcggcactggcgcagccgaggcggactgcaaaggctatattccggcggcgttagcggcctcgacagtgccaagcgaggcaatcccatcgcctgagcggtcatccaccagctgtccctgggccgattggccgagaaactccgagcgcgctcaggccacgcgcccggccgtcagcggatagcctgcctcgcgccaggccttcatgccgccgtccagcgcgaccgcgtgcagaaaacccatgccgcgcagcgtcgacgccgccagcgtcgagatgtagcccagctcgcagcaggtgaggatgcgccgcgtgggatcgggcaggtcctggttgacgcgcagctccaactggccgcgcggcagcaggcgcgcgccgggaatgtggccggcctcgtaggcgtcgcgctcgcgcacgtcgagcacgatcaggtcgtcctccgcggcctcgacgcgcgccttgagttcggccagcgacatgaagggcaccgcggccgtcgcttcggcgagcaggctcgccacggtcttgccgccgctcatgttcgtgcgcagcgcctcggtgatgtgcgtcggcatcgtgaggttgaggctgcgcatcatctcggcgaaggcttcgcggtcgcgcgcctgcaggcgcgggttggatgcgatttcctcggcgatcgtcgagtgggtgcgtcccttgtagtcgtgcgcggggcagaccttgagcgccgggtccattcgcagcacgcggttgaacaggctgtcgtagagcgcttcggggttgccgctgggcaggtcggtgcgcccggtggcgccgatgagcagcgtgtcgccggtgaacaggcggtcttccacctgaagacacatcgagtcggcggtatggcccggcgtgtgggtgacctgcagccgcaggcgcccgacgacgatcatctcgccgtcgccgatgcgcatgtccacgaagggcgcggggctcgcgtggtgcatgaccacgggcaccttcagctggcgcgcgagttcgcgggtcgccgagaagtggtcggcgtgcgtgtgggtgtcgatcaggtagcggatgcgcacgccgtcgcgcgcggcgagcgcgatgtagtgatcgatctggctcagctccggatcgatgagcgcggcggcacaggtctggtcgcagccgatgaggtaggactggcagccgccggtcgcgatctgcgcgaagaccatgatgctgcgctcgcgatcaaccgggctgcttcaccacgcgcaggtagggcttcggcgacttccagcccgcggggaacagcttcttggcgtcctcgtccgacaccgagccggcaatgatcacgtcctcgcccttttgccagttgacgggcgtcgcgaccttgtgcgccgcggtcagctgcatcgagtcgagcacgcgcaggatctcgtcgaagttgcgcccggtcgtcatcgggtaggtcagcatcagcttgacgcgcttgtcgggcccgatcacgaacaccgagcgcaccgtcgcattggtcgccgcggtgcggccctcgaacgtgcctggctcgtcggccggcagcatgttgtacagcttggccaccgcaaggtcggtgtcgccgatcatcgggtacttgggcaggtagccttgcgtttcctcgatgtccttggcccagcggtcatgggcatcgaccggatcgacgctcaggccgatcagcttggcgttgcgcttggtgaactcgggctcgatcttcgccatgtagcccagctcggtggtgcagaccggcgtgaagtccttggggtgcgagaacaggatcgcccagccgtcaccgatccattcgtgaaacttgatcggcccctgggtcgtctgggccgtgaagtcgggggcaatatcgttgatgcgcagtgacatgatcgctccttgaacaggttgacgacaaacgctctttcttgccggccatccggcaggactcaaagcatagaacggcgcggcgacggacgccagtgccggcgactcgtcagttccgctccgacagttgttccaggatggccgggttctccagcgtcgaggtgtcctgcgtgatggcctcgcccttggcgacggaccgcagcagcctgcgcatgatcttgccgctgcgggtcttcggcaggttgtcgccgaagcggatgtccttgggctttgcgatcgggccgatttccttggcgacccagctgcgcagctcgttggcgatcttcttcgcttcatccccggtggggcgcgcgcgcttcaggaccacgaaggcgcagatcgcctcgcccgtggtgtcgtcggggcgcccgaccaccgcggcttcggcgaccagatcggtgcacgacaccagcgccgattcgatctccatcgtgcccatgcggtggcccgaaacgttgagtacatcgtcgatgcgcccggtgatcgtgaaatagccggtcttcgcatcgcggatcgcaccgtctcccgcgaggtagtagcccttgagctccggcgggtagtagctggccttgaagcgttccggatcgccccagatcgtgcggatcatgctcggccagggcttcttgaccaccaggatgccgccttggccgttgggcacgtcggcgccggtctcgtcgacgacggccgccgcgatgccgggaaagggcagggtgcaggagcccggcaccagcggcgtggcgcccggcagcggcgtgatcatgtggccgcccgtctccgtctgccagaaagtgtcgacgatcggacaacgcccgccgccaatgtgctggtggaaccactcccaggccgcggggttgatcggctcgccgaccgagcccaggatgcgcaggctcgacaggtcgtagcgcctggggtgcacggtttcgttgccttcggccgccttgatcagcgagcggatggccgtcggcgctgtgtagaacacgctgacctcgtggtcctggatcatcttccagaagcggcccgcgtcggggtacgtgggcacgccctcgaaaacgacctcggtggcgcccagcgccagcggaccgtaggcgatgtaggtgtggccggtgacccagccgatgtccgcggtgcaccagaacacgtcgtcgggcttcagatcgaaggtccacttcgtcgtcagcgcggcatgaagcaggtagccgccgctggaatgctgcacgcccttcggcttgccggtcgaaccggaggtgtagagcacgaacaggggatgctcggcgcccacccattcgggttcacaggtctccggctgggcttgcgtctcgtcgtgcagccagcggtcgctggaagggttccatccgatcggcccgccggtgcgccggtagacgatgacgttcttcacgctctcgcagccgcccagcgcgatggcgtcgtcgacgatggccttgagcggcagctgcttgccgccgcgcacctgttcgtcggcggtgatgaccatcacggcgccggcatcctggatgcggtcgcgcaggctttgcgccgagaacccgccgaacaccaccgagtgcgtggcgccgatgcgcgcgcaagcctgcatggcgaccacgccttcgatgctcatcgacatgtagatgacgacgcgatcgcctttcttcacgccgcgcgccttcagcgcattggccatgcggcaggtgcgcgcgagcagctcgcggtagctgacccgcgtcacctgcccatcgtcggcttcgaagatgatcgcggtcttgtcgcccaggccccgctcgacctggcggtcgaggcagttgtaggacacgttcagcgtgccatcctcgaaccacttgaagaagggcgcctggctctcgtcgagaccttgggtaaacggcgttctccagctcaggaactcgcgcgcaaggcgcgaccagtagccgctgtagtcggcctctgcctcggccaccagcctgtcgtaggcggccatgccggccacgtgggcgcccttcatgtccggtatgggaaacagagggggcgttatttcgttgctgctcacgatggatctcctgttgctcgattcaagacgtcaagtggcctgtccggtttcacgggtcggcatggctgttgagccatgccgcaatcgccgcggcactgcgaaagtcgtcgcaggcgcgagccggaacggtggggtagcgctgattccacatgcgcgccagcgcctggcccggacccacttccagcacgcagcgcacctgccgcgcctggatgttttccatgcattcatcccagcggaccgttcgggcaatctgggcggccagcgcaacgcgggcagactccgcattccggatgcggtcccccgcattgctgaacagcgcgacccgaggcgcgtcgaacggcacctgcgcaagcgtccgcgagaagctctctgccgcatcgcgcatccagggcgtgtgcgatgcgacgttgacccgcaagcgcgtgcactgcgcgcccagcgccgcggccatgcgttcggcgctattcaacgcggcgatcgggccgccgaggatcacgctggcgttgccattgcggatggcgagttcgaggccggcttcgacccgcaaccgttcgagctgctgctcggaaacaccgctgacggccagcaggccgcccggcacacgggcggcgcaacggtccatggcctcggcgcgctgcggcgccagcgcggccgccgtggcgggattgatcactccggccgcgctgaaagcggccagttcgccgacgctgtagcccgccaccgcggccggcgatgcgagcaggggcgccagctgcccccaggcggccagggcaaggccggtcagcagcgtctgcgcgttgtcgttccgctcggcccacgccggatcggcgagtgcaaggcgccaatcgtcgacgcccagccgtgcgcacatgtcgtgcacccgtgcgtcgtccgccagccagggcagcatggtgggatgctgggtgccctggccggaaaaaagcagtgcgaagctcatgaggctggacacacgcgctggatccagcagaccgcggcaagcgtgtcggccgcgccaccgggcgacaggcgccgccgcacgaaatcgtcggcaatggcttgcgctgcccggagcccatccggccgcgcgacgcctcctcgatccagaaagtcttgcgcggcgcgctgagcccagcgcaggccggcgaggccaccgcggtgcgcgagattgctgtcgtccagcacggccatgatgtggaacaaggtgtcgagccgggcctggcggggcgtgaggccctgcgccaatgcctctttcagtgcgggaagcgcggtgtcgaacagcaccggaaacgccagcgccgcttcttcggatgcgctgcgcaggccgtggcgccgtgcagcgatgccgccgggcagagcggatggccgttggcttcgcctgtccagtgcgccgccccagtgccggcgcagcgcatcacgcaatgcttccggccgcaatgcgccgccttgttctcgcagcgcagcgcccgctgctgcgcacaacaggccgagcatgaagatcgcgccgcgatgcgtgttgacgccgccggtggcggcgagcatgcgtgcctccgccgcgatgccgcatcgttcgagcacggcgaaatccgcgccgccgaatccggcctcggcgatctgcgcgaagtagcggcgcaacgagaacaggctgcgcatgaaggtgtgcgcgtccatgtcctcgtggctgccggcgtcgatcaacgtcaccagaccaggcttgggtgccagcgacagttcgtcatacagcgcgagcgtggcggcgcgtccgatggccgcaggcgtgagcggtgaatactgtgcctgccaaagggcgacgtttctcacgcggcgacctccaccagcccggcgtgttcgcaccacgcggcatcgcgctgcagggacacgccgtccagccgcttgaccatcaccgcccgcgcgcgtccggcgcgccagtcgcgccattcgcgccacgccaccgccgctccgtcgccgaagatgagctcgccatccagccggggccgtaccgcgtcgaacgactcgagggcacgaaccgcggcatccgcatgtaccgccccctcgatggggatcgacagatcgagatcggaatccgttcgcacgtgatcgagaccgctgatcgcttgccagccgtagctgccgaacacccgtgccgtcgcatggcacgcgtcgagcctgccagccagctcgcgcacggcatcccgcgccgaaggtggcagcagctcctggactgcggccaggtgcgggaactcctcgatgccatgcaccgcatcacgtggcacctgcaatgcaagccgtcgcctgccccagcgcgcgggggaaggcaaacccagcgccatcgatccgctggacgtggaatgaaccgattggcgcgtcacgaccaggggcagccgatgcatcgcccaatgcgcgaggcactcgcgcgcctcttcatcccatggatggcgcaggacggcggcccagccgctcccggagagccgggcgagttgatggcgacgcagcggaaccatggcgatcatgcaaattcaggcggcgtccagcacgcgctgcacgaccgcggcggcaagctggcggcctccccgttcggcgccatcgcgtgcgcgccggtcgtctgtcggcgcgggagccagcgcctcgcgcaggcaggcctgcaggtcgccccgccaaagcgcacgcacgccccccattgccacgtagttctgcacgccgggagcgaacaccgggttggactgcgacagcgccgtgagtttctcttccggcaacttggtcacgcgcgccatggcggggatgcgcatcacgcggatctcggcatccggcagcgcatagcaggcatcggcaatcaaccccgaggtgatgaagccgccggacagcgcctggtcgtacaccaggcctatcacgcggtggccgcggcgccgcgccaggtcgatgcttgcgccgaggtgcgccatcgcccggttgatgccgagcagttcgtcgcgccggcgcagctgctggccctgggtgtcgatcagcagcaggatcggccggcccgggtgccgtgtgacggtgtccagggtcacgcgggcctgcgcgagtgcgagccggaccccgatcggcgcatgatttgtcgtgccgatcaccgtgagcggctcgccttcgaagatcacttcgccctgcagaaaatcgccgtcttcgcgcatgccgtggtaggggccgaagagctgggtgactagagaactccactgcatgtgatgctcctcggttaaatggtgcgcaatgcgcggacggcttcgaccgaaagctccgggacctgctgcgcatcggcgatgccgagcgcgctccagagccgcatcgcttcgtcgattccggcgttgttggcgctgttggcgccgtcggcgttctcggcgggcagggcgtgcagccgtgccgtgagcaaggcgtgctcctgctccagcgccgccagggtcaatggcctcgattcgccgatcgccgcgatggccaccgcacgaaatgcggcaacatcgtcttcgaccagcgcatcgcagtcgccggtcagccagcggtgcttgccgccggtcgtgcgccagaccagcgcacggtcgcgcgagtcgaattcatccacgccgtgggaggcttcgatcacctcgggccccgacatggccagccgcccgacgtcgctcatcacgatgtagtcggcacagcgcgccacgatgcccatgccgccgaagcagccgttggcgccgccgatcagcaccagcaccgggatgcccgcggcgcgcacgtcgagcagggcgcgcatcacttccgacaccgcgatcaacccggcgttggcttcgtgcagtcgcacgccgcccgattcggccagcagcagcacggcagccggccggtcgcgcagcgcgcgctgcatcaggccgaccagcttggcgccatgcacctcgccaacgccgccgcccatgaacgcgccttcctgtgcggccacgaacacgctgcggccgtcgagcatcgcgcggcccaccgccacgccgtcgtcgaatgcgcagggcacgcccagttgcgccaggtgcgggctcgtgacgcgctcgctcggaggcagccattcatgaaaactgccggcatcgagcagcagggcgagccgctcgcgcgccgagcattcggcgtagctgatcatggccggcctccggcgatttcggccaccgcctggtcgagccgcaggctcaccaccgcgggcgtggcgcccatgtcgttgatcgaaacgcgcacgccggccagcggatggcgcgcgtggaagtcgttcatcacggcctgccagatgggaccgaagccgcgcgccgacgtctcgacgcgcaccgcgcagccgttgccgccggccggctcgagcagcacctcgaggttgcctgagccgacgacgccgaccagcaccggcgcaaaggcaccggccggctggccgccggaaaaggaaaagtccagggtttcgagccctgcgggaacgtcgctcatcatgtatctcctgctaccagtttctgaagcgcttgggcggctgatacaagccgccggaggcgcgcaccaggtcgcgcatgttgcgtgcggccagcagattgcgcgtggcctggcgggggtcgatgcccaggtcctgcggccggcggatcacgccgcggtcgcgcaggttctcgaccgcgcgcttgtcgcgcgccaggcccactgccgtgtagccggccacgccgcggatggcctgctcgcgctccgcatcgctgcggcacatcagcaggttggcaatgccctcttcggtgaggatgtgcgagacgtcgtcgccgtagatcatgatcggcggcaggtccatgccggcctgctcctgcagcgtccaggcgtcgagccggtcgacaaaggccggctgcatgtgctcgcggaatgtctcgaccatctgcaccaccagcttctgcccgcgcggcgtgccggcggcgcctgtgcgcccggcacgcgcctcgcgtccggccttgagccaggccgggctcgcatggcggcggccgcgtgcatcggcgcccatgttgggggcgccgccaaacccagcgatgcggcccagcgtggcggtggagctgttgccatcgaggtcgatctgcaaggtcgagccgatgaacatgtcgcaggcgtagtggcccgccgcctggcagaacgcccggttgctgcgcagactgccgtccgggccggtgaagaacacgtcggagcgcgcgcggatgtagtcctccatgcccagctcggagccgaaggaatgcacggactccacccagcccgcctcgatggccgggatcaatgccggatgcgggttcaatgcccagtgcttgccgatcttgcccttgaggccgagtgactccgcataggtcggcagcagcagctcgatggccgcggtgtcgaagccgatgccgtggttcaggcgctgcacgccgtactcggcatagatgcccttgatcgccatcatcgccatgaggatctggacctcgctgatctgcgccgggtcgcgcgtgaacagcggctcgatgaaattcggacgcggggccttgaccacgaagctcacccagtcggcgggaatgtcgatgcgcggcagcctggtggtcttgccgtcgaccatctcgttgacctgcgcgatcacgatgccgcccgagaacgccgtagcctcgacgatggccggcgtgtcttcggtgttggggccggtgtagagattgccctcggcgtcggcggcctgcgcggcgaccagcgcgaccttgggcgtcaggtcgacaaagtagcgcgcgaacagttcgaggtaggtgtggatcgcgccgatctcgatgcgcccggccgacaccagcttggccagccgcgcgccctgcggccccgaaaagctgaagtccagccgggcggccacgccgttctcgaacacgtccagatgctccggaagggccagcaccgactgcaccatgtgcaggccatgcaccttcgccggatcgacctggaccagtgcgcgcgcgagaaagtcggcctgcttctggttgttgccttcgaggcagacgcggtcgccgggcgagagcaccgcttcgagcagggtggcgatggcttcggtctcgacacgcttgccggcgagccggttcccgagcgcttcggcggcgcgcgccagccgggcattgcggtcgtcggccttggtggtccaggagctgggagtcataggaagaggagttgagggtcgatcgaaaaaaagaagacgcgcctcacaggaccacgaagagcagccacaccaccacgggtgccaccagcgtcacgatggcaccgtacaccatcagctgccggaagaacacgtcgcggtctatgcccttcgcattggccagtaccagtgcgccgttggtcgagaacggactgacatcgacgatggtggaggacacggccatcgcagcgatgaagccgatggcgctgacgcccgtgtctccctgcaggaacggcaccgccaggggaatcagcgagccgagcaccgcggtcgacgaggcgaaggccgagaccacggcgccaacgaagcacagcagcaacgcggccaccatgggcgaggtgagcccggccacgctgtgtccgacgaaatcgatcgtgcccatcttgtccatcacgcccacgtaggtgctgacgcccacgatcagcatgatctccggccacgacacctggcccagggcgcgcctttgcagattgggcgccatcagcgtcagcaccaggccgatggtgatggagacgaagccgatgtcctgcttgaagaacagcgtcagcaccgccagggccagcagcccggcgacggtggcgatctggtagcggcgcgaaccctggtcggccgggaccgccggcgctgcgtccatgagcgactcgccggccgcagtcgcgacgcggcgctcttccgcgagcgattcggcctccgcatcgccgaatacctgcgccccgccctgcgcatgtgccgtgcggggcgttgctggtactgcgccggtcacgtcggccttctggcgcagcagcttcatgccgcccatgaggaagaacagcagcagcgacacggacaggttgacgccgaggctcgcaagcatcgtcgtgatctcgctgagcggcagcccggccttggcgacgatcttgttggtgatgccgccgtagatgctgatcggcgagaagccgccgccttgcgcgccgtgcacgaccatcaaccccatcagcagcggattgatgccgtacttggcggcaaagcccagcgcgatcggcgcgatgatggccaccgccgccgggctgaccgcacccaccgccgtgagcagcgcggcgatgaagaacatgatccagggaatggcggcgatgcgcccacgcacggcgcgcaccgccagcctgacgagccaatcgatggtgccgttgttctgcgccagcgcaaacaggtaggtaatgcccaccagcgtgagaaacaggtcggccggaaagccgcccatgatcgctttcgcgttcatgccggcgaccagcgtgccgaccaggaaggcgccgacgaaggcgatcacgcccatgttgatgggcagcaccgtggccagcacgaacatgccgaccagtgcgtagatcgaaatccaatgtgaactcatcgatgcgtctccggtgttttaagtgcgacgcacatgcaccgtgcgtctgggtccgtacggtacgcaccccctccgggacgatcaatgaagcggcgtctgcgacctttacgctcagtgaaacgatcgagggttaaccctcgatcaggccgacgctggaggctcgcgctcgtgcgagatcggcacgctgaaggccgccagcgtggcaaagtcgatcagtcgacgtgtactcaaagccgtgccgtgccgccgaccgaggcacatcaacgccgtcggggttaagttagtgccattcctatctgacacctggagcaacgcatgatcgtcgaacgcatctggaccggcaacgcctatcgcaactacaactacctgatcgtttgccccgaaagtggcgaggctcttgccatcgatcccctggaccaccagaaatgcctggcggccgcaaaggacaagggctggcagatcacgcagatcctcaatactcacgagcatcacgaccacactggcggtaatgaggccgtcgtcgccgcgaccggcgccaaggtgatcgcgcaccacaagtcgggctctcgcattgccggcatggaccgcggcgtcaaggccggcgacgtgatcaaggtcggcaagaccgtcgagctcgaatgcatggacacgcccggccacacgatgtgccacatctgcctgcgctctcacaccgagaggcctgcactgttctccggcgacacgctgttcaacgccggcgcaggcaactgccacaacggcggtaatgtggaatccatgtacaccaccttcgtcgagcaactcgccaagctgcccgacgacacccgcgtctaccccggccacgactacatcgagaacaacctgcgtttcacgctcgcgcgcgagcccgacaacgctgccgccaaggcgctgctgcccggcgtggaagggcatgatccggccaaggcccgcgtcacgacgctccgcgaagagaaagagatcaataccttcctgcgcctgtcgagcccgagtgtcattgcggcgcttcgcgaggcctttcccgatctgcccgacgagccggatccgaagaccgtgttcgtcaagcttcgcgagctgcgcaatacatggtgagccgctggtcaacactacttcgcccgccgcggggccggatagcgccgcaccgatcgatcaggtgcctcgcactcagccgaggtcggcttttgccacgcggcacaccgacagcagcgcgagcaggttgggatcgcgctcgcgcgtgcgcaggaaattgagcgcgatggtctggcgcatcaggtatctggactgcaacgggatcagctgcaccttctgcggcatgacgccccgcacccgccccggcagcagcgtgtagcccacgccgccgctgaccaggttcatgagcgagaagatgtcgtcggtcttcatcaccacgttgggcgtgaagccggcgatgcggaacgtttcgacaaaccccctgtaggtgacgaagccttcgctcaggctcacgaagcgttcgccggcgcaagtgctcaggtcgatctccttctgcgccgaatagggggagcccacgggcgcggcaaactggatgtcgtcctcgaacagcggctccgattcgacatcggaaacatcctccggaatcgccatgagcgcggcgtcgatcgcgccatcgcgcagcttctgcagcaggtgcgcattggacccgagcacgagctcggtgtgcaggtccggcttgcgcagcttcattcccatgatcagctgcggcaccgtgcggctcgtcagggaatagagcgagccgatgcgaatgcggtcggccgagtagccggcgacttcccgcgtggcgcgaatgccctgcgccatggtgcgaagcacctcgcgcgccacctccgccagcgcatgagcggcttcggtcggatgcagattgcggccttcatgccggaacagcgcgcagcgcagcccggtttccagcgaatgcaaggcgcggtgcacgctgacggcgctgatgtcgagcttttccgccgcgcgggcgagattgccggtctccatgaaggccagaaggacttcgagcttgcggaaggtgatctcttcgtcgacgtggaggagcatgggcggcctgcggatgaatgcgaatcgtaagccctgccggttttgaagccgcaatcaggtgaaggccaacgacgcgcgcgtgcttgagccgatggatgaggcgagcttggcgcgtcagccaaccaaacgctgcacatcgatgctgcgaagtgtcattcaattgaattacaattcatcagttgttctctaacttggaggcgcctgccatggctgcaaacgcattggtacagacccgcatcgacgctgacgtgaaggagcgtgccaccgcagtgctcgacaacatcggcctcaccgtctcggacgtgatgaggatcgttctgacacgtgtggccaaggagggcgcattgccggcggggtttaccgttgacgctgcggcccatgacgcctggttccgagccaaggtgcaggaggccctggatgatccgcgtcccgcggtcccgcacgagaaagtcgaagcgcatttcgccaaacgccgagcagcggcgctgcgcaaggcgggtgaaggcgacgcgtgaggctggagtggtcaccgctggcaacggatgaccgagagcggattttcgatttcatcgagcaagacgacccgcgcgcggcgattgcagtggacgagcgcatcgccacgcaagtgctggtgctgttgcagtttccagagggcgggcgcccagggcgcgtcgaagggacgcgcgaactgatcgttcgccgcacgccgtacatcgtggcctaccgggttggaaaggattacgttcgcatcctgcgagttcttcacagcgcgcagttgtggcctggcgaactgacagacctgctgtgaagagggagtcttcacgttcttgtcgatgacgatctgcgacagtccatcgcgtccgtgcacgacggcaaatcggctcgaacgggcgctgaaatccggaaaacagctggctgcgaagcgctacgccagttcgcccgactgtgttcggtgcgcgtgcagcgcttcgaagatcggtccgtcgctgaagcggaaaagatcgagcgtcccctggctgcctgcgtcgcagtgggccgcaaagggctgccacgacggcacgacgaacatgtcgccgcgttggacgctccattgctgctcgcccaccttcaccgtgccgctgccctcgaacacctggtagaccgatgagccgacctcgcgctgcaccagggtgctcgcacccttcctgatgcggtgcatttcggtgcggatggtgggcagcacgtcgcggccgttgctcgggttcgtgaagcgaaccgccgcgtggcccgggctcaatgtggcgggatggccttcatcctccagcgccagctggtcggccagggcgcggtcggtatcgacccagcggtaggccaggagcggcgtcgcggccggtgcctccggttgcgacagcggacgcaggcccgggtggccccacaggcgctccgagcgcgagcgctccggcgtggccttctcggtcgtgctgacgcgctcgcgcccgaactcgaagaactgcgactccgtgtagtacgagaacggaatgtccaggccatcgatccacgccatcggcgcgctggccgcgttgtgatgggaatgccagttccatccggcctgcggcaggaagtcgccgcgcgacatccgcaccggatcgccgttcaccacggtccacacgccttcgccttcgaccacgaagcggaatgcgtgctgcgagtggcgatgctccggtgcgtcctcgcccggcatcaggtactggatggcggcccacagcgtgggcgtggcaaacggcctgccgccgagggcaggattggccagcgcgatggcgcgccgctcgccgccgcggcccacgggcacgatgcgcccggcctcgctggccagctcgaccaggcgatcccagcgccagagatgaggcactgccttgctgcgcgggtgccgcggcatgaggtcgccgatctccgtccacagcggaacgagcagttcgctttcgaagccccggtagagctgctcgagtgcggggctgggctcgggttggcccggaccggcgacggccttcaggcgcacgggggagggtacggtgtcgactgtcatgaagttccttcgtggggaccgctgcagcgagcgctcgcgtggcgcttctgtccgctgtgtcgttttgtcgggagccgggctacgtcggctcttgcttcactcggccgggccgaccgtgagcgtgatctcgcccacgccggccacgctgccctcgacgcgatcgcccggctggagcgcacctacgccttccggcgtgccggtgaagatcaggtcgccgggctgcaggtggtagaacttcgacaggtcctcgatcagttcggggatgttccagatcagcttggaaagatcggagcgctggcgctcctggccgttcacgctcagcgccagtgcgccttgctcgagcacggtgccggccatgggaacgacctcggacaccaccgacgactgctccacgtccttgccgaggtcccagggccggcccttgtcgcgggccacgagctgcaggtcgcgccgcgtcatgtccaggccgcaggcgtagccgtagatcagcttgtgcgcatcggcgcggtcgacacgaaaaccgggtgccccgacgacgagcaccagctccatttcgaagtggtagttggccgtgccggggggataggccacggtggcgccggactccaccagcgtcggcaggctcttggtgaaatagaacggcacttccaccgtcttgtcgaccggccgccccatctcgatggcgtgggcgtgatagttgcggccgacgaagaacagccggttgacgggcaggcgctccgtcttgccgcgaacgggcagcgaggcgatcggaggaggggtccagaggtaggtggtggtcatgatgtttacagtgcggggatcgggccggacgcgcgttgcgcgtccgtatgtcaaagcttggcgagcggtacctggaggtcggcgagctgcgccgcgtcgacgctggtgcggcgctcgatcaggcgccgcgcaaagcgcaggtcgcgcgcggcgttcgggcccagcgcggcgacgaccttgtcggcgtcgaggaagaacatcacgaaactgctggccctccggtcgccgcgcaacaccacgcggtgcgccggcgcaggcatgccgaagatctgcaggttgacgtcgtactggtccgaccagaaccagggcagcggctgatggttcaccatggtgccgagcgcggagcgcgcggcggcgatgccttgctcctgcgcgttctgccaggattcgagccgcatccgccgtccggcccattcgcagtgccaggccgccacgtcgcccgcggccaggatgtcggggtccgacgagcggcattgcgaatcgaccagcacgccgccatcgcacgccaggcccgcctcgcgggcgagttcgtcgttgggaacgaggccgacaccgatgaggacggcgtcgcaatcgagcgtgcttccgtcgccgaacgacgccatgaggccgccttgcgcgctctgcgccaggcgctcgatgcccgtgcccaggcggacatcgacaccgtgggaggtgtgcagctgcagcaggtagtcggaaatttcggacggaacggtgcgctcgcacagccgccccatcgcttccacgacggtcacgtccaggcccttcttccgggccgtggcagccacctcgagcccgatccagccgcccccgacgacgagcagccgcttgcccgcagacagtgcggcaccgagcgccgccgcatcctcgatgctgcgcaagctgaagacgccgggcagatccgcgcccgggatgttcagccggcgtgcccgcccgccgttgcagagaatcagcttgtcgtatgcaacgggctctccatgcgtgaggcgcaactgcttcgtcgccctgtcgatgaaggtcgcaccgacgttcggccgccagtcgatgcccagcgcatcgaaggcttccgctttcaagagatgcgtcgtgtccgcatgggcgtctccggagagcaccgccttggacagcggcggacgttcgtagggacgatggggctcgtcgccgatcaggaccacacggcccgcgaagccctcgctgcgcagcgtctgcgcggcccagccgccggcctggccggcgcccacgatgacgatggtttcggtggtcatggattcaaggccatggaagaaaggagaggcatcagtccagcgagaggaacacgcggcccgcgtcgatcttcacggggtacgagcggatcgcctcggtcacgggggcgcaggtcggcttgccgttgcgcacgtcgaacttgccctggtgcagcgggcattcgatctcgtgcccttcgaggaagccctcgcagaggcgcgcatggccgtgggtgcacacgttgtcggtcgcgtagatctggccgtccacgttgtacagcgcgatgtcgcgcccgccgaccaccatgccgaccacgtcatcggtgggcacctcgtcgacggttgcggcgtcggtccattggaaatcgctcatggctggcctcagaggggatagatgacggagttggggatcatttcgctgtcgtagatgacctggcgcgaggcgaacttcagtccttgctcggtgcgcacgacgacgtcgatgtagcggcccacgctgaagacgctcgaaagctcggacagcttggtgcggaacaccgcgtagttggcttcgcactcgaagcggtccgcctcggccttcaagacgagcggcgtcccgacgacgtggcgctggtagtaggggtcgtggaacaaggtctcgcgaatgccgtagacgcggtccttcagcatgcccttgctctcgaacgacagcgtggccagcggaaagccgcggtcgtagttctcgcgcggctgcagccggtagctgcagtcgtccgtgaagaactccggccagagttcccattcgccggagctcacggcctgggcgtagcgggcgtagagctgggtcaggtcgaagtagtcctggaagttcatctcaagcctccatgaccttgcgccagtactcgtacatgccccgtatcagggtctcggtgaccatgtggtccgtgtcgccgacctcgcggccgccgagttcggcaagcgtgcggtggaagggcttctgttcgaagcctttctgcgaaagctcgatcacttcgccgtcgtcggcggagacgaaaccggccgggccgaagagattggcctggcgcagccgtcgcagcgtcattgcgtcgtcgtcgtcctcgaagccgaagtgcgtccagacgaaatcgaaggcgccggggccgctcggctggatgtgccgggtcgagacactgttgacctgctgctggaagatcacgctcgggaacagcgtcatcatcaccgccgtggggcccttccaccacggctcgggcacgatgtccagaaagcggtcgtcgttgagcttcatgctttccttgaagctcgacacctgcgtgaccccgtcggccttgccgctggcgccgcgggtcgagatcatggccgcgtgccggtgatggctgtccatcttcagctccgacttgttgtccgcgcgccagaggccgaaggtgacgaaccacgtatgcaggaggcccgggtggtacgggtccttgatgttttcctgcatcagcttccagttgcccggaatgcgctggcggttgtagccgaggatcgtcagcttgcggccgttgaacagccggtcgaagtaacccaggatttccgggcccatgaagtcttcgagtgactccacgtccgcatcgaaggaagcgaacaccacgccgccgcgggtcgcgaccttgagtttgttgaggccgtggtcggcgggcttgaagtcggctggcatcccgccgttgaccttgccgtcctgcttgacgccgcgccggaagggcacgccttgcaggtcgccgcccagcgaatagttccactggtggtaggggcaggtgaacccgctggccttgcggttgccgtgccgctcgcggcagaactgcatgccgcggtgcgcgcacacgttctccaccacgctgatggagtcctcggcatcccgcaccatgatcaccgagcgttcgccgatcaccgtgcgcttgaaatcgccgacctccggaatctcggcctccaggcccacgtagcaccagtggccgcggtagaagaggcgctcgagctcgcgccggtgctggtcggcatcggtataggccatgaaggggatgcggctcgtgcccttgtcttcccagtggatcttctgcggaaagactgctgatgtgtcgtccatgtttgtctcctgtgcggccgtgtcgcatgggccgcttgtctcgtggtacccgatgatcggcagttcggccccatcgttcaatagaatgtgccgaatacctcatatagatttcgcgaatgggagccggcgtggagctcaaggacatcgacctcaacctgctggtggtgttcaaccagctgctcatcgatcgacgggtgtcgaaggtggcgacgaatctcggcctttcgcagccgggcgtgagcaacgcattggcgcgactgcgcaagctgaccgatgaccccctgtttcttcgaacgccgaagggcatggagccgacacccttcgccgagcagctggccgcgccgacggcgagcgcgctgcagacgatccatgcggcgatcaaccagcgcagctcgttcgatccggccacttcgacgcgcgccttcaccatcggcatgaccgacatcggagagatatattttttgcccaagctcatgaaggagctggcgcgcgtggcaccgggcctctcgctcagcaccgttcgcaacacggcggtcaatctccaggacgagatggaatcaggccatgtcacgctggccatcggcttgctgccgcagctcaagagcggctacttccagcggcgattgttcaagcagcactacgtctgcatgtttcgccgcggccacgcgctcgacaagcggcagatctcgctggccgagttctcgcaggccgaccacgtggtcgtggtttcggagggaaccggccacggcaaggcggacgagcttctcagccgcaagaagatcgttcgcaaggtcgtgctgaccgtgccgcactacgtggcggtcggccatatcctgcacgactccgacctggtggcgaccgttcccgagcggctcgcccaggccttggccgggcctttcgggctttcatatgtccgccatccggccaagctgccggagatcgcgatcagcctgttctggcatggacggtatcaccgcgatcccgccgtggcctggatgcgtgccttgatcgtgcggcttcacggggaaggcgccgctgcctgaccgtctccggcagcggcagcggaagcggaagcggaagcggaagcgccggccattgcagctgcgagcctgccgcgacggcgagccccggcgccgcacatgcatcgggcgcccccccgatcgcctcgcaccgctcactcggctgtggccgggtcgatcacgctgtacacccggtctacccggtcggccgggaagccgccgagttccgcgtgccggcgcaccagggcttcgtcggtggattggtagacgcaatagatccggtcatcggtcacgtagctgtggatccactggatgtcggggcccatgctgctcaacacgccgcaggacttttgcgagatggccttcaggtccgacggggtgaattggccggcgccggggatgtgccgttcgataaggaatttgggcatggcgatactcctatctagaatcatcggtcaaaggcgaccaagacccatggtgccgacgcgaagcgcccttgtattgctcgccactccggacttgttgactgaaaccccgccctcgccagcctgagaggtgaccatggatgtcttgtcggacgtgctgcggaccatccgcctggagggcgcgctgttcctgaacggagacatgcatgcgccctggtgcttcaaggtgcccaggggcacggacatggcgcagctcctcaagcccggtgcgcagcggctggccatctgccacctggtgctgcaaggcgaatgctgggcccaggtcgaaggcggggagccgatccgcgcatatgccggcgaagtgattgccgtgccgcatggcgactcgcatgtgctgggcagcggcctgcaccatgcggcggtggacgtggcgcatgtggtcagtccgcgcgcacccgagctggagcgcatccgctacggcggcgacggtgaccgcaccgtgctggtgtgcagctggttcgcttacgaaggcgatgcgcccaatcccgtcatggcgaacattccgcgcctgttcaccacctcgttgcgcagccggccggcgggcccgtggatcgagcaatccgtcaatttcgtgttggccgatgccgcttcgcacacgcccggttccgagatggtcgccgccaaggtggcggaggtgctgtttgccgaagtgctgcgcggctacatcgaatccatgcccgccaacaaccctggctggttggccggcctgcgcgacccccacgtgagccgctgcctggcgctgatgcatggcgagcccgcgcgcaactggacggtcgacgcgctggcgcaggaaacccacatctcgcgcagcgtgctggcggaccgcttcgccgaactggtgggcgtgccgcccatgcagtacctgacgcgctggcgcatgatcctggccgccggcttgctgcgcaaggaccggggcaacctggcgcgcattgccgaaggtgtcggctatgaatcggaagccgctttcaatcgcgcattcaagcgcgagtacggggtgtcgccgggggtttggcggcaaaacggggttgagctcccggccggttccgagcgcaccgcatgatggtacgaacgtctatggcagagggagctcgcgcatgaggttgctgcgcacccacgtgaacgcgccggactggacgttgttcgcttgccagcggcggaactcgggatcggctgacagcggatccgtcaccttcgcgtattccgtcgcgttctcgaactgcacggtcagaacatagttgcccagttcgcctgcgaccacgctccaaagctgagggctgggtgcgccatgcttcttccagagcgccgcacccgccttcacggcttccatgacggcctcgagatcggctccggggctgggtcgcaggacatatcgcgcttcgtaggccatagaagtctccttcgtcatagcaagagcgacattgaagcaccggcgcgcttggggggcaatcgacaattgcggcgctaaagtgcggctgatcgcccgcttccgacgccgctgaatcgataggacttcaatgctcgaactcttgacggaccctcaggtttggattgcctttgccaccttgacggcactcgagctcgtccttggtatcgacaacatcatcttcatcgcgatcctcgtcgacaaattgcctcccgccaatcgggagttcgcgcggcgcgccgggctgttcatggccatgttcatgcggatcggcctgttgctggttctggcctggatcgtcggcctggtcgctccgcttttcacggtgttcgatcaggaaatatcggggcgagacctggtcctgatcctgggtggcctgttcctcatctggaagagcacgaccgaggttcaccagtcgctggagggggagcacgagcacaaatccagtgcagccaaagcgaccttcgcttccgtgatgcttcagatcgtcctggtcgatatggtgttctcgctggactcgatcatcaccgcggtcgggatggtggacgacgtgcgcattatgatcgccgcggtgattgcgtccgtgctgctgatgatgctgttcgccggcccgatcgggcgcttcgtctcgaaccaccccaccatcaagatgctggcgctggccttcctggtggtcgtgggtgtcgtcctcgtggcggagggcttcggccaccatgtgcccaagggctacgtgtactttgcgatggccttttccgtggccgtggagatgctcaatatccggatgcgcaagaaggcggccaaagccgtgaaactgcacccgccccgcatgccgggcgattgaagaagaactgaagccgccaatcagtcagccgcaggcggcgcagattcctccgtccaccgcgcatgcgacgcgctcaggtgatgcagcatggcggccaccgcggcctgcggatcccgcgcttccagcgcgcggtagatcgcctcgtgctcggcgaacgccgccttccacgcctgcgaattctcggtgcgctcgctcatgcgggacgagatcgggctgtgccgcccgtcgaagagttctccgaccagccgcacgagaaccgagttgcccgtcatctcggcaatggtgatgtggaagcggcggtcgttctcgatctgcgtgcggccattgaggccgtcctggcgcatgctttcgagcgatgccctgacgcgctccagaagctgcggcgtgacgcgggccgaggccagcgtgaccaccgagccttcgagcatcgcgcgcgcctgaatcatttccgacgggctttcgccgaccgcgggcgttgcgcgctccggcgcgtcctgcgacgcgcagacatacacgcccgaccccatccgtatctcgacgcgtccgtcgatctccaaggcgatcagcgcttcgcgcagcgaaggccgcgacacacccaactgcaaggccaactcccgctccggtggcaagcgcgcgccgacgggcagattgccgttgcggatgaaagcccgaatctggtccgcgatctgttggtagagccggcgggtgtcggcgggtttggtgggggggaacatgagaagggggtcggcaatctggtcatgccagtttgccatcctctatgtagtgattgctactaatgagcggtactttacgggaaaacccgacaagggtttgttccgttaaggccatttttgacgttatggcaaagtggcctgccaaattggtaaggccaaaacagatggcggcgttccgttttgacgagactggagggtgccagacagcatgagccaacgcatcgactcgcatcagcatttctggcggcccgcgcacggcgactacgcatggctgcgcgccgatgtgcccgccctcgcgccgctggtgcgcgactttcttcccgcgcacctcgcgcccctcctgcaagcgcatggggtggagcggaccgtgctggtgcaggccgccgactcggaagccgaaaccggcttcatgctcgaactggccaccgcgcacgacgtggttggcggcgtggtcggctgggtcgacctggccagccccgatgccgtggtttcgctcgagcgcatggcgcggcatcccaagttcaagggcgtgcggccgatgctgcaagacctgcccgatgacgactggatcgcacgcatgccacggcccgatgccattcaggcgctcgttcgcctgggcctgcgcttcgatgcgctggtgaagccgcggcacctgccctcgctgatgcggttcctcaaagactggccgcaactgcccgtggtgatcgaccacgccgccaagccgcccgtgggcgcgcacggcagcgaggccttcgcggcctggcgcaaggacatggccgagctcgccgcgctgccgcaggtgtgctgcaagttctccgggctctggggcgaggcgccgcaggctgcgcaccacgacgtcgacgtggcggcacgcgccgtgcgcccggtgtgggagcagttgctcgagagcttcggccccgcgcgcctcatgtggggcagcgactggccggtgctcacgctggccggcgactacgcaggatggatcgcggtcagcgaagcctgcatcggcgggctgtcggccagcgagcagtcgcacctctggcgcggcaccgcacaacgcttctatggccttccgacggactgaatgcgccatgcaacccatcgtcaccatccgcgacctgtgcaaatcctttgccggcgtgcgcgcgctcgacaaggcgcagttcgacctgctgcccggcgaggtgcatgccctgatgggcgagaacggcgcgggcaagtccacgctcatgaaagtgctggccggtgtctacagcaaggactccggcgaggtgatgatcgacggcgagcccgtggacatcgcgagcccgcgcgcggcgcaggcgctgggcatcgggatcatccatcaggagctgaacctgatgaaccacctgagcgccgcgcagaacatcttcatcggccgcgagccgcgcgggcgcctcggcttgttcatcgacgaagacgggatgcgcgccgaggccgagcgcatcttcgcgcgcatgaacctgcggctcgacccgcgcacgccggtcggcgagctcacggtggccaagcagcagatggtcgagatcgcgaaagcgctctcgttcgattcgcgcgtgctcatcatggacgagcccaccgccgcgctcaacaacgaggaagtggtcgacctgttccgcatcatcggccagctcaaggcgcagggcgtggccatcgtctacatctcgcacaagatggacgaactcaagcgcatcgctgaccgcgtgaccgtgatgcgcgacggccagtacatcgccaccgtgtcgatggcgggcacgccgatggacaccctgatcgccatgatggtgggccgccagctcaccgaggtggagaacgactttcccgacacctcgggcaacgagatcgtgctcgaggcccggggcatccgtcgcggctcgatggtgcgcgatgcgagcttcgtcttgcgcaagggcgagatcctgggctttgcgggcctcatgggcgcgggccgcaccgagctggcacgcgcagtgttcggggctgaccccatcgacgcgggcgaggttcgggtgcgcggccagcgggtgtcgatcaagtcgcccgaggatgcggtgtcgcatggcatcggctacctctccgaagaccgcaagcacttcggcctagccaccggcatggatgtggaaaccaacatcgcgctgccgagcatgaaaaaattcctgtcgatgggcgtcttcatcgaccaggccgccatcgaggccgcaggcgagcgctatgtgaagcagctcagcatcaagacgccctcggtgcgccagcaggtgcggctgctgtcgggcggcaaccagcagaagatcgtgatcgccaagtggctgctgcgcgactgcagcgtgctctttttcgatgagcccacgcgcggcatcgacgtgggcgcgaaggccgagatctaccgcctgctcaacgaactggccgccgagggcaaggccatcgtgatcatctcgtcggagctgcccgagatattgcgcgtgagccaccgcgtgctggtgatgtgcgaaggccgtatcaccggcgaactggcggggcgcgaagcctcgcaggaaaagatcatgcagctcgccacccggcgtgaaaccaccgttgctgctgccgccaccgcatgacgactggagacaaagccttgacaacccccaccgccaccaccgccaccgcgcccggcttctcgctgaaggcacggctctttcgtcccgccacgcggcagaagctcctggcctttgccagcctgatcgcgctgatggtgttcttcagcgtcgcgtcgccgcagttcctgcagaccgacaacctcgtgagcatcctgcagtcgaccgcggtgaacggcgtgctggccattgcctgcaccttcgtgatcatcaccgcgggcatcgatctttcggtgggcacgctgatgactttctgcgccgtcatggccggggtggtgctcacctacatgggcatgccgctcgcgctcggcatcgcggccgcgatcttcttcggtgcgctggcggggttcgtgtcgggcgtgctgatcgccaagctcaagataccgcccttcatcgccacgctgggcatgatgatgctgctcaagggcctgtcgctcgtgatctctggcaccaagccgatctacttcaacgacacgccggactttccggcgatctcgcaggattcgctgatcggctacttcattccgtcgctgccgattccgaatgcggtgctgatcctgttcctggtggcggtggccgcgagcatcttgctcaacaagaccatcctcgggcgctacaccttcgcgctcggcagcaacgaggaggcggtgcgcctgtcgggcgtgaacaccgacttctggaaggtcgtggtctacacggtgagcggcggcatctgcggcattgcgggcctcttgattgcctcgcgcctgaactccgcgcagcctgcgctgggtcaagggtacgagctcgatgcgattgccgcggtggtcatcggcggcacctcgctcagtggcggcaccggcaccatcgtgggcacgatcatcggcgccttcatcatgagcgtgctgaccaacggcctgcgcattctttcagtcgcgcaggaatggcagacggtggtgacgggcgtgatcatcattcttgccgtgtatgcggacatcctgcgccgtcgcagcagcagcgcgcactgaccctgtttctacaaccgaaggagacattcgcatgattcaaagaagagcagtcgcaaccacgctggccgcgtccctcatcggcctgtcgggttttgcccaggcacagcaggcgcaagagatctacatcccgctcgtgtccaagggcttccagcaccagttctggcaggccgtgaagtccggcgccgaacaggccgcgaaggacctgaaggtgagggtgaccttcgaaggccccgagaccgaggcgatggtcgacaagcagatcgacatgctctccgccgcgctcgcaaagaagccgcaggccatcggctttgccgccctcgacagccaggccgccattccgctcttgaagaaggcgcaggccgcgaagattcccgtggtggcgttcgactcgggcgtggacagcgacattcccatgaccaccaccaccaccgacaacaaggccgccgcggcgctggcggccgacaagatggccgagctgatcggcaagtcgggcgaagtggcgctggtggtgcacgaccagaccagccgcaccggcgtggaccgccgcgatgggttcgtcaaccgcatcaagtcgacctacccgaacatcaagatcgtgagcgtgcagtacggcggcggcgaccagctgaagtccaccgaaatcaccaagtcgatcttgcaggcctcgccgaacctgaagggcatcttcggcgccaacgagggctccgccatcggcgtggtcaacggcgtgaaggagatgaagcggagtggcaaggtcgtgatcatcggctacgactccggcaagcagcagaagaacgccatcatcgacggcagcatggccggcgccatcacgcagaaccccgtgggcatgggctacaagaccgtggagatggcggtgaaggcggtcaagggcgagaagctgcccaaggtggtcgacaccgggttcttctggtacgacaagaccaacatcacagacccgaagatcgccgcagtgctgtacgactgattctttcccggaagactcgttcatgaccatcgttcgatccatgcacgtactggacgtgcgctttcccacttcgcagcagctcgacggttccgacgcgatgaaccccgacccggactactccgcggcgtacgtcgtgctggaaaccgatcagccggggctcgaaggccatggcctgaccttcaccatcggccgcggcaacgagatctgctgcgcggccatcgaggcgatgcgtcacctggtcgtcgggctcgatctgcagtgggtggccgaggacatgggccgcttctggcggcacatcacgtccgacagccagctgcgctggatcggccccgacaagggcgccattcacctcgccaccggcgcggtggtcaatgcgatgtgggacctgtgggccaagtccgaaggcaagccggtgtggcagctggtggcggacatgagccccgagacgctggtgcgctgcatcgactttcgctacatcaccgactgcatcacgcccgaagaagcgctcgcgctgctccgcgatgcggccgttggcaaggccgagcgcgttgccacgttgcaggccgagggctacccctgctacaccacgtcggccggctggctcggctactccgacgagaagctgcgccggctcgcgcaagaggccgtggatgcgggcttcaatcacatcaagctcaaggtggggcgcgacctgcaggacgacatccgccggctgaccgtggcgcgcgaggtgctcgggcccgatcgccacctgatgatcgacgccaaccaggtctgggaggtcgaccaggccatcgactgggtgcggcagctggcattcgccaagccttggttcatcgaggagccgacgagccccgatgacgtcgaaggccatcgcaagatccgcgagggcatcgcgccggtggtgaaggtggccacgggcgagatgtgccagaaccgcatcatgttcaagcagttcatcatgcgcggcgcgatcgacgtggtgcagatcgatgcgtgccggctcggcggcgtgaacgagatcctggcggtgatgctgatggctgcgaagtacaagctgcccgtgtgtccgcatgccggtggcgtggggctgtgcgagtacgtgcagcatctgtcgatgatcgactacctctgcatctcggggacgcgagaagggcgggtgatcgagtatgtggaccatctgcatgaacacttcgccgagccttgcgtgattcgcggcgcggcgtacatgccgccgacggccgccggcttctcgatcacgatgaagcccgaatcgctcgagcgttatcgcttccgtggatagtcgaaaaatagaaaggcatcgcgcagtcatggacctgaacctcaaagacaaggtggtgctcgtcaccggcggcggcagcggcatcggcgcggccatttcgctcacgctcgcgcgcgaaggggcggtgccggtgatctgcgggaagaatccgctggatgcggcattcgaggaagagctgcgcgggctgcagccgcgggcgcggtttctccagttcgagttgatggaagaggcggcttgcggcaaggccgtcgaaagcaccgtcgcggagttcggccgcatcgatgggctggtcaacaacgccggcgtgaatgacagcgtggggctcgaagcggggcgcgaggcattcgtcgcatcgctggaccggaatctcattcactactacgtgatggcgcatttctgcctgccgcacttgaaggccagccgcggggccatcgtgaacatttcgtcgaagacggcgctgacggggcagggcaacaccagcggctattgcgcggccaaaggcgcgcagttgtcgttgacgcgcgagtgggctgccgcgctcgcaccggacggcgtgcgcgtcaacgccgtgataccggccgaggtgatgacgccgctgtaccagcggtggatatcggccttcgacgaacccgaccgcaagcttgctgccatcaccgacaagattcccctcggccgccgcatgaccgcgccgcaggagattgcgagcaccgcggtgttcctgctctccgatcaggcctcgcacacgacggggcagtgggtgttcgtggacggcgggtatacgcacctcgatcgggcgttgacctgatcacctttcactcttcctttctttcatcgacgatcggaacgaaccactcatgcgccactgccttgcccttgacctgaaagacgatgcggcgctgatcgccgagtacgaggcctaccaccgcaacatctggcccgaggtgcgcgcgcatctgcatgcgcatggcgtgacgggaatggagatctatcgactcgggacgcggatggtgatgctgatggagacggacgacgcgcgctatgacgccgaggccatggcagctgcgacgcggaacgatccgaagatccgggcgtgggaagaactgatgtggaagttccaggcgcctacgccttggacgcctgcaggagaaaagtgggtgggcatgcagcggatattcgagttgtagctgcttctcgaacgcagtcgcactgccaaccgcagcctgcaaccggttgctccggcatctcttttttgtcgacctcgacctgagcgcgaaccaaaactgtcgcatgtggagtccgaagcgacgctccatgtcacttttcggggtcaacgcgcgtgttcttcccccgcggggaagtgggcatggatcgtgcgcccgtgtgccacggccggtgacgccgttggacatgaatgcccacggcaagtccccggcaaagcggcccaggcggcagctgattctctttgccaggacattcaccccgacatcgtggacacctacctcgtgggcgtgggcgcgggcgcctggcccacctggaacagccccgaaggggcgtacatcacctacaccgcgcaggccatccaggcttacggcgcgaccccgatgttcacgctctaccagatggcaacgagcggcgagggcaacttgagcgtcctcaacgacgcgagcttcatgaacagctactgggcgcaggtccggctgatgtaccagcgcgttgcggccctcggcacgcccgtcctgatcaatctggagccggatttctggggattcgttgcgtcgcaagcacccaatcgcgacgcgacgcagctgacggccctcgtgaacagccagtccgaatgcagcggcctgccgaacaccgccgcaggcctgggccaatgcctggtgcaaatgggccggcagatcgcgcccaaggcgctgctggggttcccgcccgcgttctggagcggcactcctgcggcaatcggcgcccagatgcgcgcggtcggggcgcatcaggcggacttcatcgtcgcccagacgaccgaccgcgacgcgggctgcagggaggtcccgtcgccgcccgcggaatgcacgggccgaagcggtccgttctactgggacgcaagcaacatcgccagcccgaacttccacgagtcgcagcgccagatttcggactatcgggctgccctgggcaatgggctgccgatcctgtggtggcaaacgccgatgggcgtgccatccgacacgcccggtggcaccgacctgcactatcgcgacaaccacgtcgactacatgctgcgcaacgcccaggagtacggcgacacccacacctttgcgatggtcttcagccctggcgggagcgttcagacctcgatcagcaccgacggcggtcaatttgcccgcctgtcggctcagtacctcgcacgaggcggcgccaccttgaagtagcggcggcaaccgggaaggccgagaggctgatttgtccgtcagggtttgtcctgacggtgcaacggcgcaaatgtccttcgcgcaacaaacgcgacgagcctatgttcataggcttcgcaagcctgagggaaacatgcaatgagagctcgatctggtttggtcttcgcccgtgtcgttgggtgaccgatgctgcctgccaaggatctgagcgctttctttgagcgatgcatctggccgcgcgccttgacgcaggcagaacgaaccaaagcgttcgaggccctgtacgttcggcatcatgaagcgcactcctatgtgtgccaacgcgacgagatcgccgacagctggattggggtgctggagggcttcctccgggttcaggacaccacggtggacggtcgcctgatcatgttcaccggggttgcagccagcggttggatcggcgaagggtcgctcctgaagccagagcagcgcaagtacgagatcatggccacgcgaccgaccatcacggtccatctgccaaggaccacgttctcatggttgctcgatcgaagcatcccgttcaaccatttcatgctttcgcatctgaacgagcggcttggacaattcatcgcgatggtgaagttcgatcgactgctcgaaccgacggcgcgcgtggcgcgtggcatctccagcctgtttcatccggtgctctatccgaacaccgactcgacgctgcgaatcaaccaggaggaaatcggcttgctcgtcggcatctcgcgccagcgcgtcaacgtcgcattgaccgaactggaaaccgcgggcctcatccaacggggctacggctacatcaccgtgatggacaggcaagcacttgccaggtactcctagcgaggctgccgcacatcgaaaccggagggtttttccttagaaatcagtggccagaatgtcggtctcggaacagttggccaagggctcgcctttcagaatctcctgggcatcgcgccatctcgttgcggtgcgcaggctgacaactgataaaggaatagagacatgcacttcttctccccaaaggcacccttggctcgcgcgaagcttcacgctgctgccgtcagcgtggcgatgctggcagcttgcggcggcggctccgataacggcggcgcgttccccctgctgctccctggcccgccaacagcacaacccgaaagtcctccatccgcaccggttgtgacggctcagaaggcctgcaccgacctgaccggaaaaaccgttgcaggcgccgccctgacggccgtgatggtgactgcgacggcggacgttcccgtgtactgcaaggtcaccggcaccatatcacccgcgttgaacttccagatctctctgccggaggcatggaacggcaagctctactaccagggaggaggcggctataacggcgccatttcgccgccttcggtgccggccctgggcctgggctacgccgtcatcgccagtgactccggacatcaggacaatgccttgagcgcggacttcgcgctgaccgatacctttgcggcccagctgttcggcagcctctcggtacccacggtgatgtcgacggcgaacgagaccctggcggctgcctatgggtctctgccggcaaagtcgtacttcgagggttgctccaacggcggacgcgaagcattgatggcggtgcagcgctcgccgaatctcttcgatggcgtcatcgcacgtgcccctgcgtacaactgggtcgggttcatgggcgctttcaatcgaaattccagggcgcttgccgcgcctggcggtgcattcaccgctgcgaagacggcgctcctgagcaagcatgtgcgagacgcctgcgatgggctcgacggagtcgccgatggcgtggtgtcgaaccgggccgcatgcacgccggcgctcgtcaacgtggccgccctgcgctgtgccggcggaaccgactccggcgacagctgcctgtctgatgcacagctcgacgtggtggcgtcctggaccacggaagcaagcttcacgggtagcgccagcttccggaacgccggttggaacctgacaggaaacgaggacgatccgggcgcctggagaacctgggtcacgggcgacggcaatgtaaccatggcgctgcagtttctgttccaggatacgacggtcaagaactatctggcccgcgacagaacggtgagttcgctcgcctacacaccttgggatcagaaccagaatgcgctctatgccatggccgcgctcaatgatgcgaccaacacggacatccggcccttcatcaacagcggcggcaagctgatcttgtggcatggcgggaatgattcggcgctcagcgcgaaatcgaccgcggagtactacgggaatatgcgaagctcggtgggcgccgcggcggccgacgcgtcgacgcgtttctatgtggcgccgggggtcaaccactgcagcggaggaccgggtgccgatacctccgatctgctgacagccctcgaccaatgggtgacgaaaagcgaagcgccctccacgttggtcgcggagaagcgcgatgcacagggagcggtcgtcctgagccggcctctgtgccagtacccgcaatatccaagatacacaggtcccgccaatgatgccgtcgcttcgaagtcagctgccaactacacctgcagctcctgagtgattgggccgcagttctttgcgcagaatctttcccactgctgatttgggcaatgattcgagaaacgtgatgtggcggggcaccttgtacgccgcaaggagcttgcggcaatgcgcttccaactcctccgcctgcaagcccggtgcgcgccgaacgacgaagaggtggggcgcctctgccgagcgctcgtccggcaccccgacgcacgcacattcgagtacgtccgggtgcatggcgaccacgccttcgatctcgttcggatagacgttgaagccggagaccaggatcatgtccttcttgcggtcgacgacgtacatcaggccttgcgcatccatggtgacgatatcgccggtgcggaaccagccgtcctgcgtgaaggacctgcgcgtttcgtcctcacgattccagtagcccgcgaaaacctgcgggcccttgatgagcaactcgccgggcgtgcccagcggcacgggctcgcccgcatcgtcgacgatcagaacatcggtggagggcacgggcgcaccgatcgtgccgttgcagccgggcgcattgaaggtagcgctgggtgatgtttcggtgagcccgtaggcctcggtgatgggcggaccaccggctttcacccacttcgcggcaactgcttcctggattgaagcgccggcgccgatgacaacgttgcagcgggagaagtcgatgcccgcgatctcaggcaaggtcaccatggcattgaacatcgtgttgacgccgatcagcatgtcgaaaggcgcccgcttgagttcggcgcaaagcgcctgggcatcgcgcgggttgacgaccagtcggttgtgggcgccgctggcaagggcggtcaacgtcgtcccgagcggaaagatgtggtacagcggcagcggcgtcacgatctcgaagttgtcgatgtcgagcgccagtgccaaccatgaccgcatctgcagcgaactggcaaggacgctgcggtgcgtcaggcacgcgcccttcgaaacgcccgtcgtgccgccggtgtattgcaggaacgcaagatcagatggaccgacctgctcgctggtgaagtcggcgtctgccagcaccgacatcgcgtcgcgcagactcacgatgcgggcgccgtcgttcgcggccgcagcatcgggttggccggccgtcgcgaacaatgactgcttcacctcccgcatcggtacggtcatgacataccggagctgtgtctggtcgagaatttcgttcacaaggcccatgaagggctcggccgctaccagcgcggtagccccggaatcggccaactggtacgccagctcgcgcgccgtgtagaggggattcatggtcacacccaccatgcccgcacgcaggatggcagccaatgccaccgggtagacgaggttgttgtgcagcaggagggccaccctgtcgccacgcttcagaccggccgcttgcagggaccgcgccagcagtgccgacgcatggtcgacctgggcgaaggtcagggattcgccagcgcaggtcacggccgtcctggcggcgtacctcgtgaaagcgcgttccagcagggtgacgagggtttcactttcgtcgaggatgatgtcgtgcggaagccctgccggataggaggcatgccagagtcggtgttccatgtggtttccttcgtgcggtgaacggggttcaggactgcagcgcttcgcgaacgaagtccatccggtcctggccgaagaacatctggtcgccgacgaaaagcgtgggtgcgccgaacacgccgcgctcgaccgcctcttgcgtcgcggccttcagcgcggccttggtctcgacgtcctgcgtcaggcgctcgatctcggcgggatcgaatccaccttcggtcaggatgtgcgccgtgagttgcgcatcgttcaggttgagcgcgtcgatccagagcgccttgaacacgcagcccagcagctgctgcagctgctcggggcggcgcagctgaattccggtgaccgcgcgcatgaggaacagcgtgatgacgggaaagtgcggattgccctggaagggcacgccataccggcgcgcgtggcgctcgtagtccatttgcgtatagcgtcccttgacgggaatcgtggcaggcgaggcgttgcccgtggcctggtagacgccgcccagcagcattggccggtagacgagttcggcgccatggctggcgcacaagcccggcagctgcgtccacgcgaggtacgacgacggactgccgacatcgaagaaaaaatcaaccgacttgcgcattcatggctcctttaagttaacggacgtttggtaaacggaagctatgtgattaatgcaaccccgtcaacggggtttcactgggttcttcttcgattgacaaacgaacgttcaccaattaacgtccaatgacttaacgaacgttttttaaaggagaacgcatggacccatcaaccaatccccgcggtgtggctctcgtcgtcggcgccggcgacgccactggcagcgccattggcgcgcgtttcgcccgcgagggctacgtcgcgtgcctgacacggcgatcggcagacaagctggagccagccgtcgaacgcatccgcgcggcaggcggccaggccttcggctatggcagcgatgcacgcaaggaggacgacgtcgtcgccctcatcgaccagatcgagaaggagcgcggccccatcgaggtgatggtgttcaacatcggcgccaatgtgcccagcagcattctggaggagacggggcgcaagtacatgaagatctgggaaatggcggccttcagtgccttcctgaatgcgcgcgaggtcgcgcgaaggatggtcgcgcgggggcgtggcacgattctcttcaccggcgcgacggccggcatccgcggctcggcgaatttcgcggcctttgccggagccaagcattcgctgcgcgcactggcccagagcatggcgcgcgagctcggcccgcgaggcattcacgtggcccacatcgtggtcgacggcgcgatcgacaccgagttcatccgcagcaacttcccggaacgctatgcgctcaaggcgcaggacggcatcctgaaccccgagcacatcgcggagaactactggtacctgcatacccagcctcgagacgcctggacgttcgagatggacctgcgcccttacatggaaacctggtgaaagacgacacatgaaaacacgcatcacggaactcttcggcattcgccacccgatcatccagggtggcatgcactacgtcggctttgcagagctggccgcggccgtctccaatgccggcgggctcgggctcatcacgggcctgacccaaaggacgcccgagctgctggccaaggaaatcgcgcgctgccgcgacatgacggacgagccctttggcgtgaacctcacgttccttccaaccttgtcttcgccaccataccccgagtacatcgcggcgattgccgagggcggcgttcgcatcgtcgagacggccgggcgcagtcccgaggcctacatgcccgcgctcaagaaggccggcatcaaggtgatccacaagtgcacctcggtacgccatgcgctgaaggccgaggccatcggctgcgacgccgtgagcgtggacggcttcgagtgtggcgggcacccgggcgaggacgacatgcccaacatgatcctgctgccccgggctgccgaggaactgaagatcccattcgtggcctccggcggcatggccgatgcgcgcagcctggtggcggcccttgcgcttggcgcggagggcatgaacatgggcacgcgcttcgtggccacgcaggaagcaccgattcaccagaacgtcaaggacgccatcgtggcggccaccgagctcgacacgcggctcgtgatgcgtggcttgcgcaacacggagcgtgtgctgaccaattcatccgtcgagcaattgatcaggatcgagaaggaaaaaggagccgatctcaagttcgacgacatcatcgaccaggtcgccggcgtctacccgcgcgtgatgctgcaaggcgagatggatgcgggcgcctggagctgcggcatggtggtcggcctgatcaacgacattccgacggtgcaagatctgatcgatcgcatcatggaggaggccgagcagctgatcacacggcggctctcagggttcctcgagcccgctctggcttagcctttgggcatccgccggctcactccgcagagtgagccggcttctcgaagaggcgaaccgctgctagacgcgttcgaggcacagggcaatgccctgacccccgccaatgcacagcgacaccacggccttgcggccgccggttcgctggagcgcatgggccaccttcgtgatcaggatcgcacccgttgcgccgatggggtggccgtgcgcgatcgcaccgccgtcgatgttgtagcgtgatggctcgatcttcagctcgtcgcgcacgacgatcgcgatggccgcgaaggcttcgttgacctcgaagcggtcgacgtcctgcacgttccattcggcacggccgagtgcctggcgaatggcgggcagcggccccaatccgaagaagcccggctcgaccccggccacggcgacactgcgaatggcgagcatcggcgtgaggccggcttcgcgcgcgaccgaagcctcgcaaacgaccatcgcggcggccccgccgttgatccccggggcgttgccggcggtgatggtgccgtcgggacggaacgcgggcttcaggcgtgccagcgtctcggccgtggtgtcaggacggtttccttcgtccgcggcgaagaccgtggatgccttgccgcccttgatcgtcagcggctcgatctcgtcattgaaccacccagcctcttgcgcggcggcgaatcgctgctggctctgggccgcgaacgcatcctgcgcttcgcgcgtcacgccgtatttctgcaccaggtcttcggtgtgccagccagaatgtttgcctgagaaggcgtcgttcaatccatcgagcagcagagagtccatggcctcggcatttcccatgcgggcgccgaagcgcatgcccggcaacaggtacggcgcccggtccatgttctccacgccaccggcgatcaccatgctcgacaccccggcgagcacttccgcataagcggtcgcgacgccctgcgcgccggatccgcagacgcggttcacggtcatggcgggcgcacccactggcaggccggcgtggaccgcggcctgccttgccacgttcattccgttgcccgcctgcacgacgttgcccatcaccacggaatcgacgcgcgccgggtccaagccggagcggcgcaacacggcggcgatggcgtgcgcgccaagcgatgcggtagaagtggtcttgagcgatccgccgaagccggcgatcgcgcttcgcgcaggggaacagatgacgatctctttgctcatggtggactctccttggttagataacggtcgcgcagcaacttcttgtagagcttgccggtcgcgtggcgaggaaaatcggactcgaaatcgatgctcctgggcaccttgatcggcccgagcaattcgaggcagcgggccttcagcgcatcggcgatccccgtgcccgtgaaatccgaatgcgccggctggatgacggctttgacttcttcgccgtattcctcgttcggcaccccgaagaccgcggcatccgcaacgcgagggtcctgcagcagcacgtcttcgatctcttgcgggtagatgttcacgccgcccgagatgatgacgaagtccttgcggtccgtcaggtagaggtagccttcatcatcgagatggccgatgtcgccgaacgagcgccagccctgcggactcgtcgccgcgcgggtcttggcgggatcgttccagtattcgaattgggcatcgctttcgaagtagacctgcccggtttcgcccgtgagtagttcatggccggcgtcatccaaaatgtgcaggatgccgtcggtcgcgcggccgaccgagcccctgtgctggagccattcgcgcgaggtgatggccgtggagccgatgccctcggtgcccgagtagtactcctgaagaatcggaccccaccagttgatcatcgcctgcttgacgtgcaccgggcagggcgccgcgccatggaccgcctgcaccatgaaagccatgctgtagcggctgcgtacgcccgcttccaggcgcagcaggcggtggaacatggtcggcacccagagcgaatgtgtacatgcgaaatgcgcgatggcggcgagcgcgcgctcggcgtcgaatttcgccatcacgatgctggtggcgccggcatgaatggccgccgagaggaaccggttgggcgcgctgtgatagagcggcgatgtggagaggtagaccgacgaggcgtcgagtgcgaacgaccgggccaccgcggcgttgcggttgtcgaccgcatcgaagtcgccttcgaagggcggcttgcgcacacccttgggccggccggtcgtgcccgatgaatacagcatctcgcgtccgggcgcgagcacgggcggcagcttgcccggcgcagccagaaagcgcgcatcccaggattcgatggccgaatccgcaaagccgatcccgacgcgccgtgcgccacccaggtccaacgacgaagccgtttcggcgctcatgcaggccgacgacacgaccgcgaccgacgcccccgagtccttcacgatgtactcgaaatccgcagccgacagccgcgtcgaggcgagcacgtaatacagcccgatacgctgcgcgccgagtgcaagaaagagcaaagcgggcgcgttctcgatgcacagcacgatgcagtcgccccgcttcaggccgagcgacagcaaggcgttggccgcccggttcgcctcgcgttccagctgcgagaagctgaacgcctcgcccgattcgagaaagtgcaccgccaccttgtcgggcgtggcaactgcgaagcggctcaggtggtacatgccgcgcggttagaaaagatcgatggccggttccatcaatgcggacgatcccgcccggatctcaccgcacagcgccgcggtctgcggcagcagccgctggaagtagaagcgggccgtggcgatcttcgatgcatagatcgggtcggtggagccggcgttcttgaacgcgacttcggccatgcgggcccaactccacgcgagggccaggtgcccgaccaggcgcagatagggcgcagccgcggcgcctgcggcgtgcgggtcctgggccgacgtcgccaccagctcgccggtgagctgtctgatgtcggcgaccagcccggcgagcggctccgcgaactcgcgcatcgactcgcgcgggctgcaggtctcggcgaatgcgcaggccatgtccaggaaggcgcccatctgccgcccctggtcggccagtaccttgcgcgcgagcaagtccatggcctgcacgccgttcgtgccttcgtagaggcccacgatgcgcacgtcgcgcagatgctgctcgacgccgttctcgcggatgtagccgtgcccgccgaacacctgcatggcgagcagcgtgcactccaccgcgaggtcgctggacagcgccttgacgagcggggtcaaaaggcctagcagttcggccgtctcgttgcgtttggcggggtcgggatgaaggcgctgaagatcgctcagctgtgcggtccacagcgccagggcacgtgcgccctcgatattcgccttctgcgtgagcagcatgcggcgcacgtcggcatgcccgatgatcgggtcggccacctcactggaagatctcgcaccgctggcacggccctgcaggcgctccttcgcataggccagagccttctggtaggcagcttccatcagcccgatggcgatcatgccgaccagcacgcgcatgtggttcatctgcacgaacatgcccgccagacccttgttgggcgcacccagcagccagccggtcgcgccgtcgaagttgatggtgcaggtcgagttgccgtggatgcccagcttgtgctcgatggagccgcagaccaccgcattgcgcgcgccagccgcgccgctcgcatcggggatgaacttcggaacgatgaaaagagaaatgcccttcacgccgggcggtgcgtccggcatgcgcgccagcaccaggtgcatgatgttgtcggtcaggtcctgctcgccgcccgagatgaagatcttgctgccggtgatgttgtagctgccgtcgggctgcgccacggcgcgggtgcgcatcaggcccaggtcggtgcccgcgttgggctcggtcaggcacatggtgccggcccactcgcctgaggcgatcttcggcaggtagagcgccttctgctcctccgatccgttggccgccacgttcacgtaggtggcatgcgacatgcccggataggacgaccacgccatgttcgcgccgccaaagacttcgtagaccgcgttggccacgaccgaaggaaagccctggccgccgaactcggggctgcacgccagtccggcccagccgttcttcgtgaattcgtcgtaggctttcttgaagcccggcggcgtctgcaccacaccggccgaaggcatgctgcaaccgtgctcgtcgcccggcgcgttgagcggcgcgatcacctcggatgcgaactggccagccgcggtgagcacctggtcgatcgtcgcggcgtcgagctcgggctggccgcaggcctccagcatggccggcacctggagcagctcgtgcaatatgaattggaagtcccgcattggggcctggtagctcatggtgatattccttccttgcctcaagccacttcgaacaggcccgcggcgcccatgccgccgccgatgcacatcgtcacgacgacgaagcgcgcgccgcgccgcttgccttcgatgagcgcatgccccaccagccgcgagccggtcatgccataggggtgcccgatcgtgatgccgccgccgttgacgttcagcttttccggatcgatgcccaggcgatcgcgcgagtacagcacctggcaggcgaaggcctcgttcaattcccacaggccgatgtcgctcaccttgagcccgtgggtcttcagcagcttgggcacggccaggaccgggccgatgcccatttcctcgggcgccaggccggccaccgcgatgccgcggtacgtgcccagcgccttgagcccgcggcgctccgcaactgcgcgctccaccagcacgcaggccgatgcgccatccgagagctggctcgaattgcccgcggtgatgacgccgccttcgatgaccggcttcagcatggaaaggccctcgagcgtcgtatcggggcgattgccttcgtcgcggtccagcgtgacgtcgcggtagctgatcgcgcccgtctgcttgtcggccacggccatgcgcgcggtgatgggcacgatctcgtcatcgaacaggtgccgctcctgcgccagcgcggtgcggcgctgcgcttccgcggaatacgcgtcctgcgactcgcgcgaaatgccgtacttctttgccacgatctcggccgtgttcagcatcgggatgtaggcgtgctgcacgcgcgcgatgagcagcgggtcggcctcttcgcccacccacttgacgaaaggattctgcacggcggagatgttctcctggccaccgcccacggtcacgtccatgccgtccacgatgatctgcttggccgccgtcgcgatggccatcaggccggacgcgcattgccggtccatcgtctgtcccgggaccgactgcggcagtcccgcggcaagcgccgcgaggcgtccgatgttcatgcccgcagttccggcggccatcgcgctgccgacgaccacgtcctccacttctccgggattgatgccagcccgctggacggcatgctggatcgcatggcccatcagggtcggcgacttgatgttgttcaatgcgccgcgaaaggcccggccgatgcccgtgcgcgcggtggaaacgatgacggcttctctcatggttcaaactccaaggggttcggtaaaaaggtcggcgtagcggctcgccacgaccgagcggttcaggcgcagcgcgggggtgagttcttcgtcgccctgatgcagcgagcgcgggatgacgcgaatggtgcgcacacgatggttctcgggcaggcgcccgttcgcgatctccacctgcgccgcgatgagcgcagtgatctcgggcaggccgagcaggctggcgtagtcggtgaaggacaagcgctgctgctgcgcatgcttcctgatccgctcctcgtccagggcgagcagcgcggccgaatgtccgccttccgccggcacgacgatggcatcggcgatgtacgcactgagccggaatgcgtcttccgcaatttccgggctgatggattcgccccgtgcgccaatggtctgcgcgcgcacgcggccgagcaattgaacgcggccttgtgcgtcgacacgcccgaggtcgccagtccgcagccacccgtccgcaagggtcacggcggggctcagcgttccgcgcacccagtagcccgggcgcgggatcgcaccgcgcaccagcacttcgccatcgggcgccagcttcagctgcgcgcctgtttcgaacggcgcggaggcggtctccgtcgagcggctggcgagaacgatcctgcagaagccggcctcggccatgccgtagcagtcgagcatgggaacgccgatggcgtcgaaccagtcggccacctgcgcggggctggaggcgccgcccgcgagcgcgacccgcacgttccgcaaacccagggcggcgcgtatgcgcgcctgcgtcctgcgctgcagccaaccgggccggtgcgccgaaaggcacgaggcatacgtggttcgggcgactggcacggcctcctgcatgaacagctcggtcgttccttgcagcttctcgaaaaagcgtggggctgcgaacaggaagtgcggctcgacctcgctcatgtcgttgaacaccgtcgcgccgttctccggcaagtggagcaaggcttcgtgcatgagcatggccttctgtgccaacatgcgttcgccatagtgcgcgagcgacatgatcgacaaggtccgatcccccgggcgcagttgcagccagtggctcattgctcgcacttcccgcaagaagtcatgctggtgacgcgcgatcagccgcgccgggccggtgctgcccgccgtggccgcgaggaatgcaatctgatcgccggtaccggcgtcgattcgctggtcgaacagcgctggtttcctggccgcggcttgcgaaccgcgcgcaagccattcgtcgtaggaactgacttgcgggtccgtgaagcgcgagagcccgcgtgtctcgaggaccacgatgtggcgcaggtcgggacaggtgtcgcgtactgcgagcactttcaccagctgatcggcgttctcgacgaagaccacccgcgttccagcctcgacgagcgcatgcccgatttgcgcagccgtgctgcaggggtacatgccgtgagacacgtaacccatggcctgcgccgccatgtcgacgatcaaccatcggggccgattgtccgaaagaaccgagaccgcctcgccggcttgcagcccggcatcggccatcgcgagaccgatggcccgcgcctcgctgaaatagccgctccacgacaggccctgccagatgccgcgctccttgtgccggagcgcgggccgatcgccccattcggcgcatcggcaccgccacaactgaggcagggtcgtgaggcgcgcctcgtccgcggccagcgatgccgacacgtggatcacagggagctcttggccgggtcgaccacgctggagcgcgcagtccagcgaccctgcacgacttgctcgacccgcgtccattccgggtcgatgtggttgttggcgaagcgctgcgtgtcgtacgaagccacgcccttgaaggtggacgcctggagcgccttcaccagcttctcggtcgtcaggtcgcggcccgcggtgcgcagttcctggaggaaccagctggtgtagtcgtagaaggcagcggccacgtcgtcaggctccgccttgaaacgcttgcgatagccctcggcccacgatttctcggcggcggtggcctggtcgggcgtcgcgatgcgccaggtgccaacgccgtacacgccttccatcgcatctttgccgagggcgatggtgaggccggcacggcccgggctggcggtcagcacgttgacgccggtcaagccgagcttcttcacttcggccgccaccgcgatggtttcgcgcgtggtggttgcgcagacgatgaggtccacgcccgcggcctgcatgcgtgcgacgtgcgaggagaagtcgagatcgccgaccttgtagctggcctcggccgcgagcggcatgcccttggctgagagtgccgcctttacacccttgccgaccaggtcgccgaaggggccttcctggtagacgaagccgactttcttgctgcccaggttgccggtggcccacttcacggcggccgatgtcgtgctgtcgtagttcaggttggtcgtgaaaagcagcggcgtctggccggccgcctgccgcacgaggcccgaggcggcatacggcgcgaaacagatcacgccggcatccaccgctttcttgaccgtggccacgttcggtccggaaccgaaggggcagagcagggcaaagacctcgtccttgcggatcagcttgtccacggcacgcaccgcttgtgacggctggctcgcgttgtcttcgatgaccagccggagcttgcggccgttgatgccgccggcctcgttggcctcgtcgatgcgcatctggatgccgttgcggatcacgggcatggcgattgccaccgggccggaaaggtccaggtgcgtgcccaggacgagctccttgtcgcccacacccgcagcgcgcgcggatgttgcggcggtccacagggcgcctggcgccgcggcggccagggttgtcttcagaagggttcggcgatcgagtgtcatggcagggtccttttctcagttccaggaagggcgtcgccgcgccggccggatcccgccagcgacaccttgcggtagatggtgcgatgcgccacccagataaaactccttgatgtcttcgcgctgggagagggcctcgcagctgccagcggcagcgacgcgccccagctcgatgacatagccgtggtctgcggtggccagcgcgatcgccgcgttctgctccacgaccagtacggccgtcctggtctgctcgcggatgcgcttgatgattccgaagatgtccttggtgaacagcggcgagaggcccagcgacggctcgtcgagcagaagcaggcgcggccttcccatcagcgcgcggctgatcgccagcatctgctgctcgccgccggaaagcaggcccgcctgttggcgctggcgttcgcgcaggcgcggaaaccagtcgtacatctgctccatgtcccgcgcgatttccgtatcgcgccgtgcgaatgcacccatgcgcaggttttccgcgatggtgaggaacggaaatatctggcggccttcgggcaccagcaccacgccgccgcgggcgacttcatcggcgtccgtgccgccgatgggtcggccttcgaactcgacggttccattggagggcgcgagcacgcctgcaatggtgttgagcagcgtcgtcttgccggcgccgttggcgcccagcacggtgacgatctgcgcggcatgcacttcgaggctcacgccgtgcagcgcgcgcacggggccataccatgtctcgagattgcggacggacagcagcgaagtcatgagttcaggtccccagataggccgcgatcacgcgcgggtcggcttgcacctgcgccggcgtgccgtcggtcagaacctgtccctggtccatcacgaccacgcgatcggcgaccgcggcgaccagcgacatgtcgtgctccaccatgaccacggtgacgcccagttcggcctggatgtcctccagccagtacgcgagcctgcgcgtctcttcggggttgagcccggaggcgggttcgtcgagcagcagcaactggggttccgcagccagcgcgcgaccgagctcgacgaccttgcgcacgccatagggcagttccgcgaccggccgatgccggaatgcggcgagatccagcaggcgcacgacgtcttcgacgcgttcgcgcgtgtgggcttccgcccgctgcacggagggcaggttgaacatctgcgagaagaagttgccgtggttcgcgcggtggcggcccagcagcaggttctccagcaccgtggcgccttcgaacaattcgatgttctggaatgtgcgcgcgataccctggcggaccacgtcgtgccgcgccaggcgcgagatgtcgtgcccgttgaagcggatgctgccgctgctggcgtcgaacacgcgcgtgatgaggttcaagagcgatgtcttgcccgcgccgttcgggccgatcaccgcgaggatctctcccgcacgaatcgaaaagctcacgtcgcgcacggccttgacgccaccgaaggacaggctcagatgctcgacttcgaagaatgcggcgctcgatagggcccccacgcttgtcacttcgtgtactgcgctgccccccgggggggccttcgcgccttcgggcggccgtgcggcgctcatcggtaacgctccgatttcatgtagaccttggtctggtgaacactgctcttgcgcacccacgggaactcggccagcaccttgcggatgcgaacccagcgcgcgttgaggccgcccggctcgagcagtacgaagaaggtcagtacggcgccgtagacgaaaagctccagcccgaactgagcgccgagcctggcaggcagcgcttccttcagcgaggagatgaacgcgggcaggaggccgatcaggatcgcgccgaggatggctccgcgcaggcttccgagtccgccgatgaacaccatcaagacgagctgtagcgacagcgccaggccgaacgcttctggcgtgatgtgttgcatctggtgcgcgagcaatgcaccggccaggcccgagcacgccgctgaaaggctgaaggcgagcaccttggtgcgggcgacgtcgatgcccaggccccgcgcggcggcctcggagtcgcgaatgccgatgaaggcgcggccggtggcggaccgcatcaggttgaccagcaggagcaagaccaccgccagcaccaccaggcaaaggaagtagaaggcgcgcggaccgccgaggctgagcccgaagagggtggggtccggcacggccatcccgctgtggcccccggtgacgctcttccaacggccgagtacatgctcgcagacgatggcaaaagccatcgtcaccatcgccaggtgcagccccgacacgcggatggccggcatgccgacgagcaagccgccaagcgccgcgcccgccgtggtgaggagcagcgacaccggcagcggcacgccctgggtcaggaggatggtgtggatgtacgcgccgatgccgacgaacgccgactggccgagcgacacctgcccggtgaagcccgtgagcatcatgaggccgaggctggccacgcacatgatgaggatgaacgtcgcctcgccgatgtgatacgccggcagcatccagggtgcggcaatgagggccagcgcgagcaagccgtacgcaagccgctcgggcttgccgcgcagcagccgccggccatcttcgaatcccgtttcgtagcgtgccatggcgtcagaccctccgtccgtggctttcgcccaggatcccgcgcggatacaggatgagaaccgcgatgagcaccaggtaaggcgccacgtccttgatgccgtccggcaggtagacgccggcgaactgttcgatgaggccgatcaggagcccgccgatcacggcgcccggcgcactgccgaagccgccgagaaccagggccgccagcgccttgagcatgacgaaccacaggcccaggtcgaccagcgtgatgggcgcaagcagcagcccgcacagcgcggcgatggcgccggagatggcccacaccagcgaattgagccgcttcacgcgcacgccgcacagataagccgccagctggttctgcgacgtcgcgtggatggcaatgccgagcgtggtgcggcgtaaaaagtaatacaggagtgccgtcacgcccatggcggcgccgacgatcaccaggttgagctcggccaccacgctgccgccgagctgcatggattggcctgtccacggcgtgggatagctgcgcgactcgggcccgaagaacatgctgacgccgccgcggatcatgaagccgatcccgatggtgagcatgacgcccgagaactgggggcggccgacgatcctgcgcatgatcttcgcttccagcagaaagcagaacgcggccgagatgcacagcacgacgacgaagctgagccagaagggaaggccggccgcgacgacgaaaccccagccgaggaatgcggaaagcatcaccacgtcgccctgtgcaaagttgagaacctcggtcgccttgtagctgagtacgaggccgagcgcgacgagtccgtagattgcaccgctggagatgccttgcacgatcagttgggtcagttgcgtcatcacatcattcgcttggctttaaataacgatcgtttggtaaacggtggtgaactataggtttgcaaagagggcagcgtcaacacgccggagcgggtttggcgcagggacaaaccctcggtcaatcgaccggtgactctgataaaacacggtcgtttaccaaacgatcggcatgctatgatggaggccccacgattgctgaggcccattcatgcgctatccgacaaaccacaaagaggaaacccgcaagaagctgctcgcgaatgcccgagccatcgcgaagaagggcggcttcggaaccaccggtgtcgatgaattgatggcgagcatcggcctgactgggggcgccttctatggacatttcccgtccaaggaagcgctgttcgccgaactcctagaacacgaaatctcgaacagcaccgacatgctggccggggaccgcgactcgccgcccgaccacgtcgccaagcggctgcgcagctacctgagctcgtaccacgccctgcacccggaaaccgggtgcgtcctgccggcgctgggacccgagatcgcaagggcggggcccgaggtgcgtgcggccgtcgaggaggggctgaagcgcctgcagaagagctggagctcgcgcatcggcgaccctgatgcggcgtgggcgctgattgcccagtgcgtcggcgcactggtgctgtctcgcgcagtcgaatcggagcgcacccgcaaggaaatcctggcctccagccgccgcttcatcgaccagacgcatgcgctggacgaagctcccgcaaagccgtccaaggcatcctgaccgccgaagccgatgttgtctcggcgcaccactcctgcacctgcgctgatgcaaacgctctttgcaccgcagacatgcgcggttgctgccgccagccttcagcggtcggcctgcaccgacaccaaggcgcatcagctcgctcgcctggtcaggcagcactatgacgcggaactcggcaaggtcggtctcagaatcacgcagtaccggctgttgatggaggttctggcacatgggcccgtgcgcccctgtgacctggccgagacgatgtcgctctctccatcaacgctgacacgcactctcaggcctctcatctcggcaggctgggtggatcttggacagggcgctgacggacgcacccgcagcgtgcgcatcaccgctgcgggccgcaggaagtgtgccgagggcctgcctcactggaacggtgcgcaggccagggtgcatcagttaatcggtagccaaaatgtcagcgcattgcatgccctcataggggaatgcttgataagcatgtctgcagcggatagatgaccaagtgccttggtcttcgccgcggagcgcctttgagccaaggattccacgccaaggcgtcactggcccgcactgcttgcgcgcagctggggcgtagtggcttctacggtcgcttccttcttcattcaagttcacctggagatcgacatgaaatactacttggccaaattccttccaccccgcgccgactttctcgccaccatgacccctgctgaagttgacctgatgaaggagcacggagccttcctcaacgatcttcttcagaagggagtggtcgtggcgcacggcccggtggacgatccggcaggcggatggggcctctcgctctaccaggtggaggatggccaggatgtcagtgcaatcgccgcgaacgatccaatggtgaggtctggcggcgcccgctatgagatctttccgatgcggcatctgaaggcacgtggctgacaccacccacggctacgggacgccccgacggactggcgaccagcgctgtagtacgccgcttggccacgaagcggcgccgtcaattcacgaaccatgagcccaccatgacccatcgtccattctcgctagccctctggattgccgtgagcgccgtggccctgacacaggttgcctgcgcctacaaggccggggacgcagtcgatgcaggccgctcgaccgccacaaccgtaaggaccgagaacggcagcatcaaaggccttgcgaaaggagatgcagaagtgttcctcgggctgcctttcgcggcgccgccaatgggaagcctgcgttgggcaccccccgagagagccgcttcctggcagggcgtacgagacgggacggtcgcgggacccagttgcccgcagatgggtggttccccggtcatcggtcgaacggagaacgaggactgcctttacctcaacctctatcgtcccgcaggcatcgcttcgggcgcatcgctccccgtgcttgtgtatgttcacggcggggccaatacggtcggcggcgcagtccagatcgacggcgctcgcatggcggcagaaaaccgggttgtggttgttgccgtcaatcaccgcctcggcgcactcggtttcttgaatcatcccgcgctcgcccagcaggccaaggatcgcctggcgggaaactatgcattgctcgacatcaaagcagcactggaatgggttcaacgcaacagcggtgcattcggcggcaatccccacaaggtaacgttgggaggaacctcgtcggggggaaccaacgtttgcgcgctccttgtcaaccctggtaccgctgggcttattcatgcggcgattatttccagtgatgattgcttgcgggacgtcgatacggccgcgcaatcggaggcgcgcgcggcagcctttgcagccaagcttggatgcacggatccggtgagtgtcgcgacctgcctgcgctccaagagcgccggcgagttggtgactgcgggcggcgcttggaatccacatgtcgatcccaaaggcttccaccgcaagcctgcgatcgacgcgatcgcggcaggcgaatggaggccggtgcctgtattgatgggcagcatgcgcgaagaagggcgtggttccggcgtggctttcgccaacttcacggcccaggcgtacgcagcctgggtcacccggctcgtcggggctgaccgagtgccagcgctgctggcagcctatcctgcggacaaatacgcgggccagtacgcgctgccctacgtcattggcgacttcattaccgacagcggaatgcgcggtctcggcggttgcaccaacctggcgctggcgagatctctcgcgcggcaaacgcccacctactactaccagttcgaggatccaagcccaccggcgccctcgacgccgcccggctacgagtttcgcgcgtcacatggtctcgataccccgttcacgtggcccgattcgccgcacatggcgcagtcctcctcacggttcaccgaagcgcagtggcagttgtcgaaagagatgacccgctactgggccgctttcgccaagaacttcaacccggaggttcccggccaggcggcttggcctcgactgatcgcggacggatcgttgatgtcgctgcggccgggcggacggagccaagcctcgcctgtcgcacagtttgcagagctccacaagtgtgcactgtgggaaaagatgccctgggtgctcgatcgcggcgaacgctgatctgctgcgatgcggagcggaaaagacttgcgtcaggccgcaagcggacagcagggcaaacgacagcgttgggtgcgacatcgtcctcatgtcttgcgcccgagcgatttcggctcagatgcaggtggcgaaggcggttgcgccgcttcgccggatcgaccgggatctcaatgcgacatgattgctgccgctctgatgggctcagcctgccagccgccgcccagcgccttgaacgcactgaccgccgcgcgcgccgactccgtttgcgcttgcgctcttgcatcggccacgcgcagcacgctctcgtcggcctgcagcacttcgatcaggctgaccacacctcgctgatacgccgcgaacgatgccccccgcgcacggccgagcgatgcctctccctgcgcgagcacggcggcctgttcctcgcgcttgaccaaggtggagaacgcgttttccacgtcttcggtcgcacgcagcgcggcaagccggtaggccgcgagcaactccgcgtcctgccccttggcgagttcgatctgcgcatcgatgcgcccgaagtcgaacagccgccagcgcaggccgagcagggccgcagcctggctggcgcccccggtgaacaggttgccgctggccaccgacgtggcgctgccgatcgttcccgccagggacagcttcgggtaatactcggccacggccatgccgatgcgggcgttcgatgccgcaaggcgccgctcggcggcgatcaggtcgggccggcgccgcagcaattcggcaggcgatccggcggcgctgatgcgcggcgcgacgggaatggccgcggctgtcgcgagttcggcgcggtgcgcgcccggcgccgcacccagcatcacgtcgagcgcgttcatggccgcggcctcgcccgcctcgagcgcgggcaccgacgcacgaacctgcgccagcgcgccctcggcctggcgcaactgcagctctgcggccagccccttgccgtagcgcagatcgatcttcgacagcaggtcctgctgcgtgcccacttgccggcgtgcaatgtccaggcgggtttgcaggccgcgcagggtgatgtagatgtcggcggtctgcgcggccaccgccaggcgcgtggcggccgcgccggcctccgaggcctggtagtcggccagcgcggcctcgcgtccccggcgcaggccgccgaagatgtccagctcccagcttgcgccgaggtttgcttcgtaggcgttgccgtagcgatcgaaacccggctgcgcgttcagcacctggcccagcggcgtctccaccgactggtaggccctggcggcttgtccgccgagattgcccgaaggcagcaacgccgcgttcgctgcaccgaggctggcccgtgcctgcgccatgcgggcggaggcctgcgcaagatcgagattctgtttcagcgcctgttcgacatagcgggccagttgcgcatcgccgaagccggtccaccaggccgccagctcggcgttggcggtggccgatcgccggtcgagcactgcctcgccaatgaagcggtccggcagggtcggggcaggccggacatagtcaggcccgacagcgcagcctgcgagcaggctgaacagcaggggcagggcaagcgtacgttgggacatgggttgctccgagacggcggacgggaaaagcagaaggaagtgtgtgactataattcaatttggtcacttgttgtcgtttgtttgtccgggcagtaagctccgggcatgaacaacgcaacttcttctccgccggctgcgcggggaccggccgatcacgacgtgcgcgcgcagatcgtcgtcgcggccaccgagcatttcagccagtacgggtacgagaagaccacggtttccgaccttgccaaggccatcggcttctccaaggcctacatctacaagttcttcgagtccaagcaggcgatcggcgaaatgatctgctcgaactgcctgcgcgagatcgaggcggacatccgcgcggcggtcgacgcggccgatcggccgccggaaaagcttcgccgcatgttcaaggccattgtggattcgggccttcggctgttcttccaggaccgcaagctctacgagatcgccatctcggcggccagcgagcgctggcagtcggccatcgcccatgaagaatgcatccggcagatgctcctcgagttgctcaagcaggggcgggagtccggcgacttcgagcgcaagaccccgatcgacgagaccgcggcggccatctacttggtcgtttatccctacgtcaaccccgtgatcctgcagctcagctccgatcacacggagcaggcgccggcccagttgtcgggtctggtgctgcgcagcctgtcgccatagacgaataattttgttggtgactattgactaaaatggtcactgttatcagaatcggggccctgatcgattcgtcaatgggcccctcatgcactcgcgccgcttcctcacctccgtcttcgtctgcgccttgccgttcgcgttggtcgcctgcgacgacaaggctccggccgatccgcgcacccagacgccgctggtgcgcgccgccaccgtccaggccgccgcgtcggcatcgcgctcgttcacgggcaccgtagccgcccgggtccaaagcgacctgggcttccgcgtctccggaaaggtgctggagcgctttgtcgatgcaggccagacggtcaagcgcgggcagctgctcatgcgcatcgacccggtcgacctcaggttggcggcgcgcgcgcagcaggaggcggtcagcgctgcgcgtgcgcgtgcgaagcaggccggcgacgaagaagcacgctaccgcgatctgcgcggcaccggcgccatttcggcctcggcgtacgaccaggccaaggcgtcggcagatgccgcccaggcccagctcagcgcggcggaagcgcaggccgaggttgcgcgcaattcgaatcgttattcggaactcaccgccgatgcggacgggaccgtgctcgagacgctggccgagcctggccaggtcgtcaacgccgggcagccggtgatccgcgtggcgcaggctgggcgcagggaggccgtggtgcagttgcccgaaacgctgcgcccggtcgtcggctctggcggacaggccacgctgttcggcaaggaagatgttgccgtgcccgtcaagctccggcaactctccgatgcggccgacaagctcacgcgcactttcgaggcgcgctacgtgctcgatggcgagctcgccaatgcgcccttgggcgccacggtgacggtccatgtcgcggacggcaagcctgtccaggcaggtggcgtccaagtgcccatcggcgccttgttcgatacaggcaagtcgacgggcgtctgggtgatcggtggcgatccgtcgacggtgcgctggcagccagtggccgtcgagcgtctggacggcgaacgtgccctggtggccggccaactcaagcagggggatcaggttgtcgcgctcggcgcgcacctgctgcgcgaaggcgagaaggtgcgtgtcgcgacctcggccgcgacacctgcggcgggcggagcccgcccatgagcgaaggccgcttcaatctctcggcgctggccgtacgcgagcgatccatcacgctgttcctgatctgcctgatctcgctggcggggctggtcgcgttcttcaagctgggccgtgcggaagaccccgccttcaccgtcaaggtaatgacgatcatcacggcatggccgggcgccacggcacaggagatgcaggaccaggtcgccgagaagctcgagaagcgcctgcaggagctgcgctactacgatcgcacggagacctacacgcggcccggcctggcgttcacgaccctgacactgctcgacagcacgccgccggcgcaggtgcaggacgagttctaccaggcgcgcaagaagctcggcgacgaagcgggcaacctgccggccggcgtgatcgggccgatgatcaacgacgagtacgcggacgtcaccttcgccctgttcgcgctcaaggccaggggcgaaccgcagcgcgtgctggtgcgcgacgcggagatgctgcgccagcggctgctgcacgtgccgggtgtgaagaaggtcaacatcgccggtgagcagtcggagcgcatctacgtcgagttcgcgcacgaccggctggcaaccttgggcatcgggccgcaggacgtgttcgccgcgctcaacagccagaacgcgctcagtcctgccgggtccgtggaaaccagcggcccgcaggtgttcattcggctggacggcgcattcgacaccctgcagaagatccgcgacacgcccgtggtcgcgcagggccgcaccctgaagctgtcggatgtggccacggtcaggcgcggctacgaagacccggccaccttcatgatccgcaacggcggcgagccggcgctgctggtgggcgtcgtcatgcgggaaggctggaacgggctcgacctgggcaaggccctggacgtggaagcccgcgcgatcaacgccgagctgcccctgggcctccgcttcaccaaggtcacggaccagtcggtgaacatcagcgcatcggtcgacgagttcatggtcaagttcttcgcggccttgctggtcgtcatgctggtgagcttcctgagcatgggctggcgcgcgggcctggtggtggccgccgcggtgccactgaccctggcggtggtcttcgtggtgatggccgcgaccggcaagaacttcgatcgcatcacgctcggctcgctcatcctcgcgctcggcttgctggtggacgacgccatcatcgccatcgagatgatggtcgtgaagatcgaggagggctacagccatgtggccgcgtccgcctatgcctggagccacacggcagcgccgatgctctcgggcacgctggtcaccgccgtcggcttcatgcccaacggctttgcgccgtcgaccgcgggcgagtacaccagcaacatgttctggatcgtcggcatcgcgctgatcgcatcctgggtggtcgccgtggtgttcacgccttatctgggcgtcaagctgctgccaaacttcaagaagatcgaaggcggccatgccgcgatctacgacacgccgcgctacaaccggctccgtcgcgtgctggcgcgcgtcatcgcgcgcaagtggtcggtggcgggggcggtcgtcggcctctttgtcgtgtcgatcctcggcatgggcgtggtcaagaagcagttctttccgatctccgaccgccctgaagtgctggtcgaagtgcagatgccctacggtacctcgatcacgcagaccagcgacgcgacggccaaggtggagagctggctgtccacgcagccggaggcccagatcgtcacctcctacatcggacagggcgcgccccgcttctacttcgcgatggggcccgaactgcccgacccgtcgttcgccaagatcgtggtgcgcaccgccagccaggaggagcgcgaagcgctgaagcaccggttgcgtcaggccgttgccgacgggctcgcgtccgaggcgcgggtgcgcgtgacccaactcgtgttcggcccgtactcgccgttccccgtggcctatcgcgtcagcgggcccgatgcgaacgagctgcgcaagatcgcggcagacgtgcggcaggtgatggatgccagcccgatgatgcgaaccgtcaacaccgactggggcacccgcacgcccacgctgcacttcaccctgaaacaggaccgcctgcaggccgttgggctgacctccagcgccgtggcgcagcaactgcagttcctcttgagcggtgtgccggtgacgaccgtgcgcgaagacatccgcaccgtgcaggtggtggcccgttcggccggcagcacccggctcgatcccgcgaagctcgtggacttcacgctcgccggtgccggcggccagcgcattccgttgtcgcaggtcggcgaggtcgaggtgcgcatggaagaaccggtcatgcggcggcgcgaccgcatgcccacgatcacggtgcagggcgacatcgccgaggggctgcagccacccgacgtgtcgaccgcgatcaccgcgcaattgcagccgctgatgcagaagctgcccgccggctaccgcatcgtccaggccggctccatcgaggaatcggagaaggcgacgcaggcaatgttgccgctgttcccgatcatgctggcgatcacgctcctcatcatcatcttccaggtgcgctcgatctccgcgatggtcatggtgttcctgacgagcccgctggggctgatcggcgtggtgccgaccttgctgctgtttcagcagcccttcggcattaatgcgctcgtggggctcatcgcgctgtcgggcatcctgatgcgcaacacgctgatcctgctcgggcagatccacctcaaccagcaggaggggctcgacccgttccacgcggtcgtcgaggcgaccgtgcagcgtgcccggcctgtgatcctgacggcactcgccgcgatcctcgcgttcattccgctgacgcattcggtgttctggggcgcattggcatacacgctgatcggcggcaccttcgcggggacgatcctgacgctggtgttcctgccggcgatgtattcgatctggttcaggatcaaaccaggcaacgcgacccagcccgcgcactgatgcgcttcatcatcattcatcgaaatcgaaggaaccagtcatgtcgagttcatcagtcgtcgtagtgacgggcgcgtcctcgggcatcggacgcgccgccgcagaaatgttcgtggcgcgaggctgccgggtgttcggcaccgttcgcgacctgcgcaaggcacccgcgctgcccggtgtcgagtttgtcgagatggacgtttgcgaagaaggctcggttcagacgggcatcgactccgtcatcgagcgggccatgcgcatcgacgtgctggtcaacaatgcgggaatgatgatgatcggcgcggtcgaggaaaccgcgacggccgaggctgcggtgctgttcgacaccaacgtcttcggcatgctgcgcgtgacgcgcgcggtgctcccctacatgcgtcagcaaaaacgcgggcgaatcgtcaacgtgagctccgtgctcggtgtgcttccggccccgtacatgggcctgtattcagccaccaagcatgcggtggaagggctgtcggagtcgctggaccacgaggtgcgccagttcggcattcgcgcaacgctggtgcagccggccttcacccgcaccaacctcgatgccaatgcaccccgtgtcaaggcgcggatcgcgggctatgaccgcgaacgcgaactggtgtcgctctcggtggctaacagcgtgagcagtgcgcccgagccgcacggcgtggcgagcaccatcgtcgaggcggcgcttggcccctggcgtatgcgctgcacgccgccggggcaagcgtcgctcttgacgaagttgcgccgcttcatgccggcgggaccagtggacacgagtctgagaaaacagctcggactcggcggttgctaagccgttgctcctccgcacaatggcggaagacttccggattttctggcgagccggctcgagcctgcgggattgcgcatgaggatggattcaaaatgacgacttgcctcaataccgcagcgaaccaaagaccgccgatacatgatcacccttcaccattgcgtcagcgcacgctcgttccggcccttgtggacgcttgaagagatcggcctctcctacgagctcaagatgctgccctttccgccgcgcgtgctgtctcggtcgtacctcgaggtcaacccgcttggcacggtgccgatgctgtccgacggcgccatgcgaatgaccgaatcggccgcgatctgccaatacctggcggcgcgattctcggcgggccagctggatgtgggtcgtgacgagccagacttcgggccgtacctcaactaccttcatttcggcgaggcgaccttgacctttccgcagacgctggtgctgcggtatgcacacttcgagttggcggagcgaaaacagccgcaggtcgccgacgactatgccaagtggttcctggcgcgcctgcgaacgctggagccgctgctcgcagaacgcgactacctctgtgcgggccgcttcaccgcggcggacgtgtcggtcggctatgcattgttgcttgccgagcatctgggcttggcagagcgcttcacgccctcggtgacggcttactgggagcgtctgcaggcacgaccgggtttcaacgcggcgatggctgcgcaattgcaagctgccaaggcgcagggtgtctcctcgacccccgcaccggccatcagacccgatagtccttgacggtgcccgcggcccccatctgacgcttcagcaagcggcgctttgggattgcgccttggcctgcacccgggcgtggcggagtggctgaaacccttcggcgactgtttgtggccgagtgggaaagccatcgtccgatccgcagtagcgggccacggcgcgtcccagatgcgtgatctcgttcactgtcgcacggggcggtgctgcgccgtgcggcggtgagaatgccaccttgatgtacccggcgtcttccaggtgcttcagttgatcgatgacagcgttgccccagaactgcatcggcagccgcgcagccaggacttgggtgaacaacgtatgccccatgtgcctctccagtcttcaatcctggatcacatcaatcgcgctccgcgggaaaatcgcatcgaggtcggagcgaagttgcgaatgtcgcccaacttcgcgatctcggcgaggccttcgtcggtgatcccctccaccgtcgccatcgaaacctgtgcgtaccgcccagccggctcaagggttgcgaacctggcctcgatcagccccgtggccatgagcacggacacggctcgaatttcttctggctcaacgacctgcaccggcagttgagtgtggagaagcctcatcaagaacaagagtggcattcggtcccccggttgccggcgcttgctttgcgcaatgtgccggcttgttttgggacggaaagtgtgttcccgggtgtgagaggtcgcaaccgggcttatctgcaaccagggggtcaatatgtgaaaaacatcacatttggagacgtattcaggtggagagatgccccgtgggcacgttcgacatcactctcgagcagggtgggattcggattgatagcccgattgctcatcgctctgcaactccaccagtgcccggtacagttgctcgggtgagatcggcttgtgcagcaggggaatcccgctggccagggcttcgcgcagacgctccggggccgtgtctccggtgatgatgagggcgggtgtatggcggccttcctgccgatgcaattgctgacgcaattcggcgatggcgtgagccccggtgcgcggcccacgcagtcgatagtcgctgatgatgcacgcggggggattctgcagcgccagcggcagggcttcctccagggattcggcgttgtcagaggggcagccccagctttgcagcaggtgcaccatggcgctgcgcacagtggcatcgtcgtcgatcaccagtacccgcatgggttgcaactgcggccccttttgcagcgggggtggcaccggtgcgaccgacaagggcagctccagccggaacacgctgccccgctcaggcttggacgacagcgtcagcccatggcccaatgacttcgccagtccgtcggcaatagccaggccgagccccaggcctttgtgccggtcgcgttcagggttgcccagttggtgaaactcccgaaagatggcttgctggtcggctggtgcgatgccgatgccggtgtcccacacctcgacactcacggtgtgccgacgttttcggcaagtgaccagcaagccgccgcgctgggtatagcggatggcgttggagaccaggttgcgcaccaccatgccgaccaggatggcatcggattgcacggcaagccgggtttcccgcgagcggtagaccagccccttggcatcggccagcggagcaaagtcgttctcgatctggtacagcaggtcttgcaggagaaagggttgtatctggggctgcaccacgccggcttcgatgcgcgaaaagtccagcagggtgttgagcatgtcgctggaggcgcgccaagccgaccgggtgctgaccaagacctcgctctgatacatcgacagcggggtacgcgacagcacgtccagaaacaggccttgggcgtggatgggttggcgcaagtcgtggctggcggcggccaggaaacgcgacttggccaggttggcttgttcggccgcttctttctggacatgcaggcgttcggccaagtcggcaatctggaagcgagcccgcagcgattcggtcagcttgccgttgagcgtccgggcaaagcgcaccgccagcagcgaataggcaaaaatcgtcaggccgacggcctggtacaagcgagtgccaagcatcagattgcccgcgacggcactcaccgcgcagggcaggaaaaagccatgaaaggtcggcagatggatggtctgcgaaatcagcgaactcgagaccatgccggccagcatgagggtgaccagcaagcggtgctccacttcgccgtattggagcaagcacagagcaccgccaccccacagcaaccccgaggcgagcgacaggaccgtgtgcagatgaatccggcggctcacctccgcctctgtcacggtctggtgccgcagccaccaccagcatgccaggcgcaccaacgcgtgcccaaccaacaacccgctccacaccagcagcacggccaagggaagaacctcgtgcatcacccacagcagtgcagtggccaccagcagactgccaaggacgatgaacggcacgttgctctgcaacgtgatgaactggtgcaactggatctgggattcggccttggaagacagaggcgcaggagcgggaggcgggttcattgaggcagtcttcggcaactaccggagcctgagttgtttcacgttgaggatttgcctgcgcagcgccccgctgcgtgagtcctgttaaccaatcagcccgttttggcgtgccgcaaacgtggcctgcgagcggctgttgacccccagcaggcccaacaccgcttgcacgtgcccgcgcacggtgaactccgacacctgcaggcgccgggcaatgagcttgttgggcagaccctcgcacagcagatccagcacctcgcattggcggggggtcagccggggcacgctgggctttgtcggggcgctgttggcgaggtgcggctgctgcagatgcgccagggtgtcgcgaatcaccgagatgatcttgtccggggtatcgcccttggacacgaaagccgccgcgccgcgtgccagagcctgggcgatggtgtccggcgtcgcgatggaggacagcatcaccaccggcacctgtggccagcgctgccgaagcagccccagcccttccagtccgttgacaccctgcagctgtatgtcgagcagcaccagcgcggggggctcgtccgtcgtgcgcacggcttgttccagggacgctgcctccaatacctcgacgtcggccatgccctgcagcaaaaccaggcgcagacccgagcggaaaagcgcgtggtcgtctatgagcagcaaacgcgagagggacatgcgcaaattacaacattggttgcaaaaagtttcaatcagtcaaaattgactatatgcgtgcctgggcgccgtgtgcacgatgcaattttttgatacaaaaaacaggggctatttctccatgaaccacgcctaccgcctcgtctggagcgacgccgccgcacgctttgtgcctgcccccgagaccgccaagggccgcggcaagtcgtcgggacgcggcgctgccgtcgtggtgctctgtgcggcactgctggccagcggcgcgtgggccggccccagcggcggcagcgtgagcgccggcagcggcagcatcagccagaacggcagcaccaccaccatcacgcagggcagccagaacctggccatcaactgggccagcttcggcattgccgccggcgagcgcgtcaacttcgtgcagcccggcaccagcgccattgcgctgaaccgggtcatcggcccggagtcctcggtcatcaacggcagcctgagcgccaatggccaggtgtggatcctcaaccccaacggcgtgctgttcggcaacaccgccagcgtcaacgtcggcggcctggtggcctccacgctgagcttgagcgatgccgacttcctggccggcaagcgcagcttcagcgccaatggaagccagggcacggtagtcaaccagggcagcctgaccggtggctacgtggccctcttgggcaagcaggccagcaacagcggcaccatcaccaccgccaacggcacggcggcactggccgcgggcgacaagatcacgctggacttcagcggcagccggctgctgtcggtgcaggtggacgaaggcaccctgaacgcgctggccgagaacaaggggctgatccgcgccgacaacggcacggtgatcctcacggccagcgccaaggatgcgctgctgaacacggtggtcaacaacgagggcgtgatcgaagccaagggcatcgacgccgcgggcggcaccatcctgctgctgggcggcctcaacggcggcaccgtcaaggtggcgggcacgctggatgcatcggccagcggggcccacgacggcggcttcatcgagaccagcggcgcgcatgtgcaggtggccggcggggcgaaggtcagcacgctgtcggagacgggcaagaccggcacctggctggtcgacccgaccgacttcaccgtcagcgccggcagcgcggccggcaccacgagcggcatcggtgccgacacgctgtcggccaacctggcaacgaccaacgtcacgctggccaccgacaacagcacgggcaccgacagcggtgacatcaacgtcaacgcggcggtgagctggggggccaacaccacgctgacgctgaatgcgtacaacgacatcaacatcaatgcggcgatcaccgccacgggcaccagcgccgggctggtgctgaaccacggcaactacgccagcacgggaacggtcaccagcggcacggactacaacgtgaaggcgcccatcaccttgagcggggccagcgccgcgctgggcatcaacggcacggcctacacgctgctgcacagcatggctgagatcgacgccatcgacagcaccggcctgagcggcaactacgcgctggcgcaggacctcgatgccggcggcaccacctacaccagcgcgctggtgggctcgaacagcttcgtcttcggcggccgctttgccggcctgggccacacgatctcgaacctgaccatcagcgccggcagcgccaacagtgtgggcctgatcgcgcaaaacttcggcaccctccgtgatctgggcttggtcggcggcagtgtgtcgggcggcgaccgcgtcggttcactggtgggcttcaacggcagcagcggcaggatcagcaacgcctatgccaccggcagcgtttcaggagacgactacgtcggcggcctggcaggctacaacggcgtcggcggcagcatccgcaacgcctatgtcgccggcagcgtttcggggactggcgacttcgtcggcgggctggtgagcgtgaattacggcacgatcagcgacgcctatgccgccggcagcgtttcgggaaccagcagctgggtcggcgggctggtgggcgtgaacgcgggcagcggcagcatcagcaacgcctatgccaccggcagtgtttccgcggctgccggcaactacgtcggcgggctggtgggcttgaacgacggcggcgcgatcagcggcgcctatgccaccggcaatgtcctggcaaccggcggattcgtcggcgggctggtcggctacaacaacggcggcatcggcaacgcctactgggacagcagcaccaccggccaaggcgccgcggtgggcacgaacagcggcacggtcaccaacgtcaacgccgtcaccagcggcaccgcctacagccacggcagctacgccaacctgggcacctggaccgaaacggtttcgggctccggcgtctgggtggccaaggacggcagcggcaacccgcagtgggtgatggtcgaaggcgcgacccgccccttcctgtatagcgagtactccaccagcatccgcaacgcccaccagctgcagctgatggcctacaacctctccgccagctacagcctggccgccgatatcgacgccagcgaagccgccggctccaaccccagcggcatgtggaccacggcgggcttctcgccggtgggcaatggcacggtggcgttcagcggcagcctggacggccaaagccacaccatcgccgacctggtgatcaaccgcagcacgacgtcgaaggtcgggctgttcggccagaccggcagcagcagcgtgatccaaggcgtcggtttgctgggcggcagcgtcaccggcggcgacgaggtgggcagtctggtgggccacaacgaaggcagcatcagcaacgcctacgccacggggaccgtcagcggggccaacggtgtgggcggcctggtgggctacggcttcggcggcagcatcagcaattcctttgccacgggcgccgtcaatggcgccggcgactgggttggtggtctgctgggattcagctacgccagcagcatcagtaatgcctacgccacgggtgccgtcaatggcgccgggaacgatgttggcggtctggtgggctacagcggcggcttcaacggcagcatcagtgatgcctacgccaccggcaccgtcaatggcaccggcaacgatgttggcggcctggtgggctacaaccgcggcagcatcagcaatgcctacgccaccggtgccgtcaccagcgcgggcaaccatgtcggcggactgacgggtcttcactaccttggcagcatcagcaatgcttacgccacgggcgctgtccgcagttccaacgcggctggcgtcgtgggcggcctggtgggctacaacgacaatggcagcatcagcgatgcctacgccacgggtaacgtcactggctccggagacaatgtcggtggcctcgtgggcctcaacgacggcgtcatcagcgatggccacgccacgggggccgtccgcggggccaccgccgttggcggcctggtgggccgcaacagcggcagcatcggcagttcctacgccatcggcaccgccacgggtacgaacgacgtgggcggcctggtgggcttcaacttcggcgtctacagcttcatcggcaatgcctacgccacgggcgccgtcagcgcatccaacgactatgccggcggtctggtgggccgaaacggcgccggtcgcgtcgtcaatgcctacgccaccggggctgtcagcgcggccaatgactatgcgggcggcctgatgggctggaatgacggggacatccgcaacacctacgccaccggcgtcgtcagcggcgccggccttgtgggcagcctggtggcccacaacgccggctacgtcacggcatcgttctggctcggtgcgggcaacactggcgtgggcctcaatgcggggtcggtcgatgcgctgacacggggcctgagcatcagcgaagccaccagcgccagcacctacagcgccgccggctgggacatcgccaccactggcggcagcagcgcggtgtggcgcatctacgagggcaacaccatgcccttgctgcgcagcttcctgaccgcgctgaccgtcacggccggcaacgtcagcaagacctacgacggcacgaccagcttcagcgacagctacgccctcagcgatccaggtgccgacaccagcctcatcacggggaccgcgagctacgacaccagcagcaagaatgtgggcagttacgccatcaccgtcggcggcctgtattccagccagcagggctacgacctgatttcagcgggtaccgccagcatcaccgccgccacgctgaccgtcagcggcgcgactgcggccgacaagacctatgacggcacgaccggtgccatcgtgagcggcggtagtttgagtggcttggtcaacggcgacacggtgacactcagccagagcggcagcttcagtgacaagaacgtcggcaccggcaagaccgtcaccgagaccttcgccatcagcggcagcgatgccggcaactacgtattggccagcagcagcggcattaccacggcaaacatcactgccgccacgttgaccgtcagcggcgcgactgcggccgacaagacctatgacggcacgaccggtgccatcgtgagcggcggtagtttgagcggcctggtcggcggcgacacggtgacactcagccagagcggcagcttcagcgacaagaacgtcggcaccggcaagaccgtcaccgagaccttcgccatcagcggcagcgatgccggaaactacgtattggccagcagcagcggcacgaccacggcaaacatcaccgcggccacgttgaccgtcagcggcgcaactgcggccgacaagacctatgacggcacgaccgccgccaccgtgagcggcggtagtttgagcggtctggtcggcggcgacacggtgactctcagccagagcggcagcttcagcgacaagaacgccggcaccggcaagaccgtcaccgagaccttcgccatcagcggcagtgatgccggcaattacgtgctggccagcagcagcggcattaccacggcaaacatcaccgccgccacgctgaccgtcagcggcaccaccgccgcgaacaagacctacgacggcacgaccagcgccaccgtgagcggcggcgccttgagcggcgtgatcggcggcgacaccgtcgcgctcggccagagcggaaccttcagtgacaagaacgtggccacgggcaaaacggtgagctacaccagcagcctctccggtaccgactccggcaactacgtgctggcttccagcagcggcaccactaccgccgacatcacggccgccacgctgaccgtcagcggcagcaccgctgcgaacaagacctacgacggcacgaccgtcgccacggtcagcggcggtagcttgagcggcctggtcggcggcgacacagtgacgctcagccagagcggcagcttcagcgacaagaacgtcggcaccggcaagaccgtcagcaccaccagcagcctttcgggcatcgacgcgggcaactacgtgctcgcatcgagcagcggcagcaccacggccgacatcacggccgccacgctgaccgtcagcggcaccaccgccgcgaacaagacctacgacggcacgaccgccgccacggtcagcggcggcttgagtggcctcgtcggcggcgatgcggtcagcttgagccagagcggcagcttcagcgacaagaacgccgcgaccggcaagaccgtcagctacaccagcagcctgagcggcaccgacgcgggcaactacgtgcttgcgtccagcagcggcagcaccacggccgacatcacggccgcgacgctgaccgtcagcggcaccagcgccgccagcaagacctacgacggcaccacggccgcctccctgagcggcggcagcctgagcggcctcatcggcggcgacaccgttgcgctcggccagagcggaaccttcagtgacaagaacgcggccacgggcaagacggtgagctacaccagcagcctctccggcaccgacgcgagcaactatgtgcttgcgtccagcagcggcaccactaccgccgacatcacggccgccacgctgaccgtgagcggcagcaccgccgtgaacaagacctacgacggcacgaccgccgccacggtcagcggcggtagcttgagcggcgtgatcagcggcgacaccgtggtgctcggccagagcggcagcttcagcgacaagaacgtcggcaccggcaagaccgtcaccgagaccttcgccatcagcggcagcgatgccggcaactacgtgctggccagcagcagcgccaccaccacggccagcatcaccgtcgccgcgttgacggtcaccgccaacaacgacagccgcgtcgccgacggcagtgcctacagcggcggcaacggcgtcagctacagcggcttcgtcaatggcgagaccagcagcgtgctcggtggcagcctggtctatggcggcagcgctcagggcgccaccgcggccggcagctacaacatcgcggccggtgggctgaactcgggcaactacgcgctgagctatgtcgacggcgcgctggtgatcagcgcggcggtggccagccccgtgccgtcgagccccgtgccattgggcgccaacccgtcgcttggcgatgcgcagcagcgcgcactggccagccaggccgacttgccgaagccgccggccaacccgcccgagcggctgagcatcgaacagtgcgggctgcgcctggacgaacccgcgaccgacttcttcacccttaacgagaacaagctttcatgcatgtcacgcctcgaatcccgctgagcctgctgggcgcttccctggcgctgagcgccgcgacggtttctgccgccacgccggacgccgggcagatcctgcaggagccccgcgcgcccttggcggtaccgagtggcagcgcgccggtgctgagcatcgacaaacctggcgccggcactgtgccggagggcggcgcgcgggtccggctctcggccatccgcttcagcggcaacaccgctttcagcaatgccgcgctgcaaagcctgctgaccgacgcggtcggcaacgaactgacctttgccgagctgacccgattgaccgatcgcgtgacgcggcactaccgcgaagccggctacctggtcgcgcgcgcctacctgccggcccaggcggtcaaggacggcgtgctcgacatcgcggtgctggagggcaatctgggccaggtcacggtcaccaataccgctggactcaaggactccgctctggcgcctttgcaggcactgccattgaacgccccggtacaagcccagagcctggaccgcaccctgctcacgctgtcggacttgccaggcacccgcgtgcagtcgaccctgcgcccgggcacgaccgtgggagcctcggacctgctggtggaggtgaacaagacccgcgccttccagggtattgccgatatcgacaacttcggcagcacctacaccgggcagtaccgcgtcggcaccagcatgtactggaacaatccgctggaccggggcgaccagatgagcttgcggctgcaggtcagcaacaccagcatgcactacgcgcgcctgggctaccagttgccgctgggtcgcgatggcacgcgcgtgggcgtggccgtgtcgcacctggactaccgcctgggcaaggactttgcggcactggacgccgacggcaaggccgataccttcagcctgtatgtgcgccaccccttgctgcgcagcctggagagcaactggtatgcccagctccagatggacgccaagaatctgcgcgacaccgtgggcagcaccgccaccacgtcggtgcaccagctgcgcaatgtcgtgctggggctgaacggcgactggcaggatgcggtgggtggcggtgccggcaacagcctggccctgaacctgaccaccggccagctgcggctggacaacgacagcctggcgcaagacgcggccagcacccgaagcgccgggcacttcaacaagctgaactaccagctgcaacgcgtgcaggccttgcgccccaactggtcgctggcactcaacctcagcggccagctggccgacaggaacctggcttcggcggagaaattcagcctgggcggcaacaacggggtgcgggcctatgcgcaaggcgaggccctgggcgacgcgggctggctggccagcgcggcgctgcgctggcagcctgcgccgggctggcaactgcaagctttctacgacgcgggaggcgtgcagctcaaccaccgcgcgtgggaccggaccggcagcacgagcaaccgcgcgcatctggccggcgccggtctgggcgtgggctgggcgacggacaaggtggcgttctcgctcacctcggcctgggccaccgagggccgggccagcgatggccgccgcggcgcgcggctgtgggcgcaggcgaccgtggcgttctgaatcgttgaatcaagcgggttcgccggcctgagcgtgacgcgggccagcgcgagagggcgagcacagcagacttgccgcgcgtcgatgttcgccacgagcccgagtcggccacctgcacttgcggctgtgcgctcgagcgcatcgcgaagacgtggccgagacgctcgaccacgttctcggtgtgtcatccaaaaatccgtttgacactgcgaataccttcttctatccttcgcgccacgacgaaacccatcatcgggtgagtcgggcagcaacatcgctgcttcacataccggctatgaaagccctcgaacaacgcgcaagcggggtcgagggcttttttgtttttggagcttcaatgacatcgaccgacaaggtccctttgagcggccaggccttcccggacctgatcgtggcgagcgtgcagatggaaccgcgggtgggccacacggccgccaacgtcgcctgctcggtcgagcgcatcgaacaggccgcagcacagggcgcgtcgatcgtggtgctgcccgaactggccaacagcggctacgtcttcgaaagccggcaggaagccttcgctctcgccgagaccgtgcccggcggcccgagcacgcaggcgtggatcgacgtggcgcgccgctgcaaggtgcatgtggttgccggcatcgcggagcgcgggggcacccggctgtacaacgccgccgccgtcatcggtcccgagggatggctcggcacctaccgcaagctccatctctggggcgacgaacacctgttcttcgaagcaggcaacaacggcgtgcccgtcttcgataccgaatggggtcgcctgggcgtgctgatctgctacgacggatggttccccgaggtgtaccggctgctggcaaggcagggcgttgacatcgtctgcatgcccaccaactgggtgcccatgccgggtcagcctgccgaccaacccgccatggccacgacgctcgtcatggcgaacgcgcacagcaacgggctcagcgtcgtgtgtgccgatcgcgtcggcaccgaacgcggccaggccttcgtggggcagagcgtgatcgtcggctcgcagggatggccgctggcggggcccgcctcgctcgaccgcgaggaaatcctctacgcgcgcatcaacctgaaggcctcgcgccaggggcgccacctcaacacgttcaaccacgtgctgcgcgaccgccgcgacgacgtctacgacctgatgccgggcagcggccgactgctgtcgcggcattgacgtgggaattcttcggcctggcgccgtcgctccctgttttctccttccgtttctcaactccaacctcccgaggactttgccatgaagagcttttcgtcattcacacgcatcggcgcatttgccgccttcgctgcgctcacggcctgtgcggaggccgcggacccgatccgcatcggcgtggccgtgggcctgtcgggcgccaacagcgtggtggcgcccgcggtggtgcaatcgtcgcagcttgcggtcgagcagatcaacgcggccggcggcatcctcggccgcaaggtcgaactggagatcgtggacgatgcctcgggcgcagtaggcgcgcagaaggccttcgacacgctggtcttccagaagaaggtccaggccgtcatcgccatggagaccagcgccgcgcgcaatgccgcgctgcccgtgatcagcaagggcaagattccctacatctacacctcgttctacgagggccgctcgtgcaacccctggatgtacgtgaacggctgggtacccgaacagcaggttgcgccgatggtcgactatttcgcgagcgccaagggcgcgaagaacttcttcctcgtgggcaatgactacgcgttcggccgcggcatgctggaattcaccaagaagtacatcgagaagaagggcggcaaggtcgtcggcgaggaatacctgccgatcgacggcagcgactggacctcggtggtctccaagatccgctcggtgaagcccgatgcgctgatcagcgcgacggccggtggcgctcctaacgtttccctggccaagcagctgaagggcgctggcctcacgctgccctatggcaacctcgcgatcgacgaaggcacggcaaagacgatgggcgacgtggccacgggcctgtacatgtcggcctcgtacctcacgggcatcgacacgccgcagaacaaggaattcatcgccgcgatgacgaagaagtttggtgccgacctgaagacgcccaacgaactgtccgagccccagtacgaagcgttcttcctgtacaaggcggcggtcgaaagggtgggttcgacggactcggccaaggtgacccaggcgctgggcgaggtgtcgtacaccggcccgcgcggcgcagttgcgatgaacagcagccgtcacacgcagctttcgatgcggctggggcatgtgcaggccgacggatcgatccagatcctggagactttcaagaacgtcgatccgggcgcacagtgccccaacatcaagtaagcgctgacagaaagcgcaactgactgaccttcggagcccctcatggtgctattgctggacttgctcacgacggcggcgatgctgttcgtcgtcaccgcggggttgctgatgatcttcggagtcatgaagatcgtgaacttcgcgcacggtgccttgctcacgctcggcggatacgcgagctacgtggtgacccagctcaagctggacccgtggctgagctggccgatcgcgctcgttgcggggatgctggtcggcatgcttgtcgagtggctgatcgtgaagccgctctacaagcggccgctcgacgccattcttgcgacgtggggcctgggcatcatcatcgggcagctgatcgtgctgagcttcgggcgcgaggtgcagttcgtcgacgcgccactctccggcacctggtcggtgctgggcgtggactactcggcctaccggctgctgctcgtgccaatcgccatcgtcctgtgcctgttgctcacgggactcttgaacggcacgcgtttcggtgttcgcacgcgtgcggtgatcatgaacgaggcgcttgccagcggcctgggcatccattccgggcgcgtgcgcttcatcaccttcagcctgggtgcgggcctgggtacgctggccggcaccatgatcacgccgctgtcgagcgtggatccgaacatgggcctgccgtggctggtgagcgccttcatgctggtgatggtgtcggggcattcgatgctcagcctgctcgcaacgtgcgttgtcttcggtgcctgccaggtgctggtgagcacctatgcgagcccggtgctcggcggtctcacgatcgcggtgctggcggcggtgaccctgcgcatccgcccgaaaggatttgcccgtggctgaagcaatcaacatggcgagaccatcttcttcaatgcgccgcacgctccagtcggggcgcggcatcgccgtgctcggggccgtggggctcgcgctggtcatcgttgggccgtgggtgttcgacacctacctgctcaacatcctgatcaaggccttcttcttcgcgatcgcggccatcacggtggacgtgctgtgggggtacacgggctatctgaccttcggccagtcggctttcttcggcatcggcgcctatgccgcggggctcgtgttcacccacggcggcttcagcgtgccgatggtgttgctggcgttcggcgcggccgtgctgacgtgcgccgcggtgggtgcactggtcggatggctgtctttctaccgaggtgcgtctcccttcttcgcgacagtgatatcgctcgtgctgcccatcgtgctgacgcagctgctgttgtcgggtggcgaatggaccggctccagctccggcctgacgggctatgagaccttcgatctgtcgatggaggcctggtactgggtgtccggcaccatgctgctgctggccggcgttctgggctgggtgctggtgcgcagcgatgccggccgggtgctcgcagccatccgcgacaacgaatcgcgttgcacctatctcggcattccgatcgagttcgtcaagattgcattgctggtcgtcatggccgtcgtggccgggcttgcgggcttcggctacggtgcgttcagcggcgtggtggcaccggagctcaccggcttcgcactcgggaccgaactcgtcatctgggtggcgctgggcgggcgcggcacgctgtgggggccattgatcggcgccgtgctgatcaacgtcgccacggcttacctgagcagcagcatgccgtttgcgtggcagttgatcctgggtgtggccttcgtgctcgtgatcgtgctgctgccgcaaggcctggtgccgttgctcctcaagccgttcggcctcggacggcctgccgggcacgtgccggcgctggccgagcgtccgctcgatgaagcgcccgcccaggacgcagccccggcccttcgcatgcaccaggtgacgcgacacttcggctcgctcaaggtcttgcagggcatcgatctcgaggcccatgcgggcgagctggtcggcctgatcggcccgaacggcgccggcaagaccacgctgatgcggtgcatgagcgacggcgcggaccgcagctcgggcacagtgacgctgtgtggcaacgacatccgccagctcccgccggaggcctgcgtgcgcttcggcctgggacgcaagttccagaacgccaacatcttcgagtcgctcaccgtcgctgagtgccttcgcattgccgggacggtgctcgaatggccatccctggtgcgccaggaccgcacgttgcgcctgccgccctatgcactggacgtggtgcgcacgaccgggctcgatgcgaagctcgcgaccatcgcgcgcgacctctcgcatggcgaacagcaggcgctggagctggccatggtgctggcgctgaagccgcgcatcgtgctgctcgacgagccgacggccggcctcaccaagacagagcgcacgcaggtgggcgtcatcctctcgtcgctggcgcaccgctaccgcctttgctgcctgctggtggaacacgacctcgattttgtcgaggagattgccacgcgcatcgtggtgctgcaccagggcgcgatcgtgatgcagggcagcttcgaggaagtggtgaattcgtcgctggtgaagaccatctattcgggcagcgcccatgcgtcaagggaggccgaatgagccaggctgcattgaggctggaggacgtgaccagcggctacggcgaatcggtggtcctgcgcggactttcgttgagcgtgggtgcgggcgaggccgtggcgctgcttggcaagaacggcatgggcaagagcaccttgctgaagaccgtgatgggctacctgccgaagaagggcggcgccgttcatctggccggcgccgacatcacgcgcatgccgccgcatcgcgtcgcgcgccagggcgtcgcgtatgcggcgcaggagcatgcgctgttcgcggatctcagcatccgcgacaacctgcggctcgggctcgccagggagtccgagttcgacgatcgcttcggggagatcgaaccgctgtttccggtcttcaagagccggctggcgcagtatgcgggcacgctctcgggtggcgagcagaagatgctgctgctggcccgggccctgatgatgcggcccgcgctgatcctgctcgacgagatcaccgaggggctgcaaccgtcggtcatcgaccggctcgccaatgccttgctgagcgagcgcgcgcggcatggcacggcactgctcgtcatcgagcagaacgtgccgttcgcgctgcaggtcgccgaccgctatgtcgtgctcaagcagggcgagctgatcgacacgggcgacgccaaggcgcacggcgccgtcgacaaggtgttcggccatttgcgggtatgagccgcttgtcgcgtgaggctggaggatgactgaagacatgactctccctatctgcgtcctggtcgctaccggcggcacgatcgcgatgaagatcgatcccctgcggaaggtgcccgtgccggccttgtccggcgaggatctgctggcggcggtgccgggcatctcggagctggcccggctggaggtgaacgacttctccaacctgccttcggaccacatggggccggataactgggcgttgctgagccggacggtcgacgccgcattgcagcggacggacgtggcgggcgtgatcgtctcgcacggcaccgacacgctcgaggaggccgcctggttcctggacctgacgctcgccagcgagaagccggtggtgcttgccggcgcgcaacgcaacgcgtccacgccggatttcgatggcccgcgcaacctgatgaacgcggttcgcgtttgccttgcccccgaagccaaaggaaagggggtgatggtcgtcatgaacaaccagatccatgctgcccgcgatgtcaccaagacgcacaccagcgaggtggaatccttcaagtcgggcgacttcggatttctaggctcggtcgaccaggaccgcgtggtcttctcgcgctcgccgctgcgtcgccagcatgtggcgctgcgcggcaaggcgctgcccccggtggagatcgtgccgatgtacggcggtgcgagcggcgccatgctgaacgccgcggtggtgcagggcgccgggggcatcgtggttcaggcattgggcctgggcaacgtcaatgtcccgatgttcgaggcgatcgagtctgcgatccggcaaggcatcgcggtcgtcgtctcgacccgggtacccaacggacgcgtggcgcccgtctatggattcgtgggcggcgggagtacgctcaaggcggcgggagcggtcttcgcggacaacctgagtccgcagaaggcacgtatcctgctcatgctggcgctgcaggaaaaccccgacccgcatttcttgcagaccctgttcgaccgatgaaggaaacgccgatggtcaccgacacagacatctccgccgacgacggctggcgcatcggcgtgttgtactcgcgctccggtgccacgggcgtgaccgaatcggagcatttcttcggcacggtgctggccatcgaggagatcaaccggctggggggcgtgctcgatcggccattgctgccgatcgcctatgaccccaagggcgactccaccgaataccgccgccttgccacccaattggtgctggaggacgaggtcaacgtgatcttcggctgctcgcgctcgtcgagccgcaaggccgtgctgccggtgatcgagcgcaacaacgcgctgctgtggtactgctcgttctacgagggcttcgagtattcgccgaacgtgatctacacgggcgccgtgcccaaccagaacagcgtgcagcttgccgcctacctgctcaagaacaggggatcgcgcttcttcctggtgggggccgactacatctacccgcgcgagtcgaaccgcgtcatgcgcgagatggtcgagcagcatggtggcgaaattctcgacgaggtctatctgccgctggaggcgaccgaagccgaactgcaggaggtcgtgcgcgacatcgtggccgcgcagcctgccgtggtgttctccacgatggtgggcgagtcggccaggcgcttctaccagatctaccgggagcatggcctggagcccgaccgcgtgccgattgccagcctgtcgatggcggaggaggaagtccggctgaccggcgccggcatctgcgcggggcacatcaccgcggcaacctacttcaactcgctgcagaacgaaagcaacgcgcgcttcgtcgaactgtggcgcacgcgcttcggcgaccggccaaccagcacctggtcggagatggcgtacagccaggtccatcttttcgcgcgcacgctggagcgaaccggcagcctggacacgcgcaagctcgtcaaggcgtcgcatggcgtgcatttcgagtcgccggaaggccgcctgtcgatcgacgccgagaacaaccactgcatgctgacgccgcgcatcggcgtctgccgcgccgacggccaattcgacgtcgtgtggcagggcgcggggccggtgaagcccgacccgtacctttcgaccttcgggttctccgagttctggctgagctgaggccatgagcagcctgcgccgcctctacgacgatctccgcagcatctgcgtggcggtcgtctatccgccgggcgaagaccgggacgtgctgctcgaccagctcaagcgaatcggttgccgcctgaaggtcatctggccgttcccggccgagccgccgaagggaaccgacgtcatcttcttccaggtgtcgcaggaactgcagggcagcgcgagctggagcgccagtgccgtcgaggccacgctggttgcgctgtcggactacgagagccccaccacgctgaagctgctgctcgacaccagcgcccacggcgtcatcacgcggccgtttcgctcgagcggcgtgctgagcacgctggtgctggcccgttcgtcgcggggctaccaggagcggctgcaaagcaaggtcagcaagctcgaggaaaccatcaagtcgcgtcggcagatcgagaaggcgatccggctgctgtcggagacccagggcctgcaggaggcccaggcctacgagcacatgcgggcacgcgccacggccctgcgggtcacggttgcggaagttgcgctgatggtcgtggacgcacacgaagcgatggagaagctcggcctgggaaagccgcctcgcggcggctgaggggatcacgagcgctgcttcatcgatgagggctagtccgagttcttgaagacgaactcctgaacggcaacaacatcggtcggctgattggcacatttgtactgtgccgcggcctttttcactgccgcgtgaaataccttcggccccgaaacgatcgttacctcacgcacgatgccttcacgcaccagcagttgcgccttcacgacgccatcgacaccatctcgaagtgctgccgcaggcatttcgggccggacctgtgtcggacaggccacgccgatttcgacgcggcctggagccgcgggcggcgcgatgggtgctgtgggcgctggaggagccacagcggccggctccagcgcgggtgcaacggaaggcgctgacgccggctcaatcgccggcgcggccaagggggtcggcgccggcggcgtgggtgcgcgcgacatgggcggcgcgggggccgccttggagaccacgcgttttacctccttgggcgaaggaggcggtggcggtggtggcggtggaaggaacacgtcctgaatgaccacggcttccatcggcttcctggtgctttccggtgtgccccgggtggtaccgctcagcagcgcgtatccaaccacaacatggacacccgcaacgacggcccaaccgatgacgcgacgcgacggatcactgccgcgatagtcttttctcgacaacgtgctcattggacaaactgctcactgccgataacggcgatcttggaaagccccatgcgccgggaagaagacaggacatgggcgaaggccgcatagctgcagtccttgtccgggcgcaggctgatctccggctgcaccgcaggccgcgaagcctccagaagtttgctgccaagttcttccgcggtcgtgggcatcccctgccaataaagggcatcccgggcgtcgatgtcgatttgaatcttctccggcttgatgggcgctgccgtcgatgtgccgacgggcagttcgatgttcaccgcgtggagctgaagcgggatggtgatgatcaacatcacaagaagcaccagcatcacgtcgatcagcggcgtggtgttgatgtcgggttcgatttcgtggtcgccgcctcttctcgcgaagcggcggctcgtttttcttgccatgcaagttccctttttgatgagtgcgaggctagccgtcgagcgcggggggttgggtaatgaaagccactttggcgatcccggcgcgctggcattcgagcaggatgcggccgacactgtcgtaccgggcgtccatatcgcctcggatctgcacctcgggttgtggattcatggccgtcagcggcctgagcttttccgacagcgcttgcgcatccttcaacttcgcgtcgaaccaatagatacttccgcctttgtcgacagaaacgatgaccgtccgaggcttggcctcctggacctccatgcgttccttcggcaaggaaacgggtacggaggcggtcaccgccggtatggtgatcaggaagacgatgagcagcaccagcatcacatccaccaagggtgtcgtgttgattgccgaaatcacgtcgccttccgccgagggtccggccgtcattgccatggtgtactaccttgaatgagcaaggtgctcatgccgccgccatgcggcccagggcggcatccggacccgccctcatcgatggcaccgtggagccgaccacaaccgcgttgagttcctcgctgaactcccgcacctgatccatgacggccttgcttcgcttggccagcaagttgtacccgagcaccgcaggaatcgcgacagccagaccgatggcggtcatgatcaatgcctcgcccacagggcccgcgaccttgtcgatggaagcctgccccgacagcccgattgccgtcagcgcgtgatagatgccccacacggtgccgaacaagccgacgaaaggggacgtggatcccaccgtggcgaggaatgccaagcctccgtgcgcattcgcatgcacccgatccacggcgccctgcacgttcatgggaatccagtcgggaagcggaatgtggcgcttgaggcccgagtgattggcaaccgcttccgcccctgcttgcgcgacataccggtacggactgtttttctcgagcgccgcagccccctcctgcaccgaggatgcattccagaacttccgattcatgctcccggcatagccgtgcatcctcgccaactcgatgaacttggcgaccatgatgtaccagctccccgcgctcatcagcgcgagcagaaggagcaccgtccgcgcgaccaggtcggagcccctccacagcgcctgaaccccatacgggttctcgatcgggtcgacgttcttcctgtcggaactcttcacttccgaagcggcagccatcccggactgcactctttccggcgctgtggccacggacggcggtgtcgcggcggcagcctgggcgaaagcaggaggtgccgcttgaagggcaatgcacagcaagccaacgctcacggcccgcgcaattttgtttgctcgataagacaaggtaatcctcgcaaaggtagaaatgttgattgcagggccgacggtggccctcgaacgcagtcgccgcagatacggtgcggttcaaggcgaatcgaccgaagcggcacagaagagaaaaaaacttcaggtcaaaggctcgatgacctccatcacttccggggtgccgaccatgacgaatccatcgcaatccgaaagcggcgcgtggcgcgccaggagcccggcttcttcgcacaatgccaggccgccggccatgtcccagatcttcacgctgtgctgcatgtgaccatcgaggtacccgatggcggcaaatgccatggcagtggctgttgaacgataggactccaccacccatccggcacggcgcagcgcaatcgtggtcgccgccgcgcggtcgatgtctgaatgcgcatcgccgaccgagaccacgcggacggcatcgaaggccgtctcgcgcgtggcgggcaacccgttcacgaacaggcccgcacctcgctgcgcacccacgatcaagcccaatgcgggcatggcaatcacgcccatcgttgcccggccctcgctgatgaagcccaatgaaacgccccacaaggggatgccgcgcaggaaattggtcgtcccgtcaatgggatcgacgacccaggtgctttccgccaacgcgccggaggcccgttctccatcgccgaattcctcgccgtaaacgggttcgcccgggtgggttcgcgacagctgctcccggatgtacctttcgacggtctcgtcgacagccgagacaaagtcctggggctgcttcgtgcgcatggacacgtcgcggcgatgtgtgaagctgtgcagcgcggttgccgcagcgctctccacaatgccatgtgcaagcgcgagccgaggaggcatgctcacgccggatgaaagttcaagcattgaattggtctcttccaagttgggcggtcctgcaggacctgacgacgtgttccggcatcacaccttgcccatgcccgcagccaatacgtcgtcgcgcatgattcggcccgcgaccaggaaaatcaccagggcgggaatcagcaagacgatggccaccaccgatgcaagcggaaactgcaaggagtagggatcgaggtactggtaaagcaggatcggaagtgtctggaccgcgggagcgcccaccacgaaggatttgtcgaactcctcgaagctggccacgaacgacagcagcccgccggccagcagcgctggcaccgacaagggcagaacgacatgcacgaaggctctccacgggcttgcccccaggcagcgcgcggcgtgcagaagttcgtcgggcatggtctcgaaggccgcgaccagcaatcggatcatcaaggggagcgtgccgaccatctgcaccagcaccacgcccgcaaacgtgtacatcagtccgagtcgcaggaacacctctcccaagcccaccgcgactaccacgcccggaacgatcaatggcgccaggatgaaaatctcgatcaaccgcttggcgcgcatcggaaacttggccagcgcccacgccgtgggaacggaaaccactgcagtcagggccgtcacggtcagcgcaatcagcacactgctgaccacggcttcgatcatcgagtcgtcgcccaggatccgggtccaatgcgccagcgtatagcggccaggcagcagccccggcggtgaccagcgttgtgccgtgctccacaggaacatgagcaccagcgggagaccaacggtcaccgccaatgcggcgtagagacccagcgagacccacacacggtcgtctgcggtgaagcggcgcggacgcaccggggtgtctcgatcggcggcagcggcagatctagtcatcatcgcgctccgctttgcccgacagcagctgcgtggcccggcccacgaggtggtagtagcccagcaggaccgccactgcgaagacgctcagcaccatccccatggcatagaccagctgcaggttcccattgccgaattcggcgaccatgtgcacggtcagcggctggggagccgccgcgccaatcaggtccggaatggcaaatgcgcccatcgacccgatgaaggtcagcaatacggcggcggagatgcccggcaaggccattggcaactcgacatgcagcagcgtgcgccaacggccagccccaagggtgcgcgacgcgctgacgatgtcttcgggaatggcggcaaatgcaccgccgatcacaagtgtcatgaaaggaagctgcttccagaccgtggtcaggatcacgccgacaccccgtggatcgcgcaccagcggtggcagatggagtccgaatggcgccactgccctgtcgaggaaacctccgcgttccgccaccgtcaggacaaccagtgcggcgatgatgccgggcaccgcgatcggcatcttgtacaggccattgaacagcttgcgtccccaaaagtgtctgcgcaggaccaaggcaagagctatcgacagcaccagcgtcacggtaaccggtgcgatgccgaagtacatggaccggatcagcgcgcgctgcagcgtggggcggttgaagatttccgaatagtgggccagcgtgaatccgcttgcctcggccgtgatgcccacgcttccgagaacgctccagagcaggggcgtgccgaacagcaagccgagcaagcccagtcccggcaacagcaagcccacagcccggatcgaggcgccgatgcgattcgatctcatcgctcagcctccatgccttcttccagtggatgcagttctgaactcagcgccacggacacgcgctggcccggctgcaggatggcgccgccgcccgaggtcgtcgcccgcagcgtggtcactcccgtgcgcaatgtgtagttcacctgaggcccggtgaaggagacggattcgatgctggccgctccgttttcatcggcggcgaccgcaacgtcttcgggtcggatcgagacccggacggttgtcctgttggccgcggaaagaggcacgcgagctccccagggaagaagagcttcgcggccttgaacctccagcgtcagcaggttcgtctgccccaggaactcggcggtgaacgtccgggccggtcttcggtagagatcgatgggtacccctatctcgaccacgcgcccggcattcatcagcacgatgcgatcggacatggccatggcttcggcctgatcgtgcgtcacatagaggctggtggtgccgacgcggcgatgcaactcggccaattcgtggcgcaggctgtcgcgcagcttcgcgtcgaggttggacagcggctcatcgaagagcagcagcgccggctgcatgacgatggcgcgcgccagcgcaacccgctgctgctggccgcccgagagttcccgcggcatgcgatccatcaagctgcccagccggcagatctcgaccgcgtgtgcaatccgctcggcctgggcgcccgccggaacgcgcttcatcttgaggccgaaggccagattgcgccccaccgtcatgtgcggaaacagcgcatacgactgaaaaaccatggcgatgtcccgacgctccgggggcaacgcttctatcctcgcgccccgcagactgatctctcccgaactgggcgcagtgatgccgctgatgatccgcagcagggtcgactttccgcaacccgacgggccgaggatggtcacgaactcgccgcggcgaacgtcgagatcgatgggatgaagcgcggccgtggtgccatagttcttgcacacctgccgcaaagatagttcggtcaccggaaaggccctttcagcgctgcgagagcaccttgtcttcgaacgccgtcgtcaacgcgcgcgctgctgcccagttcatcggcacggacagcttttcgtactgcgcagcgggaaccatcaatgcggcggtttccgtgctgaggacctgttcggcgcgtacgtccgggcgcagcgaacgcgagccgtaggtcgccagcttccaggcctggaattccttgccgaacgccatgtcgatgaacaacagcgccgcggccggatgggtcgtgttggcgggaacgatcaggccatctccgctggccgcctcgccgctggccagaagcgtcaggcgcaggctcggtggcacgagctgcgcacgctggaaccgaagcacctggtcctcccagacggtgccgatcgtcgcttgaccgttgttgatgagattcaaggtatccgcattgccattggcgagctccgacaccttcatgaggctccgcaagtaaatccaggccgcctccaggcatgggtcggacatggcccagctgcgcgcatcctcggggctcgcctgtgtcctgtagagcttcgtccggcaggcgtcgtccggcgcgaaatgcagcgccgccgagaacaggaatgcgccgccggcaccgcctttggcgggagaggtcatcacgaacctgccaggattgcgctgcgcccatcggagcaattcttcgtagctgcgaggcacctggtctgcgggcaggaccgcactgtcatagccgatcgcagtttggccgacgtgcaccacgggccaggtgccgcgcgtgcgcacgccgaacaccacttctgtcagcgctcggggcaccgtggccaattcgggcaggagcgctcccaggtccagatccgcaatgaccccgttcctggacagggcggcgaagttgtcgctgctcccggccagatagacatccgccggggagttttgacggaccttgtgcaccgcgatgagctgctggttcgccaagccgttcctcacgttgcgatagcgcacgcgcacgccatagcgcgcttcgaagcggggaatcaggccgttcttccagatgtcttcaaaacctcccgccgagttgtaaagcatcaactcgccctcttttctggcaagaggttcgagcaccgcgtaaaagttttctcgcgtcagtgcccgaacatcgaaggtcgcgttcttcatcggcacctgcgcatgcgagggctggaacgcaaacgcggatgcaagcaccgaggcgcacctggcgatggcaaggacatgccgccgaaggcgggcggcccatatgtgcgctttcatgcgaatttcacccgtctccggaagatgacagtgcgagttgagcagaacagttttcaagcctgatgaacgaccctgaacgcgaacatgtcgcgaaacgcgcagaactgaagcttgcgaatcaacaacggctgcccgagttctgaaacattgcgcgcccagttttcgctcgcctggagcatctcggccgattcctcgggcgtcaggaactggtgcaggtagccgagcgtcaggtgatattggtagcgctcatggttggcgtcccgcaggccggtcaaccgggacagctgtccccgcacggcatccagccggttcttggtctccgcgcgagcgggcttgagcttgatctggagcgtgccttcgctgcgaagggcaggtttcccgtcgacgacaaaatcgtagggctccgttgttgtggcgtccagcgcccgcatgcgctcggcatagatgcgcgtgacagcctccatgggcgtatcgggcgagaactcgccgggccacctgggcctgccgcgatccacctcgttcagtccgacgaagacggtgacgtgatagctcgacggcggcaggatgctgagcttccttgcgaaagactggcgcggcaggtctcgatagacgtccagcagccggtcgaacatgtcgaagtcggcaccctgctgcccgacgtgcccgatgaaggtgtttccggcgaagggctgcacggttccgtcggccctgaactttcgaccgacgtcgtggggtgcacggtgcggctgcacggtgtgcgcaggcgcctcgctcgatgccgattcggcacatacggcaccggtgccggcgagagccgcaacgcaccccacggcggagccgcgggacagaaacagacgacgctgaagcatggtggagatcctgctgaagtgtggataaggaagagcgaacatcacagcttgtaggtaaggccgacgagaaccgagggcgcaagcttccatgccgattggacgtactcctgcgaacggccgaagttgtattgcatgccctggcccgtgaggttgaggatgtccagcgtcaggctgagctgcttcgaaacgtcgtaggcgatctgcaggtccacattcctggtggactgctggtagcggttcgcatagaagcccagcgcgctgtagttcgggaagcggtcgtcccagagcttgctgacgtagttccaggcgatctttgcgtgcagcggaccgcggtcgtagtagagcgcgatgttcgcgatcttccttggctgctgcggcagtgcggccagcttcgtggtcgatccatccgtcagcgtgaccggatagttggcgtgggtgaaagtggcgttggcgctgatgcccaggccattgaagggagccggcaggaacgtgaggtccttcgtcgctccgagctcgatgcccgacagcctgaccagcccgtccacattgcgtgcctgcgtgaccagcaccggtgtcgacacgccactgacctgcatctgctgggtttgtccgtagttgaagatctcgttcttgatctccttgtagaacgccgcgacggaaacgatccctcgcccgttgtcgagataccagtcgtggccgatgtcgacgttgttcgacagccgtggtttcagatcgctgttgccctgcgaaagggtcgcgacgcttccgccggacgccaatgctcctccgcgagtcgccatttgatcgaagcgcggcctgcccatcgtttgcgacaagcccacccggagcttgctggatgacgtggtgtcgtaaacggcaacgaccgagggaaggagcttgtcgtagtccttcttggccgacaccggattccaagcgccattggtggaaaggaatccattggtgttgaaactcgtgtgctcgaaccgcaagccgcccgccagcaggaagcggtccgtcttgtactggccttgggcataggcggcatagacgtcttcgcggtagccgtaggttccgccgtactgcgcggccgtgtcgatcgcagcctgcaccctgccggcgttggcggcaaatgccgcatcggcaaggcccggatcgatcaccggaatgccgctgccgttgcaattgaagccgcaaatcgtgcccgagctgacggcagccaggctgtaaggcatcccgctccatgtcgagcgcgaaaaggaggtgtcggcgcgtgtcgaaacaaaacgcgcgcccaggccaaagccaaaccctcggctgtcgctctccatgttgcggcgcgtgttcgcctgcaggtcgtagaccgtctgcgcgtactccgtggcgtcttcccggtggtagttcagcgggtagcgagccaggttgcccgcatcgagcggtttcactgcgttgaacacgggcgtcgcaccgctggtgtcatagttgaaggacatgcccttctgcacgaagttgtcccaggtctgggggttggacacggacgaccgggagacgcttccccgcacgtcggccgtccaccccggctcgatttcataggccagttcgccatttgcgccgtagagcatccgctgccagcgcaagcgccccagctgggcggtctgatcgatcgagttcaaggtgcccgacgtgggcgtctgattggcattggcagccgttccattcacagccgcgacgaggtcgtttctgttggatttttcgttctgcttgagcatgtaggcgctcaggtggccagacaacggcccttccggcctccagtccagccgcgtcgtcaacccaagacgctcgcgcttgttgtcatagttgtaccagcgccgctcggtcggaaccgcatagccgttgccggagtagggcgtggaactgcgtttcccgttgcggtcataccagttcagagtgcctccggattcgatttgcggcacattgatgctgcggctccagtagctggccgttgtcagcaagccgaattcgttgtgatcgccgaagcgcttcgcccacttgcccgcagcctcaccgcctggcttcgagccgccgtacttgtcgcccatcaggttctggcccagcttcgcggatacgtcgaccgtgttgtccgggagctggaaggcgttggcggtgacgatgttgacgatgccgccgatcgcggcgccatcgctttgaggcagaaagctcttcgtcacatcgattcgctgcgcaatattcgacggaagcatttccatcagtatctgccggcttccgatgtctgctgtcgcaaaggcgaagccgtcgatctgcgtgacgttgtagttggcattcagtccgcgaatgatgacgaaccgaggctccccctgatagctcagcgtgttgacgccggtcactcgcttgagcgcatctccgacgttgaaatcgggaagcttgccgatctcgtcggcggcgatggtatcgacggccaccgcggactccttcttcgcggcaatcgtctttgcgttggacgagcgcacccccgtgaccaccacggtccccagcgaaggctccgacgtcggtgccgcagcttgctgcgcgtttgctgcggaagcagcgagaacaagaagaacagctgcggtgatcgtcgatggccgacctgcagggtgagcagtggcgtggcgcctgccgggcggcttctggatcgcgggacttgggcttgacacgggaacgctcctcgaggggtttggtttggaatggcaattactttaagttcattaaattaaaataatgtgacatcccgccgcctacactccgttgcatgaccgcagatcgccaagccacgacgctcagaccgcagttcctccggcgcgaaggagcatctcccgtcaatcccaatgaacgcgcactcctggacgccatacgccgatccggaaccatttcgagggccgatctcacgcgcgcttccggcttgagcgcgccgggggccaaggcactcatcgacagcctcagcgaacgccagctcattgaactgggcacgccatcgatccgtggacgagggcagccgagcgcatccgtcacgctggcaccggatttcgcctactgcatcggcacgtcggtgatggtcgacggcttcggcgtgacgctttcgaatttctccggacagctgctcgaaacccacttcacgccaacgtttccgatgcgccttgcggccgtggccacgggggtgcgcaaatcagtcgggatgatgctcaggaaacatcgcatcgatcccgagaaggtgttcggcatgggactgagcatgacggggccgttcatcggcagcggctcgcgcgtgaaccccccgctgtccatgcccgaggagtggatgcaggaagaattggacgcgtacttccgtgcccgcctggagatgccggtgtggctcgataacgacgcaaattgcgcggcgatcgcggagagcctgttcggcgtcggtcgatgggcatcgaatttcgtctatctgcatttcaccgacgggctgggcggaggcgtcatcaaggaaggcagagtggtgaaaggcagccacggcaatgcaggcgagctgggccgcatctttcctttgaccggcttgaagcgcccgagcctggaaggactgcgacagcaggtggcccagcgcggccgtgatgtgccgaacatcgaagccatgctcgcgatctacgaccccgaatggccggagatcgaagcctggctggacgaggtcggcccggggctgtccatcgtcatcgcggccatcgccgcgctatgcgatccgcaggctgtcgtgtttggggcgagacttccttccgatctggcccatcgcctcattgccaaggtggacctccaacaacaggcgcggcgcgacgcgcccatgccggaccctcgactggtcgtctcggaaggacctcgggatgcggcgtccattggagccgcgaatctgccattcaaggaacacttctttctgtgagcagcaggcatgctttcgctgaaataccgaccgtacgacaaggccgaagagaccgaggcggcaaggctcgagcctgccgccgccttcagaagttgtgctgaatgccggcgcccacggcgcgcaccacgtcattggcgacacgattgtttggatcgcttcgatcaaggaaggcgtacaggttggtgcgtttgctcaggttgtagaggtagcccagctggaatcgcttgagcttggcatcgcgattggtctggacatccttggtcatgtagttgccgacgagcttcccgttccccaggtcccaggacgcaccgacgtaatggacatcggtcttgctccgcgctgtcggaccgccctgagtgttgtcccggttgaagagcacccatgcacggatggcgccgaagtcgtatgaggcaacagccatccacttgtctttgacgtcattgaccagggcgccgccccgtttcttgttctgcccatagcccacgccgaggcccagcggcccactaccctcaccgtagctgagcgatacgtcggcttgcttgtagtcgctctcgaaacgcacaggcgtgttggcggcctccgtgatcccatcgccgttgaggtagtagcccgcgcgaaacacaaagttgttgacgatggggctcgcatagccgatggcattcgactcccgcgtccgtgcgttcaggatcgaggtgcccacggcggttgcaccggcatcgtggatgacgaactcggtatgtcgcgtgacgagtgcgtacagcggtgtccgccgaccatcaatgaagccgcgagcggcgacgtgcagtcccacgccgcgtccatcgcactggccttgacgatggacccggtgcgtgagctcaggccaaaccggaacgggtgctcaggtcaaactggaatgggtgctcagggagcatcggaatacgcacggtacggctcctatctgggggagatcagtccggcgcccgagaacctcatcaatcgcgacttccacgccgcagcgccgaatgagaagtggctcaccgacatcaccgagttccagatcccggccggcaaggtgtacctctcgcccgtcatcgactgcttcgatggtctggtcatcagctggtccattgggacgcatccagacgctgagctcgtcaacacgatgttggatgcggccatcgagacggtggtcgaaactaacgaccggcccgttgtccactcagatcgcggcgcccactatcgctggcctggttggctatcgaggatcgcagatgcgaagctcattcgctcgatgtctcgcaaggggtgctcgcctgacaacgctgcatgcgaaggcttcttcggtcggctgaaaacggaattgttctaccctcgggactggagggccgtctcggtcgagcaattcatcaaagaagttgattcttacatccgctggtacaacgagaagcggatcaagatctcccttggctctcgcagccccatcgagtaccgagagagtcttggacttgcggcgtagaaccagtccaagtttttatccgcacccccgccgggtgagttttccgtggcaatcaacaccgagctggcaccttcatcaagccaaatcgaagcagcaaccggcgtagtacggcttgtcgccgccctcgacgaatggcacttcgattgtcaggacctcgttgcgccaggcatcgcggcgcttgtagccagcgcttctgagttcggcccacagttcttcgacgtgctggatgcgataggggcagaacgcaatgccgatgctgttgatcgtgtagagcgtgcgttcggggtgcaccgccgtcgtgttcagcacgatgcgtttcggctttactgcgagaacggccaggatctcggcgattcgctgcggcaaatactgcaggctgcccgaggcatacagtacgtcgcagccgcttgcatccttgtaatctatggtgaagtccatctgggcgggcgcgtcgcgctgaacggccagctctttccctgtttgcaccacgccggggacgtcgcagactgtccagcgcaggtcatcgggataaggcagaacacggcgaaacgcgtaatactttattcccacgttgccgcccaggtcgaaaacgcgccgcatgccatcgtcgaacgatcttccgagccaaaaaaggccgggatagtcgtagaagtaaatctggtggctgtagagctcaccagccgccttggcgttgctgtatcccacagccttcgaatcaggcgccccggcctccgcggccgcaaagctctcaaacgagcccatgaagaggttttcggtttcattgacgaggaacttgcgccgatacgcgtggacgcggtagcgcaagggcagcaggttggcaagcatgagctggtttcctctttggctgaaagaacaccactgcgcgacgccctaacggcgcgccgccgcggagaactgcgatctccgaatcctagcgattccggccagatcttggtggcaccgtctccgaacgcgagttcgggccaccacatcaccgggaaaatgccagcgtgacgaactgctcagcttttgctagggggcgaatggggctgcctgcagctcgccgatgcgtaccggcgcggccgaccgggctcgcttcgagcatgtggcggtagcccgcgccgcgcttgccccagcgcaccgcttcggccatcacgcgcagcgaattgccgcgtttggaaatctggtaggcgtgcagcgaggcgtctgcggctgtcgagcggatcagcggcaggccgagcaactgctcggcgggcgtggtcgccagtgccacgtcttgtcgaactgctgcatcacatccacaagagcctgttcaacctcggccgtctgcaatttctgcatcagagccgttggcgcttcctataatccgcccggtcggtagaaccctccttgctggagcgatctccgccacggttcgaaggtgccccccatgccggaaatggtttgggaggttaaacgggaagcaggtgcgcgcgtcgatgacgcgcaatgcctgcgctgcccccgcaacggtaagcggatagagaagtttcgagtgagcacctgcgggtgttcgcagccactgcgcttgaatcgagcgtgggaaggcgaggcttctgttgttgtgcgcaagcgcatgacagcaacccgcgagcccggataccggccttcgcaatcgccttcggacgctgcgggagtgcgtttgtccgggctgctcggcacctgcgtgccgggttggcatcggctcgtgcaattgcagcgtgtgtctcttggaacagcccagcgggaatgcgggctagaggaacagcatatgcacaagcctgccgagctcgggatccggccccgggtttcaggtcctttcacgacccgacacatcacgatcccgggccttgtcgccttgctcgccagcacgtctgcgctggcgcaagagagcttgcgaccgatcgaggtgacggccccccggcaggatcaggcgccagcgcttcaggcaacaacgaccgaagttgccggcaggctgggcctgagcgtgatggaaacgccggcttcggtcgaggtcatcagccaggaaaccatggaacggcgtggcgcacggactttcgaggaggccttgcgcggcggggtgggcatcactgccggtggagcgcccggatcgccatcggtgatctcgacgcgcggcttcaccggaggtttcatcacctatctgttcgacggcgatcgcattgcagtgccgacgatggtgagccggccccaggacacctggaactatgagcgcatcgaagtcttgaagggcccctcgtcggtgctctacggtgaaggcgccatcggcgcggccgtcaacttcgtgaccaagcgacccgaccgcagcaaccccggggccgaggccatgttttcctatgggagcttcggcacggccagggccggcgtcggcctgggtgtcaacgtgggcgaggccagcgctttccgactggacttcagccaccagcagaccggtgggtacatcgaccgcaacaagcagcgctacgacaacctcaccatgggcttcagcacggcattgacgcgtgagctcacgcttgaactgtcgatggactacgccagggacagtgcgctgtcctaccagggcacgccgctcgtgccgcgcgcctatgcgctccagccgacggacatcgtcagcgacgccagcgggcgattggtcgatcgcggcatcgcgtttcgcaactacaacttcgacgatgccgagatgagtgcgaacagcctctggacgcgcgccaagctcagctggcagatcgcgccggaatggaagctgcgcaaccagctttcctactacacggcggacagggcgtggcgcaattcggagtcctttgccttcgctgcgccgggccgcatcgtgcgcgacctggtcggcatcacgcacgaccaccagatcctgacgaatcggctcgatctcacgaacacgtcgccgatcgggggaatgaagaaccggttcgttggggggcttgaatacacgaagaccgacttttcttccaaccgcgacttctccaacggatcgaccgcagccaacaatgcgctctcggtgagcgagttcgccaccatcccgggacgctacggcaactttgccgcgaaccccgccctgttcgcgggtgccggcaatcgcacgatcttcgacgcacggattcccacgggatccatcttcatggaagatgccctgtccgtcagcgaccgattgaccctcgtgggcggcttgcggcaggactacgtgaagctggcgcgccagaacatggacctcaacaccggggcccgggcatcgttcacgcagaagtacaagcccacatcggcgcgtctgggcgcggttttcgcgatcgaccaccacacttcggtctacgcccagtactcgaacgcgagcgcgccggtcggtacgggcaacctcctgctgctctcggcggccaacgccgccttcagcctctcgacgggcaagcagctggagctcggcctcaagcagtcggcgatggagggccgccttgactacacgctggcggcctacaggatcgaactcgacaacgtgctgtcgcgcgatttcagcaacccgacgctcacagtcaacagcggcaagcagtccgcgcagggcctggaactcgccgcggtctggaaggcgacacgcgagctgacactgagcggcaatctcgcatgggtcgatgcgaaattcgacagcctcatcgaggccggcaacgtctcgcgcgcgggcaacaccccgccgaacgtgccgggcgcggttgccaatctctgggtcgactacaaggtgccgggatggccgctgcgcatcggtggcggcgtcaaccgaaccgggtacgcctacgccaacaacgccaacacggtccgcatgaacgggttcacgactgcgaccgcctatgcgacctggagcctgcagaagggcgaaatcacctttcgcgttcgcaacctgactgaccagttctacgcgtattggagcggcgccaattcgaacaatcaagtcatgatcggcgcgccgcgcagcttcgaagtcagctaccgggcggccttctgatgagcgcgcgcgggagagccattcctgcattcaggccacggcgccatgcgccggcggcacgggcatgaagcgcgcactgatcttcatccacaagtggctcggcatctcgttggccttgctgttcctgatgtggttcgtcaccgggatcgtgctgtactacgtgccgttcccgaacctctcgcaggccgagcggcgcgcggggttgcagcctctggcgctcggcgctggttgctgcctgaccgccgaagaggctgccaggcgggccggcgtgagcttcgccgaggcacgcctgggcatggccggcccgggagagccggtctggcgactgctggtcgacgccgggcaggcgaaggccgcgcagtggcaagccttcgatgcccgcaccggcaccgcgacggccccgctcggcgccgtgcaggccatgaaggtggccgagtccttcagcggccgacgcgcgctttcggccgaagcgctggagcgtgaccaatggacggttccgcaaggcttcgatccataccgtccgctcttcaaggtcagcctggaaggagacgacggtctcgaactgtacgtctcgagtactgccgccgaagtggtgcgcgacacccgccgcagcgagcggttctggaactggatcggtgcggtcccgcactggatctatccgaccgtgctgcggcagtttccgcaggcgtggaaccaggtggtcgtctggctgtcgatccctggcgtggtgctggccgcgaccggactggcgctaggcatctggcagttgttcctgaaccgaacgcgctggattccctatcgcaagttctggatgcgctggcatcacatcgcgggcctggtcgccgcggtgttcacgctcacctggatcttctcgggcctgatgtcgatgaatccctatggcgtgttctcgtcacgcgggctgtcggcttccgagcgcgagcgctggctcggccctggccgggacgcggtcctggcgccgccgcttgccctggctgcggtctcggccggcgaggccggtgcgcagccattggaactggagcgggttcgagtcggcgcgcaggtctggtatcgaatccagggcacggaccggcggtggtgggtgcgcgctgacgacgtgagcgccgcatcgacattggatccggcactgccagatgcgctgatgtcgggcgtcctgcggcatctgcgtggcgaagacaggcctgcgtcgagcgtggtgcggatggatcgctatgacgatgcctactacgcgaagaatccaggctcggccgaagcctcggagggccggcccttgccggtctggcgcgcgcattggtccgacggcacggacctctatgccgatcccgcctcgggcagggtgctgttgcgggtcgaccggtcgggacgatggcagcggttcatgtaccagggattgcacagcctcgatttcgagccgctgcgcgaacggcctcggttgcgcgaggcgttggtgctgatcctgtcggccctgggcattgccttgtgcatcacatcgtgcgtcatcggctggcgcgccctggtgcccaaggcggtggcgcgcaagacaaccgggcggcgcaccgcatgagtggaggtgttccgctatgatcagcctgttggtgctcgcttcgtctttccggtcgaagcagttcaacgggaatcaggaggggtggcgcggcaagccatcgcgcgccctaacctgagctgcccccgcaacggtaagcgaacgtgagccctcgtgctcgccgctcgtgtctatagcccactaggtgaatccgcgcaatctgcgctgcctgggaagggaacacgggtcgtcttcgccagcccggataccggccaacgaggcggcgcgctgcgcgaacggcgcgccttgtggtgcgtacctgcggggaagcgggtgagcatggctggcgcggtattttctctatgacacgcatccccttcaggcgacatggtcctggctcacgccgctgtatgccgctgtgcggtggcgttcacgcgctgcgagtggccggcaggccgatgagggtcgagggatgattgcacccgcagacttcagctgtcccgcgctgctggtcacggccccggcctcgggccaaggcaagaccaccgtcactgccgctttggcgcattggcatcgcagccagggccggcgcgtgcgcgtgttcaagaccgggccggattttctcgaccccatggtcctcgagcgtgccagcggcgcgccggtgcagcagctcgacttgtggatgggaggggaggcgcactgcgccgagctcttgcaccgtgcggctgcagaggccgacctgatcctggtcgaaggcgcgatggggctgcacgatggagcgccgtcgagtgccgatctggcgctgtatttcggactgccggtactggccgtgatcgatgcatcgtcgatggcgcagacctttggtgcagtcgcccacgggctggcgacctatcgccccggcctgcagctggcgggcgtgctggccaatcgcgtgggcagcgcgggccatgcgcagatggtgcgcgagagcctgccggccggcatggcctggtacggcgcgctgccgcgcggcgggcactacgcgttgccgtcgcgtcacctcggcctcgtgcaggccggcgaggtcgacgacatcgccgagcgcatcggagccgccgcgcttgcgcttgccgagcacggggcgctgccgatgccgcctgccgtggaattcaacgcgccgctgcgctcggcttcggattcaggtctgcccgcctcgctcgccggcgtcaccatcgccatcgcgcaagatgccgccttctcgttcgtctattccgccaatctcgagctcctgcgtatgctgggcgcgcaactgtgcttcttttcgccgctggccaacgaaccggtgccgcaagaggcgcacgcgctgtaccttccgggcggttacccggaactgcacttgcaagcgctggcgggcaatgcagcgacgcgcgaatccatcgctgcgcaccatgctgcgggtcgcccgatggtcgcggagtgcggcggcatgctggtgctgctggagtcgctgagcgacgctgccggccacaaggcgcccatgctgggtttgctgcccgggcagggcgcgatgtccgaccggctcgtcaacctcggcatgcacagtctggagttgcccgaaggcgaggtccgcggccacacttttcatcacgcccgcatcgacacgcgcgcgccggctgcactgcacacgcgggcccggcgccaccacggccaagccgaagcggtcttccgccagaaacgccttttcgcgtccttcatgcatctgtactttccgagcaatccggcggccatcgccgcgttgttcaagccctgatcgcgcgctggcaacgccgcacgcgaccccacagaaccaccacagcccatgcaaacctcgacgcccacgcccatgcaaagccgcaagatccccgccaccatcgtcaccggctttctcggcagcggcaaaaccacgctgctgcgccacctgttgcagaacgcccagggccggcgtatcgcggtcatcgtcaacgagttcggcgaattgggcatcgacggcgagttgctgcgcggctgcggcatcggctgcgacgagaccggggcgccggacggccagttgttcgagctggccaacggctgcctgtgctgcaccgtgcaggaagagtttgcgccggtgatggagcaactggccgcgcggcgcgatcagatcgatcacctggtcatcgagacctcgggcctggccctgcccaagcccctggtgcaggccttccaatggccggcgctgcgcaacgcattcacggtggacgcggtgatcacggtggtggatgcaccggccgtcgccgccggccgcttcgcggacgacccgctggcggtagatgcccagcgccgcgccgacgaaaacctcgaccacgattcgcccttgtcggagttgttcgaagaccagctcgcgaccgccgacctggtggtcgtgcacaagacggatgggctcgacgcggcgacgctggccggcgtggaggccgtcattcgcgccgagaccgcgacaggcgtgaagctggtgcatgcgcagcacgggcgcatcgacctgggtgtgctgctgggcatggagcgggcggtggaggatgcgatcgaccagcgcaagactcaccacgacgaggaggaagaccacgaccacgacgccttcgactcggtctcggtgaccctgcaggtccctgaccgcggccgcttgctggccgccttgcagagtctggtcgagcgccacgagatctatcgggccaaaggcttcgtcgccctgcccggcgcagcgatgcggctggtggtgcaaggcgtcggcacgcgcttcgacagctacttcgaccggccatggcgcgccgacgaggttcggcagacgcgccttgtgctgatcggggcaggcctcgatgcggcggtcttgcaagccgaactggacgcggtgctggacgtggccgcggtggcctgacgcgtcgccgaaagccctcatgcatctgctgtccacccgccccggcggccacgtcgaagacggcggccagggcgtcgtgcgcgtggcgcagacgcccgcctcggtggtcgtgctcagcgccgccgacaccaccctgtcgctgctcgccgacgcggccgggcatatgggcgccgactatcccagcgtgcgcctggccaacctgatgtggcttcgacagccggcttccgtggacatgtatgtcgacgacgtgctgcgccatgcccgcgtggtggtgatcgaccatctgggtgccccgagcgactgggcctacctggtggagcgcgccatgtcctcggcacgcgaacgcggtcaatggctggcgatattctcgggcgatgcctccgaagacatgcagctgctcatgcgcagcagcgcgccgcatgacgattgccgccatctttggcggtgcctgcgcgaaggagggctcgacaatgcgaaggccttcttctcgctgatcggccatgcggcgttcgggctgggcagccggccgctgcagccggtgaccctgccttcggccgtgcgctatcggccacgggaggctgccggctgcgccacctggaaggcagaagcgccggtggcgctgctgctgttctaccgcgcccatctgcaggcgggcaacacggcggtgttcgacgccatgctggaagcgctgtcggccgccgacctgaacgcggtggccctcgccgtggattcgctcaagaaccccgacagccacgccgcggtgcaggcgctggtcgcggaacaccgcgtggcgatcgtactgaacgcgaccagcttcgcggtggcgtcgatcgacggccgcgacgatgggagcgcaggcgacggcgacccgtcactggcgacgctggccacgctggccggggacgcccccgtgctgcagctcattacggccggcggcacgcaggagcaatggctggccgacccgcacggcctcgcgccgcgcgatctggccatgcaggtggtactgcccgaggtggatgggcgcatcctcacgcgcgccatcagtttcaagggcatggcccggcgctgcgagcacaccgagctcgatgtgcttcgctaccaggccgagcccggccgaatggccttcgtggccgaactggcacgccgctggtgcgtgctgcgcgacaagcccaacgccgacaagcggatcgcgctgatcctggccaactacccgatcgacgatgcgcgcatcgccaatggcgtcgggctggacactccggcgtcgaccgtggtcgtgttgcaggaactgcgggccgcggggtacctgaccggggatctgcccgccagcggcgacgccctgatcgcagcgctgttgcgcggcatcaccaacgacagcgacgccaatggcggccggcccgccgcgcagagcttttccctggccgactacctggaagatttcaatcgattgcccgccgacagcagggcggcggtcaacgcccggtggggcgcgcccgagcaagagccgtcgctgcgcagcgggcgcttcacgattgccggcctgcgcttcggtcacgtcttcgtcggcattcagccggcgcgcgggcgtgccgtggacctggcggccacctaccacgacgcggacctggtgccgccccaccactacctggccttctacttctggctgcgccgcgccttcgcggtcgacgcgatggtgcatgtgggcacgcacggcaatctcgagtggctgccgggcaagagcgtggcactgagcgaggcgtgctggcccgacgccatcctgggcccgctgccgcatctctatcccttcatcgtcaacgacccgggcgaagggagccaggcaaagcggcgtacccaggccgtgatcatcgaccacctgatgccggcgatgacgcgcgccgagacctatggcccgctccagcagttggagcggcagatggacgagtactacgaagccctgtcgctcgacccgcgacgcgcgcggctgctgcgcgaggacatcctcggacgcaccgtgcgcgaaggcttgcacgaggaactgggtttcgcgcggccgaccgacgagagtgcccgggagagcctgttgaaggggctggacgcctatctttgcgagatcaaggaatcccagattcgtgacggcctgcatgttctggggcgttcgccgcaaggccgccagcgcatcgacacgctgctggcgctggcgcgttttccgggcggcacggccgccagccagaagagcctgctggtcgcactggcgcaagaccttggcgtggagggcgcggacggcttcagcgctctggcgccggactgggccgcgccgtggcatggtccgcgtccgaaggagttgcaagcgctcagtgccgaggcatggcgccacgccggccacacgcgcgagcggctggaactgctggccgcgcgcctggtggcggcgcaggcggtgtccggcgacacccgggcgggcgctgcgcacgatgccttcgatgtccatgactggccgcatgcggcaccggtgctgcagcgcctgaagaaggtgctggccccccgcctcgatgcctgcggcccccaggaaatgacgcaattgctgcgaggcctggccggacgcttcgtgccccctggcccgagcggcgcgccgtcgcgcggtcggcccgatgtgctgcccaccggacgcaatttctacagcgtcgacacccgtgccgtgcccacgcccacggcctacgccatgggtgcggccgcggcggaaagactgatcgagcggcacctgcaagaccacggcgcgatgcctggcgaggtgggcttgtccgtctggggcaccagcaccatgcgcaccggcggcgaagacgtggcgcaggctttcgcgctgctgggcgtgcggccgaagtgggccgacggcagcgcgcgcgtgatcgacatcgaagtgctgccgatggctgtgcgccatcggccgcgtgtggacgtgacgctgcgcgtgtcggggttcttccgcgatgcctttcccaacgtgatcgaccttttcgacacggccgtgcgcgccgtggccgcgatcagcgaagacgatgaatccgacgaggtgaacccgatccgtgcccgcgtgcggcgcgaggccgccgaggccctggcggccggccagcccgtcgaccaggcgcagcgccaggccacgtggcgcgtgttcggcccgcgccctggcggctacggcgtgggtgtgcaggaggtgctggacggcggtcgatggcaacacagtgccgacatcgcccaggcctatctgcaggccggtgcctttgcctatgggcagggcgaacacggtgttgccgcgcgcgcctcgttcgagcaacgtctggggcagctcgatgcggtgctgcacaaccaggacaaccgcgagcacgacgtgctcgacgctgccgatcacgctcagttccagggcgggatggcggccgccgtggcgcatcttgcgggcgcaccggctgcgctctaccacggcgatttcagcgtgccggggtcgccgcgcatccgcagcttgcgcgaagaggtcgcgcgcgtggtgcgatcgcgcgccgtcaacccgaagtggctggacggcgtgcagcggcacggctacaagggcgcggcggagatcgccgccaccgtggacaacctgttcgcgtacagcgccaccacgggcgtggtcggcgatcaccagtacgcgctggtggccgatgcctacctgcacgacgacaagacgcgcgagttcctgcagcggcacaacccgctggccttgcgcagcattggcgaacgcctgctggacgccatgcggcgcggcttgtggcaagaggccggcgaccaccgcgaacgtatcgaacaccaccttctggcgctggagcgccggctcgaggaccacggcgaagggccgctctgatgacaccccattccaccgaagcgatcgccggcccgaagctcgagcccgccggccgcacgaccttccccttcagtgcgctgatcggtcaacccatgttgcaacgcgcgctgctgctcgcggccatcgaccccggtatcggcggcgtgctcatcagcggaccgcgcggcaccgcgaagtcgaccgcggcgcgggccttggccgcgttgctgccgcctacgcccgcttcatcggctgcgcccttcgtcaccttgccgctgtccgccaccgtcgagcagctggtgggaacgctggacgtcgaggacgtgctgcgcgatgggcggctgcgcctggcaccgggcctcttgacgcgcgcccaccatggcgtgctgtacgtcgatgaagtcaacctgctgcccgacgcgctggtcgacgcgttgctcgatgtcgccgccagcggcgtgaacaccgtcgagcgcgacggcatttcgcaacagcacgccgcacgcttcgtgctggtcggaaccatgaatcccgaggaaggcgaactgcgcccccagttgctggatcgtttcggcctgtcggtggcgctggccaacccgagcgaggccgcgcagcggatggcgatcgtgcgcgcgcgtttgcgcttcgacgaagacccgcttggggtggccgaagcacatgccggtgaacaggcccgcctggctgcggcggtcgttgcagccagcgccgggctggcgcgcctggcgtggtcggatgccgtgctgcagcgcgctgcggaatgcgcgctcgcggctggcgtggacggcatgcgggccgaccttgtgatgctgagagcggcgcgtgcgctcgctgcattcgagggccgcaccgaagtcacgacggacgatgtcgatgcggtggcggaactggcattggcccatcgacgggaggagggcaggagcagcccggcgccggagccgaaagccgacatgcggcaggcggcgccgacatccaccggcagttccgcaccctccgccaacagttcccccatgggcgactggggtgcgctgccgccgattcccgaagccactgcccgcgtgctgcccgaaggagggtggcccgcaaaaaaagcgtgagccaccgcagccgcctcatgcgcgccgggcgcggaggtctgcggtggctgaatccagctcggcagccattgctggcgccgcctgcacatccggatgccgggccttcgcgggcttccatcgcatggttgcccaccctgctggccaagggcccgcagcctttgcaaggcgggcatctgcgctacacccagcgctcggtgcaaccggcgcgtctgcacctgatcgtgctcgacacctccggctcgatgcgccagcgcgggcgactggcactggccaaggggcacgccacttggctgatcgagcaggcagcgcgcgccggcgacagtgtggccatgctgagctttggcggtcagggcgtcgagctgcggctgccgcccggtcgggcgcgcgcgtcttgcagggaaaaggttcgggcgctgggcggtggcgggggcacgccgctggcgcatgctttggcacaggccgacaaggtgctgcgccgcgccgagcgtcgcgacggcccggccgaatcctggctctggctgctgaccgatggccggacgctggagcagccggcggcacccgaggccccgcggcatgtcgtcatcatcgatttcgacgaagccgcgcgcgccatcggccgctgcgccgactgggcgcagcgctggggcgcggaacatcgcctcgccagccgacccgagtgaccccacgaataaagtagaaccatgtcccacgcagctcacccagcgcccaccgcgctgctcgccgattggctgcgccctgccgccaagggcaggtgccccggcgcgcatcgcgccatggcttccggcgatggcctgctggtgcgggtgcggccgcagctggcgcgcttgacggtcgcgcaggccctggggttgtgcgagctggcctctcgcctgggctcggggctcatcgacctgacccatcgtgccaacctgcagttgcgtggcgtgacgcccgacgcccacggcgcggtgatcgatgcactctgcgccctgggcctggccgatgcggacgccacgcgggaagcctggccgctggtcctcgtggcgccttgctggcaggcgggcgatgacaccgaaggcatcgccacggaattgttgtcgcgcctgaacgaactgcccgcgctgccgcccaagttcgggttcgcagtggatgcggggccggcgccggtcctggctgcggccccggccgacgtgcgcatcgagcgggcccgctcgggtggcctgctggtgcgtgccgacggcgccgcggccggacatcccgtgtcccgtgccggggcggtggatgcggcgcttgcgatggccgactggtttgcggcgacggccaagggggtcgaaccggcatcgcggcgaatgcgtcgccatcaacagatcttcagctgggccgacggcccgcagccgctcgaacccgcggccgcctcggcctcgctgcccacacccggcatgtcctcgctcggatcggtctacggcgtgcccttcggacagatcgaggctgcggccctcgccacgctgttgcgcgacagcggcgccgtggcgctgcgcctgacgccgcatcgcgccctggtcctggaaggggggcggtggtgcgatgcgagggctttcatcaccgtggccggcgatcccttgctgcgcgtcgatgcctgccccggcgcgccttcgtgtgcctcggcaacggtggcgacccatgcggtcgcccgcgcacttgcttcggggctggctgcggcgggcaccgatgcaccccgcagcctgcacgtgtccggctgcgccaagggttgcgcacgtgcgcgcccggccgatgccactttggtgggccgcaacggcgccttcgatctcgtgcgcagcggatgcgcctgggatgcgcccgtgcaaacccgactgtcccctgaagccttgtgctcactcatcggaatgccctgatgcacgtctttgaaaccgatggcgcggaaatctaccgtcgctctttcgccatgatccgggccgaggccgatctctcgcgcttcgatgccgacgacgagcccgtcgcggtgcgcatgatccacgcggccggcctgatcgggctggaagcgcagttgcgcttccagcccggcttcacccgcgcggcgcgggcggcgctggcggccggcgcacccatcctgtgcgatgcacgcatggtcagcgaaggcgtgacccgctcgcgcatgccgggcggcaacgaggtggtgtgcaccttgcacgaccccaaggtgcccggtctggccgcggccatgtcgaccacccggtctgccgccgcgctggaactgtggcgacctcggctgcagggcgccgtggtggccatcggcaatgcaccgacggccctgttccatctgctgaacatgctgcaggacccggcctgcccgcggccggcggcgatcatcggttgtccggtcggcttcgtcggcgcggcggaatcgaaagacgcgctgtgggccgaacagcccgcgccctgctgcatcgtggccggccgcctgggcggcagtgccatcaccgtggcggcgatcaacgcgctggggagtcgtctggaatgaacccgcgcggcaccctgtacggactgggcctgggccccggggatccggacctgatgaccgtgcgcgcgcaccgcctgttgcagcgcgcgacccatgtcgcctactttcgcaaggccggccggcccgggcaggcgcgccgcatcgtggacgatctgctgcccgaagcggtgacggaacacgcgatggaataccccgtcaccaccgagatcccggtggacgatccggcctacaaccaactgctgtccgccttctatgccgagtgcgcgtcgcggctgcgggcgctgtcggacgccggccacgacgtggtcgtgctgtgcgagggcgatccgttcttctatggctcgttcatgcacctctacacccggctgatcgagacccacccggtgcaggtggtgccggcgatcaccggcatgtcgggtgcatggacggccactggccagcccatcacctggggcgacgacgtgttgaccgtgctcatgggcacgctgcccgaagcgcggctcgcgcgccacatggccgacagcgaggcgctggtcgtgatgaagatcggtcgccacatcgacaaggtgcgccgtgcattgacgacggcgggtcggctgcaagacgcctggctggtcgagttcgccaccatgccgggtcagaaggtgatgcggcttgcggaggccgaaggccgcgtcacgccctatttttcgatcgtgctggtgcatgggcaaggacggcggccatgagcgccgcccggccgcccgaaggcgctcgcaccgcagtgcgcagcacggaggtcgcctgatgagcgtgccgacgcatgccgcgggctggctggtcatcgccgggctgggccctggcgccgatggctgcgtgacacccgaggtgagcgcggccctggccgatgccaccgacgtggttggctacatcccctacgtggcccgggtggcgccgcgcgccggactcaggctgcacgcgagcgacaaccgcgtcgagctggaacgcgccgcccacgcgctgcgcctggccgccgaaggccggcgcgtggtggtggtgtcgtcgggcgacccgggtgtgttcgcgatggcctccgcggtgttcgaggcggtagaggcgggcgatgctgcatggcgcctgctggacgtgcgcgtgttgcccgggatcaccgcgatgctggctgccgccgcgcgcgccggcgcgccgctgggccacgacttctgcgccatcaacctgtcggacaacctgaagccatgggcgctggtggaacgccgtctgcggctggcggtgcagggcgatttcgcgatggccttctacaacccgcgctccgtgtctcgcccgagcggcttcgcccgaacgctggacgtccttcgcgaggcctgcgcagcggcgggaagcccggcgcgtccggtgatcttcgcccgtgccgtgtccacgcccgacgagaccatccgcgtggtcgcacttggagatgcacagcccgaaatggccgacatgcgtaccgtcgtcatcgtcggctccagtctgacgcgggtcattgcccgcgagggccgaccctgggtctacacgccgcgctcggcgccgcgcgaggtgggcgcatgatgcgctgcctccagccacagcagcacctcggccacgcgcgtcgcttcctgccgcgcgggcagcggtggccgcgccaccatcacgatcggcagctcgagctcgcgggccgcgtgcagcttggcctccgcaccggtgccgccggcgttcttgcagaccaggacgtccacgcgctgcgcgcgcagcagggcgatgtcgccttccaggtcgaagggcccgcgcgagacgatgaccgtgtgttgcggcaagggcggccgcagctcgggcaggtcgaccagccgcaggatgtagtggtgctgcggctgtgccgcgaaggcagacaggtgcatgcggcccaaggccagcatcacgcgccgcggtggtccgctcagcgcggcgacagccgcgggcaggtcgggcacgggctgccagcggtcgccaggacctgcctgccagccggggcgagtcaaggccagcaagggcaggccgcactccgcgcaagccgccaccgcgttcgcgctcatgcgcgcggcgaagggatgggtggcgtccacgacgtgcgtcacccgctcttcgcgcaggtggcgcaccaggccgttcacgccgccgaagccgcccacgcgcacggcgatgggctgcgccttgggctgggccacccggccggcataggacagcacggcgcgttcgcccctttcggcgagcgcccgcgccagcgcgctcgcttcgagcgtgccgcccaggaccaggacattgcgcatggctgaattcacttctgaagttaccccgtggttgacgatcatcgggctcggcgaagacgggtgggagggcctgccttccgccagccgcgcggcactcgatgcggccgatctggtggccggcagcgcccggcatctggcgttgttgccccatctccgcgccgagcggctcgaatggccggtgccgtttgccgatggcatcccgatcctactggcacagcgcggtcgccgcgtggcgatgctggcctcgggcgacccgttctggttcggcgcgggcagctcggtgacgcgccatctcggcgcgcacgaatggcatgccttgcccgctgcatcgaccttcggcctggcggctgcgcgcctgggttggccgctggagcacttgacctgcctgggcttgcacgcggcgccgctggcgcgtctgcgaccgcacctgcacacgggcgagcggctgctgctgctgctgcgcgacggtgccgcagtgacggcgctcgcgcgctacctcgtcgacaacgatttcggcgccagcgcgatgagcgtgctcgaagcactgggcggcccgcacgagcggcggcgcgacgtcgctgcgtgcgccttcgacctggccgatgtgcggcatccggtggccgtggccttgcagttggccggaacgggcatggccatgccgtgcagcacaggcctgccggacgacgcatttgcgcacgacggccagctcacgaagcagaaggtgcgtgccctggcgctgtgcgccctggcaccgcggcccggcgagcggctgtgggacatcggtgcgggctccgggtcgatcggcatcgaatggctgctggcgcatccgaggtgcgaggccgtcgccatcgagggcgaccccgaacgcgcgatgcggctgcgtgccaacgcggaccggctgggcgtcgatcggctcgttttggtgacaggcagcgcacccgaagccttggccggcctgccgccgccggatgcggtcttcatcggcggcggcctcagcgatgcaatgctggcgcatctgtggcgcttgcttccgcaaggctgccgcgtggtggcccatgcagtgacgctggaatccgaagcgctgctgagcgactggcacgcgcgcgccggcggcagcctgacacgcatcgagctggcggaggccgcgccattgggaacgcggcgcgcctggcgcgcttcctacccaatcgtgcaatggagtgcgacgcgatgatggtggcgggtttcggcttcagaagcggcgcgacgctggcatcgctgcgcgacgcgttggcgcacgcggccgcggccttgcaacccacggtgccggtgcagtcggttgcctggctcgccgctgcgcaagacaaggccgacgcaccgtgcctgcgtgcgctggccgaggcgctgggcgtgccggtgtgcgccgtggaggctgcgcgcatgaacgccaccgtcaccctgaccgaccacgcccgggtgcgtgtgctgcgcggcagcggcagcaccgccgaagccgcggccctggcggcagccctgatgcacgtcggtccgggtgcaacgttgcttcatccacgcgtggtgtcgaccgaccgccttgccacctgcgcgatcgccgcgcgaacccaacaaccggagtttcgaccatgaccatccacttcataggcgccggtcccggtgcgccagacctgttgaccctgcgcgggcgcgacctgatcggccgctgccctgtctgcctctatgccggctcgctggtgcccgaagaaattctggcgcactgtccacccggcgcgcgtatcgtcaacaccgcgccgctcgatctcgacgccatcgaggccgaattcgtcgccgcccatgcggcagggcaggacgtggcgcggctgcattcgggcgatctgtccgtgtggtcggccatgggcgagcaattgcgccgtctgcgggccgtcggcatcccctacacggtcacgcccggcgtgccctcgttcgccgccgcggcggccgcgctgggtgccgagctcacgctgccgggcctggcgcagtcggtggtgctgacgcgcacatccggccgcgcgtcgcccatgccctcgtgcgagaccttggcgggcttcgccgccaccggagccacgctcgccttgcacctgtccatccacaagctggccgaggtggttgcagagctggtgccgttctacggcgccgaatgtccggttgccgtggtctatcgtgcaagttggccggacgagcagatcttccgcgcgaccttggccaccatcgaggcgacgatgggcgagggcgtggaacgcaccgcgctgatactcgtcggccccgcactggccgcagaaggcttcgccgaaagccgcctctatgccggcgactacgatcgaaggttccggccgacacgcgccgaaccgggcaatccgccaagcacctgacatcgcatttctcgtttcctcccatcaaccccctcgcagctccgcgcagcggactgcactcaccctacggagccccgccatgcacatggaacccggaatcgtcgacggcagcaagatcgtgctgtcctatgccacggcgagcgcctgcgcgctctatgcagtgaagctgtccctgaaccacattcgcgaggagggagtgggctcgctgctgctgcgcagcgtgctcgccgccatgctggtcttcgtcttcttcgaggtgttcccgcacgcgccggtcggtgtgtccgaggttcacctgatcctgggctcgtcgctgttcctgattctgggcgcagcgcccaccgccatcggcctggccgcggggctggcgctgcagagcctcttcttcgagccgcaagacctgccgcagtacggcatgaacgtcaccaccttgctggccgcgctgttcgccctgcaggcggtggccaagcgggtgctgccggccaagcttccctatgtcgagctgggctacgtgcatgtgctcaagatgtcggtggtgttccagggagggatcgtcacctgggtggctttctggacgatctacggccgcggcttcggggcggagacgctgcaagccgtgggcagcttcggcgccgcctacatgacggtcgtgctgctggagccgctggtcgacctggccgtgctggcagcagccaaggggctgcgcgggcgggcagggcagggtgggtcggtgctgctgacgcggcgtctgcaccacgcagcctgaccacgagttggccgattgccgcgcaggcccgctgatggatgccgtttccgtttccacgatcgaactgatgctgattggcatcggcaccggcaatcccgagcatctcacgctccaggccatcggtgcactgaaccgcgccgacctcatcctgattccgcgcaagggcgccgacaaggccgagctcgccgacttgcgccgcaagatctgcgcaacgcatctgaacggccaggcccgactggtcgagttcgatctgcctgtgcgcgacatcgccgcgcccagctatcttgacggcgtgcacgagtggcacgccgccatcgccgccgtgtgggcggagcagatcgccacatgcctgcctcatggcggtcgcgtggcactgctggtctggggagacccctccctctacgactccagcatgcgcattgccgaacggttgcaaacggctggcatggcgctgcgggtcgaggtgattcccggcctgagcagtattcagttgttgaccgccgcacacgccatcccgctcaacaccctgggggccccggtgctgatcaccaccggacgtcagttgagggccggcggctggccggcaggcctggacacggtcgtggtcctgctcgacggtgccggcgcttttcaggttctacccccggagggcattgagatctattgggcagcgtatctggggatgccgcaccaattgcttcttgccggccctctggccagcacgggaccacgcatctctgcgcttcgcgcagcagcccgcgaggagcacggctggatcatggacagctaccttcttcgacggaactccgcaaccgtcacctacgaagacgatttgatatgacttgcgaattcgagcagcgacttccgctgtttggtgtttagctgaccgaaccacaggatgagtttggcgagctcgtcatccggtgcgtaaaagtatcttagtcgaacatctttcgccgctctagtcgttcatgctgcaggcgcaggggcaatgggtggcattggcagtgcacccacgccccatcaaatcccccgggtccgaatcttcatgctcgaccgacgcagcgcaaacacgccgtcgaaggtccggcaccacacgatatcctgagagcttgcgatgaggcgtgcaggcatcggatacccgccgcccggtgtcagcagttccgtcgagaagacgaactcccgctcgggcggggccttcgcggacgcgtccttcctgccggcttcctccctggcgatgaaggccgcgagttcgccgaagccctgcgcggcctccgaagcgagcttgcgctgaaggtcctccgagggccgggccagttcgtcgaggctgtagatcgagggcaactggtacatgtacaggcccgaccaccgatcggccccgctgccctgttcgagctggactgccgcagccgccaccagcctgccgttgggcgacttgctgatggagagatagggcgttgcgcccgtgcgcactgcgccgccaacatcggcgagctcgagcccctgccggatcgccgcatcgaggaacaactgccgcggctcgagcctgagcttgcccttcatgcgggccgcatcgaggccggtctggctgtcgaccatgcccatgttggcgagcgcgcccagggcaccgaacaccaggccggccgtcagactgccgccctgtgtctgcgtgtagacgatggtcttcgcgtcgtcgaggtggcgagtggcgtgccgcggctcctccacgatcgccgcatgcgcgagcacgaacatcgacggtgcgtccgccgcgacgggacgattcctgtagctcggcggcgccacgcaagccgtcaggccggctagcgccagcagcgcgcacactcccaccgcgcgacgatgcgcgcgggcctcgaaaccgatcatggctttttctcctcactccgtggtccgacaagccgctcttcggcggcgggcggatcatagccgccggaccgtacgcaaccgttgccggtcggttcgcagacggccagtcgcatggacgccttcggcttcggtggcccgacgccggtgatgaatcagcgcgagcggcttgattgctcgaaaaggtggccgaccgattggaaagaaggttcgacgccgcccgcgtgactagcgcgcaagttccgcgtcgaaaaggggacggtgctgcgcgccgtgtgtgggggcgctcgactcggtgctgtgccgcctgggtcgaggcgagagggggagggaggggatgcggtgagccgcgttcggtgcgctaggctgaaggcgcgggcaggcggtccttcagtgcttgaacccggactcgcgctgggctcgcagtgccaggatgaagacggtctcgatcccagccaggtaacggtacagcgccacatagccgcggttgcccttgccgatgatcagctcgcgctttccgcctgcgacggggcggccgatcagcgggctgcgcgaaaggatctgaatggcctcgagaatctccccgacccggctcgccacatcggcgacctggtgttgttccagatggtcgatgaagcggtcgatgtcatccagaacctccggtgccagctcgatgcggaccatggcccggtcagggcgccggcctgcgcgccataggccggcgcggtttctggccggccgcgcgtgccttcaagtaagccgcagcgtcctcccaggcgaccgattcgccggtgcgctgcagcgccgcccaccgcttgtctgcgatccgatgcaattcctcgtccaattcgctgcgctcgaccatgtcggacagcgcgtccagaatgaacgcgtgcgaagacctgcccgacctcgcagccgcagccgcgatgcgggccttgagctcatcttcaagacggatggtcgttgtcggcatgttgatggacctcatgacgttgacggtgtgcaagtgtagcacacttgtagcacatcgggtcttgcagctcgcatgtctttagtgcccatactcgaaacaggacagaaagtttcgaattgctgtcaaattgcggtatggagccctgctgcgccgcaggttcgcaggtgccgattcggagcttcgggtatgaaacgcaggtctaaaagcgagacggcggcatgggctccgaggcttttcgcggccgaacctgttccgcatgcggcagttctacgagacctatgtcgacgcgggcgagaaagtctcggcactgctgagacaaatcccctggtcttgcccgcgccggggtccagcctcggctctcgaactaagggactgagggccgcaaccgatccgttgggcccccgccgcactgcgcagaacgcagcacagctcaatgcggctgattcgtatcgcctgctgaatcccggtcagggtcctccagcaccgggagcagaggggccactatttcaccaatgtgttgagcgttcctggcgccgatttcgcgcatctccggtgagagccgcgggtccgctgcggcggctgtccagaagcggtgtgccgcttcgaacgcctgctcccagacctcaggcctggcccccagcgactgaaacgatggcgtgacgagccgcaagggcggctcgatgccgcctccgacgggcgcgtacatcatggggagcatgtcgtaggccggcgatacctcggtaggtcgccctcgctcgtcggtcatgagcgagagattctcaaagtgtcgatcgccattgccgatcagctctgagaaggcggtcagcacgaggatccgccgcacggagtcaggcccgatcattcctgcttcctcgcagcgctgcgcgaacgatggccagttgtcccgcatcctgaacagctcgtcatcgatcgcccctgcggagatcattccccggcggccgaaccgcccgactcggtcgaagcgctcgacctcgaggaagccgtactcctccatctcgaagtagcgagccggagccgctggcatcccggactcgccgagggcgcgcaacgccaagtcctccaggagaagcatttccgaggagcgggtcccgacgcgtgcaaacttcacaatgagatgcccattcgcctctgtctcgcacgtgaacttgggctgttcgccgcccgcgctgctgccggcgcccgtctggctcgtcgcgttcgccaaatcctgataggcccgaggaatgtcggcggtcgtgatcggcgggacctgccgcgacgccatgtgggccgcgaacgaactggcgccccacatgagcgccccagccacatccgacccgaccgagcagaggaacttcacccggtgatcgtcggaccagtcgcgaagggaggagggcaccccaatttctgtggccacgaccttcgcgatccgtgcgccgaggtagccggacggcgccgcgaatgccatggccggcggcagcccttcgtgcaagcggctgtctggcccgccaagatcgacccaggtgccacctcggagaaagttgacggcgccaatctctgtgacccgaccatcctcgctcacccggaagatgggctgaggggtgggcacgggttcggtgcggacgagtgcgtagcggggcgtgcgcacgccaggttcccggaatcgaagaacttcggcaccgaattcgtgaatggtccgagagaaggttgcttgactgacttgaaggagcgcaagcagctcgccaacaggcctcggtccctgggaaagagcgtgacggacgagcgtctttctgtctgcctcgcgggctcccgatgatcgggttgcggcgctcattgaatcattgaatgaatagttcggtgaacgacaagtctactacatcgcgacagcgtcggcgcatatggcccatgccgttcggtcacgacgccagcgcctctgctaccttcggactttttgagcgagttcgaatgtcgatgacacttcgcgatacccccgccgaaaaacggcaaatctaccgcgacgccttggccgcagagcaggcccgctcattggctgcgaccgacaattggtgccgacatgaaggccttccaccaggcctatcaccctcgcatggtcgaactgcttggcgaggcgatggccctgtacgcgcagcagctgccgcctggccgatcggaacgaagctacaagagccatctccagccacgctgcgccgctgcgtggatcgcaaagctcgctgcccctgtctcgactgcgactgcctggtgtcctcatgatttgccaggaaagaaacttctgctccaaaataacttaccgtgcgacaggtaatatcttattgaatttcaaggagacatgatggctttcaacacgttgcagctagtggtcaaggatcggatcgcggtggtcacgctcgatcgtcctcccgtcaatgcccagaacgccgaactgcgcagcgaactgactcaggcgttcgacgagctttccgaccgcgaggacgtgtcggtggtcgtcctcaccggcagcggcaagaccttttcggcgggtgccgacatccgcgagcgccccaatctcggcgcgacgccgggcgcctacggccgccacaaccggttggtgcgcgagtcctactatgcggtcgtcgagtgcgccaagcccgtcatcgccgcgatcaacggtccggcgatgggtgcgggtttcggcctagtcatggcttccgacatctgggttgcctcggaggacgcgttcgtctcgatgcccgagatcaacgtcggccttgccggcggcgtgacctttctgcaagaggtgttcgggcgctcgcgcgcacggcgcatgttctacacgggcatgaaggtcactggccaggagttgtaccgactcggcctcgtggaagcctgtctgccggccgacaagctcatgccctatgcgatggaaattgccgcagagatcgcctccaagagcccgatcgcgctgcgcctggccaaggaagctgcgcgcatgacacaggtgatgccttcgcgcgatgcctaccgctacgagcagggcaacacggtggcgctgtcaaaaacggaagacgcgaaggaagcgcagcgcgcctttctcgagaagcgcgcgccggtctacaccggacgctgacggcaggcggtgcccggccgtgcgccacgcatgtgcgtgctattatttttgatcccgcgggttcgcgcacctgcgtatccaggcgctcccgcgggcttccacgccagaacttcaagaggaccttcgccccatggccaccctgtccaacgtcgccgaggcgaccgatccggaacggggctctaggcgcaagtccgacgtgcgccaagagcagttgaccgagatcgcctgccggctgttcgccaagaagggctacgaaggcacttcgctgcgcgacattgccgacgaagccaagatcaccaaggctgcgctctactaccacttccccaacaaggaagcgttgtacgaacgcatcgtgctcgagtcgatgcagacgctggtggactcggtgcgcgaggcgatgtcccgcggcacgagcccgctggacaaggtgcgcctgttcatggagtcgtcggccgacttcctggaccgcaaccgcaattcgtggatcgcgggctccaacgccttctggtccggcagcgagggcgatccgcgcgcgggcgccgtctatctgcgcgacgagtacgaacacctcctgcgtgattgcatcgccgaggccatcgccaagggtgaggttcgcaaggtcgaccctgccattgccgggcgcatgctgctgtcgatgctcaaccacatctgccgctggcattcgcccaaggggcggctgagcacgcgcgaggtgatcgagcagtacctcgacatggccttcggcggcctgcgcgcgacaccgcgcacctgatcttccggacacggtggcgcgaatgcgcgccgcattgcccgagagggtaaacccggttattaacttaccggccgttaagtaaactttgctcgagattcaacgatgcaagcccttcaacgattccttctttcggtgtgctccggcgtactggccgcggcaccggttctggccctggcgtttcctgacaagccagtgcagctgatcgttccgtacgcggctggcggactgaccgacaacctggcacgcgtcattgcgccagcgctgtccgcacgctggggacagccggtggtgatcgacaaccgaaacgggggagggacctcgatcggcaccgccgcagccgcacgtgcgcccggcgacggctacacgctgctgctcaccgccttcggctacatcggcaatccgctgctgatgaagaacctgccctacgaccctgccgcgctggtgcccgtcaccatcgtggcagatgcgcccagcgtgctgttcgtgtcggccaagctgcccgtcgataccgtgcccgagttgatcgcctatgccaaggcgcatccgaagcaggtggtgttcgcatcttcgggcaacggatcgagcccgcacatcgctgcggaattgctggcttcgctggcgggcatcgacatcgtgcatgtgccttaccgcggcaacgggcccgcgctgaacgatctgctgggcggccaggtgcaggcgatgttcgattcccctgcatccatgtcccatgtgcgcgccggccggctcaaggcccttggcgtggccagcgacgcacccgtggcgcgcttgcccgggctggtgcccatcgcgcgctcgggcgtgccgcaactcgcgggcttcgccgcaggcggctggttcggtcttttcctgccgagcaagacgccggccgaactgcagcaacgcatttatgccgacctgcgcgctgtgctggagacccccgagatacgcgcggccatcgagcgcgccggcgtggagccgcgcctcatgacccagcccgagtttgcagcctacctgcgcgccgagcacgaccgctgggcgccagtgatccgcgagcgccgcattcagctcgactgaggaagacccgatgtccagcagctttcattgagacccgacaagacacatgacaagtccaacatcgaccgatccctacgccgctttccgcgaggaactgcgccagttcgccgccgagcagtgcccggaagacctcaagcgcttcgtgcgcagcaatcgcaagatcacgcgcaacgagtaccgcatctggcaggagaagctcttcgcccgcggctgggccgcgcccaactggccggtggcccacggtggcacgggctgggacctgcagcagcgctacctgttcgaggagatcaccgcgcaggccgattgcccgccgcagtaccaccacggcctgggccacatcggcccggtgatcctgcacttcggcaccgaggcgcagaaggcgcgcttcctgccacgcatcctcgacggcagcgagtggtggtgccaaggctactcagaacccggtgccggttccgacctggcttcgctcaagacatccgcacggcgcgatggcgatcactacgtgctcaacggccagaagatctggacctcgcacgcgcaggaggccgacatgatgtacacgctggtgcgcacctcgagcgaagggcgcaagcaggccggcatctcgctgctgctggtgccaatgaacgcgcccggcatcgaggtgcgcccgattcccaccatcgaccactggcaccacgtcaacgaggtgttcctcaacgacgtgcgcgtgccgtgcgaaaacctggtcggcgccgaaggcgagggctggaaatgcgccaagttcctgctcgaccgcgaacgcctctcgcccgcgaccgtgccgcgcctggcccggctcgccgagcaggtcgaggagctcttgatggctcggcgcggcgccaatcccgccgcggccgcctcgcccagcttccatgtgctgctggaacgcctctacctggcccaggccggcgtgaagggcgcgcgcgagatgctgctgagcgccatccaggaggagatgcagggcacgctggcggcgtccaagtcgtcggcgctcaagctcttctgctccgacctgtcgcagcagatcatcggcattgcactcgacattgcgggcccggcgtacgcggcgcggctggtggcgtccaccggtgtcgatgccgagcaggacgtcgacctgcagcgcgagctcgtgcacacctatcttttctaccgctcgcgcaccattgccggcggcaccagcgaagttcaaaagaacgtcatcgcgcgcgacctgttcggagcttgatccatgccattccatgctgagccgatgttccccggcgacctctacgacacgaccttgcgcgtcgcttcttccgcagccgccacggccggtgccgacgccgatgcccgcgcggcgggtgcggcctggcgccagttcctggacctgggctggcaagccgtgctggtggccgaggccaggggcggcgccggtgcctcgctgggcgacatcgcggccatcgccgaggcggccggccgccatgcgctggccgcaccgctggtcgaacgctgcgccgtggcgccgaccttgctgtcgcgcatcgccggcaaccccgccgccgatgcgctgctgggcgagattgcaagcggcgaggcctcggtctgtccggtgctggcactcgacgagcccgcacctacggcgcgcctggagggcgggcgcgtggtgttcgacggctgcctgcgcggcgccgacctgaccgagccggtgacgcacctgctcgtgctggccgcgctggatggcaaggacgcgctggtcctgctgccgcgcgccgcgctggccgagctggccgcctccgcgcgcggctacatgggcatcgatgcacgccacaccgcggacatcgacgtcgcggggctcgcactgcccgaagccgccgtgctgctgcacggcgacatggttcgcccgctggtggggcatgccaatgcggtgggtgcgttgctgtcgtgcgcgcagatggtcggtgccatcggcgccatgatcgagcagaccatcgagtacctgagcatgcgcgagcagttcggcgtggcgctcgccaccttccaggccttgcgccacaaggtggtggagatgtacgtggcctacgagaacgtgcgcggcatggtgcgccagcaggtgcaggtgctggacggcttgcgcggggcgctgccggggcgcgaggcgcgccgcgaactcgcactcgtgaagctgtacctggccgtcaccggccgccaggtcgcggagacggccatccagctgcacggcggcatcggcatgtcgcgcgaactgcctgcggcgcgcctggccatgcatgccctcgcctgcagccagcagtggggcgatcgtttcagccagctcgatcggctcgccgccgatgccgcgctgcattgaggagcctgtgatgcattcgcttgattcgctttttcatccttcgtcggtggcgttgatcggcgcctcgtccgatcccgagcgcatcggcggacggccactgcgcttcatgctcgaaggcggcttcgaggcgccgctctatccggtcaacaggagcggcgacaccatccagggcctgcccgccttcgccagcgtgctggacattccgcatccggtcgaccaggccgtcatcgccgtgccggtggccggcgtggaagcggcggtgcgcgacagcattcgcaagggcgtgaaggcgatccaggtgctgaccgccggctttgccgagatcgacgacgccggccgggcgctgcaggaccgcctggtgcagatgtgccgcgatgccggcgtgcgcatggtagggcccaactcgctgggtctgctcaacgtgcccacgcgcttcttctcgaccttctccaccgcgctgaatggcctgaagcccaaggccgggcccatcgcgctcgccacgcaaagcggcgccttcggctccgccgcctatggcatggcatcgctgcgcgggctgggcttcagcaagatcatcgcgaccggcaacgaaggcgacgtcgacgtggcggagtgcatcgactatctcgtggacgatgccggcacgcgcgtcatctgcgccgcgctggaatcctgccgcgacggcgagcgcctgcggcgcgcgttgctgaaggccgccgccgccggcaagcccgtgctcatcatgaaagtggggcgcaccgaggtcggcgccgccgcagcctcgacgcacacaggctcgctggccggcaacgacgcggtctacgacaccgtctttgcggagtgcggcgcctggcggcccgaatcgcttgaggagatgctcgacatcgcctacgtgttctcggtcgcgaacgcgctgccgcacaacgccggcatgggcatcgtcaccggctccggcggcatcggcgtgctgatggccgacgacggcggtgggcgcggcatgtcgctgccgccgctacccgaggctgcgcgccgtgcggtgctcgagctgctgccgttcgcggtggcgagcaatccgctggacatgacggcgcaggtcacatcggttgccagcggcgtgtcgcgcaccgtgggcatcatgttggaccacacggactatggcaccgtgttcgcctacctggcgcacgtgggcctgtcccccgagcgcttcgcctcgacgcaggccgaactgatcgcgcagcgccagcggcatccggaccggctcatggtgctggtgatgctgtcgaagcccgaggtcaaccaggcgctcgaacagcacggcattccggtcttcgaggacccctcgcgcgcggtgcgtgcgctggccgcgctggcgcacatccgcgcgcgccggctggccctctacacgccggtgcagcgagtgcccgccgcgtcgctgcgcggagacgtttcgaccgaggacggcgccaagcgcgcgctggcgcaagccggcctgcccgtgccgccggagcgcctgtgccgcagcgccggcgaagccgcggctgccgcgcgggccctgggcttcccggtggtcgccaagatcgtctcgcccgacatcccccacaagaccgaggtcggcggcgtcatgctcggcctgcaggacgcagcggcggtcgaggcggcgtacgcagcgctgatggcgcgcgccggcaaggcgcggcccgacgcgcgcctggagggcgtgctgatcgcgccgatgctgcagggcggtgtcgaggtcatcctgggcatccaccgcgacccgacgttcgggccgatggtgatgtacggctcgggcggcacggccgtcgagctgttcaaggacgtggccttcgcttccgcgccgctgacgccggcgcgcgccgccggactgatcgagcgcgttcgctcgacgcaactgctgcgcggctggcgcggcgggccgcgctacgacgaggctgcgctgatcgatgcactgtgccgcctgtccgacttcggcatggcgcatgcgcacgagctggaaagcgtcgacatcaatccgttcgtggtgcgcgccgaaggcgccgcatgcctcgacgcggtgatcgtgctgcgtgaaacggaaacgaaggagcattcgcatgccatctgaagaacgcctggccgcgctggaggcgcaactcgaaaccttgaccgcgcgcgaggccatccgtacatgcctctaccgctattgccgcggcatcgaccgctgcgacgaggcagcgctgcgctcgtcctactggcccgatgccaccgaccgccacggcccctacagcggcagcgccaacggcttcatcgactgggcactggccaagctcaaggagagcggccgggtgatccacatgatcggcaacatctcgatcgagctgcgcggtgccgaggcggcagtggagagttacttccaggctttccaggtcgacgcagacgcgcaaggcaaggagcgcgagacatttctcgtcggccgctacatcgaccgcttcgagcggcgcggcgcgggcgaatggcgtgtggccgcccgcaccgtggcgtacgactggatccgcgagtcggcggcgccggtcggcaccgaagccgagcgcttcggcgtgcgccagccgaacggcggccgctttcccgacgacccctggtacgcgctgacggcatcgctgccgtagccggcgcctcaccgctgcgcacccgcccgaagagacaagagtccctcgctttttttcctgattgccgcccctggccttgccggagggtggctttctgcgtgccggcctgcaggcgagtcctgaaggcggccgggctcccttcaacgggcccgcgctcaaaaaatcccctacgaggagacaaatcttgccgagattcttcaagccattcgcagccgccactgcaattctttgcggcacaccgttcgcattcgcccaacaggcgcagaaagaggagttgagacagatcgtgctgcccgccggaggcatggcggcgtcgccgtcgagcctgacggtctatgggctgatcgacaccagcctggcatatgccaccaatgccggggggcgcgtgaagcgcctggacagcggccacatgaacggttcgcgccttggcttcaagggcagcgaagacctgggcgacgggctgcgcgccaacttcctgctggagatggggctcaactccgacgcgggcacgctggggcagaaccagggggcgggcgccaagtcgttcggccgcggatcgattgtcggcctgtcgggctcgatgggcgagatccgcctggggcgcaccgtggtggccatcggctccgaggtccaggcggtgggcgacgcattcgggcttggcggtggcggcaatcttcaagggatccagcccgcgccgggacgggtcaacaacaccatctggtaccagtcaccgaacctgggtggcttcatcaccaagctgtcttactcgcccggtgaaaccacggtcaccagcggcacggcagcacgctccaaggccggcgcgagcaccgccgcttccgtgttctacgtggggcatggggtgagtgccgccatcggctattcgacctacaagcaactggccgatgccagcaccttgcgctggttccactccgcggccgcttacgacttcggcgtggccaagctgttcggctcgtacgcgacctttcgcaatccgggcatcgcaaccacaccggccacccacgcggcagcggacaacaacatcatgttcgcgggcttcccgctggtgggctactacagcgggcagaaagaccgcagcgcgtcgatcggggtggcggtgcctttcggtttgagcaccgtgcttgcgcaggtggtgcgcgtcgacgacaaggggccgctgaaccgggacgcgacgcagttcggcattgcctacatctatgcgctgtccaagcgcaccagtctgtacgccgaccatggccgcgtgcgcaaccgcaacggcgcgtcctacgcagtgaccggcgccaccacgcaggcgggcctggaccgcggcggcaacagccgcgccacccacgtcggggtgcgcatggcgttctagccggcctcatggttcgcccgctagggaaaacgcatgcggggtcactaccatcgcatgcgtgatttctgaaggacatggatgcccaccggaaccgtcaaatcggccacgcgcgtgctgcaggtgctggagtattttgcgcagctgcgcacgcctctggcgctcaagcagatcagcgatgcgctgggctatccgcagtccagcacgaccgtgctgctcaagaacctcatcgctctgggctacctcaattacaaccgcgccgatcgcgtgtacttcccgacgccccgcgtggcctcgctgggcgactgggtcacgcaggcgctgttcgggcaggggcgcatcgtcgaggtgatgcgcgacctgcacagcgccaccggcgagaccgtctcgatctgcatgctcaacgatatttacgtgcagtacatccgcgtgatccagtcgacgcatccgttgcgctttcacaccgacgagggaagcatgcggccgctcacgctctcggcggtcggctggctgctgctgaccgaccgcggcgatgccgagatcgagaacctcgtgcggcgcgccaacatcgccgtaccgcgcaaggaagaccgcgtggcgctggatgtcattgcaccgcaggtggccgacgcgcgcgagcgcaagtcgctctacatggagaacatgccgctgcttggcggcgccaccatcggcgtggtgctgccttgcctggtgcaggggcgcatcgcggtgctgggcatgggcggtaccatcgagcgcatgcgcccgcaccgcgcgcgctacaccgcgttgatgcggcggctcgtccagccgctgggcgaatcccggtctgcatagcccctcgcaagccctacggaaaatcatggatgtgatcttgttcgccgcaagtgtgattttcttgatgacctggcaggtggtcggcatcatttccttgcatgaggtccgcgccgccgcggccgcaacaaacaaggagacacacacatgaccactgagcctcgcaacctgcatccatctcgccatccattgaatccgcacaccggggcccagcggctcgacgtggtcgtggtcggtgccggcttcggcggcatgtacgccgtgtatcgcttccgcgaaatgggccttcgggtccagggcttcgaggcgggaggcgatgtcggtggtgtctggtactggaatcgttacccgggcgcacgcgtcgacctgccgagcatcgactacagcttttcgttctctcccgagatcgagcaggaatggacctggtcggagcagttcgccgcgcagcccgagctgctgaggtacatcaatttcgtggccgaccggctcgacctgcgccggcacatccagttcagcacacgcgtgacccgcgcggtgtgggacgagtcgcgcaagctgtggaccgtgatcaccgatcgcggcgacacgtacgaggccacgtactgcatcatggcgaccggcccgctgtcgattcccaaggaccccgagattcccggcatcgaccgcttcaagggccagctgctgcgtgccgccaagtggccgcatgaacccgtcagctttgcaggccgccgcgtgggtgtcatcggcacgggatcgaccggcatccagatcgtccaggaagtgggcaaggaggccggcgagctcttcgtgttccagcgcacgccgagcttcaccatgccgatgcgcaacgaagcgctcgagccggcctacgtggccgaggtcaagcgccactatgccggcatccgcgagtcggcccgcaacagcgcggtgggcggtgtgcgcccgcaatccacgcgcgccttcttcagcgtgacacccagccagcgccggcagctccttgaagacgcctggaagaacggcggcctggccatgctcggcaccttcgcggacctgctgaccaacgcggaagccaacgagcaggtcgccgagttcgtgcgcggcaagatcggcgagatcgtgaacgatccgcagacagccgagaagctgaagccgcgcgggtatcccatcttcgcgcgccggccctgcctggacggcagttactacgagaccttcaaccggccgaacgtgcatctgaaggactgcacctcggaccccatcgaagagatcaccgagcgcggggtgaagacgcaggccggcgaggtcgaactcgacgcgctcatcttcgccaccggctacgacggcctgacgggcgcgctgctggccttcgacatcgtcgggcggggcgggcgcacgatgaacgacaagtggaaggacggtgcgcgctcgcacctgggcctgatgatggaaggcttccccaatctcttcatgaccaccgggccgaacggtcccgccgcgctcgccaacatcatccgcatcagcgagcatgacgtcgactggatcgcggccgccatgacgcacatggacaagaacggactgtcgaccatcgagccgacgccgcaggcagaacaggcgtggatggacatcgtcttcgcgctctcgcagcgctcgctgctcctcaaggccaagacctggtacgtcggtgccaacgtgaaggacaagccccaggggctcacgctcttcacgggcggattccagaaatacagggagcattgcgccgcggcagtgcagggcggctatcgcgacttcgtgttcgaacacgcacaggaagccctcgcagcctgacgtcatggcccgggacccgcgtgcgcgggtcggggcgtggccttacacggccagcgtgccgccgtctaccggcaaggtgacgccgttgacgaagctcgcaagccccgaggccaggaacaccgccggaccggcgagttcgtgcggctggcccaggcgcccggccggaatgcgctgcatgaagcggcccagccgcgccgggtcggcacgcgtggcttcggtcatgggggtctcgatcacgccgggtgcgagcgcattgacgcgaatgccgtccggcgcgaggtcgagcgccagcgactgcgtgagcatcttcaccgctgccttggaggccgaatagcccagtgcgccgccttgggcgatgaacgcggcacccgacgccacattgaggatgcagccgcgcgtgcgccgcaatgccggcagccatgcgtggacggtgttgaagacgccgaacaggttcacgtccatggtgcgatgaaggttctcctgcgcgcgtggactgtcgatgccttcgcggatgatcacgccggcgttgttgaccagcgtgtcgatgtcgccggcggtgtccttcaccgcttccgccagcgaaaggcaggcctgggcgtcggacacgtccagtgcgtaggcccagccttcggtgcccgccgcatgcacggcctgcagggtttcggcgcagcgatcgctgcgcaggtccgtcacgatgacacgcgcacctgcctgggcataggccaccgcgatggcgcggccgatgccgctggcggctccggtcaccagtgccagccggccggagagaagccctggcgtggccggccaggtcgaaggaaggtcatgggctgccattggcatgctcctcagggtgccgcggccgcgcggcgctgccggcgggtggcgagacaggaatggaactggccgacgatgcccttgcggaacagcatgacgaccagcacgaagacgacgccctggatgatcagcacccattcggcgaaagacgcgagatagttctccatcgacacgatgacgatggcgcccaccacagggccgagcagcgtgtgcatgccgccgacgatgcagatcagcagcgcctcgcccgaagtcgcccagtgcacgtcggtcagcgaggcgagctggaacaccagcaccttgagcgagccggccagccccgccagcccggcggacagcacgaaggccagcagcttgtagcggttgacgcggtagcccagcgactgggcgcgcggttcgttgtcgcggatggcacgcaggatctgtccgaacggcgaatgcaccacgcgatggatcagccagaagccgaagacgatcagcgccgcgacgaagtagtagagcgtcagcgtgttctgcagcgagaacagtcccagcaccatcggccgcggaatctcctggatgccgtcttcaccgcctgtgaagggcacgcgcagcgcaatgaagtacaccagctgcgcgaaggccagcgtgatcatcgagaagtagatgcccgagcggcggatggccagcaggccggtgaccagccccacgagcgccgccgcggcgatgcccgcgagaacgccggcggcgccgtcccagccccacaccttgaccgcgtgcgccgtgacgtagcccgcggcgccgtagaacatggcatggccgaaggagagcaggccgacgtagcccaccagcaggttgaccgaggcggccagcagtgcgaagcacatcagcttcatgaggaacatcgggtagaccgcgaaaggcgcgagggcgagcaccgccagggcggcggccagcaatgcggtgtgggtgcggcgatgcagggtgtccatgtcggtttcctcagtgggcgcggccgaacaggccgtgggggcggaccgcgaggaccaggatcatcacgacgaagatcaccacgccggcgccgtcgggatagaagatcttcgtcaggccctcgatcgcaccgaggccgaagccggtgaagatcgagccgaggatcgatcccatgccgccaatcaccaccaccgcgaacaccacgatgatcaggttcgagcccatcagcgggctcacctggtagatgggagcggccatcacgccgctgagcccggccaggcctaccccgagcccgtaggtcagcatcagcatgcgcggcacgttgatgccgaaggtgcgcaccagcggcgcgttctcgttggcagcgcgcaggtaggcgccgagctgcgttttctcgacgaagaaccaggtgcccatgcacaccgccagcgcggccacgatgacccacacgcggtacatcggcaggaaggtgacgcccacgtccaggccgccagacaacggattggggtagggctgcccgctcacgccgaactgcaggcggaacgcgccttccatgagcaaggcaacgccgaaggtcagcagcagcgcatagacatggtccagcgtgtacaggcgccgcagcatccagcgttcgaacaacagcccgaaagccgccaccaccagcggcgcgatgacgatggcgccccagtacccgatgccaaggtactccagcagcccccaggtgacgaaggcgcccagcatgtactgcgcgccgtgcgcgaagttcaccacgcgcagcagcccgaagatgatcgacagccccaggctcatcagcgcatagaaggcgccgttgatgagcccgaccatcagttgcccgatcagcgccgccggggagattccgaatagcccgtccatcgtgtgttcgtcctgcgttgattgctttgttcagagccccagcagggactcgatgcggccgcgctgcgcgtccagctcgtcgcggcggaaatgcgccgcgacctgcccctcctcgatcacgtagaagcgatcggccagcgtggaggcgaagcggaagttctgctccaccatcagcacggtgaagccgcgctggcgaagcatgccgatggtctggccgatgcgctcgacgatcaccggcgcgaggccttccgtgggttcgtccagcagcagcagccgcgcgccggtgcgcaggatgcgcgcgatggccagcatctgctgctcgccgcccgacagccgcgtgccggggctgtggcggcgctgcagcaggttggggaacagcgtgtagatctcttcgacgctcaggccgcccgggcgcagtaccggcggcagcatcaggttttcctgcgtcgtaaggctcgcgaagatgccgcgctcctcggggcagtaggccagcccgagccgggcaatggcttcgggctgcaatccgatggacggggtcgagccaatgtggatctgcccttcgcgccgcccgagcaggcccatgatggcgcgcagcgtggtggtcttgccggcgccgttgcgtcccagcaggcagaccacctcgccttcgtgcacttcgaggtcgataccctgcagcgccagtgtctcgccgtaccagccgcgcaggccgtccacgcgcagcatggccgttgccgcggcctcacgcatgcacgcctcccacatacgcttcgatcacgcgggcatcgcgcgacacttcgtcatagctgccctcggccagcacctggccggcctgcagcacggtcacctggtcgcacagcgcctcgatgaccttcatgttgtgctcgaccatcagtaccgtccggcctttggcagcatcgcggatcagctcgaccaccgggccgatgtcttcatggcccaggcccgccatcggctcgtcgagcaggatcatctcgggctccattgcaatggtggtggcgagctccagtgcgcgtttgcggccgtagggcagttcgccggccagcgcatcgcgccagtgagccaggcccacgcgctccaacagctccatggcgcgggcgtccaggctgcgcagcacgcgcacgttgcgccagaaggcaaagctgccgccggccttcttctgcagcgcgacgcgcacgttctccagcaccgtcatctggccgaacacggccgagatctggaacgagcgcaccaggccggccatcgccaccgatgcggggtcgctgcgcgagatgtcccggccattgaagatcacatggccggcgctcggccgcaggaaggtggtcagcaggttgaaacacgtggtcttgccggcgccgttggggccgatcagcgcgtgcacggaatgccggcgcacgcgcaggtcgacgttcttcacggcaaagaagccgctgaattgccggctgagctgccgcgcttcgaggatggtgtccatggcgtgagcgatccggtgctcagagaaaggcgtgcgtcacgccgccgtccaccagcagcgattcgcccgtgatgaagctgctgtcggatgaggcgaggaagcacaccgccttggcgacgtcgtccaccgcgccgagccgcttcatcggtgtcttggcgagccgcacctgggccttctcgggcgtgagattgatcttcacgccctcggtctcgatggacccggggcagatcgcgttgacgcggatgccgcgcggcccgaggtcggttgccgccgaacgcgtgagccccagcacgcctgctttcacgccgcagtacagcatgccttcgggcaggcccaggtaggcggccgatgaggcaatgttgacgatgctgccgccttcgctcatggcctcggccgccacctggatgccccaggcgaccgagttgaagccggtgccgaccatgcgctcgagcatctcgggcgtgatggcatcgatggggccgtagcgcacccagatcgcgttgttgaccaggatgtcgaagcggccgaacttttccttcagcaccgggatggactgggtgaaagtgtcgcggcgcgccacgtcgccgccgaaagccatggcccggccaccccgggcctggatggcttcggcggcgtcgcgcgccaggtcttcctggcggtcgagcacgccgacgatggcgccttccgcggccagggcctccgagatggcgcggccgatgccgcgtgcgccgccggtgaccagcgccaccttgccttcgaaacgttgagtcatgttgtctgccttgtcagatcggttgagaggcgtcggcaaagcgggactccgcgagtccgcgcacgccggcgccgtgaatggcgaacaccgcgcccgcgtccggatggtcgctgcgcagcaggttgccgctgttgctgatcgacgtgaggtagatcacgtcgagctcggggccgccgaagcaggggcaggtgacataggtcacaggcaactggatggtgcgttcgagccggccttcgggagtgaagcgcgcgagttgcccggcctgcaccagcgccacccagaggtggccctgggcatcgacggcggcgccatcgggaacggagcccagtgcgcgcgtgtccaccagcacttcactcgggcctgagacgccggtggccgtatcgtagggatggcggcggatctggtgcgtgtggctgtccgcaaagtaaagccagcggccatcggggctgaagcaggtggcgttggcgacagcaatgccgcgctccagcgtggccaccgtgccgtcggaagccagctggtacagcgcaccctggggctcggcgcggcccagggtcatcgagccgaccacgaagcggcccgcgcgatcgacgcggccgtcgttgaggcgcatgcgctcggcggggtgcgtgacgctcgcttccaagggtgtgagcgagccgctgtcggggtcgagcagccagaagtcgttttccagcgccagcagcaggcggccgctctcgcacagcgcgatggagccgatgtgctgcggtgcatgccattgcgcgctcgcgccggtggcgggcgtgtggcggtggacccgttgcgcgcggccgtcgatccagtagagcgactggctgcgcacgtcccacagcgggcactcgccgagcaggtcgcgccggggatcgaggatgtcgatccgcaatggctgggcagaggaggcggtagccatggggcgactacttgcccttgatgaaatcgcaactgctctcggccagcgggcgccaggtctgctccggcgggatctcggcgcgcaccgtgtagtagtcgttcgcgcccttggactcggcgggcttcttcacctgcacggcatagacggggcgaagcgcctggccgtcctcgcggatcctgacgtccttcgagaagaaatcgttgatcggcatggccttcatcttcgccgcgacggtggcgccgtcgtcggtgcccgcggctttgacggcgttcaggtaatgcatggtcgcgctgtaggcgccggcatggatgtaggtcggtaccacgctcttgttgcgggccatgaagcgcttcgaccattcgcgcgaggcatcgtcgcggtcccagtagaagggcaccgtcagctgcaggccctgggccacgtccaggcccatcgccgccacgctgttgatggtcatgccgaacaccgacaccacctggccgttgcgcgtgagcttgtattcggccgcctgcttcagcgcgttcgagaggtccaggcccgcgttcaggatgacgatggcctgcgcgccgctggcctgcgcctgcagcaggtacgacgagaaatcggtggcgcccagcgggtgcttgacggagcccaccaccttgccgcccgcggcctggatgaaccgggcggcgtcgtcctggaaggcctggccgaaggcgtagtccacggtgatgaagtagaagctcttcacgccctgcttcatcaggctctgcacacccgccttgggcagcgcataggtgtcggtgaggaactggaagttcatcggcgagcacgacttgttggtcagctccgcgctcaccgtgccggcgatcaggtaaggcttcttgcgttccttgagcagcgatgacacgcccagcgcgatggaggaggccgagccgccgacgatggtgtcgactttttcggtgtccagccatttgcgcgcgatgttcaatcccacgtcgggcttgttctggtcgtcggccagcagcacctcgacgggcttgccgagtaccttgccgccaaagtcctcgacggccatcttcacggccagcgaagagccgggaccgccgttgcccgaataggggcccgtctggtcggccatgacgccgatgcgcaccacgtcgtcgctgatggcgctgccttgggccgaagcggccgcactgacgagaagggcgaccgcgcaggccgcgaggcggaatcgatgttgcatgtctgtctccgttgtgtgtgtgagggttgctgtcgcttgagctctgccgcagctccggtgccttggattgccgaagggaaagaggaagcctcagccgccgggtatgtccgtaggcaaccggtggccgcggaactgctcgcgcagccgggtcttctgcagcttgccggtggcggtgtggggcaactcgtcgacgaagacgacgtcgtcgggcatccaccagcgcgccacgcggtcctgcatgaagccgaggatttcctcggacgtgagttgctcgccctcgttcgggaccacgatcagcagcgggcgttcctgccacttgctgtggtacgcgccgatgaccgccgcctccttcaccttgggatgaccgactgcgaggttttccaggtcgatcgacgagatccattcgccgcccgacttgatcacgtccttcgagcggtcggtgatctgcacgtagccgtccttgtcgatcagcgccacatcgccggtggcgaaccagccgtcggcatcgagcgacgcgccgggctcctggccgtagtaggccgacaccacccaggggccgcgcaccttcagttcgcccggcgtgtgcgtgccgtcgggcagcctgcgcccctcggcgtcgaacaccgcgatctcgacgccgaagatggcgcgcccctgccgcgcctgcacgtcgaagcgctcctcgagcgggatgccctcgtggcgcggcagcaggttgcagatcgtggccagcgggctggtctcggtcatgccccaggcctggatcacataggcgccgaacagatgctcgaatttctcgatgacggcgcgcggcgcagcggagccaccgaccacgacgcgttccaggcacagttcggcgcgcgtggccgcatcgagcttctccgcgtgctggaagaagccgagccacacggtcggcacgccgagcgaaaaggtgcagcgctcgtcgcgcatcagggtgaagaggcgctcgccgccgaggtccggccccggcagcaccagcttggcgccgcacatcgcgcccgcatacgggatgccccaggcgttcacatggaacattggcactgcgagcagcacgctgtcgtgcgcgcgcagctgaaggccgtcggccgcgcacgccgcccacgagtgcagcaccgtcgagcggtggctgtaaagcacgcccttggggttgccggtggtgccggaggtgtagcaaagcgaggaagcggtgttctcgtcgaggtcgggccactgcgccagcggctcggcctctgccaccaggtcctcgtagcacagcagcggcccgggcaggtccagcgcgggcagctccgcgtgggagcaaagcgcgacgaatgccttgaccgacttcagctggggcgcgacctgcgcgagcagtggcgcgaacccgagatcgaagaagagcaggtcgtcggccgcatggttgacgatgtagccgatctggtccgggaagagccgcgggttgaccgtgtgcagcaccgccccgatgcctgagacagcgtagtagagctccaggtgccgatgcgtgttccaggccagcgtcgcgacacgcgcgccgggctggatgccgcgcgcctgcagcgccgatgcgagcctggccgcgcgctgcgccacctgccgccagttcgttcgctcgcactgctgggcgttgacgtgcgagacgatttcgacgtccggatggtgccgcgccgcgtgctccagcagtttggaaatcaggagcgcgttgctctgcatcaaggcattcatctcgttgtctcgtgtctttcttctgtcacgtcgagcggtttgccggttttgtttttacatgccggccggtaagttaacttatgctagcagctttgattgcccactacaacgcgagccggcccggggaaacccggggaatagggccggtggcaaccacccgtggcgggctgatccacgcaacttttccggcaacttttccgatccaacatgaacattcgacgtcacgtctgcgctttcattctcggagccactttcgcgggagcgcatgcacaaaacgcagcgcccgcgatggcatccactctgttgtcacaggccctgctcctgtccgatggcgcacagccccaggtggtcgaatggcgccggcatattcaccagaaccccgagctggcctaccaggaaaccggcaccgcgaagtacatcgcccagaccctcgctggcatgcccggcctcgaggtgcgcaccggaatcgccggcacgggcatcaaggccgtgctgcgtggtggccgtccaggccctgtggtggcgctgcgggcggacatggatgccttgcccgtggaggagcgcaacgacctgcccttcaagtccacggccaaggcggactggctgggcaagcccgtcgccgtgtcgcatgtctgcgggcacgacgcgcacgtcgccatgctgctgggcgcggccaaggtgctgtcgtcgttgcgcgagcagttggctggcacggtggtcttcatcttccagccggccgaggagatcggcccgggcctgggcaagtccagcggcgccatggcgatggtgcgtgagggcgtgctcgacaaccccaaggtcgacgtcgtactcggccagcacatcagcaaccaggcgccttccggcgcgatccgctacaggccgggcccgatgctggccagcatcgacgtgtttcgtatccagttcaagggcaccggcggccacggcgcggcgccgtgggcctccaacacgcccatgctggccgcggccgagaccgtgctgggcctgcagaacatcgtgagccaccggctcaacccgaccatcgacggtgggccgacgatcgtgaccaccggcatgttgcagagcgggaaccgcttcaatgtgcttcccgagacggccgagatcgccggcacgatccgcgcgctctcgccgacgaaccagaagatcgcccaggaggaaatccgccgccgcgccacgggcatcgcggccagctacggcgtgcaggcggacgtcaagatcgacagcggagacggctacgaggtgctggtcagcgaccgggacgccacgctctcgctggtgggcgccttcggtgccgccgcgggaggtgccgcgaaggtgagccagatgcctgcctccatgggatcggaagacttcggcgccttcggttcgaccggtgtgccggtcgtgttctggatgctgaacgcctcgccgatgggcgacaaggacgggccggtgaatcactcgccgttgttccagatcgacgaatcggcgatgcgcgtgggcgttcgcgcactgaccgcggcgacgctttcccagttggccaacgagcggtttcagagtcgctgagaacctgaggcagcagcgttcggtgtcccgacctgcctgaacgcgaaccccgtgaacggccgccgcgtgagaaaccaccagcttgatctaggaggctgggcggcagaagcttctgagaagccttgccgatgaggccaattcagtttggcgaaggccacatgcggcgtgcgcgccggttctgacgtactgcgcagtctgttggggccgcatcgcgaggcttgagggggcgttcgcagctggttcctcgcctcgtcgctaatccttcagaggcgagatgccttgcaccggcccgatcagccgttcgaacaggcttttcagccgctcgacgcgcgcgcggtcacgcatgaaggccaggaagtcggcagggctggtgttgtacttgtcgatggtcttgaagccgggaggcggcgcgacgtccttgcgcagcgggaactggcgcggcgcggcattctccggaagggacagccgccagctcacgtagagcttggctgcggcgggatgcttggcgtccttgaagatagcgccggtctgcgcccaggtcaggaaggggtcattcgtcggcagcacgaaacgggtattgaccgactcgactggcacgaaaggtcccgaggtcccggtggccactgcatacttgcccacctccaccgcgtcgcgcggcgtctgggtgccacgcacccactgcacgccattggcctggagcttctcgatgaagtcgatgccgtacttctggatgatcttgtcgaagacatagagcaccgcatcgtcgtcgttcgggtaggcgatgatgatcttgttcttgaactcgggcttcagaaagtcggcgtagtcgcgcggttcgttgccggcttgcacgagattcttgttgtagctgttcgcgaacgtcagcatgaacaggcccgtgaatcggccctgggggtccttgtaagcgtcgggcacctggtcccatccgatcggcttgtagggcagcagcaggccgcgcgccgcccagtcgtcgaagtcgtgcaaggtttgcagatgcgccacatccaccttcaagttcttgcgcagcagctcttcctcgatgcgggcgtcgtggtacttgctcaagtccatcacgatgtcgagtttcataccgggaaactggcgttcgaatgcagccttggtgccgaagccctgcgtgacctcgtcgccgccggcgtacaccgtcagctgtccgccctcctgcagggcggcctggtaaagctcctggagcgaacgccccgcaccgtcgcgctccacgggagcggtcaccgatgtggtcgtgggcgcaggggctgcctgttgggcgctcgcgggggcggttgcggcgagcacggcaaggccgacggcagcaagccatgcgcggagacagacatgtctatggatcatcgaatgagtctttcgtgagtgggctggccacccggggttgagagaaggtgaggcgagtcgggcagcgctgcgcggggcaccgcgagccacagtcactgcggctgccggcgcgtcctgatccttgttgttgcggtgcgctgttcagaaagcctttcgggtcgaccagaggattggcatcccctggtttgcgtgccttcaacagctctttcgtttcggtgaggccgttggaaaacgcatgcgtcgtcaggtgcgtggtgaccggatcgaccctgtcttcggtgagcgcacgtatgcgtttgaggctggagatgtaggcctccacctgctcggggccgcgaatggcattgagcccgaggcctccaaccgtgaaggcgcgatagcgcttcgtgccgtcgaatgcgtcgaatgagaacgacgcggtgcccatcgtatggcccggcgtctcgaaagattgcaggggcacgccaccggctttgaccatttggccgtcggtcagcacttggtcgggcgcgatcatcgtccagcggtccggccggccggccgactgcgccgcgttctcggccgcttcgcgccagccctcggcggtcattgcgaaacgggcttgtggcagttgctccttgagccgggccgcaccgccggatcggcgccgactcgcagcgcgtggtgagtggttcttgggcttcagcactgagcccagcggcggccagccccagggcgagcagggtccgtgtcgtgatccggcgaatcgcggggcgcatggagcgatggagctttgtcatgtcttcgtggcgttgcgatggatgcgccatcgagtgtcgcgggcctgtcggagcgagacaatcaatcgcttgtgagagcttttaaagcaacgcttgataatgcgtggcatggccttcacgcgattcacactgcgccagatcgagaccttcattgcggttgccgaggttcacagcttcacggatgccgcatctcgcctgggcctcacgacgcaagcggtcagtcagatcgtcgcggaactcgagggcgtcatcggttttcgcctgttcgatcgcacgacgcgcaagtgcacgctctccagcgccgggcgtgactttctcggctctgcgcagaccttgttgcgccatgttcgagcatcagagagcgctgcggacgatgttcggaaccgggcctcgggcgtggttcgcgtaggcgcgccgctggtgctggcgtcgaccttgctgccgatggcgatgcgggcctatgcgcggcagcggccgaaggtggtggtgcgcatccgcgacgtggcggtggacgccttggtcgacagtgtcgccgccggcgatgtcgacctcgcgattggtccggatcttgtcgtcgacgacaacgtgatcgccgaagcgttgttcgacagcgagtgggtcctgtggtgcgctcgaggacacccgcttgcccgccggcgcgctgccatccggtgggccgacctgcgcgacgtgcccctggtcgcctcagggcgcgatcatgaacagagcgtggcgcagatgcgcgtgagcgcgccggatggtttgcgcgtcactccggtgcacgttgtggacaacatctccacagcatttgggatcgcggcgcagggactgggggcgaccctcgcaccggcgtacgtcggggttttcgccaaggcgttcggtctggagatgcgccgagtgactgatccggagacggtccgcaaggtctgcttgtaccgttccgcattgcgtgatccgtcccctgcagtcgaaggcttcggtgcattcttctcccgttggctgatcaggtggcatgcgtcggagaggcgaaggctttccgaaacagaccgccccggttcggcaaaaggcacgaagcgctgaacggtttgcgtcacccatcctgacgttctcgttctatcagcggggcgcggtgccaccgaaacgtggctggcggcgtggccgagcccaccgcggcttgccgctgtcatttcccacaagggctgccgcaacaagttgctccgtacggctgatgtgcttgcatagcagctccgtcgccctctaggcatcgcgcgcgagaactgtattcagcagttgctgatgctcgtcgtgcttacgccgtggctcttggcggaacttgactgcccagcgtcgatagcgttcggcgttgtcgaagaggacgtcggccaagtccagcaacaggggagatgtgcttggccgccgatgaggatgtcttcgccgtatatttaacataagatacattgtattgtttgtggatgtagcggctgattagaaatgtcgcatggtcgcctccgcccagcttctggagcgaccacgcatgttcgaagaccgcgcgccatcgtgcacgctgctggtatgtatcgacgatgcgactagccggtgatgcagctgcgctttgtgcggaccgaatcggcatcgcgtatttcgaggccacgcgaggctatatcgagcagcatggcaagcccgtggcgttctacagcgacaaggccagcatcttccgttcggtgcgcgactcgaccgacttcggccgtggcacgacccagttcgggcggatacttttcgagctgaatatcgacaccatgcgcgcgaacaccagccagaccaagggccgcgttggcttgcctggttccgacgtcagccgagcatcgggttcactacggcttggaaacgaacagccccaattcggaaagatccgtaaaagctccgtcgccattgttggctgtgatgttgagccggtagtagcggtaggagcccggattcgcgatcgcgtaggtcttcagctccaggcgttcggcaaacacctggtcgctttgcgtgtcgagcgtggtccaggcggcgccgtcgctggagacctggaactgccagtccttcggatcgcgcgagaccaggtcggaactgctggtgaccgcataacgcaggacgcgctccgtgtgcccgaggtcgtactgcagccagccggtcgtgccagagtagaaccattgcgtcgccgagttcaggtcgaaggcgcgtttcgcgttggtcgcgttgcctgcactgtcgtttgcggtgccgccggtcgcgacgttcaccatcgaaggaaccggcgtggcgctgtccgcaggagaactatcgctcgttccggcggagttgctcgccgtgacggtgtagtagtaggtcgtgccattggtcacggacgtgtccgtgtagtttctgcccttgacgcccgacgcgatcgtctcgtagggcccgtcgctgaactcggagcggccgaccgtgtagctggtagcgccaaaggacgcctgccagcgcagcgggacggcgccatcgcccggcgatgccagcagcatggcgggcgccgcggggatgacgctcggtgcaccgccgttgccgccggtgatctggacgttgctgaacgtggagctgttcagggtgccctgggtcgccccggagaccaccagaccgacatagagcgtatcgggaacgggcccgacgatgcggccgagatcggtggcggcccaattggtgccatcgggagaaatatagccggtgatgatgtttccgatgcgctcgagcttcacccaattaatgggcccggaggtcccatcggtcaatatcttgttcgcgtagtacgagccgccatacaccgccaggttcgtcatgttctgtaaggcttggcctttgtcgcttatcgccatccaggcgcgtggagcgcctggatccagacttgtgcgcatcatcacgcctgccactccggagctctgaatcgactcgactttcgcgatgatggcgccgttgcccgtgatggccttgtaggtgaagtggcaactgtcgcttgcaccccagatattggccccagctccccgaaccatccatttgccgttggcgtatgtggccacaccggccgggctggcgcccccgatgtcggcgctgctgaaccccgaggtgatcgaggtggtcgaaggaatgggcagcgccggcggcggcgtcgccttcgaggtgtcggattccttgaggtacatgaagctggtgccgtccacaggtgcccacaggcgtcgctgcgtaataaagggtgcctggagacccttgcgcaggacgtaggcaccatgaagctgagtgagtacgacggtcccacccccgccgccccgccagccgcgattggtgacgtcggaggtgtagtagcgatcggtggtgccgaaaggaagcgctgtcgtcgggacgagctcgttcaccctcgcgaaatactcacccgtcgctagcaggcggttgtcaaagtctgaatagatgtcgatgccttgggtccagagcgcttccgccagcatggtcagtgaccgaagctgcccatagccgtgcccctggtcacggagatagtcgccgagcatgccgatgtcgttggaattgcgcagtccgatatgggccagcgtgcgcgtctggtatacgacccggtccaatgtctcaatgtcgtcgttgtagatcgccataagtcccaaagcgacgagggacaacgcgcccttgttgcccgccccaaactgactctcgccatagggattcgctgccggcatcaggacgtttttgaagtacttcttgaccgtcgccgtgtcggcctccgtccagcccgggtaggtgctgcgcaggatttccgcaccgccaacgaactgaaacgcgtaatcgcccagatcgagcatggactcgcgacccgagaactcggtctgggtggtggcccacccaagcagcaggccccttgcaatcttcgcgtattgctcgttctgggtgaaataccacatctgcgagagttccgagatcgcgatcatgtcgcggcgccaagcatggagattcacgtcgggggcgcggctcaccttcgcgaacgggccaccggcccctgcgtagctgagcctggcgttgggactgttcgccaattggttgtagccggacttccacggctccttgccttgctcgacattcgccttgagcgtctgaagatccgacagggtgagcccagcgcctgggtgcttgatcacgcgggccaccggggtgtctctcggggcggcggggatttcgggggtgactcccgtggtggcgggaatctccggtgtgcctcccgcgacagcgggaacctccggggtgtcccccgcgacagcagggaccggagcgcctgcctggaaacttcccgaatttccgcccccgcaacccgggagcacgatcgcgctcaacacgagcaacgcagcagcaaaatcggttttatcaaacataggatccttcatagccaatgcgcggaaaagtcgcggagcccggcacggcgccgccagctttcgttgaggcgttgatttcagtgataagcctgcgatccgccgtgaaggcctttcggcccgcgaggcgggcgaatcctggcgttcgtccaagaagaggatgcgagcgctggagtgttgatttccatcgaatatgaatctgccctctttgtgagcctgatggctcaggatataggtaagcttttggttttcacttgagcttggactgcctgaacgaggtgcgccgcgctgtgttggatcggacgctttcattgaggcgctggctataaaagtgtaacatgcacgatacaattacgggcattcaatgcctttgatgatcgacctattgctagctgcagccagcaacggcgaatcccgaggagccgaaaatcgctactggaccaaggcctcctcggagcgctcctccaccaaatccgacgacagcttggcgaagatccgttgcgcatattcctgcacggcctcgaaaagcgcatcctggtgtcccgccagaacgcgtcaacgccttggaccttctcactcgcaggtgactgcttggcgcagcggcgcgcctaatccctccgtccaaagcatcgcggatgcgttcacacaagcgcgctcgatggcgcatcactgcctctccggcgcagaccatgccttgtccgcgccagccagccagcaggtgtatgcgacgctgctcgttgcctggttcaaacgacgggtttcaactcctgacgcgatgagaccgcccccatgagcggcggtgccaaggtcctttcgacacgccacgttcagggcgttccctgcctccgtcgcgtcaaccgagtatcgggttcactgcggcttcaaggcgaacagcccgaattcggaaagagccgtgaaagtgctgtcgccgttgttggctgtgatgttcagccggtagtagcgataggaggccggactcgcgaccgcgtaagtcttcaactcgaagcgtttctggttgctttgggtgtcgagcgtggtccagttggagccatcgttggagccctggagctgccagtccttcggatcacgcccgacgagattggcgtcgggagtgctggtgaccgaatagcgctggacgtgctccgtgtggccgaggtcatactgcagccagccagttacgccctcgtagagccattgcgagtacgtgttcaggtcgaaggcgcgtttggcgttggtcgcgttgcctgcactgtcgtttgcggtgccgccggtcgcgacgttcaccatcgaaggagccggcgtggcactgtccgcaggagaactatcgctcgttccggcggagttggtcgccgtgacggtgtagtggtaagtggtgccattggtcacggaggtgtccgtgtagctgctgcccttgacgcccgacgcgatcgtctcagagggccccccgctgatgttggagcggtgaacggtgtagctggtggccccgaaggacgcctgccagcgcagcggtacggccccatcgcccggcgaggcgagcagcatggcgggcgccgcggggatgacgctcggcgcaccaccgtcgccgccggtgatctggacattgctgaagacgctgttgttcagcttgcttgtgaccgacgagaccaccaatccaacatagatcgtgtcgggaacgggggcgtcgatacggccgacatcggtagcggcccaattggtgccatcgggagaaacgtagccggtgatgatgttcccgatgcgctcgagcttcacccagtaagtgggcccggagctcgcaaccttgttcgcgtagttcgagccgccatacaccgccagtttcgtcatgttctgtaaggcttcacctttgtaatttatcgccatccaggcgcgcggagcgcctggatccaggcttgtgcgcatcatcacgcccgccattgcggacgggtgggtgttctggagcgactcgactttcgcgatgatggtgctgttgccggtgagggccttgtaggcgaagtggcaactgtcgagtgcgccccagataccccagcctgccccagccacgttccatttgccggtggcgtatgtggccgcgccggccgggctggcgcccccgatgtcagcactgttgaaccccgaggtgatcgaggtggccgaaggaatgggcagtgccggcggcggcgtcgccttcgaggtgtcggaatccttgaggaacatgaagctggtgccggtcaggggcatccagaggcgtctctgcgcgatgaagggtgcctggaggcccttgcgcaggacgtaggcgccataaatctgagtgagcgccacgtttccgccattggcgccctgccaaccgtgcccggtgcggtcggaggtgtagtacgcatcggtggtgccgaaaggaagcgctgccgtgggcacgagttcgttcacccgcgcgaaatactcacccgcggccagcaggcggttgtcaagatcggaatagatgtcgatgccttggctccagagtgcctcggcgagcgtggtcagtgacgcgagctgtccataggcatgcccctggtcgcggagcgagtcgccgagcatgccgatgtcattggaatttcgcaacccgatatgggccagcgtgcgcgtctggtagacgaccttgtccaatgtctcgatgtcgtcgttgtagatcgccatcagtccaagcgcgacgagggccagtgcgcccttgttggcggccccgtacgagctttcgccataggggttcgccgccggcatcaggacgttcttgaaatacttcttgaccgtcgccgtgtcggcctccttccagcccggccaggtggcgcgcaggatttccgcgccgccaacgaactgcatggcgtagtcacccagatccagcatcgattcacgacccgagaactcaacgtgggtggtggcccacgcaagcagcatctcgcgcgccttgtccgcgtatcggtcgtcccgagtgaagtaccacatccgggagagattccagatcgcgaccatgtcgttgcgccaggcttggagattctcgtggggcgcgcggctcactttcgcgaacgggccgtacctttcgtaggagagcctggacatggggctgttcgccatttgctcgtagccggatttccacggttcccttccttgatcgacgtaggccttgagcgtctggagatccgagagggtgagcccaacgcctggatgcttgatgacgcgggccaccggggtgtctcccggggcggcggggatttcgggggtggctcccgtggtggcgggagtctccggtgtgcctcccgccacaacgggaacctgcggggtgcctcccgtgacaacagggatctctgcagcgcctcccatctgggcatttcccgcatttccgccaccgcaacccgggagcacgatcgcgctcaacacgagcaacgcagcagcaaaattggttctatcaaacatgggaaccttcttagtcaatacgcgaaaaagtcgcggagcccggcacggcgccgccagctttcctcgaggcgttgatttcattggtaagcctgcgatccaacttgaagtttcttggctcgcgaggcaggcgaatcctggtgttcatccaagaagaggatgttgtgagcaccggggtgttgattcccatcgagtatggattcgccctttttgtgagccagagcggacggggttcagttgctgtacaacacgccacggccggtgccgctcacatagatgcgtccgtagatgttctgatcggccgccatcgcgccgatgccgccgaactggtgcgcgtcgtcgttgaagcgagtccaggtgacgccagcgttgtcggagcggtacacgccccacacgccgttcaccacgcccaccacgtagaccgcagccgagtacgccgcgccaggcgctgccttgcccaaggccaccaaggtggcgccctggacgtcgggccacgggttgctgcccatgatcgacgcaaagtggctcagcttcttccaggttgcccccgaatccaccgagcggtacacggcgttgccgtcggccagccagaggtcgccctcggcgttggggttgaccgccagcgacgtgttggcgaagtagttgggggccagccctgcggccaccgaaccctggctcagcgtgaacgtgcggccgccatccgtcgacacgtagaccttgcccggcgtgccccaccagtggccgcccgaatcgtaggcatagaccttgttcgggttcttgcgatcggcgaccaggtggtaggcgcgagggaagatggcattgatcgccggcagattggtcgggatccaggtggcgccgttgtccatggtgtaggacggcaccgagttgccaggcgcccagaccgccttgttgcgcgtggtgaccgcgatgctcgcttcctggcccttgttttccgcgacgcccggcgggtaggtggcgaactttgcccaggtctcgccgccgtcgccggaccacatgccgaagccggtgctgttacccagcacgacgccgatggtggccatgtactgcgagtcagaccacgccatgtcggtggcgaagccgttgctccagtcggtggccggcgtcagcgtcggcttggtcgcgaggttggtgtgcacccaggcgccgacgtcgcccgaactgttgatcacggtgtaggttgcgccggccggcggcgtggcgaggcccagcacggctgtctcctcgattccgttgaccgtgctggcccaggttggcgtggccgaggaggcgttgtgtgtctccatgacgccgccggcgacgtgcaggatgtggttgcggtcgaatggatcgatctcgacatcgtcgatccagccccaggcgacctcgcccggcgtcatcgcttcgatctcgcgccagttccggccggcatcgtcggacagctggaggatttgctggccggggtagttgccccaggtgttggtcacccccagcgcaatgcgcgtcgtcgcgccggtgccggagacggacacgccgccgtagccgaccgagtcgtcgctcttgagcaaggtccagttgctgccgtcgaacttgtacagacgggcgggaccggcggagccgggaccggtgtccttggtgaagaccacatagaacgtgccgtcagcggcgcgcaccatgtgcgggatgtgatagccggagatcggcaccgagactggggtccacgaggcgccgccgttgctggacttgtacaggttcgaggccaggcctgctgtctggacgtagtccggcgcaatgggggcgtagatcgtctgcgtggccgagccgctgcccttggtgccggtgtcgtagacgatcgtctcgacgcccattgcgctgttcatgcccaaggcattgacctggtcctgggtcagcttggcgctcgacagcgacgtgacctgcgcccaggtgaggcccgagtcggcgctcttccacaggccggccgtgcgcgagccgtagaacagtgtcgacggcttgttggggtcgaccatcaggcgttcgccgatggcccggccggggttgttgccgcccagggggaaaggcagggcgacgtaggtccactggtcaccgcggttgccggagatgtacaggcggccgttgcccccggacgtgtacatgccggcggccatgtagacgagctggtcgttgttcggatcgacggcgatgctttcgatgccgtggaacccttcctcgcctccgccgaaccccagaccatcggtgatgggcgtccaggacgaagcgccctggttccaacggtaggcgccaccgacgtcggtgcgtgcgtacagcaggttggcggtggtcgggtggaacacgaggcccgtgacgtagccgccgccgccccacttcgcgctcgtccaggtggtggcctggcccggtgcgggtgcagttgcagttgcgggtgcgggtgcagtcgcagtcgcagtcgcagttgaagttgaagttgcagttgcagttgcagttgcgggtgtgcctgcaacgagcgctgctgtcgaagtgcccgacgacccaccgccacaagccgcgacccatgtgctcagcaggccgatcgcgatgagccgcgcgcgattccagttgcgggggatcgtcgacggaaccggcgacgatcggtcaatggacacctcacccattcttcttgaaatctgtgacatttttggcatattgtgtgtaattgtataaatgccgcaagaaccgaaccactcagatcgtcgccgcacgaccgtgaaaaagcgaccagatgtgtcacccggatcgatgcgccttggaccttcacatggatggctgcgatcggcgccctgccctttgaactgatccaagccgattccgaaggcacggaacggtgccgcggcggttgcaagaggcggcactgccgcttcttatgcacgcatcggctaagcaataccgaaaggcttctttggccgccttgcaagcgacgcgtagtctgtggcgattctttcaaggagccccagatgaacgatcgtttgaaccgccggcatgcatcgcgctccgccgccgtgaaggccggactcgaccacccggtgatcgacacggatgttcacgtcaacgactacgcccccgtgctcgaggactacgtggcgcagtacggcggcagcaagctggtcgacgcgctgcgcaaggcgctgggcgggcgcttcgtcacgcgcaacggcggcggcaaggactggtaccagcagacggccgaagaacgccagttccaccgcacgctgcgcgcgccctggtgggcccgcgtgacgcgcaacacctacgacctggccacctatacgttgccggcgctgctgtatgagcgcctgggcgagcaaggctcggactactcgatcctgtttcccaacgacgtgctctcgcccgccgcggcgggcagcgaataccgccagccgctgcaccgtgcgatcaaccactttcatgccgaccagtaccggccgtacgccgaccgcctgacgccggtggcgggcattccgctgcacacgccgcaggaaggcatcgaggaactggaattcgcggtcaagacgctcggcctgaaggtgatcaacatcgctggtggcgtgcgccgccccattcgcgccatcgccgagaagtacccgcccaaggaccacccggagatcgccaagcagaccggctacatcgacttctatggcatcgacagcgagcacgactacgaccccttctgggccaaggtggtggagttgggcgtgcctgtcaccacacactatggcagccagggctggacgagccggcagtcgatcagcaactacatgaacaaccacatcggccacttcgccgatggctcgcaagcctttgccaaggcgctgttcttcggcggcgtgacgcggcggtttccggccttgcgcgtgggcctgctcgaaggcggcgccgactggggttcgcatgtctacgcgcacctggtcgaccgctgggagaagcgcaaccggaatgccgtgcgcaactacgaccccgcggaagccgacgtcgacctgctcgcctcgctcttcgaacgctacggcagcgaccttctgaaaggccgcaagctcgacaagtcgaagctgctgcgcgacagcctcggcatttccgcgctgccgcacagccgcgagccgaatgaatcggagatcgacgacttcgcgctcgccggcatcgagaaggtcgaggacatccgcgaccgctgggtgaacaacttctacttcggctcagaggccgacgaccgcacggtggctgcggccttcaataccaaggtgaatccgctgggcacgaagatcaacgcgatctggtcgtccgacgtgggccactgggacgtgcccgagttcacagagccgctggtcgaaacctgggacctggtgcagcaaggcgtgatctcggccgcggatttcagggcctttgtcttcgacaacccgcatcgcttctacaccgaagccaacccgcgcttcttcgaaggcaccgaggtgggccgcaagctcgccctgaaaggcgagaagtgagcggcacgacacgcgccctgctcgcccgcctgcgccgttgggcggcgccgctcggccttctcgcgctgatggccggtgcgctgcctgcgcaggcggccccggagaccatccgcatcggcgtcgcgacagcgggcggcggcgatcccgtcacctggggcggctcgcccggcggcgtcgcgcgcgtcagcaactggctggaggacgagttcaaggccaccggagtcaaggtcgaatggctgttcttcaagggcgccgggccggccgtgaacgaagcgctgtcgaacaagcagatcgatttcgcctaccagggcgacctcccgtcgatcgtcgggcgctccaacggcctgaagaccaagctgctgctggtgagcggcgcgcgcaacaacctgtacctggtggcgccgcccaagtccgacatccggtcgatcaaggatctgagggaccgcacggtctcgatcttccgcggcaccaacggccacctcgtcgccatcaacgtgctggcagctgccggactggccgagcgcgacatcaagggcgtgaacctcgacactggcagcgcgcaagctgcgctggtgtcgaacggcgtggatgcggccttcggtggctacgagtggttcaaggtgcgcgaccagggcctcgccaaggtggtgtattccacgcaggggcaggatccggccctcacacgccaggcctcgctgctggttcgctccgacttcgagcaggccaacccggccgaggtgcagcgcgtggtcgacgtgttcgtgcgcgccgcgcgctggtcgtcggacgagaagaaccgcgatgaactcttccgggtctgggcgcgcagcggcacgccggttgcgtcctgggcggcggagttcgatcagcagcaactcgcactacgaaattcgccgctcgtcgacgacttcatcatcggtcgctacaaggccgtggtggccgacgcgctcaagctcaagctgatccgccgcgaggtgtcggtagacgactggttcgacacgcgctacctgaagaatgcgttgaagaagcaggggctggaaacctactggacggcctacgacgccaagggacagccgaaggtgggccagtcggtcgcttcaagatgagccggctgtcttcttccctctcccgcttgcgggagagggccagggtgagggcatcggccttcacacgagcaccgcattcccacgtgccgctggccctcaccccagccctctccccaagggagagggagcaatacacatgagcgccgaggtcgaactgacagccgtcccacagcctcgcgacgacacgcccgcgtcgtcgctgccctggcgccacatcggcgaccgcgccttgccctggctcctgcccatcgcgctgctggcgctgtggttcgcgggcgccgagcagggctggatctcgccgcaggtgctgccgccgccgcagttcgtgtgggaaacccttcgcgatctcgccatgagcggcgacctgtggctgcacgtgagcaccagtttcacgcgcgtgggcgtcggcttcacggccggaacacttctgggattggcgctgggctcggccatgggcctgtcgcgctgcttcgaagcctacgtgctgcccaccttcaatgcgctggtgcagatcccggtgctggcctggctgccgttcgtgctgctgatcgtgggcatcggcgagccactgaagtacatcctcatcgccaaggcggcgctggtgccggtggcgctcaacacgctgcagggctttcggcagaccccatccgcgctgcgcgaagtcggccaggtgtacggctacacccggcgtcagcaggtgctggaggtcgtgttgccgcacgcggtgcccacgctcttcaccggcgtgcggctgggcttcaccaaggcctggctctcgctggtcgtggtggagctggtggcttccagcgaagggctgggctacctcatcgtctatggccggcagctgttccagctcgacctggtgatggccgccgtgatcgtggtgggcgccatcggctatgccatcgaccggctgctcgaccgccttgaaaccgcggtgcaccagcgccaacctggtggagccgcccgatgagcacggccacgcgggacgcagccgagctggctgccgtacagccccttcgacccgagcagcgcagccgctggcgcggcttcgtgctgcccgtggcggctgtcttgctgtggtggctgctgtcgtcgctcggtgtcgtgaactcggcgctgctggtctcgccggccaaggtgttcgacaccgcggtcgaccaggtggcgagcgggcgcctctggcgcgccctcagcgccagcctcgcgcgggaagcaacgggcttcctgatcggcaccttctcgggtctcgtgctcggcgctttgctgggtttgtcgccgctcttcaaccgcatcgtcggtccgagcttcaacaccttcaagcagatctctctgttcgcgtggattccgctgatctcggtgtggtttggccttggggacgtcgccaaggtggtgtttctctcgctggccgcgctggtgccggtggtggtcaacacctgtgacggcattcgcaccgcaccggccggcctgctcgaggtggcgcgcgtctacggctacacgcgctggcagaccgtcacgcaggtcgtgctgccggccgccctgccctcgatcttcacgggcgtctacctggcgctcatctattcctggctcgcgaccatcggcgccgagtacctgctggtggccggccacggcatcggcaacacgctgatcgagggcagcgagcatttccagatggacctggtcatcttcggcatgttcgtgatcggcctcgtgggctggctcatgaacgcctcggcccgcgcgctggagcgccgcctggcgcgctggactgggcgcgcatgaaccacgcagaaagaactctcctctcatgacctccctccatgcgaacccttccaacgagctagacatccgcgggctcggcaagcgctatgcgaacacgcaggccagcggcggcgaactgcaggtgctcgaaggcatcgacctgcatgttccggcgggccgcttcgtgagcatcgtcggcgccagcggctgcggcaagtccactttgctgcggctcatcctcggactcgatgcgcagtacgagggccggatcctgctggacggcgaacccatctctggaaccggacgcgagcgcggcatcgtcttccaggaccatcgcctgtttccctggctcacggtggagcagaacatcgctgtcggcctgcgcaacgcacccttcagcgccaaggaaaagcgcgatctggtggccgagcatgtcgcactggtcggcctcgagggcttcgagaaatcctggccgcaccagatctccggcggcatggcgcaacgcgtggcaattgcgcgcggcctggtgaaccggccacgcgtgctgctgctggacgagcccttcggcgcgctcgatgcgctcacgcgctcgcggctgcagaacgagcttcagcgcatctggcagaaggagcgcatcacgatgctgctggtcacgcacgatgtcgaggaagccgtcttcctcggcgatcgcgtggtggtgatgcagccctcgcccggccgcatccggcgcacggtcgaggtcgacctgccgcacccgcgcaaccgcagcgacccggcattcatcgccttgcgcgacgacgtgctcggcgacttcctcgatgtcgataccggccgcacaccgattgcggcaccgcaacccgaagcggccgcagccgggctgccgcagcgcctgcagctggcgtggtgagcgggcgcggcccgctttctctcccgtgcaggtaggcgccgagggcgccgggcagccgcaccagtcaggcgcggcgctgccccgccaaccgccgcaccacagccaccagccggtcgatctcgtcgaaggtgttgtagaaggccagcgatggccgcaccgtcgtctcgacaccgaagcggcgcaggatcggctgcgcgcaatggtggcccgtgcgcacggcaatgccttcgtcgttgagcgcatggcccacctcctcggtggtatagccgtcgagcacgaaggacatcacgctggccttgtcggccgccgtgccgatcaaccgcacaccgggaatggcgccgagctcagccatgccatacacgagcagatcgtgctcgtagcgcgcgatgttctcgatgccgaccttgttgacgtagtcgatggccgcacccagcgccacggcatcggcgatgttgccggtgccggcctcgaacttgttcggaatcggctggaacaccgtcttctcgaaggtcacgtcggcaatcatgttgccgccgccctgccagggcggcatgtcttccagcacttcgcgcttgccccagaccacgccgatgccggtcgggccgaacaccttgtggccggagaagacgaagaagtcggcgccgatgtcctgcacgtccacgcgcatgtgcgagaccgactgcgcgccgtcgaccagcgccttcgcgcccgcgcggtgcgccagctccacgatctccttcaccggtaccacggtacccagtgcgttggacacttgcgtgatcgcgacgatcttcgtgcggtcgttcagcagcttgcggtattcgtccagcagcacctgtcccgaatcgtccaccggaatcacgcgcagcttcgcgcctttggcggcggcgagctgctgccagggcacgatgttggcgtggtgctcgaggttggacacgatgatctcgtcgccctcgcccacatgctgcccgccccagctcttggccacgaggttgatggcctcggtggtaccgcgcacgaagattacttcttcgacttccggtgcgttgatgaacttccgcacgcgctcgcgcgcgccttcgtaggcgtcggtggcgcgcgcggccagttcatgggctgcgcggtggatgttggagttctcgtgcgcgtagaagtacgcgatgcgatcgatgaccgactgcggcttgtgcgtggtggcggcgttgtcgaaccacaccaactgcttgccgttcacgcgctcttgcaggatggggaagtcgcgccgcacggcgtggacgtcgaacggtggatgccggccgctgccggcaatgggtgtggcatcgggcccgcgcggatcgggcttggctggcgtgacgaagccactgggcaggcgcaccgcgtcgacgaagtagaactgcggctgctgactcacctgcggttggctgctgctccctcgcccctctggggagagggttggggtgaggggcgaccccgcaccttggttcgtctgcaggccctcaccccagccctctcccgccagcgggagagggggcaagacctgtggaggggcggacacggcagaagccgcgccggccgacggatgcccgaagctgttgttcaggaagtagaacggcgacgcgcccgtttgcggcgcggaaggcgcggcaggcgcgttgacctgctgcggcacgcccagcaccgaactgccgaggcgcggctcgaaagccggcgccaccgacagcacgctgtccggcacgccattgcccgccaccgcgtgcggcgctaaggccggcgcacggttcgcaagcgaaggcaattgcgtgggcgatgccggcaccaggttggcgccgggaatctgcccttgcgggatcggcgtgccgggcacgctcggcccgaagccggcaggactcgccagcggcgagcccggcggcgcgatgttggcggggaactgcgcccccggcaccagggggttggccacgcccggcaacgcgctcggcggcgtgccgggcagcgcggcgaacatggcgctcgccatgcgcgcgagaacggccggatcgaacggcgcctcgcccggaatcgagggtgtgatgctcactgcggcttacttgtaggtgtcgggatagtcgtggtacttgccgatctcgacgtcgtcgagcacggccagcgcatcggtggtcagcaccgccagcgagcagtacagcgagatcaggtaggacgcgatcgcatggttgttgatgcccatgaaacgcaccgacaggcccgggccctgctcacccgacaggcccggttgaaacaggcccaccacgccctggcgcttgtcgcccacacgcagcagcaggatcttgctcttgccgtcggccaccggcaccttgttcgaggggatcagcggaatgccgcgccaggtgatgaactgcgagccgaacaggctcaccgtcggcggcggcgtgccgcggcgcgtggcctcgcgaccgaaggcggcaatggccagcgggtgggtgaggaagaaggcgggctccttccataccttggtcagcagctcgtcgaggtcgtcgggggtgggcgccccggtcagcgggaagatgcgctgctcttcgctcacctgggccaagaggccgtagtcggggttgttgatgagctcgctctcctggttctccttgatcgtctcgatcgtgaggcgcagctgctccttgatctggtcgtgcgggctgctgtagaggtcggagatgcgggtgtgcacgtccagcacggtgctcacggcattgagatagtgctcgcgcgggttctcttcgtagtcgacgaaggtgcgcggcagctgattttcctcttcgcgcgaggtgcaggtgaccttgatcgattcggggttcctgaccttgttgacgcggtagatgcccgcctccaccggcacccattgcaagaggtgcgtcagccagcgcgggctgatggtctccagctgagggactgtcttggtggcattggctagctggcgtgcggcgttgtcgccaagggcggtggtaccaccgactgttgcgctcatggatcaaggctccgtattgagaagaaagtggccgcaagtgtcaggcggcatggggttttccctcaacaggctatagccgccaagttgatccttcgcacaagacgcgattgctccagctgctcgcagcgcagcagcagacccaccatgttgatgtccagggccgcagccagtttgtgcgccgtgacgatcgaggggatgacgcgcccgcgctccacttcgccgacataggagcggttcaggtcggcctgctcggccagtacttcctgcgaccagcccttgccttcgcgcagctggcggatggtcacgccgaagtcttcgacaaaatccttcatgcaccgactccctgcggcgcgttctgcaggctggcctgcgtcacgctcgcgcccgcgggcacgtcgtcggtgatccacacgttgccgccgatgaccgcgcccttgcccagcgtcactcgtccgaggatggtggcgccggcatagatcaccacgtcgtcttccaccaccggatggcgcggcagacccttcctcgggttgccctcggcatcggtgggaaaacgcttggcaccgagcgtcacggcctggtacaggcgcacgcgcttgccgatgacggcggtctcgccgatcaccacgcccgtgccgtggtcgatgaagaagcctgcatcgatctgcgcgccggggtggatgtcgatgccggtctgcgcatgcgccagttccgccacgatgcgcgccagcagcggcagcccgagcttgtagagctcgtgcgccagccggtggtgaatcatcgcgagcacgcccggatagcacagcagcacctcgtccacgctgcgcgccgccgggtcgccctggtaggcggcgagcacgtcggtgtcgagcaggcggcgcagctgcggcagcgcgctcgcgaaccggcgcaccgcatcggtcgcggcatcgtcgatctcgcccggcgaacgcggttcgtgccgggcgttgaattcgagctcgaggcgtgcctgtgccagcagggcctgcaaggccgaatcgagcgagtggccgacgtagaagtcttcgctttcgtggcgcaggtcgggcgggccgagccgcatcggaaacagcgcgcccttgagcgattcgacgatctgcgcgagcgcatcgcgcgacggaaactcgcgtgcgccgggctcgcgcgagcgccgctgtgaatcgcgccattcgtcgcgcacgccatgcagcgcgcgcacgatgccgctcacctcgaaatgagccatgtggttgttctccctggaaaggaacgctgccgtcagtcctgcacccacggcaggccgtggaagcgccagccgtcggaaccgccgcggtgctggtgggcatcgatctcgccctcgaagccttcgagcacgttgaacacgtgcgtgaagccggccttggcggccgcttccgccgcgagtgccgagcgcttgccgctgcggcacagcagcagcgccaccgcatccttgccgccgtgcttcgcaagcctggcctcgagctcgcgcacaaagcgcggattgcgcgtgagcgccgtgccggtcgcccaggccacgtgcaggctttcgggcacatggcccacgaacttgcgctcttcgcccgagcgcacatccaccagcacagcctgagcaccctgcaccagcgcccatgcgatgggcggcgtcacgccaccggcgtagttccatcccgcttcggccgcatgaacgcgcgcttcctccagtgcgggcggcaagacgacgacatcttcaacttccactgacatgcgcttgggctcctgtgcgttgcttcactcgccatccggcttggtggcgatggccatcactgtaggagcggggcggcgaagctccaacaaccgaaaagtcggttctaaacaaccaactggtctaacgatccaatgcagctccaagcggaaaaaacgcatatcgatagtcgaaggcgtacgttgcggcggcagccacggcctcggtgcaccgaggcggccaccttgccctcgcgcacctctgcgccctgccagggcgcccggatagccgcgcacgcgtgtcaccggggtggctgcaagcctttcgcggcgcgcgaacaggtgcaccgctgcggcgccacttttttaaaccgatacgcctccgcagcaacccgcgcattgctagatcagcggcaattcgatcgcaacgcgaagtccgccccactgcgacgccgaggccgtgatgcgtccttcatgggcctgcacgatgttgcggcagattgccagtcccaggccgctgccgccggtcgcgcgattgcgcgactgttcgacacggtagaagcgctcgaacagcttctccagcttgtcgtcgggcacgccgggcgcgctgtcctcgatgaggatgagcgcggtggcgccgtgccgggcgcagcccacgcggaccatgccggcgccgtccgtgtagcgccgcgaattctcgagcagattgccgaacaactgatgcaggcgcacctcgtcgccgctgacgatcagcggcacctctgcaatctgcagtaccaattgcagcgacgccgcgtcgagccgctgccgcatgctctcggccgccgccaggagcaccgtggccacattgatgggaacccgccagtacgccatggcccccacatcgctcagcgacagatcgtgcaggtcgtcgaccagcttgccaagccgctcgacctccatgtgcatggcgttcgtcgactggatcgaggatgaacggatgccgtcctggatggcctcgagttgggcgcgcagcaccgcgagcggcgtccgcagttcatgggaaatatccgccatgaagccccgccttgcccggtcggcatgctccagcgtctgcgccatgtggttgaagtcacgcgccaacgctccgagttcgtcatgcgctccatccgaaatgcgcgatgcgaagtctcctgcggccaggtggtgcgtggcccgggccatatcgcggacccgccgcaacagagtgcgtgcgagcatgaatgccagcaaagccgccacgaggatcgatccgagtccgaccatcgtcaaggcagtgaactggtgttcgagaaagcgcttgtcgttcttcggaatcacggcctcgaacggcaccgtcgcgatccagcccactgtccgtccctcgaccatgatcggaacgcggatcgaattggtgtcgatgctcggattgccgatcacccggcgcatctgtgcatccagcaggcccacgcgcgtaagtgcgccggtctgatcggaagaagccagccgagacgcaggatcactctctgtttcgccaagaaagggcaacatcaggttcatccactcccggaagtcggagcgcaggaagtcccaactgccacgaacggcataggcttgctccaggcgtggaacgatctcttccagccgcgtgcggctttgctggttgaggtagcccaggaagccgcgctccatcacgagccgcatggcgatggcctgcaccacgaccactgcagcgcaggccagcagaacgaacaggaagagctttgctcggatgccgaatttcatgtgggctggaggtctgccggtcaggctacgcgtacgaggagccgcgatccaccgtcatcctgcgggcttgccggccgatgcgtagccacccaggaacacctgcacggcgcggcgcgttgcctcccgcagttctttgcgggtcaacggtccctggatgcccaggagactcggcctgacggtttcagagtccagcagcgccatcaggtggtttgccgccgtggcgggttcggccgttcgcatgcggcccttgcgcatctgccgctccaggaaacccgccagctcggcgatgcccttcttggggcctccttcgaagaagagccgcccgatgtcgctgcggccggattcggcgatcacggccctgtgcgcctggatgacctcttgcgagcacatcgcggccaggaccttctcgccgaaccgctgcagcacgggctccaggtcttcatcgccctcctcggccagcgccgcgaagatcggctcgaaatggctcttcgccgaggcgtggatcaccgcgacgaacagctcctccttggagctgaagtagccatagagcgtggcgcgcgaaccgcccaggcgggcggcgatctccaccatggaagcgccttcgaaccccagttcccgaaagacctccgacgccacctgaacgatggcatcgcgcttggcttctgttctgactcgcatcgggtcccctatttatttctgtacatgactgctcattattgattgacatctcctggaagtcaaaatacatttctgtacagcactgtatatttaaacgcggaccgaccttcaaaccgtcgttcggtcatctttcaggaaccctgtcatgcgcccctctttcacctatagcctgacctttgcctcggccctcgtgtccacctgcctgctcgtcgcctgcggcaagccgccgggcggcccgcccccggcgctgggcacgcccgaagtcggcgtggtcactgtccagccgcagcgcgtggcgctgagcaccgaactgcccgggcgcaccgtgccattcctcattgccgatgtgcggccccaggtcaacggcatcgtgaaggcgcgcaagttccgcgagggcagcgacgtgaaggccggcgagccgctctaccagatcgatcccgccacctacaaggccacctacgacagcaacgtggccgcgctggccaaggcggaagccagcctcaagaccacccggctcaaggccgagcgctacaaggagctggtggccatccaggccgtgagccagcaggactacgacgacgctgccgcctcgctcggccagggcgaggccgacgtcgcatcggccagggcgaatgtcgagaccagccgcatcaacctggcgtacgcccgcgtggatgcaccgatctccggccgcatcggcaagtcgagcgtcacgccgggcgcactggtcaccgcaagccaggccagcgcgcttgcgaccatccagcagctcgacccgatctatgtcgacgtgacgcagcccagcgcggcgctgctgcggctgaagcaggcaatggcccgcggcgagctgcagaaggccggcgccaacaccgccaaggtgaagctgctgctcgaggacggcagcgcctatccgctggagggcaagctcgagttctccgacgtgaccgtcgaccagaacaccggcgccatcacgctgcgcgcggtgttcccgaatccggacgccgacctgctgcccggcatgtacgtgcgcgcggtgctgcaggaaggtgtgaaggagcagggcctgctggtgccgcaacaggcggtctcccgcggcagcacgggcaagccgaccgcctacgtggtgggcaaggacaacaagctgcaactgcgcgccctggagaccgagcgcgccgtgggcgaccagtggctggtgagcagcggcctgcaggccggcgagcaactggtggtcgacggccagcagcgtgccgcccccggtgccgaggtgaaggtggtggcatggaaggccaagcccgccggcgcaccggcggccggcgcgcccaagagcacggctcactgatcggcgaaagacatccatggcacgttttttcatcgaccgcccggtcttcgcctgggtcctcgccatcatcgtgatgctggcgggggcgctctcgatcttcacgcttccgatcgcccagtatccgagcatcgcgccgcccgcggtcgccgtcaccgccaactaccccggcgcttccgccaagacgctggaggacaccgtcacccaggtcatcgagcagaagatgaaggggctcgacaggctgagctacatggcctcgaccagcgagtcgtcgggctcggtcaccatcacgctgaccttcgagaacggcaccgatcccgacaccgcccaggtgcaggtgcagaacaagctttcgctggccacgccgctgctgccgcaagaagtgcagcagcagggcgtcaccgtcaccaagtcggccaccaacttcctgaacgtgctggccttcacctcggaagacggcagcatgaacggctccgacctgtccgactacgtggccgccaacgtgcaggacgcgatcagccgggtcgaaggcgtgggcgacaccacgctgttcggctcgcagtacgccatgcgcgtatggctcgaccccgacaagcttgccaacttcaacctcacgccgatcgacgtgaagaccgccatccaggcgcagaacgcgcaggtctcctccggccagctcggcgggctgcccgcgacaagcgaccagcagatcaacgccaccatcacctcgcagacgcggctgaagaccgcgggggagttcgagggcatcctgctgcgcacgcagaccgacggctcgcaggtgcgcctgcgcgacgtggcccgcatcgagctgggcagcgagtcctacggcacggtcggccgctacaacggcaagcccgccgcgggcctggcgatcaagctcgccgcgggggccaatgcgctcgacacggtgagggccgtcgatgcgcgcgtggccgagttggagaagttcttcccgccgggcatgaaggtgcaaaagccctacgacaccacgccgttcgtgcgcatctccatcgaggaggtcgtgcgcacgctcatcgaggcggtggtgctggtgttcctggtgatgtacctctttctgcagaacttccgagccacgctgatcccgaccatcgcggtgccggtggtgctgctgggtacgttcggcgtgctttcggccttcggcttcaccatcaacacgctgaccatgttcgccatggtgctggccatcggcctcctggtggacgacgccatcgtggtggtcgagaacgtcgagcgcctgatgacggaagaggggctttcgccgaaggaggccacgcgcaagtcgatgggccagatcaccggcgcgctcgtcggcgtggccctggtgctggcggcggtgttcgtgccgatggccttcttcagcggctccaccggcgtgatctaccggcagttctcgatcaccatcgtctcggccatgacgctctcggtgctggtggcgctggtgctcacgccggccctttgcgccacgctgctcaagccggtcgccaagggccatgcgatggcgagcaccggcttcttcggctggttcaaccgcaatttcgaccgcggcaaccgccgctaccagggcgtggtgcgccacatgctgggcaagggctggcgttacatgatcgtctatgccgtgctgctggcggccgtggtcttcggtttcatgaagctgcccgtgggctttctgccggacgaagaccagggcacgatgttcgtgctgatccagctgccgccgggcgccaccagcgcgcgcaccgaccaggtgatccatcaggtggagcatcacttcctggaggaccagaaggatgcggtgtccggcgtattcgcggtgtcgggcttcagcttcgcgggcagcggccagaacaccggcttcgccttcgtcaagctcaagccatgggacgagcgcccgggtgacgcactgagcgtgaccggcgtggcggccaaggccggcgcgttcttcgcgaccattcgcgatgcgaaggtgttcgccttcgcgccgcccgcggtggcggagctcggcaatgccaccggcttcgacctgatgctgcaggaccgggccaacctcggccatgccgcattgatgcaggcgcgcaaccagctgctgggcgaactgtcgaacgacaagcgcctggtggccgtgcggcccaacggcatggaggacacacctgagttccgcctggaagtcgatccgcacaaggccggagcgctcggcctttcgatggccgacatcaacaacaccttctctaccgcctggggcagcagctatgtcaacgacttcatcgacaagggccgcgtgaagaaggtgatgctgcaggccgacgcgcaataccgcatgctgccggaggacatcgaccgctggtacgtgcgcaacagcgccggcaccatggtgcccttcacctcgtttgccaaggcggggtggacttctggctcgccgcggctggagcgctacaacggcgtgccgtcggtggagatcctgggcatggccatgccgggttccgcttcgagcggagaggcgctggccatcgtggaagcggcggttgccaagctgccgccgggcatcggctacgagtggaccggcctgtcgcgccaggagaaggcgtcgagcggacagaccggcctgctgtatgcgctgtcgatcctgatcgtgttcctctgcctggccgcgctctacgagagctgggccatcccgttctcggtgatcatggtggtgccgctgggcgtgttcggcgcgctgctcggcgcggtgctgacctggaagatgaacgacgtgtactttcaggtgggcctgctgaccacgatcggcctggcgtcgaagaacgcgatcctgatcgtcgagttcgcgaaggagctgtacgaaggcggcatgagcctggtggagtcggcgctgcaggccgttcgcatgcggctgcgtcccatcctgatgacctcgctcgccttcattctgggcgtgctgccgctggtgctcggcagcggtgccggcgctggtgcccagcacgcgctgggcacggcggtgatcggcggcatgctgtccggcaccatcctggccatcttcttcgtgccgctgtttttcgttctcgtgctgggcatgttcaagcgcaagcccgctgagccggcgtcgcccgcatcccacacccctgcgtctgccgccgctgcttcggaaggtctctgacatgaatcgcttcaccttgacttccgtgacgcttgcggcgctgctgctcagcggctgcagcctgatgcctgcctaccagcgacccatggcgcccgtgccccagaccttcgcaggggacaccgcggcggccgctgccgcgccggtcgccgagatcggctggcgcgacgtgttcaccgaccccgccttgcagcgcgtgatcgagaccgcactggccaacaaccgcgacctgcgcgtggccgcgctgaacatcgaaaaggcgcgagcccagtaccgcgtgcaggatgcggcgctgtttcccaccgtcaacgccagtgccggcggcaacggcagccgcacgccggcggacctgtcggccagcggcagtgcgcaggtttcgcacagctacagcgcgtcgctcggtttcagcgcctacgagatcgatctgttcggccgtgtgcgcagcctcaatgcccaggcgctggagcagttcttctccaccaccgaggcgcgccgcagcacgcagatcagcctggtggccgaggtggcgacggcctacctcacgatggccgccgaccaggaccggctccgcctcgcgcaggacacgctcgcgagccagggccgcacctaccaactcaaccagcgcagcttcgaactgggcgcggcctcggcgttgacgctgcgccaggcgcagacgagcgtggacaccgcgcgcgtcgacgtcgagcgctacaccgcgcaggtggcgcaggaccgcaatgcactgaggctgctcgtgggcgccgaagtgccagacgaactgctgccgcatgccctgcccaacacggcggcggcggccgcaagcccgctggcgaccattccgccgggcctgccttcggatctgctgcaacgccggcccgacatcctgaaggccgagcgcgatctcaaggcggccaatgccaacatcggcgccgcgcgcgccgcgttctacccgcgcatcagcctcacggcctcggcgggcagctcgagcgcaagcctgtcgaacatgttcaccggtggctcgcgcagctggagttttgcgccgcagatttcattgccgatcttcgatggcggtgcgaaccgggccaacctcgacatcgcacgcaccgaccgtgacatctacgtggcgcagtacgagaaagccatccagacggcttttcgcgaggtgtcggacgcgctcgcacagcgcagcacgctgggccggcagctcgacgcccagcagtcgctggtggacgccacggcggagagctaccggttgtcggacgcgcgcttcaagcgtggcgtcgacagctacctgagcgtgctcgacgcgcagcgctcgctctacaccgcgcagcagaacctcatcggcacccggctgtcgcggttcaccaacctggtgaccttctacaagacgctgggcggcggttggatggagacctcggaaacccagagcgcatccgcacgcaccgcggaaccggcgccgtgagacgcaatcgcgcagccaccgaaatcacccgcacccgggtgctccaagccgctctggaagcctttgctgccagcggtgtgcgcgccactacgctggaaaatgtggcgaggctcgctggcgtgacgcgcggcgcggtgtattggcacttcgagaacaaggccgcgctggtggccgcgatcatcgatcagcttcgatggccgatggacatcgggccggacatggtcgcctatcaggcacacccggagccgctccaactcctgcgagagcaaatgtggcgacaaatgacccgttgcatggaagatccagatcaatggcgcgctgcccaattggtgcttcggcacccggcgcagggcgagttgcctgtcggcgtggtgactcggattgggcgcacgatgggagacacggtggcacgactgagtcgagtgatgactctggcttgcgagcgtcgtcagctgaaggagggacttcggccggcttgcgtagcgcgctgcctgcattcggtgggcatcgccgttcttgccgagcatgccaatcaacgggaaaaacgcagacggcgtgcatcgttgttgttgtgcatcgacctcttcatggccggggcctgcagcgatgctcctgcgattcagtcgtgagctgcgctcggctgtggcgtcgccggcctgatcctggccgacccgcctggggcaagcactcggtgccactgggcgtacccgaaggctgcggcacagctctgaaggaccatgatgaacattcagaagagtaaaccgaagccatacggcccaccgagatggtgggagaccatggcaggcgcgcctttggcatatttcatggtgctgggcgccttatttctggcactttttcttttgaggaatctactcggggcttaagagcctcacctcacctcggcacgaatgtcgagaacgccagatcgcgtcgatgcgccggtcgaagcgatccagcttgcggccaccactgcgcgccttccgaccgctcgccatgatgacgcgggcgagtgcgctacactatttttcgcccctgctgcctccggctgctcctcgaaggagtgccgcccctcgatacgtattcacactatcgacagtttcgctcctgtggacacgtctcaaaagcgctcgaagcaccgctcctctgctcaggccgattcgcccgaagatcaaagcgatgtcgatgggcgcttgttcgtcggttcgatggagaagggaatgcgcgtcctcgaactgttcaacgaacatccctccaccctttcgatcggcgacattgcggagcacacaggcatgggccgcagcgcggcgcagcgtttcgtctacacgcttcaccggcttggctacctcagcagggacaatgagtcgaaaaagtacttgccctccctgaagctgctgggcctggtgcgcggcatccatcgccatcatccgcaacgagagctggcgtatccactgctcgagaagctcgcaagggagacgcgcgagacggtgtcatgggtcgaactggacggagacgaggtggtcgtgctgctgaacatccccggatcgcacatcacggccatcaatcttccggctggaagccgctttcctgcgctcacctcttcctccggccaggtgcttctctcgcaagctccgcaggcacagctgtcgaagatgcttgacgccctgccccctgagacgcgggcccgcttcggcagccgcagccgctccgaggtgctctccattttccgcaaggcggcggaagacgggcattcattcaccgagaagaatttcggcgatgacggcgtgtccgtgtccgtaccggtgacggatttctcggggcgccccatcgccgccctcaacgtatcgaccgtacgttcgcgctacagcatcgcccaggtgcgcgaactgatactcccccggctcgaactggcggcacgcgaagcctccatctgagcgcggggctcgcccccgctgcccatcccttcttttcttctggctgccggatgtgccgaccgtcggttcgagcgccgcatccggggtggtgcgcgtatcccgtacttgacgtggtgagacataccgccgaagattaaattgaaatgcaagtttgataattgcatatcaattatcaagatctttcggtttgccttctccagcagggaacaagatgccgcaaggaacccttttgcccggatcggtcgccatggcttcgctcagcgaggagaccatcggtgagttgctcgctcgccgcgcccgctcccacccgggagacatctattgcaccttcagggacgagcgcgtcagcctcgggatgctcgaccagcgtgtgaatcaagtggccacgctgctgaagtcgcaaggtttgaaaaaaggcgaccgggtcggcgtcatgctgcccagccatcccgatcacctctacctgatctttgcgctggcgcggctgggcatggttcgcgtaccgatcaacgtgcacctgctgggcgcgccgctggcccacctcctcgacgagctcgcgccacaggccatcgttgccgacggtgcctaccgtgttgcgctcgaagaactcggaagcgacctgccccaggtgatctggcgcaatggcatcgacggggagttcgatcgcttcgccctctgcgatcaggacgatgccgcgcccctcgtaaaggccgacgagatcattgccctcagtccgagttcgggcaccaccggcgcacccaagggcgttctgaagtccgaccgccatctgcgtgccgggcccatggccatccttcgcctgacagaggccggacccggtgacgtctttctgttctgggaggcgctccaccacggctccggggtggccgtcgcgattgccgcactgatgggaggcttccagctggcaatgctggaacgcttcagcgcttcgggattctggggcgacgttcgccgccaccgggccacgcacatccattacctgggcagcgtgctgccgatgctgctgaagcagccggagcgccccgacgaccgcgaacacggcgtgcgcatcgcctggggaggaggctgccccgccgatgtgtggcacgcatttgccgaacgtttcggcgtgtcgatgcgcgagggctacggtctctccgagctgatcaccttcgtgaccgcgaacatcgatggcccgccgggctccatcggcaagccgctgtcgtactacgagatctcgcttctcgcggacgatgggtcaccggtcgagccaggcgacaaaggcgagatcgccattcgagcgctcgatccgagcctcggcttcctgggctacttcagaaatccgcaggccgatgccgccgcgcgccgcggtgagctgttcctcagcggcgatctcgcgcaccgcgatgcgaacggcaatctcttctacgcggggcgcaagaaggacatgctgcgacgccgcgggatcaacatcgcggcctgggatgtggagagcgtctttgcgcagcacgatgcggtggccgaagtggcattggtcggtgttcccagcgagcttggcgaagacgagctcaagctgttcgtgcgcctgcgcgaaggggccgacatcacgccgctcgacctgatccgctggtgcagcggcaagctgccgtacttccagattccacgctacgtcgagttcatcgacgccttccccaagacaccgactcagcggatccagaagaaggaactgtctcgcagcctgaccggtgtgtgggacgccgacgccgccggctttcgcgcggtcaagcactgactcccaaccgattcaaggtctccgtcgatttccccgattgctcaactgaaaggaaaagtcatgatccgagttcgcttgaatcgctggcgtcaggcgatggtgatggtttccggcctcgccttctgcgcatgggcccaggccgccctcgctgacaagcccatcaccctggtcgtggcctttccggccggcggcggtgtcgacgtggtcgggcgcatccttgcgcagggcatggcacagaagctgaagctgtccgtggtggtggacaacagggcgggcgcctccggtgcgatcggggcgcaattcgtcaagcgggcggcgccggacggccacaccctcctcatggcaccgaccacttcttacgtcatgtcggaaaagatgtccggcgccgaggccgtcggctacgaaatcgccaaggacttcaggccggtggccacggtcggtgagctgcccttggtcatgctcgcgtcgaaggcaagcggcatcatctcgtacgcggacttggtcgccaaggccaggcagcagccgggcaagctcgcctacggctcgtcgggcaacggctcgaccgaacacatcgtcaccgagtggttccgccagcaagcggccattgaactgctgcacgtgccctaccgcggttccgcgccggccatggccgatctgtttgcgggcgagatccagttcatggtgaccacctcgcccaccgcgctcaccaacctggcctcaggaaaggtggtggccgtgggcgtggcaagcccgcagcggctggacatcttcccgggcctgccaacctttgcggagcagggcctgccgcagttcgttgccgcctcggtgtatgcggtgctggcgcccaaggggacgcccgatgacgtgatcgccacgctgaatgcggcgctcaacgagacactggcagacgaggcggtcaagcgccgcttcgcgcagattggagtcgaggctgttcacagcacgcccgcccaggcgcgcgaccggctgcagaacgaatcgaccaaatgggagcaggtggtgcagcggatcaaggttgcccgctagaaccccacacgcatcttggagccaaccaatgactgaaacgctttccgcaaaaccttgcgtcactctcgccatcgagaagggcgtcgccttgatcacaatggatcgcccgaacgcgatgaacgcgttcgaccgcacgcagcgcgaactcttccagtccgcccttctgtcggccgacgccgacgcgggggtgcgcgcgatcgtgatcaccggcgccggcagggccttctgcgcgggccaggatcagcacgagagcgctgccatggacgcggcagggtcggccgcgcggatcgacagctacatggccctgtacgaggtgtttcgtgcgctcggcaagccggtcatcgcacggatcaacggcgtggccgccggcgcaggactgcagatcgcgctcatgtcggaccttcgcattgcttcaacccaggcgcgtttcggaatgaccgagttcaaggtgggctccgcagccatcttcggcagcaccttgctgaactccatcatcggcgaggccgcgatgaagcggctcgtgctgctcgccgagatcgtgccggccgcgcagtccctggcgctcggcctggtccacgaagtcgtggatgacgcccgcctggacgagcgggtggcagaaatctgcgcgcaggtgtcgcaatggtcgccaacctccgtggccatcaccaaatcgtggtggaaggagatgggcgacgagatgttcgccaaggccgcaaccgctgcccggcgtgggcacgccatcaattttgcgtccggtgcctactcgctcggcgccaggaaattcaccgagcgcaaggcgaagccggccagcccgtagccacgcggcacagcttgcggcgtacggcataggagtcttccggtcgccgattgcccacgaccggcgctgcaaagtcttcagcacggtgcgatggcactatgaatcaaccgcggccgaccgaccaggtccagacaatcagcatcatcagaaccagcgcaaggccgctgagcgagaacgcgttctcgccaagttctattgctggcatcagtgccttgccgatgttgtacgcagccacggcatacgagatgcagacgatgagccagcccagcacccggcggtagcggcgggcggcagcctgcccgtcggtgcgtcggtcgatgctgcagatcagccggccgtccagcgtgtcggtgatcatcatgccggcggtgaagaccaacccggcggcaagcgcagcggacaggccgccgccgcggtggctggccacgtatccccaagccgctgcctgcgtcgcagtgtcgaacaccgtggcgaacaatacgcccgtcagcaccaccgcccacgggctggcgtgcaggcgcaggcgctgcgggaccagctttaatttccatccggcaggcgcgaaggcaacatcgcggcgccgcaggaggcgcaggttcatcgtcccgaccagcacaagcagcaccgtgggaatccagtcgaacaccgtcaccagagcttcaggcacgcgcacgtcatgagggagctggctcacccccgctgcgatcgcggtgacgagcaacccgtggccgagcgcgaacaacgtgccgatccagggcgcgtggccgtggtgggcactgcggtccagagcctgccaggtcaggccgtcgatgcaggcaatgtggtcggggtccaacccatgccgcagccccaaagcgaacatcaggaccaagcccgaaaaggacagccactcggtgctcattcatggctccgcaaaggcggatcggccaggactccggccagttcgcgttcagtcaccacctgctgccgctccagaacctgcagcagcgccccgaagaaccgctcgtagtagtcccacggcggctgcgccgcgcaatcgagccgttcccaatcgccgatcgattcgatcaggtgctggcggaagtcttcccagtcgaagtggccctgcttggccaaggccagcgtcaacccgaagagctggcgttgccaggcctccgcaaagaacagcttgccctggctgcgcggcggcgagtcggcatggcccagcatctgagaggccgcatattcctcgaagcgagtgaacatggcaccccgcctcaggccgttgtaggcggcggtaccagcgcaacgcccatcatcgcctccggcgtgaccagcgcagccagctgctcttcgctgaagccgtcggtgtttgccggccgctcgggcacaacgaaccagcggatctgcgcgctgctgtcccacaccttcacttcgatgtgctcgcttatcggcacgccgaactcgcgcaggaccgcgcgcggctcgcgcacgcctcgcgcgcggaacaccggatccttgtaccagtagggcggcagcccaagcaccggccacggatagcaggaacagagcgtgcagatgatcaggttgtgcacgcccggaccgttggccactgcggccatgtgctccccctcggcgccctccatgcccaatggcagctgaagttcggcaatggccttgggcgtgtcggcgagcaggcgctgcttgtaggcgggatcgacccatgctcgcgcaacgattcgcgcgccgttgaacggtcccgcggtcttctcgaaatgatcgagcaccgcatcgaccgaatcgctgccgatcacgcccttctcgatcagcagggcctccagtgcgcgcaccttcgcggcgctcgctgcttcgcgctcttcgttgtacttgaacagatcgctgctcatggcgttttcttttcctcgggcgttcggcattgcaggtagacctcgaagaggtcggcgtagatcgtcgtgttcggttcgcagaggtcggggccccagatgtcgcgcgcatcgaacgcgacgcggtacaccggcatcggtccttccagcccgtcaggcccggtcgaacagaaatactcgaaggcaccctggtacacctcgcggacagtgcctttcttgttgcgcaggtagccgggtagccgcgtgtggtcagccgccgccgggtcggccacctgcaccgtctgaccgagcgtgaaccgcggcgcatgcggcaacggccgctggctggagtcgccttgcagcagatagtcgacgatctgatgtttgatcggctcgctgggccgctcgggcagtggcgcgtcgggctggacgcgatagtgcgcggtccaccacgccagctcttgggcggtgatgtagccctcgtcgacaaaaaactggctgatgcccatcagccatttctcgtagtagcggaacttgaagtactcgaagggctgcatgccctcggcaccagtgcgcagcgaggcccaggtccaggtgtgcttgaacgtggtgggtaagctggccatcggatatctgggcaatgcctctgcgaggtgggcgctctcggccatcatcaccgtgtggatgccaaagatgcgcttctcccactcctgcacgaagacccgggtttcgaggctcacaggcccgaggttctcgaggccgcccagcgcatgctggagtttcatgggtgctccgtttcggattccatggcacgctccagcgcccgatcaggttgaaccgcgaggcatccgaggaagccctcgcgcaaggcgtccgccgcaagttcccgcccgatgaagaccaacttgctgcggcgcggctcgtcggggccccaccgccgtccaggccgcgcgtcgagcagcatgtgcacgctgtgacagtggaactgacgcgcctcgccgtcgaagtgaagcacgcccttcgtgcgcatcagccctgcgccttcgcgttgaacaagctggttcatccaacggctgaaccggtccgggtcgatggcgccgtcggtttccacgcagcacgagccgatcgaggtgtcgtgctcgtggtcatgagcctcaccgtccagcagatcgggctcgatcgacaggacgtgcggcagcgagaagcgcctcgtgcccagcagctcggcggccgggacccgcgcgcgctccgtcctgaccagatgtgcggccggattcagccggcgcagctcacgctcgagttgctccagcttctgcgcgcggggaatctcgaccttgttgagcacgatcacgtcggcgaaggcgatctgctcgcgcacgatgtcgtcgccgatgtgaatcaggatatggtgtgcatcggcgacggtgatcaccgcctcgagttccacgcgttgcaacaggtcagcatcggcgagaaagctctgcagcaccggcgcgggatcggccaggccggaggtctcgatgatcagccgctcgatcggacgttcggcgcgttggagcagctcgttcaccgccgccgtcaggtcctttcgcaccgtgcagcagacgcagccattggtgatctcgatcagcggctggtcatcagcgacgatcagctgcccgtcgatgccgacctcgccgaactcgttgacgatgatgccgatgtaggtgccgctgcactgcgccagcaggtggttcacgagcgtggtcttgccggccccgagaaagccggtgacgatcgtgacggggatcttggcgggagccatggcggtccgggctactgttgcgacgcagcgagcttcgaagcggcatgcggcgtttccgttgtggctatcggctcgcgcatgtcgagcccccggcggtcacggatgcagatcgctcctataaccagcgtaagcagcgatacgccaatcgtgtagatgaggccgcggaagatatcgccgctgctcacgaccatcgcagtggcgatgaacggcgcgaagccgccgatccagccattgccgaactgcagagccacggagacgccgctgtatcgcacctgcgttggaaactgctcgaccaggaacgcgcccatcgggccgtacaccatggtcgcgagcagcaccagaatgaacagcatcagcacgaccattggggcatccacgcgtgccggatcggccgtgagcggcatgccgcgctcgaccagcacgcggcgcagagccgcttcatcgaaaccggtcagcgtcgtttcggcgaccacgaactgcagctcgcctgcctgcggccgcaacgtgtacggcacgccttgcgcagccaggaacgagcgggcgcgcgtgcacggcttggtcgccttcggctggaacagctggccgacgaaggactggtcctcacggcagtcgccgccttcgatgacgacctgggtgctggcgcggaactcctccagggccggattgccgtacttggccatgccctggaaaagcggcatgaacaggattgcggaaagcaggcagcccgtcagcatgatccacttgcgcccgatcaggtcggacagccagccgaacagcacgaagaacggcgtggccagcaccagggcgatcgtgaggtaggcgtaggcggactgcggcggcagcttgagcgtcgcggtgaggaattgcaggctgtagaagtgcgcggtgtaccagatcaccgcctgcccggccacggcgccgaagatcgttaccagcacgatgcgcagggtgcgggggttgccgaaggtgtccttgaccgggttgcgcgagcccttgccgtgcgccttcatctcgaggaacaccggcgactcctccagccgcatgcgcacgtagagcgagtacgcgagcagcccgatggacagcaggaacggcacgcgccatccccacaaggcgaaggactcgacggacatcgacgagcgcagcatcaggatcacgcccagggaaacaagcagtccaatggtgccggtgatctgcagccagctcgtcatgaagccgcggcgccgcggatcggaatgctcggcgatgtaggtgaccgcaccgccgaactcgccgccgattgccaggccttgaagaagacgcagcagcaccaggatggcgggcgcggcccagccgatggtttcaaacgtcggcaggaatccgatcgtggcggtggcaatgcccatgatcatcatcgtcaccaggaaggtcttcttgcgcccgaccagatcgcccagccgcccgaagatgatcgcaccgaagggcctcagcacgaagcctgcgccgaaggtcgcaagcgacgcgagaatggccgccgactcgttgcccttcggaaagaacaacccaccgaagaacacggcgaggctgccgtagatgaaaaagtcgtaccactcgaatacggtgccgagcgcggcggcgaagaccactcggcgcgtttcacgcgaacgctcgggcgtggcgggggaagtctcaactgctgttgtcatgtccatactccttgatgtatggcggacgcgcgtcaagcgccgctccgcttgtcgatgcgggcgatgaagtcgcgcaggatcgcattgaaactctcgggctgctcgagcatcggaaaatgcgcggcactgggcaccagcttcagtgtcgcgccgggaatgccggcggcgagcgcatgcgactcagccggcggcgtgatggcgtcctcctcgccgcagacgacgagcgtcggcaacgccaggcttgcgagttgcgcgcggctgtcggcctcgttgagcgaaacgatggcttcgcgggcgacgaattccggcgtctgcgccacctgttcgcgcgcgaaggccaccagctcggccgaggcggcggaggcgaacgagcggtcgatcaccgcctggctcgccgcaatgacacccagggtgtcgatggcgtgcagcacattcttcacgttcacgtcagggccgagcccgtgcggcgtggcgcccaccagcaccagcgcgcgcaagcggctcgggtgcgcgagcgcgaaacgctgggcgatcgtgccgcccatcgacagccccacgaggatggcatcgtcgagatgcagcttgtcgaacagcagcacgaggtcgttcacgaacgcgtcgatcgtgtagcggcgcgagcgtggtgatgccgagcggccgtggccaggcagatcgggcactaccaatcggtggtcgtgcgagaacgcgcccatctgctggcgccagaactccccggtcgtggtgaagccgtggcaaaagacgagcgccgggccgtggcccgccacgcgcacgtgcatgtctccgattgaaatgatgtcgttcatgtgcatttccaggtgaaaggacggaagccgccgcgccgcttcgactgcgggacggagggcacagagcaattcggaggcccgctcgaccgacctcttcgcaatttcgacaagtgcttgatttgcttggacaaatgctcaacacggctttgattgacggcttggaacccatgccttagtctcagtattgagtcttaatgtcgcaactacgagacgaaaaatgccctttcccgaatggttcggctccggccagaacgaggcagagttcctgcgccgcgtgctcgaccatgtgtccgactgcctggtggcggtcgacaccaatggccgcgtcgtgctcatcaatgcgccctactgccgcctgctgggcggcccccaggaagacttcatcggccgacacatcaccgatgtcgtgtcgccgaagacgcgcctgcaccacgtggcgcgcggcgacctctccgtgaccatgatgccgctcgaagtgcggggccaccagttgctcgcgcggcaggtgcccgtctaccaggacgagcgaatcattggcgctgtcggtctggcgctcttctccaacatggcggcgctgaaaaaggcggtcgctgtcgtcggcgaccaggggcgcgccatccatagcccgcccacgccgtggaccgcgcgctacggcctcgacgacatcctgggccaaggcgcccggatggacgcggtgcgcgcggccatcgaacaggccgcgccgctctcgctgcccgtgctcgtccagggcgagaccggcagcggaaaggaactggcggccaacgcaatccacgcgctgtcgccgcgcgcccggcgtccgttcgtgtgggtcaactgcgcgtccattccggaatcgctgatcgatgcggagctcttcggctacgaaggcggtgccttcaccggggcgcgaacgcgcggcaagcccggcaagttcgaactcgcgagcggcggcacgctgtttctcgacgagatcggcgacatgcccctcagcctgcaggccagcctcttgcgtgccgtgcagaaccaggagatcgtgcgtgtgggtggcgtatcgccgatcccgatcgacacccgcgtggtctgcgccacccatcgcgaccttcaggagcgcgtgggcgcgggccagttccgggccgacctgtactaccggctcaatgtgctcggcgtgcacatgcccgcgctgcgcgagcgcgacgacctggagtggttggccgagcagttgctcgagcgcatcgcgctgcgcgaaggcctgccggggcgccgtgtgccctcttccgttcgcgcgcgatggttggccttcgactggccgggcaacgtgcggcaacttgaggctgctctgctgcgctttctgctctcgggcgagcccgggctgccggaagtgcccgccgcgaagcacccgcaggccgttgccggccagcggggaacaacggcaacgaccacgttgcaagcacaccttgaccgcgagcgcgatgcctgcatacagaagacgctcgcggagaccgccggcgacaaggacgaggccgcgcgccggctgggcatcagccgcgcgacgctgtaccgcgagctacgacgctcgaccgagtcgatttgacgagcccggccttattgcccgaacacgtcgcggatccgcgttccaaggagccgctgtcttcgggcttgtagctgcgcccaattcttcgagaagaatgatcttgaagcgagccttcgactctcagcggccgggcgacggtgccagggtgccctcctccccaaggtagctgcgcaaacctccaaggtcgatcacctcgacgccgccatgctccacccgcagcaagcccgcgcgctcgagttcatgcagtgccctgttggcgcgctggcgagagacggctgacaagagcccgatctcatcctggctcaggcgcacgaaggtgctcgcctgcggataaagaatcggatcgaacagactggccaggcagcgtgcgacacgcgcgtcggggcccagcaagcggtcgaactccatgagcccgatgaacaggctcaggcgagcgttgatgtgcgacagcaggaaccgattgaagccgaggttcgtcgacaccaggcgctcgaaggtgtggcgcggcacgcaggccacgcgcgtcgggcgcatggccacgccgtcgtagcgccacgggccgggattcagcagcgagccttcgccggcccagccgccggaggtcacgccggtgaaagtggagacgcggccatcggcctgcgagaccgacatcttcacgaggccttcgatcacgccgaaccacagatcggccggctcgccctggcgcatgacaaagccgccaaccggtgcctcgcgctcatgcgattcgcgcaccacgcggtcgagctcctcggcggtcagggtctgcgcccacaagctctcgcggagcatggtctccatggccttcgacggcatacgtgcttcccactcgcttgttggttgctcgctcttctgcgcgccgggcctcgtggggaggccggcgaacacgcccgtaagtaatgtctctgaaacgacatttttggcgcggcgatcatgacatattgactcctgttcgccacaaccagaagacaggagacaaggatggaacatccggaatccgccgcgggccccgcgagtgcaccgcatcacgatgatgaatcgcccggcatgcgcaggcgcaatctgctggggtacgcggcttccgcgcccctgctgtcagccgtcgccggactcggcgggctggcggcgccctcgtcggccaatgccgcgatactgccgatgacgccacccgacacgaccgaccagctcgacatcggcgatgcagtgacggtcacggcgctgccgaccatgccgcttgtcaagatcagcaacatcgggaacggccgcgtccggctggagcttccgcgcttcgaatcgggccagggcatcgccaccgccgccgccatgatgctggcggacaagctgggtctgccgctgaacgcgatcgaggtcggctccgccgacgccagccccgagctgttctacaaccagctcaccggaggctcgtcgagcgtgcgttcgctgcatgcgggcatgccgttgctcggcggtttgggtgggcagccctcgggctccgggagcgcggtggtcggccaacgcgtgacgcggctcgacgcgctggacatcgtgaccggacgcaagaagttcacgctcgaccaggccgtgcccgacgcgaagcccaccatggtgtgccggccaccgaccatcaacggccagttcgttcgcatcaacaacacgaccgcggtgatgggcatgccgggcgttctgggcattgcgccgattcccgccacgaacggcatcgtgcccacgccgcccggcgtggcggtgatggccgaaacattcgggcaggcctgggccgcggtgaatgcgctcgacgtcacctggagcgcaagctcagtcgccggcgagtccaatgccagcatccagcagaagctgaaatccgcgctgctgcccttcctgctgccgccgctgggcgcgctgacggtcgagggagagttcgagttcgcggcggtctcgcactgcccgatggaaacggaatgcgccatcgccgatgtgcgcgccgaccgggcggagatctggtccggcctgcagagccccatcgtcacgcagcaggcggtggcagccgatctgggcttgccgctggacaaggtcaaggtgcatgccgtgccctcgggcggctccttcgggcgccggctgttctgggacgcgacgctgcaagcggtacagatctccaaggcgctgggccgcccctgccgcctgatgtaccaccgcaccgacgacatgcgccacggccgcgtgcgcccgcccatgttccatcgggcgcgcgcgacgatgctgctgggccaggtcatctctttcgagcagcgcatcgccggcgtgcggctcgatacgcgccatggcttcggcgagatgctgggggccgcggccatcgcgctgcccaatggctttccgcagacggtgggcaacttcgccgtcgagcaaaccatgttcaagaccatggtcagctcgccgtacaacttcggcgtcaccaccaagctcttgacgccggtggcgatggacatcaacacctgctcctaccgttcggtgcacatccagccctcgcgcctggtggaagagattttggtcgacgagatggccagggcgttgcgcaaggaccccgtggccttccgcctcgaatacctgcgcctgccgcgcgcacgggcggtgctgaaggcggtagccgaggcagcgcaatggggcaaggccatgccggcgggcttcgcgcagggcgtgggtgtgcaccaggaatcgaagtccttcacggcctgtatcgtcgagatcgacgcgcgggtgccgaccgacctcaaggtgacgcgcgccaccatcgcgattgacgtcggcacgcccatcaacccctcgggcatcgaggcgcagatgcagggcggcctgtgcgaatcgatctccatcgtgctgacggccggcctgcacatccagaacggcctgccgctggaaggcagctactcgcaataccactttgcgcggatgaagaactacccgaaggacgtgaaggtcatcatcatgccgtccagcagtggcgaggcgatcggcggtctgggtgaagtgggcctgtcggccagctcgggcgcaatcgccaatgcctatgcgcgcgccaccggcaagaagccgcgaagttttccgctgaacttccccgtcgatttcacccccatccccccgggcaagctgcccacgccggtcaccgtgccggtccgcacctgaggagctccatcatgcccgtgcaatctttcaaggtgaacggcggcaacgtcgacgtcgaggcgcctgacgatatggcgttgctgtgggtgctgcgcgacaagctcggcatcacgggtccgaagtacggctgcggcatcaacgtgtgcaaggcctgcacctgccatgtggacggcaaggcggtcaccgcctgctcgacgcgggtggcggacgtgcgtggccggcgggtgacgaccatcgaaggtctggccaacggaaccacgctgcatccggtgcagcaggcctggatgaacctcgacgtgccgcaatgcggcttctgccaaccaggacagatcatggcggcagtcgatctgttgcggcgcacccgcaaccccaccgacgccgagatcgacgccatcgaaaacgtgtgccgctgcggcacctacggccgcatccgcgaagcaatcaaggcagctgcggcgatgatgggttagcgggtcgccccggtcaaggcctgcgccagatcttcccgcagatcgtcaacgctctccaggccgatcgagaagcgcagcagatgtcccgcatagctctgcttgccgctgcggatgcttcccatgtcatagggcatgaccagactcatgggaccgccccacgacaggccaatgccgaacaaccgaagacggtcacagaaagcatcgacttgtgcgggggtacgggactcgtcgatgagcactgaaaagaggccggcggctgcgctgcagtgcgtcgcccagtgttcgtgccccgggcatgattccagagcgggatgcaggaccctgcggatgccgtcctgcccggccatccatgaggcgagcgcccgagccgtggcgtcgtgcaggtcgtagcgagccttgatggacgccaagccccgcagcaccagttctgcatcgttggcgcccacgcccatgcccaggtccaggtaggcgacgcggagcttgtcatgcagcttgtcgtcgttggtgatgatcgagcccatcaagacatcggcaccgcctgaagggtacttggtcagggcgtgaacgctgatgtccacgcccatctcgaacggcgcgaacgcgatgcccgccccccaggtgttgtcgagcgcgacgattgcaccggcgttcttggccgttgccaccagtgtgcgaaggtccggaaattccatggtaatcgagcctggcgcctcgacccagacgagcttggtacgcccgctgagcttggcctgcagatcggcgacgtccaaggggtcgtagcactgatgggtgatgcccatctgcgagagcgtcgcgcgtgcatggcgcagcgagggcccatagacgttggtgggcagaagcatctcgtcgccgctcgacagcaggccgaggttgaccgaggcgatggccgcctgcccgctcggacaaagcaggcagtgccgaccgccttcgagcgtacacaggcgctgttcgagcgtgtacgtcgtcggtgtgccgtagaggccgtagctgtacccgtcgcggtggccgaatgctttggcacgttcgcgcaccgttgccacgttcgggaacaagacggtcgagcccttgaacacgcccggcggaaccgcctggtagccggccggtggaacgtagccgtggtggatcagtcgggtgctgatgtcttgagacatggcgggaactcttctgcaggatcaggagcttcaatgtatcggaacatggggcgccgcctgtgccgccccctgggcaaatccgcacgtcgggttgcgccgatgcggcaaggcgtcctcacgtacgcatgtcggctagccgcgcggctgcgcatccgcggggccgttgagccagtcttgcttcgactcgaagagccgatgaaggtactcggtgacagcgcggatgcgagccgagtattggaggtcgtggtgcacgctcacccagagcgttcgcgtcacgctcgccgtgtctgcaagcaccggcaccagggtgtcctccttcaccacggagaacttggggagcagcaccaggccgagcccggacgctgcggcggccatctgcgccagcatgctgttggactggaagctcatcggaggccttgcgaccagttcatcgagccagcggaccgcgtcgagctggatcaggtcgtccaggtatcccacgaactggtgctttggcagatcggccagactcgcgggcactccgtggttctcgagataactcgacgagccataaaggtacaacgcgaacgagcccgacgtctcgcaggccaatccctggccaatcggtttgaaaaagctgacgaagacgtcggcttccctgcggctcacgttgacgatggacgaagacgtcaccagttccacgcgcagcttggggtgcttgcgcagcagcggctcgagatggcgagccacgaacatggcgccgatcccttccatcatggcaatacgcacactgcctgaaggctccctgtcggttccgccgagttcctcttgcagcgacaacactgcccgctccatgttctcggcctgcagcgcgaggacatgtgccagctcggtgggtttgagtccggcgcggtgacgttcgaagagtgggccgcccaggcaaagctccaactgcgagagtcggcggctgaccgtcgaatgatcgatgtgaagctgcctggccgcctgggaaagactcccggtacggttgatatgcaggaacaggcgcacatcgtcccaatcgagattggcgaggggtaccttcttggtcgtcatgcggccttctcttgcgttgtcgtatgcagtcctgctccatcggcccaaccggccggtggtttctggatagcatttcacatcgagatgggcaacacaagggaaagcgcagccgagcatggccgcttctcagtccgggcacagtgccgtggaagattgccagggcgacctcagcccgtgggctgctcgacatgcgcttggcgccggtacaggaagtccatcagtgcgcgcctgcactccgcataggtcggatcggtcgccaggctgacgcgatcgcgcgggcgcccgatggggacgtccaggatctccccgatccgtgccgcgggaccattggtcatcatgacgatgcggtccgcaaggagcaccgcctcgtccacgtcgtgcgtgaccatgacgacggtgctttcggttttctcgacgatgccgagcagctcgtcctgcaacttggcgcgcgtgagcgcgtcgagcgcaccgaagggttcgtccatcagcaggacctgcggttccatcgacagtgccctggcgataccgacgcgctgcttcatgccgccggagatttcgctgggcttcttgtgcgcggcatgcgccaggccgaccatctcgagcgccgcctgggtgcggcgatcgaccgcggaagcagactccgcacgaaacacgctgcgcacggccatgcgcacgttgtcgaagcaactgagccacggcaggagagaatgattctggaacaccatcgcgcgccgaggtcccggcccgcggatgacctccccgtcgcacgagacggttcctgcggtcggcgatgccaggcccgccagaagattgagcagcgtggatttgccgcaaccagaatggccgatcaatgcaacgaactcgcctctgcggatctccaggttgatctcgctgagcgcaggaaattcgcctttgggcgtgctgaaggtctgccgcacattgtgaacgcgcagaaacccgggcgtggcggtcgaggcagtcgaaacagtcgggaaagttggccgcaacatggtctgccctttcattcgcgaaagctcagctgcttcatcaatgcgcccagcaactggtcgagcaccaggccgacaatgccgatcatcacgatggcgacgatgatgctggagatctgcaggttgttccattcgttccaaacgaagaagccgatgccgctctggcccaccaccatttccgccgccacgatcaccagccaggcgatgccgatcgagatgcgcatgcccgtcaggatcatgggaaccgccgccggaaagacgatcttgcgcgcgcgctccaagggcgtgagtccgatgacgcggccgacattggtccagtcctggcgcacgctcgcggtgctgtacagggtgttgatcaggatgggccagatcgaacagatgaagatgatgaagatcgccgaggcgccgctgtctttcagcgtgtagagcgcgagcggcatccaggccatgggcgagacgggccgcagcagctggatgaaaggattcagcgcctggcccagccatggaaccagtcccagcaagaagcccaagggaacgccgaccagcacggccagcgcgtagccgctgaagacgcgcctgagcgaatcgagcaagtgccaggcaatgcccaggtcgttctcgccgttgcggcggaatggatccgcaaacagttcgccggcgcgcttgaacacgtcgacgggcgtcgggatggccgagcgctccacggttgcaccggggctcttgcccatcagcttgtcgtagtctgaaagctccgctggcgcgctgccgccgccgctggaggcgagtacctgccagaccgtcagcaagagcaagccgatggccaaggtggccagccaggagcgtgaggtcgagatcgcgccctgcatgatcacgccttgcccagcgatttcagatagtcggccggacgatcggagtcgaagctcttgcccaggatggtttccttgcggaatccgacttcgggtgccctgccgccgcgctcttcaatgaggcgctttgcatcggtggccagcatgacttggcgggcgagacccttgtagtccaggtcctccttgatcatgttccatcggcgcatctgggtcagaagccacaccgcgctcgagtaatgcggaaagggctggaagtcgatgcggcgcggcagcgtcttcacgttgccgaggccatcggcataccggccggtgaggacctggtccacgaccgtttcgggctgattgagatattggggctgggcaaggatcttggccattcccgcgcgattggcaggctcggacacatgcaggctcgctgcgatgatcgcgcggtaggcggccatgaagctgttcggatgggccttgatccaggtctcggttgccgtcaccgagcagcaagggtgttccggccagatctcgctcgagaccaggtgaatgaaacccgccccttcgtacacggcacgctggccgcctggctcgccgccgaagaaaccgtcgatgttgcccacgcgcaggttggagacgtactcggacggaggaacgacgcggtaggacacgtcgcggtccgcgtccagccctgccgatgccaggtagtggcgcagctggagcatctgatgggactgctcgaacggcaccgcgaacctgaagcccttccagttcttcgggtcacggttgtccttgtgcttcatcgcaaggaccagcgagttgccgttctggttgagcaccgtcatcacacgggtgggaatgggagcgccgccgatgccggcggacatggccagcgcaacgggcatcacctgctgggagatgtccagttcgccgttgaccatcttgtcgcggatcagtgcgattccggcgactttctgcaggctcagctccaggccctcgcgtgggaagagtccgagttgctccgcatagatcagcggcgttgcgcaggtgatgggcaggaagccgacagcgagccgctttttctccggcacgcccttgctgctgcgctcctgcgcgacggcggcaagctgggtcagcggcgtgagcgccgtgagtgcggccagcgcccctgccctccccagcgtcttgacgaatgcccgccgcaggccgcgctcgggaaagaggccgtgcagcatgccctgggccatggcgccggccagcgcatcgtcggcgttcgcagccgtgttctccgcgaggcactcctcatcgtcaccgtgggtactgccgcatgcgcaagggccggtgcgggaaaggcgaacatactcatgtgatgggtccatgggccctccagtgtgggttgaacggatcaggtccgcgacacgtcaatggtgagcatgttccgtgcaaatagccgctgggaaattcacaacccgctgtgcgcagatgctccatggacccgtggagcccgcaaaaacgcacctcttgttgcgtttttcgagcatctgtgcggctgtaccggcaactatcctgtgggcctcagcaacgcacagcgagtacctgacatgagttcattgccccgggtgaaggttgccgccgcccacgcagcgccggtgctgctcgataagaccgccacgaccgaaaaggccgtgtccatcatcaaggaggccgcccttcatggcgcgcaggtgatcgcgttcccggaaacctacattccggcgttcccggtgtgggcggccctgtgggcgccgatctacaaccacgatctgttcgaggccatggtcgagaacagcgtctacgtgccggggcccgaggtggccttgattgccgcggccgccaagcgctttggggtgtgcgtgtcgatgggcatcagtgaacgcagcaccgtgagcgccggctgcatctggaactcgaacatcctgatcggcgagtcgggtgaattgctcaaccatcatcgcaagctggtgccgaccttctacgagaagctggtctgggcggcaggcgacggacagggacttcgcgtcgccgagacccgcttcggacgcatcggcgggctgatctgcggcgagaacaccaacccgctcgcacgcttctcgctcatggcgcaggcagagcagattcatgtctccagctggccgccgatgtggcccacgcgcaagccgtcgggcggcggaaacttcgacaacgttgcggcaaaccgtattcgggcgtccgcccattcgttcgaagccaaggcattcggaatcatctgcgcgagcttcatggacaaggcgatgcgtgactttctggtggatcgcgatccggccgtggcagaagtggtcgacggcacgccgcgcgccgcatcgatgttcgtggaccctaccggcacgcagatcggcgacacgctccagaacgaggaaggaatcgcctatgccgagttcgacctgaacaagtgcatcgagccgaagcagttccacgacgtggtgggctactacaaccgattcgacgtcttctctctgggcgtcgaacgccgccgccacgagccggtcgcgtggtcagggccgtccgatccgcagtttccgcggctgctcgacgatgagatggctgccggggtgctggatgaatagctccaagttcctgccaccgctgcccgaaggaactgagcgctcggtcgtcattggccggtctcccggattccatctgaagccgccacccgcccctgcggcgctgcgcgacttcatcacatccgatgcgcagctcttcgagaccatccacatgggcgccgtcgaagtcgatgccaggcgctggcggctgcaaatggacgggctcgtccgcaggcctttctcgatcgatctggacggtctcaggcagctgccttctgtcaccgtcacggccttccacgagtgctttggcagccccctggtacccgccgagctcaatctatggcgcgtgggcaacgtccgctggaccggtgcgccgctggccgtgctgctcgagcaagcgcagctcgagccgggtgccactcatgtctggtcagacggcctcgacagcggcgagttcggcggccgcagcatgaatcggtatcgcaaagatctgccgatttcgaaagcgctatcgcatgaggtgctcgttgcttacgagatgaatggcgcacccctgacttgcgagcggggcggcccggttcgcctgatcgtgccaggctggttcggcaccaacatgaccaagtggctctgccggctgtcgatccaagaccggcgtgcgaactcccccttcacgaccgattggtacaaccgcgacagcgagcacgaaggcaaagtcattcgagagccggtgtgggccgtcgaacccaattcgatgatcacccatccggcacccgacgacaccatctccacggatgatgtggaagtcaagggctgggcctggagcaacaacggcatcggtggcgtggcgctcagcgctgatggcggggcaacgtggcaagaggccgaagtccggccccgccgagaattcgaatggcagcagttcgcggcgacgcttccgctgcagcgaacggccggcccggtgagcatcgtcgcgagagcccaggacgccgatggatcgatgcagccgttgagcggagaacgaagcgcggcccactcggtccagatccagcgggttctatccggctcttgaacgaaaatgtcggaattgatgcgcaacaccagcggggcgaactgacgaggcctgcacgacacatgtacacatccactttcacattcgcaacgggcgagttcgacgacgagttccatgccttggacaacgtcattgcacagctcgccaaatccattcccggctaccttggcgaagaaagctgggagaaccctgcaacagggctcgtctccaacgtgtactactggaagacgatggaggcgctccaggagctcatcgggcaccctgcacacatcgctgcaaagcagcgccaggcgctttggctcaagggttaccaggtggtcattgcacaggttgtccgctgctatggtgatggcggcattccgcacccgctcgccgatggcgccgcggcctcacacagcggctgacccggcaacaccggggcgatcaaaacacttgaccggcagctgcggtcttttctttgcagtgatcagggtttcagcggcttcacggcaccgtcccagtgcgcgacgattttgccgttctcgaggcggaacatgtcgaaccaggtcgtcgtgtactttcgcgttgcgtcctgcggttcggggtactcgcgcacgaagctcaatatcaccgtgtcgcgctcggcgacgatcgagaccagcggggccttgatgcgagcctctaccggcagaggcgtcggagtccgtcgcgagatgaatcccaccatggccgcacggccggtgggcacgttggggttgtgctggatgtaggactcggcaacatacttgtccgcctgcgccacctgtcccgcctcgaagacctcacgccagaagtcgtagaccaggcgcttgttggcgcgcagcaccggatcagcgctcgcgagaagcgcctcctggtcggcggccggttgaaccggaacctgtgctgccgcggcgaggggcaagatggctgcaagcgcaaaaaggatatgtgcgaacagagggttcttcatggatcaaggcagttgttgagggacgctggactgcagcagacgatcagcgcggcctttgtgctcgccgatgaagagatcctgaacacgtctcaaaaagccctccggacatcgcgtgacttgtactggcgggcggcggccccgccacgagtttccgatgtcatattccgctgaaccagttgtatccctggtcttcccaatagccccccggattcgtgttcgaaacgaagatcgcggcgacgtgcttcgcgctcttgaatccgagcttggtcggaacactcagccgcagagggaagccgttggacgttggcagcgcttcgttgccaaagtcgagcgcaagcaacgtctgcgggtgcagcgcgctggccatgtcgaggctcgagtgatagcggtcagcacatttgaagccgacgaagcgcgccgtcgtgtccgcgccgatgcgctgcaggaatgtcttgagcggcacgccgcgccagtcgccgattgcactccagccctcgatacaaatatggcgcgtgatctgccgcgcttgcggcagcgtgcgcaggcgctcgacggtccacgctgtcttgtcggcgacgagtcccgagacttcaagccgccaactcgacacgtcaacttggggcgcgtcgaactctgggtagaacgcgttgaacgggaacggcttcgtgacctggcttgcctcataggtcggcgcgaggcggctgccgctgaagagacgggcctgcacgcggtcgttccagcgcgacagcgcccacaggaccttgtcgacctggtcgttgtcctgcaggttgcagccggacagcatcgagagcgcgccaaccgacagcgacgaacgcagcagcagccgtcgctcgaggttcacgatctgcgtcttgtgatcggagagcttgatcatgatgcggtacggtgagaggcccgcgcacgtccgatgaccatcggcagcagcgtgcgcggcacgaggaggacgagcagcagatggatcgcgatgaagccaacgatgccggccattgccgcgaagtgcacctttcgcgcgaaatcgaagccaccaaaaaggccgaccagccataccagctgcacaggcttccagatcgccagccccgatgcgacgacgagcacgccaagcagcagcacgatgacataggcgaagcgctgcaccacgttgtagcggccgacttcatgcgggagccgcaacgtcagcgcacgtccggtgtcgcgcagcaactcgctggcgcgaatcggaaaaaactcgcgacggaagtgaccgctggcgatgccgtacagcgaatacagcaggccgttcgcgacaagcagccacatcgccgcaaggtgccacgcaatggcgccaccgagccaaccgccaagcgttgcccaggcgggaaactggaatggcaggatcggcgacgcgttgtagattgtccaaccgctcatcagcatgcaggtcatcgcgaacgcattgatccaatgggcggcgcgcaccgccagcggatgaatcatcgtgctcttcatcttcacatcggcggcgtcacgccgtccttgcctgcggagatgaagtttgcagacaggcttgaatcggcttcctttttcgcgaacagcacgaccttggtgccgaccgtgagcaatgagcggtcgccgggttcgaggttgacgatcggcacgtcatccggcacgacgatcttcttctcgccgcccttgtacttgaggatcagcgtgcggccgttggtcgcgaccaggtcacccaccgtgccgttggtcatggtgctcttgggcgcgaggtcccaggcacggtggccatcgccggtgcccgccatcgcgggcgggaatacatgcacctcaagcgctttcagcgaaccgtcgggcagcggagtcgccgccgttccgatgtagctgccgggtttgatgtcggtcaacttggcgagcgtcaccgcgcgaacctgagtgtccttgttgatcttgatgctcaggtcttcgccgcggttggtatggaccttgatcgcatcctcgctgacggcggtgatcgcgccgcgcacaccgaccggcggcggcgtctgggcgtgcacggcgcagctggcgccaagcaggccggcgctcatcaaggtcgggagggcgagggtccgaaggagttttccgaatctgatgttcatgaatgagccgtagaggatgaagacaggccactctagggatcgcccatgctcatgggcatgacattcggatgacaaaaaagtcatgaaccgacgccgcaccgcgagagagaatggcaaacacaatcccatgagcatccttgttatcgaagacgacccgaagacgggcgactacctgaaaaagggcctgaaggaaagcggctacgccgtggaccttgcgcgcaccggaacggatgggcttcacatggcgcttgaacacgcctacgacctcgtcgtgcttgacgtgatgctgcccggcatcgacggctggcagatcatgcaggccttgcgcgacaagcgggacctgcctgtgctcttcctcaccgcgcgcgaccgcctggacgaccgcatccgcggcctggaactcggcgccgacgactatctcgtcaagcccttctcgttcaccgaactcgtattgcgtatccgcacgctgctgcgtcggggcatcgtgcgagaagccgagttctacgaattcgccgatctgaaggttgacgtgctgcgccgcaaggtcactcgcgaaggcaaggagattgcgctgacgaacaaggagttccttctgctgcaactgctgatcaagcggcagggcgaggcgctctcgcgcacgctgatcgcctccgaagtgtgggacatgaacttcgacagcgacaccaatgtcgtcgacgtcgcgatcaagcgccttcgcgcgaagatcgatcagccgttcgagaaaaagttgatccacacggtgcgcagcatcggctattcgttcggcgacgcgccatgagatggctgccgcgatcgctggcagtgcgcgccaccttgctgcttgccctgatcacgtgcgcggtcaccggcatgctcggcgcctactttttttattccgcgcgatcggcaatcaccgagcagctggacacgcggctgatcggtcgcgtcgagcacttccgccgcctggtgggcaacgtgcagacgatcgctgacctgcacgagcggccgtcgctgttcacggccatgctcggtgccgagagcgatgtgctgctgctgcgccgccccggcgaggcgcctttcatcgacgtcaacccccgcggttttccggtgcccggcgctctggctccggtcgcggtcgatcgcgatctggcgatcggcaacgtgctaaaagttccgatggcggatggcgtgccgatgcattgggttgcggcgctcgcgcgttcgggccgcgatggcaatatggtggaggtggtggccggccacccgctgaccaacgaggtcaagatgattcgcgccaaccgagatcgcgtaatcctcagcgccatcatcgcgatgctcgcttcgaccattcttgcgtatctggtgcttcggcacggcctgaggccgctgcaccgagttgccggcaaggcggccttgatcaatccgatcaatctcgctgtacggctgccagagcatgacgcgccgctcgaagtgcagcatatggtcgtcgcgttcaacgccatgcttgaccgcattgccaccggctatgagcgtctttcacaattctctgccgacctcgcgcacgagatccgcacccccgtcggcgcgctgatcggacagacgcaggtcgcgctgcaacgggctcgcagcgccgatgagtaccagcagcttcttgaatcgaacctcgaagagctgaaccgattgcgccagattgcggagaacatcctgttcctcgcgcaagccgaccatgcatcgctgacgatcgagcgagccccgattgcgctgcacgccgagctagagaagatcgccgaatacttcgaaggcccggccgatgagagcgggcttcgattcgaagtgcaagccagcggtatggccttcgtcaatgccgcgttgtgccggcgcgcggtcaacaacctcgtcgtgaatgcagtgcgccacggcacacgggggacgaccgtgcggctgatcggtgcgcaagacggcgacgtggcaacgatagctgtcgagaacgaaggggtgccgatcccgcccgaacagcttggacgcctgttcgaccgcttctaccgaggtgacgctgcacgcagctataccgaatccaacggcctcgggctcgcgatcgtcaaggcgatcgtggcgttgcacggcggcgatgtgtgcgcttcatgccccgcgcccggcttgattcggttcgagttgcgctttcccgcgatgagggagtgagtgccgcaggtcccctggggtcgtctccttccgtgcccagtatcggctggcaatcacgcagaccagaaaggcaagaggaacagtgaccaaggcaggcggatctatcgggaaaacggggctcgcgtgtccaagcaccttgacccagatcgccgggccaagcaccgtaagcaccagggaggacaacagacccacgcttcccccaaccaccgcgccggtggctgtgaggcggttccagtaaatcgcaagaaccagcaccggaaatgtcgacgagcaggcgatcgagaacgccaagctgatcatgtaggcaacgttctgccccttgaacgcaatgccgagcgcaatcgcaaaaagacccaatgcgatcgtggccacacgaacgatccggatttcatcccgagcgccggccatcttgtgtcgaaacagcgcgccatagatgtcgtgactgatcgccgaagcaccagatagggttaggccagcaacaaccgccaggatggtggcgaacgcgacggcagaaaccagcccgaacatgatctcgccgccaaggatatgagacagatgcagtgcggccgtattgctgccgccgatcagcaagcctttcgcgtccatatattccggatgcgtgcgaagcaaggcaagcgcgccgaatccgatgatgaaaatcattgcatagaagcagttcatgaagatggttgcccagagaaccgaagtgcgcgcagccttggcatcgggcacggtgaagaagcgcatgagcacatgaggcaggcctgcggtaccaagcatcagtgcaataccgagcgaaagccccgacagcggatccttggcaaacgaggtcggcgtgaggattgcgtcctttcctgggtgcacctcgaccgccttgcgcagcaatgcgcccatgctgaagccaaactgtttccacaccaggaacgtgattgccgctccaacgccgagcatcaacacggccttgatgatctgaacccacgtcgtggccatcattccaccaaagacgacgtaaagcaccatcaacacaccgaccagcacgatggcaaggttgtagtcgatgccgaagagcagttgaatcagttgcccggcgccgaccatctgggcgatgaggtagaacgcgacaatgatcagtgatgcgcatgcggagaatacccgtatggcactgccattgagccttgaacaaacgacgtcggtgaaggtgaattttcccagctggcgcagctttcccgccatcaggaacacaacgatcggcaagcccgtcgtgtaaccgatggcgtagatgaggccgtcgaacccgctcgagaagaccagcgcggtcaaaccgagaaatgcgccagccgacaaggcatcgccggtgatcgccaatccgttctggaatcccgagatgcgtcctcccgccgcgtagaagtcgctggtcgacgacgtacgccgtgctgcccaccatgtgatggcgagcgtgatcgaaatgacgacgaggaaaagaaacacagaggttgcggagggagagccaatggcccctcccgccgccaacgcatgggtcgccgtagcggaagctgcgaatgcagcaatcaatttcttcatgtcagccatccatccgattggttcgaacaacgtagatgacggtcaacacgatcccgcacaggatcacgagcagaccgaaagcgaatgcgaaagggatctcgagcacaggcaccgtgaatgccattcctctcgcgttgaagcagcacatcagcacaaacgtaaagtagacaagaacctgcacggcggtgagcgccaggccgaagcccagcgattcgccgcctccatcgttgaggtcgcgacgcatgaaaatctccgtcaagttgattcgatccgggcgcaaccatatcgatgcgcccgaggtggcagaaacgattaatttcgatgagaccgatccgtcgcccagatgccagatgaaggtgcattgcttgcaccaaggcggacagcctcgtgcccgctgagctagagccctaacgcttccaccatcgccatgtgggcgctgtcgaggagcgctagcagctgctcgtcgtcccgtccttgaatgacatcgaacttcaagagtggcatctgcggacccctcagacgcagcgtcgcgcgttgttgatgatgtcgtacgcttgccgggcggtccggcgcacgacatcggccgccgacgggatgtcgtcgatcaggccgatggcctgtcccacggtgacgttcgcgcagtcgtagtcgccggactcatgcgccgcctcgacggcgcgcagttccgattcgcgcagaccccgaagcgcctcttcgttcccatgccagcgatgaatgaagtcgttgcgcatgaggcggccggtgtattcctttggccaagccttgccgcgcacgatgtcatacaccgaggtgcgaatcgtctgcgacccgcgcgcctgcgtcacgcgagccttggcgttcgggtggatgagggcctcttgggttgcccagaagcggctccccatcaagaccccgtcggcacccagcatcaatgcagccgccaggccgcgtccgtctgcgatgcctccagcagcgaggaggatcgtctccggactcttcgccgcgaggtagtcggccacttcggggatgaaggtcatcgtggtttgccgatcgaagccgtgccctcccgcctccgtcccctgcgccacgatgacagccgcgccgacgtcgagtgcacgctgtacgtgctcgagcgtctgcacctggcagatcagcggaattttcgccgcatgcactcttacggcgaagggctcgggatcggagaacgagagcatcaggcatcgcggccggcgcgccagcgccctgtcgagcagcgacacatcccgcgccatcgaccaggtgatgaagccgcagccgatcgacgcgtcgcccgccagggcgaattcacgttccaggacttcatggcttccgtatccgccgcccaggaggccgagtgcgccggcattcgacaccgccgcggcgagcacgccgccagaggcagggtccatgggcgcaagtgcgatcggatgttgcaggccgaacttttcggtgaagcgattggtgagcatgggttcctcgacatgtggtggaaggcccggatgctaggaagctgatcggatcctgagaaacgatttgttttgatgtcggcaatctatgcagcagattgcttgccgcccacttctggcgccgccgccagcctcgcggccccgcatgcacctaagggctaaccatgggctcgatgctgccaaaactgcctacgatgcccctctgtggggcgcattcgcaccagctttctcgtcgcgcccggatttttgcaggtacgcatcttgcgaaagctgcttgctgattgagtcatcagctatttcgatctgatctggagatgcatatggaagttggcgatctcacaacgttcgctgcggtggctcgctgcgcaggcatcaccaaggcggccaaggagctccacacggtccagtccaacgtcaccagtcgcatcaaggcgctcgaggacgaggtcggcgtaccgctgttcgaacgccacagccgtggcgtcgccctcaccagcgcagggatgcgcctgttgccttacgcatctcgtgcagtggcactgctgcaggaagcggccgccaacgcgcgcgacgacggccaggccagagggccgctggtgatcggctccatggaaacaaccatcgcggtgcgtctgccggaagtcctgggccagttcaacgcccgccacccggccgtcgagctggtcgtgcgcaccgggcccacggccgagctgattcagagcgtcatcgacaacgaggtggacggcgcgtttgttgcgggaccgatcgatcacccccggctgaaggccgagaagatcttcgatgaggaattagtcctggtcacgtcgcggcgctggccccacctcgcggctctgcgcaatgaggcagcgccgctgaccgcgctcatgttccggacgggctgctcataccgtcagcgcctggagcagttgctcgtccagctcggccgcccgtcctatcggcggctcgagttcgggacgctggaaggcattctgggctgcgtcggcgccgacgtcggcgtcaccctgcttcctcggtatgtggtcgcaaggtcgtttgctcacgagcgcctggtcgtgcacgagatcgatgcctcgatctcccgggcgccaacgctgctcgtcacgcgtcgagacgccttcgagtcaaccgcgatgcggatgtttcgcgagtgcctgggggggccggcgctgcgccagcttggcgattttccggtgagcgacatgtttgagccggtggctgctcagtgaacgagttgggctctacttcgccgtgggcatcacgaactcggcacccttgccgatgctctcgggccagtgctgcatgatcgacttctgcttggtgtagaagcgcacaccttcctcgccgtaggcatgcatgtcgccgaagagcgaacgcttccagccgccgaagccgtgccaggccatcggcaccgggatcggcacgttgatgccgaccatgccctcctggatgcggcggctgaactcgcgcgccacgttgccgtcgcgcgtgaagcagctcacgccgttgccgaactcatggtcgttgaccaggtcgaccgcgtccttgaagttggccactcgcacgcaagagagcaccggcccgaagatctcttccttgtagacggcgtgatgcccgccaccacgccgagcggctggcgcagcgtccagttgtcgatgccggtggaaacctggtcggtgaagtcgcccatgagcagctgcggaatgccgcaggcgaactcgacgatgtcgatgccgcgcgagacctcgccctgcgcgtcggtgaacaccctgccgtgctcgaaggcaatcgcatgcgccagctcacccttgttcttgttgagcagctccagaaacttgaacatcacgcgggcgcggcggattggcggcgtgtcggcccacttgggaaacgcagcctgggcagcagccactgccgcgtcaacgtcggcatggttggccagggccactcggccggttacccaccccgtggcggggttgctcacctcggtgggccaggcagcggcggcgcccctgccttttgagcaatgaacaagtctccccattccttcatcgctttcagaaccggggccaacgtggtgccgaagtcggtcagtgagtactccacgcgaggaggaatctccgcaaagatttcgcggcgcacgatgccatcggcttcgagttcgcggagctgaagcgtgagcgaacgttgcgagacaccatcgagcaacttctgcaattcgccaaagcgccgagttccctgcaagaggtggaacaccaacgggggcttccactttcctccagcaacgtcgacggttgcatccacagcgcaacgataggttttgaggtcagatttcatttaacagtatcaagcaggtgcctatcggcaagaaatgtgcgtacttgcggggcacgcatgcgggccctagcatccggcctgttggcccattccgggccggtatcgggagtagcgttgaaggcagcatattttgatcagcaagggccggccgaagcagtgctgaaggttggggacatctcggacctgacgccagggccaggcgaggtgggggtaaggatcgaggtgtccggtttgaacccgacagatatcaagacgcggacggggtttgctggggcacgcatgccgtttggccggatagtgccgcatcaagacggtgctggggtcatcgatcaggtgggtcccggagtctcggacaagcgactcggagaacgtgtttggctgtacgaagcacaaacaggaagaccgttcggtacatgtgctgagcggactgtcgtgccctcctctaacgcggttccgttgccccctggcgcttccttcgacgtgggggcgtgtcttggtattcctgcgatgacagcgcatcgctgcctgttcgcagatggcgacctccggggcaagaaggtcttggtgcaaggcggggcaggagccgtaggacttgcagcgatattgttggcgaagtgggctggtgcgtgggtcgctaccacagtgagtcgggcgaaccagtgggcgatcgccagtgccgccggtgccgacctcgtgatcaatcgccgtgatcaggatgtagcagaagtcgtaaagagcgctctgggtggcgctcatatcgatcgtattgtcgaagtcgatctgatgtcgaacgcgcaaatcgattttgcgtgcctttcgcccagcggcgtgatcagcgcctatgccaccgatgacccctccgccgaactgcgattgcccttccttcgcacgatgttcggcggctatgtgattcgctttgtgttcgtgtacacgatgccagaggacgcgaagcgccaagcggcccgcgacatcagcgcatgcgtggctacggaaaaatatgtgccggcgatcgccagtcgatttgccctgggagacgtggctgccgcccatcaatcgctggaaaatggagacgctccaggaaaagttttggtgtatccggcttggcctacggccgcccctaccaacgtttagttcagccgtagaggggcgaccgtcgacgcgatagcctctcggcggcgtgcgggcgtcggcgacaactatgaccgtgtcaatttgtcgcgctgctgcctgcatgtgatgtgaggcaactttcctcgcggcctccgtccctaccgccgactgagcagccactgcaggttccgtcggacgccgggccactcagtcgcaacaatgctgtacacgtacgtatcccgaagcaaattgctctcgacaatctgatggcttctcaaaatgccgtccagattggcaccaagtcgttcgatcgcggcccggctgcgcaagttgaaggaagacgttcgaaactcgacggcaatacaagacagcgtctcgaacgcgtgcttgagcagcagctccttgcattcggtattgaccgcagtgcgctgggctgatgctcggtaccaggtcgagccgatctccaaacgccgatgctgaggctcaatattcatgtagctggtcatcccaaggacacgagcggtctgcttctcttctacgacgaacgcaagcatgcttcccgcttcctgcaaagccagccgcctttcgatctcagcctcaactttgtcaggtgccggtattcttgtgtaccagagattccatacctcaccatcggcaacagcctcgcttagtgcagcggcatgtcgacaggccagaggcctgagcgcgactgcctcgccgatcaattccacgggttcaatccatgccaaaggtcatttctcctctgctacaaaggaatcgacaatgtcatgcatcagcgcgtttcggcgaaggcgtcatgaagagcctcgacgaggcgatcaatctccaccttctccgagataaacggcggcgcaagctggatggaatccgcgccctgacgcacatagaagcctttgctccagcacgccttggcaatgtcgtagggccgccggtcgggagtggcagctatgccgatgccagcagccaatccaaagttgcgtatatcgacgacatgcttcgcctgggcaagtgaatgcacggcatcttcgaagtagggagccagggccgccgcacgagcaacgatctcgtcgttcacaagcacgtcgagcgtcgcgatccctgccgcgcaagcgaccggatgggccgaataggtataaccgtgaggaaactcgaccgcaaagtcaggggacgccactcccatgaacgtatcgtagactttgcccgaggcaacaacagcggccaatggctgtgcgccattcgtcacctgcttggcgatggtcatcatgtccggcacaacgccgaatgcttccgcacccgtcatcgcgccaagacggccgaatccggtgatgacctcatcgaagatcaacaggatgtcgtgcgccgtgcagatctctcgcagccgctgcagatagcccttgggcggcaggatcacgccggccgaaccggagatcggctcgacgatcactgcggcaatgttcgacgcatcatgcaaggcgatcaggtcgatcagttcgttggcaagctcggcgccgtcctgaggtagcccgcgaacaaaggcgttgcttgcaagctgtgtgtgagcaagatggtcagcgtcgacaccagggccaaagagcttgcggttgccgccgaggccgccaacagatatccccccgaaattgaccccgtgatagcccttttgccgaccgatgaagcgggtcttggttccttgcccccgcaggcgccagtaggcacgtgccagcttcagcgcggtatccacagcctccgatccggagctggtgaagaacacatggtccagcccttccggcatgagcgccttgatcttgttcgcgagctcgaattgggcaggatgaccgtgctggaaagcaggcgagtaatccagcttcgcaatctgcttggagactgcttcggagatttcgtctcggccgtgccccaaccccgaacaccacagacccgaaagcccatcgaagatcttccggccatctatatccgtgaagtacgctcccttggcttcaacgatgacccggggcgattccttgaactggcgattgccggtgaatggcatccagcaggcgtcgatccattgcggatccaggctgagggacggtcgttgacgcttttcttgaaaagtatgcatggctgcttccagttgaagatgtgaattccgttgatcaggtcgcgccgacgctgaggtatcgatccttgacggcatcgtctgcaaggaactgcgcgttgctgccctggtacacgatcgttccttgctcgatcacatagtgccgatcagccagctgggtgcagacttcgaggttctgctccaccagcaggactgcgacgccggcacgccggatctccttgagctgggcaacgatctcttcgacaatgaccggggccagtccctcgaccggctcatccagcatcagaagcttggggttgttgagcagcgcgcgtccgatcgagagcatctgctgctccccaccggagagctgccctcccccgttctttcggcgctcgcgcaggcgcggaaagatcttgtagatgtcggtcagcgaccatggagagcctcggcgctgaccgagcaggaggttttcttcgaccgagagcagcttgaagatccctcgatcctcgggcaccaggcaaacaccgcgggaagcgatctggtgagaaggcaagtcttgcaactcaacgcctccaaacacgatcttgccgcccgtggcgcgaacagcgccggcgatcgtcttgagcgtggtggacttgccggctccattgcggccgagcagggttaccagttcgccgttgccgatctgaaggtcaacgccttgcaggatgtgacttttgccatagtggctatgcaaccgatccaggcgaagaatcatttgcggcctccggtgatcatgcttccgaggtaggcggttcgcacgcgctcgtcatcacgcaccgactgaggcgttccctcgaccagcacccgtccctgctgcatcaccgtcactgtgtgcgatatgtccatgacgattcccatgttgtgctcgatcaagacgacggtgtagtcgcgacccaggtcggcgatcagcgtcttcatatcgtccagatcgtcgatccccatgccggaggtgggttcgtccagaaagatggctttgggctcggccgccagggccatgccgacctccaatcgacgctgctgaccatgcgacagggaaccagccgccgtacgctcctgattccgcagtccaaggcgttcgatcactcggtccaccatctctgcgcaagaccagcggccctgcggtgaacgccagagattgaacgcccttcttgcgttcacgccctgcgccgcaaggcgcaagttctcgcgcactgtcagggtggggaacaggctcgtgacctggaacgatctggccattcccttgcgcacgcggacgtggccgggttcacgggtgacgtcctggccatcgaaggcaatgctgccaccggtcacacccagcgtgcctgtgagcatgtggaacagtgtcgtcttgccggcaccgttggggccgatgaccgaatgcaccgtgttgcgtctcacgcgcaggtccacgccgccaagggccacaaacttgccgtagtgcttggtaacctgccgtgcttccagaaggaattccgtgctcatacctgcttctcctcgactcggatttcaccggtccgcttgaaccgcgccgtcaaggcgagaaagccgtcttcgatgaggccccacaagccgcgctgcatgcccaggctgatgaccacgagcagcacgcccagcaacatcagccagcgcggccacagtgtcgacagccaatcggccgcaagcacgtagaacagggcaccgatcaacgacgcggcaagattgccggcgccaccgatcaccgtcatcacgaggatcatttcactcacatgaaattcggcgttcgcgagtggtgcgacaccgaccatcatcgcgttgagtgcgccggccagcgcagtcacggcacccgagagcacgaaagcgagcagtttgaagcgcggtacgttgtagccaacggcgctggcgcgcacctcgttgtcgcggattgccagcagcgtgcgcccaaagatcgatgtcgtcacccggtgcaaagcgacgaagaccaacaggaagatgaccgccaccatcacatagaactgccacgccgtggtgttgtcccagagaaccactccgaacgcagacaccggcggtctcggaatgttgagcagcccgttgtcgccccccgtcagggacggaacgctataggccagaaagtagaacatctgcgcgaaggcgagcgtcagcatgacgaagtaggttcccttctgtcgaatcgacacgatcccgaccagccccgcggcgaggccaccaagaatgatcgaggcaaccagcgcaaggggcatgggcagcccggtgcgagtcagcatgaggccgatcgtgtagcttccgagtccgaagaaaatgccctgcccgaaggacagcagcccggtatagcccagcagcagattgcatcccagaacggccagcgcgtagatgaggatctcactggccaaggagcctgaactcaacagcagcggcaatgccacaactacgccaagagcaactgcgatatcgatgtttcggcgcatggttcaggctccctttccaagtaggccattggggcgcagcagcagaaccgcagccatggcaacgtagatcatcagacgggcaccctcaggccaaagggtgctcatcacgctctgcactacgccgatgagaatgccgccgacgagtgctcctgtgaaacttcccaggccaccaactaccacgacaacgaacgcgacagcgagtgcctcgatccccatgaatggttcgacaccccggatgggcgccgcaaggacacccgcaatcgccgccgtcgccgcaccgagagcgaaaaccaaactgaagagacgaaagacgttgatgccgagcagagagaccatttcgggtgactcgctcccggcccgcaccgcactgcccaggcgagtgccttcgagcacccaccagagcaatacggccaaaccggctgtcactccgatcacgaacaggcggtacttgggatagatgaagtcgccccacatgaccacgccctccaggctcggcgggacggccacgctgtcgcccagcggtccccactgcacgatgaccagctcctggatgatcagcgcgacgcccaccgtgatgaggatgtggaactcgtgcggcttggcgtagacatgccgcagcaaggtcttctcggcaacccacccgacggccgcgatcaacagcggaaccacaagcaaggcggcccagaagctcattccttgcctgacggcttcgaagcaaaaatatgcccccagcagatagaaaacgccgtgggcaaaattgacgaatcggagcaagccgaaaacgatggacagcccaacggccagcaggaagtacaacattcctattccgatgccgttgacagtctgcagaaggtaaacgctcatatgcggcgactccggtagttcgcggccggcttttcagctcagcttgcagccggcttgttcgacggtcaggaacgactgtccggaactgacaacatccacatagtcgtccgcgtccttcatctgcttcttggcctttccgcgcaccaggtagtagtctttgatgacctggtggtcttccttgcggatctgctcctggcccgtgaggccctcgaacttcatgccctccagcgccgagatcaccgccttcggctcggtcgaacccgccttggcgatcgcgtcaatgacgcatttggtgcagatgaacgcagctgccaaggtgtagttcggcgtgatcttcagctctctggtgacctgcgtgatcagctcgcggttggtaggagactcgacgctgtgccagtactgcgccccgaagtagatgccctcggtggagtctgcgccgagcgactggaactgctccagcccggacgtccatggcacgaggatcgtcatcttcttgtgcagcccgaagctgatggcctggcgcagcgcatcggtcgactgcgtaccgaagttgagcagcaccaggacgtccggcttggccgccatggcattggtcagatagccgctgaactctttctccgccagcgagtggtagctgttgccgaccagctccacgcccttttccttcagcacatccttggtggccgccagcattccttcgccaaagacgtattgggcggtgatggtgtaccagcgcttcgccttgggctgtgcctcgatgagtggccgcaccgtctgtgcgacggcgccataggcaggcaccggccaccggaacgtcgcgggattgcattccttgcccgtgatctcgtctgcaccggaatagcagaagaagacgcctccgagtcggtggacttctttgcccatcgccagagcttcaggggacaggatcccgccgacaaagaacttggtgttcttttgctgcgcagcctcctgcaccttgcgcaccgccgtggccggctttgcctccgtgtcaaacacgctgtacgcgaggcgacgaccgatcacggtcccataccgctggattgccatgcgaacaccgagctccccatacttgccgttgacggcaaacgggcccgacatggggaaaggcgccccgaactcgatcccttcggccgcctgcgccgacgccaagcgggagagcgacattggagcaatgccggccgcggccagcgctagtaggtcacgtctattcatattttctctttgatgtttcagttggggaaagtgacgacggccacggcgacccgggggatcaccgcgagggaacctaaggcgagttgggaagttgcgcgacggcgcccgctaccgaaagcaatcggctgtcttcgcctcgggccccgaccagttgaatgccgacggggcgaccgtctgcagtcagcccgcaagggatcacgacggcgggttgctggctcaggttgatgggatagctgaagccggcccaatcggtccatcgggtcatgccgctgcccggcggcacctcgtgacccacctcgaaggcggccactgccgtggcgggcgagacgaggacgtcgtactcgtgcagcaaccgatccattgcgctaccgaactcggcccgccgcatctgtgcagaaaccaggcccgcggtcatctttccgccgtcgcgtgcggcctccagcaacccgggatcaatgcagcttcggtcttgctcgggtatcgagtcgatgcgggccgctgcaccgcaaagccagtggtgcttgaaaatgtccaggacgtcgtcgcggggcagctgcacgggctccacgcgggcgccggcgcgttcaattcggcgaacggcccgttcgacgatctgcatgacctctggttcgactttcccggtcgcgggctgcgaccagtagccaactcgcgtgccggcgagcgcggtctggccgcagtcagacgatgtgaggccatgcgcgcattgggtccagtcgcgcatgtccctgcccgccatcaccctgaacatggcctctgcgtcagcgacggttctggcaatgggcccgatgtgggacagggttccgaacgcactcactggaaaggtgggaacgcgcgcgtaggtcggcttgaatcccaccgttgcggtgaaggaagcaggaacgcgcgccgatcccccgccgtccgtggcgagatgaaggacaccggcgccggtggcggccgccacggccgcaccaccagacgatcctccggcggtcatgctgggcatccaaggattgcgcgtgatgccgctcgacggactgtccgtgaccgccttccagccgaactcgggcgtggtggtcaggcccaggagaacggccccggagcagcgcagtcgctcgaccgctggtgcgtcctcacgttgtggttgcggctgcgtcgtcagactgccgaagcggaccacccagcccttgacccggacgatgtccttgatcgttgtcggaatgccatcgatcggcgacagcggggtgcccgtccgccagcgctgttcggacgcacgagcctgctccatcgcgccgttgtgatcgatgtacgtgaatgcgttgaagggcctgttgatcgcttcggccctggcgagggatgcacgcgcgacctccacgggcgagacttcgcctgagcgatacagcgcggtcagtgccgccacgccgaggcggcaaagtggatcggcatccaagagaggcgagctgatttgcttcatgaaattttccaactgacatgtattcgaatgcgctgaaaagagagcggacgcggcttcccctggcgatgtccaaccgccatggtgaatggattccagcgaagcacggtgctatgcgtgcgcgcagtcggggggcttggggggaggaccttccgaagcagacgatccgtggctcgaagtccgtgcaagcacgtctttgaattctttgatggggcctgcgatgtctcgaactgaaccgattgcgctcacgccgcgcagaattccctcggcatcggaggagagaaaaagtcgcgaacgtccaatcgtctcgaccttggttgtggagcccagggagggaagtcctgcgacctggagcgcgaagtcgtactgattgctccagaaccaaggcaccgcatcaaactcgagttgctggccgagcatgtttcgggccgcggtgtctgcttgatcctcggcattgcgccagttttctatccttacggcccgcccgtagagttggctgtcgtaacagcacacatcaccgcacgaaaaaattcgttcgtcgtcagttcgcagatactgatttgtccgtatgccgttgtcggtcgccaaacccgccgtttcagccagatcgacattcggtcgaacaccaaggccatagaccacgatgtcacatgccagggcctcgccagtcgaaaggcgaacggcctgcaccctgtccgtcccctcgagtgccacgatcccgacaccgaaccggacatccacgcctcgtcgttgatgctcagccaccactgcatccgagacgatcgccggcacactcctgcccattgcttgcggtgcgcgctccagcaccgtgaccgtacaaccgcgttccagagccgcggcagcaacctccaggccaatcacgccggcgccgatgaccaccaggcggcagccacgttgcagtgagtccgcaatcgcttttgcatgctggggcgtgcgcagcggcaataccccgatcagatccgaacctggcaccgtgagcggattgatgctcgcccctgttgccagcagaagccggtggtaggcgatctcccgcccgccttcgaggatcgcacgcccagtatctcgatcgatgcgagcgacgcattgggcaagctgcagatcgacttcattctccgcgtaccaggagtctgcgtagaaggcgcattgttcgcctgttttcttgcctagaagcaccgccttggacagcggggggcgatcgtaaggaaggcaactctcctcaccaatcaggctgataccccccgtccaaccatgcttgcgaagagcagcagcggctcgggatccgctatgacctgcgccaacgatcacgatgggctcttggcaagtggtcatggctttctcttcgcgcccgtctttactgtgctgccttgacttctgcgcacgccagcatggcgtcaccaattacccgctcgcctttcgcattcagggcttccccggcgctctggatatcgcgcacgtccttgttctggctcagcttggccttgcccacgaagcgcgttacctcgatctcgattccgacgatcgcctggagcatcgtgtcgatgtagtccttgggaccatcggtcatcttccacggcgttggctgcgacgcctcgtgagtgcgggtgagccgggccaccatgccgcggacatatcgctcatcgtcccgaatcgtggcgcgcccgtaggcatggaccacgatgtagttccaactgggcacttgcttgtgaaactcctgcttgctcggataccactggggcgagatgtaggaatctccagcccgaaacacaaccatcacttcgtcgccgctgacgatgtcctgccacaccgggttgttgcgcgcgacgtgcgagtgcagcactactttggatccctccttggcgtccagctcgaacggaatatggttggcatccaagccgctttttccgtgcgtaaacaaaatacccagtggattcttggcgatcaggtcgtgcagaacttcagggcgcgattcatcgaagtgggcaggaacgtacatatctctatctccgaaattggttgctgaggacggaaaacttcgaccaggctcgattcagatctcgatcatttcgaaatcggctttgccggcaccgcattcagggcacacccaatcgttcggcacatcctcccagcgcgttccggatgcgatgccttccccaggcaggccttgctcttcgtggtactcgaatccacagagcacacaaagccagctcttgaaggccacggcttggttcttctcggttgcgcaatcactcatggggtgcctcgctcatgtcatgccggcttcgaaaacaagccgtcgtcaaaaagtagtatggtgtattcaggttcagtgagatggaccagtattcacttatctcaggagaccagaatccaatgccacggacagccaagacgccggaagttccagcgatcgggccactcgatcgggaggccggcggtctcggacggcagctcgcccacaagttgcgtcaggcggtcaagagaggcgacctccaagccggcgagatcctcccgtcgacgcgcgctctcgccaagtccctgggagtcgcacgcggtaccgtcctcgaggctttcgaacagctgattgccgagggatttctcgaggccgaacaaggcggcagcacgcgcgttgccgcatctttggctgacatgccattggttgcagccgacgcgcgcgaaagcaaggcgagcgccaagcctctgccactgcccttgccttccgcggcgttcgcccagatcgctcggcagttcatgccgttgccaccggtgccttttgctgtgtcagtgcctgccggtgctgccgctcccggcgaggtctggcgccgcctgggaaaccagattcgcgcgcgcggcaagggggggccaagcggctatggagaccctcagggcgccctgcctctgcgccaggcgatcgcagaatatgtgcgacggtctcgctcagtgcgttgtgaccctgctcaaatcattgtgactaccggcactcaacaagggctgtatctggcctgcctggtacttctcggcaacgaagaccacgcgtgggtcgagaacccggcctattggggcatcacggcaatattggaaaccttggggcctaaaggtcgcatggtgcgcgtgccggtcgattcggaaggtttgatcgtcgacgagggcttgcgcttgagacccgatgcgcgcgccgcgtttgtgaccccatcgcatcagtaccctttgggcatgcctttgagcatggcgcgccgaaacgccctgctgacctgggcacgcacaaatgcagcctgggtcgtggaagacgactatgacagcgagttgcgatacgcgggacatccatttccggcgttgcaaggcctggatcctgaccatgtgatctatctggggacattcagcaagatcctctttccatcgctgcggctcggatatgccatcgtgcctccgaggctcgtcgaggcgttttgcggtgctcgcatgctgttggaccgccatccgccgagcgccgatcagcatgtcctggcggctttcatcgccgaggggcatctggatcggcacatccgacggatccgaggcgtttatggagaatgccgcagccagctttcgcagctttttcaggacatgcttcccagtgacttggcatggctgcagcccagtgatcagggcatgcactcggtgctctggctggcgcctggcattgacgatcaggccgtttccgttcaggccgccagagccggcgtggctgtgcggccagtgtctcgcatgtacgcggaaggcagcgaacgttcaggcttgatcctgggcctgggagcattcactgccgatcagattgcggacgccgcgcggcgactggcatccatcgtcactgctgccgctccagcaggacgccgcagggtccggagcacgatccgataaacgggccgtcatggtcgccagagtcgcaggccaagagactggactggcgctcactcccacttgagagagcgttccaccgacatgtccggatcactgcagacttcgatcaacgccggcccctcggcgctcatggcttgctcgacgatgcctgcggcatccctggagtgctcgatcctgaatccgcgggcgccgaaggcctcggcaagttttgcaaagccggggttcgccaggtcggtgccgctgacgcgatggggaaagtgccgctgctggtgggtgcggatggtgccgtacgacccgttgttggacaccaccacgcgcaggttcagccctctgtcgaccgcggtgatcagttcgttgccgttcatgagaaatccgccatcgccgacgaaggcgagaacttctcgccccggatggcgcaaggcagccgctatgccggccgggacccccgttcccatggctccgcaagccgagccgagcagccggttcgccggcgtcatcttgaagatgcgatgaacccaggctgcaaagttgcctgaatcggtcgtcaagaccgcatcgttctgggccaaccgtgcgatcgccatgatcgtgtggcccaggacgtcgttcgccaccacattctgtggctgccagccatgcgcacggtcggccgccgcgcgcacccgctcgagccactggctcgacaccgccccggagccgccatggcgcaatgcggcacgcacgaagccatgcgccgtcgagacgatcggcagttccgccgagaaatggcgcccgatcatggacggatcgggatacacgtgaacgaacttctgcggattggtgccttgccgcggaaaggcgaaccccagggacgacacatcgcccatgcggctgccgatcgcaacgatcaggtcggcctcgctgaagagcgccgtgtgcgcgggcgaggtgaagaagctcagttggcccacccagcgagggtctgtgttggagaactggtcctggttcttgttggtgacggcaacgggaatgttccactggtcgacgagcgcctggagatcgttgcggaaatcatcggtccggcactcaccgcccacgatcaggatcggccggctggccttggaaagcagatcatgcacacgcgccgcgtcctccagggtcgcctctgcgagtgccacgccgtgaacccgcgcgggctgtcgctcgaccagttcggtcaggacgtcttcgggcaactcgaccgcgaccggtcctggcgttcccgaggcagctgtggcaaaggcgcgggccatcacttcggcggcgcttgccgccttgtcgatgcgcccggaccatttcaacaagccggaaaaagctttgccagtatcgatttcctgcacggcgccgcggcccaggttcggcgtttcgacctggccaatcaagaggatcagcgggaccgcttcttcggccgccacgtgaacgccgatcgcggcattgaaggccccgggccccctgctcgccatgacgatgccggcgcggcccgtcagcttggcgtccgcgatcgcggccagggccgcggatccttcgtggcggcatgtcaccagatcgaaatcgcgccgcgcgtgaagcgcgtcaagcagcgccaggaagctttcaccgggaacgctgaacgcccggtccgcgccgtgcgcgaccatgctgtcgacgatggcctcggcaactctgtacgtcatgaacgtccttctttcaagacgcgttcacgtcgacgaccacgcggccccggatctcgccccgcatgagccttgcggctgcatcgatcgcttgcggcagcgcgatctcggtcgcaatgtcttccaggatcgggccgtgcagatcgcgcgccagccgctcccacgcggcgacacggtctgcctttggccgcatcacgctatcaatgccgatgaggctcacaccgcgcaggatgaatggcgcaaccgacgcaggcaggtcgagcccctgggccaggccgcacgcagtgaccacgccgttgtatcgaagctgcgcgcatacgttggccagcgtgtggctgccaaccgaatccacggcggcggcccagcgctccttctgcagcggcttgcccggttcgctcaactccttgcgatcgatcacgtcgctggccccgagccgccgaagatagtcagattcgcccggccgccccgtggacgcagtgaccgtgtacccgagcttggccagcagcgcgatcgcaacgcttcccacgccgccgttcgcacccgtcacgagcaccggcccatcgcctgccttgagcccgtgccgctccagggccatcacgcacagcatggcggtgtaccccgcggtcccgatggccatggcatccctggtgctgaaacgcttcggaagcggaatcaaccagtcgcccttcacgcgcgcccgctgtgcaagcccgccccagtgcgtctctccaacgccccagccgttgagcaccaccgtgtcacccggcttgaattcgggatggtcgctctgctccaccacgcccgcaaagtcgatgcctggcaccatgggaaagctccggacgacgggcccctttccggtgatggccaggccgtccttgtagttcagcgtgctgtattcgacgcggaccgtgacgtcgcctgcgggcaggcggtcttcatcgatctcggccagcgaggcgcggtaaccctgcgcgtctttttccacgacgatgcctttgaacatgtttcgctccaataaaaaaatcagtggtccgccgcgtggcggggcgaggccggggcgcgcgcgcccaggctggacagatatgcctcgatgaaggtcaccaggggacggtccgactgcaccagcctggctcggagcacggccccctcccaggcgatccagaagaactcggcgagttgctcgacgtccagcgttgccgagatggttcctgcggcctgagcctctcgcaggcagcgagccacccgctcctgccagccgacaagaatggcatcgagacgttcgcggaaatccgcaggcagggcacccagttcctggctcaggttgccaaccaggcatccccgcgtgaagtggtgcttgcgcatgcccctggatgcatcggcaatgaagtcggcaagccgatcgagcggtgcgcgttcctggttcaacagccaccggtctagcttgcgcttgaagtagtcgtcgtaggcgtccatcacggccgctccgaacgcgtccttgttcgcgaagtagtgatagaacgagcccttgggcacggtcgcccgcttcagcacggcatccaggcccgtcgaactgaagccctgctctgtgagcagctccatcccgcatcggatcagtacatcgcgcgttgccgcatacgccggcgacggcctttggctgcgcgccacgcccgctttggatttttcggtcatgcgtcaattctagaccgatcgtctagagaacatctactgcaccctctcagttgtcgtgcatctcaatgggttgcaccaatatgcgaccgcgcacgcacgttcattgggcaacttgcaccttcgcgcgcgccatcgggcttgatgccgttgatctgaccgcgcttcacggcgggcccgagtcttgctcgtaaaccccaatgcgagtcctaattgacacaatgtgtcctatcaccaatactttcatcacctcctcacttctgcggaaggaagccccatgaagccccactccatcaagaaatggcttgtcgccaccggcctggcctgcctggctgtctcaacggcgctggccgatgagtcgtatccgtcgaagccgatcaagctcgtcgccggcttcccgccgggtgggcccacggacatcattgcccgcgtgattgcgcaggcactggggaaggagctcaatggcacgatcgtcattgacaaccgcgctggcgccggcggcgtcatcggcgctgacgccgtggccaagtcgaagccggacggctacaccctgctcgttgcggtggagtcctcgcagacgcgcggccaagccttgaacccgacgctttcctatgaccagctcaaggacttcgcctatgtcaggaacgttgccaagcagcgcaatctcgtcgtcgtgaatcccgacatgccggtcaacagcatcaaggagctcatcgccttcgccaaggcgaaccccggcaagctgaatttcggcggcaccttcggcgccacgtcgcacatcggcggaacgctgttcgacgcgcgaaatggcacgcaacttacgttcgtgaattacaagggcggcgcgcaacccatcaccgacctcatggccggcgtggtacaggtcggcttcttcaccgaggcgacagtcgcccagcacatccgcgccggaaagatcaaggccctggcagttgccgcgccggagcgttcgcccgcgttcccagacctcccgacactccaggaagctggcagcaagccaatcgatctttccccttggttcggcattgcggctcctgcgggcactccgggcccagtcatccaaaagctggcggcggcgctcgacaaggttgtgaggaatcccgagtttcttgggcagctggagacgctcggtgccgttccggtgaaggagtcgacacccgatctgtacaccaaacaggtggccaaggagatcgtgttctggaacgattgggcgaaaacgctgacgactcccttggcccgctgaacgactgccgagtattcgaaaccgatgaacttctacgacctctacgacgagagactgtccgcggcggaaagatcactggtccaggctgccagcgacttctgccgcggcgaattcagcgcccacctcctggagtcgcacacgcagggtcgcgcctacgatgcgtcatggatcgacaggtgggcaaaggaaggcttcctggggcttcaagcgccaagggaattcggcggccacgatgcttcgttcatctgcaagatccgcgtggcgcagacgatggcggaacatggctttgccgccgcctttgccatcaacaatctgcaaggctccgtgacccgcgtggcgcgcttcggttccgagaagcaacgtgccgagctcctccacgccatgctgggcgggcgaacgctgtgcgcccccgccatgtccgagcccgatggcggcagcgacctggccgcactgaagacgaaggcgcggcgcgtggacggcggatggctgatcagcggcacgaagtcgtggatcaccaacggttcgatcatccagtgcgcaaccctgcttgcaagagttgacccgctcggcgcggaagccggcgacatcgcgtcttttctggtgccgctgaccgatggaccgacgcttcgcagggaagagcttgtcatgccgggcgccctgtccttccggctggcatccctggtcttccaggatcatttcgttcccgactggtgtctcttcgacccaccggggcaggcgttcaagtcttccatggcgtccgtcaatgccgcgcgcgttcatgtcgcggcgatgtgcgtcgcctctgccagggcagccttggcagagacggtgggctacgcggaatctaggcaagccttcggcaagccgctgctcaggcaccagggactcgggtgggagctcgcggaggtctcactgcgcctggaggcagccaatgcactcgtgctgcgcgcagcgattgccgtgcaaacaggaaagccggccctgacgctggccgcccaggcaaaaaagttcgccgtcgacgtggccgtctgggcactcgaccagtgccagcgtgcaatgggcgccaccggcgcgagcgccgatcaccgccttgccatgctgtcgagcgaaacacggctggcggcattcggcgacggcaccagccagatgctgctcgaccgcatcgccaagggtctggccaaagactatgggccttcgcccgcgcagaaggaatctgatcgatgagaaatgtggtcgtcaaggatgcgaacgccgcagtcagcggtttgcgcgacggagatacggtgatggtcggaggcttcggcggcgcaggcgttccgcgcggaatgatcgaggcggtgctggacctgggggtgcgcgaactgaccgtcatctccaacaacgcaggctccggcggccaggacctctcgctttggttcggtgcgcgcatcgtccggaagatcgtctgctcctacccgcgaagcgcggacgtgttcgccgaccaataccgggccggcgaagtcgaactcgagctggttccgcagggcacgctggtggagcgcatccgggccggcggtgcgggccttggcgggttcctgactcccacgggtgtaggcaccgtgttcgagaacggcaagcagaaggtcgtggtcgacggccgcgagttccttctggagacgcccttgcgcgcgcagttctcgctgctgaagggccggcaggccgatgtgctgggcaacctgaactacaacaagacggcacgaaatcattctgtggtgatggccactgccgcagaggtggttgcggtggaagtcgacgaactcctggagcccggcgagctcgaccccgaaggcatcgtcaccccctgcatctttgtcgaccgcgtctttctctcgaggcccgcatgaactcgctatccagactggaactcgcgcgcctggtcgcccaccagcttcccaagcaagggttcgtcaacctcggcatcggagcaccgacgggcgtggcggaccatcttccctccgatacctcggtcatgctccacagcgagaacggcattctcaatgtcggtcccaaaccggccgagggagaggaagacctggacctcatcaatgccgggaagatgcctgtcacgctcgcccgcggcggatctttcttcgactcgagcctgtcgttttctatgatgcgcggagggcacctcgacatcgccatcctgggtgcgttccaggtctcccagcacggcgacctggccaactggaccacgggcgatctgaacggtgcgccgccggccatcggcggagccatcgatcttgcggtgggagcaaagcagatctgggtgatgatggagcacaccacgcgcgacgcccagccgcgcctggtcgagcgttgcaccttgccgctcacggcagtgggtgttgtggccaaggtgttcacgaacctcgcgatcatcgacgtcaccgccgatggattcgtggtgcaggcgcttttcgagggagcctcgcttgaatccgtgcagcagctcaccggagcgccgctgaagccggcgcccacgctgaggcgattctcttcggacggggtgctcacgccgccccgttgaggccggcgttcaggcggcagcacgagccgtgcctcgggaccttatgcggtggcggcaatcacgaccagggccgaagccggctcatcggtgagcgcggtgagcttgtgcggaatggtggagtcgaactgtacgcagtcgccgggctccaggcgctccttgcgggctccgatctgcatctcgatgtggccggtgagaacgaagaggacttcttcgccctcatggtggctcatgatccggccgcgcttctgggtttttcccgggcgcacgatgaatgcccgcatcacgcggtcgtcgcgaaggcccgcgaccagcgagagatgcgtcgtgggatctcccgcaatggatccattgccccggacgatcgaaacgacgtcttcctccggctgttgcccgaagagccggtccaccgtcacacccagggccttggcgatattgagggccgactcgatcgacggcgtggatatgccacgctcgatcttcgacagatagctgcgcgtgagccctgaatctcgagccagattctccagcgtcaatccgctttggacgcgcaggtacttgaggtgtagtgccaaggctttgaacgggtctgcggcaggccgatcggctgctcgcaacccactggaaattgctgcggggcccgattctggcacgagtgtgtcgcccgcagcctagatgtcgagaaccaggcgcgggcccgcacactccgcaacgcacacgatcacttcatgcgcgcgctcctgaggactcaggacgcggtcgtgatggatcggcggtccctcgatccagcgcgtacggcatgcgccgcagatgccaccggcgcacgacacagagatatcggcgtccatcgcttccagggtggccagaaggcccacctcgggccgcacttccatctcgcgtccgctcttggccagcaccacgctgtacggctgcgcgttcagggttggaacaagcttgggcgcggtgaaccgctcgacgtgcttgcggctttcaggccactcggcgacagcggactcgaatgcatcgagcattccggcggggccacagcaaaatgccttcgcatccgggccggagccctccacgatggatcggatgtcgggcgggctgacctcgagcgtgttgtagagatggacccggccacccttcaccgccggcgccagcatgtcgatcaggctcggctctcccatgctggcccagtgcaactggtagttcgacttgccttcacgctccattgccaggatggcagacacgaacggcgtcacgccgattccgcctgcgacaaagatgttcataccggtgggcgagagctccaacccgcttctgggtaccgaaacaccaatgacttcgccggcacgaagctcgtcgtgtatgtggcgcgacccgccgcgccctgcttcttcgcgcttgatcgcaatgacgtatctccggcagtcggcgggctcattgcacagcgaataggtgcgtacgagcccattggccaaatggagatcgatgtgtgctccgggcctgaaggcaggcaagcgccaaccgtcctggtcagccaataccagccgcttgacccccggcagaggctcatcgatttctcgaacgacagcttgaaggtgtttgatcgccttcggcatatcacgccccgtggacagcgtcgcccacgcggatgacgccacccttcagaatccggcagttgaggcctgatctattgatcaatggatcgaacaccgccttcccgaggatctcttcgatatggcggcacggcgtggacagccgggttgcctcaaggagagtttccccgacccagaactggcggccgacgagatgattgagcggcacaccttgcacggtcacgtttcttcggtgctcttcaggcagcatctggatttttgcatcgcgcgccagggcttccagcgtctcgatctcgaacagcgtgatctgccgcccctcctccggcttgtgggagtagaagccggactcccggccgatcatgtatcggtctccctcgatgcccttgccggccacgagcgtcaactcgtcgaacgactccatgggaaggaaggctcgaggcgtgatgtgcagatgtcgaacgacccccgcccaggcgggaacgacctcccgctcgccgagctgctgttggtgggttgctgcagtaagcatgtaagacgctccttgataacggcgatccagccggtctgatgaaggaacgtcattataggacactttgtgtcctatgggactcgttcaggcactgtgagaaccggctcgaagcgcgaggtcgctgtccataccgatgcggcacagccctcaggattcctcaggtgctgccgtgcgcaccccatagagggccgtcctttgttctaaaaaggggtcggaccgccgattgaacaaggccatgatctgagctcgcagccattggcagctcggttccttctgtgtgcgccgatgccagtactggtgaatcgtgacggaaggcggcgtgaagggaagcggcaagacctcaagctccccggagcgcgcgaaatcaaaggctgcgggcagaggaacggtcgcaatgaggtctgttcttgcgatgatgtgaggaagactgaggaggttgggcgtactgagaaccactcgccgccgaactcgatgacgctccagtgcagcctccagcaatatggtcgaccgggccggcaagtcgagcacggcatgtccgagatcttgatacgccgcgcggctcatgcctcgggcgaccaccggatgtccccggcgaacgatgcacgcatacgtgtggctgaaaagagattggcgaaagtaggcatctttttccaatgcgggaaagtagccgatcgccaaatcaatgtcgccgctggcgagccgctcgtggagcggcaagacgatcggcgaaacgatgtgcacggaggtgcgtggcgcatgctcggccagatgcgccatcaggacaggcatgaagagagattcggctgaatcgggcatcgacacgcgaaaactggtctcgctgttttcgagatcgaatgcgccgctgccaaggacgtccttgtcgacctgatcgagcatgacgcgcgctgtttccgccaacgtcacggcccttggtgtcggacgcattccggatccagcgcggacgaataactcatcgccgagttgcttgcgaagtcggctgagcgcggtactgaacccagactggctcatctgaaggctttcagccgcacgacccaaatgacgtgtgctgtcgagggcgaccaggaggcgcagcaggttcagatcgagttgcttcatcgtttttgcagataacggatgttcatcttttccggttgagagtgcttcggtgggcgcctattctctggcgcagaccaacaggagacaacattgccgagccctgtccagagccatgcagaggaacgccggaaacatcttgccgcgatgcaacgagccgttcccgtcacgaggatggtggactatggcgtgccgctgggtgacgcgctccacatccatggcctgatcgcgacggacgattcagccggctgggacgaaatctgcgaacggctggcggcacggcatcatggctttgcagaggccgcagagaaggctggccggtcccctaccgcggctcaggcatggcgagccgcatcggcgctgcttcaatgcgcgcagctcgcgttcaatcaagacgtgcctcgcaaaagagcgctctacgaacaggcccatgccgcgctctcccgacatgcacacttgagcggagatcttgcggaggtgcaactatcgacgacatacggagctcttcatggttggatcgtccgtcccgaaagtgtggctgcaacggctgcggtgatcgttgtgggggggttgagcggctgggggagcgtgtaccttgacatcggacgggcgctcgcggctcgcggcctgctcgcgattcttgccgaagggcctgggcagggcctgactcgtcttcgaggcggaatgcatctcgacgaccgaacactgccgctcttcagcgctttcctggatcacgccgagtctctgggcgtgcgccggtgcggggtgtggggcaacagctttggcggcttgttcgctgcacaactggccgcgagggaccgaagggtgcgagcgctttgcgtcaacggcgcgccgatgattccctcggtccctccgttccgaaccgcccgcgagcaaatggaagcggtattcggtgtcgatgacgggatttctctaggtcatcgattgcaatcgctggccatgaacccacgccgtcaccgcatcgatgcccatctgctggtcgttcaaggcgggcgcgacgcgttggttccattgggcgagcagacgtcgtacttcaccttggtgccagcccacgagaaagccgtactcacgtgggcggatggcgagcacaccatctacaactacgcccaggagcgcaacgcgcaagcggcggattggtttgccgagcggctggatccagcggcggctttgatcgagaacaatgaaggagacatgaattggaagaatccacaagctttgaatttgacgtgatcgtggtcgggtatggacccagcggtcttgtccttgcttcgctgctgggacagcaaggccatcaggtggcggtcgtcgaacgctggccgaacttgtatggcaagccgcgcctgacacatatcgacggcgagacggctcggctgatttccgtctgcgcggatgctgaccacgccctgcgggacgcgtggaccacgccccactaccactggttcaatggcaaggggcagctcctgctggacgtgggcgggtttggcaatacgcgccggatgctgtgggatgaccatatctcggtccatctgcctcacatcgaggaggcgattcacgagcgaatcacgtcccttcccaatgtgcacctctatcggggatatctcgccaatggcctcgaacaggactccgagggcgtcaccctgagatgcgtgccgtgggggaaggcgaaggatccctctgcttcgccacgatccgagttgagcttgcgcgctcgctacctcgttgggtcggacggatcgaacagcttcgtgcgcgaggccctcggcgtcgaccggatcgacttcggcttcaatgagcgttggctgtgcgtggacaccgaacctcgtcgcaagctgccatcgaagttcgacgaaaacgccatccaggtgtgcgatccccgccgtggtcacatgttcatgccgattggcacgaagcggcaacgattcgagttcgctttgctgcccgacgagaccacagaggagatgcagaccgtcgatgctgcatttcgcatgctcaagcagtaccacgggctggagccggaagacctggatctcatccgcaatctcgtctacaccttcgagtgccgtctggccaagtcctggaaggtcgggcgggtctttctagccggagatgccgcacacacgaatccgccatacctcggacaaggtgcctgctccggcatgcgcgatgccgccaatcttgcgtggaaattcgacctcgtgcttcgcgggctgtccgacgcgagcctgctcgatacatacgaatcggaacgcacgccgcacgcccagcagatcatgctggactcgcgtgcgctgggactggttgccaacacctcgaaccccgtgaaggccgcggtgcgggacctgctgttcaagttcaatctcgcgccgaaacccaagtttccggtgctcaccaatggcattctggccaaaggggccgatggaagacccatgcggcaggcagggaccttggcaccacagggccgcatcacggtggacggtcgcacgatgcgcttcgatgagcatgtcgggttctctttcgcccttctcgcaaaccccgaagtgacagacgagttgcctgcgacgctcaaggccgcgctgcgggcggtcggtgtccggttcgtcgagctggcacctgcttcaggtgtgtgccagggcgatcgcgtgatagatgccgacggcgtgtacgccccatttctggagtcgctcgacgccgaggccgttctgacgcgccccgacttcgtggtgtatggacacgccgatcgtgcaggtctcgtgcatctggccgaaagcttcctgcagcagttgcagcacacctcgacaaggcggcatcattccaccatcagcgtccctagtccttgaaaaggccaatgaagagattgcggatccagtggtgcgcggggtccgattcgaagcggcggctccagtgcagcgacacggtgaaggcgctgcggggaagctccgccgggagcaccacatagcgcttcggctcgatgaacctgcgcgcaatcgcctgcggcatcacgacggcaaaatcggtacgcgcaatgatcgccggcagcgcaaggaagtgcgccgagttgagcaccagcctttcatcgaggccgagctgctgcaggatgcgaaaggtctccgagtgcgagcgcacggccacgtactccaggcgccgcaggtcctggatcgtcatgcggacatccgaggccttcgaggccttggccatcggatgccctgcacgcaccaccaccgcgtagcggtcgcgcagcagctcgacgcgctccgttccgctgaccgagggcagaaacccgagtgcgaagtgaatggcgcccgtctccagggcatcggtgatctccccgtgcggcagcggagtcgtatgcacccgtatgccaggtgcctggcggtgcaaggcttccatcagttccggcagcagccgagcctcgccgatgtcgttcatatgcagccgaacggtcattcgcgagcgcgaggggtcgaaggtgtcttcgtcccgcagcacatcctcgatggcggccacggccggctgaacgacgcttgccagccgctccgcgcgcagcgtcgggcgcatgcgcccgttggcgcgcacgaacagcgcatcgcccaaggcaagccgcaatcgcgtcaggccttggctggcggccggctgcgacaaccccagcgcatcggcggcgcggctgacgctgcccaggcggtacaccgcttcgaacagacgaagcaggttcatgtccagcttttcagtatgcatataacttattttgctctagacatttcattgtattgatgaatacagcggcaagcgcaaaactgcagacctcatctaggagcattcatggatcgacacgtcgaagttcccgcgcaagcacccctctcggccagcagcaccctgaccgtgcgggacgcggttttcaggctgctgcgcgcgttcggcatgaccagcgtgttcggcaacccgggctcgacggaactgccgatgttcatcgacttccccgaagacttccgctacgtgctcgggctgcaggagtccgtggtcgtgggcatggcggacggctacgcgcaggccacgcacaacgcggcattcatcaacctgcactccgcggccggcgtcggccatgcaatgggcaacatcttcacggcctttcgcaaccgcacgccgctggtgatcacggccgggcagcaggcgcggtcgatcctgcccttcgagcccttcctcggctccacgcaggcgcccgagctgccgaggccctacgtgaagtggagcgtcgagccggcgcgggccgaggacgttccgctggcgattgcgcgggcctactacatcgcaatgacgccgccgcgcggccccgtgctggtctcgatcccgtcagacgactgggacgtccagaccttgccggtcgatgcacgggaggtcagccgccacgtgcgcgcggatcccgatcttctcgcgcgcattgccgcggccctcgatggcgcccgctccccggcgttcgtggtcggtgccgcggtcgatcgcgacgaggcttggaaagaagcggttcaactggccgagcggcacaacgcccgcgtgtacgtcgcgcccatgtcgggtcgatgcagtttcccggaagaccatccgctgtgggcaggcttcctgccgccaatgcgcgagcgcatcgtcgaacggctcgacggccacgatctggtttttgcgctcggtgcgccggcattcacctaccatgtgccgggccacgggccgcacctgcccgaaggatgcgagctggtgcagctcacagacgatccccaggttgcggcctgggcgccgacaggaacctccgtggtcggcagcatccgcctcgggttactcgatctgctcgagtgcagcacgccgcgcgatcgtccggcaccacctacccatgtgcggccgccgcgcgttgcagagcccgagcccggcgaacgcctgccggttgcgtgggtcctgcagacgctggccgatgtgcgcgcacgcgacagcatcctggtcgaggaagcaccgagcgcacggcccgtgatgcacggccacttgccgatcttcgagtcggaaactttctacaccatgtgcagcggcggcctgggtttcggccttccggccgcggtgggggtggcgctgggcaagcccggcgcacgggtcattgcactggtgggcgatggctcggcgatgtacgccatccaggcgctgtggagcgcagcgcagctggcgctgccggtcacggtgctgatcctgaagaaccgccgctacgccgcgctgtacgagttcgcgcgcatcttcggctaccggcccgacgcgcatgttccgggcaccgacctgcccgatctcgattttgtcgcgctggctggcgcgcaaggcatgaaggggctgcgcgtcgacacggcggagcaactgcgtcccgcattgcaccaggccctgcaatcgaccgcaccgatgctggtcgagatcgaagtggcctgacagtttttttcgcttttccaaatctacaaggagacaagacgatgggcacgatatcgatgttgatcaatggcgaggaccgccaggctgcgggcggtgccaccttcgagcgccgcaatccgctcgacggcacggtggcgaccgtcgcgccggccgccacgaaggccgacgcggtggcagccgtcgaagccgccgcagccgcgtttccggcctggtcccgcaccggcccgggcgagcgcagggcgctgctgctgaaggcggcacaggccatcgaggcgaaggcccaggccctgacggatgccatggcatccgagaccggtgccggcgccccatgggctggtttcaacgtgcacctggccgccggcatgctgcaggaagcggcgggcatgacgacccagatcaccggtgaggtcatcccctccgacgtgcccggcagcctggccctgggcctgcgccgaccggccggcgtggtgctgggcatcgcgccttggaatgcaccggtgatcctcggcgtgcgagcgatcgccacgccgctggcctgcggcaacacggtggtgttcaagggctcggaactcagcccggccacgcacgggctgatcgtcgaagcattcaaggatgccggcttcccgccgggcgtcgtcaacttcgtgaccaatgcgccggcggatgcggccgaggtggtcgaagcgatcattgcccatccagcattgcgccgtgtgaacttcacaggctccacccgcgtcggcaggctgatcgcacagacctgcgcgaagtacctgaagccggcggtgctggagcttggcggcaaggccccgctggtcgtgctggacgatgccgacctcgacgccgcggtcaacggcgcggccttcggcgccttcgccaacagcggccagatctgcatgagcaccgagcgcatcatcgtggaccgcaagatcgcggacgccttcgttgcgaagctcgccgccaaggcagtgcagctaccgctgggcgatccgcgcaaggggccggtggtgttgggttcggtggtcgatgcgagcaccgtcgagcgctgcaacgcgctgatcgacgatgcccttgccaagggcgcgaaactcgtgtgcggcggcaaggccgacagcacgctgatgcccgcaacgctgctcgaccacgtcacgccgcagatgcgcatctaccatgaagagagctttggtcccgtgaagccggtggtgcgtgtcgacggcgtcgacgaagcggtgcgtgtggccaacgacaacccctacgggctttcctccgccgtgttcgggcgcgacatcgcgcgtgcctgggacgtggccaaccgcatcgactccggcatctgccacgtgaacggcccgaccgtgcacgacgaggcgcagatgcccttcggcggcgtgaaggattcaggctacggccgcttcggcggcaaggccggcatcgacgccttcaccgagctgcggtggctcacggtgcagaccaccgaccgccactatccgttttgatgaagcgcaggagacagcccatgaaatccctgctcgcaaccgcggcgctggtgctcggcctcgggccgtgcggcatcgcccaggcccaggattggcccaggcagccgatcaagatcatcgccaacttcgcgcccggcggcgcggccgaccagctcgcccgcgtgatcagcgcgcccttgcaggaagcgctcgggcagccggtgatcgtcgagaacaggggtggcgctggcgggaacctcggcggcgatttcgtcgccaagtcgccgcctgatggctataccttcctgatgagttccggcggcatggtgtcgatcaatccgcacatctacgcaaagatgcccttcgatccggcgaaggatctcgtcccggtcgcatccgtcgcacgcgtgccgttctacctggtggtccgtgccgacagcccggtcagggacttcaagggcctggtcgccgacctcaaggcgaaccccggcaggcggtcgttcggatcgcccggcaatgggagctcacctcatctcgcggcggagatgatgacgggccagacagggacaacggccattcatgtgccctaccgcggcgcggcgcccgcgctgacagacctgctgggtggccagatcgactttctcttcgatccgggaatcagcatccagcacgtcaagaccggcaagctgcgcatgctcgcggtggcaagcctcaagcgcgcgccccagatgcccgaggtgccgacgctcgacgagctcggactgaagggcttcgacgccgacgcggtgttcggcctctacgcccccgccggcacacggccggccgtgatccagcggatcaatgccgaagtcaaccgcgcgctggcactgccggccgtcagggcgcacatcgaaaccctcggcaacgtgccggagccgctgacgcctgcagccttcggcgacaagggcgcggccgatttcaagcggctgggcgccgtgatccgggagcgcggcattcgcgccgactgatgcaagaagaagaaagaactcgatgaccgccactccccggcctggcgccggccaccctcccctcatcgccacggacgtgctgatcgccggcggcggcccctgcggcctgatgctcgccaacgaactcggccgtcgcggcatccgctgcttggtcgtcgacgccaagccaggcacggccttcaacccgcaggccaatgcgacacaggcccgaacgatggagcatttccgccggctcggcttcgcgcacgagatccgtgcgctgggcctgcctgccgatcaccccacggacatcgcgtacttcacgcgcttcgccggccatgagctggcgcgcatcagtctgcccaccgcggccgaggctgcggtcaaggtcaaggcgatgacggggtcctggagcgccgccgagctgccgcatcgcgtgtcgcagaagttcgtcgagcaagccctgcgtcgccatgcgcaggcctggccttccgccgatgtgcgctatggctggcggctggagcggttcagcgacgacggtgagtcggtgagcgccacggtgcggccgagcgaaggaggtccggcgcaggacgtggtcgcaaagttcctgatcggtgccgatggcgcgcgcagtctggtccggcaacagctgggcatcgagtggggcggcgtgagcggcatccagcgcgagttcatgggcggcaagatgtttgccatctacttgcgtgcaccccagtttctctctgcgctgcaatctcccaaggcctggatgtacgtggccgtcaaccacgaaaggcgcgccttcatggcctcggtggacggcgtgtccgagtacgccttccatgcggcgctgcgtcccggcgaagacgccgagggctggaccgagtccgatgcgcgccgcgtcttcgccgaggcgctgggcgccgaggtgccgatcgaaattctctccatgggcacctggctcgccgggcatgcgctggtggcgcagcgctttcacaagggccgggtcttcattgcgggtgacgcggcacacctgttcacgcccaccggcgggctgggctacaacacggccgtcgaagacgcggtcaacctcggctggaagctcgcgagcgtgatccgcgaccaggcaccgctggcgctgctcgacagctacgaagccgagcgcaggccgctggccgagcgcaacaccggctacgcgcgcaagttcgccgactcggtggggctcttcgcggcaaagcccgaactggaagaaacctccgtgcggggcgaagccgagcgcaagctcgcgggcctgcacttcgatgcgcatgcccgcctcgaattcaacattccgggcgtgaccttcggcggccggtacgacagttcgccgatcatcgtcagcgatggcgctgcgctgccgccggacgagccgaatgcctacacacccaccgccagtccgggcggccggcccccgcacgcgtggctcgatgacggacgctcgctgttcgacctgttccacgccgaatggaccctgctcgcgctggggcctgatgcccccgctaccgaggccttcgaagccgcggcccgcaatttggaaatggatctgcgcgtcgtgcggctgccgcagccggccctgcgcgaactctatgaagcgccgcttgcgctgatccgcccggaccagatcgtcgcatggcgcggtgcagccgcggacgatgcagcaagtgtgctgtctcgcgtcacggcccggtctttcgccgcagcgccgcacgccacgtcaacaccttcaacaacaatctccgtcgatgcgacgggaggaaaccgcgcatgaaagtcagcaccccacttcttcgtctcgccgtccttgcaatggccttggcgatggctccttcggcattcgcgcaggcttggccaaccaagccggtccgcctggtggcggcatttccgccgggcaccccgggcgatgtgatcgccaggttgatacagccggcgcttcaggccgcctggaatcagccggtcgtcgtcgagaacaagacaggcgccggaggcaacctggccgccggggaagtcgcgcaagccaaggatggccacacactgctcgtcgggcccgacacgatcctcaccatcaatccccatctgtacaagaagctgggcttcgatccgagggcttcactcaagccggtcacctacttcgcgagtttcaaccagttgctggtgtgcaatccagccgccgaggtcccatcgctcgcaaagttcatccagttgccttccacccggctgtatgcctccggcggcgcgggctcgccaagccacatggcaatggagatgctgctggccacgaccggaacgaggctcacccatgtgccctacaaaggtcccggcccggccgcgcaggacgtgatgggcggccatgtggactgcggcttcatcgtctcctccgtcgtcctgccgcatgtccagagcgggcggctgcgggcgatcgccgtctccggcaaggaacgatcgggcctgctgcccggggttccgacggttgccgagagcggacatccgggcttcgatgccactttcttcgagaccttggccgcgccgtcgagcttgccagccgctaccgtcgagaaaatccagcgcgacgtgcgtgccgccctccaggctccggccgtgaaagcacgtctggcggagatggacctgcgtgtcgagggctacagcacgccggaggcgcagcggcgcagcctggaggacttcgccaagtggggtacggtcgcgcagcggacccaactgcaactggactgaaggagagccatcatgcgcaatctgaaccatcacaccatcaccgacgccgtgcttgcgcggcaggcgcaggcggccgacccgcggctcaagcgcatcatggacagtctcgtgcagcacctgcatgcctttgcacgcgaggtggaactgaccgaagaagagtggttcaagggcatccaattcctgacccgctgcggccacatcaccgacgacaagcgccaggagttcatcctgctgtcggacgtgctgggcctgtcgatgctgacggtggcgcagaacaacgacaagcctgccggctgcaccgaggcgaccgtgttcggcccgttccatgtggaaggggcgcctcactacgaacttggcgcggacatctccaatggcgcgcggggggttgcctgcgtggtgcgcggcacggtgcgcggcatcggcggagagccggtcgccgacgcccgcatggacgtgtggcaatcggacgaagacggcctgtatgacgtgcagcatccggagatcgaccatgcgcaggcgcgcggcatcgtgcacgccgacagcgagggccgctaccacttccgttcgatcctcgccgttccctacgccattccgcacgatggcccggtgggcgatctcttgaaggccaccgggcggcatccctggcgtcctgcgcacctgcacttcctgatcgaggcggatggctacgagaaactgatcacgcacgtgttccgcagcgacgatcgatatctggattcggacgccgtgttcggtgtgcgccagtcgctgatcgccgactggaagcagcaagccgacggctcctacgtcgttgaatatgacttcgtgctgaacaagcgggacgctgcggatgcctgacaactcgccttcttcaacaactgcaaaggacacgcaatgatccggcacatcgtcatgtgggacgtgagcggagacacggccgaagaaaagcagcgaaacatggactgtattcaaagcggcttccatggcctgcgcggctccgttcccgggttgctccacctggagatcggtgtggatgccagcaacgttgactatgcctgcgacgtggtgttgtacagcgagttcgaatcctgggaagcattggccgcgtatgcggtgcatccggaacatctgcgggtgcgcgacgaactggctggcgtccgcatcgcccggcatcaggtggactacgaagtccgggccggcagagcctgggctgagcacgatgcagcggggatcgcatgaaggacttcgtctacaacagccagccgtcgcgggtggtgttcggcgccgggagcttggcgcatctggagcgcgagatcgaactgctcggggcgcgccgtgcgctggtgctgtgcacgcctgagcagcaggaccaggcgcagttggtggccgggcgtcttggcagccgcgcggcgggcatttttgcgcgcgccgtcatgcatgtgcccatcgagacggcgcgcgaggcccgcgacgaggcgcgccgcctgggcgcagactgcgccgttgccatcggaggtggctcgaccaccggcttgggcaaggccatcgcgctggaatccggtctgccgatccttgcaatccccacgacttacgcgggtagcgagatgacgccgatctacggcatcaccgagggcggcttgaagaagaccggcaaggacgcgcgggtgctgcctcgcaccgtgatctacgaccctgagctcacgctgacgctgccagtggccatgagtgttacgagtggcatgaatgcgattgcacacgcggccgaaggtctgtacgcgcgcgacggcaatcccgtgatggacctgatggccgaggaaggcatccgcgcactggccagggcgctgccggccatccgccggcgcagcgacgacatcgatgcgcgcgcagatgcgctgtatggcgcgtggctgtgcggcacggtgctcggcaatgtgggcatggcgctgcaccacaagctgtgccacacgctgggcggcagcttcaatctgcctcacgccgaggtgcacacggtggtgctgcctcaggccatcgccttcaacgcgccggcggcgcctgaagccatgtcccgcatccagcgcgcactcgggggagcagcgcaaagcagcgccgcggcgagcctgttcgatctggcgagagacaacggggcgccggtggcgctgcgcgacatcggcatgaaggaggatgatctcgaccctgcggcagatatcgtcgtgagcaatccgtactggaacccccgagacgccggcttggcacagcgcggcgagatcaggcaactcctccagaacgccttcgatggcatccggcctgagtaggctcctgttgtggtccaacacaggtacgctggcgagcatgctggacctcgccatggcgatgggagtcttgtcgcagctgaagccaggctgtacatgcgccaccatcagcctgaccgtgaacatgcaaagcgccggccaggaaggccagttcattgcggtcgcgggggtcgaccggatcggccggcagattgccttcgcccacgcgaagctctatgacgcggagcgctcgcggctgattgcaagtgcgacatcgtcgctcgccgtcattcggctgcgcccctagggtggtgcgctggcccgcctgcgcagaccggtccttcgactttcgcgatcagggtttcggcggcttcacggcaccgtcccagtgctcgacgatcttgccgttttcgaggcggaacatgtcgaaccaggtggtcgtgtactttcgcgttgcgtcctgcggctccgggtactctcgcacgaagctcaatatcaccgtgtcgcgctcggcgacgatcgagaccagcggtgccttgatgcgagcctccaccggcagaggcgtcggagtccgtcgcgagatgaagcccaccatggctgcacggccggtgggcacgttggggttgtgctggatgtaggactcggcaacgtacttgtccgcctgcgccacctgtcccgcctcgaagacctcacgccagaagtcgtagaccaggcgcttgttggcgcgcagcaccggatcagcgctcgccaggagcgcctcctgatcggcggccggctgaaccggaacctgtgctgccgcggcgaggggcaagctagcggcaagcgcaaaaaggagatgtgcgaacagagggttcttcatggatcaaggcggttgttgagggtctctggaccgcagccgttatagacgatcaacgcgggccttgtctttgaaaaggccgatgaagagattccgcgccaaggctctattggtagccacgatgctgccctcgtcccgatcgcgccggctcgagtacgacagcccggttgccccagcaacgccggccgcccatgtcggcgttttgtcgaggttctgttgtcgacaagagacaagcgaagtgaatcgagcaaagaatcaatccgttgagatacacaaaaacacatatttcattgaaagtaacacctcgcctttttttgattgatctgccgcgtctcaagtcttccctcgggaactgaatattgcgttcgtgcagagccacgtcccgaggacattgcttgttccattccccatcaagtcgactccgaacggacggcatctcggtcgacgctgccagagacggcaaacatgcactccgtgaattctccggcttgcaactggcgccgtttcttgcgtcggccctcttcacggtcgccatggcgcgccctgtcgtcgctcttgcagccacgacctatgaaggaaccgttaccggcgttcaggccaacgaccaggcaggcggaaccggcaactattcgccggcctacgtcatcacgccctcttcgggcacgctgcactattcttttgcggcagacgacagcatcgatgtgcggggtgcgagtggcgacgtgtatggcgtcctgttgacttcgacttccggctcgtcgcccgtggcactcgattccgctggcggcaggttgaacatctcctcgaccagaggcacggcggatccgggttggggattgtcgatgggcatcaatgccgagggcaacagcctcacggtcaatggcaatgcgtcggtctatgcccagtccgacagcgcaaacagcgccgccatcggcgtgcgtgcatatcaaagcacggtcaccttcaacggcgatacgtcggtgcgcaccagcacgccgggctactcgcagggcgtgtgggtctaccagggcgtcgtcaccttcaacggggacaccaccatcgtcgtgagcgcgaagcgggagaacaccgacggggtctacaactccggcggcggcgtcagcagcgtcactttcaatggcaacctgaccattgcaacgacgggcgagtatcccagcgacaacgcgcacggcatctacaacaacaaccagaacagccggctgcatgtcgcgggtgatctgaagatcacggccatcgcgaatggctcgaccgtcttcggcatccgcaaccagggcaacctcagcgtcgggcaggatgccagcatcacggccaacggaagccgatccgcgttcggcattgccaacacgcaccgtaccgcccgaatgagcttcgcaggcaacgtggacattgcggtcgtcagcacgacggggtatgtccccttcggcaatccgacggggatcggcaacagctatccggacacgtcctccatcaacttcggcaaggcggtcacggtcaatgtatccgccgcggccgaggcctatgccgtcaacaacgccagcacgctgaatttcaactcggcaacggacaacgtggcgctgcaggtggcgtcgtcatgcagcggctgcgacgtctacggcatccgcaacgacgccggcacggtgaccgccgccggcgggttgagcatctcgacttcgccaagcggcacaggcaagggctacgcgatctggaacgtcgcggcggacggccgagacgccacggtcacggtcaacgccgcaggcgggcaggcggtgaagctgcagggagatctgctgaccggcagcgtgacgaacgccgccggcacaaagtacaccggcgcgctgaatctgaacctgaacaccgcggactcttacttgcgcggatcggtcggaagcttcgtggaccccgacacgtcggacgccacggtctatacggccggctcgcccaacctgtcgttctcccagggcgcctcctggattcccaccggcaccggcaccatggctgccgacttcggttcgggcaccctggcgctggccagtggcggtgcgatcgacatggccgcaagctggggaaccttccgtcctggaagcatccccgcccactcgctgcgtgtgctcgatatccaaagctcgaccaacgcggccacggtcagcctgggggatggcgccacctttcgcatcctgagcgatgtccgcaatggcgcggccgacaagattcagttcagcagtggggtgacgagcttcaacgcgaccggcacgcaggtggtcaatgtcgtgtacgaccccgcgctcaacgacaccagctgggtcaatgccgcgacgatgaaaaccggcaccgtgattccagcgagcacgcccatcgtcgtgatcgatgcgtctgccgcagcaggcggtacggcgcgcctgcaggccgttcagggcgccacagggcaatggagctatgagaacgacctggtgcgcttttcttactcgcccagcgtggcgctcagcgcggatggcagcaaggttttgctcaccggcctgagcattgcggggacgggtggggacgccagcacgggcacggcgaccagcacgagcacgagcacagccgtaagcagcgcaggcagccagtccggaatcctggcgcgcatcactccctcggagacggtgaagaccgcggccgacgcaggcgacagccttcgcagcctctgggctttgcgcgccaacggcatcgcgcgcagaaccgagtcgctgcggcgcgatacggcctccgaaacctcgggcatctgggccgaggtggacggcggcggcttcgacgccaagacggggtactccaggtcataccgccagagctatggcgccctcgccgtcggcgtcgatcggaatttgggcgacttcggcggctggaaaagccatgcaggcggctccgtcagctacgtcaattccagcgccacttatgaacgtggaaacgggaaggcttccgccatcgaactcgcaggctacggcctgtggaccaacggcagcgcaacctatctgcagattggcgcacgcaccgcgtcgctcgaaaacaaatacgcttcttccgactcgctcgcgcggcaagtcaccggcacgtatcgaacgcagggatacgaagtcagcgccgaggccgggcatcgcttccccctgccccaggacgccttcgtggagccgcaactggcattgaccgcgagccgcctcgcggacggcaagcacgtggcgagcaatggcgtgaccatcagccacgacaacgtcgacggaggctcggtcagggccggcgtgctcctgggcaaggccgtacgctttctcgatctgagcggcgacgtctatctccggctctcggcgatcaactacttcggcgatggcctggcgatcaccgcggccaagggaagtggcagccttcctgtcgaaagcgaaagccgcaacggaacaggcggcgaggtcgcactgggcggccgttttgcgtttctgccgcggcgaggctttgtctacttcgaggcttcgagcctggccgccaacggcatccggcggacgtggagcctgcgctctggcttgcgctacgagtggtactgatggcaaacccgcgacaccggctggccgtctggtcgcgtggccagagagccttggcttcactgctgttcgcaaccggcctggttttcacgtctggcctctcgatggctgcagagggcgacggaaaaaacttcgcgtggggcacgcaggtgacgcgagacaacgtcgccttcgaattccaggaagccaagtacgccaatctggtcgtggacagcagcagcaacaacaacgattcaccgaagcaatacaaaggcaactttgtcctgctccaggtgaacgtcacgaacaccgcagaccagccactgttcgtgcggtttcaacccgtgttcaggttgatcgacgcttcgggtgcactctatgagccgcatgaaatgctgacgaagctggtcaatccggtgcaagacggccaaccggtctttggcgcgccgctcgcagcgggccagaccatgcagcggcgtgtgctcttttccgtgccgaaacagctctatcgagccgtcgtcatcgttccacgcagcgccgacaaggccgacgacggtgtcgtgacgtactcagggccgtacttcttctacgacctggcgccccttcgatcttcaccaatggcaaagaacgccaagacgacgccgaaggtcccctgaaggatgcgctggcggattcattggccggtgtcgcatgcccatttgggcgcctgctcagaagctaggcgcatccttttccggcggcttggcgccgagtaccctttgctgctccgcgaatatctcgccgatgtagctcaggaggccgtctcccccgatcttcggcgccggggcgcgcgcatccttgggtgcggccttggcttggtcgacctgggtcccatcatccgcaagttcaagctgcggtccgctctgctggcacgcagcggcagcgaggccgaggcctgtgagtgccgctgcgtgaaatattctggtgaagtccatgtcgactcctcggtggatgggtggacgcgtcatcggaatcgatgatgcggcgctgctgttgctgtcgttgtggcgccttggaagcgctgcctttgcgcgagccggccagcacggtccgcgccacgccatcccggtttctaccgtgcggtagaaatccagattcgaccttcgtaaaggtctcgggtcacaggaagaagccgcccgtgcgcgggaacttatcggtgcaaccgaagcacagcgtactcctgccattcggcgcccacaatggaactaaaggcatagagagactgaaatttcaggcggcctgcgttgtaaaacacaagttgaaattcgtcgttaacggcggtgacatctcaatcaaacggcagatcgaaaatctatcccgtaatgatcggccgcagcgtatcgatctcttcgatcatgaagtcgaagaacgccgaaacgcgcggcgtatgccgcaagtcggcgcgggtaagaagccgccagattcgcgccagttcgggcacgggaccgagcacacgcaccagctcgggttccgcatcggcaatggcggtaggcagcggcgcaatgccgacgccggctttcaccgaatagagcaagccgagcacgctgttgttgcgcgcgaccaccctgccgtggggagccacgtcgcgcaaccatagagccgcacgatggttggccatcgtttcgtcgaacccgaccagatcgtgctgcccgagcgcctcgatccgatcgggctggccgcagcgttcgatgtacttgcggctcgcatataccgcccacagcgaatcaccgatcttgcgcccgaccaggtcgttgtcctcggtatcgccagagcgcagggcgacgtcggcttcgcccttcatcaggtcgaggtacttgtcgctcatcacgaactcgacgcgcagcccggggtaccgcgcgtgaaaacggtcgagcagcgtggtctgcatgatgcggtagaccagcggctcggggcaggtcacgcggatgacgccgactgcttcgagccggtccgattcgagttgccgttcgagggcggccacggcctgcgcgacgctctcggcatggggcagcagcgcctcgccgaattccgtcagccggtagccggtgggatggcgccgcacgagcgggcggccgagacggcgctcgagttcggcgagccggcgctgcacggtggactggttcacctgcaaagcccggccggccgccatcgtgctgtggtgatgggccaccgccagaaagtacttgaggtcgttccagtcgaacatggcgcgagctatgcgtttgtgcggccccattctgcattcctgcggcttacggtggggcatgtcggcgcctatgctggatctagccaggggagtgccagccagccgatgccgcccgaccaggcgaatgaaaggatcgatgatgacgaacccgttgatcgcacccgaagtggacgtacaggcgttcaagacagccatccgtgcggagtgggaccgcgcagccccggggtggaacggccatgctgcgcagatccgggagtggctgcgccgtgccaccggggccatgctcgacatggccggcgtgacggcgggggcgcgcgttctcgacgttgccgccggcgcgggcgaccagaccctcgacgtagcgcaacgcgtcggccccgatggcttcgtgctcgcgaccgatctgtcgcccgtgatcctggcgctggcgcaggagaacgcccggcgcgccggctacgccaacgtgcagaccgaagtatccgacggtgaaaagctcccggtcgagtcggccagcttcgacgccgtggtgtgcaggctcggcttgatgttctttccgaatccgctggaaggtctgcgcgagatgctccgtgcgctcaggcccggaggcggtgcctgcacgctggtgttcggacggcccgagcgcaatccgtgcgtgaccatcctgatgtcgacggccatgaagcacgcagggcttgcgccgcgcgacccgttccagcccggcgccctgctgagcctgggccgcccggggctgatcgacgggctgttcaaggaggccggttttgccgaggtggccaccacgacgatcgatgcgccgttcaagctgccctcggcgcgccactaccttgatttcgtccgggagtcggcaagcccggttcggcagatcctgagccgtttggacgccgccgcagctgccgccgcgtgggccgagatggaggagcgcctcgccgccttcaacaccgcgtccggctgggaaggcccgaacgaactcttgctgacggcgggtcgccgatcgccgcttcagcagccttcgaccgccaccaggtagtcgactgccgccggctgccgcagggccagcagcggtgcgtactcgggcgaggcgaaccagtcgcggatgtgctgcatcgaaggaaactcgatcatcaccaggcggctgggcttccagtcgccctcgagcacttcgagtgtgccgccgcgcacgatgaagcgcccgccgaatttctggatgacgggcaagacctgcgccttgtatttgtcataggtctcgtggtcgtggatctcggtctgcgcaatcaggtaggcggtcatggcgggctccttcttttgccggccatcatgcggatggcccggcgcgcgaagcaataccctgccggcgctctcaagcctccagtgcttccagcggcccgaagaactcgtagcgcagctgctgcttcggtacgccgagcgcaaggccgttggcgtacaccgccttcatgaaaggcttggggccgagaaagtagagatcgacgtcgcggtcctcgggcagttgctgcgccagcaactcgcgagtgacaaaacccgtggcgtgcggccggtcggcatcgcgcggcgtgtcgtacacatagaccggcttcacgttggcatgcttggccgccagcgcatcgacgcgcgcgcggaacgcatgagcgcctccatggcgtgccgcgtggatgaaatgcaccggccggccggtgtgcgccatcgactcgagcatgctcatggccggcgtgatgcccacgccgcccgtcaccagcacgagcggacgcgcgctttcgcccgcaggctgcagcacgaagtcgccgcagggcgcctgcaccttcagcagcgcgccgacagtggcagcctgatgcagccagttcgatgccctgccgccctcttccttcttgacgctgatgcgataccagggcttgcccggcgcatcggacagcgagtagttgcgccgcaagggttcaccgtcgatgttcagcaccagcgtgaggtactgccccggcgagaacgccagcagcgggccgccgtcggtcggctccaggtagaacgaggtgatgacttcgctctcgtcctcgcgccgggcgacgcgaaactcgcgctcgccgcgccagccaccggtttgcgcggcgttggcacggtagacctcttcttcggcggcaatcaggagtgccgcgagcgattggtaggcctcgccccatgccgcgatgatctcgtcggtcgcggcgtcgccgagcacgtccttgatggcacgcagcaggcaggcgccgacgaccgggtagtgctcgggcagcacgcccagcgcggcgtgcttctggatgatgcgcggcagcgcgccggcaatttcatcgaggcggtcgatgtacgtggcataggccagcaccgcgcctgcgagtgcacgcgcctggctgccggcggcctggtgcgcctcgttgaagaacgccttcacctccggatggctctcgaacatgatccggtagaaatggctggtgatggcctctccgtgcgcctggagcgcgggcacggtggctttgacgatggcgatggtctgcgggttcatggtgggactcgattcggaagtgaacgacgttgatgcctctcacgatccgtgccacggggacgacacccgccaagtgcccgtggatactggggattcttctttcgtggtcaaattcgcaacaggattcatgttgtatttatgaccaccaacagtgtcagtcagaccaccgatgcggttgccgacccagtcgcctccgcgagcgaaggcagccgctaccgctcgcttctggctgcggcgcgcggcctggtgcaatgcgatgccgccgcgctgctgcggctggacggcgatgtcctgcggccggtggccgcggacggcctgagcgacgagaccctgggccggcagtttccgatcgcgtcgcacccgcgctttgcgcgcctgctcgaaagcggccgcggcctgcgcttcgcccacgactgcgggctgcccgatccgtacgacggcctcgtggccggccagccgggaatcctgcccgtgcacgactgcatgggcgcgccgctgcgcctgcgcggcgccgtctggggcctgctgacgctggacgcgctcgagcccggcgcattcgagaccgtgagcccggagcagctcgatgcgctggtcgcgctgttcgagaccggcatcgaggccgccgacaccatcaaggacatggaagcgcgcgccatgcgcgagcaggccgtcgtccaggccctgcggtcgggccacggatccacgcgcgagctgctgggcagcagcgccgcgatgaagcagctgtgcagcgagatcgacacggtcgcggtgtccgatctcacagtgttgctgctcggcgagaccggcgtgggcaaggacctggtggcgcagcgcctgcatgcgcattcgcgccgccgcgagcagccgctggtgcaggtgaactgcgcggcgctgcccgagacgctggccgacagcgagctcttcggccacaagcgcggcgcgttcaccggcgcgatgcaggaccgcagcggcaagttcgaaattgccgacggcggcacgctctttctcgacgaggtcggcgagctgccgctgacggtgcaggccaagctgctgcgcgtgctgcaaagcggcgaggtgcagcggcccggcagcgaccggacgctgaaggtcgacgtgcgcgtgatcgcggccaccaaccgcgacctgcccgcggcgattgcgcagggccgctttcgcgccgacctctatcaccggctctcggtctatccgctggtggtgccgccgctgcgcgaacgcgggcgcgacgtggtgacgctggccggcggcttcctcgaagaaaaccagcatcgcctgggcgcgcgcaatctgcgcttgtcaccggcctcgaaggcggctcttcttgcgcacggctggcccggcaacgtgcgcgaactcgagcacgtgatcagccgcgcatcgcttcgggccttcacggaacagcgccgcggcgcacgctggacggcgatcgagccgcatcacctggcgctcgacgctgcggccgccggcagttcccagggactgcccgcgccgcccctgccctcccctgcgtctgcggcggtgtcatctggccctctcgcgggcgttgttgccgcgggcggcacgctgcgcgaagccacggaagccttccagcgggcgtggcttgcggacgcattggcgcggcaccatgggcacgtggccaacgccgcgcgcgaggccggcatcgaccgcagcaactttcaccggatgctgcgcaagctaggcatgcggccgtccgcgtcagacgcctgaacgcgcaccgcgcttcgtcgccggcgtcggcgctggcgccggtgccggtgccgggcgaagcgactcgaaggcctctgccagcgacagcacgcggccgcagttcaccgcctggtagcccggcagccggttcaccgcctcctgataggcatcgctgcgcaggatggccagcatccgctgcacgatgggtgcagtgagcgagcgctcgtcgcacagcaggaagtagcgctccacctggttggagatgaagtccagcttgaactggcgcgccggcgtctccacgccatagcccgcatcggccatgccgctggccacgaaggccgccacggccgcatgcgtgaactcgcattgctcgtagcccttgatcgactcgggcgcgatgccctgctcgcgcaattgcaggtcgaacaggtagcgcgtgcccgagcccgcctgccggttgatgaagcggacaccgggacgcgccaggtcggccagcgtgtagatcttcttcgggttgcccggcgccaccatcaagccctgatggcgcgtggccatgccgatgactttctgcgtgtcggggttgagccaggcgccgtagtgggcgatggcttcggcctcgaacgcccccagcggcacgtgaaagcccgccacgtcgcaactgccgtggtgcagcgaggccacggcttcttcgctgccgcagtagcgcagatcgcccggcacctgcgccgcggccaggaagccgtgcagcgcctcgatggcgaagccgtggctcgcgtagatgcgcagcagcgtgggcgcggtgggaatcagcttctcgatctcggcgcccagctcggaagccagcgaatcgagcagcggcgacaggcgcgcggtgatgcggcggtcggcccacaccagcttttcgcccaatggggtcaggctggaacccttgccgcgctgcatggccaccagcggctggccgaacatggtttcgccctggcggatgagctcccaggcatggcggtaggacacgccgcttgcggtgcaggcgctcgacaggctgccgtgctccagcaccttcaccagcagttcgatcacccgcggcgccagcgccgcgccgtcgggctggcgaatggtccattgcggcttgatgtgcacttcatgcatgagtttcggcttttgaaagcatatttattgggttgtgcgcttcatattgtggcgtcttcagtcgctccatacactcacgcaaccacgaatatcgcaactccgagtttaggagattgaaggcatatgcaaaacctgggcatcgcgaccaccatcgccgccgcgcacaaggatgttcccggcgggctgctgcccgcgctgcacgtcatccaggatgcgctggggcacatcccgcccgaggccgtgcccctcattgccgagcagttcaacctgtcgcgcgccgaggtgcatggcgtggtcagctattaccaccacttccgttccgcgccggccggccgcgtgctggtgcaggtctgccgggccgaagcttgcaagtccatgggagcggatgcgctgctggcacatgcggcggatcggttgggctgcggcgtgcacggcacttcggcggacgggcagtgttcgctggaaccggtgttctgcctcgggctgtgcgcatcgtcgccggccatcgcggtgaacgacgaggtgcatgcgcgcatcacgccggcgctgttcgacgccatcgtcgaagaagcaaggagcgcctcatgaccgtcaccctccatgttccgcgcgactccgcggcgctggccgtcggcgccgagcgggtcgcccaacggatcgcggcggaagcccgtgcgcgccatgcggacgtgcgcatcgtgcgcaacggctcgcgcggcctgttctggctggagacgctggtcgaagtggcaacgccggcgggccgcgtggcctacgggccggtctcgccggccgatgtcgccggcctgttcgatgccggttttctttccggcggcgcccatgcgctgaacctgggcctgaccgaagagattccctacttgaagaagcaggagcgcctgaccttcgcccgcatgggcgtgaccgatccggtctcggtggccgactacgaggcgcatgaaggctttgcgggactgcgccgcgcgctcacgcttgcgcccgcgcaaatcgtgcagcaggtgctcgactccgggctgcgcggccgcggcggcgccgccttcccggccgggatcaagtggaagaccgtgctggccgcagaggcgccgcaaaaatacatcgtctgcaatgcggacgaaggcgactcgggcaccttctcggaccgcatgacgatggaaggcgatccgctgatgctggtcgaaggcatggtcatcgccggccttgcgaccggcgcgaccgaaggctacatctacgtgcgctcggaatacccgcattccatcgccacgctgaacgaggccatccgcaatacggaacaagcgggctttctcggcgaagacatcctggggtcgggccactgctttcgcctcatcgtgcgcaaggcggccggcgcgtacgtgtgcggcgaggagaccgcgctgctcgaaagcctggaaggccgccgcggcatcgtgcgcgccaagccgccgctgccggcgctgcaggggctgttcggccagccgaccgtgatcaacaacgtgatcacgctggcttcggtgcccctcatcctggcgcgcggcgcggacttctacaagcactacggcatgggccgctcgcgcggcacgctgccgtttcagctggcgggcaacatccggcatggcggcctggtcgaaaaggcattcggcctgaccctgcgcgaactgctctacgacttcggcggtggcagcgcgagcggccggccgatcaaggcggtgcaggtgggcggcccgctgggcgcctacgtgcccgaatcgcaatgggatctgccgctcgactacgaggcctatgcggccgtgggcgcggtggtcgggcacggcggcatcgtggtgcacgacgacacggccgacatgtcgcagttggcccggtacgcgatggagttctgcgcgatcgagtcctgcggcaagtgcacgccctgccgcatcggctccacgcgcggcgtggaagtgatcgacaggatcaccagcaaccagaaccggccgcagcaggtcattctcctgcgcgacctgtgcgacaccatgctgcacggctcgctctgcgccatgggcggcatgacgccctaccccgtgctctcggccatcaatcactacccggaggacttcggcatcgaagcccccgaccgcgctgcggcatgaatcgacgagcattccaggagacacccccatgctgaacccatcgcaagagatcgactacggcacgccccggcgcgaatccatcgaggaagtcacgctagagatcgacggcacgccggtgacggtggccaagggcacctcgctgatgcgcgcggccgtcgatgccggcgtgcaggtgcccaagctgtgcgcgaccgacagcctcgaacccttcggctcctgccggctctgcctggtggagatcgacgggcgcaagggctacccggcgtcgtgcaccacgccggccgaggccggcatgaaggtgcgcacgcaaagcccgaggctgcaggagctgcgcaagggcgtgatggagctctacatctccgaccatccgctcgactgcctcacctgcgccgccaacggcgactgcgagctgcaggacatggccggcgtcacgggtctgcgcaacgtgcgctacggctatgacggcgccaatcacctgaagagcgccaaggacgagtccaacccctacttcacctacgacccgtccaagtgcatcgtctgcaaccgctgcgtgcgcgcctgcgaagagacgcaaggcaccttcgcgctcaccatcagcggacgcggcttcgaatcgcgcgtgtcgccgggccaggaccagcccttcatggaatccgagtgcgtgagctgcggcgcctgcgtgcaggcctgccccaccgccacgctgcaggagaagtcggtgatctggctgggccagcccgagcacagcgccatcaccacctgcgcgtactgcggcgtgggctgcggcttcaaggccgagatgaagggcaacgaagtggtgcgcatggtgccctggaaggacggcaaggccaatgaaggccattcgtgcgtgaagggccgcttcgcctggggctacgccacccacaaggaccgggtgctaaagcccatgatccgcagcaagatcaccgacccgtggcaggaggtgagctgggacgaagccgtcaattacgccgccagcgagttccgccgcatccaggccaagtacggcaccgattccatcggcgggctggtgtcctcgcgctgcagcaacgaagagggctacctggtgcagaagctggtgcgcgcggccttcggcaacaacaacgtcgacacctgcgcgcgcgtgtgccactcgcccaccggctacgggctgaagcagaccatgggcgagtcggccggcacgcagaccttcaagtcggtcgagaagtccgacgtgatcatggtgatcggcgccaacccgtcggacggccacccggtgttcgcctcgcgcatgaagcggcgcctgcgtgccggtgcgcggctgatcgtgatcgacccgcgcaccatcgacctggtgaagtcgccgcacgtcaaggccgaccatcacctcaagctcaagcccggcaccaacgtggcggtgatcagcgcgatggcgcatgtgatcgtgaccgaaggcctggtcgacgaagccttcgtggccgagcgctgcgaggccaagtcgttcaacgagtggcgcgaattcgtcgcgcgcccggccaattcgcccgaggcgatggaagcggtgaccggcgtgccggccgccgacctgcgcgccgccgcgcggctgttcgcactgggccacgacggcaagcggaacgccgccatctactacggcctgggcgtcacggagcacagccagggctcgaccatggtgatgggcatcgccaacctggccatggccaccggcaacgtgggccgcgaaggcgtgggcgtgaatccgctgcgcggccagaacaacgtgcagggttcctgcgacatgggatcgttcccgcacgagctgccgggctatcgccatgtgtcggacagcaccgcgcgcggcagtttcgaatccgcctggggcgtggagctgcggcccgaaccgggcctgcgcattcccaacatgttcgatgccgccatcaccggcagcttcaagggcctgtattgcgaaggcgaggacgtggtccagtcggacccgaacacgcagcacgtggccgaggccatgatggcgatggaatgcatcgtggtgcaggacctgttcctgaacgaaaccgccaagtacgcccacgtgttcctgccgggcgcgtcgttcctggagaaggacggcaccttcaccaacgccgagcgccgcatctcgcgcgtcaccaaggtcatgccgcccaaggccggctatgccgactgggaagtgacgcagctgctctccaacgcgctgggctaccccatgaactacgcgagcgccgaagagatcatgaacgagatcgccgcactcacgccgaccttcacgggcgtgagctacgccaagctggcaaggctgggcagcgtgcaatggccgtgcaacgaggccgcgccagagggcacgccgaccatgcacatcggcgagttcgtgcgcggcaagggcaagttcatcatcacgcagtacgtgccgaccgacgagaaggtcacgcgcatgtacccgctgatcctgaccaccgggcgcatcctctcgcagtacaacgtgggcgcgcagacccgccgtaccgagaacaaccagtggcacagcgaggaccggctggaaatccatccgaacgacgccgaggaccgcggcatcgccgagggcgactgggtcggcatcaagagccgggccggcgaaaccgtgctgcgggccaccatcaccgagcgcgtgcagccgggcgtggtgtacaccaccttccacttccccgaatcgggcgccaacgtgatcaccaccgacaactccgactgggccaccaactgccccgagttcaaggtgaccgcggtgcaggtgatgccggtgatgcagccttccgaatggcagcaggagtacagccggttcaatgccctgcaggaagagctgctgaacaagcggctcgaacaggcggcagaaacggcggcagccaaatgaacctggccgacataccgctgcggccaggaggtgcggagctcttgcccgtgcgcggcgtgcgcgcacgccaggctttcgacaaccgcgactgggtggccgtggaggtgccggtcgcgctggagttcaacggcatcgcgcacgccgtgatgcttgcaacgccgaccgacctggcggactttgcgctgggcttcgcgctcagcgagggcatcctgctcgggcgcggcgagctctacggcatcgaggaggagtttgcgcccgaaggcatcacgctcaagctcgacgtggcgggcgcggctttcgcgcggctgaaagagcgccgccgctcgatggccggacgcaccggctgcgggttgtgcggcaccgagagcctggcgcatgtggcgcgtgcgctgcctcccctgccgcacggcccggcgctttcgaaaaatgccgtcgcccgcggcatgcgggagcttgcatcgctgcaggtgctgcagaaggtcaccggcgccgtgcacgcggcggcctggtgcaccgcaaatggcgaagccctgctggtgcgcgaggacgtcgggcggcacaacgcgctcgacaagctcgtgggcgcgctcgcaaaaagcacggtggacgccgccgcgggcttcatcgccgtaaccagccgcgcgagtttcgagatggtgcagaagaccgtcgcggccggcgtgccgctgctggcggcggtgtcggcctcgacctcgctggccacggcggtcgcgcaagacgccggcctgacgctggcgggcttcgtgcgcggcgacgacctggtcatctacacccacccgtggcggctgaacggcctgcccgccaacgcctgaggtttttctgcaatgcacgtcgaccagttgattcgcatggtgaaccagatgggcagcttcttcgaggccatgcccgaccgcagcgaagccctgcacgacctggcgcagcatctcaagcgcttctgggaaccgcgcatgcgcagggagctgctcgcgcacctggacgccgacggatccggggaactgaacccggtctcggccgaggcgatccgggttcaccgggcgctgctcgaataacgcgaaggctgcgtgaagcgccgcgccgggtaacctcgcggcatggattccctgattgccgcttccgcgcgtgcgctcgccgccggcgacgcactcggcgccctcaagcgggtcgccctgcgcgaagacccgcccgcactggccctgcgcggcatcgcgatggcccagctgggcgagcatccgcgcgcgcgcgaactgctgcggcgtgccagccgcggcttcggggcccacgaagaactggcgcgtgcacgctgcgtcgtggccgaggccgaggtggccatggccatgcgcgatttcggcggctcgccgcgcgcgctggcggcggcagcggccacgctcgatgcgcacgccgaccgcgccaacgcgatgcaggcgcggctcatcgcggcgcgccggctgctgctgctcggccgactggaagcggccgcggctgcactggcgccgctggatgcacgcgacctgcctccttcgctggccgcggtggccgagctgaccgcggcggagctggcgctgcgctcgctgcacatcggtccggcacgcgccgcgctcgcccgtgcgcacgaggcggccggccgcgcgcgcgtgccggcgctgctggccgaggtggcggagacgcaggccgcgctcgaccgccccgccgcccggcgcctctttcccggtggcgagcagccgctgcgcctgggcgaagtcgcggcgctgctggcctccgacgcgctggtggtcgacgcctgccgccgcggcgtgggcagcggccaagcctggcggccgctggcgcgccggccggtgctcttcgcactggcacgcgcattggccgaggcgtggcccggcgacgtcgaccgcgaagccttgatcgcttacgcgttcaacacccgccgccccgacgagacgcatcgcgcgcgcctgcgggtcgagatcggccggctgcgcgcgctggtcgcggcgcaggccggcatcgaggccaccgcgcgcggctttgcgctcaagccgcgcgatgcacgcgacgtggtcgtgctggcgccgcccatcgacggcgagcaggcctcactggtggcgctgctgtccgatggcgcggcctggtcgacctcggcgctggcgctggcactgggcgccagccagcgcacggtccagcgcgcgctcgccgaactggaggccgaaggccgggtgcgctcgatcggccgggcgcgggcgcagcgctggctggcgccgccgctcgcgggattcacgacgatcttgttactccccgccgcgctgccgattgaatagagttgtctccacggcaccgatcccggcgcccgcccacacaaggagcaactgatgaacagcaccacagccagcaagaaagacaagtcccaggtcgtgccgcatgcggccgagatcgtgcgcgaatacgggccctttggcggtgacggcagcgtggccggcgtgacccacgacggccagcgcgtctgggcggctgcggggacgaagctggtcgccttcgatcccgcgagcggcgagaccacgcgcaccctcgattgcgtctgcgatgcaggcaccgccttcgacggcacctacctctaccagattgccgaggcgcgcatcgacaagatcgatccggccagcggcaaggtgctgtcatcgatccctgcgcccggccacggcggcgactcggggctgacctgggccgagggcagcctgtgggtcgggcaacaccgcgatcgcaagatccaccagatcgatccggtcagcggcgctgtgttgcgcaccatcgaatcgaaccgcttcgtcaccggcgtgacctgggtcgacggcgagctgtggcacggcacctgggagaacgacgagagcgaactgcgccgcatcgaccccgccgacggcgccgtgctcgagcgcctggagatgccgcgcggcgcgggcgtgagcgggctcgagtccgatggcgccgacctcttctattgcggtggtggcggcagcggcaaggtccgcgccgtgcgtcgcccgagaaccgccaaggcctgaaaggcgaaggagaaacgcatgaacaccgccatcgccgaaaccagcaccgccaaccatcccgtcgtgtcgaaggaccgatggctcgcccagcgcaaggcgctgctggcccgcgaaaaggaactgacccacttgcgcgaccagatcgcccgcgagcgccgcgcgctgccgtggagccgcgtcgacaagaactacgtcttcgacacacccgagggcccgcgtgcgctggccgacctgttcgaaggccgccggcagttgctggtgcagcacttcatgctcggccccgattgggagcagggctgcccgagctgctcctacatgtccgatcacctcgacgggatgaaggtgcacctggagaaccgcgacgtcacgctgctggtggtttcgcgcgcgccgctggccgagatcgagcgctttcgccgccgcatgggctggcagttcaagtgggtgtcgtcgcacggcagcgacttcaactacgacttcaacgtcagcttcaagccgcaggagtgggccgaaggcaagggcgaggtctactacaactacagcgtgcggccgtttccggcgcaagaggctcccggcatcagcgtgttctacaggaacgatgcgggcgaggtcttccacacctactcgacctacgagcgcggcgtggaagccatgatgggcacctacaacctgctcgatctcacgcccaagggaagggatgagcccaacccggtccatgcgatggactgggtgcggcaccacgaccgctacgagccggcgcccatggcgaagccggcggccgcggcgggttcgtgctgccacgcgccggactgaacgccgagcgcgctgaacctgcgagaacgtcatggcaaatctctggccgtggctggcggtggcgggcgtcggtgcccttcacgggctgaaccccgccaccggctggatgtgggccgcggcctggggcgtgcgctcacgcgaccgcacgcaagccttgcgggccctggtgccgatcgtcatcgggcacgctgcctcggtggcgctcgtggccgcggcggtggccttcggcgtgtcgatggaccgcgtggtgctgcagatttcggcgggcgtgctgatcgtcgtctttgcggtgcttcacttgtcgagccgcacaccgagcgcggcgcgcgcgccggccgggcatgcgggtatggcgctctggtccttcatggtgtccactgcgcacggcgccggcctgatgctggtgccggcgttgatcccgctgtgcatgggcgatgcctcggcccgcgagaccggcgcatcgggctcgctgatgctggcgtttgcggcggtcggcgttcacaccgtggccatgctggccgtgaccggcgccatcgcgctcggtgcctgccgcggcttcgatgccggcgcgcgctggctatcgaggctcaggcggaagctgccagctgcggcagcgcatcgcttttgaaacgctgcaacggctggcgactcgccatcgcgagcgccgccgtcagctgcagctgagacgggcgagcgccttgcccgcgccagccaccgcaggcagcttctgcttcacgcaggccgggtcgtgcgccgtgtacgcgtaggggatggcaaccggaaaggtgccagtcgtgatccagtcggtcgcgtcgcgcgacggagaggacgaactggccacccaggtgatcccgaaggtgctgaagtcggccggtgtcttgatgttgttgttgcgcagttcccagaagccgatcgccgagctgtcgcgcgaggtcacgggattcttcgcgttctcgaagtagttgccttcgatcagcgaaaagccgcccatgcggatgttggcacccgaggtgatcacgccgctgtacaggttgttgtacaggtgcgtgtagccgccgcgctgcagcggcaggcgtgagccgacgttctcgtagacgttgtgatggaaggtgatgaagcgatcgctggaatcactgtcgctcgagccgatgaggccgaccttgtggtgatcgtggatgtggttgtaggaataggtgatgtggtgcgcgccggccttgttgtcgagcagtccgtcgaactccaggtcgccagcgcccgagcattccttcaggctgctgaacagtgtgttgtggtcgatccagatgtggcccgggaacttgccgctctgcccctcgatgccgatcgcatcgatcgaacccggcagcaggccgatcgtcatgttgcggatgatgatgttggtggcatcggccttgatggccagcccgaagttggccgacgagttgtccgcgccctcgatggtgatgttgcttttgtcctcgatatcgacgatggcgccggccggcaacttccactgcgtgcaggcatcggtgatgctggcgaaatcgaacgttccgttgtagcggatcacgagcccaccgtcgccggtgtagccgtcaatggcagcctgcatttgcgcagcggtagacaccgtgatggccgcgaccttgccgcctccggtgacctcgccggcaaatccgccgctcaggctgtccgaggtgattgcaggtccaggcgcaggtgcaggaccaggtccaagagcaggagcaggagcaggagcaggagcaggagcaggagcaggagcaggagcaggagcaggagcaggagcaggagcaggagcaggagcaggagcaggagcaggagcgggatctgcagcagtagatgtcgatgtcgtggatgcggatgcagttgccactgagggcaagcccgtcgcgccgccgccaccgccgccacccccgcaggccaccagcaagagcgaggtcatcagagcacccgcagcgcgcgaacgggggcttgtgtgcttcattttcttcatgagattttttgtgtgttgatgccccgatggaatgacgaatgtcaaagcgggagaccacgtcgatacgcacactgcgtgccgctgacgcatttcggtttcttgtcgtcgatgtggacgcactttgtcggaaacggtcgagatttcgatggaaggggcagtcggcgcaacccgcaaacgacaatttgtgtctctttgtgacaaaacaaagcagccgggaggcgctgttcagcgcatctcaaatattcgtcgtttattcgtcaggaagataattgacaattatgtgttagggagataaagtgcacttattcgcatcacgaataatttgcatgcagtaccccttgtcgaatccggtgcagctggctcacctcctcatgtccgcccgcaaggccaagggactcacgcaggccgcggcggccgcgcgcgtcggcatgagccagagccgcctgtcggtgctcgaaacagacccctcgtcgctgacgttcgaacagctgctcgccttgatgagcttgtacgagctgcgcgtgacggcgcacgacaagcacccggccagcgcgccggggagctggtgacatgggcaggaaatcccacgcccagacgctctcgatctgggccaacggcttgcgggtcggcatctggcgcattccggcgcgcggcgcggtcgagctccagtacgaccgtgcctggaaggattcgccggccggccggccgctgtcgctctcgctgcccttcggcgtcgacgaggcaccgctccggggcgagcgagtgcagaactatttcgacaacctgctgcccgacagcgacgccatccgcaagcgcattgccagccggttcggcacaggctcggtcgatcccttcgacctgctgagggccatcggacgcgactgcgtcggtgccgtgcagttgctcgaggaagacgaaacacccggcaacgtgcaaggcatcgacgccacggtgctcggcgatgaagccatcgaacagctcctcgagcaaacggtttcctccgcggccttcggcgcgaacgccgacgaagacgacttccgcatctcgctggccggtgcccaagagaaaaccgcgctgctgcggcacaagggaaagtggctgcgcccgcatggcgcgacgcccaccacgcacatcctcaagctgcccctgggcctggtgggcaacaggaagatcgacctcggcacttcagtggagaacgagtggctgtgcctcaatatcctgcgggagttcgggctgccggtcgcgcagaccgacatccacaccttcggccggcaaaaggtgctgagcgtggcgcgattcgaccgccagctgcaccccgacggcagctggtatctgcggcttccgcaggaggatttctgccaggccctgggcgtgccgccgcacgccaagtacgaagccgacggcggccccggcgtcgaagacctcgcgcgcatcctgcggcagtcggagaacgccgaggcggacctgcgcacgctgctcaccacgcagatcctgttctggatgctggccgcacccgatggccatgccaagaacttcagcctgcacctgctcgccggcggcctgtttaggatgactccgctctacgacgtgatgtcgatctggcccgcggcgggcaccggcccgaaccagttcaactggcaccgcgccaagctggccatggcggtctcgggcaagaaccggcactacctgatgaaggacatccagcgccggcacttcaatgccatggcggccaggtgcttctttgcgtcttcggcggagccgatcatcgagcgcatcctggaacagacgcccgccgtcatcgacaaggtggcggccgccctgccccgcggctttccgggccacgtcagcgacggcatcctgaacggactgcgcgggtccgcgaagcaactcgcgggcatggcgccggaataaagaatcaagcacttgcgcaaagacgcggggtcatgcgcgaactgggcaaagtgacagcctcgtcgagacgacgcgggccgaggcccgccccatctgccaaagtcagttcgtcgcgaagcagtacatcagcccagcgctgccgctcattttgagttggtcgacgctgcagccgcgcgtaccgtgcgaagagttccacgaagcattggctactgggtcgggattggtgcccttgcggtcgtggtgacccacgatggcggagccgccgtcgcttttggtccaattgccgcatgtggtgtccttaccgggctcgggcacggccacggtgccgtcagggcgcgagccggtgaggatgtcgtggcggttgaccggatcgccggcgccggagacaacctcgcccttctcggtcagcgaggtgtccttgccgagcttggcgttggcgctgtgcaggtcggccacgctggtggcgacaaccactcccttggcattggtccaaggaccagcgccgatccggtcgcgcgcattgacagccggctgcccgtccgcggcagcggtgctcaaataagcgcgccacgttttgttgcccgcccccgcactcgtggcgagcgactggcagaagcggtcggctccggccaagcctccgaggtcgccgcccttgccggggttgacgctggtgatgaagaagctcatggggttgccgcccgatgaacgcatggcaccgcaaccgatgatcagcgcggtggctgcgacggcagcgccagtggaaagaaataagcgactgggcatcgacagactcctggctgtattggagccagaaggctaccgcaccgtcgtgtcagcggcaatccaagccagccctcatgcggctaccgcagcgcaacatcataggctcctcccgcaggacagataccgccgtctacaggcttcgttcccaagcgcgtaaattccgattccatgtgcgaaggcggtcgtccaatgcttctccgccggcgcccgagctggtggccaagagctggtcgagcaggatctgctgatcggtgctgagctgttgtggaaatatcggcaccagcgtgaccagttggtcgccacgcgtgccgcggcgctgtaccgggaagccctggcccttcaagcggtaggacagcaggtcgcggctcaactgcagcgcctggaagccggtgacggtcggcaccttgacctgccgattggcgatccatgcgaatccatcgaccggcatttcgcatcgaatggtgccgtcgtcgtcgagctttaggaacgcgtgctccgacacctcgacgcgaatctcgacgtcggtggaagggccttcggcgcgcacgcgacgtccgtcgacatggagcagatcgccgtcgcgcactccgtgcggaatgcgcacgttcatcttgtagccgcgcggtgccatcttgccgaccccgctgcacgccgcgcacggctgcctcgcgatgccgccgcccaagcaagcctcgcactcggccacaccagcgggccaaccgaaaaaggagcgcttcgggatcgcgcccgatcccccgcaccgagcgcaatttccgcccagcacctggtgcccggcgcccgcgcacgtggcgcagatgtcggtgaccttgccccgcagcaccttgatgcaaccgacggccgcttcctccagggtcatcctgaccttgcggtgcagggtccggcgctgccgttgcgttccgtccgcgtgggatgctgccgtggcttggttggcgtcgaatccgtcgggggtgttgttctccggtgcgccgggcgtgtcgacgtcggcgttcgccggggcgccgaatccggcgcggcggatctcttcgaatgcctggttgatgcgctgcatcttggccacagcaccggcgctgtcattgcggtccggatgccattgcgaggccagccggcgccatgccgccttcacctcgcgctcggtcgcgtcaggtgccagtcccagttcggcgaaagcgttctcggtatccaaatcaataaaccttgtccagggaagccgtccacgatggcacatggaggcggcggccggtcagcgtgaatgttatccgagggagcagcatgcaagccgtgtgccacgcgcggcgaggccgctcactccctgatcgcggcactccagaatgcattcgtcgccttccccaagagatcgctgtctcgataaagcctgatttccagcggaacggcccactcgctgctcgctgcggcgacaaggcgcccttggccgatgtcttcctccaccagggtctgcggcagccatgcgatgcccctgccgtccagcgccatcgtcctgaggaccgaggcgagatgggccgtgaaaacaacctggacagacagcggctccagtcgccggctgaccagggcacgcatgatgcgtcccagcccggattcctcggtgtacaagagcaccggtacggccgatgccccctggcgtgaaagctgatgcagcggcttgccagagtcattgggcgcggacactgcaatcagcaagtccccaccgatccgggctgatttgtacgggtctgcatcgagcgcgccatgcgcttcaggatgcgcgtggctcagcacgaactgaaccttgctttgcagcatcagcgattcgcaacgctgaaggacgtcggacatgagctgcacgggccccagcgtgatgctcgactcgaggctgcgaatccatcgcggcaggaaagtcatggaaagcgcatgcgtgcacgcaatgcgcagggtgaccgaactggcctcggcaatcttcctggcgtcgcccggcacgcgggccaccctcgcggtcaattcctgcgccacgccggcaaaccattcgccaacttcggtgagtgtggctggctgcgtgctgcggtcgaacaagtcggcgccgatccactcctccagtgcgcgaatgcgacggctgaatgcgggttgggagctatggcgctcatctgccgcacgcgagaagttccccgttgctgccaacgccaggaagtcgtcaagccagatcaggttcatgtccggttcgtccagcgcatagaagttgagaaattgaacattggccgaaaaagacggcgtggccgaccattcagtcttccactcaccccctctggagacaaccgtgaagatcgtcgaaatccgcgagaagaccatccccatcagctcgcccattcgcaacgcctacatcgactttagcaagatgacgctgagccttgtcgcagtcatcaccgacgtgatccagggcggcaagccggtcgtaggctacggcttcaactcgaacggccgctacggccaaggcaagctgatgcgcgagcggttcatcccgcggatcatggaagcgaatccgtcgtccctcgtcagcgacagcggcaacaacctcgatccgcacaagatctggaacacgatgttcaccaatgagaagccgggcggccatggcgagcgctcggtggccatcggcaccatcgacatggcggtgtgggacgcggtggccaagatcgaaggcaagccgctgtttcaattgctggccgaccgctatggcgacggcaagcccaatcgcaagatcttcgtctacgcggcgggtggctattactacccggggcaagaccatgggaagctgaaggacgagatgcgcagctacatcgaccgcggctatacggtcgtgaaaaagaagatcggcggagcctctctggacgaagacctgcgccgcatcgactcgatcatggaagtgctgcaggacggccagaagctctgcgtcgacgccaacggccgcttcgacctggaaaccgcgattgcctatgccaaggccctgtcgcagtacgacctgttttggtacgaggagccgggcgatccgctggacttcgaattgcaagccgcgctgcgcaatttctacaagaacccgatggccacgggtgaagaccttttctcgatgcaggatgcgcgcaacctgatccgctacggcggcatgcgtccggaccgcgactggctgcagttcgactgcgcgctcagctatggcctggtggagtacctgcgcacgctggagatgttgaaggaacatggctggtcggccagccgctgcatcccgcacggcggtcaccagatgtcgctgaacatcgcggccggccttggccttggcggcaacgagtcgtaccccgacctgtttcagccgttcggcgggttccccgatggcgtgaaggtcgagaacagcttcgtgaccctgcctgacttgccggggatcggcttcgagggcaaggccgatctgtaccgcgagatgcaggcgctttcggcctgaagcagatggcccccaaggagacaacaccatgaaaagcatttggcgctacggcgctggcatcggcctgctcgctttggccacgttggcctccgcagactttccggacaagcccgtcacgctggttgtgccgttcgcggccggcggcccgagcgacaagatcgcccgcgacttggccgaggcactgcgcaagccactcggccagaccgtgatcgtcgacaacgctgccggtgccggcggcaccatcggctctgccaaagtggcgcgcgccacgccggacggctacacgctgctggtgcatcacatcggcatggcaaccgcgccggccttgtatcgcaagctcccttacaaggtgcctgatgacttcgaaatgctgggtgtgatcaacgaagccccttcggtggtgatcggcaagccgagcctggaagccaacagcttcgcggatctgcgcaagtggattgctgcaaacggcggaaaggtcaacctggcccatgccgggctgggctccgcgtcgcacctgtgcggcttgatgttccagaacgccttgaagaccaacatgaccccggtgccctacaagggaaccgcgccagccatgacggacctcattggtgggcaagtcgatctcatgtgcgagcaggccaccaacgctgtcccgcagatcgaaggcaagaaggtcaaggtctacggcatcacaagcctgaagcgcctgccgctgccatcgctcaaggacactgccacgctgtcggagtccgggctcaaggacttcgacgtgcaggtctggcacggcttgtatgcacccaaggggacgccgccggcggtgttggacaagctcaacgcggcgcttcgcaccgctttgaaggacccggacctcatcaagcgcgaagaggcgctgggcctcaccgtggtgaatgacgaccgcttgagcccggccggccacaagaagtttgtggaagctgagaaggtccgatggtcgaaggtcatcaaggacgccggcgaatacgccgattgactggcgaagcgcctaacgcacagattacgcgccaaaccctgtgttcaacgcgtgagccggcagccctactgcgcttcgatcccgaactcccgcatgcgccgggtgatgacgtcgaaatcgcgcttgtagttgactgcgaactgctcgggcgtggtgttgagcatttcgagcccgcgctccgccatgcgcacctgaacctcgggcatggaggcggcggtgcgcagcgcaagtgtcaagcgctcgatggccgcgggcggcgtcttggccggcgcgacgaaagcgatccacacggcggcctcgaacaacgggtcgtcgaaacccagctcgcgcattgtcggcacctgcggcagcacggaggagcgctcgcgtcccatgatggccaacggaacgatcttccccgcctgcacgtgctggcgcgcgaggccggcggacgtgagcccgacactcaccgtgttgctcagcaggtcggccatcacgggggcctccccgcgctgcggcacatggaccatgcgtgcttcgagcttgcggttgagcgcctcgcccgccagatggccgaggccgccgggtccccaggtgccgtaactgagcttctggtccggcctggcggccagtttgcggaagtcgtccatgcccttgacgccgagctcgaggttggccgagaggatggccgggctgcgcaccacctgcgtgagaaaaacgaagtcgcgctgcgggtcgtagggcaacgtcttgtacagcgcgacgttgttgatgagcgagtcgccgagcgtgaccgcgatcgtgtagccgtcgggcgcggcccgcgccacctcgcccaggcctacggcgccgttcgcgccagcgcggttgtcgatgacgaaaggctggcccagcagcttggcggcatgctcgccgatcaggcgcgccacgaagtcgttggccccgccggcttgggccgtcacgacgacgcggatcggcttgcctgggaatgtcccctgcgcaatgctcgcgagcggcagcccggcgagcaaggcgaaacccatggtgagaaagtggcggcgcatcgaggactcctttgtctctgtgtgtcttgggattcttcgtgtggctcagccggcggccggcatgccccgctcgcgctcgatctcttgctgcagcagccggcggtactggaccagcgccgcgtccatgcccagcggcagcatctgcgcttcggaatcgatgttccggtattgcgcggtgatcatttcgcggtcttcctcgaatgcggtaacgaggcctcggtagatggtctcggtgaccgcggggtcggcgatgctgcttcggtgcgattgctggaagaagtagtgcgtggttgtttcggtctcgggcgtgagcgtctggcagctgtgcagctgcacgccgccgcgcaggtcgccctcggcctgccccaccggcgcgccgcccgatttcatcaacaaggtgccgggtagcacgaagtcatagatgaaatagcggtcgacgttccggtcgaagctctggaacgatttccagaagggcgacggaggaacgtcgggcacatgccgcgtcacgcggatgccgcgcggcaccttctcgatcttcggaacggcctgggcgatggccgtcgatccgccgagcgtgccttcgtgcacgtagctcaggtgcgagaagtccagcaggttgtcggagaccaggagatagggtgtgtcgtagtggacatagccgggcttgtggcgccagtcgggatggtcgcacgagaagttgtcgggcaagagagccggatccgccagcgtcggttcgcccatccagacgaacacccatttgttgtgcgagaccaccggataggttcgcacgcgcgccttcacgggaatgttcgccagcccgggtgcctccacgcaggccccgtcgggcgcgaacttgagaccgtgatagccgcagcgcacgcagtcgccttcgcggcgaccgcgagacagcggtgcatgccggtggcagcagcggtcctgcatggcgacgagttcgccggtctcggttcgatagaccaggatcggctccttgagcaccgtgcgcgtgaacagcgcgttggcggaaatctcgtgatcccacgcaatgacgtaccagcaatttcgaacccacatgcctgtctccaagagtccaggcaatgtagaaattcgcgcggcttccgtctgtccccgtcgaaggggacaaaaccctcagggcgatccctagtgagtaaaacgcagcagctgctgccgaccgtggatcgacagcttcagataggcgcgcttgcgcagcgtcgtcaccgtcgacgaggcaacgcccaggtcggcggcgacgccatcggcacccatgccgcaggcaatgcgcgcgcacacctcgcgctcgcgcgccgagagctgcggtgccgtgcgctgcagcgtgcgttcgatgcccgccacgcgcaatggcgtatcgggcgatgcaagctgcgcgaagagcgaattgcggtgcgcccgcttcaaaaggggcgccagccccagcagccgcgccacatccccctcctcgaactttccgttctgccggttgcggtagaggttgattgcaaatagcgtccggggtaccggcgagtagagaaagctcagccgccctgtcaactgccgcccaatgaagatctgctcacgccatgcggggtcggggatgtccgccgcgtcgtacagcatggcggtcacgggtgcgtgcgccggcgcctccgcactcatgcgcgcggccaggcgggtgatgtcgtccgcatgccggaagcgcttcttgtaaagcgaaaagcactcggccgtgatgttgtcgtgccggccggccgcatgcccttccacctgcgacggaacgccgtcgatgtactgcacgagcgagatgtattcgaccggcacgacatggttgatgaagtcgagcatgttgagcgcaggcgcctgctcgctgcctgcatcgagcaggtgcgcgacggcgccggcgtccagcatctggcccgcaggcggcgtgtcgagaaaccaggtggaaggcatcgcggctcaatataggcgagcggcgcccgattcaacagagtggaagcccgcgtgggccaggaggtcagcgaacacccatcgcgtggtcgagcgacagacgtccgccgccgcgacccaccaggtacagcagcagcgcagcccacgagaggtgcgtcggccatgcgtccggatagacgaacacctggatcaccagcgtcatgcccagcaaggccagcgccgacaggcgcgtgaagaggcccagcaccagcagcagtgggaacagatgctcagagtaggccgcgaggtgcgccgcaatctcgggcggcacgaacggcaacttgtattcggtgcgaaacagctcgtaggcgctgtcggtcagggtgagaaagccctcgaccttggtgcggccggagtagaagaagatcgccgccacggccacgcgtgtggccagtgccagcgcatcgtggctcacgatgcgcgtgagccgttcggccaccgagttccaatgcgcgcgaagaccacggtggttgctgctgtcgaccggcgcggaagcctgaaggtgggtgctcatggtgctctttcgttggatgcgggcgatgcacaggtgccggtgaatgcgccggcgcgcagcagggttgcaaagatggccgagatgtctgcctccgggtcggcagccagcgcgcgctctgccgcatcggcaagggtggcgccacccgcgcaggcgtcgagaaagacgcagcctgccttggtgatctcgtgccagttcaccgcgtcctgcggccgcgtgagcaatgcaccctcgcttctccaggccagctcaacgcctgtggcactctgctggcgattgcgctcccagatgctgtagaccggctgcgcgtcgaaccaggcccagcgtgcggccggatgcggtgcgagcacgaggcccgcgatccgctccggcgtgtggcgtgcgatccatgcggcgtcggcggcaggtgcgtcgggtgcggcatgggcttcgcgccagaggatgtcgagttgcgcgacgccgggcaggtagacgagttccgcggccggctcgaagccgcgcaggaaatcgggaaagccgccgccgtagtgcagcaggcgtccgtcgcgcggcacgtcggagaccacgtagagtgcggcggcggcgcgaaaccactgctcgcccaccagctgcgcaacggtgggaaagttggcctgcagcgcatcgatgcaggccttcatcaccgtgttgcggtacaccgagaaagcaggctgcatggcgagtgcccgcaccgccggatgcaccgcctgcaatggatcgaacagggcctctgcaaaggcctgctgaaactggccgtgcggcgtgttcatgccgtcgcctcctgcgccgcgcggtgcagttcaatggcagcttgttcctgctcggccatgagttcttcgaaggccggcacattgccgtcgcgctcgatcagcgtgggccgtgcgcccgcgctttcgacgaagcgccgatacagctgccagacttctggcgcgatgggcgcatcgtgcgaatcgatcagcagggcgtcacccagcgtgggatcggcggtgtggcccgcaaggtgaatctcgccgaccagtgcctgagggaaccggtcgatccaggccgcggcagaaaaaccgaggttgcgtgcggacacatacacgttgttgatgtcgagcagcagtttgcagccggtgcgccgcgccagctcggcaagaaaatcgatctcgtcccattcgtggccgtcgatgtgcaggtagtgcgacgggttctcgatggcgatcgcggtgcccagcgcgtcctgcgtgcgcgcgatgttggaagcgatgcgatgcagcgcggcggtggtgcgctgaaaaggcaggagatcgggaaagtattgaccgttccacgtcgaccacgccaggtgctcggagatcaaggcgggctggatgcgccggacaagctccgccagccgctcgagatgcgcggcgtcgggttccgcttcgcccgcgagcgagagtgagacgccatgcagcgacaccggatggcgcgagcggatcgcttcgagccatccgatgcgcggcccgcccgccaccatgtagttctcggggtgcacctcgaaccagaggccctcggcacgcgcgccgagcgcggcctcgtagtgctccggcttgaggccgagaccggccgcaagagtggcagacatggcggcgtgcgcagtgcgtcgtcgatcaggatttgatcggtgccagtgagcccatgcccttgggcgtcttgatcgtggtgcaggtgccggccggaacgttcttccaggcgttgccctggtagtcgaccttggaggtgcccgcgcaggtggtgccggggccggcggcgcaatcgttcttgccggccatcgagacgccgtagcacttttccatcgtggccatcttgtcggccatcggtttgtcttgcgccatggcggagccggcggcaagggcacccagcgcaagggcggtgatcgcgaaggaacggttgatcatggatgaactccgaagattgattgaagatttgcaaccacgccccaatgcgcggtcacttgctagttcgcaagttgcgcggccggggttacaccgcagtggacgatgggccagatttttttgcaccatcgatcgttgcaacgagcagcgatacactgaggccgatatgagcggacatcgctacttccgacgttgcacgaccgcgttcctcgtggtcctgtcgctgctgttttcgcagctggcgctggcgagctacgtctgccccggcgaagcagaggcggcatcgatggccggaatgacaatggcggcgggcgagccgtgcgaaggcatggatgccgcccagcccgtgctgtgccaccagcatgccgccgacatgtcgctgtccttcgagccggtgaagctcgcgacgccttcgctgcccgccatcgcgcaggttctgctcgtgccgctgatgctggagccgcaagaccaggcgctgccgcagcaggcgcgtcccgaacggcagcatccgccgcccgatcccgtctttctcgcgaccctccgacttcgcgtctgaaatctccgtcgaccgactggtgccggcgcggctcgtccgcttgccggcgattgtctcgttcgtccgcggagttgccatgtccattcttttttcccgcgcaaccgcaatggttgttgcgctgctgccgtgccttgcgacggcggcccccctttccctcgaggccgcgctccagctcgcggcccagcgctccgaaaccgccagggccgcccgcgccggagtcctgagtgcgagggaggcgtcgcatgcggcggcacagcttcccgacccgacgctgcgtgtcggcatcgacaacctgccggcgacagggcccgaccgttttcacactgcgcgcgaatcgatgacgatgaagcgcattggcatcagccaggaatggctctccgccggcaagcgtgcggcgcgccaggcggccgccgatgcggcggtcggccgggaaacggtgcaggcgcaggctgccgccgccgagacgcgcctgcagaccgcgctcgcctacctggatgccttctacgctggcgagagcctgaagctcgcaacgcgcatggagcaccatgcgcacgaagagctggaggcctcgcgtgcgcgcctgtcctcggctgcggggagcagccaggacgtgctggcgctgacgggcgcacgcggcgtctcggaagacggcacggcagaaatccggcaacagcagaacactgcccgcgtcgcattgcagcgctggatcggcgtgcagccggacgagttgcagcccccaggcgccgttgcgcttcctagcgaagaggcgtatgtcgccgcgcaccccacggttgcggcgatgcagcgcgatgccgatgtggccagacaggccgcggcggtcgctgcgtccaaccgcaagcccaactggacctgggagcttgcctacggccagcgtaccggctattcggacatggtgtcggtgggcgtgagcattccgctgcccgtggcacccggcgaacgccaggaccgcgacaccgccgccaagctggcgctggccgagaaggcagaagccgaactggccgaggccacccgcgccgccacggccgagtaccgcaccctgcttggcgatgcgcagcgcctgcagcagcgcgtcgaccgctaccgcactggtgtggtcgtgcccgccggccagcgcacggccgccgcgatggcttcctaccgctccaatcagggcagtctgctcgccctgttcgaggcgcggcacgccgaagtcgaagcgcagcgcaagctgctggcgctgcagcgcgatcttgccaagacacacatccaactggcctttcggccgctgactgccgaggtggcgcaatgaaccggacactgaccatcggcgtatcgctgctgggcgccctgctgctcgcagccggcactttctacctgggccgcaagacaggccagatcgcaaccatggcggccgcgccggcagccagcgccacggcggacggtcgcaaggttctctactggcacgaccccatggtgccgggaccgcgcttcgacaaacccggcaagtcgccgttcatggacatgcagctggtgcccatgtacgccgacaacgccgcgaacgaagccggcgtcagaatcagccccgccgtgcaacagaacctcggcattcgatatgccagcgttcggcggaccgaaacctcctcgtcgttcgatgcgatcgggacggtgcagttcgacgagcgcctgaacgtggcggtgcagacgcgcgtggccggctatgtcgagcagttgtcggtgcgggcaccgatggagcgcgtgcgcaagggccaggccctggccaccgtcttcgcacccgactggctcggaccgcagaacgaatggctcgcgctcaagcgctcgggggtctcggccgatctggtcgcggctgcccgcgaccgcatgcgggccctgtccattcccgccgagctcatccggcgcagcgaggaaaccggcaccgcacaagcgcgctacgtgctcactgcgccaatcgacggcgtggtggccgagctgggcgtgcgcgagggtgtcgctgttgcgccgggcaccacgctgttccgcatcgcgggtctgcagaaaatatgggcagtggccgagatcccggaagcgcaggcggtgcgcctcgcgcgcggccagaaggccaaggccgttctgcaggccgatgcgtcgcagtcgttcgacggaacgctcgacgaaatcctgcccgagatcaatgcaaccactcgcaccttgaaggcccgcttcgaggtcgacaacaggaacggaaagctcacacccggcatgctgctgcgccttcaggtggcgggaccggccatcacgcggctggtggtgccttcggaggccgtcatccgcaccgggcgacgtgccgtcgtcatcgtgcgcaaggccgacggcgccttcgagccgcgcgacgtgtcgctgggcgcggatgcgggggacgataccgaagtcgtctcgggcttgtccgaaggtgaccaggtcgtggcaagcgggcaattcctgatcgactcggaagcccggctgcggtccgtgctcggcagcatgacggcgaccgcaccggcatcggcaccggccgcagtgctgcacaaggccgaaggcagggtcgagggcgtggcgcccgatggcatcaccatttcgcacggacccgtcgcaacgctccagtggccctcgatgaccatgggcttcggcaaggcgtcgcccggcgcgttccccgagatcaagccgggtgaccaggtacgtttcgagttcaaggagggcggctccatgggctatgagctcgtctccgtgcagcgcgcgcaaccgggcgcccaacgatgatcgccgccctgatccgctggtcgatcggcaaccgcttcctggtgctgatcgccaccgtgtttctgatggccgcgggatggtggtcggtggcccgcacaccgctcgatgccttgcccgatctctcggacacgcaggtcatcatccgcacgccctaccccggcaaggcgccgcaggtggtcgaggacctggtgacctacccgctgaccaccaccatgctcagcgtgcccggtgccaagatcgtgcgcggctactcgttcttcggcgactcgttcgtctacgtgctgttcgacgacaagaccgatccgtactgggcgcgctcccgcgtggtggagtacctcaaccaggtgcaggccaggcttcccgcgggcgccagcgcttcgctgggtcccgacgcgacaggcgtgggctgggtctacgagtacgcgctgatcgaccgcaccggcacacgcgacatcgggcaactgcgcgcactgaatgactggttcctcaagttcgaactcaagaccgtacccgacgtggccgaggtcgcgagcatcggcggcatggtgcgccaataccaggtggtgctcgaccccgaccgcatgcgcgcgctgggcatcacgcagtcgacggtcgtggaggcactgcaaaaggccaaccaggcatcgggcggctcggtcgtcgaattcgcggaggccgaatacatggtgcgttcgcggggctacctgcgttcgctcgacgattttcgaacgataccgctctcggtgacgggcacgacgcccgtgctgctgcgcgacgtggccgcggtgcagatcggccccgagatgcgccgtggcatcgccgagctggacggcgaaggcgaagtggccggcggcgtcatcgtcatgcgctcgggcaagaacgcccgcagggtcatcgaggccgtcaaggcaaagctcgaaacgctcaagcccagcctgccgccgggcgtggagatcgtgcctgcctatgaccgctcgctcctgattgaccgtgccgtcgagaaccttcgcagcaagctgatcgaggagttcgtcgtcgtggcgctggtctgcgcggtcttcctttttcacctgcgctcggcgctcgtggcggtcgtgaccttgccgatcggcgtgttggcggcgttcgtcgtcatgcattggcagggcgtcaacgccaacatcatgtcgctgggcggcatcgcgatcgccatcggcgcgatggtggacggtgccatcgtgatggtcgagaacgtgcacaagcacatcgaagccttcgagacggcaaagggccgccagcccacggtggcggagcgatggcaactcgtcgccgatgcgtcggtggaggtcggtcctgcgctgttcttttcgctgctggtgatcacgctgtccttcgtgcccgtgttctcgctcgaggcgcaggagggtcggctgttctcgccgctggcattcaccaagacctatgcgatggccgctgcggcaggcctgtcggtgacgctgataccggtgctcatgggctatctggtgcgcggacgcattccgcgcgaaggcgccaaccccgtgaatcgcttcctgatggcggtgtaccggcccgcgctggaactggtgctgcgatttcccaagggaacgctcgccatcgctgcagtgttgctggtactgaccgcgatcccgctgacgcggctgggtggcgagttcatgccacccctggatgaaggcgacctgctctacatgccctctgcgctgcccggcctttcggtgtcgaaggcgtccgaactgctgcagcagaccgaccgattgatcaagaccgtgcccgaggtcgagcgcgtgttcggcaaggccggccgggcagacacggcaaccgacccggcgccgctcgagatgttcgagaccaccattcagttcaagcccagggcgcaatggcgggcgggcatgacggccgacaggctggtcgaagaactggatcgtgccgtgaaggtgccgggcctgagcaacgtgtgggtgccgccgatccgcaaccgcatcgacatgctggccacgggcatcaagagccccgtcggcatcaaggtggcggggaccgacctggccaccatcgacgcgctgaccatgcagatcgaggcggcggtcaagaacgttcccggcgtctcgtcggcgctggcggagcggctcaccggagggcgctatatcgatgtcgacgtcgatcggctcgccgcggcgcgccatggcctctcggtggcggacgtgcaggccgtggtgtcgacggcaatcggcggcgagaacgtcggcgaggtcatccaggggcgcgagcgctatcccatcaacctccggtatccacgcgagatccgcgattcgctggagcggcttcggcagctgcctttcgtgacggcccagggcgcgcagttgctgctgggcgatgtcgcgaagatcgccatcgccgacggaccgccgatgctgcgcagcgagaacgcgcggctgtcgggctgggtctacgtggacgtgcgcggccgggacctgcgctccgccgtcaacgacatgcaggcggccgtcggccaagccgtgaagatgcccgccgggtacgcgatgtcgtggtccggccagttcgaatacctggagcgcgcgacggagcgcctgaagctggtcgttccggcaacgctggcggtcatcttcgtgctgctatacctgctcttccggtccttcggcgaggcggccctggtgatggccgccgtgccgttctcactcatcggcggcttctggctcatctgggcgatgggccactcgatctccgtggccacggcggtgggcttcatcgcgctggccggcgtggcggccgagttcggcgtggtgatgctcgtctatctgaagaacgccctggcgcgacgcctcgaagccggggagccgatgaacgaccagaccctgctggccgcgatccgcgaaggcgccgtgctgcgggtgcggcccaaggcgatgaccgtggccgtcgtgatagcgggccttctgcccattctctggggcagcggcaccggttccgaggtgatgacgcgcatcgccgcgcccatggtgggcggcatggtcaccgcgccgctcctgagcctgctcgtggtgcccgctgcgtggtacctgatgcgccggcgcgcccagccctgggctcacccgccgtcggtgcagcgaaccggcagcgcattcagcggaatgcgcaggtagcacacgccgttgtcatcgggcggaggcagccggccggcgcgcacgttgacctggatcgaaggcaggatgagcgtcggtacatccagtgtggcgtcgcgcgcgcggcgcatggcgacgaactcgtcctcggcgatgccgtcgcgcacgtggatgttgcgcgcgcgctgctccgcgaccgtggtctgccactgtgccatccgcgatgcgggcgggtagtcgtggcagacatacatcggcgtctcgggtggcaggtcgagcaggcgccgcatcgatgcgtacagctggtgcgcgtcgcccccggggaagtcggcccgcgcgctgccgaggtccggcatgaagagcgtgtcgccgacgaaggccgcgccgccgatcagataagccatgtcggcgggcgtgtgccccggcacgaggatggcggtggcctcgatgccgccgatgcggaaggtctcgccatccttgaagagatggtcgaactggctgccgtcgggcaggaagctgcgctccaggttgtagagcttcttgaaggtggcctgcaccgtgcggatgttctcgccgatggcaatgcgcccgccgatccgcgcctgaaggtagccggccgccgaaaggtgatcggcatgcgcatgggtctccaggatccagtcgacctgcagcccgtgttcggcgacgcacgccagcacccggtcggcgcaggcggtggcggtgtggcccgacttgaagtcgtagtcgagcaccggatcgatgacggcagcccgcaacgtggccgggtcccatgcgaggtaggagaccgttccggtcctcgggtcgaagaaggcctggacgttggcggatgtgttcatggctgcctcgcgggtctattaattgatctatcgataaatattctatatattggtatattgttgtcaacgccgatgaaatggacgaccgactcatgcctgctgtgcgaaccatgaaatccccgccccccgtcttcgatgccgaggtgctgcgcggcgccgccgctcgcgcggtcggcgtgatgaaggtgttggccaacgaggaccgcatgctgctgctgtgccagctttcgcagggagagatgtgcgtgagcgagctcgaagcgcagctagacatccgccaaccgacgctgtcgcaacagctgggcgtgctgcgcaacgagggcgtggtcaccacgcgacggcaaggcaagaacatcttctacgccgtggccgatccggcgctgctcgagatcctggccctgctctaccgcatctactgcccgaaggaagaatgatgaccatcgactggactgtatttacgccatggacggcgctggcgggcggcgtgctcgtcggcgcggccactgcgatgtttctgctgctcaacggccgcatcgccggcatcagcggcatcgttggcggactgcttcggctcgtcagcggcgacgtggcgtggcgcgtggccttcgttgccggccttgtcgttgcgccaatggtctatgcgatcttcacggactggccgaagccgcagatcgaggccggctatggcacgctggtgttggccggtctgctggtcggcgtgggcacgcgctacgcggcgggatgcacgagcggccacggcgtctgcggcctgtcacgcctgtcgccgcgctccttcgcggccaccgcggtcttcatgggggccgggttcctgaccgtgttcctcatgcgccaccttctgggtctctgaggaacactgccatggccttcttcacttcatttctcgccggtctggtgttcggcctgggcctgatcgtctccggcatggccaatcccgccaaggtgctcggcttcctggacctgggtggacgatgggatccgtcgcttgctttcgtgatggccggtgcgattgccgtcggagccgttgcgtttgcagtggccaggaggcgcacgcagtcgctgctcggcgcggcgatgcagctgcccagcctgcggtcgatcgatcggcgcctcctcattggcagcgccgtgttcggcctcggctggggcatcgcgggtttctgtccgggcccggcgttggtggcagtgggcatgggacaagccaaggcgctggtcttcgtgatcgcgatgctggccggcatgggcgtttttgaatggctcgaggggcgcaaggaagcgaagcacccgcgagagaagcgttcgaaggcgcatggacgccggcgatccgtgtcgcgttgatcgagttgcgcgtgccgtcgagaaagagtgtgaatagcgtcggttcgccccgtcactgcagcagcgcaggcgccggcgcgaggcagcgctgcacgaaggccgacaaggcacccacgtcggggatctgcacgtcgcggcggcccttctcgacaaactcgatgaccttgtcgcgtgcgagccgcgacagcgcccggctcacgctctccagcgtcatgcccaggtagttgccgatctcggcacgcgtcatgcgcagcgtgatctggtcggtccgcatgccacgctcggccagcgactcggcccagtagcgcagaaaatccgccacccgcgcatcggccggcagcgtgcacaccgacatcagcgaatcgcggtcatgggcgatctcgcggctcatggcggtgtggaacacctgcagcaacgtgggttcggccaggcaggcggcaagcagcgattcgtacgagaccacccagacctcgcccgtgtccatggcgacggcgtcgcacgaatagtgtccgccggcgatgccgtcgaagccgagccagtcgccgcggaacttgaggcccaccacctgctcgcggccgtccgcggacaggttcacgatcttgaacaaacccgagttcacgatgtacaggttgccgaagcgctcgcccgactggtagatcacgtcgccggcgtgcaccacgcggcgttgcggggccaggcgctcctgcaggagcttctgcgtttccaccagcttctggcaggcccgctcatgaatcgccctgccttccggcggcaacgcgcgcgttgcgagaaagccggtcatcgccggtgcggcggtttcggtgcgggcggggttgtacatgtgaagagctcctggagatgtgtatgtcgcgggtcgatggaggaatgctaggaagcgcgcggcaacacagtgacaacactcgaagtcggtcggtaacgctgggtgaatggtttgtgtccggtgggtaacagcgcccacccgcgcgccgctttgatctgcatcaagagcggccggcccgctgcggctagccttcctgcgtcacacaagggagttcatgcgctttcccttcgaaatccataattcgtcggccttccagaccttgctgcctgaggacgagacagccctgctcgggcgcgcccgtctcctccaggcggcgtggctacgcgccgcttttccgctgcagctcaaggggaagaatctcgggatcttttgtgacgaaggaagcgaaggcagcgagagccgggcgctgttccaatgcgcggcggaggcgctgggcgcgcatgtcgcgaccattcgccccgccctttccagcctgggcagccccggtgaggtccggcacacggcacagatcctgagccgtttctacgacgcggtggagtgccaggggatggcgccggaactcgtgcggcagatcggccgggaagctgccattcccgtctatgacggcattgcctgcggggcccatcccacggcggcgctcgccgatcggctcgacgaccggacatcgcctgaggacaacaggcgattcgtgctgcaggcgttgctgctgggcagcattggctgaggagtgagcggggcgccttcgtgcggcatgatgcccttgcccctccaagtaaatacactaacggcaagcggattagcaacaaccacgactgtccaaggctctaccccatcgcctgttctccaacatcaaggcccgccgttagcgtatttttatgtcgtcacttccactcttccccgagccctccggcgaatcgcatcaggccgctttcgaccgttggctcgcggcgcagcaggaaaacggggccttgcggcagccctcttcgatcgcggtctaccgggacatgtggggcagtttcacggcctggtgcctgggccagtcgcccgccgtgacactggcgtcgctggacatgggcgacctgtcggcgttccagcaggcgcgcttcggcatgaagagcgacgacctgtcgctgtctccgcgttatgcgctgcgcctgctccggctcatcgaccgggtgctgcgccaccatgcggagacccacggaacgcccgccaacgccgcggcctcggaatggatcgcgacccagcccgaggttcgctatgcggattcggcgcgggcggatcccctgccggaatttctctcggtctccgaggcccggcatctcatcacctttctttccagcgcccggccccggcccggcgaccggcacggccaggccgcgctcagctggcaggcattgcgcaatcgggtggctgtcgccctgcagctgggcgcggggctcacgcccggcgacgtccgcgtgctgcggctcgacgcgccgacatcgcagatcgccggccggcgcgaacgtccgtggaaggttgccgtgccgggcaacggcaactcgccggcgcgcgaggcacccatcgctccttgggcaggcgagctgctccagcattggctgaaagtgcgcgccgagacgacgattgcgggcgacttcctgtttccggccacgcgcaccggcaagccctggagcaaggaagcgcagtatgtggccgccaaacaggtgctcgaagacgcgggcatcgatgccgccggcggcgggtcgttcctgctgcgccacaccttcgcgctgcgccagctgcgccgcggcgccaagctcgaccaggtggcgcgctggctcggcatcgagcccgaggcgatgggcaaatatcagcgcgtgctcacgggtccggccgaagtcatctgagcgccagccggcggctccgcgccggcatcagtcgacaagcgcgcgcttgacgtcttcctgcagactgcgcagatgcgcgcgcatcgccgcgcgcgcccgttcgggatccctcgcgcgcaaggccgagatgatctcgccgtgctcttcatggttttcacgctggcggtgcaacgggctgtgcagccggaacagccgtgcgttcacgcgcagttcctcgaccaggcgcggcagcaccacattgccgctggccgacgaaatgagttgatggaatcggtcgtcgaagtgccagtgctcgatctcgtcgtgctccccggcgtcgagcgtcttcagatcggcgtccagttcatcgagctgcgcttcggtgatcttgtcgaccgccagcacgatggcctcgcactcgatgatctcgcgcgcccgcatgcagtcgaagtactccttggtgcccagcgcgcgcaccgcgtatgaacgcgcgtcgcggcgcacgagcaaaccttcgcccgcaagccggacgagtgcttcacgcatcggcgtgcgcgaaatccgcagttcgtccgcgaggcggccttcctgcagcgggctgcccgccgaaatcttgcgatcgaggatcagcgtgcgcagtctcgagtaggcctgctcggccaggctcgcggagcggacttcgagcggcgcgatggtgattgtggctggctgagccgggctgggaaggcttggcatgcgtgagaagttgattgccacgaaaggtggggaaacgcctggaaggccagccgcggcggggctgaaagcttcacagccatttggcgagcggattctcggcgttgggcgcgcgcgggcgcaggcagggctggaactctcccgcacctgcttccgccgagaacacgccattttcccataccacccgccccctcgaaagcgtgattcccggccaggcgcgcatcttcatgccctcgtagggcgtgtagtcggccgcatggtggagcatgtcgttgcggatgactttttcgtggccctcgccgaacgtgtcccacaccaccaggtccgcatcgctgccgaccgcgatcgtgccctttttcggatacagcccgtagagccgcgccggattggtcgacgtgagttcgacgaagcggtggacgtcgatgcgccccgtcagcacgccttcgctcatcagcagcggaagccgggtttcgacacctggaatgccgttgggaatgcggtcgaaggacgcatcctcgccggccacgcgcttgccgtcgctgccatggatgttgaagggcgcatggtcggaagagaagatcgtgaaaaggccgctcgaaagcgcgttccagatgaactgctggttggccttgtcgcgcggcggcgggctgcagatgcagcgtgcgccgtgcatcggatcgttggggtccacccccaggtcttccgcgctcaggaaaaggtactgcgggcaggtctcggcatggatcggcaacccgcgcccgcgcgcccagtgaatctgctcgaccgcctcgcggcccgagacgtggacgatcaggatcggtgtatcgatcagctcggccagcgcaatcgcgcggtgcgtggcttcgcgctccaccgccatcggccgcgagctcccgtgatagcgcggcgccgtcagcccggcatcgagcaactgctcggtgagccaggcgatgcagtcgctgttctcggcatggatcatggtcatcgcgccgtgccggcgcgccaccgcgagcacctcgatgatctgccggtcggcgagcttcaggtcgtcgtaggtcatgtagatcttgaacgaggtgtagcccttctcgatcaatgccggcagctcgcgctgcgtcacgtccttggtcgcgtccgcgacgatcagatgaaacgcatagtcgatcaccgccttgccttcggcgcgccggtgatagtcgtccacagcttcctgcatgctgcgccccttctgctgcgcggcgaacggcagcaccgtggtggtgccgccgcaggccgccgagcgcgtgccggtgaagaagtcgtccgagaagcgcgagccgtcgctggtcggctggtcgaagtggcagtggccgtcgacgccaccgggcgtcaccagccggccggccgcgtcgatctctcgcgcggcgctgccgtccagtcgatgggcgatggcgctgatgcgcccgtcgcgcacaccgatgtcggcgcggtagcggtcgcccacggtggcgatgtcggcattgcgaagaatcaggtcgtaggagctcatcgatgggtcccggtcaacgttgttcgagcacggcatcggccaccaccggcgcgtcggtgccggtggtgccgttgcggtaggcgcggccgtagtggcgctcgatgcggcgctggatgaaatcccacgccgtggtcatcagcaggtagtagatggcggcgacgatgaacagctccagcaccatgaatttctcctggatcagcacctgggtgcggcgcagcagttcttccatcgagatcaccgaggtgatcgaggtggtcttgagcaggccgttgatgctgttgcccagcgtcgggatgatcagccgcatcgcctgcggcatcacgatgtagcgcatgctctgcgcactgctgaagcccatggcgcgcgccgcgttggtctggcccaccggcaccgactggatgccgccgcgcaccacctccgcgaggtaggccgcctcgttgaggatcagcccgagcagcgccgattcgatcaccgacaacttgagcccgagctgcggcagcccggtatagatgatgatcagctgcaccaggagcggcgtgccgcggaagacccagatgtagaaatgcgccggtgccaccagccagcggtggcgcgacaggcgggccagggccagcgcacatccgacgaccaggccgcccgcgatcgacgcgagggtcagccagagcgtggtgagcgcaccgttcaggatgtacggattgaacaggtagtcggcaaaccccgaccagctccagccttgtcccatggactttccctctcgaactcagtggtggtgcggcgcgcttagctggcggggcccttgacgacgacggcaccgtcgatcgccttgacgccgtattgatcgaacagcttctggaagctgccgtcggccttcatgtcgttgagcgccttggccatcgcaaccgacaggtccttgtttttcgcggccagcgccaccggggtggggaacaggccgctcagcacgcggtcgaaatcgccgcgcttctggtactcggcaccggtggagtcgatcgacagcgccacctccacctgcccggcgcgcagcgcctggaaggccatcgcgaagttctcgaaggtccggatggtcatgcccttcatgcccctgtcggtcagctgcttgtcgagttcgcgcgccttgcgctcctcgaatccgccgatctcgacgccgatgctcttgcccgacaggtcatcgggcttgctgatcttgagcgggttgccgcgcgcggtgctgatgctgatcgcctggtcctcgtagggcagcatctgcatcaacttggcacgctcgtcggtgtagaagatgccggtgttgatcacatcccagcggccagcctgcaggccgggaatcatggccgagaactcgatgcgcacgtattcgggcgtcaggcacaggcgcttggcaatcgcttcgccgagttccacccgcatgcccttgagggcgccggtctggtcgacgaactgcatcggcggcaaggtcgggttgaccgacatgatcagcgtgcccttcttgatcagcgccgagtcgggcaccggcgacttgcaggcctgggcgttcgcgatgcccatgccgaggatgaaaagaaccgtggccgacgtgagagcgggaagcagtttcatggtgatttcctggtggagatggagcgaggcaagagatgggggattgaagggtcgggcgctgctcaggccttgatcgagccgagcaggccgaggcggtcgagctcgcgccgcaggtcgatggcgtcggcttcgggcagcggcaggcgcggcgcgcgcggctggccgaccggcaggcccatcattccgagtccgtgcttggaggccgcgacatagcggtggccgccgacccagcgcacgatcggcagcatttccttgtagagggcgagggccgcgggcatgtcctgctcgtcggcgaccagttcgaacagccgcgccgacatcttcgggatcaggttcgagcagaccgcgacccagccctgcgcgcccagccagaacgactcgtagcccaggatgcccgcgaacaccgtcatgcggtcgccgcagagctcgatgatgtcgcgcactcgcgtcacttcgagcgtcgattccttgatgtacctgcagttgtcgatgcgcgaaagccgcgccaccagttccggcttgagatcgacgttcgccgtggccgggttgttgtaaaccatgatcggcacgccgatcgcctcgcccaccttgcggtagtgcgcgaacagttcgtcgtcggtgggggtgctgtagaacggcggaatgatcatgacgccgtcggcgcccatggtctccgcctcgcggctcagccgcacgcactcgtcggtccactcggcgccggtgccgatcagtacgggcacgcgttttgctgccgtctgcacacaggtctcgatcaccaactgccgctcctcggccgtcaacgacaggaattcgccggtgctgcccaggggaatcagcccgtggatgccctcttcgatctgccagtcgacgagcctcttcagggccggcacgtccacctgctttccgtcggcggtcatgggggtgatgagcaccgtataggtgcctcggaacgctgtcattccagtccttattgaaaaaattggggcgacgaagtatttgtatacgttcagtatacgtatacattagaccatgtccaagtggttttttgcttcgcacctgtttcaatgagcacccgactgacccattcctccatcgctgccggcggacgcccgatccgcttctggtacgacggacagcccgtggacggtctcgagggcgaaaccgtggctgccgcgctcgcggccagccatctccggcagatgcggcacacgcagggcggcggacgccgcggcctgtattgcgggatgggcgcctgcttcgactgcctcgtgaccatcgacggccgggccagccagcgcgcctgcctgaccaaggccgcggacggccagcagatccgctcaaccatgccggccgggacgcctgccgatccattgcatccgctggcacccgacgcgggggcccggccgttggcgcgcgaggtcgacgtgctggtgatcggcgccggcccggccggcctctcggcggcgctcgcggcccggcgcgcgggcgccggcgtgttggtgctcgacgagcggctgcagtccggcggccagttcttcaagccgctggcaccgtcgcaccaggccgcgacaccgccggaccgacagtttgcggacggcctggcgctggagcgcgaagtgctcgccgccggcgtcacgattcagcaaaacgcgcaggtctgggccgcgttttcgccgcacgacgtcagcgcgctgatcgacgggcaggccacccacatccgatgccggcagctggtgatcgcgccgggtgcctacgagcggccggtgcccttcccgggctggacgctgccgggcgtgatgaccaccggcgccgcccagacgctggcgcgggcctaccgcgtcgcgccgggacagcgcgtggtgatcgccggcaacgggccgctcaacctgcagctggccgcggaactgcttgccggcggcgcccaggtcgtcgcggtgctcgaatcggcggcccgcccgtccgcgcgcgactggcgccagctgctcgccgccgcccgcaccgcgcccgacctgctgcgccagggctggggctacttgcggcagctgcgcgcccacaaggttccgctgctgtggggccatgcagtggtcggcgccgaaggcgaggccgaactgcaggcggtgcaggccgcgcggctcgacgcccacggccgtgccgcgccttccccggcgctgcgcttcgaggccgacacgctgtgcctgggctacggcttcatcccctcgaccgagctggcgcgcatgctcggctgcgaacaccgcctggccgaccggcacctgggctacctcgcgaccgtgacgggcaccgacggcgccaccagcctgcccggcgtgttcgtggtcggcgacggtgccgacatgggcggctcgcgcgtcgcattggcgcgcggcgcgctggccggcactgcggcggcacgcaacatcggcctgaccgcctccgaaccgtccggcgccggggaccggttgcgccgcgccgagcgcttccagcaggcgctgtggtcgctttaccgcgcgccgcccgtggcgctggccacggtcagcgacgacacgctgctgtgccgctgcgaggagatcagcttcggttcggtgcgcgagcagatccgggccggccgcgacacgctggccgcgctgaagcgcaacacgcggctcggcatggggcgctgccagggccgctattgcgcggtcaccgcggccaggttgatcggcgagatgacccggcgcccgaccgaggtcgagcagtatttcgcgccgcggccgccggccaggccggtgcccgcgggcgcactcggcttcgagaagcccgaatggggcggccacaagccggcgatcacgccgaacctcgcgcggcctgtcgaacgggcggcctttcacatcctccgcaccgacgtgctggtgatcggcgccggcgtgctcggttcctgcctggggtactacctggcgaaggccggccaggaagtgacggtggtcgaccgcgacgacatcaatctgcaggcctccggcgccaacgcgggaagcctgcatgtccagctgctgtccttcgacttcggcgccaaggcgcagcaaggtggcggcccggccgcagccaccctgcccctcggcccgatgtcggtgcggctctggcaggagatccaggccgattgcggcgaagaagacctcgagatcaagatcacgggcgggctgatggtggccgacagcgaggccggcatgcgcttcctcgaggccaaggccgcgctcgagcgcagccatggcatcgacgcgcaagtcatcgacggcgccgaactgcgccggctcgcacccgcgctatccggaaaactgctgggcgccgacctgtgcccgatggaaggcaagatcaaccccctgcgcgcgacctatgcggtggcctcgcgcgcgcagcagcagggcgcgcgctttcttcgcggctgcgacgtgatgcgcatcgaacgccggccgggcagcggcgccggcttcgtcgttcacacctcgcgcggcaccatccacgcaggccgcgtggtgaacgccagcggcgcctggtcgagcacggtcggcgacatgctcggcatcaggatacccgtcaagggcgcaccgctgcagatgatcgtgaccgaaccggcgccgccgctggtcaaccacctggtggcacatgccgaccgccatctgagcctcaagcaggcggccaccggcggcctgctcatcggcggcggctggacggccgcctttcacgaaggcatgcgcctgaaccgcgccgagcgcgacagcatcgaaggaagcctctgggtcgcgcgccaggtgctgccggccgtgagcgggctgcacatggtgcgctgctgggccggcatgaacgtcaacatcgacggcgcgccgatcatcggcagcgtccccggcctgcccggcttctacaacgccgtgacctccaacggctacacgctggcacccatcaccgctcacctgttggccgacctgatcgtgcgcggccgcaccgacatcgacatcactcctttccacatcgaccgctttctttgacgccatgacagacctttcaacctcgcgcgacacgctgcgccaattcatcgacacccatttcgaccatcaggtcgaaaccctcgcgcggctggtgcaatgcccctccgacaacccgcccggcgactgcgccccgcacgccgaactcacggcccggctgctcgaggccatggacctgaaggtcgaacgccatccggtgccggccgcattcgcagagcagcacggcatgcgcagcgtgaccaacctgatcgtgcgcgagcgcttcggcgatgggccggtgattgcactcaatgcacacggcgacgtggtgccgcccggctcgggctggagcggttcgccctatggcggcgaggtgcgcgacggctggctgtacggccgcggcgccgcggtctcgaagtcggatttcacgacctacgctttcgcgatgcgtgcgctcaggcagttgcagtcatcgggcgcggcgctggccggcacggtcgagctgcacttgacctacgacgaggaaaccggcggcatgaccggccccgcatggattctttcgcagggcctgagctggccggactacgtgatatcggccgccttctcgcatcacgtggtggtggcgcacaacggctgcctgcatctggaagtgacgctgcgcggcaagtccgcccatgcggcgaggcccgacaccggcgtcgacgcgatcgaggcttcggcgaccttgctgccggcgctctaccgctatcgcgaccagctggcggagcggccctcgcaaacgccgggcatcacgcatccgacgatgatcgtcggcctgatcgaaggcggcatcaacaccaacgtggtggccgacgcgctgagcctgcggatcgaccgccgcatcgtgcccgaagaagtgcccgaggacgtcgaggccgaactgcgccaggtcatcgagcaagcctgcagcggcctgccggggatctccgtcgagatccggcagatcctgctggcccggccgttcgcgcccgcccccggcgcagaggccttcgccgagctgatgtgccgcgaagccagcgccgtgatgggcaagccggtcacgccgatcggcgtgccgctctacaccgatgcgcggctctacagcgaagccggcattccgaccgtgatgtacggcgcgggccccgcgtcgctgctcgaagccaacggccatcgcgccgacgagcgcgtgccgctcgatgaactgcacaaggcgaccgtcgtggtcgccaacacgctgctgcaactcctgacccagccggagaaatcactgctcgggccgacgccatagccagatggcgacggccgccatgaagagcggcgcgccgatcttcacggcgacgggtgcgccggtggcaagcagcacaagcgcgctgaaggtcatcatcacggtcgcggcccatttcgctcggcgcggcaccgcgcctctttcctgccatcgccggatgtactcgccgtagcggggatgttcgagaagccagcgctccaatgcaggccagccgtggcccgccgcccaggcggccgcgagcagaaagggcaccgtcggcagaacggggagaaaggcgccgatcaggccgagggcgacaaacaccagcgccagcacgcgccagagcagcctcgcgacgggacctttgggccgcatcaggacgcgtgcactccgaaaaagcgatctgcggggaagtgcgaagcgggcatcggcggatggtaagccaacggtccgcccggaggatgcgcttcaagccgcatcgggcccgccatcctggttccagtagccgccgttcatcaggctggcgcgcaccatggcccgggcgcgatgcagccggctcttcaccgcctccacgctcaggcccaggctttgcgccacctcgggggcggtcagttcctcgacgtcgcgcaggatcagcgcgacgcgataggcctccgggagcgcggcaatggctttcgtcaggtccaggcgcaggtcggtcggaatccgcggcgccgccagctcgtcggacagcggctccgacagccggcccttggccgcgctgcgcctgaagatccggtagcactcacgctcgatgatccggaacagccaggtggcaaaggcggccacggtcccgagcgtgccgatcttccggtgcagctgccacagcgccacctgcaccgcgtcttcggcgtcctcgctgttggcgcaggtgcggcgcgcgaaacgcttgagatcgggctggcaggtgcgcagcagctgcgacagcgccccttcgtcccccgcacaggcggcctcgatcagcggcgcggacgcgcggatcatttcagcggcccgatggccctgcggccgagcatcgcgcaggctgggcagaacccgacgacggcggtggcgccgagcatgcccgccgcggcgaagcccagcacccggagcgcgccgggcggcagaaagtagagcgcgccgagcgcggcgatgacgcccaggcacaggcggatcacgcgttcccaggccggaatgttgcgtttgagatgaaacacgttgtagctctccaaatgatattgacccctgcatggagggccgcgcgtggcgcaaaggattcagggaaagaaagagaaattcagaggcgtgccgaggggagatccggcgccgcttggtgggggccctgttgctgccgcgcgacggccggaagccctcaatctctgtgacttattaccgaagttcacctttagaaacattacatttgaaaatgagaacttaataactcacacaaatgtgattctttagttacactccgggtttcctcccgtcccaactttagccaaaagcattcattttcatgaaaaaacttcttctgatcgccgcagtggccgccaccctggctcccttcgccagccaggccgaatcgaatttcgtgacggcctctggctcgagcacgccgagcgccagcgccaagctcgacttcaagatcgtcgttccgaaggtgcttttcctgcaggttggcacgggcagcagcatggcggacaacacgacggtggataagctcacgttcaccgtgcccgcaagcgatatcggtaacagcgttgcggtggcaggcacgggcggcgacctctctgccggcgccgtcacggttcgcgtgctcggcaacagcggcaacgtcaccctgtccaacattaccgcaggccagctcagcaacggcgtgagcggcgatccgaccgtgccgtggaccgacattaccgtgacggccggcgcattggcgacgaccacgtccggctataccaacgcggccatcgcccacccgccgttcaacaacggcgctaccggcggtgcgtcggcaacggccaccacgctgaccgcttcggccggcctcgtgcgccgcgaaggcagctggaccttcgcctatgccaatacgtccgtgatgccggccggcacctacggcgacacgattgcgaacaagggccaggtgacctacaccgcgaccgctccctgagcgccagcacaacctttagatacgcgcggatttcgacacacgacgaccgaaggcgggccggtcccgccttcgcgatctgttgagaacgagcggcatgaaatcttcgtcactcccgccgtcccgcgcccaacatgccatgctggggctcgccctggtgtgcggcgcctggctgcccagcgcgcatggcttcacggccaccatcttgcccgggcagcgttcgctgttcctgcaggtaggcgcgggcaccatgtccgggggcaatttcaacttcggcggcacgccgggcgacaacccgacggtcaacagcgcatcggtcacggtcccggcggcccagctgggcacgggcgcagcgcagctcatgacgacggacagtaccgtcacggccagtccctgggatgggaacgccttctgcacgtcgcccgccaccaccggtcaggtgtacgtgggcggattcttccgccggcccggggtggggagcggaggcaacgaagccctgctgacggtcactacaccggccgcgctgaccaacaccaacggcgacacgattccgttcagcaggattgcatggacctcttcgggcatcggtgacgccactgccaccattccgagcggcaccttcgtcggcggcacgcaagacctgctgaccgtcagccgcaacacctggttcgagagctgtctcgcctttcgctacctcaattcagaggtcgtcccggccggcaccttcaccggcacggccaccttcacgctgaccgccccatgaaagcccgacgcacgcttgccatgctggccggcctgctggccctggggaccgtgatccccgcggctgccgccacctaccgcatcgacgacaccggcacctatgcaagccaaccggtcacgcagatgcgctggcgccggctggcgcccggccgcgcgggcgaccacacggtggagggccgcgtgtccgtgtcgctgcggctcaacctgtcgcagtggctcaaccggcccgcgcgcatctacctgtcgctggcgccgaccgacggcgaacagctggtcgccacgtggcgcacgcagggccgcctgcttccgggcacggtccgcggcggcggccgcacgctggtgtacgagggcgtggtgcgcgagtctttcctgcaggaaagcatcgtgctcgatctcacggccgatggccgcaaggtcgagcacgcgcagtccctgcaattctttttcgagatcgaggtatccccgtgatgcaccgagtcgcaattcttttccgtggccgctgcgcggccgtttttctgcttggggccctggcgatgggcacgacggcgcaggcgcagttttcccttgccgtgtcgccgccgcgcttcgagctgtcgaccaagcccggcgagcgcgtgcgcgaggtgatcgaactcacgcatcgcgacacgccgaccggcgcctacaagctcaagaccgccgactggaccttcaggcccgacgcctcggtcgacttcagcgacgagctgttgcccggcagttgccggccctgggtggccatcgagcggcgcgagctcaacatcacgtccggacggccctaccgctttcgcttcgaagtgacgccaccagccgacgcgccgccgaccgaatgccgctttgcggtgttgatcgagggccagcaacccaccgcagctccgggcatgcctgtggcgctgggcgcgcgcatcggcgtgatcgtctatgtggccgtgggcaacgtggcgccagtgctggaactcgtgggcagctcggtgcagacgatcgacggccgtcccacgcccatgctcaagatccgcaacacgggcacggcgcacggccgcctggccggcttccttgcgggcaccgatgcgggcggcaccgccctcgaactgcaggccggcaccacgccgatcctggccggcgaaacccgcgacatcgcgctcgtggccaacaagcccggcgacaccgaaaacgcggtctcggtgcgtttcccgatcaccatcgccggcaagctggagtggggcaagagcggctcgctgccgatcaaccaacgcttcgccccatgaaacgctggctccgttatggagccctcggattgtgcggcgcaggacaggtgctgaccggcacatccgcatgggcgcagccccaggggacgcagtacgtcgatcgcgtgctcgacgacagcccgcaggccgcgccggtcgatgagccccaggtccagggcagcggctggccgcgcggctggaccatcgagggccagtccacccagcaaagcgggggctcgcgctcacgcaacgattcgctgctgttctcgggctacctcgacacgcccgactacggcacgctttccgccaatctgaacctgaaccgaaattccgtgccggtcagcggcattgcgctgtatggcaccaccggcacgccggtcacgcaggtgccctacacctaccgcagcggcagcacctggcgcatcgaccagcgcgccatgcctttcaacggcggctggttcggcaacaacagcatcggcaacatcaacatggcgagcacgccgctcgcacgcggtgtaggccgggtctacctgcccagcctgccgatcgagggcgcgtcgctcagcatcgagcagccggggcgaaccatgttgaatgcgtcggctggccggctgggctatttcgacggcatttcgtcccagggcttcacgtccgggcggggcaccgcggcgggcgccggagcccagacccagctgagcggcagcgacggcccctacgcgctgggccgcaccgatgcggcggtccagttggtggaaacgcgcaatttcaacgccaacggcgtggccggctttgcccaggacacccgctcggtgtggagcgccgtctcctggcaaggccaggcaccctgggccgagtcggtcggcaaaggctatggcggcatcggcgaacgcgtggggggcctgcgcgtccaggccaacctggcgcacagcaccgggcagccttccgacgcctcgtcacgcgcagcgcgcgattcagccaccggcggctgggtcgacgcgacctggcgcacggcgctgatgcagcagagcgcatcggtgttctatttccagccctcgctgcgctggggcggcgactcgctgccgagcgacctgcggggtgcctcgtggcgcggcgacgtctcctcccgccaatggcaactgggcggcaacatcgaggtgagcgacagcgtgagcgggctgcagcgccgctcgctgtacggcaacctcttcggccgttttcgcttcgattcgcgcgactcgatctccggcaacgtggccgcccgcaccggcaactatgccgcccagtcggcgcagctcacctgggagcacaagtccgactggggctacagccagtggcgcaccgacgttgcgcacggcaccgacctgcgcgtgctgcgcaccggcatcgaccacgcctggcgcgtcagcgaggaccagacgctctcgacctcgctggcctacgagcaatcgcgccaggccggggtcgattcgcgcaccgtgcactggggggtgctgggcaccacgccgctcgcggccggcgcccggctcgacctgagcctgcgcggcagcaacggcatcggcgacaccgattcgcgctatttaagcgccaacgcgcgcctgagctggccgctgggcctgggctggtcgttcatcgcccagtacgccgcctcacgcgggcaggagtcgctcaaccccgccgtggtgtcggcgctgacgacggccatgcagcaggccgtgcgcgtgctgccctccaaccgctcgttcatggtggcgcttcgctacgagagccgcgccggcgtggccagcgcaccgatcggcggcgcccccggggccggcgcgggcaggctcgagggctatgtcttcttcgaccagaacaacaacggcctgcgcgaggccagcgaaggcggcgttccgggcgtgacggtggtgctcgatcgcaactacgtggcccgcaccgacgcccagggcctctacagcttcccctcggtggccgccggcagccaccagatcgagctggtccaggacaacctgccgctgccctggagcagcgcgggttccccatcgcggcgcgtcaacgtctatgtgcgagacgccgccatgaccgacttcccgatccagaaagaccggtgaatccgacgaaaggcagttgcgctcaccgcgcctgctgtatttacttgcccctgcggtcttcacttttgaagcccgctgccgatatacgaaggtcgggcatcgccaagatgccttcagcccagtgtttttcggggggtcagccttatgtccgggagcaggatatttgcaggggtgtgcatgaaaggcgccctgtccgcattgcttgttctgccgcctgtgtgcacggcggagaccatgcccggggcgatggccagcagcgccacgcgccagctgagcttcaaggtggtcgtgcccccggtgatgcgcgtggtgcaggtcacccccctcaaggacggctacgaataccgcatctggaccaacacccgatcagcctcgttcaacggccgcgagtaccgcttccccaaggtgggcgagtacacgctgaaggtgccttcgtccccgcgcggggtgtacctcattcacggcctctgaaacccccgggccgcggctgcaagcgacagtcggcgccgggttgccgtgcccgcgcacggccggccccagccattccacagcctgcatagccaaatgaagacctcctattggacccgcatgtgcgaaaactgcgggcacggccgactggtgttgcagcacgacatcacgaatcatcggatctacgtgcactgcgaagactgcgagatgggatggctgcgcgcagccgaccaggccgacgtcggcaagggatttctggcgatgctcggcaattttggatccgtggatccgacctttgacgagatcgcccggtccgaatgggcggaccatgtctgcgggtcgttcgacagatgagggagaagtcgcctaggacgtgacgccagtcgtcttcggcatggccccgcggtgaagaggcaaccagagcgtgaagcgggttccggctctgctcgactcccagctcacggcgccgccgatggccgatgcgcgccgctgctggttgcgcaacccccggccacttcgacgcagggcctcgtccacggcaaagcccgccccgttgtcttcgatcaccacgcacacgccctggccatccgtggcggtactgaagcagatgctggtggcctgcgtgtggcgcagcacgttggccacgcattcctgcatgatgcgcagaatgtgcagcgcgctgcccgggtccagccacggcagcgcaggcaccgactgcacttcccagcgcagcgcgagtccggcgctctcgatgcgcggcgccaggcgaaaacgcaaggtcgccagcagcagcagcaaatcggcgtccacgctttccatggagtcgatcgccagcttcaggtcctccatgcagcccttgagcacgcccgagatctcggccttgttcatggcgccctgctccaccgaacggatggcgctgatcagcgacgaacccagcccgtcgtgcatgtcctgcatcaggcgccggcgctcggcaccgagcatgtgctcgttctcgatcacgcgcatccgctggtagctttgctccagctcggcttcgcgcgcttgcaggcgctgggccaggcccttgttcagccgggccacctcggcaaacgcgcccgtgtacagctggaacatgatgtacgagaagatgaagaacaggccgatgatggcgtagggtgaggtgtacacgctctccgggctgaccaggttgttttgcaggagcccgtcgtacgaggtgaaggccaccgccagcacggcccagcccgccaccagccgcccctcgggcaatttggcgcgcagcgccttgcgcatgttcaccgcaaagatcagcaccgccaccggcagcaccatcaggttgagcagcggcgtgagcaggtacaggctggcaaacgacgcgtgaggcagcgtcgcgatgctgctggccgccgccagggccaccgacaaacgggtcagccagaccgagggctgctggtgcaggcgctgcagaaacaggtgaatgaggatgatcaaccagagcaacgaggccacggtgatccactcgaaccactcatccgagatcgggaggttctcgccgctcacgtagtagtgcagcgtgcgcaggaaagccatcgtcgagatcgcaaagaacagcaggtagagcgattcgcgccttttgcccacccacaccgccaaggcgaatgcacccaccgcaaggaacgcggcgctgcccatgaacggcaactgcacctgcagcaactcgcgagcctggtagcgccagatcagcgaatcctggtcgccgacccataccgtcgaaaatccgctcccgctgctgcgcaggcggtcgacccgaatcagcacggacgccggggacagcgtatgggccgctgcattcaacggcagcaacagcggtcggttgtagccgttgtgcacggggctgccatgcgattgataaagcagcacgccgtcgccatacaccgcgatgtggcccagggtcttccagcgcggaaggtagagaaagcgctgccgttccgatgacgccagccgggccagatcgatgcggtaccagtcggtgacggtccgctcgccccccgtcgaggtggggaccagttcgcgaccggccgtgtgcggaagatcgaccgtcttccacccgtcgctcggcaatccggcatcgtccgcacgccgcggaggggcggaatagcccgaaccggaaacggacagcaattcggcctgggtgatgtggagaacgctgcccggctgctgcacctcgtccgcggccggtggctcattcgcgtgcgcgcaagacaaggctgccagcggcaaggccagccacagctttgcgatccaccggcccgcccaccaaccaccgctgcggccgggcttcatgaattgcgtctgccttcgacgcaagcatcgaccgccaccatcgcgacacgaggagtgtggtggccaagggcaacggaggacgctttcatcaggtcacaattatgtgcgcggccgaaccacgcgctcatcgaacggacggaactgcttcagtcccacctctggtacaaagccgcatgagcagcgtcccactcgcggcctccctcgtcgatctcttgctcgggctcgaactcggagcttccgacaaggccgctcgcgatcgctggtcgctcgagggcgtcacctggcaacccgaacaggacggcgtgatcgaagtcggcgcccggcaattcgaggcgagcgcgctccgccttgcttcgggggcgctggtgctggagatcgatcgcattgccgtgcatgaactggtggctcagctgcggaccgatgccggcttaccgcatctgtctgccatccaagcggtcgaggccgagctctcgggcgtgaagctgcatggcccgttgaccgtgccgccgcagatgcgcgccgcgtgggacgccctgcggagtgcgggcgcggccgcaacccacgcgccgccggccgacgcatggagcctcggcccgctcggcgaggcagacggcacgatccgcggggaaatcaccgacgcccacctgctgttcgacgccgaggtcacggtgccaatacgacaggggcagatcgacttcaacgatgcgacggtcgagcatgtgggaccggattcgcgcatgggcgtgagtcgcctgggcctgtatgtcgatgcgccgaatgggcgcagctatctttatcagttcgcatcggcaccgctcgcgggtgtggaattcgaacgccgcggcgcattgctgagtccgtgggtttcggaacgcggcaagctgtacctgaaggctttcggcgagacgatgctgcgccagagcggtggtggccagggccagggactgacggagcaggcgcgcctgctgctgggccgcaccgcgctttccggcgaggtgcaactcggtgatggactctttgccgtgccgggcctgcaagtgcgattggaggggcgaggcgaaggccgcaatgcggttgaattgcactccgacgccctcggccagggcctggccatcgagatggcttcattgtcggccgccaatgcagtggcccattggcggggcgcgcagctgagctgcgacagcatcacggcgcggctcaagctccagcttgttgtcgatgggccgcacatgcgtttcatcctcgacatcgggaactgcaaggttgcaggggcgcgggtcgatcttcgtccgcatccgggcgtgccgccggacgcgtagccggggcaggccactcggccgcctcgcaagcatgtcggccgtgagcgccttcgaagacaatcggataagcccagttcgaaaatcacagccacgaccatgccccgtctcgacgaccccctccacgacgccgaaatcggctcccgcgacagcacgctcgacaccacccggatcgacgacgtgcgtatcggcgccgttcggccgctcatcacccctgccttgctgcaggaacgcgtgcccgtgcgcgacaacacgctggcgctggtcgaaggcagccgcgcggccattgccgacgtgctccacggtcgcgacgaccggctggtcgtcgtggtcggcccgtgctccatccatgaccacgaccaggccatcgaatacgcacagcgcttgaagaccgtcgccgactccctgcaggacgacctgctgatcgtcatgcgtgcctatttcgagaagccgcgcaccaccgtgggctggaagggctacatcaacgacccgcacctggacggcagcttcgcgatcaacgaaggcctggagctcgcgcgccgcctgctgctcgagctgaccaccctgggcctgccgacgggcaccgagtttctcgacctgttgagcccgcagttcattgccgacctgatcgcctggggcgccatcggagcgcgcaccaccgagagccagagccatcggcagctggcgtcgggcctgagctgcccggtcggcttcaagaacggcacggacggcagcgtcaaggtcgcggccgacgccatcctcgcggcccgcgcgccgcatgccttcatgggcatgaccaagatgggcatggcggcaatcttcgagacccgcggcaacgacgactgccacgtgatcctgcgcggcggcaaggcgcccaactactcggccgccgatgtcgcggccagctgcgaggcgctgctggcgaacggcctgcggcctcaggtcatgatcgacgtctcgcacggcaacagcagcaagcagcatcagcggcagatcgtggtcgccgaagacgtggcggcccagatcgcggccggcgagcggcgcatcacgggcatcatgatcgagagccatctcgaggaaggacgccaggacctgaagcctggcgtcgcgctgaagcacggcgtctcgatcaccgatgcctgcatcggcttcgcccagacggtgccggtgctcgaggggctggcttcggcggtcaaggcgcggcggcgcttgtcttaagccggccagcagccctccctcaatgcggccgtcatgcggccgtcacgcggccgtcttccgctactcctgcggttccagtgccatgggagccggtcccatggcgcttttctttcgggcctggagaacgaaagcgaccacctgccacacgacgaagaccccgatcaggctgagcaaggtgccgctgatgggacgcgtcacgaaggcgccaaagcttccccggctcagcagcatcgcgcggcggaagttctcctccagcatcgggcccaggatgaagccgagcatgagcggcgcggcgtccagttccaggcgcatgaacatgtagcccatgaagccgaaggcggaggtgatgaagacgtcttccagattgttgttcacgctgtaggtgccgatgcagcagaagaacaggatcgacgggaacagcacgctgtacggaatcttgaataccgagagccagtagcgcaccagcggcacgttcagcaccaagaggaacacgttgccgatccacatgctggccaccaggccccagaacagctcggggtgggcgccgatcatgttcggccccggctggatgcccttgatgatgaaggccgccagcatcagcgccatgacggcgttctcgggaatgccgatgctcatcagcgggatgaagctggtgcgcgctgccgcttcgtcggcagcggcctggccggccacgccctcgatgcagccggagccgatctcgtgcttgtacttgctgaccttcttgtcgagcgcgtaggcagcgaactgcgcgatggtggggccgccgcccggcaggatgcccagcagcgagccgaccacgctgccgcgcagcgcgctggggatgatccgcttgaattccgcccaggtgggaatgaggttgatcttgccgttgaagggcgaacgctcctcgcgggagtcgaggttcttggtgatctcggcaatgccgaagcatcccagcgcgatgctcacgatgccgacgccgtcggtcaggaagggcatgtccagcgtgaagcgcgccatgccgctgttcacgtcggtgccgatcgttcccagcagcacgccgatcatgcacatcgccaggccgttcagcaggctgcccgttgtcacgaagctcacgcacacgaagcccaccagcatcatcgcgacatagtcggccgggccgaacaggaaggcgacctcacccagcatgggcgcgaagaacgacagcaccaggatggccaccgtgccgccgatgaagctggagaacccggccgtgaagagcgccaggccggtctggcccttcagcgtcatcgcgtacccgtcgatgcaggccacgatgctgctcgcatgcgggatcttcatggtgatggcgctcacgctgtcgccgtattgcgcaccgtagtagatgccggccagcatgatgagcgcaccggtggtgggaatcgaataggtcagcggcagcagcaggctgatggtggccagcggccccaggccgggcaacaggccgaccagtgttcccaccgtgcagccgatggcgcagaacatcaggttctgccacgtgagggcgtgcgaaaaaccgaacgccagattgttcaggacttccatgatcgtggcctcagtggcctcagaagagcggcaggttcaggccgaggagtttctgaagcgcgaatgccatggcgatcaggccggcagaaatcttgacgttgcgcaaccatgagttcgagctgccggcgaaggccgagcagaacaccatgaagacgatgcccgcgaccatgtccaggtacatcgagatcaacgcgaagccgcaaaggcttccgaggatgagtgcgatgttcttgaagtggaggtccagccgcaccggcgcgacgaggaacgatcggaccaccgtcgaggcgccgatcagcagcagcaggctgctcaccatgacggggaacagacccggcccggcccggctcaggtctccaatggggtagcgaagcgccgtgaggccgaaggccaatgcgattgccatgaggaagagtcccctgacaagatttctgtttctcatacgttcccgatgcggtgggtttattgaacgcaaccggcgcaggtgaagccggccgggcttgtctccatccggctggcactccggacgatcgaatgctctttcgccgagctgatcgcaatctgaccccgaggcgaggggaactacgtacccttcgctccgaagggctccccggtcatccgtcgcttcgaggaaaatgcggcccagaagccggagctttcgaatgacccccaccatcaccgccttcgaacgatcgcccgatcgcggcagaggattggcgcgcgacatgcgcgtgcgctgggcgcttgaagaagtgggccagccctacgacgttcgccttgtttcgttcaaggagatgaaggagcccgcgcatcgggcgcttcatcctttcgggcagattccgacctatgaggaaggcgatctcgccctgttcgagtcaggggccatcgtgttccatatcgccgagcgccgtgccggcctgctgccggacgatgcgaccgcacgggcgcgtgcgatcgcatggatgtttgcggcgctcaacacggtggagccgccgatcctcgatcgcgagatcgccacgctcgtggagcgtgacaagacctggtacggggagcgcctacctgtgctcgaggatcgcgtccgcatacggctgggtcaactctccagccggcttggcgatgccgattggctcgatggtgccttcagcgctggcgacctactgatggtgacggtgctgcgcaggttgagcggatcggggttgctggatggatatccgaacctctgcgcgtatatcgcccgcggcgaggcgcgaccggcctacaaacgcgctttcgccgatcagctggcggttttcactggcaaggcccagagccgctgatggggtctgctccaggagcaagaagcgcatccatcgatcctgggtggcacttcagaaaagaatcacccattcgccgcgaatgtaccggtactggtagctgggtccggaaaaggtggtgcttcgactgtagccggcaccaaatcgaaacacctgcgaccctctgacgggactttggagactgaagtccagcaatttcgttggctggctcagctcgtgattgatggtctcattgccgagccccgccgtcacagccgcggtccatccctggaaacggtgtcgccaactgaccgccagcatcgactcggcgtagctcttcggattgaaataggccctgtcgacatcctcgtgggtacttcggtacgttcgatagcgcgcctgcagcgtcagccccagatcgagcgacggctgatagatcagccgcaggcggccgtggtcccgccgattgccgtcggagaaatactgctgtgccagcaggcccaccagggtcacgtggctcccgagcccctgatccacggcgaccccgacgaaggaaaaatcgattccgcggtccagtgacttgggggtttcgacccagtcgcgcgtcagaagaaactccaccgccgtactctttgtcggggacatgcggtagctgccgtcgagtgtcagcagcgtatgccctccctgttgaaacacacccgcctccatcgcccctccgtcgcccgttctggtttcgatcgagcgggcgagaaacgagatcttctggccatttcttcgccagttgtcctgcttgtattggtaatcgcccagccggaaccccaggaagcgatccgcgttttcaaaggcgggaaaaaactccacggacacgcgccgcgattgaaaatgatcgctgtcattggtcagaaagaattccgtcccaaacgccatgccggctgctttttcgttggttttttcttcctctgccttgcaaggagaaatcaacgccgcgaagcccaaaagaccggccagaccgcattggagtcccccgctcatttcgtaccccacgacttcggctttctgaacagttcatccagatatcccagaatgctggccggctgcagaatgaggctgtacagcagcacgtagacaaagaatccctgcacattttttcgcacgaccaagcctgttttcttgaacattcggcgttcgatcgaaaacatcagaagactcaatgcgaaagcggccggcagcagcgcaagggtcatcaaccccacaatccagtaatagccgaagaaggcaaggatcaatccaggtatgaatccgaaggtgaacgccagatccaaccatggaaacaaaaggttccagtaaacgaaaaatgtcgacaaccgggatttgaggaggatccccggatgcttgatgaaggcttccgtcatgccacgcgcccatcgctggcgctgcttgaccagttgtttgacggtgctgggcacgttggtaaacaggcatgcatcctcgcaatggccgacccgatagcccgccttcagcagggcccacgtgagcacgatgtcttctcccacgcactccggccatccgcccacctcggccagcgcggcacggtcgtagacggaaaatgcaccctgcgcaaccaaagtgccctggaacagcgattgaacccgcttgatggcagaaataccgtggaaatagtcccattcctggcaacgggtgatccagttttgccgcgaatttcggaccaggatctttcccgcaacagcgcgcgtattcggcggatccgcttgataacgctcgacgatattgaccagcgcccctcggtacagaaacgaatctgcatccaccgtgatgacaaggtcgtgcagaacctccttgagcccgatgttcagcgcgcgagccttgcctccgttctttttcaggtcgacgaaggtcagccacgggtaccggtcctgattgcgctgaacaacaagagaagtgccatccgtggatccatcgttgatcacgatgacctgcaattcgccggggtatttctggtggccgatgctgacaagcgtctcctcgatcgaagcctcttcgttgtatgcggcaaccagaatggagatcgggggatagacggacaaagcgcggtgcggcggccttttgtccaggaccaggcttatcgccaggaacgcattcatgaagcccggaatgatggcgatcccatacaccaggaaaatcgccaaagcggggccgacatggaattgaagatcggcgaaccaaggccccgcggcccatattgaaaaccccatccaggcgctggcaccaatcaatgcgatgagaaattttcccgacaccggcaggtaaagtattcgctgcagcgctgtttggccatcttcgttcatgtcgccctcgatagttccaaaaatgtaacgcgcatggagcccggggaacagtctgtttacactgttcgaggcgcgttaacaactatgaatcgagggcgttgcttcgcccggcgccgccggcgggtcggtaggtgaccgtcagagggccccgacgatttcaactcagcgaagagctccgcatcctgtttcgagctatctgcagcgtcctgcccattcgtcggggttcgttgagcatcttgttgatttccgccatgccgtcctccgtgatgcacgtcacggtggctgttcgggcgacgttgtacttgccggccgagtccgaggcaggcgcgatctctgcttcaatgagaccggtcgctttcaatacgctcacatgctgaacgtcttcgggtctcgccaccaccttcggcagggcgacgtactgcaggcttagcaaatagaacaggggcatggccgttacctcattcgatgcgttttgttgtcgagatggggcgcttgctcgcgtcgctccttcgttggagaactcgaagatatgccactgccccggccagcctgtcggacgccaaccagcagctctgtagcccaagaaacctcctcagggctgccgatcgctccgtcgaacaagcctggatcaatgactgtggccgggtctgccacaggctgtgctcgcggggtctggatatcgatttccgcagtctccagacataagcaaattcttaactcggccaaatgacccagagcggcgtagttggtcgagatcgccttgaggacgaccagcaccatcgggtcgtccttgccgatcggcatcccgttgatctcgtcgcagatccgttttgcctgctggtattgaagctcggtgactttcgcggcgtacgcaatccggcgtttcgccacttcggaaagttcgacctgggagtcgtcgctcattttctgctccgggttgcgagtccccctacggcacatggccgagacaggaggcgaatcggacgagccaggcagatgacccgacatggacgaatatccatggagagaaggtcgcggccattggagccggtcatatgcttccttggtgaacgccggaaggcggcctgtgtggtctcgacgatgtattggattgcgccgacgacataagcacatggaaggaatgtcctctccttctcgttcgataagtactggaatagcactgaagagctgggacttttgtcctgttgaagcatccgcccgcgggcgtgttggcttttgcggagctgggccagcggcaatgacgtgtgcacgtcccaaccgtcgcgctggcgacgaccgctggacgacgccgcgccaaagcgcggcccgaaggccagcgggtcagcgcgtcttgggagcgctcgcagacggcgctggcgttgcgcccctttcagaacgcgagcgagtcgggccgtgcgggcgggccgcgccgcggcgtcgcagcgtgcgccgatgccacgccatcaggctggttgccacgctgatggcaaacagcccggcaacctgctggatgagcttggcggtggccacccgcgtgcgctcctccagcacccgccgggtgtcctcgacgttcgcaagagcttcgagttttcccgtttcgtgctggcgcacggcggcgctttcggtgccctgctcggcttgctgcgccgcgatttccgtcgcggcctgtgccttgctcgcggcaaccgatccatgggcgttggcatagaccttggtgaattccgcgccgagcaaaaagacctgcgccgcgtagtacacccatgccaacagcaccaccagcgatccggccgcggcgaacgattcggtcacgctgctcttgccgagatagaggccgatcagaaccttgccgacctcgaagagcacggcggtcaccgccgcgccgatccacacgtcgggccatgcgatcggcgcgctcggcatgagcttgtagatcatcgcgaacagcagcgtgagaatgcccagcgtcaccactgcattgagcgactgcagcagcagctcccaccccggaaaaaacccgacgctccagtttcccagcgccgcgagcacggcactgacgacgagcgacaccatcagcaggaacgcgagccccaggatcagcccgaacgacagcacccgcgcccgcaaaatgccccacaggccgctcggcttggcgcgctcgggcacatgccagatgcggtcgagcgcgctttgcagttcggcaaacacggtggtcgcaccgacgatcagcaccacgatgctgatggctccggcaatcagcccgcgcgacggctcgttcgcgctcttgaccagcgcttgcaccgcctgcgcaccctcctcgccgatcaagcccgtcagctgcgcggcgatctggccctgcaccgcttcagccccgaagagcgcgcccgccaccgcgatcacgatcaccagcagcggcgccagcgagaacatcgtgtagtaggaaatcgccgctcccatgctcggcgcgaaatcgtccacccaggccatggcggcctccttgcacaggcgcaacagatgcttgagcttgttcatggcccatcgaagctcgcgctttcacgcaagattcgctgtaggtagacaccgcttcagcgtgcaaggtccgcgccgtctgcatgcggctgcatccatcggccggcatgatcgcgcagcgattcgatctgcacccggaccatggcgagctcggcccgaaaaagccgggcgatgtgatcggccgcctcgtcgccatcggcctcctccaccgctgtcgcgggatcgatcggcttcggggccgcttcgccgccgccatccggcgacgcaccttccataccttccatgtacgaggccaacgcatccagcgcgcttgccgcgccttcggcctcggcatgcagcgcggccagctgttgcggcgcgtgcagcgccgcgcgatgcgcgccaagcgcggacaagtagctcaggagcgcgtgcgactggatcaggaaccgcaacgcgacgcccgcgcgcggccgcacgaggcccggttcgcgatacatctcgaacacggcgccggacagcgtggcgtcggcgttgtgggcattgcgcctcgcgagccgataggccaggtcgtcgcgcgcccccgagcgatattggctggcgatctgccgcaggtagtgcccgtggttgcgcagcgccgtcgcagccagatcgctgaagcgccgcgactgccaatggggcagcacgaggatcatcgccagcgcggcaatcacgctgccgatggcggtgtcgatcagccgaggcacgatcagcacgtcgccatcgcccacctggttggagcacatcagcaccagtaccgtgaccgcggccgtggcgagcaggtagcgcgtggcacgcgtggcgaagaagaagacacccgcggccacggccaccagcgattgcagccagggctggggaaagagcgccagcaaggcccacccggccaccacgccgaccgccgtgcccgcgatgcgctggcccatgcgcgacacggtatcgccccaggcctgctggcagacgaacagcgtggtcagcaggatccagtagccccgcaccgggtggatcagcagcatcacgccatatcccgccatgagtgcgacggccagccgcagcgcatggcgaaacagcgccgactgcggcgtgaactggcgccgcacgcgctccacccgctcgcgccaggaacgcggcgagcggtcgaacagccccatgtcggcgcgcccggcccgggccgatggctcggtggcgccggcgagctgcccgtcgagctgcgccagattccacgccagcgcctcgacggacgcgagcagcgcaagccggcgcggttcgcgcacctgcgtgcgctcgtggtcgatggcgctttgcagctctgccagcgcgcggcccgtctcggggccggcgacgaagggttcgcgccgctcgatcgaatgcgcaaggcggcggcaggcttctccctgcaagctcagcacgcgctggcagcggtacagcaggtcgctgtgaaagaacgcatcggccagcgcgttgtagtcgtcatgcgacgaggtcgcgcgctcgtgcacgtcctgtgcgatcaggtacaggccgcggtagcgagcgatgcggcccttgggtgcgcgcgcgccaatgcgccggaagatgccctccttggccgcgttgagttcgcccaccacgtcggcattgagctgtgcaagcgaaagccgcttgcgctccacgtcgatgccgcgcagcggctcgaacagcgatgccttgaagcacacgtagtcgccgagcacggagaacagcttcaccagccgcacctgcaccggctgggccggaaagaacgcgcaccacgccaccgagaacacgccataccaggcggcgcccgccagcaggagcaggacctcccgcagccttgcggcttcgcttgcggcggcgttgccgtcggtgcccagcgtggcatagatcgcaagaatgagcgtggcaaagccgatggccttgtagcgcggctcgatggcgccaagcatcgtgagcgagaacgcggccagcgcgagccccgcgatgaagaagaccggctggtcgatccaggacagcaccgcgaaggccgccaccgcgaagcaggccagcgtgacgagctgcgcgcgcaagcgcccgcgggcgctgtcgtcggtctctgccagcgcgctcgcaatggtgcccagaaaaagcggcgtgacggcttcggcgtgcccgctcaggctgccgatcgccatcaggctgcccagcgtgagcaacacccgcagcggctgggcctgcccggccagttggcgcaggcgatagcgaaaagtatccagggaaaatgaaaacatgcccgtctttgtgcacgatgcatgccaacacgcaccctgcccttgcgctcgccggcgccgctcagcctaggcgggcacgggccgcatcgatgcgcatacgcggttgcggccgcccgccttcgccgcatacagggcctggtccgcggcacggatcaactccttcggctgcgccgctccgggcacgggcttgagcgcatccacgccggcactcaacgtcacgaagccgtcttcggtgccggcatgaacgatcttcaggtcgcgaacggcgctgcgaatgcgttccgccaggatgacggcgcccgccacgtcggtgttcggcagcagcaccaccagctcctctccgccgtagcgcgccgccaggtcccccggacggcggcctgcaaccttggcgatggtgcggccgatcgattgcaggcactcgtcgccggccgcgtggccgtagatgtcgttgtactgcttgaagcagtccacatccatcatgatcagcgcgagcgtgctcgcattgcgcatcgcgcggccgaactcgttgtcgagcgtcacgtcgaactgccggcggttcgcaagcccggtcagcccgtcttccatggccagcgtgttgagcgtcttgttcagcgtctcgagcgcgtcgcgcgcctgccgcagttcgttctcggtctgggtctggagctcgaactgcttgacgagccgccatccgacgaaaccgaccaccagcgcgagcagcagcacaccggccgaatgccagatcgtctcgcgccaccagttggccaggatttcgtccttggacaaggccgcggacacgaacagcggatagttctcgaggcgccggaaactgttcaaccgcatcgtgccgtcctgcgccgagcggatgtacgcggtgccgactgcgccctgctcgacgtaggcgcgaaagaggtctgtctcccgcatgtcgcgcccgaccatgtcggcgctgtagggccggcgggtcatcatcgttccgttgtccagcaccaaccctacggcgcccgcctcgccgatgtccaggctgtcgtagaacttcatgaagaagtcgacgtcgatcgtcgcaagcgccacccccgcaaagctgccgtctgcatggttgatgcgacgcgacaccggcaccagcaattcgccgctggtgcggctcttcaccggaatgccgacgtgcggtccgcgctcctcgtgcgtgcgatggaagatgaagtattcccggctcgcattgttcaggttctgcggcgtgatgcggcgcgagttcgcgacccagttgccgtcctcgtcgtagatatggaggccgtcgagctgcggaaattcatcgacctgcgcggcaagcaccttgcgaagccgctggacggccgccggaccggtgccgtcatgttcgacgcgctcgacgatgccgaccaacgcggagtcggccgccttgagcgtgtcgtccgcctgttgcgccatggcgcgcgcaaggttcgacgtcgctgcgttcatctgccgcagttgcaccgtgcgcgactgccagctgttccagcagtcgattgccagcaggctgaggcagacgatggccacgaaggccatcgtccgaaaggtgatggagggtcggcgaagcacgatgcgtttccaagggatgccgtaacggccgctcgcactttgacacatctgcgacccgatcacctcgaatacggcaaatcgagccggaccctgagcggcaaggcttcagggtttgccctattttttagttatcacataaaactatattggttatccaagataacttcatcacagccggcccgacccggcaaaggagacaccgatgagccggatcatgttcccttcatgccacccgacatgggccgcattggccacagcctcgctgcttgccgcctgcggcggcggtggtggcggtggcgcaagcggcttcgggttccttcccgccgcgccctcccccggcggctccggggtgtcggaggcacgccccggcacgctccagtcgtgcagcgatctcgcaagccaggcggcgttcggcaacaccgcctacaccagcgtcacttcggtcgccgcgggcacgctcgtcgtcgccggcgtgagcacgcccgtgcctgagcattgcctggtgcaggggcagatgaaccagcgcaccagcagcgtggacggcaagacctacgccatcggcttcgagatgcgcctgccggtcagctggaacggacggttcttctaccaggccaacggcgggctcgacggcaacgtggtgcgcgcgacgggcggcatcggcggcggcgcgcccacgagcacggcgctgcaccggggcttcgcggtgatcagctccgacgccgggcactcgggcgcgcagattccgaccttcggcatcgacccgcaggcgcgcctggactacggctacaacgccgtcgcgcaactgacgccgatggccaagaacctgatcgccaaggcctatgggcgcgcacccgaccgctcctacttcggcggctgctcgaacggcggccgccacgcgatggtggccgcggcacggtccgcaaaccagtacgacggcatcctggccggcaaccccgggttcaacctgccgaaggccgcggtggcccagctctatggcgtgcagcaatatgccaaggtgaccaccgccaccacggcggccggcaagccggacctgcagaccgccttcacgccggccgagatgaccacggtggccaacgcggtgctcgcgcgctgcgacgccctcgacggcgcaacggacggcatcgtggccgacgtgcagagctgcaagcaggccttcgacctggccagcgccgtgcccacctgcggcgccacgcgcaacggcagctgcctcacggccacgcagaaaaccgtgctcgacaacatcttctcgggcgcgcgcaacagcgcgggcacggcgctctacagcagctttccgtatgacgccggcatcaagggcgccgactggcgccagtgggaatttgccaattcgcagaacctggacacggccgccgtgggcttcgtcttcagcacgccgccgctgggcacgagccgcccaccgggcatcgactttgcgctgggcttcaacatggacaccgatgcgccgagcatctttgcgagcacggcgctctatacggagtcggcgatgtcattcatgacgccgccgaaccccgccaatctgtcggcgcttcgcgagcgcggcagcaagctcatcgtctaccacggcaccagcgatgcggtcttctcttcggacgacacgacgacctggtacgagcagctgcgcgcggccaacggcggcgacgcgtccggctttgcccgcttcttcccggtgcccggcatgaaccattgcggcggcggcccggccaccgaccagttcgacatgctggcgccgctggtggcgtgggtggaacagggcaaggcgcccgcgtccgtcaccgccacggcgcgcgggcccggcgccaacgtggtcaatgccgaagtgcctgccgactggtcgcctgcccgcacacggccgctctgcccatacccgcagacggcggtctacatgggcggcagcatcgaatcggccgccagcttcgcctgccgatagccacggtcctcccccgcccggcccgaagcctcaggccggctccatgccgtggcggcgcttggtgtcggcgctgtccgccgagcgcatgaaatcgagcagcgcgcgcaccgcctccggctgtgcgccgccgccgatgccgggagcggccgtaaagacggtggtgatctgaaccgccggcggcagcgggccgatcaactcgatgccttcgacgccgatcagctcgctcagctgctggaacccgagctcggcatcgccgcgcgccagcagcgagccgaccggcacgccggtcggcgcctgcaccaggcggccgcggatgtcgccggcaatgccccagcgctcgaacaacgccatcagcgccgtgccgctcggacccgtcgagtaggcgatgcggggtgccgccagcacgctgctgcgcaacgcctcttcggtggaaatgtcgggacgcggcgcaccggcgcacaccgccgccgccacgcccgagcgcaccaggtcggtcttgccggcggcatcgagtttgcccgccgccgccagcttgtcgatggcgtccgaggccagcaccaccacgtcgaacggctctcccgcggacacgcgccgtgcagcctcgacacctccgatggccagaaaggagaccggcacgcccgtgtgctgcgcataagcggccgcgagttcatcgagcaatccgcgcgtcgccatcgaacagaggccctggatcggtgtcgtcatacgttgcctcgctcgcgtggtcaatcaggcttgatgttggcttcgcggatcagcttgccgtagcgcgccgcatcggtcttgagcagcttgtcgaattgcgccgccggtccgggcagggtgacgccgccggccgcggcaagctggtcgcgcacctccggcgaggccagcgccttctgcaccgcatcgtgcagcttggcctgcaacggctgcggaagccccgcgggcgcgacgaagccataccagacgctcgattcgaaaccgggatagcccgactcggccaccgtcggcacgcccggcagcaccgcggcgcgctcgccgcccatcaccgcgagcaccttcagcttgcccgacttcgcgagcggcagcacctccagcgcgttgaccgccaccacgtcgacatgtccgccgagcagatcggtgagggcctgcgcgccgcccttgtacggcacgtggcgcagtgacaggccggccgtgtgctggaacagttccatcgccagatgcggggtggagccattgcccggcgtggcgacagtgacgccgcccggcctggccttggccgcggctaccagttcgggcagcgtcttgatggccgagccctcgcgcaccgagaacaccaccggcacgcggccgaccgaggcgactggcgtcaggtcgcgctcgagatcgtagggcgcgggctcgaagagcgaagggttcaccgccagcgcgttggccgcgagcagcagcgtgtagccgtcgggcgggctcccgatgagcgccttcaccgcgatgttggttcccgcgcccggcttgttctccaccaccacgggctgcccgaggatggccgacatgcgctggccgaccgagcgtgcaatggcgtcgaccgcaccaccggcgctgtagccgaccaggatcttgatggggcgggacggataggcatcggcggcaccggcattgactgaggcgccgagcgccagcacaccgaccagggccagcaagcggcggcgaatgaaagaagtggtcatcatcagtttttcaggttgcggggatttctggtccccaggtctgcggcgcgggcatccttgccgggccagcggtgcgccgcgctcagtcgatgtagcgcaggccggccttggccagcggctcgcgcatggcgtacatgtccaggccaagctcgccggccgcgaagcgctcgcgcttggccgtctcgttggcttcgcgcgcttcggccgcatcggccacctgctgcgcgcgcgcggcgggcaccaccaccacgccgtcgatgtcggccaccaccacgtcgcccggatacaccagggcgcccgcgcacaccaccggcacgttgaccgagccgagcgtcgccttgatcgtgcccttggcatggatcgcgcggctgaacacggggaagcccatcgcattgaggtcgcgcacgtcgcgcacaccgccgtcgatcacgaggcccttgcagccgcgcgccttgaaggaggtggcgagcaggtcgccgaagaagccgtcggtgctgtcgctggtgcaggccgcaacgaccacgtcgccgggctgtatctgctcggccaccacatgcagcatccagttgtcgccgggctgcagcagcacggtgacgaccgggccgcagaagcgcgcatcgggatggatggggcggatgcgcggctgcatcagcccgagccggccgagcgcctcgtgcacggtggaaacgccgaagcgcgaaagcttttcgacggcggccgcatccgcgcgcaccacgttgcggtgaaccacgccgagctgttggagggtgttggaagcagacatgagatcagagccccttggcgatgagtgcgcggtccaggcgcgggtacacgcggcgtgcattgccttcgaacaccttgtgccgcgccttcgcgtcgagcatgggtgtcgaatcgatatagcgacgcgtgtcgtcgtagaaaaaacctgtctccggatcgatgccgcgcaccgcgccgatcatttcgctcgcgaagagaatgttgtcgaccgggatcacgcgggtcagcaggtcgatgcccggctggtggtacacgcaggtgtcgaagaagatgttgttcagcaggtggtccttgagcagcggcttcttcatctcctgtgccagcccgcgaaagcgcccccagtggtagggcaccgcgccgccgccgtgcggaatcacgaagcgcaaggtcgggaagtcggtgaacaggtccgacgtgaggcactgcatgaaggccgtggtgtcggcgttcaggtagtgcgcgccggtggtgtggaagcaggcgttgcaactggtgctcacgtgcaccatggccggaatgtcgtgctcgaccatcttctcgtacagcggataccagtggcggtccgacagcggcggtgaagtccagtgcccgcccgagggatcggggttgaggttgatcgccacgaagccgtattcgcgcacgcagcgctccagctccggaatgcagctgcgcgggtccacgcccggcgactgcggcagcatggccgcgccgatgaagtggtccgggaacagttcgctcacccgaaagcacagctcgttgcagagggcggcccaggtcgacgaggtttcgaaatcgccgatgtgatgcgccatgaagctcgcgcgcgggctgaagatcgtcaggtcgctgccgcgctccttcatgaggcgcagctggttgccctcgatcgactcgcgcagctcgtcgtcgctgatccggaggtcggcggcgcgcggcttcagcgcggcgtccgcgaggcccgcgatctgctggttgcgccagttctccagcgccttgggcgccgtggtgtagtggccgtggcagtcgatgatcattggcagttccgtgaatggcttggtggtgccgtcgccggcacatgagggagtgcgccagcccttgcggcaagtgtggttcgcgggactgccgcgtggggtgagttcgggttggcctaccatcagacttttttatcgatcagggttttccccaaatccttcagaaccctccgccgagagaacatcttcaaaaaagcaaagcccgtgcacccacgagacaaagttatcgaccggacgcacgctggcgcgctcggcatcaacctgcggcatctgcgcgcgttctcggccgtggccgcggccggcagcatcgccagggccgcggacgagcagctgtttcgcgtcgcctcgggcgtgacgcgctccatcgccgagctcgaaggcgcgctgggccggccgctgttcgaccgcggctcgcgcggcatggcgctgaactcgtacggcgacctggtgctggtgcgcgcgcggcgcatcgagcgcgagttcgaggatgcgcgcgcgcagctcatggcacgcggcggcatcggcgcctccgccgacgtgcattcgctcttcgcgtcgatcctcaacggcaggcgcctcgcggtgatcgcaagcctggtggagaagcgcaacatgccggcggtcgcgcgcgaattcggcatcacccagcccgccatcagccgcgcgctcaaggacctcgaaggcggactcggcgtcgcgctgctcgagcgcaggacacgcggcctcgtgcccacgccggcgggcgagatcgtggccttctacttcaagcgggtgctcgcggagctgcgccacatcggcccggacatcgcggccagcgagggcatgctgcagggcagcgtgaacgtgggcgcgctgccgctcgggcgcacgcagatcctgccgctggccattgcctcgctgctggcgcgccatccggggctgcacatcgccacggtcgaaagcccctacgacgcattggcggcatcgctgcgaagcggcgacatcgacttcattctcggcgcgctgcgcagcggcgccgaggccggcgacctgcagcaggaagcgctgttcgaagaccgcatctcggtgatcgcgcgcgccggccatccgctcgagcgcgccgcgcgcgtcgacttcgatgccctgcgccaggccacatgggcgctctcgcggcatggcacgccctcgcgcgaattgctcgagcgctttttctccgccgcgcggcaggcgcctcccattcccgcggtggagaccggcgaccttgccgtgctgcgcggcctgctgctcgaaagcgacatgctcaccgcgatctcggcccaccagctgcgctacgagatccgcgacggcagcctcgtcgtgctcgactttccgctcgacgaaacgcgacgcgagatcgggctcacccagcgcctcggcgcgttcccctcgccgggcgcgcgcgcgctgatggaggagatccgcgcggtggtccgccgctcgcccgatttccacatgccaagctgaatcagtacactgaacacccgcgcgaaggctctgcagaggtgcccatcatgcaaatcgcgattcccgaaatgaccacggacgtgctgcaagcatttgccgacgcgtggaatcgccacgatgtcgatgccctcatgtcgttcatgaccgacgattgcgtcttcgaatcgtctgctggcgccgatgcctgcggcacccgatacgtcggcgtcgaggccgtgcgagccggtttcgcggaggtctgggccgtctttcccgatgcccactggggcaacgcgcgccacttcgtccacggagaccgcggtgtatcggagtggacgtttaccggaacgcgcacggacggcacgcgcgttgaagtccaaggctgcgatctgttcacttttcgggccggcaagatcctgctgaaaaactcctaccgcaagaaccgcctgtcccctgccgcgccaacgcgctgagatgagatgtagccggcaagctgccaagcgtaccgttcagaacctcgaggagatctcatatggctgagagcgacaaggtgttcgcgggctcgatcccgaagttctacgacacgctgatggtccccctgatcttcgaggcctatgcctccgacatggcggagcttgccgcggcctcctcgcccggctcggtgcttgaaacggcggccggcagcggcgtggtcacgcgggcgcttgcaccaaggctcggcgccaatgcgcgctacgtggtgaccgacctcaaccaacccatgctggactatgccgcgagccgccaggggcccgacggccgcatcgaatggaagcaggcggacgcgctcgacctgccgttcgaagatgcctcgttcgacgtcgtttgctgccagttcggcgcgatgttttttcccgaccgggtcgccggctacaccgaggcgcgtcgcgtactgaggccaggcggtcgctttgtcttcaatgtctgggaccgcatcgaagacaacgcctttgccgacgacgtcaccaacgccgtggccgcggtctttccgcacgacccgccgcgatttctcgcccgcacgccgcacggctatcacgacgtcgcacggatccgcgaggaactgagccgcgcaggatttgtcgacatccagatcgagacgcgcgagaagacgagtcgcgcaccctcggcacgcgacgctgcaaccgcctattgccagggaacgccgctgcgcaacgaaatcgaggcgcgcgacgccagcttgctccagctcgcgacggaccgtgccacggaagcgatcgccagccgccatggcaaggaaggcccggtggccggcaagattcaggcgcacgtgatcgtggcagcgcgatagcggagtcccgggttcctctgctcattgatgaagctccaggccgcaatggctgcagtcggcccacgagctgacctgcgctgcgtccgccgactaccatcgagacatgactttcagcctcaagacggaccatgagcagaggcttgctgcaatggtgtctgcatccgacgaattgatggccgccttgcgagtcgtccgctcgctcggactgcgatcttggtgcatcggcgccggggccatccggtctctggtgtgggacacccttcatgagttcgaccagcgctcggccgtcgaagacatcgatgtcgtctacttcgacgcggaggctggtccagagcaggatgcagagttcgagaaccggcttcattcggccatgccaggctttcattgggaggtaacgaatcaggcaggcgtgcatcgttggtttgcctccgccctcggtcaggcggtgccgcctctctcatccctggaagaaggcgttgcgacgtggccggaatatgcgacctgtgtcggtgtctacctgaacgagggcgagtcgttgggcgtggtcgccccgcacgggcttgatgacctgttcgagctgcgtgttcggcacaacccgctccgggcaagcgtcgcgacctaccggcagcgggttgcggcgaaacggtttggtgaacggtggcctcggctttcgatcgacacagcctcgggccagaatgccgcctgacattcgattgcaccttcgatggcctaccaacctgcaacgtcgttcccggacttcatcgagaccgcccgcctgaagcttcgcccaccacatgttgacgatgcacaggcgatgttcgactcatacacccaggatgcggacgtagctcggtgcatggtctggcggccgcattccttcctggagaccacacgcgaattcattgccgactgtgtcgctcagtgggacgctggcaccacccttccatacgtcgtcactctgaagtcgaacggccaactcatcggcatgctcgacgcacgtctccatggtcatatcgtcaacatcggctacgtgctcgcacgcagccaatggggtcaaggcctgatggtcgaggccgtacaagcgtttactgctcacgcccttggtgcgccagaaatttttcgcgtcgaagcgacctgcgacgttgacaaccgatcctccgctcgagctctggagaaaagcggcttcctgttggagggccggcttgcccgccacacgattcatccgaacatctccgatgaaccacgcgactgttttatctacgcagcgtgccggcggtagtcatccggcttgccgtcattgggaaacatgcgtggatggttatgtcgttctccctcgatggctgtcgtcaccgcggaattcatgacggtcgccgaaagcggtcgtcaatcaggcgtgaaaaggactgtgccgtgagcgagaacgctggtccggtcgtctgcgcccttcattgagccttgcaattcgaggatgcagccgcccttcgggtgggctgcaatcgaagtcacgttccattcgatggaaaccgtctcgctcgccagcacgggacgcagcaaatccaccgagaagttgatccccagcacatttcccttcttggcaaagtgactggccgtcaaccccatcaacaaagacgtggcgtgagttccgcttgcaatcaaaccaccgaaacgcgtgcctcgtgcgaactccacatcatggtgcagagggttctcgtctcctgcagccagtgcaaatgtcctgacttgctcttcgtcgaaggtatggaatcgcgagaaacgatagccgggtccgatgggtgcaacggcagcgatttcgaactcaaccatggctcgcgagcctggtgatggcttcctggctcccggcctgctggcggagccggaacttctggatcttccccgtggccgtcttcggcaagctgctgaatatcacgcggcgcggacacttgaagtgggccagccgttcacggcaaaacaagatgatctcttgctcggagggcgccgcaacgcctgccttgagctcgatgaacacgcacggcacctccccccattttttgtcgggctgggcgaccaccgcagcatgcaagaccgccgggtgtccatggacaacatcctcgacttcaacggaagagatgttctcaccgccggaaatgattacgtcctttgaacgatcggtaatctgcgcatacccgttgccatgaaggacggcgacgtcgccggttcgaaaccagccgttggcgagcgctccgcgcgttgcggcctcgttcttgaagtaccccatcatcaccgtgttcccgcgcagcatcagctcccccgcggttttcccgtcgtgagggaccggatccagcgtgtccgcatcgccgaccatgaggccttcgaacatggcggctcgcacgccctggcgcacacgcagcatgccttgctcggccggcggaaggtcgtcccagccgtcttgccacacacaacctaccggcgtaccggaaacctctgtgatgccatacacgtgctccacatcgaaccccatggccaagacggcgttcagcaccgcaagcggaggcggagatcccgcggtcagtacgcgtacggcacgaggcagcttgctgttttgcgccgaatccgcgagcatggccatcacgaccggcgctgcacagagatgatcgatctggtgcttgtcgatggcctccagcaccgcgtcggcggaaacccggcgcaggcagacatgggtgcccgcggccgcggtcacggcccaggtgaaacaccatccattcgcgtggaacatgggcagcgtccacaggtactttggcgcccggggcatcgcccagttcgtgatctgcagcaggctcatgaggtaggtgccgcggtggctggcgactacaccctttggatctcctgtcgtaccggacgtgtagttcagggcgatgggttgccactcgtcgttcggccatcggccgggaaagtccgggtctccgctagccagcaaacattcgtagtcggtctcgccaatgcattcaccgggcggcgcgaggtggtcgttgatgtcgatgacaggaggaggcttgtccagaagcttcaaggcggcggcaaccgttccggcgaactcgcggtcgaccatcagcaacttgcattcgccgtggcgcaggatgaacgcgatcccttcaggatccaggcggtggttgatcgcgttgagcacggcgcctgccaagggtacgccgaagtgcgcttccagcatggcgggcgtgttgggcgacagcactgaaatggtgtctcctggctggatgcccctgctcaccagcgccgacgcaaggcgatggcagcgctctcgggtctgctcccacgttcgcgacaaatcgccgtgcaccacagccaggcgtttcggatgtgccagggcggcgcgatcgagaaagccgagtggagtcagcggcacatgattggcctcgcagcgatcgaggccttttccataggattctgcgctcatgcttttgtctcctttgcattgttgtggaatgtcgtgaatgcggcaaccggctcacgctccgtggcgagcgagttttcgatcgcggactcgtcgacgtagcccaagctcatgccgcagacaagcatctggtcggcgggaagttgcaggaactcggcgatctggcggtgaaacttcagaaaggcggcttgagggcaggtgtgaaggttccggcctcgcgcggcgaccatcacgctttgcaggaacatgccgtagtccagcaggcttccttcctggagctcgcggtctaccgtaaagaacaagcccacgggcgcatcgaagaaccggtagttgcgcccgtgttgcatgtgcatgcgctgcttgtcgcccttggcgatgccaagcaacccatagagatcccaacccaccttgcggcgccgctccaggtagggagaaaaccattcgcgcggatagtagtcgtagggctcaagcagttcccccgctcttccggggtcgtcgtcgagcgctgcaaccgcagcggacaggccggccttcacaggcccggtcaggacatgtacatgccaaggctgcatgttcatgccggaagcgctgtagcgcgcggtcgagagaatcgcttcgatctcttcttgtggcactggctcgggcaaatacgccctcacgctgcgtcgggtggcaattgcccaatcgaccgcactttgcagcatttctgcactgagcggtggcgccatcattcgattcattcctgggtcccttgcctcaaacaaactcgtggcgccgcgggtgcgacggcgagaggagattagttctgcaagggctcggcgcccatgcccggacgcctcgattcgagcggggcttttgggcatgcgagcgccctctttggtggaccccagaagtccggcgcctactcttgcgtggggggagaggagcgataggctcccgggctgacgcctgtccatttcttgaaggcgcgatggaaagcgcttgtttcctggaatccggttcgggcggcaacctcagccaccgtcaacgacgcgctcgacaacagatcgatggcgatgtcccgccgcagatcgtctttcacccgctggtagctcatgccctcttgttgcaagcggcgctggagcgtggtgccggaaacgcagagctcttgcgccagcttctccagctccggccacgcatcgggcatctggccgcgcaatcggttgcgtacctgcgcaccggtactcgcgtcgttgcggtacttgaccagcaaattggcaggtgctgcccgcagaaagttgtcgactgtctctggagattccgcgatcttcaaatccaacagatcgcttgcgaaggtgatgtgcgtggtcttgccgttgaatttgacgttctcgcagaatcgcgtgcggtagtggctgtcatcaccgggtggcgggcatcggaactgcatctcgcgcaggggaatgcgcctgtgcacgagccagcatgccaacccatgaacaagaatgaaccaggtgccatagccaaacagccggcgcagcacgccgccgtcatgcaggatcaggcaggcctcatccgccgagcgcaccagttccccacggaagtcgtccaatgtcgcgtggaggaacctgagggtccggcgcagcgcgtgctccaggttttcggcgctgaccgccgcgcgtgtcatgagtgcgtagctaccacggcgaagtccgtggctgtccaggccgaagaactcatcgtccatcaaatcggccaaagccacccacatgcgtgagtacgcagccgctgagatgcgagcacgcggcgcgttcagcagctcgcgatcgagcttcgcactttcaaggacactgctgatgtccatgttccggagcgccgcggcgtgaatcgcctcgtgcaccaactcaatggaaactgttcccttcaagcctgctgacttcatacgaactcgccaaagaatcgttgattgggacgagccctttatacgcgcgtattgcgtcgcacgagacagccacaggccgggacgtcgtatgcctagcgaggccctcaagcgcgaactggcagagcaccgctgatgcctggcgccgcggtgaaggcactgacgaggtcctgaggcgggtcgccgtttcccgaatctcgaacaagtcttgaacgaactccgtgcacgggagcccatcttttatcgtcgggaattcgggaccagtcgtggagatcttcttcgaatgacggctgacgacttctgggagatcggtgcgagtggcaggatttacgagcatgagttcgttatctctgaacttctggagcggtgagcccagccgagcgatgcactggcttgcatcgctcggcgatctgcctcagcacatcgatccccatctgcagggtgtgcaatgcgctgagaccgatcatccgttcatgccttggcgtgagcggtaggttgtcaatcagcgcgatgaattcgcgacgatgatgctggtcaagtacctcatggcgtgcaattgcgcgaaaagcagagggtgcaaagccagtgacggcagcgaggtggttcgcaaaaccggttgggggatgattgcattccattgcagcgatatggccaagcagcgagacggggtgatagtggtgcaaccagtagtactgcgcaccaaccatcgaagcgatcacgggcgaaggaatagcatgcatcacgtcttggtccgggtcgccggtggcggcaaggtcttcgcgcagccattcgtcatgacccttctcctccaacgcatggcttgcgtagtacccagccagccgttcgcacagcggatcggatgcgcgaagtcgggcctgtgcctctgctgcagtcaatagaggcaccgctgagcgaaccaccatgtgcatggtccgaaggtagatcggataggccactctggcacgctctggcatccacaagcagtgggcatagtgctgcattgttggcatggcttgggcgatcttgcgcagaaggcgctcactgggcttaccctgtgctgtgcaacggccgccatcctgcgcgggaatgaactcttctgcatgcatggctcatctccttctcgacgtttttggtgaccaggctttcaagtcgtgtgctctactggtccggggtccggcacaagccggtctatcagagtcatcaggcgatcgggctcgctgcggtcgggcatgcgctcgaagactttccagcagagttcgcaattgctgctgaagcgctcgcgggcaagcgccttgagcttggggtgctgtacgacgacacccaagcccgcggtaccaatcgcgtgcaaaagcgggtcggccgcaaaaccctccactgccgcgtcgatggcgctggcatcggagcaaggctgacgaagccgcttcggcccctgacccatgatcacaccctcattgcagcagccggtgaccacaccgtcgtagcgcagcatcggcgaacgcgcaagggcgcaggcgccgaaagattcaccccgagaccaggcaatccgcgcgaacatgccctggccacgaccgttgtcgagtggctgcaccaggttcagttcggcctgcgattgccaatcgtttcccagcgcgcgggccagcaaagatcgggctcgagcctcaccgtcaccgtacgcaacaacctgtacgaccagcgacgaacccgcacgcacgatcgttcttgcggcacgtacgaactgttcgtcaccgacgccggtggcgtggaaagcatcagtactcaaatagatgcaggcgcactcgcgcagaacctcctcgatccaaactggcacgacccttgtctgcgcccacacgccgctggtgaaaaccacgagctgcttgcccgcagcacgcaaccgctcggtcgccatgcgcagacctttgcgctcgacgaagggttcgccaccggaaattccgatgatctcgataccaatccgtgcgccgagccagtcgaggatctggtcgaacagtacaaaatcccggatcgtcggactgtcgggccgcgaatcgaccgaacagtggtcacagttcactgggcagcgatcggtgatgaacaacagcatggagcggctgcgttggtgacgcacagcctcgatctgcgcatgcgtgagcttgcggcgtggcgatggcttggtgatcgcggtcatcacgtggctccgagcagcgcgaggtcggcatagcgcgcaacgccgttgcggcgggcgaatgcgagggcaccaccttgtcgaatcagctcaccggctgccgcttcaagcactcgcgtagattgcttctgcatcgaaatcgcgatgctggcccgcacgcgttcctccaccagcgcgtcaccactcatcgccatgcaagtgcgacatcccgcggcacacccactcgggtgcatctcggcacgcgcggccaagtagtccgggccatagagtcggatcgcgcgcatcatgctcgactcgagcgtgcgctcgcgtatctgcgcccaggtatgcgtcgacgcatggccaagcaccaagtgcccaggcatccggtccatggcgtcatcgttgccgcaggccacgatgcggccatcgaaacccatcaccggccaggcagccatggtgcagggctgggcttcgacacgcgcagggcgcttcgtcatgaccatcggtgtccaagctcgcgcacggccaaagctcgcgacttggttcacgagcatcggtatgtgtatgccgaagtggcgtcggactgcggcgatacgcgtagtgaggtagggatcgtccgcatcgcggccaacgaggtggatgctcaagtccttgccatcatcgagcaatgtgcgcagaacgcgcctgacgttcggccagggcacctcagcctcgtgaaaggcatccaggctcgcggagaaatgatcaacggcgtcgatggcagcccgaatgggcgccggtatcttcgtaccgtcatgagcacgcgcgaaaaagaggccggagagcaccgagcttgtcgtcccgcagcgccgcgcactcttcgcgagcgcgcttaccagcgcgggacgcaacagcgcttcgccgcccgacatcgccaggatggctggacggctctcgtgcgaaaaactcgcgacgaagcgcttgaacagcagttcgggatgctgctcactggtcatcgaggattgcgtggaacagtgtgcgcaatgcagcgggcaccgacgagtcagccccatggagattccagcggctgggacgctgcgccagttcaggatttcagcgagatgcatcatgtactccttcttgcgttgcctgcaggtgatgacgcggcgtgcccaaggcgcaatgtgcggcgcgcggcgacggaagctgaaaacggggcggcggcttgaagtcgccgcccccagccctgcccgtgcggctcaggcgcaggcgacgcctaccagacgaagccgcccaccgtgtcggcagccttcttcagtgcgtcggtcaggccactgttgagcttggacttgatgtccgcaaggaccgcaagttcgtcgtcgtcgagcagagcgacctgcgacttcagttcgtcgttgagcgcctctacctggacggccgaattgcgcagtcgcaccgcccgagctgaagaaatcgccttgttttctgaaaccatgattgaactccgtcaagatgctccggcatgcggagcgtgggttgaatgaacatcgaactctcccgcccttgaagcagcgaatcacaggacgccggctgccatgcagactcaccatctcactggcaattgaaggctagctctcacctgcagcttgttcaatgaagcaatcggactatccctatgtgcacgaatgtatgaagcgacccgcgcgcgatgcctgactgggtgttgcgcgggtcgcgaacaaatgaagctttggaactacacccggcaagtgtcatgcgacgcgtgcagcacccacgaagaggcagcttcatgagcctgggacaagcctgcccgattcagtattgaatgagcgggcgcgaagcgcttgcgctcacctgccgaaggcgaacgtcttttgaatgttgtcgagaggaaagacgaagaaacgcgttgacgggcgatggcctcgcgaaggtgcccagttcaatgcgtgagtgctttggcactatcggcaagagaccctcgttttgattcgctccgccccacgttgcgtatcaaacgtcactacgcgccacatgacacctccccgtttgccataggtcagaggacgcatggggtctgcgcggacggctcatcgaagcagctcacggatccaggtggcgcacccggtcgcggcactcaagagatgcgactcgcaggaactcttgcaatccaacggcgaagaacgccttaaccctcaacgtaaaagtagcggtctgcgttctcgcagagatgcctgaccaagtggggaatacgctcccagtcgtccttgtagggattgtccaccgcgttgtactccgcctcgactcgatcgtggtcgagcggcgtcttggcgtactgctcgagcacgcgccgaagcgctacggcctcctcagacatgccgacttcagcatagctcgcagccgcgacatggaccagcgcctggcccgaattgcgcatacccgtcgtgaatccttcgcccgcccggctctgctcccagatgaagatcgagtacacgatcctgtagccaggtgggagttgatcgagcagttggtcggggtcgcggacgtccagttccgtcgccaactggtacatcccttcctccgggattccctcgctgtccgactgccagaagggagaaacatccgagtgagctgaactggaggcctcttcgaccatccccagaacgagcgctggaatgatgcgggtcatctatgcctttcttgattcgccgtaagcgttttggtcatgcgattctggcatcggccccacatagtgcccgcgcgggcggatgacttgcgccacgcccagttgctgaaggattcaaaacccgccgattgataatccttgccatgcccatcaacgagcttcggtccatcaccatcttcgcgaagatcgcggagctgggcagcctgcgcaaggccgcggaggcgcagaacatgacgccccaggcggccagccaggcgcttgcgcagctggagcagcacctgggcgtgcggctgttccatcggacgacgcgcagcgtggcgctgaccgacgccggccggcagcttctcgatgcctcgatgccggccgtggccacgctgcagcaggccctggcaatgacgcgaaggaccaccgaggagattgccgggcctttgcggatcgtggggccgcggtccgtgttcgcacgcgtcttctggcccctgctcgatgaattctgccgcctctatccggatgtgcagcccgacgtggagctggacgatcgcatcggcaactgggtcgaagaccgggtggacgtcggcttcaggatcggcgtttcccccgcggaaggggtcatcgcacgcaagctctttccgctgcagctgatcatctgcgcggctcctgcctacatcgcgcggcatggtgcgcccgactgtgtcgacgcgctggcttcgtacccgtgcagcgcatttcgcagtcccgccaccgggcgcgtaatcccttggcggatcaagaccgagaagcgcttcgaggagcaccagatcgagccctccctgtgcgtcaacgacgaagagctcgaaacgcaagccgtgctcgcggggcatgtgatgggacagctcacggccgtggccgcggcttcgcacatccgcgccggacgcctggtgccgctgctcacccagcatgtcgatgagcaggtgggcaccttcatctactacggcagcagggccgcgcagccggctcgcgcgcgggcgttcatcgaccttgccgtgaagcgcctcgcgggaaattccgagtgggtcctgacggccgaagaacttcgcgccgcggaagccaggggccgcaaggctgccggttgaagctggccgcacgcatgcggcccctgacgcttttcgccaatcgcccggagcggtgctgccattgccgcgatgccccgcaccgcctagattgcagggcacatgacctctttccctgaatccacggcgagcgcatccaagggtgcgccgctcgcaggcgtgcgcgtgctcgacctgacccgcctgctgccgggaccgcttggcaccatgcacctggccgacctcggcgccgacgtcgtcaagatcgaagacaccggcgccggcgactacgcgagcccctcggtgcgcgcgctcgtcaaccgcaacaagcgtgcgatccgcatcgacctgaagcacgcgcaaggcgtggccacgctgcttcgcctgtgccgcgatgccgacgtgctggtggagggcttccggcccggcgtgatgcagcggctcggcgtgggctacgaagcggtggcggcggtgaacccgcgcatcgtctactgcagcatcagcggcttcggccagaccggcccgctgtgcgacacgccggggcacgacctgaactacgcgtcgctcgctggcgtggccgaccagatcggcaatgccgcgggccctgccctgtcgaacctgcccgtggccgatctgctgggcggcaccatgaccgcggtggcaggcatcctggccgcgctgttcgatgccgcgcgcagcggacgcggacggcatgtcgacatcgccatggccgacggcgtgctggcccacgcggtgctgccgctggccggcctgcaccagcacggccaagtggcgcgcgtcggccagagcgcgctgacgggcgcccttgcctgctatggctactaccgcacggccgacgaccggcaggtggcggtcggcgcgctggagccgaagttctggcacgacctgtgccgcctgctcgagcgccctgacctcgccccgctgcaccgcagcggcgatgcagccaccgaggagcgtttgcgcaccgaactggcggccatcttcggcgcgcggccgctcgcgcactggcgcggcctgttccatgacggcgtgggctgcgtgacaccggtgctgcgcatcgacgagacactggaacatccgcatttccgcgcacgcggcatgcgcgttgcggccgatgatgcggcggcgccgcaactcggctgtcccatcaagatgaccggcttcgagcccgctgttccgcggcccgccccgcgcgccggcgagcacaccgacgagatcctgcgacaggccgggctcgacgcatcggccgtggccgaactgcgggcggccggcgccatcgattgaggcgctttctcccgcgggagcgctgcctacaatcccaacggccgagacgccgcggccgccaccgatgacgcacacccaccacaccgttgccatccagcaggtgcacagcatcctgatgggcgcgcgccatcgcggcatcgacgcggcgcgcgtgctggcgcgggccggcatcgcgccctcgctgctggagtcgccgctcgcgcgcatctcgcagcgccagtacgcattgctgatccgcgcgctgcggcgcgaactgcgcgacgaaatctggggcctgctgagccggccgctgccgcccggcagcttcggccagtgcatgcgccagctggtgcgctgcgccacgctcggcgaggccctgcgcgacggctttgccgcgtatcacctgctgctgcacgacttcgtgccgcgcctcaccgtgcagggcggcagcgcgcacgtgcagttcgtgctgcgccgcgcctccgatgcgcggctggactacgcggtgaaggccttcatgctgttcgccttcaacgcctcctcatggctggtggcgcgccgcattccgctgctcgaggtcgactacacggccgaacagaccaacaccgagacctcgcgtgtctaccaggtgccgatccgctacggccaggcgcacgtcggcatgtcgttcgaggcccgctggctcgatctgccggtggtgcagtcgccgcagagcctgcgcgaattcctcgccggatcgccggccaacctgatcgtgaagtaccgcgacaccagcagcctcaccgagcgcatccgccggctgctgcgcaagggcctgggcagcgagctgccatcgctcgaggaagtgggcgatgcgctcgccgtcacgccgcagacgctgcgccggcggctgcgcgacgaaggccgcggcttccagcagatcaaggacgagctgcggcgcgacgccgccgtcgaatacctgctgcacacgccgctgccgctgctcgacatcgccaaccgcgtgggcttctcggaagccagcaccttccaccgcgccttcaagcagtggaccggcgtggcgcccggcgagtaccggctcgcgcacgcctccgaacgctgagcggtttcgccaagccctttggcgcttcccgccatgggtgcggcgcgcggtgcgccataagctgtgccgcatcttcgttaccagccggcggcttccatcgtgtacctgacccaaggcctgcatcgcgcgctccagcgcaactccgacacggctgcgctcacccacgtcagcgacagcggcgtgcgccgccagacccatgcgcagctggccagcggcgtggcccgacaggcggccgcgctggcgcggcgcggcattgcgcgcggcgaccgcgtagcgctgctcgcacccaacagcgaccagctggtgcgggccatcctcgcgtgctggtggctgggcgccgtcgcctgccccctgaacatccgctggagcacgcccgaactcgcgcatgcgctgcaggacagcgcagcctcgctgctgctggtcgacgagaggttgcaggcgctcgcgccggccggcgagaccgcgctgctgcgcctggccgcgctggaagacgaaagcgccacgctggagcccttggccgacacgcgcaccggcggcgacgcgctggccgccatcctctataccggcggcaccaccggccgctccaagggcgtgatgctgagccacgcgaacttctggaccgcgtcgatgacgcgcggcgccgaactcaacaatgcgcccgattcggtgtcgctgctggtggcaccgctgttccacgtcgccgggctcggccgcctggtgggccagctgatcgtcggcggcagctgcgtgacgatggcgcagttccggcccgcggcggtgatcgaggccattgccgagcaccgcatcggcgacatcatcgtggtgccgagcatgctgcagtcattgctggacgatccctcgttcacgccggagcgggtgcgcagcctcacgcgcattgccttcggcgccgcgccgatgccgcccgacctgctcgaccgcgcgctggccgcctggccgcatgccgagttcttccaggcttacggcctcacggaaaccgcgggtgcggtgtgcatcaacatgccggccaaccaccggcccgagactcgcgcgctcggccggctgaacgccgtcggccgcgccggactcggcgccgagatcatcgtcgcggacgagagcggccgcgagctgccgcgcggcgaggtaggcgagatcctggcgcgcggtcccatggtgatgcagggctactggcgcaaccccgaggccacggccgctgcgctgcggggcggctggctgcgcaccggcgatgccggccgcatgctggacgacggctacctgttcatcgtcgaccgcctcaaggacatgatcatcagcggcggcgagaacgtctactgcgccgaagtggaggccgcgctgcgcagccatccgcaggtgcggcaggcagcagtcattggcgtgcccgatgcgcgctggggcgaggcggtgcacgcggcggtggtgcttgccgaaggcagcgccgccacggccgacgagctgcgtgcctggtgccgcgagcgtctggccggctacaagtgcccgcgcggcatcagcttcatgcacgagctgccgctgtcggccgcgggcaaggtgctgaagaacgtgctgcgcgagcgggtgcagacatgatgaaacccgtcacgggcgcggaccgccgcaacctgttcggccaggtgccgttcatgcgcctgctggacgcgcgccgcgagttctccgaaggcgggcgcgcgcggctcgttctcgacgagcgggccgagctcggcaacgtcatcggcgccgtgcatggcggcgtgctggtcacgctgctcgacgtggtcatggccagcgccgccgtgtcgctgttcgacttcgaacgcaccgccgtcacgctcaacctcaacaccagcttccacgagccgggccgcggccgcctcacggccgacggcgaagtggtgcagcacgacgccagcgtggcctggtgccgcgcctcggtcaccgatgcgggcggccgcgtggtcgcgcgtgcgcagggctccttccgctacctgccgctgccgcaggccgcctgacccgcaatttcaaacgacaggagacaacaccatgacgaagatgcatcgccgcgcggccctggccgcactggccgcctgcgcgctggccgcgccgctggcgcaggctgccgacccctacccgcacaagccgatccagctggtgctgccatttccgcccgggggctccttcgacccgatcttccgcacgctggccgaagccgcctccaaagacctgggccagcccatcgtgctgatgcacaggccgggcgcgggcggcgtcaccggcaccgcctcgctggcgaccatgaacgacgccgacggctacacgatctcggtcatgcacaactcggtgatccgcgcgccgctggtgcagaaggtgacctgggacccgctcaaggacttcacttacctgatcgggctggccggcctcaccaccggcatcgtcgtggccaccgacgcgccctggaagtcgctgcccgagctgctggccgacgccaagaagcgtcccggcgccgtcagctggggcaacgtcggtgcgatcagcatcaaccgcatctacgccgagcggcttgccaagcaggcaggcacctccttcaacctggtgccctacaaaggcggcagcgaggccttccaggcggtgatcggccgccatctcgacgtctacggcgaccccggcttcgggccccaggttcagggcggcaaggtgcgcctgctcgccaccttcaccgcggagcgcctgaagcgctacgacgcgccgaccgtgaaggagctgggccatgacatggtgatcgaatcaccggtgggcctggtggcgccgaagaacctcgacccgaagatcgccgccaggttgcacacggccttcagcaaggctgcgacggaccccgcctacctccagcagctggagctgttcgacatgcagcccaagctgatgagcggcgaaagctacgccgactacgcccgtgcccagttcgagcgcgagcgaaagatgctggccgagatcggcttcaagccggagtgacaggagcaatgaaccccatggacttttccgcattcgacttcaagggccgccacgtggccgtggccggtggctccagcggcatcaacttcggcatcgcgcaggccttcgcgcgcgccggtgcccgcctcacggtgctcagccgctcagccgacaaggtagcgacggccgcgcagcagctcgaggccctcggcacggaggcgctcggcatatcggccgacgtgcgccagcccgaggcgctggaacgcgcgttcgcagcgggcgccgagcgcttcggaccgatcgacgtgctggtttctggcgccgcgggcaactttctcgcgagcgcgctcgacatgtcgcccaacgccttcaagacggtggtcgacatcgacctgctgggcagcttcaacgtcgcccggctggcgcatgcgcacctgcgcaagcccggcgcctgcgtgatccagatctccgccgggcaggccttcacgcccacgcccttccaggcccacgtgtgcgcggccaaggccggcgtcgacatgctgacgcaagtgctggcgctggagtggggtccgcagggcatccgcatcaactccatcgtgccgggccccatcgccgacaccgagggcctgaagcggctcgcacccaccgacgacaccatggccgcgatggcgcagcgcgtgccgctcaagcgcctgggccgcatcgaggacatcagccggatggcgatgatgctggcgagcgactggggctcctacatcacgggcgccgtcattcccgtggacggcggcctcgcgctgaccgggccgcgcgacttcaccgcggcggctgccgcctcgaagcggggagccgcgccatgagcctgcaccttgcgagcgcgacgccggaaggcgacgaccggccgcgcagcggaccgcagcgctacgtgcccttctccgagcaccttggtctcaaggtcgagcgggccgaaggcggcgaatcgctggtgtcggtggcgttgcgccccgagctgctgaacaaccacgccaacggccatggcggcgtgctgatgaccctgctcgacagcgccatggcgcatgccgcgctctcgcgcgtcgactacgcgcgcgaggtcgtcaccgtcgacatgcacatcgccttcatgcggccggcaagcgggctgctgcaggccgaggggcgtgccaccggcggcggccgctcggtgtgcttttgcgaagccaccgtgaccgacgccagcggcgaagtggcggcgcgcgccatgggcaccttccgctaccgcgacccggcgtgagcgcgccgccaagggtgtgccaatgagcgtttcggccaatcgttttgggccgatccgcgattgttgatgccggcgcatcggccgagacttcattcatcgtcaccgcatcccatcaggagtttcaatgacacgtatgcagcgccccgtccatgtggtcggcgtgggcatgattcccttcaccaagcccggtgccagcgacccctacaccgtgatgggtgcgcgcgccgccaagctcgcgctcgacgatgccggcgtcgactattcgctggtgcagcaggcctatgtcggctatgtctatggagactccaccgccgggcaggccgccatctacggcgtcggcctcagcggcattccggtcttcaacctcaacaacaactgttccaccggctccagcgcgctgttcctcgcgcgccaggcagtcgaaagcggcatggtcgaatgcgcgattgcgctcggcttcgagcagatgcagcccggcgcgctcaagggcgcctacgacgaccggccctcgccgatggcgcgctttgccgacgtgatgtccgagaagcagggctacattcccgaagcaccgcgtgccgcgcagttcttcggcggcgccggccgcgactacatcgcgcagcacggcatccgccgcgacaccttcggccgcatctcggtgaaggcgcgccagcacgccgcgcgcaacccgctcgcggtgttccgccagacgctgacgctcgacgaggtcatggcctccccgctggtgttcgatccgctcacgcgctttcaatgctgcccgcccacctgcggcgcggctgcggccatcgtctgctcggccgagttcgcggagaaacacggcctcgacatgcgcgtggtgattgccgcgcaggccatgaccaccgacacgccctccaccttcgagagcaaggacatgcgcaagctggtcggctacgacatgaccgccgctgcggcccggcaggtgtacgaagacgccggcatcggccccgaggaactggacgtggtcgagctgcacgactgcttcaccgccaacgaactcatcacctacgaggcgctgggcctcacgcccgagggcacggccgagcgcttcatcgtcgagggcgacaacacctacggcggacgcgtggtgaccaacccttcgggcggcctcctgtccaagggccatccgctcggcgccaccgggctcgcgcagtgcgcggagctggtgtggcagctgcgcggccgcgcggagcagcgccaggtcgaaggcgcacgcctcgcgctgcagcacaacctgggcctgggcggcgcctgcgtggtcaccctctaccaagcggtttgacatgctagcccccacgcttgtcacttcgtgtactgcgctgccccccgaggggcctccagccgccttggggcggcccggcggtggctggtcatgatcgaccgccgccacatcggccacaccctgccgcccttccaggtggaagtggaaaaaggccgcctgcgcttcttcgccaaggccacgggccagaccgatcccatctacaccgacgaggccgccgcgcgcgatgcgggacatccgggcctgccggtgccgcccactttcttcttctgcctcgagatggaggcgccgaacccggccgccattcgcgagctgctgggcatggactaccgcagcctcctgcatggcgagcagggcttcagctactacaccatggcctacgccggcgacacgctgaccttccgccagcgcatcgaggacatctacgacaagaagaacggcgcgctcgagttcgtcgtgcgcaagacccgcgtcagtaaccagcagggcgaactggtggccgaactgcgctgcgtgacggtggtgcgcaatcaatgaatgaccggaacctcgcgatgacccacgccacccttcccgactggaacgcgctgcaacccggcgacgccctgcccccgctggaactgccgccgatcagccggctcgacctggcgctgtactgcggcgcctcgggcgaccacaacccgatccacgtcgacatcgactttgccaagtccgcaggcatgcccgacgtattcgcacacggcatgctgtcggcggcctggctcgcgcggttgttgaccaattgggtgccgcagcctgcgatccgttcgctcgacgttcgctttgccgccctcacccatgtgggcgagcgcatcagctgcaccggcacggtcgccgagaagttcgaccgcgagggccggcgcagcgtgctgctcaaggtcgcaagcgccaatgcgaacggcgttatcaaactgagcggcgaggcactcgtcgcctggctctgacacacccccgaggagacaacccatgaacagcagcaacaacaacagaaaactcgaaggcaaggtggccctcgtctccggctccggccgcggcatcgggcgcgagatcgcgctcaagctggcgagcgacggcgcgcgagtcgtcatcaacgacctcgacgccgaaccggccgcgcaaaccgtcaacgacatcgtggccgcgggcggcaacgccatcgcctgcgccggcagcgtgacggacagcggctttgccgaccgcttcgtgggcaccgccgtcgacagctacggcggcctggacatcatcgtcaacaacgccggctacacctgggacaacgtggtacagaagatgagcgacgagcagtgggaggccatgctggccgtgcacctaactgcgccgttccgcatcctgcgcgccgcctccagcttcatccgcgatgccgccaggcgcgaagccgacgaagggctcgaggtgttccgcaaggtggtcaacatatcgtcgacctccggcgtgtacggcaacgcggggcaggccaactatgcggccgccaaggccggcatcaacggcctgaccaaggccatggccaaggaatggggccgctacaaggtcacggtcaacagcgtcgccttcggcctcatcaagacccgactgaccgaagcggatgcgagcgcgggcgcgagcatcgacatcgagggccggcagatcaaggtcggcgtcaatccgcagatcctcaagaacgccgaagcgatgatcccgctcggccgcggcggcacgccgcaggaagcggcgggcgcggtctacatgttctgcattcccgaatcgaattacgtgagcggccaggtgctggtctgcggaggcggccgtccatgaccggcggggccgttgccacgcggccgtggatgaacgaagaactcgagatgctgcgtgacagcgcgcgccgcttcttcgagcgcgaatgcgtgccccatgaaccgcgctggcgcgcgcagcaccacgccgaccgcgacatctggacccaggccgggcgggccggactcctgtgcgccagcatccccgaggaatacggcggcggcggcggcagcttcctgcatgaggcggtgatctgcgaggagcagatgcgcgccatggcgcagagcttcagcaacaacgtgcacagcggcatcgtcgcgcactacctgctggcctacggcaccgaagcgcaaaagcggcgctggctgccgcgcatggccagcggcgaactggtggccgccatcgcgatgaccgagcccggcgccggcaccgacctgcagcgcatcaagacccaggcacggcgcgacggcgaccattggctcatcagcggcagcaagaccttcatcaccaacggcatgcatgccggcctggtctgcgtcgcggccaagaccgatgcggcggccggcggcaagggcatctcgctgctgatggtcgagaccgagggcgcggcgggctttcgccgcgggccgctgctcgacaagatgggccagaagacgctggacaccaccgagctgttcttcgacgacgtgcgcgtgccggccgacaacctgctgggcgaccaggagggctccggctttgcgcagctcatggcgcagctgccgcgcgagcgcatgctgatcgcggtcggcgcggtggcgaccatgcagcgggcgatcagcgacacgctcgagtacgtgcgcgaccgccaggtgttcggccaaccgctcttgaagatgcagaacacccgcttcaagctggccgaatgcgagacgcaggcgcaagtggcgcgcgccttcgtggacgactgcatcgcccgcctgatgcgcggcgagctcgacgttccgaccgccgccatggccaagtggtggaccaccgacacctgctgccgcatcgtcgacgaatgcctgcagctgcacggcggctacggcttcatgaacgaatatccgatcgcgcggctgtatgccgacgtgcgcgtcggccgcatctacggcggcgccaacgaggtgatgaaggaaatcatcgcgcgggccatggagaagcaatgatggtgagcgccgcacggccgcccgaaggcgcgaaggcccccctgagtgggggcactgttcccgaacgtccgcacttccgcttctggcccaagggcgtcgcgcgcgagttggtcgtgccgcaggcaacgctgccggagtacctcgaagttgcggcgcggcgctatccggacaaggccgcgatcgtctactgcggcagcgtcgtgcgctatgccgagctccagcagcgcgtggctgcgatgtcggcctggctgcgcgacacgctcgggctgcaacgcggcgaccgcgtgctggtggccagccagaactgcccgcagttcgtggtcgccagctacgcgatcctgcgcgcgggcggcgtcgtggtgcccgtcaatcccatgagcaaggcccaggaggttcggtactacgccgaggacagtggcgcgcgcatcgcgttcgtggcacaggagctgctggagcacttcgagccgggcctgtgcgaccgcatcgtggtgcacgcgtacagcgaggccgtgggcgatgcctccgatgaaatcccggattgggtgcgcgagccgctgcgtccgatctcgcggcccgactgcgcaggctgggccagcgtaccggccaccggcgatggtgccgacccgggcgtgcgccccacggaccttgcggtcctgccctacacctcgggcaccaccggccaccccaagggctgcatgcacacccaccagacggtgatcgcatccctggccgcctcgcacgtctggaagggcctgcattgcgagaccgtggtgctggccgtcgcgccgctgttccacatgctcggcctgcagaacggcatgaacatgccgatcttcctgggcggcacctcggtgatgctgccgcgctggaatccggccctggccgcgcggctgatcgagcgccaccgcgtcaccgcgtggacggccccgcccgcgatgatcctggacttcttcgcgaaccccgaggtggcgcagcgcgacatctccagcctgacgctgctctccggcggcgccgcggccatgccggaagcggtggcgaccatgatgcagcagcgctacggcatcacctacaacgaaggctacggcctgacggagaccgcctccttcctgcaggccaacccgcttgcacgcggcaagcgacagtgcctgggcattccggcgcagggcgtggacacccgcatcgtcgatccgctgacgctgaaggaacttccgcagggcgagctgggcgagctggtcacccacgcgccgcagaacaccgtcggctactggcgcaacccgcaggccgaccgcgatgctttcttcgagctggagggcaagcgcttcttccgtaccggcgacctcgcctacgtggacgaagagggctacttcttcatgcgcgaccgcctcaagcggatgatcaacagctcgggctacaaggtctggccggccgaggtggagaacatgctgtacgagcacccggcgatccacgaggcctgcatcatcggcgtgcccgacgccaggcagggcgaggcggtgaaggcgatcgtctcgctcaagcccgccttccgcggcgaggtgcaggcgcaagacatcgtcgattgggcacgcgagcgcatggcggtctacaaggcgccgcgtctcgtggaattcgtggatgccctgcccaagtcgggcaccggaaagattctttggcgcgagctgcaggaagcgcatcgcgccgctgcccaggagcaaactcgatgaacgatttctctgcgctgcgctacgagcgccacggcagcacggcgctgttgacgctcgacacgcccgccaaccgcaatgccttcacccccgccatgcgcgacgatcttgcagaggccatcgcgcaggtgcgaggcgatggcgatgtacgcgcattggtgctcgcaggcgccaacggccagttctgctcgggcggcgacctgcgcggcattgccgatgcgaagctcgacaacgccggctggcgcgcccgcatgcaggccacccagcgctggttcagcgaactgatcctgctcgacaagcccgtgatcgcggcggtcgatggcgccgcctatggcgcgggcttcagcctcgcgctcgcggccgacttcgtgctggcgagcccgcgcgcgcgtttctgcatgtccttcctgaagctgggcctggtgccggactgcggcgccttctacacgctgccgcgcgcggtgggcgcccagcgcgcacgcgagctgatgctgtcggcgcgcgaagtcggcgccgccgaggcgcacgaactcggcatcgcgatggagctgcacgcccccgagcaactgctgccgcgcgcgctggcgctggccgaaagctttgccggtgcctcgccactcgcggtgagcctggtgaagcgcgccaccggcgatgcgggcgcgctggccgcgctgctcgacaccgaggcgaacgtgcaggcactggccttcggcagtgccgagcaccgcgacgcggtgaaccgatttctggacaagaagccgctggccttccagtggccggcgaacaaggaaccaaaccaatgaccgacaccaccaccggcgtgcaggccttccaccaggccgagctggacgccggccgcttcctgctgcagcgctgcgccgactgcagccgccacgtctattacccgcgcgaaagctgcccccattgcggcggcgcagcgctcgaatggaaggcgcctgaggggctcggcaccgtgcatgcggtgacgaccgtgcggcgcaaaccggccgacggcggcgacctcaacgtcagcctggtcgagctcgacgaaggcgtgcggctcatgagccgcatcgagaatctcgcgcccggtgcggtgcgcatcggccagcgcgtcaaggcgcgggtgcaagtgaaggacggccgggggctggtgctgttcgacgccgtcgaaggagaaaccgcatgagcgccggactgaaagcattgcgcggcagcgcggccattgccggagccgccaccttcggctgcggcgagacgccgggcttcaccgacatggaactgctcgcacgcgccgcgcgcgcggccgtggccgatgcgggcctggagatgcgcgacatcgacggcctctgcaccgcgagcgcctcggccgcaatgtgggccctgcccgtggtcgaatacctgggcctcaacccgcgctacatcgacggcacgatgctgggcggcagcagcttcatcgcgcacctgctgcccgccatgcaggccatccgctcgggccagtgcagcgcggtgctcatctgctacggcagcgcacagcgcagcgcggccttcggccggcgcgagatcgtggcggcgcgccgctttctcgatccgcagccctacgagcatccttacgaaccgatgctgccggtgtcggcctacgcgctggcggcatcgcgccacatgcacgagttcggcaccacgcgcgagcagctcgccgacgtggcggtggcggcacgtgcatgggccgggctgaatccggaggccttcatgcgcgagccgcttacgcgcgaagaagtgctgggcgcccgcatggtgtcggacccgctgagcgtgcgcgactgctgccttgtcaccgacggcgccggtgcctgcgtgctggtgagcgcagagcgcgccagggacctgccgaagaagccggtctatgtgctgggcaacgccacggcggtgtggaaccggcagatctcgtcgatggcggacctcaccaccacggcggccagccagtcgggccgcgaggccttcgcaatggccgggctcgcccccagggacatggacgtggtgcagctgtacgacgccttcaccatcaacacgctgctgttcctggaagacctgggcttctgccccaagggcgaaggcggccgcttcgtggccgacggtgccattgcgccgggtggccgtctcgcggtcaacaccaacggcggcggcctgtcgtgcgtgcatcccggcatgtacggcatcttcgcgctgatcgaggccgtgcggcagctgcgcggcgaatgcggcgagcgccaggtgaagaacgcgcgcaccgccgtcgcgcatggcaacggcggcatgttgtcgagccaggccactgccgtgcttggcacagaggaggccctgtgaattgcatctactccctccccctctgggggagggcgggggtgggggctcgcggcgcacagagtgccgccaccccaatcctcccccgaaaggggaggaagaaagacaaggagactcccaaatgatccgcgacccgcaaaccctggaagccctgctcgacgccgtcaatcgcttcgtacgcgagcggctcgtgccggccgaagccctggtggccgagaccgacgagatccccgacgacatcgtgcgcgagatgaaggagctgggtctcttcggcctgaccgtgcccgaggaatacggcggcctgggcgtgacgatggaagaagaggtgatggtgatgctggccatgggccagacctcgccctgctttcgctcgctgttcggcaccaccgtgggcatcggctcgcagggcattctcttcgacggcaccgaggcgcagaagaagaagtacctgccgcgcctggcaaccggcgagctcatcgcctccttcgcgctgaccgagcccgacaccggctccgacgcggcgtcgctgcgcaccagcgcgatccgcgaaggcgaccactacatcgtcaacggcaccaagcgcttcatcaccaacgcgccgcatgcgggcatcttcacgctgatggcgcgcaccaaccccgaggacaagggcgcaggcggcgtttcggccttcatcgtggaggcggacacgccgggcatcacgatcggcaagaaggaccgcaagatgggccagcgcggcgcccacaccgccgacgtgatcttcgagaactgcagggtgccggcaagccagctgatcggcgggcgcgagggccagggcttcaagactgcgatgaaggtgctcgagaagggccgcatccacatcgccgccatctgcgtcggggtggccgagcgcatgcagcgcgatgcactccactacgcgatcgagcgcaagcagttcggccagccgattgccgagttccagctggtgcaagcgatgctggccgacagccaggccgagatctatgccgcacgctgcatggtgatcgacgcggcgcgccagcgcgacgaaggccgcaacgtggccaccgaggcttcgtgctgcaagctgttcgcctccgagatgtgcggccgcgtggcggaccgcgcggtgcagatcttcggcggcgccggctacgtctccgactacggcatcgaacggttctaccgcgacgtgcgcctgttccggctgtacgaaggcaccacgcagatccagcaaatcgtcattgcacgcaacctggtgcgcgaagcgatgcgctgagtttttccgatccacctgaggagacaacaccatgaagacatcgaagatgcgaagactctgcattgcagccggcctggccgcactgctggccgcgccggccctggcgcagacggcctatccggcacagccgctcaagctgatcgtgccctaccccgccggcggcgccaccgactcgctcgcgcgcaccatcgggcaaaagctgcaggaagcctggggacagccggccatggtggagaaccggcccggtgcgggcggcaccatcggcaacagcttcgtcgcgaaggcaccgcccgacggccacaccgtgctcattgccatcaccgcgctgatccagcaaccatcgctcatggagaagctgccctacgatccgctgaaggatctcgcgcccgtcaccatgatcgcgcgcagcccgagcatgctggccgtgccactggactcgcccgcaaaagacctgaagagcttcatcgcgatggtgaagcagagccccggcaagtacaacttcggcagctacggcgccgggacctcgtcgcacatccagggcgcgctgctgaacatgcaggccggcatcgacctggtgcacgtgcccttccagggcgccgcgccgctcgtgaccaacctcgtgggcggccagctcgcctcggccttcgtcgacagcgcgagtgcgcggccgcacctcaagtcgatgcggccactggccgtgaccggcacgcagcgcatgcccggcctgcccgacgtgcccacttttaccgagctgggctaccactcgttcgatccgtacggctggttcggtgtgttcctcccggccgccacgccggcaccggtggtgcagaagctctcggacgagatcaaccgcatcgtgcacctacccgaggtcagcgccaagatcgaggcgctggggttgcaggtggccggcggcaagcccgaagagttccagaaggtggtgcgctcggatgccgccgtctacgccaagatcatcaaggacgccaacatccgcgtggcgcagtgagcgcgacgggcgccctgaggcggcatgaagcagcgcgtgggcattgttcgccagggcgaactgggcgactacgtgatcgagcgcgccttcgtcgataaatagcgcgaagcattgcgcgagacgacggcgggtgtcgcgtccgacgttctatgactcgatagcaagggtcgaatctgcttcaagcggctcgcgaccgcctgatttcacccaggaccaggagcgccgcgcctgcagtgatggcgcaatcggccacgttgaagatggcgaagtcgtagacctcgcgccaataaagatggatgaagtcgaccacatgcccctgccacgagcggtcgatcgcatttcccagcgcgccgccgagcacaagtgccaaggccgctctgaacagcagcgttccgctgggctgcaccagcagtttgaggatgaacgcagccgccgctatggcaagcgccgtgaacagccatcgctgccagcccgaggcgtcggccaagaaggagaaggcaacgccccggttatgcgccaggacgagatcggcaaacgacgtgatggggaggacttcgcccccgcccaggaatcgtgtggcgagcgacttcgacgcctggtccagcagcacaacggcgaaggcaatgcccagacagggcgccagccgagcggctgcggcagatatgccttcgcggcgcctgtcggcagacacgaagatcgtcattgtggggtctcctgatgttgtcgggccggggcacctgggggtgcaaacacgcgtagtccaccccggtggttgatcgtcaccgccgccctggtcttctggaccacggccggcatggctgtgggcggttgcctgctatcagcgccgcaatgggtgccgatccaggctcagcacacgtgggtgctgacgggtttggccatcagcggctttctgggacagatggccatcgccgaagccttccgccacggccaggcggccgccatcgcccccttcgaatacagcgccctggcctgggcgcttgtgctggactgggcgttctggcaggccacgcccgatgcatggacgctgggtggcggtgcgctgatcgtcgcgagcgggctgtggctggcccgcatcgaggcgccaggggctgcgcggcaggagggacaggccgcctgagccgcagcgaagtgcgcgtgcgaggccacatgctgttgcggcaagttcgggcaaaaacttcgaagactgcacaacggcttggtcccaagctccggggacgggaatggccgtaagggtctcagttcggccaggaccggtcactcgctgctgccgcaagatatgtaggaagctgggcgaggaagctgccttcatcgaagggcccgaccccttaaagaaaatcgagcgtcaggctcgatccaaaatccacgcgcgaatctggtcatcgcacagggcttgggtatcggcctcggtgtgcttcgtttgcgccaccgacagcagtccgacctgccggacgtcgcgtgggtcgccggctccatctacatccggttcgccgtgagttctgtgagctgagcgcggttcgatgttctgagccagacctgcgcgccttgcattcgcgaatggaaatccgctcgcggggcttggcactgacgacattcaatgtcttcacgtcaattaagctggaaagattaataaagctgaaatcgacaccaatttcttatggaaataaatcacaagcatgaagaaaaaagcgtagacctcaaaattatttgaacaccagcaacgatcttttactagagtaacggctgaggcccggtggagattcacttgtaagcgcgtaagcggcagttgggtgaatatttaattcgtaatttgagctgtcttgagcttcttggcaggcgactttggacactggcacatcggtttgggattcgctaatttcggtattgataagaggcagagaccgttccgctggacggcttatatcaacggtgtcccgcaatcgggcatatataactttgggggttaatcatggcagtagacatgttcatgcgcgtcgagggcgcaaacggcgaatccaaggactcgaaccataaagactggacggatatcaagtcgtttgcatggggagcgacgcagcctggaaacatggtcagcggcggtggcggcggtgtgggcaaggcgagcttcaacgacctgcagattcttgcgcgcatcgacaaggcggccccgtccgtcatgaagaactgcgccagcggcaagcacctgagcaaggtcgaagtgtcggtgtgcaaggccgggggctcgcagatcgaatacacgcgcgtcacgctggaagaagtgctggtgacctcggtgcagtacacggccgagcagggcagcgatgcggtgctggtgcagttcgccttccaggccgccaaggtgaagcagcagtactgggagcagacggacaagggcggcaagggcgccgagaccgtgctggcctggaacatcaaggaaaacaaggaggcctgatcctcggacgtgcaggggccgattgtccagggcttcggcgcgcttggtttgtggctctgatcgagccgacgagggacccaagaaatgactcgcagtttcatcgtccacaccgagttgggcgagcgtctcaaattccgctccatgacggggcgggagcggatctccactctcttcgagtacagggtgcgcctcatcagcgatacgcctggcatctcggccaagagcctgctgggcaaggacatgagcatcgaggtgaacctggccaccgaattgggcggtgccgggaagcgctttctcagcgggcaggccacgcagttcacctacatcggcaaggatgacggcgacatgcacatctatgaagctgtgctgcaaccttggctctggtatgccacgcgtcgctccgatttcaagatattccagttcaagacggtgcccgagatacttcacgatgtgctcgggccctatggcttcgccatcgtggacaagttcagcggcagctaccgcagctgggactactgcgtccagtacgcggagacggacttcagcttcgcgagccgcctcatggaactggaaggcctctactacttcttcgaacacgcgcagggcagccacaagctggtgttgtgcgacggcatgggatcgcacattgccctgcccaacgggcccgagaagatcccctatcacgccggcgtgcttgcagcccaggtcctcgagcaggatttcatcgacacctggaaccatcgtgaagacatcgcctctggccatttcgcggcggacgactacgacttcaagaagcccaatgccaagatcgacacggtccggcagcagccggcgggtcatgaccgtgaccactatgaactctatgactggccgggtggctacaccgagatgggcgacggcgagaactacgcgcgcgtgcgcatcgagcagcaaaatgcgcgacgtgaattgattgccgggcacggcaacctgcgacatctcgcggcaggctacctcttcgatctgacgcgtcacccgaggccggaagaaaaccggcgctacctgatcgaggccgtgacttacgactttcaggaaaacgcgctgcgcaaggttggcgccgccgacgcggtctacgccgaaggcaccagcggcacgagctaccgccagaccttcgaagtcctgcctgacaacgccagctaccgcaccgcacggatggcgccgaagccgaggaccaccggtccgcagaccgcagtggtcgtggggcccgcgggcgaagagatctacaccgacgagtacggccggatcaaggtgcagttccactgggaccgctacggcaagatggacgagaactcttcctgctggatccgtgtctcgcagacgtgggctggcagcaactacggcaccatgcatgtgccgcgcatcggccaggaagtcatcgtcgattttctcaacggtgatccggactatcccatcgtcaccggacgggtctacaacgcggcacagatgccgccctggggcttgccggccaacaagacccagtcaggcatcctcacgcgctcctcccagggaggaacccccggcgacgggatgaaaaactcgcccggcacggccaacgcgttgcgcttcgaggacaaggccggtgaagagcaactgtggctgcatgcccagaaggaccagctcaccgaagtcgagaacgacgaggacaagtgggttggcaatgaccggcgcaagaccatcgaccgggacgagttcaacaccatccatcgtgatcgcaccgaggtcgtggaccgtaacgagaagatcaacgtgcatggctggcgcaccgaagaggtggacctggacgagaccatcaccatccatcagaaccgcaaggagcgggtggatctgaacgagacgatctccatcgggaagttcaagatgcagacggtggggataggctatacccagaacgtcggcatcttcaagatcatgtccatcggcgtggcctacatggagaacatcggcatcagcatgatgaccaatgtaggcaagacccagagcctcaacgtcggcgagaagcagaccattcaggtcggccaggtgcgcgaaaccgacatcggcaagaacgacacgctcagggtgggcgacaccctcaaggtccacggcaagaaggtcgcgatctccgcagacgatgaaatcacgctgagctgcggctccagcacgatcaggattacggcgggccagatcgagatcctgtcgccgctggacaagctcaactgctagcagttccggtgcgggcccctgacagcttcagacgataccttccgggagtgaaagccaaatgagcggcaaaccagcagcgcggatcacggacagcgtgtccggaagcaagatcgtcagcggctcgcgcacggtgctgatcggcagccagggcggcgttgcatgctcggaatgcccgggcggagtcacggtgggcaatccggtcagtccgtcgcagggcgccaaggtgttgatgggggagccggagctcgatttcgccttgcccggggcaatgccgctggtctggcagcgccagtacagcagctacgtgaacctggagcacggtgcgccgtgcagcctgctgggctatggctggagcctgcctgccgagatgcgcatcgaactgagggacgaggcctgcatcctgttcacagccatggggcgggccatcaccttcgacccgctgcccgaaggcggctcgatctacagcccgagcgaggacatctggctgctgcgcggcgggccggatgcaacttggggccaattggaacgctttcgccacatcccacgcaatctggccggcgacccgcaatgcatcatggccaccgatggagcggccggaacgttctgggtgctggggccgggagcaacgccttccgaacagacgcgggacccagcagccccccccggcatgccttacgcgctgcagtgcatgttcgatcggttcggccggcgccagcgctatgagcgcgacgcttggggccgggtcgtgggcatcgtcgacggcgtgggccgccgctaccggctgaacctgcggcagctgcacgccgcccgggccgcgcagggcctctggcaggccgacagcggctggcggctgacgggcgtcgacctcgtcagcgatccctgggcgccgggcgccagcgagccgatcgcgctcgtgcgctacggttactcggacacgggagaccttgtcaccgtgcacgaccgcgccggccggctcgtgcgcgaattcgcctggcaggcccacctgatgacggcgcaccgccacctgggcgggccgcgccacagctatcgctacgagagcctggcgcccggtgcgcgggtggtcgagcacgccaacgaggaggggttgacctatcggttcgaatacatgcagaccgatacgggcaaaacaacccaggtgaccgacagcctgcagcgtgtcgacgtctaccgcttcgaaggcgaggcgggcctgtcgcgcctggtggagcatgtgcgtgcggacggcagcatggtgcgctacgcctacgacgcggccggccgcatggtggaagccgtcgaccccctcgggcgaaccacccggctacgctacgacggcgagggccgattgctcggcagccaggatgcggatggcacacagagcagccaggatcatgaccccgccaccgggcacctgctggcaatcaccgacgccgtgggaggcatcacgcgccttgtctacgacgcctggggccgccggacacaaatcgtgctgcccgatggcagcatccagcgcgacgaatacgcggagccccaggacgcccccctgacttgcgaccttcccgtgcgccggatcgatgcgcgcggtggtgtcgtgcagctcgcgtggagcccggcaggccaactggtgggttacaccgactgttcaggccacaccagcgagacgcaatacgaccgctggggccagcgcatccagcggaccgatgccctggggcgcagcgttcgctacgaccacgacctagccggcaacctcaagaccgtgcatcgcgcggacggcagcacgatccggtattcccatgatgcggccggtcgcatcctgcaggtgctgccggtcgacaatgagccgggccacggcgttggcttcgcctacgacctctggggccgtgtcacgcggcgttggcaggacggatatggcgtgcaatacgactacgacatagccgggcgcctggtgcagttgaccaacgagaacggcgcccatgcgcacttcgcctgggatgcgatggacaggcaggtcagcgaagaaggcttcgacggccggctgcagacctaccgctacgacgccgccggccagctcatcgaggccacggacggcacggcctcgggcagcctgagtacccgctatgcctgggatgccatgagccggctggccgaaatccacgtgccggccacggagcacagtccggcgcgcgtcgagcggctgcaatggaacccggccggccaactgatcgctgcacgaagctacctgctcggtccggggcaactgcagcaactgcacactgaagccctgaccgagcgcgacgcgctgggacgcccgaccgccgaaacccaacgcctctacaagctcggcgagcctggcggcgctgcctctccaaccccgcccgatatcgagttcgagcacaccatctcccaccgactcgatgccctgggcaatcgccaggccagcgagctgcaggacctggggcaggtggactacctgatgtacggctccggccacctgcacgggctgctctacaacggccagggcttgctggacatcgaacgcgatgcactgcaccgcgaggtccggcggcaacagcgtcttcccatggaccaggtggtgcaaacccaccgcgaatggaatgttctgggccgcctgagcagtctgagcatcgtgggtgtggcgccagcggaccccgtgcccggcagcggctcgccctttcctctggtcgggcaactcacccgtcgtgcttaccgctatgacgtcttggggcagctcgaggcggttcaggccgccggcgacgcagagcgctaccgctacgacacgcgagggcgcctgattgccgcgcaatcggccagtcgccagcaacactggcactttgacccggcgggcaatcgcctgccttcgacggaggccgacctttcgccttcggggccgttcgggcgcaccgacaactggaaagcgctcgtgcgcggccaatggaaggaaaaaagcttcaatgtcctggaccagggcgaggttccgcagtccggcccagaggcgctgaatgcgcagccgcgctggcatgacaaccgcgttggccatggcgacgacacggcctacctctacgacagccggggcaaccgggtcgaagccgcagggccggacgaccggcggcttgtgctgcgctatgacggcgccaaccggctcgtcgaagcgcagacgcagggaagagcgagaaccatcgtcagccgctatgtctacgacacccgcggacggcggttgcgcaagatcgtgacggagcgggtccatggccagggagaagtcctgaaaggccgtacctaccatggctgggacggcgaccgcctggtgcacacggaacgtttgaagcccggcctggccaagcaagtcacgcacacggtgtacgagcccggtggcttcgcaccactggtccggttgagcatgcagggcaatgcaccgcccaccgggctggccgcgctcctggcacaagccgtgaacccgcagatgcagcagggcctgcgcgatgcggtgaacgacttgccgccgaacatgcgccagagcctcgaagaggaaatgcagacgttggcccggaacggcatgccggccgaggcccagcggatgcttgcgcagcaagccggcggcgacgcggcgatcgcctcggtgcgggaaacgatgcaggccgttcagccggttcaatccgtcgccgttcaccactttcactgcgaccacatgggcacgccccaggcgctcaccaacgaagccggacagctcgtgtggatggcccggtacgacccatggggcaacctgcaacaggaatacaacccgcacggcatcgagcagccaatccggttgccgggccagcaccacgacgcggaaacgggcctgcactacaaccggcaccgctactacgacccggtcatcgggtcgtacatcaaccaggaccccatcggattgaagggaggcatcaacggctttgcctatgcccgtcaggacccgctgcaggtgtcggatccgctgggcctgtatgccgatgccgctcatgccgacatgccgctcttcaatggccccggcgacacggcactgcccggcggcatcgacggcgacctgggccgcccggctcccagccagtcgaagaactgccccgattgcacgcaggtcgccggcaaggccggcgactacgtgatcctgtgctttaccgtgctgttcctgtcactcggcctcaaggtgccgccacgtccgccgccgcccccgccgaccatcagcgagcaggaaaaatcgctcaagggccgtggaggaaagaactgctcataaggccggaactcggcgcacgttgcgcacaggaaaacagcgtccgcgacgcttctaggggaggattcgaatga

SEQ ID NO: 6 - protein, 1374 aa, Variovorax sp.
MAQSSAYSYTERKRIRKSFGNRDSVVEIPYLLQMQKDAYTAFLQAGIPPKQRTVEGLQAAFDAAFPIVSHNGFVEMKFLEYNLAKPAFDVRECQTRGLTFASAVRAKVQLIIYDRESSTSQSKVVKEVKEQEVYMGEVPLMTEKGSFIINGTERVIVSQLHRSPGVFFEHDKGKTHSSGKLLFSARVIPYRGSWLDFEFDPKDMLYFRVDRRRKMPVTILLKAIGLNPESILANFFVNDNFRLMDSGAQMEFVPERLRGEVARFDITDKSGKVVVAKDKRVTARHTRELEQSATTHISVPEDFLVGRVIARNIVDADSGEILAKANDELTEALLKKLRTAGVQDIQVIYTNELDQGAYISQTLRIDETVDEFAARVAIYRMMRPGEPPTEDAVQALFQRLFYNPDTYDLSRVGRMKFNAKVGRDESTGPMVLTNEDILAVVKILVDLRNGNGEVDDIDHLGNRRVRCVGELAENQYRTGLARIEKAVKERLGQAEQEPLMPHDLINSKPISAALKEFFGASQLSQFMDQTNPLSEITHKRRVSALGPGGLTRERAGFEVRDVHVTHYGRVCPIETPEGPNIGLINSLALYARLNEYGFIETPYRRVADSKVTNEIDYLSAIEEGKYVIAQANAVLDKDGKLTGDLVSAREAGESILVGAERIQYMDVSPAQIVSVAASLVPFLEHDDANRALMGANMQRQAVPVLRPEKPMVGTGIERVSAVDSGTVVTATRGGIVDYVDATRIVVRVNDAEAAAGEVGVDIYNLIKYQRSNQNTNIHQRPIVKRGDKIAKGDVVADGASTDLGELALGQNMLIAFMPWNGYNFEDSILISERVVAEDRYTSIHIEELVVMARDTKLGAEEITRDIPNLAEQQLNRLDESGIIYVGAEVQPGDTLVGKVTPKGETTLTPEEKLLRAIFGEKASDVKDTSLRVDQGSQGTVIDVQVFTREGITRDKRAQQIIDDELKRFRLDLNDQLRIVEADAFDRIEKLLTGKVANGGPNKLAKGTKLDKAYLSSVEKFHWFDIRPADDEVATQLESIKNSLEQTRHSFDLAFEEKRKKLTQGDELPAGVLKMVKVYLAVKRRLQPGDKMAGRHGNKGVVSKIVPVEDMPHMADGTPCDICLNPLGVPSRMNVGQVLEVHLGWAGKGIGQRIGDLLQQEAKVAELRKFMEQLYNGSGRKEDLSKLSDTDLLEMAENLTSGATFATPVFDGASEEEIRGMLKLAYPDDIAKLKGLTDTRTQAYLYDGRTGDQFERPVTVGYMHFLKLHHLVDDKMHARSTGPYSLVTQQPLGGKAQFGGQRFGEMEVWALEAYGAAYVLQEMLTVKSDDVQGRTKVYESIVKGEHTIEAGMPESFNVLVKEIRSLGLDIELERS

SEQ ID NO: 7 - DNA, 36 bp, synthetic construct
  source 1..36: mol_type = other DNA; note = Forward primer for 16S rRNA gene; note (original language) = Cebador directo para el gen del ARNr 16S
gtaaaacgacggccagtgastttgatcctggctyag

SEQ ID NO: 8 - DNA, 39 bp, synthetic construct
  source 1..39: mol_type = other DNA; note = Reverse primer for 16S rRNA gene; note (original language) = Cebador reverso para el gen del ARNr 16S
ggaaacagctatgaccatgcggttaccttgttacgactt

SEQ ID NO: 9 - DNA, 20 bp, synthetic construct
  source 1..20: mol_type = other DNA; note = Forward primer 27F for 16S rRNA gene; note (original language) = Cebador directo 27F para el gen del ARNr 16S
agagtttgatcctggctcag

SEQ ID NO: 10 - DNA, 20 bp, synthetic construct
  source 1..20: mol_type = other DNA; note = Reverse primer 1522R for 16S rRNA gene; note (original language) = Cebador reverso 1522R para el gen del ARNr 16S
aaggaggtgatccanccrca

SEQ ID NO: 11 - DNA, 23 bp, synthetic construct
  source 1..23: mol_type = other DNA; note = Forward primer Univ_rpoB_F_deg for rpoB gene; note (original language) = Cebador directo Univ_rpoB_Fdeg para el gen rpoB
ggytwygaagtncghgacgtdca

SEQ ID NO: 12 - DNA, 25 bp, synthetic construct
  source 1..25: mol_type = other DNA; note = Reverse primer Univ_rpoB_R_deg for rpoB gene; note (original language) = Cebador reverso Univ_rpoB_R_deg para el gen rpoB
tgacgytgcatgttbgmrcccatma
